European Patent Application EP 4 635 975 A1 - sequence listing, part 3

SEQ ID NO: 219 - DNA, 4639646 bp, Escherichia coli (residues 1-2,319,823 of 4,639,646)
  source 1..4639646: mol_type = genomic DNA; note = MG1655 E.coli strain used
rrdatarragcttttcattctgactgcaacgggcaatatgtctctgtgtggattaaaaaaagagtgtctgatagcagcttctgaactggttacctgccgtgagtaaattaaaattttattgacttaggtcactaaatactttaaccaatataggcatagcgcacagacagataaaaattacagagtacacaacatccatgaaacgcattagcaccaccattaccaccaccatcaccattaccacaggtaacggtgcgggctgacgcgtacaggaaacacagaaaaaagcccgcacctgacagtgcgggctttttttttcgaccaaaggtaacgaggtaacaaccatgcgagtgttgaagttcggcggtacatcagtggcaaatgcagaacgttttctgcgtgttgccgatattctggaaagcaatgccaggcaggggcaggtggccaccgtcctctctgcccccgccaaaatcaccaaccacctggtggcgatgattgaaaaaaccattagcggccaggatgctttacccaatatcagcgatgccgaacgtatttttgccgaacttttgacgggactcgccgccgcccagccggggttcccgctggcgcaattgaaaactttcgtcgatcaggaatttgcccaaataaaacatgtcctgcatggcattagtttgttggggcagtgcccggatagcatcaacgctgcgctgatttgccgtggcgagaaaatgtcgatcgccattatggccggcgtattagaagcgcgcggtcacaacgttactgttatcgatccggtcgaaaaactgctggcagtggggcattacctcgaatctaccgtcgatattgctgagtccacccgccgtattgcggcaagccgcattccggctgatcacatggtgctgatggcaggtttcaccgccggtaatgaaaaaggcgaactggtggtgcttggacgcaacggttccgactactctgctgcggtgctggctgcctgtttacgcgccgattgttgcgagatttggacggacgttgacggggtctatacctgcgacccgcgtcaggtgcccgatgcgaggttgttgaagtcgatgtcctaccaggaagcgatggagctttcctacttcggcgctaaagttcttcacccccgcaccattacccccatcgcccagttccagatcccttgcctgattaaaaataccggaaatcctcaagcaccaggtacgctcattggtgccagccgtgatgaagacgaattaccggtcaagggcatttccaatctgaataacatggcaatgttcagcgtttctggtccggggatgaaagggatggtcggcatggcggcgcgcgtctttgcagcgatgtcacgcgcccgtatttccgtggtgctgattacgcaatcatcttccgaatacagcatcagtttctgcgttccacaaagcgactgtgtgcgagctgaacgggcaatgcaggaagagttctacctggaactgaaagaaggcttactggagccgctggcagtgacggaacggctggccattatctcggtggtaggtgatggtatgcgcaccttgcgtgggatctcggcgaaattctttgccgcactggcccgcgccaatatcaacattgtcgccattgctcagggatcttctgaacgctcaatctctgtcgtggtaaataacgatgatgcgaccactggcgtgcgcgttactcatcagatgctgttcaataccgatcaggttatcgaagtgtttgtgattggcgtcggtggcgttggcggtgcgctgctggagcaactgaagcgtcagcaaagctggctgaagaataaacatatcgacttacgtgtctgcggtgttgccaactcgaaggctctgctcaccaatgtacatggccttaatctggaaaactggcaggaagaactggcgcaagccaaagagccgtttaatctcgggcgcttaattcgcctcgtgaaagaatatcatctgctgaacccggtcattgttgactgcacttccagccaggcagtggcggatcaatatgccgacttcctgcgcgaaggtttccacgttgtcacgccgaacaaaaaggccaacacctcgtcgatggattactaccatcagttgcgttatgcggcggaaaaatcgcggcgtaaattcctctatgacaccaacgttggggctggattaccggttattgagaacctgcaaaatctgctcaatgcaggtgatgaattgatgaagttctccggcattctttctggttcgctttcttatatcttcggcaagttagacgaaggcatgagtttctccgaggcgaccacgctggcgcgggaaatgggttataccgaaccggacccgcgagatgatctttctggtatggatgtggcgcgtaaactattgattctcgctcgtgaaacgggacgtgaactggagctggcggatattgaaattgaacctgtgctgcccgcagagtttaacgccgagggtgatgttgccgcttttatggcgaatctgtcacaactcgacgatctctttgccgcgcgcgtggcgaaggcccgtgatgaaggaaaagttttgcgctatgttggcaatattgatgaagatggcgtctgccgcgtgaagattgccgaagtggatggtaatgatccgctgttcaaagtgaaaaatggcgaaaacgccctggccttctatagccactattatcagccgctgccgttggtactgcgcggatatggtgcgggcaatgacgttacagctgccggtgtctttgctgatctgctacgtaccctctcatggaagttaggagtctgacatggttaaagtttatgccccggcttccagtgccaatatgagcgtcgggtttgatgtgctcggggcggcggtgacacctgttgatggtgcattgctcggagatgtagtcacggttgaggcggcagagacattcagtctcaacaacctcggacgctttgccgataagctgccgtcagaaccacgggaaaatatcgtttatcagtgctgggagcgtttttgccaggaactgggtaagcaaattccagtggcgatgaccctggaaaagaatatgccgatcggttcgggcttaggctccagtgcctgttcggtggtcgcggcgctgatggcgatgaatgaacactgcggcaagccgcttaatgacactcgtttgctggctttgatgggcgagctggaaggccgtatctccggcagcattcattacgacaacgtggcaccgtgttttctcggtggtatgcagttgatgatcgaagaaaacgacatcatcagccagcaagtgccagggtttgatgagtggctgtgggtgctggcgtatccggggattaaagtctcgacggcagaagccagggctattttaccggcgcagtatcgccgccaggattgcattgcgcacgggcgacatctggcaggcttcattcacgcctgctattcccgtcagcctgagcttgccgcgaagctgatgaaagatgttatcgctgaaccctaccgtgaacggttactgccaggcttccggcaggcgcggcaggcggtcgcggaaatcggcgcggtagcgagcggtatctccggctccggcccgaccttgttcgctctgtgtgacaagccggaaaccgcccagcgcgttgccgactggttgggtaagaactacctgcaaaatcaggaaggttttgttcatatttgccggctggatacggcgggcgcacgagtactggaaaactaaatgaaactctacaatctgaaagatcacaacgagcaggtcagctttgcgcaagccgtaacccaggggttgggcaaaaatcaggggctgttttttccgcacgacctgccggaattcagcctgactgaaattgatgagatgctgaagctggattttgtcacccgcagtgcgaagatcctctcggcgtttattggtgatgaaatcccacaggaaatcctggaagagcgcgtgcgcgcggcgtttgccttcccggctccggtcgccaatgttgaaagcgatgtcggttgtctggaattgttccacgggccaacgctggcatttaaagatttcggcggtcgctttatggcacaaatgctgacccatattgcgggtgataagccagtgaccattctgaccgcgacctccggtgataccggagcggcagtggctcatgctttctacggtttaccgaatgtgaaagtggttatcctctatccacgaggcaaaatcagtccactgcaagaaaaactgttctgtacattgggcggcaatatcgaaactgttgccatcgacggcgatttcgatgcctgtcaggcgctggtgaagcaggcgtttgatgatgaagaactgaaagtggcgctagggttaaactcggctaactcgattaacatcagccgtttgctggcgcagatttgctactactttgaagctgttgcgcagctgccgcaggagacgcgcaaccagctggttgtctcggtgccaagcggaaacttcggcgatttgacggcgggtctgctggcgaagtcactcggtctgccggtgaaacgttttattgctgcgaccaacgtgaacgataccgtgccacgtttcctgcacgacggtcagtggtcacccaaagcgactcaggcgacgttatccaacgcgatggacgtgagtcagccgaacaactggccgcgtgtggaagagttgttccgccgcaaaatctggcaactgaaagagctgggttatgcagccgtggatgatgaaaccacgcaacagacaatgcgtgagttaaaagaactgggctacacttcggagccgcacgctgccgtagcttatcgtgcgctgcgtgatcagttgaatccaggcgaatatggcttgttcctcggcaccgcgcatccggcgaaatttaaagagagcgtggaagcgattctcggtgaaacgttggatctgccaaaagagctggcagaacgtgctgatttacccttgctttcacataatctgcccgccgattttgctgcgttgcgtaaattgatgatgaatcatcagtaaaatctattcattatctcaatcaggccgggtttgcttttatgcagcccggcttttttatgaagaaattatggagaaaaatgacagggaaaaaggagaaattctcaataaatgcggtaacttagagattaggattgcggagaataacaaccgccgttctcatcgagtaatctccggatatcgacccataacgggcaatgataaaaggagtaacctgtgaaaaagatgcaatctatcgtactcgcactttccctggttctggtcgctcccatggcagcacaggctgcggaaattacgttagtcccgtcagtaaaattacagataggcgatcgtgataatcgtggctattactgggatggaggtcactggcgcgaccacggctggtggaaacaacattatgaatggcgaggcaatcgctggcacctacacggaccgccgccaccgccgcgccaccataagaaagctcctcatgatcatcacggcggtcatggtccaggcaaacatcaccgctaaatgacaaatgccgggtaacaatccggcattcagcgcctgatgcgacgctggcgcgtcttatcaggcctacgttaattctgcaatatattgaatctgcatgcttttgtaggcaggataaggcgttcacgccgcatccggcattgactgcaaacttaacgctgctcgtagcgtttaaacaccagttcgccattgctggaggaatcttcatcaaagaagtaaccttcgctattaaaaccagtcagttgctctggtttggtcagccgattttcaataatgaaacgactcatcagaccgcgtgctttcttagcgtagaagctgatgatcttaaatttgccgttcttctcatcgaggaacaccggcttgataatctcggcattcaatttcttcggcttcaccgatttaaaatactcatctgacgccagattaatcaccacattatcgccttgtgctgcgagcgcctcgttcagcttgttggtgatgatatctccccagaattgatacagatctttccctcgggcattctcaagacggatccccatttccagacgataaggctgcattaaatcgagcgggcggagtacgccatacaagccggaaagcattcgcaaatgctgttgggcaaaatcgaaatcgtcttcgctgaaggtttcggcctgcaagccggtgtagacatcacctttaaacgccagaatcgcctggcgggcattcgccggcgtgaaatctggctgccagtcatgaaagcgagcggcgttgatacccgccagtttgtcgctgatgcgcatcagcgtgctaatctgcggaggcgtcagtttccgcgcctcatggatcaactgctgggaattgtctaacagctccggcagcgtatagcgcgtggtggtcaacgggctttggtaatcaagcgttttcgcaggtgaaataagaatcagcatatccagtccttgcaggaaatttatgccgactttagcaaaaaatgagaatgagttgatcgatagttgtgattactcctgcgaaacatcatcccacgcgtccggagaaagctggcgaccgatatccggataacgcaatggatcaaacaccgggcgcacgccgagtttacgctggcgtagataatcactggcaatggtatgaaccacaggcgagagcagtaaaatggcggtcaaattggtaatagccatgcaggccattatgatatctgccagttgccacatcagcggaaggcttagcaaggtgccgccgatgaccgttgcgaaggtgcagatccgcaaacaccagatcgctttagggttgttcaggcgtaaaaagaagagattgttttcggcataaatgtagttggcaacgatggagctgaaggcaaacagaataaccacaagggtaacaaactcagcaccccaggaacccattagcacccgcatcgccttctggataagctgaataccttccagcggcatgtaggttgtgccgttacccgccagtaatatcagcatggcgcttgccgtacagatgaccagggtgtcgataaaaatgccaatcatctggacaatcccttgcgctgccggatgcggaggccaggacgccgctgccgctgccgcgtttggcgtcgaacccattcccgcctcattggaaaacatactgcgctgaaaaccgttagtaatcgcctggcttaaggtatatcccgccgcgccgcctgccgcttcctgccagccaaaagcactctcaaaaatagaccaaatgacgtggggaagttgcccgatattcattacgcaaattaccaggctggtcagtacccagattatcgccatcaacgggacaaagccctgcatgagccgggcgacgccatgaagaccgcgagtgattgccagcagagtaaagacagcgagaataatgcctgtcaccagcgggggaaaatcaaaagaaaaactcagggcgcgggcaacggcgttcgcttgaactccgctgaaaattatgccataggcgatgagcaaaaagacggcgaacagaacgcccatccagcgcatccccagcccgcgcgccatataccatgccggtccgccacgaaactgcccattgacgtcacgttctttataaagttgtgccagagaacattcggcaaacgaggtcgccatgccgataaacgcggcaacccacatccaaaagacggctccaggtccaccggcggtaatagccagcgcaacgccggccaggttgccgctacccacgcgcgccgcaagactggtacacaatgactgaaatgaggttaaaccgcctggctgtggatgaatgctatttttaagacttttgccaaactggcggatgtagcgaaactgcacaaatccggtgcgaaaagtgaaccaacaacctgcgccgaagagcaggtaaatcattaccgatccccaaaggacgctgttaatgaaggagaaaaaatctggcatgcatatccctcttattgccggtcgcgatgactttcctgtgtaaacgttaccaattgtttaagaagtatatacgctacgaggtacttgataacttctgcgtagcatacatgaggttttgtataaaaatggcgggcgatatcaacgcagtgtcagaaatccgaaacagtctcgcctggcgataaccgtcttgtcggcggttgcgctgacgttgcgtcgtgatatcatcagggcagaccggttacatccccctaacaagctgtttaaagagaaatactatcatgacggacaaattgacctcccttcgtcagtacaccaccgtagtggccgacactggggacatcgcggcaatgaagctgtatcaaccgcaggatgccacaaccaacccttctctcattcttaacgcagcgcagattccggaataccgtaagttgattgatgatgctgtcgcctgggcgaaacagcagagcaacgatcgcgcgcagcagatcgtggacgcgaccgacaaactggcagtaaatattggtctggaaatcctgaaactggttccgggccgtatctcaactgaagttgatgcgcgtctttcctatgacaccgaagcgtcaattgcgaaagcaaaacgcctgatcaaactctacaacgatgctggtattagcaacgatcgtattctgatcaaactggcttctacctggcagggtatccgtgctgcagaacagctggaaaaagaaggcatcaactgtaacctgaccctgctgttctccttcgctcaggctcgtgcttgtgcggaagcgggcgtgttcctgatctcgccgtttgttggccgtattcttgactggtacaaagcgaataccgataagaaagagtacgctccggcagaagatccgggcgtggtttctgtatctgaaatctaccagtactacaaagagcacggttatgaaaccgtggttatgggcgcaagcttccgtaacatcggcgaaattctggaactggcaggctgcgaccgtctgaccatcgcaccggcactgctgaaagagctggcggagagcgaaggggctatcgaacgtaaactgtcttacaccggcgaagtgaaagcgcgtccggcgcgtatcactgagtccgagttcctgtggcagcacaaccaggatccaatggcagtagataaactggcggaaggtatccgtaagtttgctattgaccaggaaaaactggaaaaaatgatcggcgatctgctgtaatcattcttagcgtgaccgggaagtcggtcacgctacctcttctgaagcctgtctgtcactcccttcgcagtgtatcattctgtttaacgagactgtttaaacggaaaaatcttgatgaatactttacgtattggcttagtttccatctctgatcgcgcatccagcggcgtttatcaggataaaggcatccctgcgctggaagaatggctgacatcggcgctaaccacgccgtttgaactggaaacccgcttaatccccgatgagcaggcgatcatcgagcaaacgttgtgtgagctggtggatgaaatgagttgccatctggtgctcaccacgggcggaactggcccggcgcgtcgtgacgtaacgcccgatgcgacgctggcagtagcggaccgcgagatgcctggctttggtgaacagatgcgccagatcagcctgcattttgtaccaactgcgatcctttcgcgtcaggtgggcgtgattcgcaaacaggcgctgatccttaacttacccggtcagccgaagtctattaaagagacgctggaaggtgtgaaggacgctgagggtaacgttgtggtacacggtatttttgccagcgtaccgtactgcattcagttgctggaagggccatacgttgaaacggcaccggaagtggttgcagcattcagaccgaagagtgcaagacgcgacgttagcgaataaaaaaatccccccgagcggggggatctcaaaacaattagtgggattcaccaatcggcagaacggtgcgaccaaactgctcgttcagtacttcacccatcgccagatagattgcgctggcaccgcagatcagcccaatccagccggcaaagtggatgattgcggcgttaccggcaatgttaccgatcgccagcagggcaaacagcacggtcaggctaaagaaaacgaattgcagaacgcgtgcgcctttcagcgtgccgaagaacataaacagcgtaaatacgccccacagacccaggtagacaccaaggaactgtgcatttggcgcatcggtcagacccagtttcggcatcagcagaatcgcaaccagcgtcagccagaaagaaccgtaagaggtgaatgcggttaaaccgaaagtgttgccttttttgtactccagcagaccagcaaaaatttgcgcgatgccgccgtagaaaatgcccatggcaagaataataccgtccagagcgaaataacccacgttgtgcaggttaagcagaatggtggtcatgccgaagcccatcaggcccagcggtgccggattagccaacttagtgttgcccataattcctcaaaaatcatcatcgaatgaatggtgaaataatttccctgaataactgtagtgttttcagggcgcggcataataatcagccagtggggcagtgtctacgatcttttgaggggaaaatgaaaattttccccggtttccggtatcagacctgagtggcgctaaccatccggcgcaggcaggcgatttgcagtacggctggaatcgtcacgcgataggcgctgccgctgaccgctttaaccccatttagtgccgcacctacagggcctcccagccccgcgccgcgcagcaaaccatgcccaagtacgctcattgctgcgtgggtgcgtaaaatgcgggtcagttggctggaaagcaaatgcgacacaccttttgccaataatttgtctttcatcagcagcggcagcagctcttccagctcattcaccctggcatcgaccgcgtgcagaaactcctgcttatgttcctcgtccattttcttccaggtattacgcagaaattgttccagtaactgttgctcaatttcaaacgtagacatctctttgtcggctttcagcttcaatcgctttgaaacatcgagcaaaatggcccgatacaatttaccgtgtccgcgcagtttgttggcgatactatcgccaccaaaatgctgtaattctccggcaatcagctgccagttgcggcgatgttgctcgggatgcccttccatcgatttaaacagttcgttgcgcatcagtacgctggagaggcgagttttgcctttttcattatgggtgagcaatcgggcgaaatttgccaactgttcctcactacaatgctgaagaaaatccagatctgaatcattcaggtaattaacattcattttttgtggcttctatattctggcgttagtcgtcgccgataattttcagcgtggccatatccgatgagttcaccgtatgacccgaaaaggtgatttttgagacgcagcgtttattgtcgttatcgctgttaatgttgatccagtcagtggtttgcccttcttttatttctgaaggaatattcaggctctgactggcgctacgggcggctttgaaataaaccgatgcaccgcttaactgtaaatcgccatggtcggcagagagttgtatgcgtttcacaatgcgacaaacaggaagtttcagcgccagatcgttggtttcgttacgcggcattgcaatggcgccgaggagtttatggtcgtttgcctgcgccgtgcagcacagcatcaggctaatcgccaggctggcggaaatcgtaaaaacggatttcataaggattctcttagtgggaagaggtagggggatgaatacccactagtttactgctgataaagagaagattcaggcacgtaatcttttctttttattacaattttttgatgaatgccttggctgcgattcattctttatatgaataaaattgctgtcaattttacgtcttgtcctgccatatcgcgaaatttctgcgcaaaagcacaaaaaatttttgcatctcccccttgatgacgtggtttacgaccccatttagtagtcaaccgcagtgagtgagtctgcaaaaaaatgaaattgggcagttgaaaccagacgtttcgcccctattacagactcacaaccacatgatgaccgaatatatagtggagacgtttagatgggtaaaataattggtatcgacctgggtactaccaactcttgtgtagcgattatggatggcaccactcctcgcgtgctggagaacgccgaaggcgatcgcaccacgccttctatcattgcctatacccaggatggtgaaactctagttggtcagccggctaaacgtcaggcagtgacgaacccgcaaaacactctgtttgcgattaaacgcctgattggtcgccgcttccaggacgaagaagtacagcgtgatgtttccatcatgccgttcaaaattattgctgctgataacggcgacgcatgggtcgaagttaaaggccagaaaatggcaccgccgcagatttctgctgaagtgctgaaaaaaatgaagaaaaccgctgaagattacctgggtgaaccggtaactgaagctgttatcaccgtaccggcatactttaacgatgctcagcgtcaggcaaccaaagacgcaggccgtatcgctggtctggaagtaaaacgtatcatcaacgaaccgaccgcagctgcgctggcttacggtctggacaaaggcactggcaaccgtactatcgcggtttatgacctgggtggtggtactttcgatatttctattatcgaaatcgacgaagttgacggcgaaaaaaccttcgaagttctggcaaccaacggtgatacccacctggggggtgaagacttcgacagccgtctgatcaactatctggttgaagaattcaagaaagatcagggcattgacctgcgcaacgatccgctggcaatgcagcgcctgaaagaagcggcagaaaaagcgaaaatcgaactgtcttccgctcagcagaccgacgttaacctgccatacatcactgcagacgcgaccggtccgaaacacatgaacatcaaagtgactcgtgcgaaactggaaagcctggttgaagatctggtaaaccgttccattgagccgctgaaagttgcactgcaggacgctggcctgtccgtatctgatatcgacgacgttatcctcgttggtggtcagactcgtatgccaatggttcagaagaaagttgctgagttctttggtaaagagccgcgtaaagacgttaacccggacgaagctgtagcaatcggtgctgctgttcagggtggtgttctgactggtgacgtaaaagacgtactgctgctggacgttaccccgctgtctctgggtatcgaaaccatgggcggtgtgatgacgacgctgatcgcgaaaaacaccactatcccgaccaagcacagccaggtgttctctaccgctgaagacaaccagtctgcggtaaccatccatgtgctgcagggtgaacgtaaacgtgcggctgataacaaatctctgggtcagttcaacctagatggtatcaacccggcaccgcgcggcatgccgcagatcgaagttaccttcgatatcgatgctgacggtatcctgcacgtttccgcgaaagataaaaacagcggtaaagagcagaagatcaccatcaaggcttcttctggtctgaacgaagatgaaatccagaaaatggtacgcgacgcagaagctaacgccgaagctgaccgtaagtttgaagagctggtacagactcgcaaccagggcgaccatctgctgcacagcacccgtaagcaggttgaagaagcaggcgacaaactgccggctgacgacaaaactgctatcgagtctgcgctgactgcactggaaactgctctgaaaggtgaagacaaagccgctatcgaagcgaaaatgcaggaactggcacaggtttcccagaaactgatggaaatcgcccagcagcaacatgcccagcagcagactgccggtgctgatgcttctgcaaacaacgcgaaagatgacgatgttgtcgacgctgaatttgaagaagtcaaagacaaaaaataatcgccctataaacgggtaattatactgacacgggcgaaggggaatttcctctccgcccgtgcattcatctaggggcaatttaaaaaagatggctaagcaagattattacgagattttaggcgtttccaaaacagcggaagagcgtgaaatcagaaaggcctacaaacgcctggccatgaaataccacccggaccgtaaccagggtgacaaagaggccgaggcgaaatttaaagagatcaaggaagcttatgaagttctgaccgactcgcaaaaacgtgcggcatacgatcagtatggtcatgctgcgtttgagcaaggtggcatgggcggcggcggttttggcggcggcgcagacttcagcgatatttttggtgacgttttcggcgatatttttggcggcggacgtggtcgtcaacgtgcggcgcgcggtgctgatttacgctataacatggagctcaccctcgaagaagctgtacgtggcgtgaccaaagagatccgcattccgactctggaagagtgtgacgtttgccacggtagcggtgcaaaaccaggtacacagccgcagacttgtccgacctgtcatggttctggtcaggtgcagatgcgccagggattcttcgctgtacagcagacctgtccacactgtcagggccgcggtacgctgatcaaagatccgtgcaacaaatgtcatggtcatggtcgtgttgagcgcagcaaaacgctgtccgttaaaatcccggcaggggtggacactggagaccgcatccgtcttgcgggcgaaggtgaagcgggcgagcatggcgcaccggcaggcgatctgtacgttcaggttcaggttaaacagcacccgattttcgagcgtgaaggcaacaacctgtattgcgaagtcccgatcaacttcgctatggcggcgctgggtggcgaaatcgaagtaccgacccttgatggtcgcgtcaaactgaaagtgcctggcgaaacccagaccggtaagctattccgtatgcgcggtaaaggcgtcaagtctgtccgcggtggcgcacagggtgatttgctgtgccgcgttgtcgtcgaaacaccggtaggcctgaacgaaaggcagaaacagctgctgcaagagctgcaagaaagcttcggtggcccaaccggcgagcacaacagcccgcgctcaaagagcttctttgatggtgtgaagaagttttttgacgacctgacccgctaacctccccaaaagcctgcccgtgggcaggcctgggtaaaaatagggtgcgttgaagatatgcgagcacctgtaaagtggcggggatcactcccataagcgctaacttaagggttgtggtattacgcctgatatgatttaacgtgccgatgaattactctcacgataactggtcagcaattctggcccatattggtaagcccgaagaactggatacttcggcacgtaatgccggggctctaacccgccgccgcgaaattcgtgatgctgcaactctgctacgtctggggctggcttacggccccggggggatgtcattacgtgaagtcactgcatgggctcagctccatgacgttgcaacattatctgacgtggctctcctgaagcggctgcggaatgccgccgactggtttggcatacttgccgcacaaacacttgctgtacgcgccgcagttacgggttgtacaagcggaaagagattgcgtcttgtcgatggaacagcaatcagtgcgcccgggggcggcagcgctgaatggcgactacatatgggatatgatcctcatacctgtcagttcactgattttgagctaaccgacagcagagacgctgaacggctggaccgatttgcgcaaacggcagacgagatacgcattgctgaccggggattcggttcgcgtcccgaatgtatccgctcacttgcttttggagaagctgattatatcgtccgggttcactggcgaggattgcgctggttaactgcagaaggaatgcgctttgacatgatgggttttctgcgcgggctggattgcggtaagaacggtgaaaccactgtaatgataggcaattcaggtaataaaaaagccggagctccctttccggcacgtctcattgccgtatcacttcctcccgaaaaagcattaatcagtaaaacccgactgctcagcgagaatcgtcgaaaaggacgagtagttcaggcggaaacgctggaagcagcgggccatgtgctattgctaacatcattaccggaagatgaatattcagcagagcaagtggctgattgttaccgtctgcgatggcaaattgaactggcttttaagcggctcaaaagtttgctgcacctggatgctttgcgtgcaaaggaacctgaactcgcgaaagcgtggatatttgctaatctactcgccgcatttttaattgacgacataatccagccatcgctggatttcccccccagaagtgccggatccgaaaagaagaactaactcgttgtggagaataacaaaaatggtcatctggagcttacaggtggccattcgtgggacagtatccctgacagcctacaaaacgcaattgaagaacgcgaggcatcgtcttaacgaggcaccgaggcgtcgcattcttcagatggttcaacccttaagttagcgcttatgggatcactccccgccgttgctcttactcggattcgtaagccgtgaaaacagcaacctccgtctggccagttcggatgtgaacctcacagaggtcttttctcgttaccagcgccgccactacggcggtgatacagatgacgatcagggcgacaatcatcgccttatgctgcttcattgctctcttctccttgaccttacggtcagtaagaggcactctacatgtgttcagcatataggaggcctcgggttgatggtaaaatatcactcggggcttttctctatctgccgttcagctaatgcctgagacagacagcctcaagcacccgccgctattatatcgctctctttaacccattttgttttatcgattctaatcctgaagacgcctcgcatttttgtggcgtaattttttaatgatttaattatttaactttaatttatctcttcatcgcaattattgacgacaagctggattatttttgaaatattggcctaacaagcatcgccgactgacaacaaattaattattacttttcctaattaatccctcaggaatcctcaccttaagctatgattatctaggcttagggtcactcgtgagcgcttacagccgtcaaaaacgcatctcaccgctgatggcgcaaattcttcaatagctcgtaaaaaacgaattattcctacactataatctgattttaacgatgattcgtgcggggtaaaatagtaaaaacgatctattcacctgaaagagaaataaaaagtgaaacatctgcatcgattctttagcagtgatgcctcgggaggcattattcttatcattgccgctatcctggcgatgattatggccaacagcggcgcaaccagtggatggtatcacgactttctggagacgccggttcagctccgggttggttcactcgaaatcaacaaaaacatgctgttatggataaatgacgcgctgatggcggtatttttcctgttagtcggtctggaagttaaacgtgaactgatgcaaggatcgctagccagcttacgccaggccgcatttccagttatcgccgctattggtgggatgattgtgccggcattactctatctggcttttaactatgccgatccgattacccgcgaagggtgggcgatcccggcggctactgacattgcttttgcacttggtgtactggcgctgttgggaagtcgtgttccgttagcgctgaagatctttttgatggctctggctattatcgacgatcttggggccatcattatcatcgcattgttctacactaatgacttatcgatggcctctcttggcgtcgcggctgtagcaattgcggtactcgcggtattgaatctgtgtggtgcacgccgcacgggcgtctatattcttgttggcgtggtgttgtggactgcggtgttgaaatcgggggttcacgcaactctggcgggggtaattgtcggcttctttattcctttgaaagagaagcatgggcgttctccagcgaagcgactggagcatgtgttgcacccgtgggtggcgtatctgattttgccgctgtttgcatttgctaatgctggcgtttcactgcaaggcgtcacgctggatggcttgacctccattctgccattggggatcatcgctggcttgctgattggcaaaccgctggggattagtctgttctgctggttggcgctgcgtttgaaactggcgcatctgcctgagggaacgacttatcagcaaattatggtggtggggatcctgtgcggtatcggttttactatgtctatctttattgccagcctggcctttggtagcgtagatccagaactgattaactgggcgaaactcggtatcctggtcggttctatctcttcggcggtaattggatacagctggttacgcgttcgtttgcgtccatcagtttgacaggacggtttaccggggagccataaacggctcccttttcattgttatcagggagagaaatgagcatgtctcatatcaattacaaccacttgtattacttctggcatgtctataaagaaggttccgtggttggcgcagcggaggcgctttatttaactccacaaaccattaccggacagattcgagcgctggaagagcgcctgcaaggcaaattatttaaacgcaagggacgtggtctcgaacccagcgagctgggagaactggtctatcgctatgccgataaaatgttcaccttaagccaggaaatgctggatattgtgaactatcgcaaagaatccaatttattgtttgacgttggcgtggctgatgcactttccaaacgcctggtcagtagcgtacttaacgccgcagtggtagaaggcgagcccattcatcttcgctgcttcgaatccacccacgaaatgctgctggagcaattaagtcagcataaactggatatgatcatttctgactgtccgatagactctacgcagcaggaaggcctgttctccgtgagaattggcgaatgtggcgtgagtttctggtgtacaaatccaccaccagaaaaaccgttcccggcttgtctggaagaacggcgacttttgattcctgggcgacgttcaatgttagggcgcaaattgcttaactggtttaactcccagggattaaacgtagaaatcctcggcgagtttgatgatgccgctttgatgaaagcttttggtgcgatgcacaatgcaatcttcgttgccccaacgctttatgcatatgacttttatgccgataaaactgtcgtagaaattggtcgcgtcgagaatgtgatggaagagtaccatgctatttttgctgagcggatgattcagcacccggcggtacagcgaatctgcaatacggattattctgcgctttttagtccagcggtgcgttaatcggcagctcccccaaagttaaggtgggggagatagattagttgtacattaccacgattttgactcggctcattatttgcccgcttgagacattgtttccatatgtacgcgggcgaataaatagaggaatctgattacttccttcatggggatgctgaaaagagtagtaattgctggtaatgactccaacttattgatagtgttttatgttcagataatgcccgatgactttgtcatgcagctccaccgattttgagaacgacagcgacttccgtcccagccgtgccaggtgctgcctcagattcaggttatgccgctcaattcgctgcgtatatcgcttgctgattacgtgcagctttcccttcaggcgggattcatacagcggccagccatccgtcatccatatcaccacgtcaaagggtgacagcaggctcataagacgccccagcgtcgccatagtgcgttcaccgaatacgtgcgcaacaaccgtcttccggagactgtcatacgcgtaaaacagccagcgctggcgcgatttagccccgacatagccccactgttcgtccatttccgcgcagacgatgacgtcactgcccggctgtatgcgcgaggttaccgactgcggcctgagttttttaagtgacgtaaaatcgtgttgaggccaacgcccataatgcgggctgttgcccggcatccaacgccattcatggccatatcaatgattttctggtgcgtaccgggttgagaagcggtgtaagtgaactgcagttgccatgttttacggcagtgagagcagagatagcgctgatgtccggcggtgcttttgccgttacgcaccaccccgtcagtagctgaacaggagggacagctgatagaaacagaagccactggagcacctcaaaaacaccatcatacactaaatcagtaagttggcagcatcacctacctcaatgtgtatcacaatatccatattctttgtgggggagtctggagattgagtagatattcttgttcagaatgtatcagccgatggttctacgattcttaagccacgaagagttcagatagtacaacggcatgtctcttttgactatctggcaaccggcagtgtgttctctcacgcatcacaaaagcagcaggcataaaaaaacccgcttgcgcgggctttttcacaaagcttcagcaaattggcgattaagccagtttgttgatctgtgcagtcaggttagccttatgacgtgcagctttgtttttgtggatcagacctttagcagcctgacggtccacgatcggttgcatttcgttaaatgctttctgtgcagcagctttgtcgccagcttcgatagctgcgtatactttcttgatgaaagtacgcatcatagagcgacggcttgcgttgtgcttacgagccttttcagactgaatggcgcgcttcttagctgatttgatattagccaaggtccaactcccaaatgtgttctatatggacaattcaaaggccgaggaatatgcccttttagccttcttttgtcaatggatttgtgcaaataagcgccgttaatgtgccggcactcgttacgtagtgatggcgcaggattctaccagcttgcggggtgtgaatacagcttttccgcgataaaaattgcagcaggcggtcagtttcttcccgtgatttgcgccatggcaatgaaaagccacttctttctgatttcggtactcaatcgccggttaaccttgaccgctgtacaaggtatactcggacgattttcactgttttgagccagacatgaagctgatacgcggcatacataatctcagccaggccccgcaagaagggtgtgtgctgactattggtaatttcgacggcgtgcatcgcggtcatcgcgcgctgttacagggcttgcaggaagaagggcgcaagcgcaacttaccggtgatggtgatgctttttgaacctcaaccactggaactgtttgctaccgataaagccccggcaagactgacccggctgcgggaaaaactgcgttaccttgcagagtgtggcgttgattacgtgctgtgcgtgcgtttcgacaggcgtttcgcggcgttaaccgcgcaaaatttcatcagcgatcttctggtgaagcatttgcgcgtaaaatttcttgccgtaggtgatgatttccgctttggcgctggtcgtgaaggcgatttcttgttattacagaaagctggcatggaatacggcttcgatatcaccagtacgcaaactttttgcgaaggtggcgtgcgcatcagcagcaccgccgtgcgtcaggcccttgcggatgacaatctggctctggcagagagtttactggggcacccgtttgccatctccgggcgtgtagtccacggtgatgaattagggcgcactataggtttcccgacggcgaatgtaccgctgcgccgtcaggtttccccggtgaaaggggtttatgcggtagaagtgctgggcctcggtgaaaagccgttacccggcgtggcaaacatcggaacacgcccaacggttgccggtattcgccagcagctggaagtgcatttgttagatgttgcaatggacctttacggtcgccatatacaagtagtgctgcgtaaaaaaatacgcaatgagcagcgatttgcgtcgctggacgaactgaaagcgcagattgcgcgtgatgaattaaccgcccgcgaattttttgggctaacaaaaccggcttaagcctgttatgtaatcaaaccgaaatacggaaccgagaatctgatgagtgactataaatcaaccctgaatttgccggaaacagggttcccgatgcgtggcgatctcgccaagcgcgaacccggaatgctggcgcgttggactgatgatgatctgtacggcatcatccgtgcggctaaaaaaggcaaaaaaaccttcattctgcatgatggccctccttatgcgaatggcagcattcatattggtcactcggttaacaagattctgaaagacattatcgtgaagtccaaagggctttccggttatgactcgccgtatgtgcctggctgggactgccacggtctgccgatcgagctgaaagtcgagcaagaatacggtaagccgggtgagaaattcaccgccgccgagttccgcgccaagtgccgcgaatacgcggcgacccaggttgacggtcaacgcaaagactttatccgtctgggcgtgctgggcgactggtcgcacccgtacctgaccatggacttcaaaactgaagccaacatcatccgcgcgctgggcaaaatcatcggcaacggtcacctgcacaaaggcgcgaagccagttcactggtgcgttgactgccgttctgcgctggcggaagcggaagttgagtattacgacaaaacttctccgtccatcgacgttgctttccaggcagtcgatcaggatgcactgaaagcaaaatttgccgtaagcaacgttaacggcccaatctcgctggtaatctggaccaccacgccgtggactctgcctgccaaccgcgcaatctctattgcaccagatttcgactatgcgctggtgcagatcgacggtcaggccgtgattctggcgaaagatctggttgaaagcgtaatgcagcgtatcggcgtgaccgattacaccattctcggcacggtaaaaggtgcggagcttgagctgctgcgctttacccatccgtttatgggcttcgacgttccggcaatcctcggcgatcacgttaccctggatgccggtaccggtgccgttcacaccgcgcctggccacggcccggacgactatgtgatcggtcagaaatacggcctggaaaccgctaacccggttggcccggacggcacttatctgccgggcacttatccgacgctggatggcgtgaacgtcttcaaagcgaacgacatcgtcgttgcgctgctgcaggaaaaaggcgcgctgctgcacgttgagaaaatgcagcacagctatccgtgctgctggcgtcacaaaacgccgatcatcttccgcgcgacgccgcagtggttcgtcagcatggatcagaaaggtctgcgtgcgcagtcactgaaagagatcaaaggcgtgcagtggatcccggactggggccaggcgcgtatcgagtcgatggttgctaaccgtcctgactggtgtatctcccgtcagcgcacctggggtgtaccgatgtcactgttcgtgcacaaagacacggaagagctgcatccgcgtacccttgaactgatggaagaagtggcaaaacgcgttgaagtcgatggcatccaggcgtggtgggatctcgatgcgaaagagatcctcggcgacgaagctgatcagtacgtgaaagtgccggacacattggatgtatggtttgactccggatctacccactcttctgttgttgacgtgcgtccggaatttgccggtcacgcagcggacatgtatctggaaggttctgaccaacaccgcggctggttcatgtcttccctaatgatctccaccgcgatgaagggtaaagcgccgtatcgtcaggtactgacccacggctttaccgtggatggtcagggccgcaagatgtctaaatccatcggcaataccgtttcgccgcaggatgtgatgaacaaactgggcgcggatattctgcgtctgtgggtggcatcaaccgactacaccggtgaaatggccgtttctgacgagatcctgaaacgtgctgccgatagctatcgtcgtatccgtaacaccgcgcgcttcctgctggcaaacctgaacggttttgatccagcaaaagatatggtgaaaccggaagagatggtggtactggatcgctgggccgtaggttgtgcgaaagcggcacaggaagacatcctcaaggcgtacgaagcatacgatttccacgaagtggtacagcgtctgatgcgcttctgctccgttgagatgggttccttctacctcgacatcatcaaagaccgtcagtacaccgccaaagcggacagtgtggcgcgtcgtagctgccagactgcgctatatcacatcgcagaagcgctggtgcgctggatggcaccaatcctctccttcaccgctgatgaagtgtggggctacctgccgggcgaacgtgaaaaatacgtcttcaccggtgagtggtacgaaggcctgtttggcctggcagacagtgaagcgatgaacgatgcgttctgggacgagctgttgaaagtgcgtggcgaagtgaacaaagtcattgagcaagcgcgtgccgacaagaaagtgggtggctcgctggaagcggcagtaaccttgtatgcagaaccggaactgtcggcgaaactgaccgcgctgggcgatgaattacgatttgtcctgttgacctccggcgctaccgttgcagactataacgacgcacctgctgatgctcagcagagcgaagtactcaaagggctgaaagtcgcgttgagtaaagccgaaggtgagaagtgcccacgctgctggcactacacccaggatgtcggcaaggtggcggaacacgcagaaatctgcggccgctgtgtcagcaacgtcgccggtgacggtgaaaaacgtaagtttgcctgatgagtcaatcgatctgttcaacagggctacgctggctgtggctggtggtagtcgtgctgattatcgatctgggcagcaaatacctgatcctccagaactttgctctgggggatacggtcccgctgttcccgtcgcttaatctgcattatgcgcgtaactatggcgcggcgtttagtttccttgccgatagcggcggctggcagcgttggttctttgccggtattgcgattggtattagcgtgatcctggcagtgatgatgtatcgctcgaaggccacgcagaagctaaacaatatcgcttacgcgctgattattggcggcgcgctgggcaacctgttcgaccgcctgtggcacggcttcgttgtcgatatgatcgacttctacgtcggcgactggcacttcgccaccttcaaccttgccgatactgccatctgtgtcggtgcggcactgattgtgctggaaggttttttgccttctagagcgaaaaaacaataataaaccctgccggatgcgatgctgacgcatcttatccggcctacagattgctgcgaaatcgtaggccggataaggcgtttacgccgcatccggcaaaaatccttaaatataagagcaaacctgcatgtctgaatctgtacagagcaatagcgccgtcctggtgcacttcacgctaaaactcgacgatggcaccaccgccgagtctacccgcaacaacggtaaaccggcgctgttccgcctgggtgatgcttctctttctgaagggctggagcaacacctgttggggctgaaagtgggcgataaaaccaccttctcgttggagccagatgcggcgtttggcgtgccgtcaccggacctgattcagtacttctcccgccgtgaatttatggatgcaggcgagccagaaattggcgcaatcatgctttttaccgcaatggatggcagtgagatgcctggcgtgatccgcgaaattaacggcgactccattaccgttgatttcaaccatccgctggccgggcagaccgttcattttgatattgaagtgctggaaatcgatccggcactggaggcgtaacatgcagatcctgttggccaacccgcgtggtttttgtgccggggtagaccgcgctatcagcattgttgaaaacgcgctggccatttacggcgcaccgatatatgtccgtcacgaagtggtacataaccgctatgtggtcgatagcttgcgtgagcgtggggctatctttattgagcagattagcgaagtaccggacggcgcgatcctgattttctccgcacacggtgtttctcaggcggtacgtaacgaagcaaaaagtcgcgatttgacggtgtttgatgccacctgtccgctggtgaccaaagtgcatatggaagtcgcccgcgccagtcgccgtggcgaagaatctattctcatcggtcacgccgggcacccggaagtggaagggacaatgggccagtacagtaacccggaagggggaatgtatctggtcgaatcgccggacgatgtgtggaaactgacggtcaaaaacgaagagaagctctcctttatgacccagaccacgctgtcggtggatgacacgtctgatgtgatcgacgcgctgcgtaaacgcttcccgaaaattgtcggtccgcgcaaagatgacatctgctacgccacgactaaccgtcaggaagcggtacgcgccctggcagaacaggcggaagttgtgttggtggtcggttcgaaaaactcctccaactccaaccgtctggcggagctggcccagcgtatgggcaaacgcgcgtttttgattgacgatgcgaaagacatccaggaagagtgggtgaaagaggttaaatgcgtcggcgtgactgcgggcgcatcggctccggatattctggtgcagaatgtggtggcacgtttgcagcagctgggcggtggtgaagccattccgctggaaggccgtgaagaaaacattgttttcgaagtgccgaaagagctgcgtgtcgatattcgtgaagtcgattaagtcattagcagcctaagttatgcgaaaatgccggtcttgttaccggcattttttatggagaaaacatgcgtttacctatcttcctcgatactgaccccggcattgacgatgccgtcgccattgccgccgcgatttttgcacccgaactcgacctgcaactgatgaccaccgtcgcgggtaatgtctcggttgagaaaactacccgcaatgccctgcaactgctgcatttctggaatgcggagattccgctcgcccaaggggccgctgtgccactggtacgcgcaccgcgtgatgcggcatctgtgcacggcgaatcgggaatggctggctacgactttgttgagcacaaccgaaagccgctcgggataccggcgtttctggcgattcgggatgccctgatgcgtgcaccagagcctgttaccctggtggccatcggcccgttaaccaatattgcgctgttactttcacaatgcccggaatgcaagccgtatattcgccgtctggtgatcatgggtggttctgccggacgcggcaactgtacgccaaacgccgagtttaatattgctgccgatccagaagctgctgcctgtgtcttccgcagtggtattgaaatcgtcatgtgcggtttggatgtcaccaatcaggcaatattaactcctgactatctctctacactgccgcagttaaaccgtaccgggaaaatgcttcacgccctgtttagccactaccgtagcggcagtatgcaaagcggcttgcgaatgcacgatctctgcgccatcgcctggctggtgcgcccggacctgttcactctcaaaccctgttttgtggcagtggaaactcagggcgaatttacctcaggcacgacggtggttgatatcgacggttgcctgggcaagccagccaatgtacaggtggcattggatctggatgtgaaaggcttccagcagtgggtggctgaggtgctggctctggcgtcgtaacctgtcacatgttattggcatgcagtcattcatcgactcatgcctttcactgatatccctccctgtttatcattaatttctaattatcagcgtttttggctggcggcgtagcgatgcgctggttactctgaaaacggtctatgcaaattaacaaaagagaatagctatgcatgatgcaaacatccgcgttgccatcgcgggagccggggggcgtatgggccgccagttgattcaggcggcgctggcattagagggcgtgcagttgggcgctgcgctggagcgtgaaggatcttctttactgggcagcgacgccggtgagctggccggagccgggaaaacaggcgttaccgtgcaaagcagcctcgatgcggtaaaagatgattttgatgtgtttatcgattttacccgtccggaaggtacgctgaaccatctcgctttttgtcgccagcatggcaaagggatggtgatcggcactacggggtttgacgaagccggtaaacaagcaattcgtgacgccgctgccgatattgcgattgtctttgctgccaattttagcgttggcgttaacgtcatgcttaagctgctggagaaagcagccaaagtgatgggtgactacaccgatatcgaaattattgaagcacatcatagacataaagttgatgcgccgtcaggcaccgcactggcaatgggagaggcgatcgcccacgcccttgataaagatctgaaagattgcgcggtctacagtcgtgaaggccacaccggtgaacgtgtgcctggcaccattggttttgccaccgtgcgtgcaggtgacatcgttggtgaacataccgcgatgtttgccgatattggcgagcgtctggagatcacccataaggcgtccagccgtatgacatttgctaacggcgcggtaagatcggctttgtggttgagtggtaaggaaagcggtctttttgatatgcgagatgtacttgatctcaataatttgtaaccacaaaatatttgttatggtgcaaaaataacacatttaatttattgattataaagggctttaatttttggcccttttatttttggtgttatgtttttaaattgtctataagtgccaaaaattacatgttttgtcttctgtttttgttgttttaatgtaaattttgaccatttggtccacttttttctgctcgtttttatttcatgcaatcttcttgctgcgcaagcgttttccagaacaggttagatgatctttttgtcgcttaatgcctgtaaaacatgcatgagccacaaaataatataaaaaatcccgccattaagttgacttttagcgcccatatctccagaatgccgccgtttgccagaaattcgtcggtaagcagatttgcattgatttacgtcatcattgtgaattaatatgcaaataaagtgagtgaatattctctggagggtgttttgattaagtcagcgctattggttctggaagacggaacccagtttcacggtcgggccataggggcaacaggttcggcggttggggaagtcgttttcaatacttcaatgaccggttatcaagaaatcctcactgatccttcctattctcgtcaaatcgttactcttacttatccccatattggcaatgtcggcaccaatgacgccgatgaagaatcttctcaggtacatgcacaaggtctggtgattcgcgacctgccgctgattgccagcaacttccgtaataccgaagacctctcttcttacctgaaacgccataacatcgtggcgattgccgatatcgatacccgtaagctgacgcgtttactgcgcgagaaaggcgcacagaatggctgcattatcgcgggcgataacccggatgcggcgctggcgttagaaaaagcccgcgcgttcccaggtctgaatggcatggatctggcaaaagaagtgaccaccgcagaagcctatagctggacacaagggagctggacgttgaccggtggcctgccagaagcgaaaaaagaagacgagctgccgttccacgtcgtggcttatgattttggtgccaagcgcaacatcctgcggatgctggtggatagaggctgtcgcctgaccatcgttccggcgcaaacttctgcggaagatgtgctgaaaatgaatccagacggcatcttcctctccaacggtcctggcgacccggccccgtgcgattacgccattaccgccatccagaaattcctcgaaaccgatattccggtattcggcatctgtctcggtcatcagctgctggcgctggcgagcggtgcgaagactgtcaaaatgaaatttggtcaccacggcggcaaccatccggttaaagatgtggagaaaaacgtggtaatgatcaccgcccagaaccacggttttgcggtggacgaagcaacattacctgcaaacctgcgtgtcacgcataaatccctgttcgacggtacgttacagggcattcatcgcaccgataaaccggcattcagcttccaggggcaccctgaagccagccctggtccacacgacgccgcgccgttgttcgaccactttatcgagttaattgagcagtaccgtaaaaccgctaagtaatcaggagtaaaagagccatgccaaaacgtacagatataaaaagtatcctgattctgggtgcgggcccgattgttatcggtcaggcgtgtgagtttgactactctggcgcgcaagcgtgtaaagccctgcgtgaagagggttaccgcgtcattctggtgaactccaacccggcgaccatcatgaccgacccggaaatggctgatgcaacctacatcgagccgattcactgggaagttgtacgcaagattattgaaaaagagcgcccggacgcggtgctgccaacgatgggcggtcagacggcgctgaactgcgcgctggagctggaacgtcagggcgtgttggaagagttcggtgtcaccatgattggtgccactgccgatgcgattgataaagcagaagaccgccgtcgtttcgacgtagcgatgaagaaaattggtctggaaaccgcgcgttccggtatcgcacacacgatggaagaagcgctggcggttgccgctgacgtgggcttcccgtgcattattcgcccatcctttaccatgggcggtagcggcggcggtatcgcttataaccgtgaagagtttgaagaaatttgcgcccgcggtctggatctctctccgaccaaagagttgctgattgatgagtcgctgatcggctggaaagagtacgagatggaagtggtgcgtgataaaaacgacaactgcatcatcgtctgctctatcgaaaacttcgatgcgatgggcatccacaccggtgactccatcactgtcgcgccagcccaaacgctgaccgacaaagaatatcaaatcatgcgtaacgcctcgatggcggtgctgcgtgaaatcggcgttgaaaccggtggttccaacgttcagtttgcggtgaacccgaaaaacggtcgtctgattgttatcgaaatgaacccacgcgtgtcccgttcttcggcgctggcgtcgaaagcgaccggtttcccgattgctaaagtggcggcgaaactggcggtgggttacaccctcgacgaactgatgaacgacatcactggcggacgtactccggcctccttcgagccgtccatcgactatgtggttactaaaattcctcgcttcaacttcgaaaaattcgccggtgctaacgaccgtctgaccactcagatgaaatcggttggcgaagtgatggcgattggtcgcacgcagcaggaatccctgcaaaaagcgctgcgcggcctggaagtcggtgcgactggattcgacccgaaagtgagcctggatgacccggaagcgttaaccaaaatccgtcgcgaactgaaagacgcaggcgcagatcgtatctggtacatcgccgatgcgttccgtgcgggcctgtctgtggacggcgtcttcaacctgaccaacattgaccgctggttcctggtacagattgaagagctggtgcgtctggaagagaaagtggcggaagtgggcatcactggcctgaacgctgacttcctgcgccagctgaaacgcaaaggctttgccgatgcgcgcttggcaaaactggcgggcgtacgcgaagcggaaatccgtaagctgcgtgaccagtatgacctgcacccggtttataagcgcgtggatacctgtgcggcagagttcgccaccgacaccgcttacatgtactccacttatgaagaagagtgcgaagcgaatccgtctaccgaccgtgaaaaaatcatggtgcttggcggcggcccgaaccgtatcggtcagggtatcgaattcgactactgttgcgtacacgcctcgctggcgctgcgcgaagacggttacgaaaccattatggttaactgtaacccggaaaccgtctccaccgactacgacacttccgaccgcctctacttcgagccggtaactctggaagatgtgctggaaatcgtgcgtatcgagaagccgaaaggcgttatcgtccagtacggcggtcagaccccgctgaaactggcgcgcgcgctggaagctgctggcgtaccggttatcggcaccagcccggatgctatcgaccgtgcagaagaccgtgaacgcttccagcatgcggttgagcgtctgaaactgaaacaaccggcgaacgccaccgttaccgctattgaaatggcggtagagaaggcgaaagagattggctacccgctggtggtacgtccgtcttacgttctcggcggtcgggcgatggaaatcgtctatgacgaagctgacctgcgtcgctacttccagacggcggtcagcgtgtctaacgatgcgccagtgttgctggaccacttcctcgatgacgcggtagaagttgacgtggatgccatctgcgacggcgaaatggtgctgattggcggcatcatggagcatattgagcaggcgggcgtgcactccggtgactccgcatgttctctgccagcctacaccttaagtcaggaaattcaggatgtgatgcgccagcaggtgcagaaactggccttcgaattgcaggtgcgcggcctgatgaacgtgcagtttgcggtgaaaaacaacgaagtctacctgattgaagttaacccgcgtgcggcgcgtaccgttccgttcgtctccaaagccaccggcgtaccgctggcaaaagtggcggcgcgcgtgatggctggcaaatcgctggctgagcagggcgtaaccaaagaagttatcccgccgtactactcggtgaaagaagtggtgctgccgttcaataaattcccgggcgttgacccgctgttagggccagaaatgcgctctaccggggaagtcatgggcgtgggccgcaccttcgctgaagcgtttgccaaagcgcagctgggcagcaactccaccatgaagaaacacggtcgtgcgctgctttccgtgcgcgaaggcgataaagaacgcgtggtggacctggcggcaaaactgctgaaacagggcttcgagctggatgcgacccacggcacggcgattgtgctgggcgaagcaggtatcaacccgcgtctggtaaacaaggtgcatgaaggccgtccgcacattcaggaccgtatcaagaatggcgaatatacctacatcatcaacaccacctcaggccgtcgtgcgattgaagactcccgcgtgattcgtcgcagtgcgctgcaatataaagtgcattacgacaccaccctgaacggcggctttgccaccgcgatggcgctgaatgccgatgcgactgaaaaagtaatttcggtgcaggaaatgcacgcacagatcaaataatagcgtgtcatggcagatatttttcatccgctaatttgatcgaataactaatacggttctctgatgaggaccgtttttttttgcccattaagtaaatcttttggggaatcgatatttttgatgacataagcaggatttagctcacacttatcgacggtgaagttgcatactatcgatatatccacaattttaatatggccttgtttaattgcttcaaaacgagtcatagccagacttttaatttgtgaaactggagttcgtatgtgtgaaggatatgttgaaaaaccactctacttgttaatcgccgaatggatgatggctgaaaatcggtgggtgatagcaagagagatctctattcatttcgatattgaacacagcaaggcggttaataccctgacttatattctgtcggaagtcacagaaataagctgcgaagttaagatgatccctaataagctggaagggcggggatgccagtgtcagcgactggttaaagtggtcgatatcgatgagcaaatttacgcgcgcctgcgcaataacagtcgggaaaaattagtcggtgtaagaaagacgccgcgtattcctgccgttccgctcacggaacttaaccgcgagcagaagtggcagatgatgttgtcaaagagtatgcgtcgttaattttatctcgttgataccgggcgtcctgcttgccagatgcgatgttgtagcatcttatccagcaaccaggtcgcatccggcaagatcaccgtttaggcgtcacatccgtcgtcccctgcaaacgggggcgattttcctccatttgcctcagtggctgcgtttcatgtaacgatacatgacagcgcccgacaagatcctgatactctttggtattcaaccgtttccagtgtaactcgtcgtcactaacattgcgtacagcgcgggctggcgtacccatcaacaactggcgtttctcgccgcgaaagcccgctttgacaaagctcatggcggcaacaatgctctcttcgccaatgaccgcgccatccataatcacgctgttcatcccgaccaatgcatcgcgaccaatcaaacaaccatgcaggatcgctccgtgcccgatatggccgttttccccaacgatagtgtcagtgtcgcagtagccatgcataatgcagccatcctgaatattggctcccgcttgcacgatcaaccgcccgtagtcaccacgcagtgaggcgagtgggccgatgtagacaccggctcccacaatcacatcgccaatcaagacggcactgggatggacaaacgccgtcgggtgaaccaccggaattaacccctcaaaggcgtaatagctcacggttgttaacgtcctttccacaccggatcgcgcttctcggcaaacgccagcggcccttcaatggcatcttccgaatgcagaaccgatggatagtgtttcaacacgccgctgcgaatatagcgatacgcttcttctaccggcatttcgctggtggtgcggtagatctctttcagcgccgcaatcgccagcggggcgctgttaaccagctgctgagccagttcgcgggcgttatccatcagttccgcctggctaaccacgcggttgactatcccccaacgcagcgcctcttctgcgcccattcgtctgccggtcatcaccatttcattgacgatggcaggcggcaggatcttcggcagacgcagcacaccgccgctgtcaggaacgatgcccagtttggcttccggcagggcgaagctggcgttatcggcacaaacaataaaatctgccgccagcgccagttcaaagccgccgccaaaggcatagccgttcacagctgcgataaccggtttgtcgagattgaaaatttcggttaatcccgcaaaaccacccggaccaaagtcagcatccggtgcttcgccttctgctgccgcttttaaatcccagcccgcggaaaagaacttctctccggcaccggtaataatggcgacacgtaattgcggatcgtcacggaaatttagaaatacttcgcccatttcaaagctggtttttgcatcaatagcattcgcttttggacgatcaagggtaatttccagaattgatccattgcgggtcagatgtaatgattcactcattccttttctccatttttgctttttcagggacgacaacatccctgcaaaaaatgcatattgttttagagtgtgattattagctggcagggtagttccctgctgtttcatttatttcagattctttctaattattttccccgagcaattacgtggcagatcttttctgatctccagataagagggcactttaaatttcgccatattttgttcgcagaagcggaaaaattcctcttcgctcaatgtttcaccttcattcagcaccacaaatgctttgatggcttcatcgcgaatcgaatctttaatacccacaaccacgatgtcctgaattttcgggtgcgcggcgataatattttccagctccacgcaggagacattctcgccgccacgtttaatcatattgcagcggcgatcgacgaaataaaaaaagtcctcttcgtcgcggtatccggtatcgccggtatgcagccagccatcggcttccagcactttcgcagtggcttgtgggttgagaaagtactctttgaagatggttttcccaggtatgcctttaatgcagatttcaccgatctcaccagccgggagcgggcgattgtgatcgtcgcggatctccgcttcgtagcaaaaccccacccgaccaatcgacggccagcgtcgtttatcgccaggacgatcgccgataatgcccacaatggtttccgtcatcccataagacgtcagcaagcgaacgccgaagcgttcacaaaacgcatctttttcctgctccgacaagttgagataaaacatcacttcccgcaggcggtgttgctgatcgttcgctgaaggcggctgtaccatcaacgtacggatcatcatcggaatacattcggtaacggtggcgcggtacttctgtacctgtccccagaaggcgcgggcgctgtatttctcgaccagcacaaaggtggccccggcagaaaacgccgccatcgccgcagtacactggcaatcgatatgaaacgcaggcattaccgtcaggtagacgtcatcgtcacgcagtgcacactgccaggcggagtaatatccagcgaagcgcaggttgtaatgggtaatcaccacacctttcggtcgggaggtggtgccggaggtgaagagaatttccgccgtatcgtcagtcgatagcggcggtgcatagcacaaggtggcaggttgttgatttttcagttgagtaaacgaactcacgccatcatcagcgggaagtgccacatctgtcaggcaaatgtgccgcaattgagtggcatcttcctgctgaatctgttgatacataggatagaattgcgcactggtcaccagcaggcacgcctggctattttgcaggatccacgcgctttcctcgcacaacaggcgggcgttaatcggcaccataatcgcgccaatttttgccagcccgaaccagcaaaagataaattccgggcagttgtcgagatgtagtgcaaccttgtcgcctttgcgaatccccagcgtataaaacaggtttgccgtgcggttaatctcctgatttaactcaagataactataccggttaacgactccgccgctggattcacaaatcagcgccgttttatgaccgtaaacgtccgcaagatcgtcccacatttgacgtagatgttgtccgccaatgatatccattgcacctctatccatttttgttcgtttgttattgggcgggcgctagtcaggcaagccgactgacgccacgcgtttagtcctcaactttggccagacctttgctgaccaactcctgaatgtcgttttcgctgtagccgatatttttcaaaatggcagccgtgtccatgccatgtgagggcattccgcgccagatttgtccggggttatttttgaatttcggcatgatgttcggccctttgcaggtgcgaccatccatcgtttgccactgagtgattgattcgcgagccacatactgtggattgctttccagttccggtacggtcagcactttggcgcaggcgatattcagttcagcaaagcgttcttttacttccgcgatggtatgtgtcgccagccaggcatcgagtttctcttcaaccagtgggccgtaagggcattcgatacggtggataagctgagtgccttccgggatttctggcgtgccaagcagatgtgcgaggccaatatctttaaagcactcttcaatttgggtaatgcccaccagttccatcacgatgtagccgtcggcacatttatacagaccgcaaccggcgtagtagggatctttacctttgctcatgcgcgggcacatttcgccgccgttgaagtaatccatcatgaagtactggcccatacgcagcatcacttcatacatggcgatgtcgatactttcgcctttaccggtttcacgcactttatgcagtgctgccagcgccgccgtggtggcggtcaggccagaaaagtaatcggcggtatacgggaaggcaggcattggctggtcaacatcaccgttctgaatcaggtaaccactaaaggcctgggcgatagtgttataggccggaagattggtgtactcctcggtgccgtactgaccaaaaccggacaggtgagcgataaccagtttcgggttgtgctgccacagtacttcatcggtaatgccacgacgggcaaaggccggacctttactggcttcgatgaagatatcggtggtttccattaatttcagaaacgcttcgcggccttcatctttgaaaatatttaacgacagcgcgtgcaaattgcggcgggagagttgcgggtagttcggttgaacgcgaatggtgtcggcccaggcgacgttctcgatccagataacttccgcgccccattctgcgaacatttgcccggcaaacggtccggcgatttcgataccggagaagacaacgcgcaatccggccaacggcccgaatttcggcatgggtagatgatccattatttgctcctgaaaaatttatgtagcgcatgactgccggatgcggcgtaaacgctttatccggcctacattcgtgctcccgtaggcctgataagacgcatcagcgtcgcatcaggcagcgcacggacttagcggtattgcttcagcaccgcacgacccagcgtcaggatctgcatttcgtcagatcccccggagacgcggtctacacgcagatcacgccagaagcggctgatgcggtggttgcccgcaatcccgacaccgcccagcacctgcattgcgctatccacaacttcaaatgccgcattggcgcagaagtatttgcacatcgctgcatcgccagaggtgatggtgccgttgtctgctttccacgctgcttcatacagcatgtttttcatggagtttaatttgatcgccatgtgggcgaatttttcctgaatcaactggaaacgaccaatagcctcgccaaactgcacgcgctgattggcgtagcgcgccgcatcttcaaaggcgcacatcgccgtaccgtagttggtgagggctaccaggaaacgttcatggtcgaactcttctttgacgcggttaaagccgttaccttcccgaccgaacatgtctttctcgtccagttccacgtcgtcaaaggtgatttcacagcagctatccatacgcagaccgagcttttcaagtttggtcactttgatgcccggtttgctcatatcaacaaaccattcggtgtagacaggtttgtccggagaagccccgtcgcgcgccatcaccacgatgtacggggtgtaggcgctgctggtaataaaacacttactaccattaagataaatcttaccatttctacgggtataagtcgttttcaggctacccacgtcggagcccgcgcccggttcggtaatcgctgagttccacatctgcttaccggtgccgcggaaagccataattttgtcgatctgctcttgtgtgccttcgcgcaggaaggtgttgaacccgcccggcaactggtacagcacataggttggtgcccccagacgtcccagctccatccacacggcggcgagagtaacaaaccccgcgtccagaccaccgtgctcttcagggatcagcagactgtcgatacccatatccgccagtgctttgacaaaacgttccgggtagacgctgtcacggtcgcactcggcaaaataggcctcccagttttcgctggccatcagttcgcggataccggcgacaaacagttcctgctcatcatttaaattaaaatccatctttcaacctcttgatattttgggggttaattaatctttccagttctgtttcgcgtctttaataaaggagagcgtcaccataatgttgacgaagaacagcgggcatcctccggcgataatggcggtttgaatcggtttcaggccgccgagcgccagcagaacaataccgataatgccaaccagaattgaccaaccgatacgcaccagcagaggtggttcttcaccatcgcgtacttcgcggcaagtggacatcgccagggtataagagcaggcgttaaccagcgtaacggtggcaataaagcagaggatgaagaagccccacatggtggcggtgctgagtggcagagcggcccaggtttcaatgatggcgcgcgccacaccgtactgttcgatcagatttggaatgttgatgatgtttttatctatcaacagcagagtgttactaccgagtacagtccacaggatccaggttgacgctgtcagccccagcaccatgccgaagcacagttcacgcacagtacgaccacgggagatgcgggcgaggaagatactcatctggatagcataaatcacccaccatgcccagtagaacacggtccagccctgcgggaagccgcctttagcgatgggatcggtatagaacaacatgcgcggcagatacatcagcaacatccccaccgaatcggtgaagtagttcatgatgaagctggcaccgctgacaatgaacacccaacccagcatcaggaagctcaggtaactacgcacgtcactggcgatacgtacccctttttgcagaccgcaagcgacgcaaatggcgttgaggataatccagcaggtaatgatgatagcgtccagttgcagggtatgcggaatgccaaacaaccattgcatacactcggtcaccagcggcgtggcaaggcccagactggtacccatcgcgaagatcaaggcgacgagatagaagttgtcgacgatagtgccgaacaaccctttggcgtgtttttcacctaccagcggcaccagtgtcgagctggggcgaatcacttccattttgcggacaaagaagaagtaagcgaaggcgactgaaaggaagctgtaagtggcccacggcagaggtccccagtggaacaagctgtaagccagccccaactctttcgcccctgtcgagttcggttctaagccaaacggcggggtggagatgtagtagtagatctcaatcgatccccagaacagtacggcagcagacgtacaggaggcgaacatcataaagatccaactggcggtgctaaattctggcggttcgttacctaaacgctttttggcatacgggccaaacaccagccagaaccaaccgaaaagcatcaccaccatataccattcaaatgcccatccccatacattggtgacgtaactgaatacagcattaataacgacattcgctgcatccagatctctgactgtaagccaacaaagtatgccgacgattattaacggcggaaagaaaaccttcggttctattcccgtttttctcttttcattcttcatgagttaattccactgtgaaaacgaatatttattttgcgttcccgtttgttttatttttgttaacatttaatataattattattaacctcgtggacgcgttaatggctaactcataatgggtattcaataagctgtattctgtgattggtatcacatttttgtttcgggtgaatagagggcgttttttcgttaattttgattaataatcagtttgttatgctctgttgtgagtaaaaaataacatctgactttcaatattggtgatccataaaacaatattgaaaatttctttttgctacgccgtgttttcaatattggtgaggaacttaacaatattgaaagttggatttatctgcgtgtgacattttcaatattggtgattaaagttttatttcaaaattaaagggcgtgatatctgtaattaacaccaccgatatgaacgacgtttccttcatgatttctggagatgcaatgaagattattacttgctataagtgcgtgcctgatgaacaggatattgcggtcaataatgctgatggttcattagacttcagcaaagccgatgccaaaataagccaatacgatctcaacgctattgaagcggcttgccagctaaagcaacaggcagcagaggcgcaggtgacagccttaagtgtgggcggtaaagccctgaccaacgccaaagggcgtaaagatgtgctatcgcgcggcccggatgaactgattgtggtgattgatgaccagttcgagcaggcactgccgcaacaaacggcgagcgcactggctgcagccgcccagaaagcaggctttgatctgatcctctgtggcgatggttcttccgacctttatgcccagcaggttggtctgctggtgggcgaaatcctcaatattccggcagttaacggcgtcagcaaaattatctccctgacggcagataccctcaccgttgagcgcgaactggaagatgaaaccgaaaccttaagcattccgctgcctgcggttgttgctgtttccactgatatcaactccccacaaattccttcgatgaaagccattctcggcgcggcgaaaaagcccgtccaggtatggtcggcggcggatattggttttaacgcagaggcagcctggtcagaacaacaggttgccgcgccgaaacagcgcgaacgtcagcgcatcgtgattgaaggcgacggcgaagaacagatcgccgcatttgctgaaaatcttcgcaaagtcatttaattacaggggatgctatgaacacgttttctcaagtctgggtattcagcgataccccttctcgtctgccggaactgatgaacggtgcgcaggctttagctaatcaaatcaacacctttgtcctcaatgatgccgacggcgcacaggcaatccagctcggcgctaatcatgtctggaaattaaacggcaaaccggacgatcggatgatcgaagattacgccggtgtcatggctgacactattcgccagcacggcgcagacggcctggtgctgctgccaaacacccgtcgcggcaaattactggcggcaaaactgggttatcgccttaaagcggcggtgtctaacgatgccagcaccgtcagcgtacaggacggtaaagcgacagtgaaacacatggtttacggtggtctggcgattggcgaagaacgcattgccacgccgtatgcggtactgaccatcagcagcggcacgttcgatgcggctcagccagacgcgtcacgcactggcgaaacgcacaccgtggagtggcaggctccggctgtggcgattacccgcacggcaacccaggcgcgccagagcaacagcgtcgatctcgacaaagcccgtctggtggtcagcgtcggtcgcggtattggcagcaaagagaacattgcgctggcagaacagctttgcaaggcgataggtgcggagttggcctgttctcgtccggtggcggaaaacgaaaaatggatggagcacgaacgctatgtcggtatctccaacctgatgctgaaacctgaactgtacctggcggtggggatctccgggcagatccagcacatggttggcgctaacgcgtcgcaaaccattttcgccatcaataaagataaaaatgcgccgatcttccagtacgcggattacggcattgttggcgacgccgtgaagatccttccggcgctgaccgcagctttagcgcgttgatccactctggcagggctgcattttggccctgccgctgacagggagctcttatgtccgaagatatctttgacgccatcatcgtcggtgcagggcttgccggttcggttgccgcactggtgctcgcccgcgaaggtgcgcaagtgttagttatcgagcgtggcaattccgcaggtgccaagaacgtcaccggcgggcgtctctatgcccacagtctggaacacattattcctggtttcgccgactccgcccccgtagaacgcctgatcacccatgaaaaactcgcgtttatgacggaaaagtcagcgatgactatggactactgcaatggtgacgaaacctcgccatcccagcgttcttactccgttttgcgcagtaaatttgatgcctggctgatggagcaggccgaagaagcgggcgcgcagttaattaccgggatccgcgtcgataacctcgtacagcgcgatggcaaagtcgtcggtgtagaagccgatggcgatgtgattgaagcgaaaacggtgatccttgctgatggggtgaactccatccttgccgaaaaattggggatggcaaaacgcgtcaaaccgacggatgtggcggttggcgtgaaggaactgatcgagttaccgaagtcggttattgaagaccgttttcagttgcagggtaatcagggggcggcttgcctgtttgcgggatcacccaccgatggcctgatgggcggcggcttcctttataccaatgaaaacaccctgtcgctggggctggtttgtggtttgcatcatctgcatgacgcgaaaaaatcggtgccgcaaatgctggaagatttcaaacagcatccggccgttgcaccgctgatcgcgggcggcaagctggtggaatattccgctcacgtagtgccggaagcaggcatcaacatgctgccggagttggttggtgacggcgtattgattgccggtgatgccgccggaatgtgtatgaacctcggttttaccattcgcggtatggatctggcgattgccgccggggaagccgcagcaaaaaccgtgctttcagcgatgaaaagcgacgatttcagtaagcaaaaactggcggaatatcgtcagcatcttgagagtggtccgctgcgcgatatgcgtatgtaccagaaactaccggcgttccttgataacccacgcatgtttagcggctacccggagctggcggtgggtgtggcgcgtgacctgttcaccattgatggcagcgcgccggaactgatgcgcaagaaaatcctccgccacggcaagaaagtgggcttcatcaatctaatcaaggatggcatgaaaggagtgaccgttttatgacttctcccgtcaatgtggacgtcaaactgggcgtcaataaattcaatgtcgatgaagagcatccgcacattgttgtgaaggccgatgctgataaacaggcgctggagctgctggtgaaagcgtgccccgcaggtctgtacaagaagcaggatgacggcagtgtgcgcttcgattacgccggatgtctggagtgcggcacctgtcgcattctggggctggggtcggcgctggaacagtgggaatacccgcgcggcacctttggtgtggagttccgttacggctgatgttggtttgatacgtaacgccgcactgactctcattgcaaaaaacaggaataaccatgcaaccgtccagaaactttgacgatctcaaattctcctctattcaccgccgcattttgctgtggggaagcggtggtccgtttctggatggttatgtactggtaatgattggcgtggcgctggagcaactgacgccggcgctgaaactggacgctgactggattggcttgctgggcgcgggaacgctcgccgggctgttcgttggcacatcgctgtttggttatatttccgataaagtcggacggcgcaaaatgttcctcattgatatcatcgccatcggcgtgatatcggtggcgacgatgtttgtttcatcccccgtcgaactgttggtgatgcgggtacttatcggcattgtcatcggtgcagattatcccatcgccacctcaatgatcaccgagttctccagtacccgtcagcgggcgttttccatcagctttattgccgcgatgtggtatgtcggcgcgacctgtgccgatctggtcggctactggctttatgatgtggaaggcggctggcgctggatgctgggtagcgcggcgatcccctgtttgttgattttgattggtcgattcgaactgcctgaatctccccgctggttattacgcaaagggcgagtaaaagagtgcgaagagatgatgatcaaactgtttggcgaaccggtggctttcgatgaagagcagccgcagcaaacccgttttcgcgatctgtttaatcgccgccattttccttttgttctgtttgttgccgccatctggacctgccaggtgatcccaatgttcgccatttacacctttggcccgcaaatcgttggtttgttgggattgggggttggcaaaaacgcggcactagggaatgtggtgattagcctgttctttatgctcggctgtattccgccgatgctgtggttaaacactgccggacggcgtccattgttgattggcagctttgccatgatgacgctggcgctggcggttttggggctaatcccggatatggggatctggctggtagtgatggcctttgcggtgtatgcctttttctctggcgggccgggtaatttgcagtggctctatcctaatgaactcttcccgacagatatccgcgcctctgccgtgggcgtgattatgtccttaagtcgtattggcaccattgtttcgacctgggcactaccgatctttatcaataattacggtatcagtaacacgatgctaatgggggcgggtatctcgctgtttggcttgttgatttccgtagcgtttgccccggagactcgagggatgtcactggcgcagaccagcaatatgacgatccgcgggcagagaatggggtaaattgttcagatttctctcttttctgaatcaatattattgactataagccgcgtgaatatatgactacactttgtgggaaaacaaaggcgtaatcacgcgggctacctatgattcttataatttatgcgcatccgtatccgcatcattcccatgcgaataaacggatgcttgaacaggcaaggacgctggaaggcgtcgaaattcgctctctttatcaactctatcctgacttcaatatcgatattgccgccgagcaggaggcgctgtctcgcgccgatctgatcgtctggcagcatccgatgcagtggtacagcattcctccgctcctcaaactttggatcgataaagttttctcccacggctgggcttacggtcatggcggcacggcgctgcatggcaaacatttgctgtgggcggtgacgaccggcggcggggaaagccattttgaaattggtgcgcatccgggctttgatgtgctgtcgcagccgctacaggcgacggcaatctactgcgggctgaactggctgccaccgtttgccatgcactgcacctttatttgtgacgacgaaaccctcgaagggcaggcgcgtcactataagcaacgtctgctggaatggcaggaggcccatcatggatagccatacgctgattcaggcgctgatttatctcggttcggcagcgctgattgtacccattgcggtacgtcttggtctgggatcggtacttggctacctgatcgccggctgcattattggcccgtgggggctgcgactggtgaccgatgccgaatctattctgcactttgccgagattggggtggtgctgatgctgtttattatcggcctcgaactcgatccacaaaggctgtggaagctgcgtgcggcagtgttcggctgtggcgcattgcagatggtgatttgcggcggcctgctggggctgttctgcatgttacttgggctgcgctggcaggtcgcggaattgatcggcatgacgctggcgctctcctctacggcgattgccatgcaggcgatgaatgaacgcaatctgatggtgacgcaaatgggtcgcagtgcctttgcggtgctgctgttccaggatatcgcggcgatcccgctggtggcgatgattccgctactggcaacgagcagtgcctcgacgacgatgggcgcatttgctctctcggcgttaaaagtggcgggtgcgctggtgctggtggtattgctggggcgctatgtcacgcgtccggcgctgcgttttgtagcccgctctggcttgcgggaagtgtttagtgccgtggcgttattcctcgtgtttggctttggtttgctgctggaagaggtcggcttgtcgatggcgatgggcgcgtttctggcgggcgtactgctggcaagctcggaataccgtcatgcgctggagagcgatatcgaaccatttaaaggtttgctgttggggctgtttttcatcggtgttggcatgtcgatagactttggcacgctgcttgaaaacccattgcgcattgtcattttgctgctcggtttcctcatcatcaaaatcgccatgctgtggctgattgcccgaccgttgcaagtgccaaataaacagcgtcgttggtttgcggtgttgttagggcagggcagtgagtttgcctttgtggtatttggcgcggcgcagatggcgaatgtgctggagccggagtgggcgaaatcgctgaccctggcggtggcgctgtcgatggcagcaacgccgattctgctggtgatcctcaatcgccttgagcaatcttctactgaggaagcgcgtgaagccgatgagatcgacgaagaacagccgcgcgtgattatcgccggattcggtcgttttgggcagattaccggacgtttactgctctccagcggggtgaaaatggtggtactcgatcacgatccggaccatatcgaaaccttgcgtaaatttggtatgaaagtgttttatggcgatgccacgcggatggatttactggaatctgccggagcggcgaaagcggaagtgctgattaacgccatcgacgatccgcaaaccaacctgcaactgacagagatggtgaaagaacatttcccgcatttgcagattattgcccgcgcccgcgatgtcgaccactacattcgtttgcgtcaggcaggcgttgaaaagccggagcgtgaaaccttcgaaggtgcgctgaaaaccgggcgtctggcactggaaagtttaggtctggggccgtatgaagcgcgagaacgtgccgatgtgttccgccgctttaatattcagatggtggaagagatggcaatggttgagaacgacaccaaagcccgcgcggcggtctataaacgcaccagcgcgatgttaagtgagatcattaccgaggaccgcgaacatctgtcattaattcaacgacatggctggcagggaaccgaagaaggtaaacataccggcaacatggcggatgaaccggaaacgaaaccctcatcctaataaagagtgacgtaaatcacactttacagctaactgtttgtttttgtttcattgtaatgcggcgagtccagggagagagcgtggactcgccagcagaatataaaattttcctcaacatcatcctcgcaccagtcgacgacggtttacgctttacgtatagtggcgacaattttttttatcgggaaatctcaatgatcagtctgattgcggcgttagcggtagatcgcgttatcggcatggaaaacgccatgccgtggaacctgcctgccgatctcgcctggtttaaacgcaacaccttaaataaacccgtgattatgggccgccatacctgggaatcaatcggtcgtccgttgccaggacgcaaaaatattatcctcagcagtcaaccgggtacggacgatcgcgtaacgtgggtgaagtcggtggatgaagccatcgcggcgtgtggtgacgtaccagaaatcatggtgattggcggcggtcgcgtttatgaacagttcttgccaaaagcgcaaaaactgtatctgacgcatatcgacgcagaagtggaaggcgacacccatttcccggattacgagccggatgactgggaatcggtattcagcgaattccacgatgctgatgcgcagaactctcacagctattgctttgagattctggagcggcggtaattttgtatagaatttacggctagcgccggatgcgacgccggtcgcgtcttatccggccttcctatatcaggctgtgtttaagacgccgccgcttcgcccaaatccttatgccggttcgacggctggacaaaatactgtttatcttcccagcgcaggcaggttaatgtaccaccccagcagcagccggtatccagcgcgtatataccttccggcgtacctttgccctccagcgatgcccagtgaccaaaggcgatgctgtattcttcagcgacagggccaggaatcgcaaaccacggtttcagtggggcaggggcctcttccggcgattctttgctgtacatatccagttgaccgttcgggaagcaaaaacgcatacgggtaaaagcgttggtgataaaacgcagtcttcccagcccccgcaattccggtgaccagttatttggcatatcgccgtacatggcatcaagaaagaagggataggagtcactcgatagcaccgcttctacatcgcgtgcgcactctttggcggtctgcagatcccactgcggcgtgatccctgcgtgggccatcaccagctttttctcttcgtcgatttgcagcagaggctggcgccgcagccagttaagcagctcgtcggcatccggcgcttccagcagcggtgtcaggcgatctttcggtttattgcggctgatcccggcaaataccgccagcagatgcagatcgtgattgcccagcaccagacgtacgctgtcgcctaaggatttcacatagcgcagaacatccagcgaacccggcccgcgcgcgaccagatcgcccgtcagccagagggtatctttcccaggggtaaattctactttatgcagcaatgcgatcagttcatcgtaacaaccatgaacgtcgccaataaggtatgtcgccatattcttttaatgaatgagtgtgggaacggcgagtcggaatacgggaatgtcgatgctgaaagggacgccattttcatcgatcatttcgtagtgaccctgcatggtgcccagcggggtttcaatgattgcaccgctggtgtactggtactcttcgccaggcgcgataagtggctggacgccaaccactccttcgccctggacttcggtttcacggccattgccattggtgatcagccagtaacgccccaacaactgcactggcgctcgccccagattgcgtatggttacggtataagcaaaaacgtaacgttcattatcaggtgaagattgagcctcaatgtagacgctttgaacctgaatacacactcggggcgaattgatcatcgttaactctcctgcaaaggcgcgttctccgccagatagttcgccatctggcaatattgcgcgacagagatattttccgctcgcatcgccgggtcgatccccattcccgttaacacctcgacgctaaacaggttgccgaggctgttacgaatggttttacgacgctggttaaaggcttcggtggtgatgcggctcaacacacgaacatctttaaccgggtgaggcatcgttgcatgaggaaccaggcgcacgacggcggaatccactttgggtggtggtgtaaaggctgacggcggtacttccagtaccgggatcacattgcaatagtattgcgccatgacgcttaatcgaccatacgctttgctgttcggtcctgcaaccagacgattcaccacctctttttgcaacataaagtgcatgtcggcaatggcatcagtatagctaaacagatggaacatcaacggcgtggagatgttataaggcaggttgccgaaaacacgcagcggctgacccattttctcggccagttcaccaaagttaaaggtcatcgcatcctgctgataaatcgtcagtttcgggcctaagaatggatgcgtttgcagacgtgccgccagatcgcggtcaagttcgatgaccgtcagctggtccagacgttcgccgaccggttcggtcaatgccgccagaccggggccgatttcgaccatcgcctggcccttttgcgggttaatggcagacacaatactgtcgatcacgaactgatcgttgagaaagttttgcccgaagcgtttacgggctaagtggccctggtggactcgattattcattgggtgttaacaatcattttgatggcgagattaagcgccgtaataaaactgccgacatcggctttgccacgtcccgccagttcaagcgcggtgccgtggtccactgatgtgcgaataaagggcaggcccagcgtaatgttcacaccgcgcccgaagccctggtattttagcacgggaagaccctgatcgtggtacatcgccagcacggcgtcggcgttatcaagatatttcggctgaaacagggtatcggcaggcagcggcccgttgagtttcatcccctgcgcccgcagctcattgagcaccggaataatggtgtctatctcttccgtacccatatgaccgccttcgcccgcgtgcggattcagcccgcagaccagaatgcgcggttcggcaataccaaatttggtccgcaaatcgtgatgcaaaatagcaatcacttcgtgcaaaagtgcaggggtgatagcgtctgcgatatcgcgcagcggtaaatgcgtcgttgccagcgccacgcgaagttcttcggtcgccagcatcatcaccacctttttcgcctgcgaacgctcttcgaaaaactcggtatgaccggtaaaaggaatgccagcgtcgttaataacgcctttatgcaccggacctgtgatcagcgcggcaaattcgccgttcagacaaccatcgcacgctcgcgccagcgtttccaccacataatgcccattttcaaccgctaactgccccgcagtgacaggtgcacgtagcgcgacaggaagtagcgttaatgtgcccgcagtttgcggttgtgcaggggagttgggggaataagggcggagggtgagcggcaaaccgagcatcgctgcccggttggtaaggagagtggcatcggcacaaacaaccagttcgaccggccactcacgctgtgcaagctggacaactaagtccgggccaatcccggcgggctcgccgggagtgatcacaacacgttgggttttaaccattagttgctcaggattttaacgtaggcgctggcacgttgttcctgcatccagcttgctgcttcttccgagaacttacggttcatcagcatgcggtatgcacgatctttctgcgcagcgtcggttttatcgacattacgggtatccagcagttcgattaaatgccagccgaatgaagagtgaaccggtgcactcatttgacctttgttcaggcgagtcagggcgtcacggaaggccggatcgaaaatatctggtgtagcccagccgagatcgccgccctggttagcagagcctggatcctgagagaactctttcgctgcggcagcaaaagtcgttttaccactcttgatatcagcagcaatctgttccagtttcacacgggcctgttcgtcagtcatgatcggcgacggtttcagcagaatatggcgagcatgaacttcggtcaccgagatatttttgctttcgccgcgcaggtcgttaactttcagaatatggaagccaacgccggaacgaatcgggccaacaatgtcgcctttcttcgcggtgcttaatgcctgggcgaagatcccgggcaactcctgaatacggccccagcccatctggccgccgttcagcgcctgctggtcggcagaatgagcaatcgccagcttaccgaaatcagcgccgttacgcgcctgatcgacaatggcgcgcgcctggctttccgcttcgttcacctgatcagaggtcgggttttccggcagcgggatcaggatgtggctcaggttcagctcagtgctggcgtcgttttggttacccacctgctgcgccagggattcgacttcctgcggcaggatggtgatgcgacgacgcacctcgttgttacgcacttcagagataatcatctctttgcggatctggttacgataggtgttgtagttcagtccatcgtaagccagacggctgcgcatctgatccagcgtcatgttgttctgtttcgcgatgttagcaatcgcctgatccagctgctcatcggagattttcactcccattttctgccccatctgcaggatgatttgatccatgatcaaacgttccatgatttggtggcgcagcgtcgcgtcatcaggaagttgctgccttgcctgagcagcgttcagttttaccgactgcattaatccatcaacgtcgctttccagcacgacgccgttattgacgacggctgcgactttatcgactacctggggggcagcgaaactggtattcgcgatcatggcgataccgagaagcagcgttttccagttcttcatactttttccatttcaattaaccgcactgcggattacgtggtaaatcaacaaatcacaaagtgttttgatacggcagaatgttcgaacgcagcatctcttgcgtacccagaccgtagttggagctcaggccgcgaagttcgatgttaaagccgattgcgttgtcatataccgcatgttgtttatcgttatcccaaccgttcagcttccgctcgtaaccgacgcgaattgcatagcagcaggagctgtattgcacacctaacatagagtcggcttgcttgttagcattggtgtcgtagtagtaggccccaacaatggaccaacgatcggcaattggccagctggcgacagcacctacctgcgaaataccattcttatattgctcagcagtggaatagtacttaggcagcgtagcctgaatatattccgggctggcgtaacggtaattcagctgtaccagacggtcttcatcccgacggtattcaatgctggagttactggtcgctacgttatccagacgtgtatcgtactgaatcccgccacgcaatccccaacgctcggagatacgccagtaagtatcgcctgcccacaccagtgaacccgttttgtcgtcattctcccatgttatgttgtcatcgccagtgcgagactccgtgaaatagtagatttgaccaacggaaatattaaaacgttcaacggcagcatcatcatatatgcgagatgtgacaccggtcgtcacctggttagcggaggcaatacggtcaagaccgccgtaagtccggtcccggaacaggccagagtagtcagattgcagcagagacgagtcgtagttatagatgtcgctctgatcgcgatacggcacgtacaaatactgcgcgcgcggttccagcgtttgggtataacccggagccagcatttccatatcgcgttcaaagaccattttgccgtcaactttgaattgcggcattacgcggttaacggattcgtccagcttggtcgtgtttctggagttataccagtcaagattggtttgctgataatgggttgccagcaacttcgcttcggtattgatgctgccccagttattagagagcggcaaattgatggtcggttccaggtgaacacgggttgcttcaggcatgtcgtctctggtgttaacaaagtgcactgcctggccgtaaatacgcgtatcaaacggaccaacatcattctggtagtaattaacgtctaactgcggctctgccgagtagctactggtgttctgttcgctgaaaacctggaactgcttggttgaaacggtggcattgaagttttgcaccgcatagccaacgctgaatttttgcgttgcgtagccgtcagtactggaaccgtacttgttatcgaaatcattgaagtagctaggatcgctgaccttggtgtagtcgacgttgaaacgccacacctgatccatgaccccggagtggttccagtagaataaccaacgacgtgaactgtcatcgttcgggtgttcatcttcatagactttatctgaaggcagatagtccagttccatcaagccagcgcccgcctgggagaggtagcggaattcgttctcccacatgatgttgccacgacgatgcatataatgcggcgtgatggtggcatccatatttggcgcgatgttccagtaatatggcaggtagaactcaaagtagttggtggtggtgtacttggcgttcgggatcaagaaaccagagcgacgtttgtcacccaccggcaactgcaaataggggctataaaagatcggtaccggacccaccttaaagcgggcgttccagatctccgcaacttgttcttcgcggtcatgaataatttcgctacctaccacgctccaggtgtcagaacccggcagacaggaggtaaagctaccgttatccagaatggtatagcggttttcgccacgttgtttcatcaggtccgctttaccgcgaccctggcgacccaccatctggtaatcaccttcccagacgttggtatctttggtgttcagattcgcccagcctttcggccctttgaggatcacctggttatcgtcgtaatggacattaccgagcgcatcaacggtacgtaccggctccggttgtcctggtgcctctttttgatggagctgcacttcgtcggcctgcagacggctgttaccctgcatgatatccacgctgccagtaaacacggcgtcatccgggtagtcccctttcgcgtggtcagcattgatagtcacgggtaagtcattggtatcgccctgtaccagaggacggtcatagcttggcacgcccaacatgcactgtgaggcgaggtcggctgccagtccctgttgactataaagggcggtggcaatcatggtggccaggagagtggggatacgttttttcatacgttgattttattgttccatcatcggtaacgttgcgcgtgacaaacggtcagagactaacgtactcgtcatctctacgctagtgttaatcctgtccgaatagcgtcagtggtgttaggcacggcattgaatgacaggtatgataatgcaaattataggcgatgtcccacaattgaccgcagccggaaaacggtaaaagcacctttatattgtgggagatagccctgatatccgtgtgtcgatttggggaatatatgcagtattggggaaaaatcattggcgtggccgtggccttactgatgggcggcggcttttggggcgtagtgttaggcctgttaattggccatatgtttgataaagcccgtagccgtaaaatggcgtggttcgccaaccagcgtgagcgtcaggcgctgttttttgccaccacttttgaagtgatggggcatttaaccaaatccaaaggtcgcgtcacggaggctgatattcatatcgccagccagttgatggaccgaatgaatcttcatggcgcttcccgtactgcggcgcaaaatgcgttccgggtgggaaaatcagacaattacccgctgcgcgaaaagatgcgccagtttcgcagtgtctgctttggtcgttttgacttaattcgtatgtttctggagatccagattcaggcggcgtttgctgatggttcactgcacccgaatgaacgggcggtgctgtatgtcattgcagaagaattagggatctcccgcgctcagtttgaccagtttttgcgcatgatgcagggcggtgcacagtttggcggcggttatcagcagcaaactggcggtggtaactggcagcaagcgcagcgtggcccaacgctggaagatgcctgtaatgtgctgggcgtgaagccgacggatgatgcgaccaccatcaaacgtgcctaccgtaagctgatgagtgaacaccatcccgataagctggtggcgaaaggtttgccgcctgagatgatggagatggcgaagcagaaagcgcaggaaattcagcaggcatatgagctgataaagcagcagaaagggtttaaatgaccctgtaaatgatgctgagtaactgcccacgattaaaggtggccgccctggcggtcacttctttgagaaaaggcgtttactcagaatggtggacaggctcaatgcacggtttacgggaggggttctgtaggttttatcgcgttgaccctgcttaaggttgagagctttacgacgagcggaattatatttttacgtcttaaaaataaaaaacacatacctgaatgagcgatttttgaaagtatatttattcagaacgcgcatcatgagtttttaactcaatgcgaggctattaccatgaaagtatcagttccaggcatgccggttacacttttaaatatgagcaagaacgatatttataagatggtgagcggggacaagatggacgtgaagatgaatatctttcaacgcttgtgggagacgttacgccatctgttctggtcagataaacagactgaggcttataaacttctgttcaatttcgtgaataaccagactggcaacatcaacgcctcagaatactttactggggctatcaacgagaatgagagagaaaagtttatcaatagcctggaattattcaataaacttaaaacatgcgcaaaaaatccggatgagttggtcgcaaagggcaatatgcgctgggtcgcccagaccttcggggatatcgagttaagtgtcacttttttcattgaaaagaataagatatgtactcagacgttgcagctgcataagggccaaggtaacttgggcgttgatcttagaaaggcttaccttcccggcgttgacatgagggattgttaccttggtaaaaaaacaatgaaaggtagcaatgatatcctttatgagagacctgggtggaatgctaacctgggcgtgctaccccggacggtgctaccccggacggtgctaacccggacggtgctaacctggacggtgctaccgtgaacggtgctacctccttatatgatgaggtaattattattaataaaatcccccccaaaaaaattgatactaaaggagttgctactgaagaagttgctactaaaaaagtactgctgaacaaattactgacaacgcaattattgaatgagccagaataagctaaggttgaaggggctggaacgccccttcaaccttagcagtagcgtgggatgatttcacaattagaaagacctgcatgatgagctagagaagaggctagtgacgcaaggcgtcgtgcaggacacggatcaccgagatgggcatcgccaaccagactgctaattagcccatgaataacaatcagaaaggaccataacagacccgttaaaatgaaatataagagacggtcaacgggtgaagaaaaagttcaaaaattcgctgtggagcaggaagggaattaccgaatggaaagcgtagccacacgcaacaactgaaagcagtttggcagaaacaaaaaatccccggactcggggatttatgtacaagaggcagcccttaggatgagggtataaacgtacaggaaaggttaaaaatccgctggcgctttaaacgtcatactattgccatacgccggatgggtaatcgtcaacatctctgcatgtagcaacaaacgtggtgccatcgctctcgcttctggtgatgcataaaaacgatcgccgagaatcggatgacccagcgccagcatatgcacacgcaattgatgcgaacgcccggtaatcggttttaacaccactcttgccgtgttatccgccgcatactccaccacttcatattccgtctgcgcaggtttacccgtttcgtaacagactttctgtttcgggcggtttggccagtcgcaaatcagcggcagatccaccagaccttctgcgggggatggatgcccccagacgcgggccacatactgctttttcggctcgcgctcgcggaactggcgttttaactcccgctccgcggctttggtcagcgccactacaatcacgccgctggtagccatatccagacgatgcaccgattctgcctgcggataatcacgctgaatgcgcgtcatcacgctgtctttgtgctcttccagacgacccggcactgacaacaaaccgctcggcttgttgaccaccataatatggtcatcctgatacaggataaccaaccagggttcctgcggtggattgtagttttccatccccattttcggctccgttactgatgcgttacaacgatcaaacgcagggcatccagacgccaacctgcctgatccaggctttccattacctgctgacggttgctctcaatggcggtcagttcgtcgtcacgaatgttcgggttcactgcacgcagagcttccagacgagacagctcggcagacagtttttcgtcggcttcgttacgcgctgcatcaatcaatgcacgggcagatttctcgatctgcgcttcacccagttgaaggatagcgtgaacatcctgctgcacggcgttaaccagtttgctgccggtgtgacggttaaccgcgttaagctggcggttaaaggtttcaaactctacctgcgccgccaggttgttgccgtttttatccagcagcatacgtaccggcgtcggtggcaggaagcggttgagctgcaactgcttcggagcctgggcttcaaccacataaatcagttccaccaacagcgtacctaccggcaacgctttgttttttaacagtgaaatcgtgctgctaccggtatcgccagaaaggatcagatccagaccgttgcggatcagcggatgctcccaggtaataaactgtgcatcttcacgcgccagcgccacttcacgatcaaaggtgatggtgatgccatcttccgacaggccagggaagtccggcaccagcatatgatcggacggcgtcagcacgatcatgttgtcgccgcgatcgtcctgattgataccgataatatcgaacaggttcatggcgaaggcgatcaggttggtatcgtcatcctgctcttcaatgctttctgccagtgcctgggctttttcgccaccgttggagtggatttccagcaggcggtcacgaccctgttccagctgtgctttcagcgcttcatgttgctcgcggcagtttttgatcagatcgtcaaagccttcggtttgatccggtgaagccagatagttaatcagatcgttgtatacgctatcgtaaatagtgcgtccggtcgggcaggtgtgctcaaatgcatccagaccttcgtgataccagcgcaccagcaccgactgagcggttttctccagataaggcacatggatctgaatatcgtgcgcctggccgatacgatccagacgaccaatacgctgctccagtagatccgggttgaatggcaggtcaaacatcaccatgtggctggcgaactggaagttacgtccttcagaaccgatttctgagcacagcagtacctgtgcgccggtgtcttcttcggcaaaccaggcggcagcgcggtcacgttcgataatcgacataccttcgtggaacaccgcagcgcgaataccttcacgttcgcgcagtacctgctccagttgcagcgcagtggcagctttggcgcagatcaccagcactttctgagagcgatggctggtcaggtagcccatcagccactcaacgcgcggatcgaagttccaccaggtggcgttatcaccttcaaattcctgataaatacgctccgggtagagcatatcgcgagcacgatcttccgcacttttacgtgcgcccataatgccggagactttaatagccgtctgatactgcgtcggtagcggcagcttaatggtgtgcagctcgcgtttcgggaatcctttcacaccgttacgcgtgttacggaacagcacgcggctggtgccgtggcgatccatcagcatcgaaaccagctcctgacgggcgctctgggcatcttcgctgtcgctgtttgctgcctgcaacagcggctcgatatcctgctcgccgatcatctcgccgagcatgttcagttcgtcattgctcagtttgttacctgccagcagcatggcaacggcgtccgcaaccggacgataatttttctgctcttcaacgaactgcgcaaaatcgtggaaacggttcgggtccagcagacgcagacgggcgaagtggctttccatccccagctgttccggggtcgcggtcagcagcagaacgcccggcacgtgctctgccagttgttcaatggcctgatattcacggcttggcgcatcttcgctccacaccaggtgatgcgcttcatcgaccaccagcaggtcccattcggcttcacagagatgttccaggcgctgtttgctacgacgggcaaaatccagcgagcaaatcaccagctgttcggtgtcaaacgggttgtaagcatcgtgctgagcttcggcataacgctcatcatcaaatagcgcaaagcgcaggttgaaacggcgcagcatttctaccagccactgatgctgtaaggtttccgggacgataattagcacacgttcagcagcgccagagagcagttgctgatgcaggatcatcccggcttcaatggttttccctaaacccacttcgtcagccagcaggacgcgcggcgcgtggcggcgaccaacatcatgagcgatgttgagctgatgcgggatcaggctggtacgctgaccgcgcaggccgctgtacggcatacggaactgttcgctggaatatttacgcgcgcgataacgcagcgcaaagcggtccatacggtcaatctgcccggcaaacagacggtcctgcggtttgctgaacaccagtttgctatcaaggaaaacttcacgcagggctacgccggactcttcagtatccaggcgagtaccgatataggtcagcaagccattttcttcttttacttcttcgacttgcatctgccagccgtcatggctggtaatggtatcaccagggttgaacatcacgcgggtcacgggggaatcactgcgtgcgtacagacggttttcaccagtagatgggaaaagtaaagtgacagttcgcgcatccaccgcgacaacggttccaagtcccaattcgctttctgtatcgctgatccagcgttgaccaagtgtaaaaggcatatgtgttcggctctatatctttaattgcaggcaataaccacccgctaccgtgcttatgaggtagtggtgttattcaggtccaggaatggaaagggcgctatggtactggatggcaaagcattcgtcacgcatcaaaatggtatctggcgaactcttttttttgctcaaaatagcccaagttgcccggtcataagtgtagcaaaattatcctcaataaaagggagtattccctccgccacgggttgtagctggcgggtcagatagtgttcgtaatccagtggtgaacgttggtagtccagcggctccgggccgttggtggtccatacgtacttaatggtgccgcgattctgatattgcaaggggcgaccacgcttttggttttcttcatcggcaaggcgagcggcgcgtacatgaggcggcacattacgctgatactcgctcagcggacggcgaaggcgtttacggtaaaccagtcgcgcatccagttcacccgccatcagtttgtcgatggtttcgcgtacatattcctgatatggctcgttgcggaagatgcgcaggtatagctcctgctgaaactgctgggccagcggcgtccagtcggtgcgcacggtttccagccctttaaacaccatccgctgcttgtcgccctcctgaatcagtccggcataacgctttttactgccggtatcggctccgcgaatggttggcatcagaaaacggcagaaatgggtttcatactccagttctaatgcgctggtcagccgttgtttttgcagcgtttccgcccaccaggcgttaacgtgctgcaccagtgcacgaccgattttcgccgcttcttcttccgaatgtgcgcctttcagccagacaaacgttgagtcggtatcgccgtagataacgtcgtagccctgtgcttcaatcaacgctttggtttgccgcatgatctgatgaccacgcatggtgatcgacgatgccagccgcggatcgaagaagcggcaggcggtggtgccgagcacgccataaaaggcattcatgatgattttcagcgcctgcgacagcggtttgttaccctggcgtttggcttcatcgcgcccgtgccagatgttagtcacaatctccggcaggcaatgtttttctcgcgagaaccaggcatcgagaaaaccttcggtactgtgctctggatcaggctgcgccatgccttccaccagcccgacgggatcaatcagaaaggtgcggatgatcgacgggtacaggcttttatagtccagcaccagcactgaatcataaagccctggccgtgaatccatcacgtagccgccagggctggcgtgcggcggcacttcgccgagattaggcgcgacataaccagcgcgatgcattcgcggaaaatagagatgaccaaatgccgccaccgaaccgccgtgtcggtccaccggcaggccgttcaccgttgcccgttcgagtaaaaatggcatgatttcagttttgtggaagatctgcgtcaccagctcgcaatctttcaggttataagttgccagcgcaggtttatcttcggcgaaacggcggtcaatttcgtccattcgatcccacgggttatcgatagattttccttcgcctaatagctcctgagcgacagtttccagcgagaatgaagagaaattccagaacgcggatttcagcgcctcgataccgtcgataattagccgacctttagcctgggcaaaaaagacgccgtttttaaagccgtgctcgcgccactccagctcgctattatcgcgcccaagacgcagcggaagacggtaacgctcggcatgtttttgcagcattcgcagatcgaactgcaccacgttccaaccgatgatcacatcaggatcgtagttggcaaaccaggcgttgagtttttccagcaactgcgggcggctggcgacgtattccagttcgaaatcaagcgaggaggcgtcgccattctccggccccagcatataaacgatgcgctgcccgcagccttccaggccgatgcagtacagctcaccgtggcgggtggtttcaatatctatagaaacccacttgagcggcggacgatagtcgggatgcggtttcagacgggcattaacgatagtgccattgtgcatatcaccctcgacccacaccggtgaggtgataaaccgctccatcagatagcgttctggcggacgcacatcggcctcgtagacggtaacgccaccttcacgcaggcgcttttcgtaattcatcaattggcgatgggcgcgacagtaaaggccatacaccggctggcggtgaaaatcctttaacgccagcggtgtcaggcgaaagccttgttcaccctgcaaaatatgctgagcgcggggaacctgatcggcgggaataaacgccacggactcttgcggtgcaagcgtaacctgcaacggcccgttgtccgtcgccagccagaaggagacttctgtcccttgcggggtgtcccgccagtgtcgggttaagataaaacctgcctgcgccacgctgaaaatccatcaaaaaaccaggcttgagtatagcctggtttcgtttgattggctgtggttttatacagtcattactgcccgtaatatgccttcgcgccatgcttacgcagatagtgtttatccagcagcgtttgctgcatatccggtaactgcggcgctaactgacggcagaatatccccatataagcgacctcttccagcacgatggcgttatgcaccgcatcttcggcatttttgccccatgcaaacgggccgtgggaatggaccagaacgccgggcatttgcgctgcatcgataccctgtttttcaaaggtttctacgatgacgttaccggtttcccactcatattcgccgttgatttctgcgtcggtcattttgcgggtgcagggaatggtgccgtagaaatagtcggcgtgggtggtgccggttgctggaatcgactgacccgcctgcgcccagatggtggcgtggcgcgagtgcgtatgcacaatgccgccaatggaggggaatgcctgatagagcagccggtgagttggcgtgtcggaggagggctttttcgtaccttcaaccacttcaccggtttcgatgctaaccacgaccatatcgtcagcggtcatgacgctgtaatcgacgccggaaggtttgatcacaaagacgccgcgctcgcgatcaacggcgctgacgttgccccatgtgagcgtgaccaggttgtgttttggcagcgccaggttggcttctaatacctggcgtttgagatcttctaacatgttgactccttcgtgccggatgcgctttgcttatccggcctacaaaatcgcagcgtgtaggcctgataagacgcgccagcgtcgcatcaggcgttgaatgccggatgcgctttgcttatccggcctacaaaatcgcagcgcgtaggcctgataagacgcgccagcgtcgcatcaggcgttgaatgccggatgcgctttgcttatccggcctacaaaatcgcagcgtgtaggccagataagacgcgtcagcgtcgcatcaggcgttacataccggatgcggctacttagcgacgaaacccgtaatacacttcgttccagcgcagcgcgtctttaaacgctggcaggcgtgtgtcgttatcaatcaccgtgatttcaatgtcgtgcatctcggcgaattggcgcatatcgttgaggttcagtgcatggctgaagacggtatggtgcgcgccaccagcgaggatccacgcttcggaagcagttggcagatccggttgcgctttccacagcgcattcgccaccggcagtttcggcagggagtgcggtgttttcaccgtgtcgatgcagttaaccagtagacggtaacgatcgccgagatcaatcaagctggcgacaatcgctgggccggtttgggtattgaagatcaggcgggcaggatcgtccttaccaccaataccgagatgctgaacgtcgaggatcggtttctcttctgcggcgatcgacgggcagacttccagcatatgggagccgagcaccaggtcattacctttctcgaagtgataggtgtagtcctccataaaggaggtgccgccctgcagaccggttgacatcaccttcatgatgcgaagcagggcggcagttttccagtcgccttcgcccgcaaagccgtaaccctgctgcatcagacgctgtacggccagaccaggaagctgtttcagaccgtgcaaatcttcaaaggtggtggtgaacgcgtggaagccaccttgttccaggaaacgcttcatccccagctcaatacgcgccgcttccagcacgttctgtcgttttttgccgtggatttgtgtggcaggcgtcatggtgtagcagctttcgtactcatcgaccagcgcgttaacatcgccgtcgctgatggagttcaccacctgcaccagatcgccaaccgcccaggtattgacggagaaaccgaacttgatctgtgcggcaactttatcgccatcggtgaccgccacttcacgcatgttatcgccaaatcggcagactttcagatgacgggtatcctgtttagagaccgcctgacgcatccaggagccgatacgctcatgggcttgtttatcctgccagtgaccggtaaccacggcatgttgctgacgcatacgcgcgccaatgaagccgaactcgcgaccgccatgtgcagtctggttcaggttcataaagtccatatcgatactgtcccacggcagcgccgcgttgaactgggtgtggaattgcagcaacggtttgttgagcatggtcaggccgttgatccacattttggccggggagaaggtgtgcagccacaccaccagaccagcgcaacgatcgtcgtaattcgcgtcgcggcaaatagcggtgatttcatccggcgtggtgcccagcggtttcaacaccagtttgcagggcagtttcgcttccgtattcagcgcattaacgacgtgctcggcatgttgggtgacctgacgcagggtttccgggccatacagatgctggctgccaatgacaaaccacacttcataattatcaaaaatcgtcattatcgtgtccttatagagtcgcaacggcctgggcagcctgtgccggggcggaagttggaagatagtgttgttcggcgctcatcgcccattgctgatagcggcgataaagctgttcaaagcgttgtgcctgctcgctgcacggttgcagggttttctctaccgcactggccattttttgctgagctgatgggatgtctgcgtgcactttcgcggcgacggcagcaaaaatcgccgcaccgagcgcacagcactggtcagaggcaacaatttgcagcgggcgattcagcacgtcgcagcaggcctgcataatgacctggtttttccgcgcgatgccgcccagtgccatcacgttattaacggcgatcccctgatcggtaaagcactccatgattgcgcgtgcgccaaaggcggtggcagcaatcaaaccgccgaacagcagcggagcgtcggtagcgaggttaagatcggtaatcacccctttcaggcgttggttagcgttcggtgtgcggcggccgttaaaccagtcgagcaccaccggcaggtgatccagagacggatttttggcccatgcttcggtcagcgccggaagcagttgtttctggctggcgttgatttgcgttttcagttccggatgctgggcggcaagctgttccagcggccagccgagtacgcgaccaaaccaggcgtagatatcaccaaacgccgattggcctgcttccagaccgataaatccaggcaccacgctgccatcaacctgaccgcaaatacctttaactgcccgctcgccaacgctctgtttgtcggcaatcagaatgtcgcaggtggaagtaccgataacttttaccagtgcgttaggctgtgcgcctgcgccaactgcgcccatatggcagtcaaacgcgccgccggaaatcaccacgctttcaggcaggccgagacgctgcgcccattccgggcataaggtgcccaccggaatatcggcagtccaagtgtcagtgaacagcggggaaggcaaatggcgattgaggatcgggtccagctcatcaaagaaactggctggcggcaggccgccccagctttcgtgccacagagatttatgcccggcgctgcaacgtccgcgacgaatatcctgcgggcgggtggtaccggaaagcagagctggcacccagtcgcacagctcaatccacgatgcggcagattgcgccacggcgctgtcctggcgagtcacatgcaggatttttgcccagaaccattcgctggaataaataccaccaatgtagcgggagtagtcaacgttgcccggcgcgtggcacaaacgggtaatctcttccgcttcttcaaccgcagtgtggtctttccacaatacgaacatcgcgttcgggttttcggcaaactccgggcgcagcgccagcacgtttccgtcggcatcaatcggtgcgggcgtcgagccggtactgtcaacgccaatcccgaccacagctgcgcgctgttcgacgctaagctctgcaagcacggttttcagtgccgcttccattgactcaatgtagtcacgcggatgatgacggaactggttattcggggcatcacaaaattgccctttctgccaacggggataccactctacgctggtggcgatctcttcaccggtagcgcagtccaccgccaaagctcgcacagaatcactgccaaaatcgaggccaattgcaatcgccatcgtttcactccatccaaaaaaacgggtatggagaaacagtagagagttgcgataaaaagcgtcaggtaggatccgctaatcttatggataaaaatgctatggcatagcaaagtgtgacgccgtgcaaataatcaatgtggacttttctgccgtgattatagacacttttgttacgcgtttttgtcatggctttggtcccgctttgttacagaatgcttttaataagcggggttaccggttgggttagcgagaagagccagtaaaagacgcagtgacggcaatgtctgatgcaatatggacaattggtttcttctctgaatggtgggagtatgaaaagtatggctgaagcgcaaaatgatcccctgctgccgggatactcgtttaacgcccatctggtggcgggtttaacgccgattgaggccaacggttatctcgatttttttatcgaccgaccgctgggaatgaaaggttatattctcaatctcaccattcgcggtcagggggtggtgaaaaatcagggacgagaatttgtctgccgaccgggtgatattttgctgttcccgccaggagagattcatcactacggtcgtcatccggaggctcgcgaatggtatcaccagtgggtttactttcgtccgcgcgcctactggcatgaatggcttaactggccgtcaatatttgccaatacgggtttctttcgcccggatgaagcgcaccagccgcatttcagcgacctgtttgggcaaatcattaacgccgggcaaggggaagggcgctattcggagctgctggcgataaatctgcttgagcaattgttactgcggcgcatggaagcgattaacgagtcgctccatccaccgatggataatcgggtacgcgaggcttgtcagtacatcagcgatcacctggcagacagcaattttgatatcgccagcgtcgcacagcatgtttgcttgtcgccgtcgcgtctgtcacatcttttccgccagcagttagggattagcgtcttaagctggcgcgaggaccaacgcattagtcaggcgaagctgcttttgagcactacccggatgcctatcgccaccgtcggtcgcaatgttggttttgacgatcaactctatttctcgcgagtatttaaaaaatgcaccggggccagcccgagcgagtttcgtgccggttgtgaagaaaaagtgaatgatgtagccgtcaagttgtcataattggtaacgaatcagacaattgacggcttgacggagtagcatagggtttgcagaatccctgcttcgtccatttgacaggcacattatgcaagcattgctggaacactttattacccaatccaccgtgtattcattgatggcggtggtgttggtggcctttctggagtcgctggcgctggtcggtttgattctacccggtacggtgctgatggcggggctgggagcgctgattggcagcggcgagttaagtttctggcacgcctggctggcagggattattggctgcttgatgggcgactggatttctttctggctgggttggcgttttaaaaagccgttgcatcgctggtcatttctgaagaaaaacaaagcactacttgataaaactgaacatgcgttgcatcaacacagcatgttcaccattctggtcggtcgttttgttggcccgacgcgtccgctggtgccaatggtggcgggaatgctggatctgccggtggctaaatttattacgccgaatattatcggctgcctgctgtggccgccgttttacttcctgccagggattctggcgggcgcggcgatcgatattcctgccggaatgcagagcggtgagtttaaatggttgctgctggcaacagcggtgtttttgtgggttggtggctggctgtgctggcggttatggcgcagcggtaaagcgactgaccgtttgagtcattatttgtcccgcggtcgtttgttgtggctgacgccgttgatttctgccatcggcgtggtggcgctggtggtgttaattcgccacccgttgatgccggtgtatatcgatattttgcgtaaagtggttggggtttaggagatagtcttgtgcgggttgcctgatgcgacgcttgccgcgtcttatcaggcctacaaaacgcactacccgtaggtcggataaggcgttcacgccgcatccgacagtgcatactaacccgtaatccccaatagtgccgaagcactcgccttaccgctcaacaactcattggtcataccctgccaggcgatgcgcccgtcggcgactactaccgagcgcgtggcgatccgcgccgcatcttccacgctgtgcgacaccatcaatagcgtcattttttgctgctggcagctcgtgctcaccagcgtcaacatctcctgacgtaacgccggatcgagcgcagagaacggttcatcgagcaataaaatcggctgttcgcgtaccagacaacgcgctaacgccactcgctgtcgctgaccgccggaaagctcgcccggtaaccgcgccattaaattatcaatccccatctggcgggcgatagcgtgcattttcccctgctgtaccgcgttcagtttcaatcccggatttagccccagcccgatgttctgtgcgaccgtcaggtggctgaacaggttgttctcctgaaacagcatcgacaccggacggcgtgacggcggcatagttgtgtgatctacgccatcgatagtcagcgaaccgctggctggcgtcagaaaaccggcgatcaaattcagcagggtacttttacccgcgccgcttggcccgaggatcgccacctgctcgccgcgttccaccgttaagctaaaacgcatcggcaaatggtggtaaagccaggtgatatcagtcagttttaacatttcgccccggtagtttttcaatcacggtaaacagcagaaaacagagcagcagcagaattaacgcggtgaccgcaccgtcctggctgcgataggagccaatttgctggtagagataaaacggcagggtgcggaaatcatcgttaccgaacaacgccaccacgccaaaatcaccaatcgacagcacgcatgcaaaggccagcgcctgcgccagtggacgtttcagggcgcgcagctccaccacttttaagcgtgaccagccttcaatccccagcgactgacataacatgctgtagcgggcggtgatatcgcgcatcgggttttccagcactttcagcgcataagggatcgccattaacgcattggtgaaaatcacaatgccgtcagcagattgtggcaggccgatagtgttgttgagcagtaaaaagaagccggtagccagcacaatccccggcatggcgaggatcaacatgccgctcatctccagcacctgacccgccagcattttctgccgcgcccgcagttcgcgactgctccatagcagcatcatggtcagcactacgcacaatacacctgccgccagcgcaatacgcaacgaggtccacagcgcctgccacagcaccggttgtgccagcacttccggcaactggcgatttaccccatcgacgatcaccgccagtaacggtggcagcaacagcagcagcgccagcacaattaacaccgtgtcgcaaatgcggctatgcagacgatcgtccgggtcgcgccagccttgcagcagcgtggtgccgggcgcaatggccttactcaatcgctgactcaacagcaccagcccgaggcagcacaccatctggagcagcgccagcattgccgcgcgggcaggatcgtagtcgtaactcagcgcctgatagattgccagctcgatagtggtcgcctgcggaccgccccccagcgatagcacggtggcgaagctggcgaaacagagcataaagataagcgcagcaaccggcgggatttgtcgccgtaaccacggccattcgacgaagcggaaaaaatgccagctacgcatcccaagctgggcggcaagttgacgctgttcgccggggatgttttccagtgcctggagtaataagcggctcgccatcggcagattaaaaaacacatgggccagcaaaataccttgcaggccgtagggcgaaaaggtccactccagaccgagcgattggcagagtgttgccagccagccctggcgaccatagacgctaagaatgccgaaaacagcgaccaacaccgggaggatcaaggtcattgcacacagacgcaacagcgccagccgacccggaaagcgcctgcgatagagcgcgcgggcgaggaatatcgcgggtatgacagagagcagtgccgagagaaacgcctgccagaaggagaagcgcaccacatgccacagatagctgtcctgccagactgccacccagtcatcctgcggcgcgttccaccacagggcgagaaacgccgccagcgcaaccgctaccaccagcgtggtggcgcttacacctggaattaaccagccgggaattaacggctgacggcgcgttgccattcgctaatccatgcctgacgttgtgccgccacttcggctggcgtgaactccaacgtggttgcgggtttggtcaatttttcaaaaccggcaggcagcgtgacgtttgccaccggatacatccagttgccggttgggatcgcattctggaaagccggagaaaccataaactggaggaatttttgcgccagctccggctgcttgctggcagcggtgcgggcggcgacttccacttgcagatagtgaccttcgctgaagttcgcggcggcgtagttatctttcttctcttcgagaatgtgataagccggagaggtggtgtaactcagtaccagatcgctttcaccttttaaaaacaggccgtaggcttcgctccagcctttggtgaccgtgaccgttttcttcgccagtttctgccaggcttgtggggcgtcatcgccatagactttttgcatccatagcaacagacccagccccggtgtactggtgcgcggatcctgataaatcacccgccagttttgatcgctctcaaccagttctttcaggctttgtggcgggtttttcagtttgttcttgtcataaacgaaggcgaagtagccataatcaaacggtacgaaagtgtcattattccagccgccgggaacgttaacggcatccgctgccacaccgcttttggcaaacagtccggttttactggcggcgtctaacaggttgttatccagccccagcaccacatcggctttactgtttttgccttccatccgtagacggttgagaagcgaaacgccatcttccagcgccaccagtttcagttcgcaattacagtcggcttcaaaggcttttttaaccaccggaccaggcccccagtcggcggcgaaggaatcgtaggtataaacagtcagaacgggtttagcgaaaacgggcgctgtgcacagcaacagcaggggcagacatttttttaacactttgcacctcaaaaaagagtggcaaaggacttgagaaggagcctcaaatcccttcgccggcgttatccggatcaggttcgacgggtattttctcagcgcacgcgtacgcgtggcaccccgttgagaacggcgttagtgtagtgattttgttatcaaccagcaatcatggatccggtggcgcaaaccacgctgatttaaaatcgaaccagccgagggtattcatgcgcaggccgcgcatactgcgttgcccctgaatgatcagccagtggtgcaataatggcaccatcgctttgctggcgaccagttgctggcaccagttcgccagattcatctcgccattgcgccagcgagcagcgtcggcttgccagtcaatgggaatgcaatgttgtagcagtggcacttcgcataaatgtgcgaaaacagagaagtccagcggcagggtaaagttggcgctgtttagccagatatcactttcgatctctcctgtatgccactgatcgtagtcgatctctttgattttcagcgtgacctggtgacttgccagaatctgctgcatgatcccggcaatcacccgatgctcactgtgatcctgataaaaggttagggtgaggctttccaggccagccggtttttcgctctttatggtgcgggcatggtgccaacgggggagcagtccataagccgggaaccacagttgctggtactgttcctcagcgaaatagaccagattagttggagaaagcacatagcttacccagtccctgacttgctgattcgccccgcgatgggtgcggctgtcgaacagtaaatagtagcaaccttcctccaggcggctttcaatctctttttcctcgccctgtggaccttttagcatcagccctccggctggctcgtcggcaatttccggcagaacccagacgttaacttcgtcgattaatgcccggtaaccgaagaagtcatcgaatgcctgaattttcagttgattggtgctgttgcgaatcaccgcatacggaccggtgccgatgggatggctggcaaagttactgagggtttcccattcgcgcggcaggatcatcgccggaacttgccccagcagtaacggtaaccagcggtccggttgcgtgagatggatatccagcgtccagggcgtcggcgacacaatgtcagcaatatgcgaatagagcggcagcgtattgattcgttttaaagaggcgatcacatcgtccatttccagttcacgaccatggtgaaaatggactcctggacgcaaaaagaaacgccagtgaagcggtgaaatttgctgccagtggtgggcgatgtctgcttccagttccccattttcctcatttatgcgcgttagcgaactgaagatttgccgggcgatatgggtttcggaacggcgcaatgcgctgccaggtagcagattacgcaacggacgatagtagagcacgcgcaggatgtgccgcccctggcggaagctgcggcccagatgagaaaccagcatttgccgcacagtcgctttgtcgccaaccaactgcaccagttgatcgatacgatcctgctccagcaggtcttccgcccgctgttgctgaagcgccagcccggtatagaggaatgtcagacgcgagcgtttaccgcgcccgacttccgcttcccacgtcagccagccgcgatcctgcatggtgttgagcagggtgcgcatatgacgacgcgagcagctcaataacgctgccagttcgttgagcgttgtgtcctgcgatttaccctcgcagcattgccacaggcggatgaactgttgttgcagacgagcagatggcataaaaggggaactcctgtgcaaaagacagcaattttattttccctatattaagtcaataattcctaacgatgaagcaagggggtgccccatgcgtcagttttatcagcactattttaccgcgacagcgaagttgtgctggttgcgttggttaagcgtcccacaacgattaaccatgcttgaaggactgatgcagtgggatgaccgcaattctgaaagttgacttgcctgcatcatgtgtgactgagtattggtgtaaaatcacccgccagcagattatacctgctggttttttttattctcgccgcgctaaaaagggaacgtatgatctggataatgacgatggctcgccgtatgaacggtgtttacgcggcatttatgctggtcgcttttatgatgggggtggccggggcgctacaggctcctacattgagcttatttctgagtcgtgaggttggcgcgcaacctttctggatcggcctcttttatacggtgaatgctattgctgggatcggcgtaagcctctggttggcaaaacgttctgacagtcagggcgatcggcgaaaactgattatattttgctgtttgatggctatcggcaatgcgctattgtttgcatttaatcgtcattatctgacgcttatcacctgtggtgtgcttctggcatctctggccaatacggcaatgccacagttatttgctctggcgcgggaatatgcggataactcggcgcgagaagtggtgatgtttagctcggtgatgcgtgcgcagctttctctggcatgggttatcggtccaccgttggcctttatgctggcgttgaattacggctttacggtgatgttttcgattgccgccgggatattcacactcagtctggtattgattgcatttatgcttccgtctgtggcgcgggtagaactgccgtcggaaaatgctttatcaatgcaaggtggctggcaggatagtaacgtacggatgttatttgtcgcctcgacgttaatgtggacctgcaacaccatgtacattattgatatgccgttgtggatcagtagcgagttaggattgccagacaaactggcgggtttcctgatggggacggcagctggactggaaataccagcaatgattctggctggctactatgtcaaacgttatggtaagcggcgaatgatggtcatagcagtggcggcaggagtactgttttacaccggattgattttctttaatagccgtatggcgttgatgacgctgcaactttttaacgctgtatttatcggcattgttgcgggtattgggatgctatggtttcaggatttaatgcctggaagagcgggggcagctaccaccttatttactaacagtatttctaccggggtaattctggctggcgttattcagggagcaattgcacaaagttgggggcactttgctgtctactgggtaattgcggttatttctgttgtcgcattatttttaaccgcaaaggttaaagacgtttgatgacgtggacgatagcggaaagcccggtcatttgaccgggcaaggggattaattcataaacgcaggttgttttgcttcataagcggcaatggcgtcgtcgtgctgcaaggtaagcccaatactgtccagaccgttcatcatgcagtggcggcggaaggcatcgatggtaaagcgataggttttctctcccgctttcacctcttgcgcttccagatccacgtcgaaatggatccccggattagctttcaccagcgcaaacagttcgtccacttctgcatcgcttaatttcaccggcagcagctggttgttaaagctattgccgtagaagatgtcagcaaaactcggcgcaatcaccactttaaaaccgtagtcggtcaatgcccagggcgcgtgctcacgcgaagagccacagccgaagttttctcgtgccagcaaaatggaagcgccctgatactgcgggaagttcagcacgaagtccgggtttggctgttggcctttttcatccagaaaacgccagtcgttaaacagatgcgcgccaaaacccgtacgggtcactttctgcaaaaactgtttcgggatgattgcatcggtatcgacattggcggcatccagcggaaccaccaggcctgtgtgtttgataaatttctctgccatggtgtgctccttatttaatgttgcgaatgtcggcgaaatgtccggtcacagcagcagcggcagccattgccgggctgaccagatgcgtgcgcccgccgcgcccctggcggccttcaaagttacggttgctggtggaggcacaacgttcgcccggattcagacggtcgttgttcatcgccagacacattgagcagccaggcaagcgccattcaaaaccggcttcaataaagattttatccagaccttccgcttccgcctgggcttttaccgggccagagccgggaaccaccagtgcctgcacgcctggcgcgacttttcgccctttggcgatctccgctgccgcgcgtaaatcttcaatgcgcgagttggtacaggaaccgataaacactttgtcgatagccacttcggtcagcggaatacccggtttcagccccatataggccagcgctttttctgccgacgcgcgttcaaccggatcggcaaacgaagccggatcgggaatattgtcgttcacggaaatcacctggccgggattggtgccccaggtgacctgcggtgaaatttcttctgcttgcagagtgacaacggtatcgaaagttgcgccttcgtcggtttgcagggttttccagtaggcaacggcgtcgtcgaaatctttgcctttcggcgcatgcagacggcctttgacatagttaaaggtggtttcgtccggtgcaaccagaccggcttttgcgcccatttcgattgccatattgcacagggtcatacgaccttccatgcttaaatcacggattgcttcgccgcaaaactccaccacatgcccggtgccgcctgcgctaccggttttaccgataattgccagcacgatatcttttgcggtaatgcccggcgcggctttgccctggacttcaattttcatggtttttgcgcggccctgtttcagggtttgcgttgccagtacgtgttcaacttcggaagtgccgataccaaaggccagtgcgccaaacgcgccgtgggtggcggtatgcgagtcgccgcagacaatggtcatccccggcaaggtgacgccctgttccggccccattacgtggacgatcccctgatacgggtgattcaggtcatacagttcgacgccaaattctttgcagtttttgatcagttcctgcatctggatacgcgccatttcaccgcaggcattaatgtctttggtctgggtagagacgttgtgatccatggtagcgaaggttttgcccggctgacgtaccgggcgaccgtgggcgcgcagaccatcgaacgcctgcggtgaggtcacttcatgcaccaggtggcggtcgatatataacagtggggtttcgttttcggcttcgtacacaacgtgagcgtcgaacaatttttcgtataacgtcttagccatgattacaccccttctgctacatagcgggcaatgatatcgcccatttcatcggtactaacggcggcagcgccacgggctaaatccccggtgcgaatgccttcttctaatgcgcggttaatggcgcgttcaatggcgcaagccgcatcatcggcatccaggctgtaacgcagcagcagtgccagcgaaaggatttgtgcaatcgggttggcgatgtttttgcctgcgatatctggtgccgagccgcccgccggttcatacagtccaaaaccttgctcgttcaggctggcggaaggcaacatccccatcgagccagtgatcattgcgcactcgtcagacagaatgtcgccaaacaggttggagcacagcagaacgtcaaactgtgatggatctttaatcagctgcatggtggcgttgtcgatgtacatatgcgccagttcgacatccgggtattccgtggcgatctcgttaacgatctcccgccataaaatagaggattgcagcacgttggctttatcgatcgacgtcactttgtggcgacgcttgcgagcagattcaaacgcgatgcgggcgatacgttcgatctcaaaacggtgatacacctcggtatcaaaggctttttcatattgtccgctaccttcgcggccttttggctgaccgaaatagatgccgccggtcagttcgcgcacacacaggatgtcgaagccgtttgcggcaatgtctgcacgcagcggacagaatgcttccagcccctgatacagttttgccgggcgcaggttgctgaataatttgaagtgcttacgcagaggcagcagcgcgccgcgttctggttgctggtctggtggtaaatgttcccacttcgggccgcctaccgagccaaacagcacggcatcggcttgctcacaaccttcaaccgtcgcaggcggcagtggttgcccgtggttatcaatggctgcgccgcctacatcgtaatggctggtggtgatgcgcatcgcaaagcggttgcgcacggcatccagcactttcagcgcctgggtcatcacttccggaccaataccgtcccccggcaatacggcaatatggtaattcttcgacatcacacggtttccttgttgttttcgttgtgttgagctttgcgttgcaactctttttcgacttctgcggcacgccagatattgttcagaacgtgcaccatggctttggcagatgactcgacaatatcggtagccaggccgacgccgtggaagcggcgaccgttgtagttagcgacgatatccacctgacccagcgcatctttaccgtggcctttggcggtcaggctgtatttcaccagttcgacgttatattcagtgatgcggttaattgcctgatagacggcatcgaccggaccgttaccgttggcggcttctgctttgacttcttcgccacaggccagtttgacggcggcggtggcgatatcgttagagccagactgcacgctgaagtaatccagacggaaatgctccggctcttcttgctgcttaccgatgaaggccagcgcctccagatcgtaatcaaacacctgaccttttttgtccgccagcttcaggaaagcatcgtacaaattgtctaaattatattcactttctttataccccatctcatccatgcgatgtttcaccgccgcacgccccgaacgagaggtcagattcagctggatttggttcagaccaatagattctggtgtcatgatttcgtagttttcgcggtttttcagcacgccatcctggtgtataccggaggagtgtgcgaatgcgccgctgccaacaatggctttgtttgccgggatcggcatattacaaatctggctaactaactggctggtgcgccatatctcctggtgattaatggcggtgtggacgttgagaatatccttacgaactttgatcgccatgatgacttcttccagggaacagtttccggcacgctcgccgatcccgttcattgcgccttccacctggcgtgcaccggcatgtaccgccgccagtgagtttccgaccgccaggcccaaatcgtcgtgggtatgtacggagataatggctttgtcgatgttaggcacgcgttcatacaggccgctgatgattccggcgaactcaaacggcatggtgtagcccacggtgtccggaatgttgatggtggtggcaccggcattaatcgccgcttcgaccactcgcgccagatcggcaatgggtgtacgcccggcatcttcgcaagaaaattcaacatcatcggtgtaattacgggcgcgtttcaccatatagatagcgcgttcgatcacctcgtccagcgtgctgcgcagcttggtggcgatgtgcattggcgaagtggcaataaaggtatgaatacggaaggcttcggcgactttcagggattcggccgccacgtcgatatctttttccacgcagcgagctaacgcacatacgcggctgtttttaacctggcgggcgatggtttgcaccgattcaaaatcgcccggcgaagagacggggaaaccgacttccatcacgtcaacacccatacgctcaagggccagcgcaatttgcagtttttctttcacactcaagcttgcctgtaacgcctgttcaccgtcgcgcaatgtggtatcgaaaataatgacttgctggctcatggtttgggtccttgtctcttttagagcgcctcgcttcgggcataaaaaaacccgcgcaatggcgcgggttttttgtttgactgcgtgctggcttaatgctggatgccgctcactcgtctaccgcgcaaagaagatgcgtttagtagtagtagaccgataaagcgaacgatgtgagtcattaaatcagctccagatgaatgcgatatgcttttagagttactggatacaaaaacggatgtcaaccctgacgcaataaaaacgtcccgccagcgtgagttctgcatccgtaaaattagctaattgtgctgcggtggttaaagtaagcgatattaatttctgcttaactaccgacgcttttcatcggttgacatatttcagcataaatttttgcatctaatcaacgaggaaaaaggggacaaaatgcacgcgttgcaaaacctatcctgatgatttgtattgaattatatgttttgcgattttttttgatattgatttggtgaatattattgatcaattaatgttaagaattaatgcattaaatatataaattaattattaaataagcacatttaatccattttgtagatgattgagtattcgcggtagttatgattagattgttttcgcaacaaaaacattatggattattatgctgtggtaaatgactcattccacggcaatggattctgtttttatcagaacccgtatctttatgttttccgaattttactcattttgctttttcttattttatatgcatgataaatcatattcttcaggattatttctctgcattccaataagggaaagggagttaagtgtgacagtggagttaagtatgccagaggtacaaacagatcatccagagacggcggagttaagcaaaccacagctacgcatggtcgatctcaacttattaaccgttttcgatgccgtgatgcaggagcaaaacattactcgtgccgctcatgttctgggaatgtcgcaacctgcggtcagtaacgctgttgcacgcctgaaggtgatgtttaatgacgagctttttgttcgttatggccgtggtattcaaccgactgctcgcgcatttcaactttttggttcagttcgtcaggcattgcaactagtacaaaatgaattgcctggttcaggttttgaacccgcgagcagtgaacgtgtatttcatctttgtgtttgcagcccgttagacagcattctgacctcgcagatttataatcacattgagcagattgcgccaaatatacatgttatgttcaagtcttcattaaatcagaacactgaacatcagctgcgttatcaggaaacggagtttgtgattagttatgaagacttccatcgtcctgaatttaccagcgtaccattatttaaagatgaaatggtgctggtagccagcaaaaatcatccaacaattaagggcccgttactgaaacatgatgtttataacgaacaacatgcggcggtttcgctcgatcgtttcgcgtcatttagtcaaccttggtatgacacggtagataagcaagccagtatcgcgtatcagggcatggcaatgatgagcgtacttagcgtggtgtcgcaaacgcatttggtcgctattgcgccgcgttggctggctgaagagttcgctgaatccttagaattacaggtattaccgctgccgttaaaacaaaacagcagaacctgttatctctcctggcatgaagctgccgggcgcgataaaggccatcagtggatggaagagcaattagtctcaatttgcaaacgctaactgattgcagaataggtcagacatgaatgtctggtttattctgcattttttattgaatgtagaattttattctgaatgtgtgggctctctattttaggattaattaaaaaaatagagaaattgctgtaagttgtgggattcagccgatttattatcaatttaatcctctgtaatggaggattttatcgtttcttttcacctttcctcctgtttattcttattaccccgtgtttatgtctctggctgccaattgcttaagcaagatcggacggttaatgtgttttacacattttttccgtcaaacagtgaggcaggccatggagatgttgtctggagccgagatggtcgtccgatcgcttatcgatcagggcgttaaacaagtattcggttatcccggaggcgcagtccttgatatttatgatgcattgcataccgtgggtggtattgatcatgtattagttcgtcatgagcaggcggcggtgcatatggccgatggcctggcgcgcgcgaccggggaagtcggcgtcgtgctggtaacgtcgggtccaggggcgaccaatgcgattactggcatcgccaccgcttatatggattccattccattagttgtcctttccgggcaggtagcgacctcgttgataggttacgatgcctttcaggagtgcgacatggtggggatttcgcgaccggtggttaaacacagttttctggttaagcaaacggaagacattccgcaggtgctgaaaaaggctttctggctggcggcaagtggtcgcccaggaccagtagtcgttgatttaccgaaagatattcttaatccggcgaacaaattaccctatgtctggccggagtcggtcagtatgcgttcttacaatcccactactaccggacataaagggcaaattaagcgtgctctgcaaacgctggtagcggcaaaaaaaccggttgtctacgtaggcggtggggcaatcacggcgggctgccatcagcagttgaaagaaacggtggaggcgttgaatctgcccgttgtttgctcattgatggggctgggggcgtttccggcaacgcatcgtcaggcactgggcatgctgggaatgcacggtacctacgaagccaatatgacgatgcataacgcggatgtgattttcgccgtcggggtacgatttgatgaccgaacgacgaacaatctggcaaagtactgcccaaatgccactgttctgcatatcgatattgatcctacttccatttctaaaaccgtgactgcggatatcccgattgtgggggatgctcgccaggtcctcgaacaaatgcttgaactcttgtcgcaagaatccgcccatcaaccactggatgagatccgcgactggtggcagcaaattgaacagtggcgcgctcgtcagtgcctgaaatatgacactcacagtgaaaagattaaaccgcaggcggtgatcgagactctttggcggttgacgaagggagacgcttacgtgacgtccgatgtcgggcagcaccagatgtttgctgcactttattatccattcgacaaaccgcgtcgctggatcaattccggtggcctcggcacgatgggttttggtttacctgcggcactgggcgtcaaaatggcgttgccagaagaaaccgtggtttgcgtcactggcgacggcagtattcagatgaacatccaggaactgtctaccgcgttgcaatacgagttgcccgtactggtggtgaatctcaataaccgctatctggggatggtgaagcagtggcaggacatgatctattccggccgtcattcacaatcttatatgcaatcgctacccgatttcgtccgtctggcggaagcctatgggcatgtcgggatccagatttctcatccgcatgagctggaaagcaaacttagcgaggcgctggaacaggtgcgcaataatcgcctggtgtttgttgatgttaccgtcgatggcagcgagcacgtctacccgatgcagattcgcgggggcggaatggatgaaatgtggttaagcaaaacggagagaacctgattatgcgccggatattatcagtcttactcgaaaatgaatcaggcgcgttatcccgcgtgattggccttttttcccagcgtggctacaacattgaaagcctgaccgttgcgccaaccgacgatccgacattatcgcgtatgaccatccagaccgtgggcgatgaaaaagtacttgagcagatcgaaaagcaattacacaaactggtcgatgtcttgcgcgtgagtgagttggggcagggcgcgcatgttgagcgggaaatcatgctggtgaaaattcaggccagcggttacgggcgtgacgaagtgaaacgtaatacggaaatattccgtgggcaaattatcgatgtcacaccctcgctttataccgttcaattagcaggcaccagcggtaagcttgatgcatttttagcatcgattcgcgatgtggcgaaaattgtggaggttgctcgctctggtgtggtcggactttcgcgcggcgataaaataatgcgttgagaatgatctcaatgcgcaatttacagcccaacatgtcacgttgggctttttttgcgaaatcagtgggaacctggaataaaagcagttgccgcagttaattttctgcgcttagatgttaatgaatttaacccataccagtacaatggctatggtttttacattttacgcaaggggcaattgtgaaactggatgaaatcgctcggctggcgggagtgtcgcggaccactgcaagctatgttattaacggcaaagcgaagcaataccgtgtgagcgacaaaaccgttgaaaaagtcatggctgtggtgcgtgagcacaattaccacccgaacgccgtggcagctgggcttcgtgctggacgcacacgttctattggtcttgtgatccccgatctggagaacaccagctatacccgcatcgctaactatcttgaacgccaggcgcggcaacggggttatcaactgctgattgcctgctcagaagatcagccagacaacgaaatgcggtgcattgagcaccttttacagcgtcaggttgatgccattattgtttcgacgtcgttgcctcctgagcatcctttttatcaacgctgggctaacgacccgttcccgattgtcgcgctggaccgcgccctcgatcgtgaacacttcaccagcgtggttggtgccgatcaggatgatgccgaaatgctggcggaagagttacgtaagtttcccgccgagacggtgctttatcttggtgcgctaccggagctttctgtcagcttcctgcgtgaacaaggtttccgtactgcctggaaagatgatccgcgcgaagtgcatttcctgtatgccaacagctatgagcgggaggcggctgcccagttattcgaaaaatggctggaaacgcatccgatgccgcaggcgctgttcacaacgtcgtttgcgttgttgcaaggagtgatggatgtcacgctgcgtcgcgacggcaaactgccttctgacctggcaattgccacctttggcgataacgaactgctcgacttcttacagtgtccggtgctggcagtggctcaacgtcaccgcgatgtcgcagagcgtgtgctggagattgtcctggcaagcctggacgaaccgcgtaagccaaaacctggtttaacgcgcattaaacgtaatctctatcgccgcggcgtgctcagccgtagctaagccgcgaacaaaaatacgcgccaggtgaatttccctctggcgcgtagagtacgggactggacatcaatatgcttaaagtaaataagactattcctgactattattgataaatgcttttaaacccgcccgttaattaactcaccagctgaaattcacaataattaagtgatatcgacagcgcgtttttgcattattttgttacatgcggcgatgaattgccgatttaacaaacacttttctttgcttttgcgcaaacccgctggcatcaagcgccacacagacgtaacaaggactgttaaccggggaagatatgtcctaaaatgccgctcgcgtcgcaaactgacactttatatttgctgtggaaaatagtgagtcattttaaaacggtgatgacgatgagggattttttcttacagctattcataacgttaatttgcttcgcacgttggacgtaaaataaacaacgctgatattagccgtaaacatcgggttttttacctcggtatgccttgtgactggcttgacaagcttttcctcagctccgtaaactcctttcagtgggaaattgtggggcaaagtgggaataaggggtgaggctggcatgttccggggagcaacgttagtcaatctcgacagcaaagggcgcttatcagtgcctacccgttatcgggaacagctgcttgagaacgctgccggtcaaatggtttgcaccattgacatttatcacccgtgcctgctgctttaccccctgcctgaatgggaaattatcgagcaaaaattatcgcgtctgtcgagcatgaacccggttgagcgccgtgtgcagcgcctactgttaggtcatgccagcgaatgtcagatggatggcgcaggtcgattgttaatcgcgccagtactgcggcaacatgccgggctgacaaaagaagtgatgctggttggacagttcaacaagtttgagctgtgggatgaaacaacctggcatcaacaggtcaaggaagatatcgacgcagagcagttggctaccggagacttatcggagcgactgcaggacttgtctctataaaatgatggaaaactataaacatactacggtgctgctggatgaagccgttaatggcctcaatatccgtcctgatggcatctacattgatgggacttttggtcgcggtggtcactcacgtctgatcctctcgcagcttggcgaagaggggcgtttgctggcgatcgatcgcgacccgcaggctatcgccgttgcgaagactattgatgatccgcgcttctccatcatccacggacctttctccgcgctgggcgaatacgttgccgagcgcgatcttatcggcaagatcgacggcattctcctcgatcttggcgtctcttcaccgcaacttgatgatgctgaacgtggcttttcctttatgcgcgatggtccgctggacatgcgtatggacccaacccgtgggcagtcagccgctgaatggctacaaaccgcagaagaagccgatatcgcctgggtattgaaaacctatggtgaagagcgttttgccaaacgcattgcccgcgccattgtcgagcgtaaccgcgaacagccgatgacccgcaccaaagaactggcggaagtcgtggctgctgcaacgccggtgaaagataagtttaaacatcccgcgacccgtaccttccaggcggtgcgcatttgggtaaacagtgaactggaggagatagagcaggcgctaaaaagctcgctcaacgtgctggccccgggtgggcggctttcgatcatcagcttccactcgctggaagaccgtattgtgaaacgttttatgcgtgaaaacagccgcggtccgcaagttccggcagggttaccgatgactgaagagcagctcaaaaaactgggtggccgtcagctgcgagcactaggcaagttaatgccgggcgaagaagaggtggctgagaaccctcgtgcccgtagttcagttctgcgtattgcagagaggacgaatgcatgatcagcagagtgacagaagctctaagcaaagttaaaggatcgatgggaagccacgagcgccatgcattgcctggtgttatcggtgacgatcttttgcgatttgggaagctgccactctgcctgttcatttgcattattttgacggcggtgactgtggtaaccacggcgcaccatacccgtttactgaccgctcagcgcgaacaactggtgctggagcgagatgctttagacattgaatggcgcaacctgatccttgaagagaatgcgctcggcgaccatagccgggtggaaaggatcgccacggaaaagctgcaaatgcagcatgttgatccgtcacaagaaaatatcgtagtgcaaaaataaggataaacgcgacgcatgaaagcagcggcgaaaacgcagaaaccaaaacgtcaggaagaacatgccaactttatcagttggcgttttgcgttgttatgcggctgtattctcctggcgctggcttttctgctcggacgcgtagcgtggttacaagttatctccccggatatgctggtgaaagagggcgacatgcgttctcttcgcgttcagcaagtttccacctcccgcggcatgattactgaccgttctggtcgcccgttagcggtgagcgtgccggtaaaagcgatttgggctgacccgaaagaagtgcatgacgctggcggtatcagcgtcggtgaccgctggaaggcgctggctaacgcgctcaatattccgctggatcagctttcagcccgcattaacgccaacccgaaagggcgctttatttatctggcgcgtcaggtgaaccctgacatggcggactacatcaaaaaactgaaactgccggggattcatctgcgtgaagagtctcgccgttactatccgtccggcgaagtgactgctcacctcatcggctttactaacgtcgatagtcaagggattgagggcgttgagaagagtttcgataaatggcttaccgggcagccgggtgagcgcattgtgcgtaaagaccgctatggtcgcgtaattgaagatatttcttctactgacagccaggcagcgcacaacctggcgctgagtattgatgaacgcctgcaggcgctggtttatcgcgaactgaacaacgcggtggcctttaacaaggctgaatctggtagcgccgtgctggtggatgtcaacaccggtgaagtgctggcgatggctaacagcccgtcatacaaccctaacaatctgagcggcacgccgaaagaggcgatgcgtaaccgtaccatcaccgacgtgtttgaaccgggctcaacggttaaaccgatggtggtaatgaccgcgttgcaacgtggcgtggtgcgggaaaactcggtactcaataccattccttatcgaattaacggccacgaaatcaaagacgtggcacgctacagcgaattaaccctgaccggggtattacagaagtcgagtaacgtcggtgtttccaagctggcgttagcgatgccgtcctcagcgttagtagatacttactcacgttttggactgggaaaagcgaccaatttggggttggtcggagaacgcagtggcttatatcctcaaaaacaacggtggtctgacatagagagggccaccttctctttcggctacgggctaatggtaacaccattacagttagcgcgagtctacgcaactatcggcagctacggcatttatcgcccactgtcgattaccaaagttgaccccccggttcccggtgaacgtgtcttcccggaatccattgtccgcactgtggtgcatatgatggaaagcgtggcgctaccaggcggcggcggcgtgaaggcggcgattaaaggctatcgtatcgccattaaaaccggtaccgcgaaaaaggtcgggccggacggtcgctacatcaataaatatattgcttataccgcaggcgttgcgcctgcgagtcagccgcgcttcgcgctggttgttgttatcaacgatccgcaggcgggtaaatactacggcggcgccgtttccgcgccggtctttggtgccatcatgggcggcgtattgcgtaccatgaacatcgagccggatgcgctgacaacgggcgataaaaatgaatttgtgattaatcaaggcgaggggacaggtggcagatcgtaatttgcgcgaccttcttgctccgtgggtgccagacgcaccttcgcgagcactgcgagagatgacactcgacagccgtgtggctgcggcgggcgatctctttgtagctgtagtaggtcatcaggcggacgggcgtcgatatatcccgcaggcgatagcgcaaggtgtggctgccattattgcagaggcgaaagatgaggcgaccgatggtgaaatccgtgaaatgcacggcgtaccggtcatctatctcagccagctcaacgagcgtttatctgcactggcgggccgcttttaccatgaaccctctgacaatttacgtctcgtgggcgtaacgggcaccaacggcaaaaccacgactacccagctgttggcgcagtggagccaactgcttggcgaaatcagcgcggtaatgggcaccgttggtaacggcctgctggggaaagtgatcccgacagaaaatacaaccggttcggcagtcgatgttcagcatgagctggcggggctggtggatcagggcgcgacgttttgcgcaatggaagtttcctcccacgggctggtacagcaccgtgtggcggcattgaaatttgcggcgtcggtctttaccaacttaagccgcgatcaccttgattatcatggtgatatggaacactacgaagccgcgaaatggctgctttattctgagcatcattgcggtcaggcgattattaacgccgacgatgaagtgggccgccgctggctggcaaaactgccggacgcggttgcggtatcaatggaagatcatattaatccgaactgtcacggacgctggttgaaagcgaccgaagtgaactatcacgacagcggtgcgacgattcgctttagctcaagttggggcgatggcgaaattgaaagccatctgatgggcgcttttaacgtcagcaacctgctgctcgcgctggcgacactgttggcactcggctatccactggctgatctgctgaaaaccgccgcgcgtctgcaaccggtttgcggacgtatggaagtgttcactgcgccaggcaaaccgacggtggtggtggattacgcgcatacgccggatgcactggaaaaagccttacaggcggcgcgtctgcactgtgcgggcaagctgtggtgtgtctttggctgtggtggcgatcgcgataaaggtaagcgtccactgatgggcgcaattgccgaagagtttgctgacgtggcggtggtgacggacgataacccgcgtaccgaagaaccgcgtgccatcatcaacgatattctggcgggaatgttagatgccggacatgccaaagtgatggaaggccgtgctgaagcggtgacttgcgccgttatgcaggctaaagagaatgatgtggtactggtcgcgggcaaaggccatgaagattaccagattgttggcaatcagcgtctggactactccgatcgcgtcacggtggcgcgtctgctgggggtgattgcatgattagcgtaacccttagccaacttaccgacattctcaacggtgaactgcaaggtgcagatatcacccttgatgctgtaaccactgatacccgaaaactgacgccgggctgcctgtttgttgccctgaaaggcgaacgttttgatgcccacgattttgccgaccaggcgaaagctggcggcgcaggcgcactactggttagccgtccgctggacatcgacctgccgcagttaatcgtcaaggatacgcgtctggcgtttggtgaactggctgcatgggttcgccagcaagttccggcgcgcgtggttgctctgacggggtcctccggcaaaacctccgttaaagagatgacggcggcgattttaagccagtgcggcaacacgctttatacggcaggcaatctcaacaacgacatcggtgtaccgatgacgctgttgcgcttaacgccggaatacgattacgcagttattgaacttggcgcgaaccatcagggcgaaatagcctggactgtgagtctgactcgcccggaagctgcgctggtcaacaacctggcagcggcgcatctggaaggttttggctcgcttgcgggtgtcgcgaaagcgaaaggtgaaatctttagcggcctgccggaaaacggtatcgccattatgaacgccgacaacaacgactggctgaactggcagagcgtaattggctcacgcaaagtgtggcgtttctcacccaatgccgccaacagcgatttcaccgccaccaatatccatgtgacctcgcacggtacggaatttaccctacaaaccccaaccggtagcgtcgatgttctgctgccgttgccggggcgtcacaatattgcgaatgcgctggcagccgctgcgctctccatgtccgtgggcgcaacgcttgatgctatcaaagcggggctggcaaatctgaaagctgttccaggccgtctgttccccatccaactggcagaaaaccagttgctgctcgacgactcctacaacgccaatgtcggttcaatgactgcagcagtccaggtactggctgaaatgccgggctaccgcgtgctggtggtgggcgatatggcggaactgggcgctgaaagcgaagcctgccatgtacaggtgggcgaggcggcaaaagctgctggtattgaccgcgtgttaagcgtgggtaaacaaagccatgctatcagcaccgccagcggcgttggcgaacattttgctgataaaactgcgttaattacgcgtcttaaattactgattgctgagcaacaggtaattacgattttagttaagggttcacgtagtgccgccatggaagaggtagtacgcgctttacaggagaatgggacatgttagtttggctggccgaacatttggtcaaatattattccggctttaacgtcttttcctatctgacgtttcgcgccatcgtcagcctgctgaccgcgctgttcatctcattgtggatgggcccgcgtatgattgctcatttgcaaaaactttcctttggtcaggtggtgcgtaacgacggtcctgaatcacacttcagcaagcgcggtacgccgaccatgggcgggattatgatcctgacggcgattgtgatctccgtactgctgtgggcttacccgtccaatccgtacgtctggtgcgtgttggtggtgctggtaggttacggtgttattggctttgttgatgattatcgcaaagtggtgcgtaaagacaccaaagggttgatcgctcgttggaagtatttctggatgtcggtcattgcgctgggtgtcgccttcgccctgtaccttgccggcaaagacacgcccgcaacgcagctggtggtcccattctttaaagatgtgatgccgcagctggggctgttctacattctgctggcttacttcgtcattgtgggtactggcaacgcggtaaacctgaccgatggtctcgacggcctggcaattatgccgaccgtatttgtcgccggtggttttgcgctggtggcgtgggcgaccggcaatatgaactttgccagctacttgcatataccgtatctgcgacacgccggggaactggttattgtctgtaccgcgatagtcggggcaggactgggcttcctgtggtttaacacctatccggcgcaggtctttatgggcgatgtaggttcgctggcgttaggtggtgcgttaggcattatcgccgtactgctacgtcaggaattcctgctggtgattatggggggcgtgttcgtggtagaaacgctttctgtcatcctgcaggtcggctcctttaaactgcgcggacaacgtattttccgcatggcaccgattcatcaccactatgaactgaaaggctggccggaaccgcgcgtcattgtgcgtttctggattatttcgctgatgctggttctgattggtctggcaacgctgaaggtacgttaatcatggctgattatcagggtaaaaatgtcgtcattatcggcctgggcctcaccgggctttcctgcgtggactttttcctcgctcgcggtgtgacgccgcgcgttatggatacgcgtatgacaccgcctggcctggataaattacccgaagccgtagaacgccacacgggcagtctgaatgatgaatggctgatggcggcagatctgattgtcgccagtcccggtattgcactggcgcatccatccttaagcgctgccgctgatgccggaatcgaaatcgttggcgatatcgagctgttctgtcgcgaagcacaagcaccgattgtggcgattaccggttctaacggcaaaagcacggtcaccacgctagtgggtgaaatggcgaaagcggcgggggttaacgttggtgtgggtggcaatattggcctgcctgcgttgatgctactggatgatgagtgtgaactgtacgtgctggaactgtcgagcttccagctggaaaccacctccagcttacaggcggtagcagcgaccattctgaacgtgactgaagatcatatggatcgctatccgtttggtttacaacagtatcgtgcagcaaaactgcgcatttacgaaaacgcgaaagtttgcgtggttaatgctgatgatgccttaacaatgccgattcgcggtgcggatgaacgctgcgtcagctttggcgtcaacatgggtgactatcacctgaatcatcagcagggcgaaacctggctgcgggttaaaggcgagaaagtgctgaatgtgaaagagatgaaactttccgggcagcataactacaccaatgcgctggcggcgctggcgctggcagatgctgcagggttaccgcgtgccagcagcctgaaagcgttaaccacattcactggtctgccgcatcgctttgaagttgtgctggagcataacggcgtacgttggattaacgattcgaaagcgaccaacgtcggcagtacggaagcggcgctgaatggcctgcacgtagacggcacactgcatttgttgctgggtggcgatggtaaatcggcggactttagcccactggcgcgttacctgaatggcgataacgtacgtctgtattgtttcggtcgtgacggcgcgcagctggcggcgctacgcccggaagtggcagaacaaaccgaaactatggaacaggcgatgcgcttgctggctccgcgtgttcagccgggcgatatggttctgctctccccagcctgtgccagccttgatcagttcaagaactttgaacaacgaggcaatgagtttgcccgtctggcgaaggagttaggttgatgcgtttatctctccctcgcctgaaaatgccgcgcctgccaggattcagtatcctggtctggatctccacggcgctaaagggctgggtgatgggctcgcgggaaaaagataccgacagcctgatcatgtacgatcgcaccttactgtggctgaccttcggcctcgcggcgattggctttatcatggtgacctcggcgtcaatgcccatagggcaacgcttaaccaacgatccgttcttcttcgcgaagcgtgatggtgtctatctgattttggcgtttattctggcgatcattacgctgcgtctgccgatggagttctggcaacgctacagtgccacgatgctgctcggatctatcatcctgctgatgatcgtcctggtagtgggtagctcggttaaaggggcatcgcgttggatcgatctcggtttgctgcgtatccagcctgcggagctgacaaaactgtcgctgttttgctatatcgccaactatctggtgcgtaaaggcgacgaagtacgtaataacctgcgcggcttcctgaaaccgatgggcgtgattctggtgttggcagtgttactgctggcacagccagaccttggtacggtggtggtgttgtttgtgactacgctggcgatgttgttcctggcgggagcgaaattgtggcagttcattgccattatcggtatgggcatttcagcggttgtgttgctgatactcgccgaaccgtaccgtatccgccgtgttaccgcattctggaacccgtgggaagatccctttggcagcggctatcagttaacgcaatcgctgatggcgtttggtcgcggcgaactttgggggcaaggtttaggtaactcggtacaaaaactggagtatctgccggaagcgcacactgactttattttcgccattatcggcgaagaactggggtatgtcggtgtggtgctggcacttttaatggtattcttcgtcgcttttcgcgcgatgtcgattggccgtaaagcattagaaattgaccaccgtttttccggttttctcgcctgttctattggcatctggtttagcttccaggcgctggttaacgtaggcgcggcggcggggatgttaccgaccaaaggtctgacattgccgctgatcagttacggtggttcgagcttactgattatgtcgacagccatcatgatgctgttgcgtattgattatgaaacgcgtctggagaaagcgcaggcgtttgtacgaggttcacgatgagtggtcaaggaaagcgattaatggtgatggcaggcggaaccggtggacatgtattcccgggactggcggttgcgcaccatctaatggctcagggttggcaagttcgctggctggggactgccgaccgtatggaagcggacttagtgccaaaacatggcatcgaaattgatttcattcgtatctctggtctgcgtggaaaaggtataaaagcactgatagctgccccgctgcgtatcttcaacgcctggcgtcaggcgcgggcgattatgaaagcgtacaaacctgacgtggtgctcggtatgggaggctacgtgtcaggtccaggtggtctggccgcgtggtcgttaggcattccggttgtacttcatgaacaaaacggtattgcgggcttaaccaataaatggctggcgaagattgccaccaaagtgatgcaggcgtttccaggtgctttccctaatgcggaagtagtgggtaacccggtgcgtaccgatgtgttggcgctgccgttgccgcagcaacgtttggctggacgtgaaggtccggttcgtgtgctggtagtgggtggttctcagggcgcacgcattcttaaccagacaatgccgcaggttgctgcgaaactgggtgattcagtcactatctggcatcagagcggcaaaggttcgcaacaatccgttgaacaggcgtatgccgaagcggggcaaccgcagcataaagtgacggaatttattgatgatatggcggcggcgtatgcgtgggcggatgtcgtcgtttgccgctccggtgcgttaacggtgagtgaaatcgccgcggcaggactaccggcgttgtttgtgccgtttcaacataaagaccgccagcaatactggaatgcgctaccgctggaaaaagcgggcgcagccaaaattatcgagcagccacagcttagcgtggatgctgtcgccaacaccctggccgggtggtcgcgagaaaccttattaaccatggcagaacgcgcccgcgctgcatccattccggatgccaccgagcgagtggcaaatgaagtgagccgggttgcccgggcgtaattgtagcgatgccttttgcatcgtatgaatttaagaagttaatggcgtaaagaatgaatacacaacaattggcaaaactgcgttccatcgtgcccgaaatgcgtcgcgttcggcacatacattttgtcggcattggtggtgccggtatgggcggtattgccgaagttctggccaatgaaggttatcagatcagtggttccgatttagcgccaaatccggtcacgcagcagttaatgaatctgggtgcgacgatttatttcaaccatcgcccggaaaacgtacgtgatgccagcgtggtcgttgtttccagcgcgatttctgccgataacccggaaattgtcgccgctcatgaagcgcgtattccggtgatccgtcgtgccgaaatgctggctgagttaatgcgttttcgtcatggcatcgccattgccggaacgcacggcaaaacgacaaccaccgcgatggtttccagcatctacgcagaagcggggctcgacccaaccttcgttaacggcgggctggtaaaagcggcgggggttcatgcgcgtttggggcatggtcggtacctgattgccgaagcagatgagagtgatgcatcgttcctgcatctgcaaccgatggtggcgattgtcaccaatatcgaagccgaccacatggatacctaccagggcgactttgagaatttaaaacagacttttattaattttctgcacaacctgccgttttacggtcgtgcggtgatgtgtgttgatgatccggtgatccgcgaattgttaccgcgagtggggcgtcagaccacgacttacggcttcagcgaagatgccgacgtgcgtgtagaagattatcagcagattggcccgcaggggcactttacgctgctgcgccaggacaaagagccgatgcgcgtcaccctgaatgcgccaggtcgtcataacgcgctgaacgccgcagctgcggttgcggttgctacggaagagggcattgacgacgaggctattttgcgggcgcttgaaagcttccaggggactggtcgccgttttgatttcctcggtgaattcccgctggagccagtgaatggtaaaagcggtacggcaatgctggtcgatgactacggccaccacccgacggaagtggacgccaccattaaagcggcgcgcgcaggctggccggataaaaacctggtaatgctgtttcagccgcaccgttttacccgtacgcgcgacctgtatgatgatttcgccaatgtgctgacgcaggttgataccctgttgatgctggaagtgtatccggctggcgaagcgccaattccgggagcggacagccgttcgctgtgtcgcacaattcgtggacgtgggaaaattgatcccattctggtgccggatccggcgcgggtagccgagatgctggcaccggtattaaccggtaacgacctgattctcgttcagggggctggtaatattggaaaaattgcccgttctttagctgaaatcaaactgaagccgcaaactccggaggaagaacaacatgactgataaaatcgcggtcctgttgggtgggacctccgctgagcgggaagtttctctgaattctggcgcagcggtgttagccggactgcgtgaaggcggtattgacgcgtatcctgtcgacccgaaagaagtcgacgtgacgcaactgaagtcgatgggctttcagaaagtgtttatcgcgctacacggtcgcggcggtgaagatggtacgctgcaggggatgctcgagctgatgggcttgccttataccggaagcggagtgatggcatctgcgctttcaatggataaactacgcagcaaacttctatggcaaggtgccggtttaccggtcgcgccgtgggtagcgttaacccgcgcagagtttgaaaaaggcctgagcgataagcagttagcagaaatttctgctctgggtttgccggttatcgttaagccgagccgcgaaggttccagtgtgggaatgtcaaaagtagtagcagaaaatgctctacaagatgcattaagattggcatttcagcacgatgaagaagtattgattgaaaaatggctaagtgggccggagttcacggttgcgatactcggtgaagaaattttaccgtcaatacgtattcaaccgtccggaaccttctatgattatgaggcgaagtatctctctgatgagacacagtatttctgccccgcaggtctggaagcgtcacaagaggccaatttgcaggcattagtgctgaaagcatggacgacgttaggttgcaaaggatggggacgtattgacgttatgctggacagcgatggacagttttatctgctggaagccaatacctcaccgggtatgaccagccacagcctggtgccgatggcggcacgtcaggcaggtatgagcttctcgcagttggtagtacgaattctggaactggcggactaatatgtcgcaggctgctctgaacacgcgaaacagcgaagaagaggtttcttctcgccgcaataatggaacgcgtctggcggggatccttttcctgctgaccgttttaacgacagtgttggtgagcggctgggtcgtgttgggctggatggaagatgcgcaacgcctgccgctctcaaagctggtgttgaccggtgaacgccattacacacgtaatgacgatatccggcagtcgatcctggcattgggtgagccgggtacctttatgacccaggatgtcaacatcatccagacgcaaatagaacaacgcctgccgtggattaagcaggtgagcgtcagaaagcagtggcctgatgaattgaagattcatctggttgaatatgtgccgattgcgcggtggaatgatcaacatatggtagacgcggaaggaaataccttcagcgtgccgccagaacgcaccagcaagcaggtgcttccaatgctgtatggcccggaaggcagcgccaatgaagtgttgcagggctatcgcgaaatggggcagatgctggcaaaggacagatttactctgaaggaagcggcgatgaccgcgcggcgttcctggcagttgacgctgaataacgatattaagctcaatcttggccggggcgatacgatgaaacgtttggctcgctttgtagaactttatccggttttacagcagcaggcgcaaaccgatggcaaacggattagctacgttgatttgcgttatgactctggagcggcagtaggctgggcgcccttgccgccagaggaatctactcagcaacaaaatcaggcacaggcagaacaacaatgatcaaggcgacggacagaaaactggtagtaggactggagattggtaccgcgaaggttgccgctttagtaggggaagttctgcccgacggtatggtcaatatcattggcgtgggcagctgcccgtcgcgtggtatggataaaggcggggtgaacgacctcgaatccgtggtcaagtgcgtacaacgcgccattgaccaggcagaattgatggcagattgtcagatctcttcggtatatctggcgctttctggtaagcacatcagctgccagaatgaaattggtatggtgcctatttctgaagaagaagtgacgcaagaagatgtggaaaacgtcgtccataccgcgaaatcggtgcgtgtgcgcgatgagcatcgtgtgctgcatgtgatcccgcaagagtatgcgattgactatcaggaagggatcaagaatccggtaggactttcgggcgtgcggatgcaggcaaaagtgcacctgatcacatgtcacaacgatatggcgaaaaacatcgtcaaagcggttgaacgttgtgggctgaaagttgaccaactgatatttgccggactggcatcaagttattcggtattgacggaagatgaacgtgaactgggtgtctgcgtcgtcgatatcggtggtggtacaatggatatcgccgtttataccggtggggcattgcgccacactaaggtaattccttatgctggcaatgtcgtgaccagtgatatcgcttacgcctttggcacgccgccaagcgacgccgaagcgattaaagttcgccacggttgtgcgctgggttccatcgttggaaaagatgagagcgtggaagtgccgagcgtaggtggtcgtccgccacggagtctgcaacgtcagacactggcagaggtgatcgagccgcgctataccgagctgctcaacctggtcaacgaagagatattgcagttgcaggaaaagcttcgccaacaaggggttaaacatcacctggcggcaggcattgtattaaccggtggcgcagcgcagatcgaaggtcttgcagcctgtgctcagcgcgtgtttcatacgcaagtgcgtatcggcgcgccgctgaacattaccggtttaacggattatgctcaggagccgtattattcgacggcggtgggattgcttcactatgggaaagagtcacatcttaacggtgaagctgaagtagaaaaacgtgttacagcatcagttggctcgtggatcaagcgactcaatagttggctgcgaaaagagttttaatttttatgaggccgacgatgattacggcctcaggcgacaggcacaaatcggagagaaactatgtttgaaccaatggaacttaccaatgacgcggtgattaaagtcatcggcgtcggcggcggcggcggtaatgctgttgaacacatggtgcgcgagcgcattgaaggtgttgaattcttcgcggtaaataccgatgcacaagcgctgcgtaaaacagcggttggacagacgattcaaatcggtagcggtatcaccaaaggactgggcgctggcgctaatccagaagttggccgcaatgcggctgatgaggatcgcgatgcattgcgtgcggcgctggaaggtgcagacatggtctttattgctgcgggtatgggtggtggtaccggtacaggtgcagcaccagtcgtcgctgaagtggcaaaagatttgggtatcctgaccgttgctgtcgtcactaagcctttcaactttgaaggcaagaagcgtatggcattcgcggagcaggggatcactgaactgtccaagcatgtggactctctgatcactatcccgaacgacaaactgctgaaagttctgggccgcggtatctccctgctggatgcgtttggcgcagcgaacgatgtactgaaaggcgctgtgcaaggtatcgctgaactgattactcgtccgggtttgatgaacgtggactttgcagacgtacgcaccgtaatgtctgagatgggctacgcaatgatgggttctggcgtggcgagcggtgaagaccgtgcggaagaagctgctgaaatggctatctcttctccgctgctggaagatatcgacctgtctggcgcgcgcggcgtgctggttaacatcacggcgggcttcgacctgcgtctggatgagttcgaaacggtaggtaacaccatccgtgcatttgcttccgacaacgcgactgtggttatcggtacttctcttgacccggatatgaatgacgagctgcgcgtaaccgttgttgcgacaggtatcggcatggacaaacgtcctgaaatcactctggtgaccaataagcaggttcagcagccagtgatggatcgctaccagcagcatgggatggctccgctgacccaggagcagaagccggttgctaaagtcgtgaatgacaatgcgccgcaaactgcgaaagagccggattatctggatatcccagcattcctgcgtaagcaagctgattaagaattgactggaatttgggtttcgaggctctttgtgctaaactggcccgccgaatgtatagtacacttcggttggataggtaatttggcgagataatacgatgatcaaacaaaggacacttaaacgtatcgttcaggcgacgggtgtcggtttacataccggcaagaaagtcaccctgacgttacgccctgcgccggccaacaccggggtcatctatcgtcgcaccgacttgaatccaccggtagatttcccggccgatgccaaatctgtgcgtgataccatgctctgtacgtgtctggtcaacgagcatgatgtacggatttcaaccgtagagcacctcaatgctgctctcgcgggcttgggcatcgataacattgttatcgaagttaacgcgccggaaatcccgatcatggacggcagcgccgctccgtttgtatacctgctgcttgacgccggtatcgacgagttgaactgcgccaaaaaatttgttcgcatcaaagagactgttcgtgtcgaagatggcgataagtgggctgaatttaagccgtacaatggtttttcgctggatttcaccatcgattttaaccatccggctattgattccagcaaccagcgctatgcgatgaacttctccgctgatgcgtttatgcgccagatcagccgtgcgcgtacgttcggtttcatgcgtgatatcgaatatctgcagtcccgtggtttgtgcctgggcggcagcttcgattgtgccatcgttgttgacgattatcgcgtactgaacgaagacggcctgcgttttgaagacgaatttgtgcgtcacaaaatgctcgatgcgatcggtgacttgttcatgtgtggtcacaatattattggtgcatttaccgcttataaatccggtcatgcactgaataacaaactgctgcaggctgtcctggcgaaacaggaagcctgggaatatgtgaccttccaggacgacgcagaactgccgttggccttcaaagcgccttcagctgtactggcataacgacatttatactgtcgtataaaattcgactggcaaatctggcactctctccggccaggtgaaccagtcgtttttttttgaattttataagagctataaaaaacggtgcgaacgctgttttcttaagcacttttccgcacaacttatcttcattcgtgctgtggactgcaggctttaatgataagatttgtgcgctaaatacgtttgaatatgatcgggatggcaataacgtgagtggaatactgacgcgctggcgacagtttggtaaacgctacttctggccgcatctcttattagggatggttgcggcgagtttaggtttgcctgcgctcagcaacgccgccgaaccaaacgcgcccgcaaaagcgacaacccgcaaccacgagccttcagccaaagttaactttggtcaattggccttgctggaagcgaacacacgccgcccgaattcgaactattccgttgattactggcatcaacatgccattcgcacggtaatccgtcatctttctttcgcaatggcaccgcaaacactgcccgttgctgaagaatctttgcctcttcaggcgcaacatcttgcattactggatacgctcagcgcgctgctgacccaggaaggcacgccgtctgaaaagggttatcgcattgattatgcgcattttaccccacaagcaaaattcagcacgcccgtctggataagccaggcgcaaggcatccgtgctggccctcaacgcctcacctaacaacaataaacctttacttcattttattaactccgcaacgcggggcgtttgagattttattatgctaatcaaattgttaactaaagttttcggtagtcgtaacgatcgcaccctgcgccggatgcgcaaagtggtcaacatcatcaatgccatggaaccggagatggaaaaactctccgacgaagaactgaaagggaaaaccgcagagtttcgtgcacgtctggaaaaaggcgaagtgctggaaaatctgatcccggaagctttcgccgtggtacgtgaggcaagtaagcgcgtctttggtatgcgtcacttcgacgttcagttactcggcggtatggttcttaacgaacgctgcatcgccgaaatgcgtaccggtgaaggaaaaaccctgaccgcaacgctgcctgcttacctgaacgcactaaccggtaaaggcgtgcacgtagttaccgtcaacgactacctggcgcaacgtgacgccgaaaacaaccgtccgctgtttgaattccttggcctgactgtcggtatcaacctgccgggcatgccagcaccggcaaagcgcgaagcttacgcagctgacatcacttacggtacgaacaacgaatacggctttgactacctgcgcgacaacatggcgttcagccctgaagaacgtgtacagcgtaaactgcactatgcgctggtggacgaagtggactccatcctgatcgatgaagcgcgtacaccgctgatcatttccggcccggcagaagacagctcggaaatgtataaacgcgtgaataaaattattccgcacctgatccgtcaggaaaaagaagactccgaaaccttccagggcgaaggccacttctcggtggacgaaaaatctcgccaggtgaacctgaccgaacgtggtctggtgctgattgaagaactgctggtgaaagagggcatcatggatgaaggggagtctctgtactctccggccaacatcatgctgatgcaccacgtaacggcggcgctgcgcgctcatgcgctgtttacccgtgacgtcgactacatcgttaaagatggtgaagttatcatcgttgacgaacacaccggtcgtaccatgcagggccgtcgctggtccgatggtctgcaccaggctgtggaagcgaaagaaggtgtgcagatccagaacgaaaaccaaacgctggcttcgatcaccttccagaactacttccgtctgtatgaaaaactggcggggatgaccggtactgctgataccgaagctttcgaatttagctcaatctacaagctggataccgtcgttgttccgaccaaccgtccaatgattcgtaaagatctgccggacctggtctacatgactgaagcggaaaaaattcaggcgatcattgaagatatcaaagaacgtactgcgaaaggccagccggtgctggtgggtactatctccatcgaaaaatcggagctggtgtcaaacgaactgaccaaagccggtattaagcacaacgtcctgaacgccaaattccacgccaacgaagcggcgattgttgctcaggcaggttatccggctgcggtgactatcgcgaccaatatggcgggtcgtggtacagatattgtgctcggtggtagctggcaggcagaagttgccgcgctggaaaatccgaccgcagagcaaattgaaaaaattaaagccgactggcaggtacgtcacgatgcggtactggaagcaggtggcctgcatatcatcggtaccgagcgtcacgaatcccgtcgtatcgataaccagttgcgcggtcgttctggtcgtcagggggatgctggttcttcccgtttctacctgtcgatggaagatgcgctgatgcgtatttttgcttccgaccgagtatccggcatgatgcgtaaactgggtatgaagccaggcgaagccattgaacacccgtgggtgactaaagcgattgccaacgcccagcgtaaagttgaaagccgtaacttcgacattcgtaagcaactgctggaatatgatgacgtggctaacgatcagcgtcgcgccatttactcccagcgtaacgaactgttggatgtcagcgatgtgagcgaaaccattaacagcattcgtgaagatgtgttcaaagcgaccattgatgcctacattccaccacagtcgctggaagaaatgtgggatattccggggctgcaggaacgtctgaagaacgatttcgacctcgatttgccaattgccgagtggctggataaagaaccagaactgcatgaagagacgctgcgtgagcgcattctggcgcagtccatcgaagtgtatcagcgtaaagaagaagtggttggtgctgagatgatgcgtcacttcgagaaaggcgtcatgctgcaaacgcttgactccctgtggaaagagcacctggcagcgatggactatctgcgtcagggtatccacctgcgtggctacgcacagaaagatccgaagcaggaatacaaacgtgaatcgttctccatgtttgcagcgatgctggagtcgttgaaatatgaagttatcagtacgctgagcaaagttcaggtacgtatgcctgaagaggttgaggagctggaacaacagcgtcgtatggaagccgagcgtttagcgcaaatgcagcagcttagccatcaggatgacgactctgcagccgcagctgcactggcggcgcaaaccggagagcgcaaagtaggacgtaacgatccttgcccgtgcggttctggtaaaaaatacaagcagtgccatggccgcctgcaataaaagctaactgttgaagtaaaaggcgcaggattctgcgccttttttataggtttaagacaatgaaaaagctgcaaattgcggtaggtattattcgcaacgagaacaatgaaatctttataacgcgtcgcgcagcagatgcgcacatggcgaataaactggagtttcccggcggtaaaattgaaatgggtgaaacgccggaacaggcggtggtgcgtgaacttcaggaagaagtcgggattaccccccaacatttttcgctatttgaaaaactggaatatgaattcccggacaggcatataacactgtggttttggctggtcgaacgctgggaaggggagccgtggggtaaagaagggcaacccggtgagtggatgtcgctggtcggtcttaatgccgatgattttccgccagccaatgaaccggtaattgcgaagcttaaacgtctgtaggtcagataaggcgttttcgccgcatccgacattcgcacacgatgcctgatgcgacgctggcgcgtcttatcaggcctaaagggatttctaactcattgataaatttgtttttgtaggtcggataaggcgttcacgccgcatccgacatttgcacaagatgcctgatgcgacgctgtccgcgtcttatcaggcctacgtgcggcatcagacaaatgtcactgctttggttcttcgctccagtcatcgctttcggaaagatcgccactgctggggattcgtttttcttcagcagcccattctccgaggtcgatcagctgacaacgtttggagcaaaatggccgaaacgggctgatttcaccccacaccaccgttttcccgcaggttgggcaattcaccgtaatagtttctgacatttttactccttagcaacaggccagttcgaaatccagacgttccggtacctgtccgttttcagtgtccagcggcataaaacgaatggcaaaacggctcttatgtccggaaatttgcggataaagctgtgaatcgagcgacagattcaggcgcagcaagtcggcatcgccaccgttatcctgataaaaaccattcaggctggtttgtttacggaagggggccgactggcgaattaaatccagcaccatggtaagtgcctgggtgagcgggttcaggctggcaatccaggtttctacctggctgtcgcgctgcgcctggggtagatgcagccaaatgtgcaatgtaggtaaatcaaagctgcaacagccgcctgggatgctcagtcgctgacgcaccagagcaatcaaacgatcttcacgcagaaattgcccgatacgcggcgcggaaattaatacgctccccgccgcttttaactgctgaattaatgcttcaatacggctctggtccacgccaggcacgccaatccaggtctggagtttacgttgctgccggtcaagttctttcaacagctcagtgcggacttcgccgcgctcgaaaacatccagtaattcactgacattacggaagaaatgcagcgcgccagcgtggtcaacgatgggtaaattaacggtgagttgctgaatcaaaaactcaatgcgcagccatgtacgcattttttcatttagtggatgttcaaaaaggacctgggtctgcattacggtttttcctgtgagacaaactgcgacgcaagctgcaaatagtgtgcgtgcaggcgggcaacatccgatgcgatagcatccggtgcgccgttattatcaatgacgtcatctgccacggcaaggcgggcttcgcgcgttgcctgagcagcaaggatttgttcgacatgctcgcgagttacatcatcgcgctgcatggtgcgcttaagttgcgtttctgggctgacatccaccacaagcactcgattcgcttttttatacagtgagttttctaccagcaatggcacaacccacagtacatagggggaagtagcttgctggatctggtgttgcgtctcttgctgaatcagcggatgcagcagggcgttaagccagtttttctcttccgggttggcgaagatccgctcgcgcaaggcccggcgctgcaatgttccatcagcagcaatcatgttagcgccaaagtgatcagcaatggcatgtagcgcaggtgcacctggttcaaccacctgacgcgcaataatatcggcatcaatgacgttaattccgagatcagcaaacgcattggcaacggtactcttgccactgccaatgcctcccgttaaggcaactatatacctcataatttatattcccgggaattcatcatgattatcaaaacgttaaaaatgagtgcacgaaagcgaaattgatgaaacgttcgctcactatttaccaggtaaatttatgggattgtagcgtaaaaaaagacaatttcgcagtcttgcgccgcattgattagtgcgtatgatagcgtcactggagttgcgctcttacccttatagccattaaccccaggaatccgcacatgcgtattgaagaagatctgaagttaggttttaaagacgttctcatccgccctaaacgctccactcttaaaagccgttccgatgttgaactggaacgtcaattcaccttcaaacattcaggtcagagctggtccggcgtgccgattatcgccgcaaatatggacaccgtaggcacattttctatggcctctgcgctggcttcttttgatattttgactgctgtgcataaacactattctgtcgaagagtggcaagcgtttatcaacaattcttccgctgatgtgctgaaacatgtgatggtttctaccggtacgtctgatgcggatttcgaaaaaactaaacagattctcgacctgaacccggcattaaacttcgtttgtattgacgtggcgaatggttattccgaacacttcgtgcagttcgttgcgaaagcgcgtgaagcgtggccgaccaaaaccatttgtgctggtaacgtagtgactggtgaaatgtgtgaggagcttatcctctcaggtgccgatatcgttaaagttggcattggcccaggttctgtttgtacaactcgcgtcaaaacaggcgtcggttatccgcaactttctgcggtaatcgaatgtgccgatgctgcgcacggtctgggcggaatgatcgtcagcgatggtggctgcaccacgccgggcgatgtggcgaaagcctttggcggcggtgccgatttcgtcatgcttggcggcatgctggcgggccacgaagagagcggcggtcgcatcgttgaggagaacggcgagaaatttatgctgttctacggcatgagctccgagtctgcgatgaaacgtcacgttggcggcgttgcggaatatcgcgcagcagaaggtaaaaccgttaagctgccgctgcgaggcccggttgaaaataccgcgcgagatattttgggcggcctgcgttcagcttgtacatacgttggggcttcacgcctgaaagagctgaccaagcgcaccacgtttattcgtgtgcaggaacaagaaaaccgcatcttcaacaacctgtaatctcccaacgctggcgtggagcaacacgccagcgttatcccatcccactcatcgcatcgcctaaatggaaaattggcagatacattgccaccaccagcgtaccaataattcctcccgttatgatcagcaacgccggttccagtaaggctgcgaggttatccgccagcgccattgtgttttcccgatgatgatgggcgaggttgtctaacatgagatccagagagccggatgcctctcctgttctcactaattgcaaacagagcgggctaaactcaccggtattttttagcgccagccagatgggttgaccgttactgatatcgtgctggatttgtgtcagaagttgcacccagtacgggcagcgcattgtttctctgacgctctctacgccctgtaaaaaagtaatgcctgcactttgtgtcagcgccagaatcgtaaagatctgcgtgagtttttgtccccgcatcagtgaacccataatcgggatgcgtaacagcaatttctgccgcactataagccaggtcggtcggcgcatcagcaacttattggctatcgccagcagaaagccgaacaacaccagcagccagctccattcgccactaaagtctgccagcgtcatgatcccctgcgttagtgccggtagtggggtgttgaaggtcttatagatagcggcaaactccggcagaacaaaatgcagcattgccacaaccaccatgattgccatcgctaaaatgatgatgggataacgtaacgctgatttcactttgtcggtcaactgacgctgggctttttgctgacgcgccagttcaaagcagcattcatccagcttaccggtcagttcacccgtgcggatcatcgcctgatagagcggcggaaatacctctgaccagggtaataaggcattggaaaaagcaatgccctgttcgagatcgtgcgccagcgattgcagcaacgcttgccattgcttactgggatgctgttccgccagcagagccagcccttcagaaagcgttaaccctgctttgagtagcgtcgccagttgatgaatgacttccgcgcttttatctcctcgccactgcgcagaattgatggcgattcgcttcaggcttagtggggtaaccatctgttgctgtagtgccataagcagtaaagtacggctctctgcccatagcatcccatcttgcgcattgccgtcgccggttatgccatgccagcgccagagttgcttactcgccatgcggcatccccagtacgcggattaactcttcaaaggtggttaagccttgctctacggccaggcagccgttttcaaaaagcgtacgcatacccgcctgtcgtgcgtgcgtttccagcgattcaacgtcggtattagcggaaataagctgacgaatgaccggcgttatgggcagaacttcaaataaggccgtacgaccataaaaaccgtggtagcaatgtacacaaccgggtgcctgccagtggggcagcggcgatggccatacattgtctggaatgtggatgggctccccttgctgccggcgacaatgtgggcaaagtttgcgtaccagacgctgggctattaccagcgtaagcgccgatgatagcatccagcgggcgacccccatttgctgtaaacgtaccagcgtttcgcaggtggaattagtgtgtagggtagacaacaccaggtgaccagtttgcgccgctttaatagcgatctctgctgtttcgccatcgcggatctctccgatcatgatgacgtcaggatcctggcgcaataacgcacgcaaaacgccctgaaaggtgagtccggcacgcggatggatttgcgtctggtttagtccggctatggggatctcaactggatcttcgacgctacaaatattaatgtcagcggtattcagcttttgcagggcactataaagcgtgaccgttttgccgctgccggtagggccagttaccagcaccagtccctgtggttgttgcaaggcatgagcaaagtccgccagttgtaacggctgcattccaagcgtgttgacatccagtgcctgacccacctgctgtaacaaccttaataccaccttttcaccaccccgacatggtaaggtcgcaatacgaaatgagacggcgtttcctgccagttcgacagtgaattgcccgtcctgcggcaggcgatgttccgcaatatccaggtttcccagcacttttaatctggcggttaatgcgactccggcatccggtgaaacatccggtaaaggatgcaatacgccgtcgatacgcaagcggatgcggtaggcattgtccgctggttcgatatgaatatcagacgcgcgttgttccagcgcagattgtaacgttcgagttagcaactctgctttgggctgatgcttctcctgaacagctacgggcaatgtctgttgtgtgcgactggcgtgaccttccatttgttggcgcgtccagcaggtgatctcaatacgtttggtggtagcgaaatgcaatgcgtccagtagctcatgcgaaggtgcatcgactaccgcaacatgaaccacctcttcgctggcatccagcaagactccatgataacgcagacacagggcagtgagctgtggaatattcattgccgctccttagttggcgtcatcaaagcggaagacatcttcgcaggcttgctgcaatgcgctgtcactttgaatattgcagttgcgcgtccagccggtgacgccgtttgcgttatcccaacccggtgtcatgacgacgcttagcccattgagactttcttgcccggtcagcgacaccacgccctttgccacactcatggctgaaacatagcgggtggtggtaggcgagggaatgccattgctgccaccgtcgcaggtatctaatccaccatgttccagcgcgcacaactctacggcggtacggtaaggcacaaaggtttgtagcatgtcggtgagtgcggctttgcgcaggtagttttgataagcgggaataccaatggcgcttaaaatggcaatgatgccaataaccaccatcagttcgataagtgtaaaaccgcgttgcttgtccatctgtttcgctccttgatttggttggcgctactttggcaaacgccatcagcacaggcgaggggcaaaaaacgaaacgggaaagcagattccgaggttttttatttcgttgcagcgaaagacaagaaatttgcgaggcgttacgaagaaagttggggaaggggagattatccgcccgcgatggagcggataaatctgtcaactattagcgaaaacgcattgaaaggtcgagtgcttgtacgtgtttagttagcgcaccgacggagataaagtccacgcccgtttcggcaaattcacgcagtgttttgtcagtgacgttgccagacacttccagtagcgccttgccgttggtgcgtttgacggcttcgcgcatctgttctgtttcgaagttatccagcatgatgatatcggctcctgctttcagggcttcatcaagttcttccagattctctacttcgacttctactggcgcatccgggtgcagccaggacgctttttcgaccgcctggcgcactgagccggaggcaataatatggttttctttgatcaggaaggcatcagaaagccccagacggtgattcgctccgccgccgcaaagtaccgcgtatttcagagctgaacgcaggccgggtaaggttttgcgcgtatccaacaactgcgtgttggtgccttccagcaattcgacatagtggcgtaccttactggcaactcctgaaagggtttgcacaaaattaagcgcagtgcgttcgcccgttaacagcacgcgggatgggccttcaagttcgaacaaggattgattggcattgatgacatcgccgtcatccacatgccagattatggtgacatcgtcgcctgccagttgaataaacacctcttcaacccagcgtttgccgcaaaagacgccattctcgcgggtgatcaccgtggcatgagagcgagaattttccggtaaaagttttgccgtaatatcattgttggcatcgactgttccgcctaaatcttcccgcagcgcctgggccaccgcgccggggatatcgagattaatgcgttccagcagctcgtcacgtcgggtgtcagggttatagcggcgaggcggcatgttaaaactccagatagctaacgaatcataaggtagaaacatgctactctgaaccgggtattagcaccacatataaggagatcctgcatgttgttagaacaggggtggctggttggcgcgcgccgcgttccctcaccacattacgattgccgcccggatgacgaaacacccaccctgctggtggtgcacaatattagcctgccgccaggcgagtttggcggtccgtggatcgacgcattattcactggaactattgatccgcaggcacatcctttctttgctgagatcgcccatttgcgcgtctccgctcactgtttgattcgccgtgatggtgaaatagtccagtatgttcctttcgataaacgtgcatggcatgcgggagtctctcagtatcaggggcgcgaacgctgcaatgatttttctattgggattgagcttgaaggcaccgatacgctggcgtataccgatgcgcagtatcaacagcttgcggcggttacgcgggcactgattgattgctatccggatatcgctaaaaacatgacgggccattgtgatattgcgccggatcggaaaaccgatcccggtcctgcatttgattgggcacggtttcgtgtgctggtcagcaaggagacaacatgacgctatttacaaccttactggtgttaattttcgagcgcctgtttaagttgggcgagcactggcagcttgatcatcgtcttgaagcgttctttcggcgggtgaaacatttttctctcgggcgcacgttaggcatgaccattattgcgatgggcgtgacttttttactgttacgcgcattgcagggagtattgttcaacgttcccacgctactggtgtggctgctgattggtttgctgtgtattggcgcaggtaaagttcgtcttcattatcatgcttatctgacagctgcttcacgtaatgatagccatgcccgtgccacgatggctggcgaactcaccatgattcacggcgtcccggcaggctgcgacgaacgtgagtatttgcgtgagctgcaaaatgcattgctgtggattaactttcgtttttatcttgcaccgctgttctggctgattgtggggggaacctggggacccgttacgctgatggggtatgcgtttttgcgtgcatggcaatactggctggcgcgatatcagacgccgcatcatcgtttacagtccggcattgatgccgtgcttcatgtactggattgggtgccggttcgtcttgcgggtgtggtatatgccttgatcggtcatggtgagaaagcgttaccggcctggtttgcttcgctgggtgatttccatacttcgcagtatcaggtgttaacgcgtctggcgcagttctctctggcgcgtgaaccgcatgtcgataaggtggagacgccgaaggcagcggtttcaatggcgaagaaaacctcgttcgtggtcgtggtggtgattgcactactgacgatttacggggcgttggtgtaaagattattgccctcaccctgtacgggtgagggcgtagagagattaatgcgcttttacggctttggcggttttctctttaaacagatagccgatacctaacacgatcagccataccgggatcaggtataccgaaatcgccattcctggggtcatcagcataatcaccagtaccgccgccataaacagcaggcagatccagttacccagcggataaagcagagcagggaagcgagttaccacgccttgttcctgcttggcgcgacggaatttcatatgcgccaggctaatcatcgcccagttgattaccagtgcagataccaccagcgccattaacagtccgaaagcggactctggggcaaggtagttaatcagtacgcacaacgccgttaccagtgcagacaccagaatggtatttactggtacaccacgtttatcgacagacgccagcgcttttggcgcattaccctgttgtgccagaccaaacagcatacggctgttgcaatatacgcagctgttgtacacggagagcgccgcagtcagtaccacgatgttcagcgcattcgccacaaaggtatcgcctaactcgtggaagatcagcacaaacggactggtatcggcggtaacgcgggtccacggcatcagtgagagcagaacggctaacgaaccaatatagaaaatcaggatgcggtagataacctggttagttgctttcggtatactttgctccgggttatcagcttctgctgcggtgatccccaccagttccagaccaccgaacgagaacatgataatcgccatcatcatcaccagcccggtgaagccgtgcggcaggaaaccaccctgatcccacaggttgctaacggtcgcctgcgggccgccgttgccactgaatagcagccagccgccgaagatgatcatcgctaccaccgcgataactttgataatggcaaaccagaactccatctcgccaaacactttaacgttggtcaggttgatggcgttaatcaccacaaagaatacggcggcagaaacccaggtggggatttccggataccagaactgaatgtatttacccacggcagtcagctcagccatggcaactaaaacgtacagtacccagtagttccagccagaggcgaaaccggcaaaactgccccagtatttataagcaaagtggctaaaggagcctgcgacaggttcttcgaccaccatttcacccagctgacgcatgatcagaaaggcgataaaaccagcaatggcgtaacccaggataatccctggccctgcggactgtattacggaggcgctacccaggaataacccggtccctatcgcgccacccagcgcgataagctgaatatggcggtttttaaggccgcgctttagctgctcgccgtgctgttgaccttccatcatgaaacctcgtgcggtggttgtttttttgatctacgcagtgatgcgtgtgtaagtttgcaattccgtttgttgtattaatttgtttacatcaaagaagtttgaattgttacaaaaagacttccgtcagatcaagaataatggtatgcggcagcgaatgcacccgctttatgcatggttgaagatgagttgcttaaaaagaaaccgtttgtaaagctcagcctcaacccctctcaatatgtagaatgaatttaaattcgttttaattgaattaaaaatcacaaaattggtaagtgaatcggttcaattcggatttttatagtttaataatcgttaaaaaactcctttcctacgtaaagtctacatttgtgcatagttacaactttgaaacgttatatatgtcaagttgttaaaatgtgcacagtttcatgatttcaatcaaaacctgtatggacataaggtgaatactttgttactttagcgtcacagacatgaaattggtaagaccaattgacttcggcaagtggcttaagacaggaactcatggcctacagcaaaatccgccaaccaaaactctccgatgtgattgagcagcaactggagtttttgatcctcgaaggcactctccgcccgggcgaaaaactcccaccggaacgcgaactggcaaaacagtttgacgtctcccgtccctccttgcgtgaggcgattcaacgtctcgaagcgaagggcttgttgcttcgtcgccagggtggcggcacttttgtccagagcagcctatggcaaagcttcagcgatccgctggtggagctgctctccgaccatcctgagtcacagtatgacttgctcgaaacacgacacgccctggaaggtatcgccgcttattacgccgcgctgcgtagtaccgatgaagacaaggaacgcatccgtgaactccaccacgccatagagctggcgcagcagtctggcgatctggacgcggaatcaaacgccgtactccagtatcagattgccgtcaccgaagcggcccacaatgtggttctgcttcatctgctaaggtgtatggagccgatgttggcccagaatgtccgccagaacttcgaattgctctattcgcgtcgcgagatgctgccgctggtgagtagtcaccgcacccgcatatttgaagcgattatggccggtaagccggaagaagcgcgcgaagcatcgcatcgccatctggcctttatcgaagaaattttgctcgacagaagtcgtgaagagagccgccgtgagcgttctctgcgtcgtctggagcaacgaaagaattagtgatttttctggtaaaaattatccagaagatgttgtaaatcaagcgcatataaaagcgcggcaactaaacgtagaacctgtcttattgagctttccggcgagagttcaatgggacaggttccagaaaactcaacgttattagatagataaggaataacccatgtcagaacgtttcccaaatgacgtggatccgatcgaaactcgcgactggctccaggcgatcgaatcggtcatccgtgaagaaggtgttgagcgtgctcagtatctgatcgaccaactgcttgctgaagcccgcaaaggcggtgtaaacgtagccgcaggcacaggtatcagcaactacatcaacaccatccccgttgaagaacaaccggagtatccgggtaatctggaactggaacgccgtattcgttcagctatccgctggaacgccatcatgacggtgctgcgtgcgtcgaaaaaagacctcgaactgggcggccatatggcgtccttccagtcttccgcaaccatttatgatgtgtgctttaaccacttcttccgtgcacgcaacgagcaggatggcggcgacctggtttacttccagggccacatctccccgggcgtgtacgctcgtgctttcctggaaggtcgtctgactcaggagcagctggataacttccgtcaggaagttcacggcaatggcctctcttcctatccgcacccgaaactgatgccggaattctggcagttcccgaccgtatctatgggtctgggtccgattggtgctatttaccaggctaaattcctgaaatatctggaacaccgtggcctgaaagatacctctaaacaaaccgtttacgcgttcctcggtgacggtgaaatggacgaaccggaatccaaaggtgcgatcaccatcgctacccgtgaaaaactggataacctggtcttcgttatcaactgtaacctgcagcgtcttgacggcccggtcaccggtaacggcaagatcatcaacgaactggaaggcatcttcgaaggtgctggctggaacgtgatcaaagtgatgtggggtagccgttgggatgaactgctgcgtaaggataccagcggtaaactgatccagctgatgaacgaaaccgttgacggcgactaccagaccttcaaatcgaaagatggtgcgtacgttcgtgaacacttcttcggtaaatatcctgaaaccgcagcactggttgcagactggactgacgagcagatctgggcactgaaccgtggtggtcacgatccgaagaaaatctacgctgcattcaagaaagcgcaggaaaccaaaggcaaagcgacagtaatccttgctcataccattaaaggttacggcatgggcgacgcggctgaaggtaaaaacatcgcgcaccaggttaagaaaatgaacatggacggtgtgcgtcatatccgcgaccgtttcaatgtgccggtgtctgatgcagatatcgaaaaactgccgtacatcaccttcccggaaggttctgaagagcatacctatctgcacgctcagcgtcagaaactgcacggttatctgccaagccgtcagccgaacttcaccgagaagcttgagctgccgagcctgcaagacttcggcgcgctgttggaagagcagagcaaagagatctctaccactatcgctttcgttcgtgctctgaacgtgatgctgaagaacaagtcgatcaaagatcgtctggtaccgatcatcgccgacgaagcgcgtactttcggtatggaaggtctgttccgtcagattggtatttacagcccgaacggtcagcagtacaccccgcaggaccgcgagcaggttgcttactataaagaagacgagaaaggtcagattctgcaggaagggatcaacgagctgggcgcaggttgttcctggctggcagcggcgacctcttacagcaccaacaatctgccgatgatcccgttctacatctattactcgatgttcggcttccagcgtattggcgatctgtgctgggcggctggcgaccagcaagcgcgtggcttcctgatcggcggtacttccggtcgtaccaccctgaacggcgaaggtctgcagcacgaagatggtcacagccacattcagtcgctgactatcccgaactgtatctcttacgacccggcttacgcttacgaagttgctgtcatcatgcatgacggtctggagcgtatgtacggtgaaaaacaagagaacgtttactactacatcactacgctgaacgaaaactaccacatgccggcaatgccggaaggtgctgaggaaggtatccgtaaaggtatctacaaactcgaaactattgaaggtagcaaaggtaaagttcagctgctcggctccggttctatcctgcgtcacgtccgtgaagcagctgagatcctggcgaaagattacggcgtaggttctgacgtttatagcgtgacctccttcaccgagctggcgcgtgatggtcaggattgtgaacgctggaacatgctgcacccgctggaaactccgcgcgttccgtatatcgctcaggtgatgaacgacgctccggcagtggcatctaccgactatatgaaactgttcgctgagcaggtccgtacttacgtaccggctgacgactaccgcgtactgggtactgatggcttcggtcgttccgacagccgtgagaacctgcgtcaccacttcgaagttgatgcttcttatgtcgtggttgcggcgctgggcgaactggctaaacgtggcgaaatcgataagaaagtggttgctgacgcaatcgccaaattcaacatcgatgcagataaagttaacccgcgtctggcgtaagaggtaaaagaataatggctatcgaaatcaaagtaccggacatcggggctgatgaagttgaaatcaccgagatcctggtcaaagtgggcgacaaagttgaagccgaacagtcgctgatcaccgtagaaggcgacaaagcctctatggaagttccgtctccgcaggcgggtatcgttaaagagatcaaagtctctgttggcgataaaacccagaccggcgcactgattatgattttcgattccgccgacggtgcagcagacgctgcacctgctcaggcagaagagaagaaagaagcagctccggcagcagcaccagcggctgcggcggcaaaagacgttaacgttccggatatcggcagcgacgaagttgaagtgaccgaaatcctggtgaaagttggcgataaagttgaagctgaacagtcgctgatcaccgtagaaggcgacaaggcttctatggaagttccggctccgtttgctggcaccgtgaaagagatcaaagtgaacgtgggtgacaaagtgtctaccggctcgctgattatggtcttcgaagtcgcgggtgaagcaggcgcggcagctccggccgctaaacaggaagcagctccggcagcggcccctgcaccagcggctggcgtgaaagaagttaacgttccggatatcggcggtgacgaagttgaagtgactgaagtgatggtgaaagtgggcgacaaagttgccgctgaacagtcactgatcaccgtagaaggcgacaaagcttctatggaagttccggcgccgtttgcaggcgtcgtgaaggaactgaaagtcaacgttggcgataaagtgaaaactggctcgctgattatgatcttcgaagttgaaggcgcagcgcctgcggcagctcctgcgaaacaggaagcggcagcgccggcaccggcagcaaaagctgaagccccggcagcagcaccagctgcgaaagcggaaggcaaatctgaatttgctgaaaacgacgcttatgttcacgcgactccgctgatccgccgtctggcacgcgagtttggtgttaaccttgcgaaagtgaagggcactggccgtaaaggtcgtatcctgcgcgaagacgttcaggcttacgtgaaagaagctatcaaacgtgcagaagcagctccggcagcgactggcggtggtatccctggcatgctgccgtggccgaaggtggacttcagcaagtttggtgaaatcgaagaagtggaactgggccgcatccagaaaatctctggtgcgaacctgagccgtaactgggtaatgatcccgcatgttactcacttcgacaaaaccgatatcaccgagttggaagcgttccgtaaacagcagaacgaagaagcggcgaaacgtaagctggatgtgaagatcaccccggttgtcttcatcatgaaagccgttgctgcagctcttgagcagatgcctcgcttcaatagttcgctgtcggaagacggtcagcgtctgaccctgaagaaatacatcaacatcggtgtggcggtggataccccgaacggtctggttgttccggtattcaaagacgtcaacaagaaaggcatcatcgagctgtctcgcgagctgatgactatttctaagaaagcgcgtgacggtaagctgactgcgggcgaaatgcagggcggttgcttcaccatctccagcatcggcggcctgggtactacccacttcgcgccgattgtgaacgcgccggaagtggctatcctcggcgtttccaagtccgcgatggagccggtgtggaatggtaaagagttcgtgccgcgtctgatgctgccgatttctctctccttcgaccaccgcgtgatcgacggtgctgatggtgcccgtttcattaccatcattaacaacacgctgtctgacattcgccgtctggtgatgtaagtaaaagagccggcccaacggccggcttttttctggtaatctcatgaatgtattgaggttattagcgaatagacaaatcggttgccgtttgttgtttaaaaattgttaacaattttgtaaaataccgacggatagaacgacccggtggtggttagggtattacttcacataccctatggatttctgggtgcagcaaggtagcaagcgccagaatccccaggagcttacataagtaagtgactggggtgagggcgtgaagctaacgccgctgcggcctgaaagacgacgggtatgaccgccggagataaatatatagaggtcatgatgagtactgaaatcaaaactcaggtcgtggtacttggggcaggccccgcaggttactccgctgccttccgttgcgctgatttaggtctggaaaccgtaatcgtagaacgttacaacacccttggcggtgtttgcctgaacgtcggctgtatcccttctaaagcactgctgcacgtagcaaaagttatcgaagaagccaaagcgctggctgaacacggtatcgtcttcggcgaaccgaaaaccgatatcgacaagattcgtacctggaaagagaaagtgatcaatcagctgaccggtggtctggctggtatggcgaaaggccgcaaagtcaaagtggtcaacggtctgggtaaattcaccggggctaacaccctggaagttgaaggtgagaacggcaaaaccgtgatcaacttcgacaacgcgatcattgcagcgggttctcgcccgatccaactgccgtttattccgcatgaagatccgcgtatctgggactccactgacgcgctggaactgaaagaagtaccagaacgcctgctggtaatgggtggcggtatcatcggtctggaaatgggcaccgtttaccacgcgctgggttcacagattgacgtggttgaaatgttcgaccaggttatcccggcagctgacaaagacatcgttaaagtcttcaccaagcgtatcagcaagaaattcaacctgatgctggaaaccaaagttaccgccgttgaagcgaaagaagacggcatttatgtgacgatggaaggcaaaaaagcacccgctgaaccgcagcgttacgacgccgtgctggtagcgattggtcgtgtgccgaacggtaaaaacctcgacgcaggcaaagcaggcgtggaagttgacgaccgtggtttcatccgcgttgacaaacagctgcgtaccaacgtaccgcacatctttgctatcggcgatatcgtcggtcaaccgatgctggcacacaaaggtgttcacgaaggtcacgttgccgctgaagttatcgccggtaagaaacactacttcgatccgaaagttatcccgtccatcgcctataccgaaccagaagttgcatgggtgggtctgactgagaaagaagcgaaagagaaaggcatcagctatgaaaccgccaccttcccgtgggctgcttctggtcgtgctatcgcttccgactgcgcagacggtatgaccaagctgattttcgacaaagaatctcaccgtgtgatcggtggtgcgattgtcggtactaacggcggcgagctgctgggtgaaatcggcctggcaatcgaaatgggttgtgatgctgaagacatcgcactgaccatccacgcgcacccgactctgcacgagtctgtgggcctggcggcagaagtgttcgaaggtagcattaccgacctgccgaacccgaaagcgaagaagaagtaatttttcgtttgccggaacatccggcaattaaaaaagcggctaaccacgccgctttttttacgtctgcaatttacctttccagtcttcttgctccacgttcagagagacgttcgcatactgctgaccgttgctcgttattcagcctgacagtatggttactgtcgtttagacgttgtgggcggctctcctgaactttctcccgaaaaacctgacgttgttcaggtgatgccgattgaacacgctggcgggcgttatcacgttgctgttgattcagtgggcgctgctgtactttttccttaaacacctggcgctgctctggtgatgcggactgaatacgctcacgcgctgcgtctcttcgctgctggttctgcgggttagtctgcattttctcgcgaaccgcctggcgctgctcaggcgaggcggactgaatgcgctcacgcgctgcctctcttcgctgctggatcttcgggttagtctgcattctctcgcgaactgcctggcgctgctcaggcgaggcggactgataacgctgacgagcggcgtccttttgttgctgggtcagtggttggcgacggctgaagtcgtggaagtcgtcatagctcccatagtgttcagcttcattaaaccgctgtgccgctgcctgacgttgggtatctcgtgtaatgactggtgcggcgtgtgttcgttgctgaaactgatttgctgccgcctgacgctggctgtcgcgcgttggggcaggtaattgcgtggcgctcattccgccgttgacatcggtttgatgaaaccgctttgccatatcctgatcatgatagggcacaccattacggtagtttggattgtgccgccatgccatattcttatcagtaagatgctcaccggtgatacggttgaaattgttgacgtcgatattgatgttgtcgccgttgtgttgccagccattaccgtcacgatgaccgccatcgtggtgatgataatcatcattgtcatgatgatgatggtcatgatcgtcgtcgtcccagtcgatgctgctgaatagtgcgtacgtggtagcaacgcccatgctatagccgaatccgcgtacaaagctgtcaacaaacggttctccggctggtggtggcagataaaccggcggatacgcagtattggcccagttcccgtaaaccacggttgggttgtagttgggaatatagaccacatcaggattggcgggctcaatggaaatgacggttgttgccggctctgtaatgacggggttggcagttaaaactgtattggatggtatgacgggtgccgtgactgtctgttttaccggtacagctttcttcgttgtggtaataactttctgttcggttgatgacttcagcgagccggtttgttgcgccagttgccgcaatcgctgtaccgagtccatcacgtcctgcggctgggccagaaaagcatcgcccaggttttgcacccattgcgggttttcgcccatcaatgccatcaattgtggaaaggccaccagtgatttaacgctggcgtcccacggctggtcagataccgcctgaatagcagcatcgccttgtttaagtggattatcgtgcgaccattgcactgcttgagcaacgtttgtcggataggttgatgccatcagcacctgcgaaagtagggcgtcgggatacagcgcgacgggcgcgacccattgatctatttgtgcagtgctgaatgcggatttgacgacggcgggtgttacgggaggtgcggaaaccgttgcaggaaacgtaaccgcggcagcgtcagacacagccagttgtgtcgattgcggttccacaggcgcttccactgtgcggctttttatatatagcccggtagaggcggcacaaagcccggcactgcaaattagcgccagcacatggggtttaaacggcaaagtcattttcataattcggatctcaaggaaatcgcaatggtcggcgaactgccacccgcaggtgctgtgaatccgagtataaagaggcggtagtttaaattttgactaatcttgggattcgttgagaaaggtgattatcaccatgcgaattaacgaagtttttacggagggaaacaatctctagaccatccttaacgattcagccacttttttatgttgcttttttgtaaacagattaacacctcgtcaaaatcctgctattctgcccgttgcggtactgggcatttaccctacaaactgctgtctcacaggagcgtgaagagaatcgcctgccgcactatgacaatgagagcgaggagaaccgtcgtgctagaagaataccgtaagcacgtagctgagcgtgccgctgaggggattgcgcccaaacccctggatgcaaaccaaatggccgcacttgtagagctgctgaaaaacccgcccgcgggcgaagaagaattcctgttagatctgttaaccaaccgtgttcccccaggcgtcgatgaagccgcctatgtcaaagcaggcttcctggctgctatcgcgaaaggcgaagccaaatcccctctgctgactccggaaaaagccatcgaactgctgggcaccatgcagggtggttacaacattcatccgctgatcgacgcgctggatgatgccaaactggcacctattgctgccaaagcactttctcacacgctgctgatgttcgataacttctatgacgtagaagagaaagcgaaagcaggcaacgaatatgcgaagcaggttatgcagtcctgggcggatgccgaatggttcctgaatcgcccggcgctggctgaaaaactgaccgttactgtcttcaaagtcactggcgaaactaacaccgatgacctttctccggcaccggatgcgtggtcacgcccggatatcccactgcacgcgctggcgatgctgaaaaacgcccgtgaaggtattgagccagaccagcctggtgttgttggtccgatcaagcaaatcgaagctctgcaacagaaaggtttcccgctggcgtacgtcggtgacgttgtgggtacgggttcttcgcgtaaatccgccactaactccgttctgtggtttatgggcgatgatattccacatgtgccgaacaaacgcggcggtggtttgtgcctcggcggtaaaattgcacccatcttctttaacacgatggaagacgcgggtgcactgccaatcgaagtcgacgtctctaacctgaacatgggcgacgtgattgacgtttacccgtacaaaggtgaagtgcgtaaccacgaaaccggcgaactgctggcgaccttcgaactgaaaaccgacgtgctgattgatgaagtgcgtgctggtggccgtattccgctgattatcgggcgtggcctgaccaccaaagcgcgtgaagcacttggtctgccgcacagtgatgtgttccgtcaggcgaaagatgtcgctgagagcgatcgcggcttctcgctggcgcaaaaaatggtaggccgtgcctgtggcgtgaaaggcattcgtccgggcgcgtactgtgaaccgaaaatgacttctgtaggttcccaggacaccaccggcccgatgacccgtgatgaactgaaagacctggcgtgcctgggcttctcggctgacctggtgatgcagtctttctgccacaccgcggcgtatccgaagccagttgacgtgaacacgcaccacacgctgccggacttcattatgaaccgtggcggtgtgtcgctgcgtccgggtgacggcgtcattcactcctggctgaaccgtatgctgctgccggataccgtcggtaccggtggtgactcccatacccgtttcccgatcggtatctctttcccggcgggttctggtctggtggcgtttgctgccgcaactggcgtaatgccgcttgatatgccggaatccgttctggtgcgcttcaaaggcaaaatgcagccgggcatcaccctgcgcgatctggtacacgctattccgctgtatgcgatcaaacaaggtctgctgaccgttgagaagaaaggcaagaaaaacatcttctctggccgcatcctggaaattgaaggtctgccggatctgaaagttgagcaggcctttgagctaaccgatgcgtccgccgagcgttctgccgctggttgtaccatcaagctgaacaaagaaccgatcatcgaatacctgaactctaacatcgtcctgctgaagtggatgatcgcggaaggttacggcgatcgtcgtaccctggaacgtcgtattcagggcatggaaaaatggctggcgaatcctgagctgctggaagccgatgcagatgcggaatacgcggcagtgatcgacatcgatctggcggatattaaagagccaatcctgtgtgctccgaacgacccggatgacgcgcgtccgctgtctgcggtacagggtgagaagatcgacgaagtgtttatcggttcctgcatgaccaacatcggtcacttccgtgctgcgggtaaactgctggatgcgcataaaggtcagttgccgacccgcctgtgggtggcaccgccaacccgtatggacgccgcacagttgaccgaagaaggctactacagcgtcttcggtaagagtggtgcgcgtatcgagatccctggctgttccctgtgtatgggtaaccaggcgcgtgtggcggacggtgcaacggtggtttccacctctacccgtaacttcccgaaccgtctgggtactggcgcgaatgtcttcctggcttctgcggaactggcggctgttgcggcgctgattggcaaactgccgacgccggaagagtaccagacctacgtggcgcaggtagataaaacagccgttgatacttaccgttatctgaacttcaaccagctttctcagtacaccgagaaagccgatggggtgattttccagactgcggtttaaaaagtcagcgcacgcgctgcgcataaacgacacaatgcccggtgaatgagattcccgggcatttttttatttctaaaccatcgccgttccgctgtttttctccggtaaggctgcgataattacatcaatggcgcaatgcgatttcggtgcattgccgggagcagaggaacacactatggattacgaatttctgcgcgatattaccggagtggtaaaggtgcgtatgtccatggggcatgaagtggtcgggcactggtttaatgaagaggtgaaagaaaacctggccttgcttgatgaagtggaacaagcagcgcacgcactgaaaggtagcgaacggtcctggcaacgggcagggcatgaatacaccctgtggatggacggtgaagaggtgatggttcgcgccaatcaactggaattcgctggcgatgaaatggaagaggggatgaactactacgacgaagaaagcctgtcgctatgcggcgttgaggattttctgcaggtcgtggcggcttaccgcaatttcgtgcagcagaagtaaataaatctggcggagcctgggagctccgccagagccgttaaacagctggcatattgcgcccgtaataaatctcgcgcatttctttccacagcgcagcggtaatttcctggcgctcgctgtcggttaagtcttccggtttggtgtggaacatgtagtgcttaaggtcgaactctttaagcaacatcttggtatggaagatattttcctgatagacgttcacatccaccatgtcatacagcgccttcatatcgtcagacataaagttctgaatcgaattaatctcatggtcgataaagtgcttcataccgttaatgtcgcgggtaaaaccgcgcacgcgataatcaatggttacgatatcggactcaagctggtggatcaggtaattcagcgccttcagcggagaaatcacgccgcaggtagagacttcaatatcggcgcggaaggtacataaaccgccttcaggatgactttccgggtaggtatgtacgcaaatatgacttttatcaagatgggcaacgaccgtttctggcagtgggccggggtgttctgttttgtcgatgagtttcgggtcaaccggttcttcactcaccagaatagtgacgctggcaccctgtggttcgtaatcctggcgggcgatgttaagaatattagccccgataatggaacaggtttctgacaggatttcggtcagacggttggcattatagagttcatcgatataagcaatataaccgtcgcgctcttcggcagttttggcgtagcagatatcgtaaatacaaaaactcagacttttggtcagattattaaagccatgcagtttcagttttttcaatttcttatcttctccttaggacggctgtgaagccagtgcgtcttgcagatactgaggtaaggcaaaagctgccgtatggattgccggattgtaataacggcatttcaggccagaggcgagaaaacgcgcctgaataatttcggttgagagatggcgtaaggcgtcgttatctgtcgcccatgcaaaagtcatgataccgccgtaataggtcgggatcgccgcctgataaaagccaacgtcgctgaagtaatggctgagtttgcgatggctgtcgatggcttcttcctgctgtaaaaagcagacgccgttttgtgcgacgaagataccgccaggattcaggcaacgtttgcagccttcataaaatgccgaagtgaaaaggctttcgccgggaccgataggatcggtgcagtcggagataatgacatcaaaggtctggctggtttgattaacgaaattgacgccatcgtcgatcaccagcttaaagcgcggatcgtcgtagctaccggcgttatggttgggtagatactgacggcagaacgatacgacacccgcatcgatttccaccatcgtgattgactcaacgtttttatgtcgggttacttcacgcagcatggcaccgtcgccgccgccgataatcagcacatgtttcgcgtgaccatgggccagtagcggaacatgggtcatcatctcatgatagataaactcgtcgcgctcggtggtttgtactacgccatccagcgccattacgcgaccaaatgcagcgttctcaaaaatgatcagatcctggtgatcggtcttttcatgatacagaacgttatctaccgcaaagtactgcccaaactggtcgtgtagcgtttcatgccactgttttttttcggccatgggttgatacctcctttgttaacacccgtaaaaaaagggcgcaacataatagctaacattgaccgcggatgcacggtcaatatttctacaaaaaggtatcagggattatttgacgtaggcaagcaggcttaaggaatcgcgggccagggctttgcattttttagcgacgggaatgccaatgccgctgagatcgcggtagctgtcttcaccgagggctttcatgtcgaaggtgtcgtaattactgaggtcccactggttttgctgagcgaaaaagaccagtgcgcgacgaatttgcccgttaggtaagttctggtaaccacaatcgttcttcagaaagacaaaaactgccgttaaatcggccatatcttcggcttcagactcgctgagcgcgtaactgtttgcgcagacggccatcaggctgccgaataacactgttctgaaaaacgtcttcattgcttctaccaggggcttaaagaagataaacgttagcacactgcgagcgaggcgacgaccattattgtcgattaaattgtgtctgcggcttgaccttcccgtaaggggaaggactatgctcaacgtttgattttgtttcgcctgcttaagaataaggaaataactatgcaacgtcgtgatttcttaaaatattccgtcgcgctgggtgtggcttcggctttgccgctgtggagccgcgcagtatttgcggcagaacgcccaacgttaccgatccctgatttgctcacgaccgatgcccgtaatcgcattcagttaactattggcgcaggccagtccacctttggcgggaaaactgcaactacctggggctataacggcaatctgctggggccggcggtgaaattacagcgcggcaaagcggtaacggttgatatctacaaccaactgacggaagagacaacgttgcactggcacgggctggaagtaccgggtgaagtcgacggcggcccgcagggaattattccgccaggtggcaagcgctcggtgacgttgaacgttgatcaacctgccgctacctgctggttccatccgcatcagcacggcaaaaccgggcgacaggtggcgatggggctggctgggctggtggtgattgaagatgacgagatcctgaaattaatgctgccaaaacagtggggtatcgatgatgttccggtgatcgttcaggataagaaatttagcgccgacgggcagattgattatcaactggatgtgatgaccgccgccgtgggctggtttggcgatacgttgctgaccaacggtgcaatctacccgcaacacgctgccccgcgtggttggctgcgcctgcgtttgctcaatggctgtaatgcccgttcgctcaatttcgccaccagcgacaatcgcccgctgtatgtgattgccagcgacggtggtctgctacctgaaccagtgaaggtgagcgaactgccggtgctgatgggcgagcgttttgaagtgctggtggaggttaacgataacaaaccctttgacctggtgacgctgccggtcagccagatggggatggcgattgcgccgtttgataagcctcatccggtaatgcggattcagccgattgctattagtgcctccggtgctttgccagacacattaagtagcctgcctgcgttaccttcgctggaagggctgacggtacgcaagctgcaactctctatggacccgatgctcgatatgatggggatgcagatgctaatggagaaatatggcgatcaggcgatggccgggatggatcacagccagatgatgggccatatggggcacggcaatatgaatcatatgaaccacggcgggaagttcgatttccaccatgccaacaaaatcaacggtcaggcgtttgatatgaacaagccgatgtttgcggcggcgaaagggcaatacgaacgttgggttatctctggcgtgggcgacatgatgctgcatccgttccatatccacggcacgcagttccgtatcttgtcagaaaatggcaaaccgccagcggctcatcgcgcgggctggaaagataccgttaaggtagaaggtaatgtcagcgaagtgctggtgaagtttaatcacgatgcaccgaaagaacatgcttatatggcgcactgccatctgctggagcatgaagatacggggatgatgttagggtttacggtataaaaagaccgtattcggaaatatgcccggatctctccgggcattaaactgatgacaaacgcaaatctgcctgatgcgctacgcttatcaggcctacgctagctgtgcaatccattgattttgcacaattttgtaggctggataaggcgttcacgccgcatccggcatgaacaacgcgcacgttgtcagcaatctgagcaagtcttacttcacatcatccggcagcgcataagccacaatatagtcgcccatcttcgtaccaaatgaaccgtgaccgcctgcggagatcaccacatactgcttaccattcacttcataggtcattggcgtagcctgaccacccgctggtaaacgaccctgccacagtttttcaccgttgctcatgttgtaagcgcgcaggtagttatctgccgtagcggcgataaacagcacgttacccgccgtggagattggcccgcccagcatcggcatacccatattgaacggcaccggaaccggcatcgggaacggcatactgtcctgcggcgtaccaatacgtttcttccacaccacttcattagttttcagatccagcgccgagatataaccccatgctggctgtttacatggcagaccaaatggtgagaggaacgggttgagcgtgacaccatacggtacaccgtactgtggctgaatgccggattccgtacccgtgcctttggcatctttcggctgctccatcgggttgccaggaccacgcgggatcagtttcgaaacaaacggcagtgccattgggttggcaatcgccacttcacgatttggatcaacggaaatcccgccccattcgaacatccccaggttacccgggaagaccagcgtaccctgttcagatggcggggtgaaaatgccttcatagcgcatctggtggaacatcacgcggcacaccagttggtcaaacatggtggctccccacatatccgcaccgctcaaatctttcgtcggacggaagctcagttcagaaaacggttgagttggggttacgtaatcgcctttcgctgcaccttggggaaccggtttttccggtgccggaaccaccagttcgccattacgacgatcgagcacaaaaatgttgccggttttcgccggagcgtaaataactggcactttctgaccattaacggtgatgtccgccagcgtcggctgtgccggaagatccatgtcccacaggtcgtggtgaacggtctggtagctccacgccagtttcccggtagtggcattcagcgccagaatcgagctggcataacgttcctgttccggtgtgcggttaccgccccagatatccggcgtggtcacgcccatcggcagatagaccagatccagcttcgcgtcataggccgctggtgcccaggagtttggcgagttaaaggtaaaggtgtgttcgtcagacgggattgcgttcggatctttcgcgccgggatcaaaagcccacagcagctccccggtgttgacatcaaaaccacggatcacgccagacgtttcgcgggttgagaagttatcggtaactgaaccggccatcacgatggttttatcggtgataatcggtggcgaagtcggttcatacagacccggtttggtgtctggcatattgctttgcagattgagcacgcctttattggcgaaggtttcgcacagtttgccgttttcagcgttaatcgcaatcagtcgaccatcattgaccggaagaatgatacgacgcgggcaatccgccatcacttccggcgaagcggtttctgctttggcttcatgataagagacaccacggcaggttacgtgctggaaagactcgttggttttcagctcaggatcgtaatgccatttctctttgccgctggcggcatcaagcgcaaacaggcgctggtgagcggtacacaggtaaagggtgtcgcccactttaatcggcgtcacttcattggtgatttcacccggatcgttcggctgcttcacatcgccagtacggaacacccaggcttctttcagattatggacgttatcggcgttaatttgtttcagcggcgaaaagcgttgaccttcctgattacgaccataggcaggccagtcctgatcggctacgggggagatagcttcagcaggtgtggcatcggcgcttaaggtgccgttgatctcctgcggatcgttaaatccggcccaggtcaggataccaccgctaatcagcagtgcgaccaccagtgcggcaactgcgccgctggcaggaatgaccaggcgacgccagacaaacggcaggatcagccagatgccgaagaagaccagaatgtcgctgcgcggagtcagcgcccagaagtcgaaaccaacttcccagacgccccaaatcatggtgccgagcagcagggctgcgtatagccaaagcgcggcgcgtttactgcgccacagcatccaggcgacgccgagcatcacaaggccagcgatagggtagtaccaggagccgccaatcgcgaccagccagcctccgccaatgagtagatacagcccgcaaagcgctgcaaaaagggctgttagcgtgacgagtaatcgtcgcgagcctgtattgttaattgccataaagagacaccatttcaattcattaatattttagtagcaattaattataggttttaacatgtgtgatcgtcatcacaattcgagctttattaacagattccgcgaatgaatagttttactggtatactgcgtgtcttgcgctttgttgcggtgccaaaacctgcccgtgcgaagtgatttgtttttaaatcatatggttagagatatgaaacatactgtagaagtaatgatccccgaagcggagattaaagcgcgtatcgccgaactgggtcgtcagattactgagcgttacaaagacagcggcagcgatatggtgctggtgggtctgctgcgtggctcatttatgtttatggcggacctgtgccgtgaagttcaggtatctcatgaagtcgactttatgaccgcctccagctacggtagcggcatgtccaccacccgtgatgtgaaaatcctcaaagatctggatgaagatatccgtggcaaggacgtgctgattgttgaagatatcatcgactcggggaatacactgtcgaaagtgcgtgagatcttaagcctgcgcgaaccgaagtcgctggcgatttgtacgctgctggataaaccgtcccgtcgtgaagtgaacgtcccggtagaatttatcggtttctcgatcccggatgagtttgtggtgggttacggcattgattacgcacagcgttaccgtcatctgccgtatatcggcaaagtgattctgctggacgagtaagtgtgaagttgccggatgtgttgcatccggcatggcatttttatttgtggttggcgtgtttcagcttgaggttggaaatcccgtgacggtaacgttgctcaagggtttcgcggttggtggcggtaacatccagatcacgcagcaagccgtcgtgaatgccgtaggcccagccgtgaatggtaactttctgcccgcgtttccacgctgattgcataatggtggagtggcccaggttatacacctgttccatgacgttcagttcacacaaggtatccagacggcgctcttgcggcatttcgccgagcaatgagctatgtttgaaccagatatcgcggatatgcagcagccagttgttgataagccccagttccgggttttcaactgcggcttgtacgccgccgcaaccgtagtggccacagataataatgtgttcaacttcgagtacatccactgcatactgaaccacggaaaggcagttcaggtcagtgtgaatgaccaggttagcaacattacggtgaacaaagagttcgcccggctcaagaccggttaaacgttctgcaggaacgcgactgtcggaacatccaatccatagaaagcgcggtttttgcgcttgtgccagtttctcaaaaaacccgggatcctcttccaccagcatttttgaccatagtgcattgttgctgatgagtgtatctatgtctttcatggaggttaacgacctgtaaccaaataattacgtttggctaatatagggcaactccgggacgatttaaaccacagataaagtgtaagaacgtaaggtaagtaaaaatttatgaccattgcactggaacttcaacagcttaaaaaaacctatccaggcggcgttcaggcgcttcgtgggatagatttgcaggtcgaagcgggtgatttttatgcgcttctcgggccgaacggggccgggaaatcgaccactatcggtattatcagctctctggtaaataaaacctccgggcgggtcagcgtatttggttacgatctcgagaaggatgtcgtgaacgctaaacgtcagttgggactggtgccgcaggaatttaacttcaacccgtttgaaaccgtgcagcaaattgtggtgaatcaggcagggtactacggcgtggagcgcaaagaagcgtacatccgcagcgaaaagtatcttaaacaactcgatctatggggaaaacgcaacgaacgtgcgcgtatgttatctggcgggatgaagcgccgtttaatgattgcccgtgcgttaatgcatgaacctaaactactgattctcgacgaaccgaccgcaggcgtggatattgaacttcgccgctcaatgtggggctttttgaaggatttaaacgacaaaggcaccaccatcattctcaccacacactacctggaagaagcagaaatgctgtgccgcaatatcggcattattcaacacggtgagctggtggaaaatacctcgatgaaggcgctgctggcgaagctgaaatcggaaacctttattctcgatctcgcaccgaaaagcccgttaccgaagctcgatggctatcagtatcgactggtcgataccgcgacgctggaagttgaagtgctgcgtgagcaggggatcaacagcgtatttacgcagttaagtgagcagggcattcaggtattaagtatgcgtaacaaagctaaccgtctggaagagctgtttgtttcactggttaatgaaaaacaaggagatcgcgcatgatgcatctttactgggtggcgctaaaaagcatctgggcgaaagagatccatcgctttatgcgtatctgggtgcagacgctggtgccgccagtcatcaccatgaccctttactttattatcttcggtaacctgattggttcgcgtattggcgatatgcatggcttcagctatatgcagttcatcgtaccggggctgatcatgatgtcggtgatcaccaatgcctacgccaacgttgcgtcatcattttttggtgccaagttccagcgtaatattgaagagctgctggtagcgccggttccgactcacgtcattattgccggatatgtcggcggtggcgtggcgcgtggtctgtttgttggcattctggtgacggcaatttcactgttttttgtgccatttcaggtgcattcgtgggtattcgttgccttaacgctggtgctcacggcggtgttgttctcccttgcgggtttgctgaacggtgtgtttgccaaaacgttcgatgacatcagcctggtgccaacctttgtgttaacgccactcacgtatttgggcggggtcttttactcactgactttgttgccgccgttctggcaagggctgtcgcacctgaacccaatcgtttatatgatcagtggtttccgctacggcttcctcggtatcaatgatgttccgctggtcactacctttggcgtactggtggtctttattgtggcgttttatttgatctgttggtcgctgatccaacgtggacgtggtttgcgtagctaaggctatttcctctcctctggatttgggggagaggagttttgacggctatcaccctttatcaacaatggtcagggtagactgattttcggctaaggaggaaggcgatgttaggttgggtaattacctgtcacgatgaccgggcgcaagagatactggatgcgctggagaaaaaacatggggcacttcttcagtgccgggccgtgaatttctggcgcggattaagctctaatatgctcagccgcatgatgtgcgatgctctgcatgaagcggactctggtgagggtgtcatcttcttaaccgatatagccggagcgccaccgtatcgcgtggcttcattattaagccacaaacactcccgttgcgaagtgatttctggtgtcacgttaccgttaattgaacagatgatggcttgccgtgaaaccatgaccagttcagagtttcgcgagcgtattgtcgaactgggtgcgccggaggtgagtagtctttggcaccaacaacaaaaaaatccgcctttcgtcctcaaacataatttgtatgagtattaacccgcgattctgatggcgcttttgctacaataaaagcgttgtttcaccctcggttattttttcatgtacaaacaagctgttattctcctgctgatgctgtttaccgcaagtgtcagtgccgcgttacctgcccgttatatgcaaaccatcgaaaatgctgcggtctgggcgcaaattggtgacaagatggtgaccgtggggaatattcgggccggacaaatcattgccgtggagcccactgccgcaagttattacgcatttaattttggctttggcaaaggttttatcgataaaggtcatctcgagccggttcaggggcgacaaaaagttgaagacggtttgggcgacctcaacaagccgctgagtaatcagaacttagttacctggaaagatacgccggtctataacgcgccgagtgcgggaagtgcgccatttggggtactggcggacaatttgcgctacccgattttgcataaactgaaagacaggttaaatcaaacctggtatcagatccgtattggcgatcgactggcctatatcagcgcactggatgcccaacccgataatggcctgtcggtgctaacctatcaccatattctgcgcgacgaagaaaacacccgttttcgccatacttcgacgaccacatcggtacgcgctttcaataaccagatggcctggctgcgtgacaggggatacgcgacactgagcatggtgcagctggaaggctacgtgaagaataagatcaatctccctgcgcgagcggtggtgattacctttgatgatggcctcaagtcggtgagccgctatgcgtatcctgtgttgaaacaatatggcatgaaggcgacggcgtttattgttacctcacgcatcaaacgtcacccgcagaagtggaacccaaaatcgctgcaatttatgagcgtttctgagcttaacgaaattcgcgatgtatttgatttccagtcacatacccattttttgcatcgggtagatggttatcgccgacccatattactgagccgtagtgagcacaatattctgtttgattttgcacgttcacgccgcgctctggcgcaatttaatccgcatgtctggtatctttcgtatccgtttggcggatttaatgacaacgccgtgaaggcagcaaacgatgccggatttcacctggcggtgacaaccatgaaaggcaaagtaaaaccgggggataatccgttgttactaaaacgactttatatcttaagaacggattcgctggagacgatgtcgcggctggtgagtaaccagccgcagggataacaatcaagcaacctgtaccggaatcgctttcgcggtacgtttcatttcattgtcgccttcaaaataggcgacgttgggtcgccaggtgcgagcttcttcatctggcatggtaacgaagctggcgatgatgacaatatcgccgacactggcgcagtgggccgccgcaccgttaacagaaataattctcgaaccgcgttctgccgcgatggcataagtggagaaacgcttgccgttggtgacattccagatatcaatggcttcgttttcgagaataccggctgcgtcaagaaaatcctggtcaatggcgcaagaaccttcatagtgcaggtccgcatgagtcactttcacgcggtggagtttgccctgcagcatcgtgcgaatcataacttctacctttctaccctgtcgttaacgaagcaggcgatgcctgctttgaggaaattctcacgcagtattgcccgatttttgtttagtgtctactcatctgacggcatttgcgtcagcagtttgcgtaccgcgccgaagcgtgccatgtatcgcctgtaacgaattgatatttctctgaacgctgctcggtaaacaataaagaggtggctgacgatagcgcgccttgactggatactgccttcacgcaaagccacacggaagacagggaagatggatgcaccgagtaccacaccgcatgacgcggtatttaaacaatttttaatgcatgcggagacggctcgcgactttctggagatacatttgccagtggaattacgcgaactttgtgacctcaacacgcttcatttagagtcggggagtttcattgaagagagcctgaaaggacacagcacggacgtgctctattccgtgcaaatgcagggcaatcccggttatctgcatgttgtgattgaacaccaaagcaagccggataagaaaatggcctttcgcatgatgcgttattctatagccgccatgcaccggcatctggaggctgaccacgataagctgccgctggtggtgccgatactgttttatcagggcgaggccacaccttatccgctatcaatgtgctggtttgatatgttttactcgccggagctggcgcgacgcgtctataacagtcctttcccgctggtggatatcaccatcacaccggatgacgaaatcatgcaacatcggcggattgcgattctcgaactactgcaaaaacatattcgccagcgcgacttaatgttattgcttgagcaactggtcacgctgatcgacgaagggtacactagcggaagtcagttagttgccatgcaaaactatatgctgcaacgcggtcatactgaacaagcggatttgttttacggtgtgttgagagacagggaaacgggaggggagtctatgatgacgctggcgcagtggtttgaagagaaagggattgagaaggggattcagcagggaagacaggaagtaagtcaggaattcgcccagcgtcttctgagtaaaggaatgtctcgggaagacgttgcagagatggcaaatttacctcttgctgagattgataaggtaattaaccttatttaagttacctgtgttatgacagatgacgtggggtaaattaataactggcgccatcagccgtagcgccagttaagtattacgccagctcgaccattttgttgtcgatcaggcgagcatcgccaagccaggcggctaccagaattactgcccgtttgctggtttcagaaacttccagcaatgtgtcggcatcgcgaatctgaatatcatcggcgcggaagcctttttcattcagttcttgccccgcaatggtaataatttcatcgagatcccgttccccagcctgcaatttgtcagcaatcgaacttaaaactttgtacagaccaggcgcaattttgcgttgttccgccgtcagataaccgttacgggaacttagcgccagaccgtctttggcgcgcataattggcacaccgacaatctcaatatcgaagcccatatcggcaaccattttgcggatcagcgccagttgctgaaaatctttttcaccgaagcaggcgatgtccggctggaccaggttgaacagcttgctgacaatagtcgaaacgccgcgaaaatgtcccggacggctggcaccttccagcatggtcgaaaggccaggaacgtcaacgtaagtgtgggtttcagtaccgttcgggtagatctcttttaccgaaggggcgaaaactaaatccactttacgtttgtttagcttctcgcagtcctcctgcaaggtccgtggataacgagccagatcttccgggcggtcgaactgcatcgggttaacgaaaatactgacgacgaccacatcggcgcgggctttggcttcgtcgaccagcttcatatggccatcgtgcaggttacccatggtaggcaccagcgccacgcgcttgccttccatacgcaggcggcgaatttgctgacgcagcagcggcagggtttcgataattaacacaacgtgactccttaatggaaactgtgttcttcgcccggataaacgccggactccacttcagccatatactgccgcacagccgcgcggatgtcgcccgtttcggcgaggaaatttttagcgaatttaggaatgtgaccgccggtaataccaaaggcgtcgtgcatcacgaggatctgcccgtcagtgacgttgcctgcgccaatgccaataaccgggatcgccagtgcttcggtaatacgttttgccagttcaaccggcacgcattccagcaccagcagctgtgccccagcagcttctaaggctaatgcatcgctgagcagttgatcgcccgcttcatcgccgcgcccctgaactttgtagccaccgaaaatattcactgactgtggtgttaaacctaagtgaccacatacaggaacggcacgttcggtcagcatttgtacggtttctaccagccactcaccgccttcaattttgaccatgttagcaccggcacgcataaccgttgcggcgttttcgaaggcttgttccggcgtggcatacgccataaacggcaggtcagccagcagcaggcagtttggtgcgccgcgacgtacggcggcagtgtggtaggcgatatcggcaacggtaactggcagggtggagtcgtgcccctgaaccgtcatgcccagcgaatcgcccaccagcatgacgttaagcccttcatcagcaaagagtttggcgaagctatagtcataagcggtgatggtcgcgaaacgttttttttcctgtttgtacttctgcagtaaggagatggtggtcggtttcataacgtatcctgataaattgatgttgtgctgtctggcattttatcagtcacattggtgggggcaatgatttatccgtagcagcactgccagaaggtgacagtgctgctacgttatcagggataggttacctggaaagtactggtggctttaaattcgccgggttcgatagcaatattcccgtcttgctttaatgttgcctggaaatgaagaggctgtgatgtgccgttaccttgattagggtaaaccccatcggaggtgtcatcttcggtttcataatctatataaacagaattcgtatcattaggttttaatgtcattagcggatttttactggttgctaaaccttcaatgagtacgccaacgcctttggcggcagtgcttccagtaagcgtattaccaagcagttgtgtgttttgagtacctacttttccagtgacgagttttgtttcaatattacgcacacgaatacaattctgaagcgagatatcaaagggaacaggtgaagcgccatttttaattgtcccagagctatattctcccattctaaccgttgaaccattgactgatggcccggtaagtatggaggtaaaacatgttggtaaggttaatttgacattattcagtgtgaaattgacataaatgtggttgctgtgatctacaacttttgtaccaggactgtaggccttaaacgaataaaggtaatttgatgaactggataactggacttgctgattaagtgtaggatcgaaattagtatctgtataaaattcaacagttatgttgtgtactataccaccaatagcccaaaacttatcgtagtcgtctgctttgttgcaacccttagtttgtagatcgctgtctgtgacggaaaagaaaaattcttggttggaaggatctccgatatagattcctggcgattgaatgtcagttattgtatcgtatgcagaccagacccttgatattaacatggtgtaatacagaccaggaacagatgtattaaatagtttatgtccgccataatctttacctgaatagaccatggcattttcaatagttattggaccaggattcgctctgccagatgtattgcagtaaagaataccaccaccggtacctgtatccaggtatgaccagtacatttttaccccagtcgggccgagctgcgtgggtttataaaaaaccaagttgcttgctgttgatgtgtaattaaaggtcatctgtgcggcagtggaggggcctcgatagttatcaactcctgcattatttcccacaataaaacttgtatatgcactgactgtattacaacaagaatacagtgctaaaaaaagaatgtacctgaagatagtcttcatttttactccaatgtttctttattgttatggtttgcgctgtttttgtttgttattcgtagtaaatatccactaacacatggctcataagttgaccagatgtaacactcaatgcaggatcgattttttgcattcgggtgctaaatttccaggatgaaccattcatgtcatccgacattactggataaacggaacgagatccgcctgaagcattaagaacattgaatgtattcgccgaatcctgagtagaaaatataactactcctacattacttgctcctgacgaaatttcattagcaaatatttgcctagagccagcagccatgacaccgctaagggctctaaaatcaatatgtaactgatttagcacatcgccagttccctgtaatgcacagtcggatacagtgatagtgaactcttttccacctggttgataactttcaggagtaacattacctgaaaaatatcccaccccaacgacgccaagatcaatattaccctggttactgattccgcttttgcaggtgctgttttttacattggcaacaaggtcaatatcctgtccagcaatggctggacaggcgatgcaaaacagtaatgacagaaacagaattattctcttcatcagcttacgttgagtgggatgcatatatagttcctgaatctgtaagtctgttagttataggttactgtaaatgtggctggtgcagaaaacttacccgcagtgacattgtttacggttttatttttttccacgaccaggcgtgcactcatcggataataaacgaccgcattggctgcagtggagattgttacctcttgtgatgctggtgttacacagctaaattgtgttgcactccctgttgccggagttacagtgctccagacttcaacggcgacagcacttgctttatctgcggctgtggaaccatttgcaaaccccgcaccgtcattagcagttccctcgcatgtggctcgcttggttaattttatttgcgcttttttattggggatacccgcacagtctttgaatttgagtttgaatgtttttactttggtcttggcattgatttcagaaatatatacatcaccaaaatcaacaacagaaatgtcctgatcagagtcatttactaatgtagcggtacaagtacccatttctacagtagtaataacggtcagtccaatactgtctgttgccgcataagagagtacgctgaacaatgaggcagccaaaacgacactgctggataatccataacgtaaatttttaaatgtcatcataattatccttcttattgatagatgaaattaaacgtcgccagtgcacgaaaattccccggtacgccttgccctgcatctgtttcacgtagcgcaacggtcatttcaagacccttatcgggctgcatctcgtctgtgctccagcgtatcttttccgcactgttaggtttaaggaaagtggcatcatcagtagtccgttttttgaaacccataccgatattacttgtcgtcgaagatgaatcaccagactgcggtataataagcttaggtgagcttgatgatgcatttccggtcagagtggtatcaatccaactgatgccactgctgcacccactggcaaccagtttaaaatcagcctgagattctgtcgttttattcgcgatcttatccagacccatcttagggattctcaatgtgtagttattattgccatcattcgtgacgttattaccagtaagtgtgatgttacaggttgtcgctttgacagtggctgtaaactctacattaatatccgttgcaaatactgagggtgataataatattcccatcagtatcactattttatgtggcgttgtttttatcatttgacgtcccttgtagttactgaatctgacaccgaattccattcagaataatagattgtgctattttttctgcttctgggctttgttgataatgcgcaagacaacttacgggtttactttgttcgagccatttaatgctgatatttccctgctgctcaataccacgaacaaatgcttgtccaccctgtccaacattaccaatgacattgccttgctcatcataaatatctgcagcaaatggaatatttttaccatcacttcgtgtgatgttcataatggctgattgcccttgcacggtttcaaaatcagcaaagacgactgaaccctgacgcggtacagctactgcactggtactttttaattcaacatcgttctcaagatcgttgatatccagcgcgatacggttttcatgataaggagaaagagcgctggtgacaccataaccccatcgatcgatagtactgttgccataatttattcgcgctccttgagcacctggagcctgaactaccgccagtgtatcggagtcgctaaaactatcattactgaaagtcagtccaccgctatgcaatacaaaaccaccgtcggtgctgagagaaacttgacggctgttatcgctatttgcagaaattgaacctgccagcgttccccatggtgactcatagctggcataacccccaacataactcaaatctttgctggctttattcatcgtatagccagtattcacgctataactgacgcgagcgttatcgctatagccactgctgctaacgttgagttggttattacccttaaagtcactgcttatttgagtatcaatactctggaaacctgaagtacgttgttcagtgccaagtaatttttcaattggaatggtgaaactaagataaacgctatcgtcagtgtcgccgtcttcattccatgaacgctgggcactgacactgtagctgccccaggatgtactgttactgtagccaatagagtaattgctacgattttgtccggaagcccagtaatcggaccaacttccggaaagataaaatgaaccgtaatcttttttctcaaatttcaacggttggttaatactgaccgtaacctgatttttcatgcgtgagtaattacgcatggatttcggttcaagatcttgttcgggatgtttcacttcatcaattagagttagtgcatcattaagaccaaggtaattctgtgtcgaatagcgataggccgcgatattcagtgaagtacttgtttcttcgaataacttgttccaggaaacacgataactttgcccctggtatgttttatcatccgggatacgaacattggaatgagtcacatcgaaagaaaatgcaccaactgaagtattcagaccaagacctaacaaaccagcggtatagttattatcggttatctgaataccggtataacccgtcagatagttattcaggccgtagtagtagcttgcttgaaataaattaggctcatcctgaatatcatcttttaagacctgaccgccgctaatatcccaacgtccaacgccagggcgtaacatttgaacaacggatgagaaaggttgcgagaatgtccgctttgagccatcggattcttcgatggtaacaataagatcgctgccgtaccctgacggactcagatcatcaatgacgaaagcgcctggcggcaccgtcgtttcataaatcttatagccaccttgcgtaatagtgactttggcgttggtattggcaacgccatgaatgataggcgcaaagctggctaaagtcggaggcaacatgcggctgtcactgtataaacgaatgcctcggatactgacggaatcaaaggtttcgcccgtcgtataagactcaccaagaatgagttgagaacgcagcgaggcgatatcacgctgaacataccgattcttaaaatcataattactgccagaatcggtcatccagttgtagttgcccgaggcacgcagtcgccatgcacctaaattcatcccaccgttaaatgcagcataaatgctttcattttttcgaccaggggtttcactatgatatccgttgaggttgtatgacaacatggccgcattaatgccgttttcccataacgatggatcaacatagttttggtaatttttcattacccaggcttgaggaacgtctatatccagacgttgatcgttaacgtcataacgaacagaagcctgagggataatttccgtcaaattgaggcaattgccgagcgtttcatccctggcaagcagaacggctttttcgttatttatatcgggagaattaatatgaaactgcaataaattctttaatgtgatacaagcctgggcgttcttttttccttcaattgcgacaaatgtaatactttggttaatgattggttggtcgtttacataaacactgacgtcgtaaacacccggtatagcggggttaccttcactgtaccggctgagatcaatattagatgcattctgccccatcaggaaggtatggtcatattcaacgagttcagcactgaaagcagtattgcaatacagcagcgcgcaaaacgtggcgatacgggtcagatgatgataatttttagtatattctatagtcacgctatgcttcctgcggaattatatccttgcctgattacagcctggcattaccttcaattgcgccaccaaagtcattaatggcgtaaaaatgcacttttgcagaattcgctttgccattaaggccattgactttcatgacctcatcactaaatggtgcaatcattttcacatcaatcggatagcgtttaccgctagcttctaaatcaccactgctaaaagagacgtagtaaggggttggattggtcactcgtaatgacgccttaccttctgaacctgaccagaaccacttcagggctaacggggcttcagagggatttcccttcaatccatccgggcgatagaaaagttttatacgtgtgcgaaatgccagttgcagcaggctttgattcgcgaccttttctgcatctggttttggtggaacttccagtacgttaaaccagaacacgctctctctgtctttaggcagtgaggtgctggctgtgtacattaatttgattgtttgcccacgtttggcatcaatacgcgatactggcggcgtagcagtaaaagggactgtaatactgccaggctcagcgttgtcatcgccagtatctaaccaactctggacaagcaacgggttattccctttattttccagacgtacgttgacacttttttgatcgcttttatatattacgcgagtacccgaaatgacaatgtccgcaatagacgatgaactaaaagccatacaggttacgaagcataaagctgttgtatgtttggtgttaaaaaacataaaccatccctgatagagttaattaaaacagggaataatataaaatagaaattattattccctgtatattcattcaatcaatttaactggtgaatacttactgataagtaatggtgtatgcagtgttagtttttacataaccagcagttgctgtttggtctgcgacggcacgaacgtaagacgctttaaaatcataaacagcagattttgtcgttgcatccagggctttagtatacacatcgccagggttgttaatttgaacctgtttgatagtggaaccatcaatattgtgtagagcgatattaacgccgtcagatgggttgttaatagacatgtcgttgttcaaagtccctttgctgttaccaaagaaaacagaaccgaaggtcattttagccgtgctacctggattcggatttgctttgctgcagtcaacggtgatgctgaaaggtttagctttagcgccaacggtgtcattcagtacgccagcatcgatttcaccaacggttgcggtttgcagcaggatcagaccatccttgttaccgccgtcaacgcgggtttcacaggtgttatcaacaaccagaccactgatatttaactgaccgccgtccatatcagcagaagcagtacctgcaaccatcgccagcataagaccagacagggcaaaacctaattttttagacataaaaatcctttaataaaattccattagtcagactacatgtttgaagaatgactattcatgacacaaataggagaaacaaatgttagatattaatgagcaatgatatttgttacccaaatttacaaccattgttcattaggtcgcctattgtgcactttagaagcttttgaacaaattaaatttacttaattcaaaattaagtaaaaataagttcacaagtgcaattggttagggtatggagatgggattgatatttatttataggaagttatattatttccgcaaagagatgtttaaactaaaatcgtaattaaggaaagagatgagatatgattttcagaaaatatttatattcgcaatataaataaattaccatttgtttaatttgtcaaatgctcttgtatgtaagatttgacgcaacatctccccatcaggaaacaccaactccggcgcgatttcaaacagcggccacagcataaatccacgattcttcatatcgtagtgcggaacggtcaggcgttcagtatttatcacttcattaccaaacagcatgatgtcgagatccagcgtgcgtggtccccagcgttcagctttgcggacgcgaccttgctgcaattcaatacgctgtgtgtgattgagtagctcttcaggtgcaagagaggtttccagcgccacggctgcgtttaagtaatcgggttgatcttgcggccccagcggtggggtgcggtaaaacgaagaaacggtaagaatgtggctttcagggatatcgcctaatgctttcagggcagcattgacctgctccagcggagaggccagattgctgcctatggcaatatacgccactgtcatgcggtaccctcacgacgtggtgcgcgtttgcgtggacgacgagtacgacgacgcggtgacggttcttcatccagctcgttgagcatccctttttggtctggtggcgcggaaacctggaactcaccccaccatttcaccagacgctgcagttcagcgttacgctcaacttcagctcgcaaggccaacaggtcataagccgcacggaacttaggatgctccagcagtttccatgcgcgtttaccctgacgacgggacatacgcaactgcaactgccagatatcgcgggttaatgtcgtcagacgtttcgggattgccagtgaacggcaggcttcgtccagcacgtcgttcatcgccagcgcgaaagcgtcgtgataggtcaggccgctttcctgggcgatcttctgtgccgtctccagcagtgggtaccagaacatggcggcaaacaggaacgccgggttcacgcgcatatcgttatggatacgcgtatcggtattcttcagcacctgttcaatgatccgctccatcgggctgtcgccattttccgtgaagtagcgggtaatggtcgggaacagcggctggaacagatgatattcacacaacagcttataggtttcgtaaccgtagcccgcttgtagcagtttaagcgattcttcaaacaggcgtgccggtgggatatcgttcagcagggtagcgaggcgagggatcggttctgcggtttccgggctgatgcgcatacccaatttggcggcaaaacgtaccgcgcgcagcatacgtaccggatcttcacggtagcgcgtttccgggttaccaatcagacggataacgccgtccttcagatccttcatgccgccaacgtaatcacggacggtaaaatccgctacgctgtaatacaggctgttgatagtgaaatcgcggcgctgggcgtcttcttcgatggagccgaaaatgttgtcgcgcagcaacatgccgttttgcccgcgttgggaggtcgtgcggtcgctgacgttaccttcgtggtgtccacggaaggtcgcaacttcgataatctccgggccaaacattacatgagccagacggaaacggcgacccaccaggcggcagttacggaacagtttgcgcacctgctcaggcgtggcgttagtggttacgtcaaaatctttcggctttttgccaagtaacaggtcgcgcacgccgccgccaaccagccaggcttcgtatcccgctttattgagcctgtacattaccttcagggcattttcactgatatctttgcgggaaatagcatgctgctcacgcgggatcaccgtcacctgtggacgggcgactgcctgttcagcctcgctttcctcgcggcttagcaccttgcggcaaaaattagcgactcgggtaaaaatagtacacctcggtagtgtcaaacatcattcaggacaaaaaaatagcggctaatcatagctcagcatgacgcatttgagaatgttgaatttacaattgccgactcgggcacggcggtaagccgccagtttttgacggctgactgaaggatttgctcgacgctgaaatcctgccagtgtgcttctgcctgctgccccagaaattgaagtgccgcgattagtaccgggcgtggatcgcctttcggcaacgcaggcgcatgattctgcttggaaagtttagcgccttgtggattaagcgccagcggcagatgaatgtaatctggcactttccagccaaaaagctggtacagcgagatttgccttactgttggttcaatcagatcagccccacgcactatttctgtaacgccctggaaatgatcatcaaccacaacagccaggttgtaggcgaacaacccatcacggcgatgaatgataaaatcttcccgtgccagtttttcgtcggcgtgaataatgccgcgcagctggtcagtaaattgcgtgaccggatgctgctggcggatacgcactgcggcgttgtctggtccatgatgcaacacccggcaatgaccgtcgtaaataccgccaatgctttgaatacgcgcacgcgtacaggtgcagtaataacttagtccttgttcatgtaaccaggcgagtgcttcacgataggcgtcgtgacgttgcgattgccagagaacatcgccgtcccagtgcagaccgtaatgttccagctggcgcaggatagtttctgcggcaccgggaacttcacgaggcgggtcgatatcttctatgcgtaccagccagcgaccttgccgggcgcgagcctgcaaatagctgccgagcgcggcgatcagagagccaaaatgaagctcgccggaaggagagggggcgaagcggccaatatactgtgtgtctgtcatctctttgaacaaaaaataaggcgggagcatttcccgcctgtggtaaacgtgatggaacggctgtaattagccagccatctgtttttcgcgaatttcagccagcgttttgcagtcgatgcacagatcggctgtcgggcgcgcttccagacggcgaataccaatttcaacaccgcaggattcgcagtagccgaaatcttcgtcttccacttttttcagcgtcttctcgatctttttgatcagcttacgctcgcgatcgcggttacgcagttcgaggctgaactcttcttcctgggctgcacggtctaccgggtccgggaagttggctgcttcatcctgcatatgtgtaacggtgcgatcgacttcatccctgagttgattacgccatgcttccagaatacgacggaagtgcgccagctgggcttcattcatatactcttcgcccggcttctcctgatatggttccaccccagcgatggcgagaatactcagggacgatgttttacggttttgcccttcttgcatgttgcttctccttaacacgcactatcgatccccatgttcgggggaaaaatgaggccgctataaatagcagatgcttttccggatagcaattatctaaacgtaacacttgacaactgtgtgaggaaaagcgtatttgcgcacgcgaccagaatgtaaattaaccagttacttactttactacaatgtaaccggcagtgattttttaagagccatgccttcagcagaaatttccgctttgtaagccagaatttctacccccctctgttgagcttctgacaatagttgcgcgtatttctcatcgatgtggcgcgcgggtgaaaaccgtgtaatggctgaatgcagcacggcgaaaaagataaccgcacgctggccttcagccgctacgctcatcaactcccgaaggtgtttctgacctcgttcagtgaccgcatcgggaaaatatccctgttcgttctccgctaacgtaaccgatttcacttcaatatagcagtctggacgcgaatccgcctgcaacataaagtcaatacggctgcgttctgcgccgtattttacttcgcttttcagcgagctatagcctgacagttctgaaattgattcattaaggatagcctctttcgtcaacctgttagcccaaagcgtgttgacgcaaataaatgcgccgctctggctttgagttaattcccaggtgtgtgggtatttccgtttggtgttgtctgaagtcgaataccagacggtatcgccaggcgttgcacaaccggtcatcgcacccgtattcgggcagtgtagcgttaattcgcgaccatcgggtgtgatcacatcggctaaaaaacgtttgtaacgctgaattagcgtcgcgcgctgtagagggggagaaaattccattgcgacaatccttgttattgcgttagcgcccagcgttttagcggcgtgtagcgtgtgcgtccacgggcaaacgaggaggcgtaaagggtgaactccgtcaccgcatacgaccagttaaaacctggcggcgggattgtcaccgcctcgctggcgtcgcgcaataaggtaatatgtggatgaaacggacgattgctttgaaaacaaccgctgcgggcagcctgtgaacggagcatattcgccagctggattaagccgcgtggcggctgacgcatccctaaccacaccacacgcgaacgcagccattgtccggcgtcatcaagcgtgagtgtgaaaccaggttgacgaatccgtccggctaaaagagaaagcgccttctctttctcggcgctcacttcgcctaaaaatgccagagtcagatgcaaattatcggcggcgaccggacgtcccgcctcaggtgggaagtgtgtggcgcgccaatggataatctgttcgcggatttctgcaggtaagtcgatagcaaagaacagacgttgcggttcagacatgtgaggcactcggttatgaattaccgcgatgctacaatgtggcgcgaagaatgttaaccctctggagcgttttgtgtcgtcgttgcccgttgctgccgtcttacctgaattacttaccgctctcgattgtgcgccgcaggtattattaagtgcgccgaccggggccgggaaatcaacctggctgccgctgcaactgctggcgcatcccggcattaacgggaaaattatcctgctggagccgcgtcgtctggcggcgcgtaacgtcgcgcaacggctggcggagctgcttaacgaaaagccaggcgataccgttggctaccggatgcgtgcgcaaaactgcgtcgggccgaatacccgcctggaagtggttaccgaaggcgtgctgacgcgcatgatccagcgtgacccggaactgagcggtgttggactggtgatccttgatgaatttcatgagcgcagcttgcaggcggatttggcgttggcgctgttactcgatgtgcaacaaggtctgcgtgatgaccttaaactgctgattatgtcggctaccctggacaacgaccgcttgcagcaaatgctgccagaagcgcctgtcgtcatctcagaagggcgctcgtttccggttgaacgccgttatttaccgctgcccgcgcatcagcgttttgacgatgccgttgcggtagccaccgctgaaatgctgcgtcaggaaagcggatcattactgttatttttacctggcgtcggagaaattcagcgtgtgcaggaacaactggcttcgcgcatcggcagtgatgtattgctctgcccgctgtatggcgcgttgtcgctgaacgatcagcgaaaagcgatcctcccggcaccgcaagggatgcgcaaagtggtgctggcgaccaatattgctgaaaccagtttaaccattgaaggtattcgtctggtggtggattgtgcccaggagcgtgtggcgcgttttgatccgcgcacggggcttacgcgactgattactcaacgcgttagccaggcatccatgacgcagcgtgccgggcgcgccgggcgtctggagccgggtatcagcctgcatttaatcgccaaagaacaagcagaacgcgccgcggcgcaaagtgaaccggagatcttacaaagcgatctttccggtttgctgatggaattactgcaatggggatgcagcgatccggcgcagatgagctggctggatcaaccgccagtagtgaatctactggccgcgaaacgtctgttacaaatgctgggggcactggagggtgaacggcttagtgcgcaagggcaaaaaatggcagcgctgggtaacgatccgcgtttagcggcaatgctggttagcgcgaagaacgacgacgaagctgctaccgcggcaaaaattgccgccattctcgaagagccgccacggatgggcaatagtgacctgggcgtggcgttttcgcgcaatcaaccagcctggcagcaacgtagtcagcaactgttaaaacgcttaaacgtacgtggcggtgaggcagacagttcgcttatcgcgccgctacttgccggggcgtttgccgatcgcattgctcgtcgccgtgggcaagatggacgctatcaactggcaaacggcatgggagcgatgctcgatgccaacgacgcgctaagccgccacgaatggttgatcgcaccgttattattgcagggcagcgcctcgccggatgcgcggattttactggcgctgctggtcgatattgatgagttagtacaacgctgcccgcagctggtacagcagtctgacactgtggagtgggatgacgcgcaaggtacgctgaaagcctggcgtcggctacaaatcggtcagttgacggtgaaagtgcagccgctggcgaaaccgtcagaagacgagttgcatcaggcgatgcttaatggcatccgtgataaaggtttaagcgtgctcaactggacggcggaagcggaacagctacgcttgcgtttgttatgcgccgcaaagtggttgccggaatatgactggccagcggttgatgatgaaagtttattggcagcgctggaaacgtggctgctgccacatatgactggcgtacattcactacgcggcctgaaatcactcgacatttatcaggcactacgcggattacttgattggggaatgcagcaacgtctggatagtgaattgcctgcgcattacactgtgccgacgggaagccggatcgccattcgttatcatgaagataacccgcccgcgctggcggtgagaatgcaagagatgtttggcgaggccaccaatccgacgatcgcccaggggcgcgtgccgctggtgctggagttgctttcacctgcccaaaggccattacaaatcacacgagatttgagcgacttctggaaaggagcgtaccgtgaggtgcaaaaagagatgaaagggcgttatcccaaacatgtctggccggacgacccggcaaatactgcaccgacgcgacggacgaaaaagtattcgtaaggttggttttctccctctccctgtgggagagggccggggtgagggcatcagcgcgcacgttcaccctcaccctaaccctctccctcaagggagaggggaccgatcgagcacaaattttgagagatatcttcttctgtcttgtaacagaagaacagaaaatcgggcttttgcgcctgaatattgcggagaaaaagcatggccgggaatgaccgcgagccaattggacgcaaagggaaaccgacgcgtccggtcaaacaaaaggtaagccgtcgtcgttacgaagatgacgatgattacgacgattatgatgactatgaggatgaagaaccgatgccgcgcaaaggtaagggcaaaggcaaagggcgtaagcctcgtggcaaacgcggctggctatggctactgctaaaactggctatcgtttttgccgtgctgatcgccatttacggcgtttatctcgatcaaaaaattcgtagccgtattgatggcaaggtctggcaactgcctgcggcagtttatggccgaatggtcaatcttgagccagacatgaccatcagcaagaacgagatggtgaagctgctggaggcgacccagtatcgtcaggtgtcgaaaatgacccgtcctggcgaatttaccgtgcaggccaacagcattgagatgattcgccgtccgtttgatttcccggacagtaaagaaggacaggtgcgcgcgcgtctgacctttgatggcgatcatctggcgacgatcgtcaatatggagaacaaccgtcagttcggtttcttccgtcttgatccgcgtctgatcaccatgatctcttcgccaaacggtgagcagcgtctgtttgtgccgcgcagtggtttcccggatttgctggtggatactttgctggcgacagaagaccgtcatttttacgagcatgatggaatcagtctctactcaatcggacgtgcggtgctggcaaacctgaccgccggacgcacggtacagggtgcgagtacgctgacgcaacagctggtgaaaaacctgttcctctccagcgagcgttcttactggcgtaaagcgaacgaagcttacatggcgctgatcatggacgcgcgttacagcaaagaccgtattcttgagctgtatatgaacgaggtgtatctcggtcagagcggcgacaacgaaatccgcggcttcccgctggcaagcttgtattactttggtcgcccggtagaagagctaagcctcgaccagcaggcgctgttagtcggtatggtgaaaggggcgtccatctacaacccgtggcgtaacccaaaactggcgctggagcgacgtaatctggtgctgcgtctgctgcaacagcaacagattattgatcaagaactctatgacatgttgagtgcccgtccgctgggggttcagccgcgcggtggggtgatctctcctcagccagcctttatgcaactggtgcgtcaggagctgcaggcaaaactgggcgataaggtaaaagatctctccggcgtgaagatcttcactacctttgactcggtggcccaggacgcggcagaaaaagccgccgtggaaggcattccggcactgaagaaacagcgtaagttgagcgatcttgaaactgcgattgtggtcgtcgaccgctttagtggtgaagttcgtgcgatggtcggaggttctgagccgcagtttgcgggctacaaccgtgcgatgcaggcgcgtcgttcgattggttcccttgcaaaaccagcgacttatctgacggccttaagccagccgaaaatctatcgtctgaatacgtggattgcggatgcgccaattgcgctgcgtcagccgaatggccaggtctggtcaccgcagaatgatgaccgtcgttatagcgaaagcggcagagtgatgctggtggatgcgttgacccgttcgatgaacgtgccgacggtaaatctggggatggcgctggggctgcctgcggttacggagacctggattaaactgggcgtaccgaaagatcagttgcatccggttccggcaatgctgctgggggcgttgaacttaacgccaatcgaagtggcgcaggcattccagaccatcgccagcggtggtaaccgtgcaccgctttctgcgctgcgttcggtaatcgcggaagatggcaaagtgctgtatcagagcttcccgcaggcggaacgcgctgttccggcgcaggcggcgtatctgacactatggaccatgcagcaggtggtacaacgcggtacgggtcgtcagcttggggcgaaatacccgaacctgcatctggcagggaaaacagggactaccaacaataacgtagatacctggtttgcgggcattgacggcagcacggtgaccatcacctgggtcggccgtgataacaaccagccgaccaaactgtatggtgccagcggggcaatgtcgatttatcagcgttatctggctaaccagacgccaacgccgctgaatcttgttccgccagaagatattgcagatatgggcgtggactacgacggcaactttgtttgcagcggtggcatgcgtatcttgccggtctggaccagcgatccgcaatcgctgtgccagcagagcgagatgcagcagcagccgtcaggcaatccgtttgatcagtcttctcagccgcagcaacagccgcaacagcaacctgctcagcaagagcagaaagacagcgacggtgtagccggttggatcaaggatatgtttggtagtaattaacatctaagcgtgaaataccggatggcgagttgccatccggtaaaataacatcccatctaagatattaaccctttcttttcatctggttgtttattaacccttcaggaacgctcagattgcgtaccgcttgcgaacccgccagcgtttcgaatattatcttatctttataataatcattctcgtttacgttatcattcactttacatcagagatataccaatggcgcgttccaaaactgctcagccaaaacactcactgcgtaaaatcgcagttgtagtagccacagcggttagcggcatgtctgtttatgcacaggcagcggttgaaccgaaagaagacactatcaccgttaccgctgcacctgcgccgcaagaaagcgcatgggggcctgctgcaactattgcggcgcgacagtctgctaccggcactaaaaccgatacgccgattcaaaaagtgccacagtctatttctgttgtgaccgccgaagagatggcgctgcatcagccgaagtcggtaaaagaagcgcttagctacacgccgggtgtctctgttggtacgcgtggcgcatccaacacctatgaccacctgatcattcgcggctttgcggcagaaggccaaagccagaataactatctgaatggcctgaagttgcagggcaacttctataacgatgcggtcattgacccgtatatgctggaacgcgctgaaattatgcgtggcccggtttccgtgctttacggtaaaagcagtcctggcggcctgttgaatatggtcagcaagcgtccgaccaccgaaccgctgaaagaagttcagtttaaagccggtactgacagcctgttccagactggttttgactttagcgattcgttggatgatgacggtgtttactcttatcgcctgaccggtcttgcgcgttctgccaatgcccagcagaaagggtcagaagagcagcgttatgctattgcaccggcgttcacctggcgtccggatgataaaaccaattttaccttcctttcttacttccagaacgagccggaaaccggttattacggctggttgccgaaagagggaaccgttgagccgctgccgaacggtaagcgtctgccgacagactttaatgaaggggcgaagaacaacacctattctcgtaatgagaagatggtcggctacagcttcgatcacgaatttaacgacacctttactgtgcgtcagaacctgcgctttgctgaaaacaaaacctcgcaaaacagcgtttatggttacggcgtctgctccgatccggcgaatgcttacagcaaacagtgtgcggcattagcgccagcggataaaggccattatctggcacgtaaatacgtcgttgatgatgagaagctgcaaaacttctccgttgatacccagttgcagagcaagtttgccactggcgatatcgaccacaccctgctgaccggtgtcgactttatgcgtatgcgtaatgacatcaacgcctggtttggttacgacgactctgtgccactgctcaatctgtacaatccggtgaataccgatttcgacttcaatgccaaagatccggcaaactccggcccttaccgcattctgaataaacagaaacaaacgggcgtttatgttcaggatcaggcgcagtgggataaagtgctggtcaccctaggcggtcgttatgactgggcagatcaagaatctcttaaccgcgttgccgggacgaccgataaacgtgatgacaaacagtttacctggcgtggtggtgttaactacctgtttgataatggtgtaacaccttacttcagctatagcgaatcgtttgaaccttcttcgcaagttgggaaggatggtaatattttcgcaccgtctaaaggtaagcagtatgaagtcggcgtgaaatatgtaccggaagatcgtccgattgtagttactggtgccgtgtataatctcactaaaaccaacaacctgatggcggaccctgagggttccttcttctcggttgaaggtggcgagatccgcgcacgtggcgtagaaatcgaagcgaaagcggcgctgtcggcgagtgttaacgtagtcggttcttatacttacaccgatgcggaatacaccaccgatactacctataaaggcaatacgcctgcacaggtgccaaaacacatggcttcgttgtgggctgactacaccttctttgacggtccgctttcaggtctgacgctgggcaccggtggtcgttatactggctccagttatggtgatccggctaactcctttaaagtgggaagttatacggtcgtggatgcgttagtacgttatgatctggcgcgagtcggcatggctggctccaacgtggcgctgcatgttaacaacctgttcgatcgtgaatacgtcgccagctgctttaacacttatggctgcttctggggcgcagaacgtcaggtcgttgcaaccgcaaccttccgtttctaatttctcttttggggcacggatttccgtgcccatttcacaagttggctgttatgcaggaatacacgaatcattccgataccacttttgcactgcgtaatatctcctttcgtgtgcccgggcgcacgcttttgcatccgctgtcgttaacctttcctgccgggaaagtgaccggtctgattggtcacaacggttctggtaaatccactctgctcaaaatgcttggccgtcatcagccgccgtcggaaggggagattcttcttgatgcccaaccgctggaaagctggagcagcaaagcgtttgcccgcaaagtggcttatttgccgcagcagcttcctccggcagaagggatgaccgtgcgtgaactggtggcgattggtcgttacccgtggcatggcgcgctggggcgctttggggcggcagatcgcgaaaaagtcgaggaagctatctcgctggttggcttaaaaccgctggcgcatcggctggtcgatagtctctctggcggcgaacgtcagcgggcgtggatcgccatgctggtggcgcaggatagccgttgtctgttgctcgacgaaccgacctcggcgctggatatcgcccaccaggttgatgtgctgtcgctggtgcaccgtttaagtcaggagcgtggcctgacggtcattgccgtgttgcacgatatcaatatggcggcacgctactgtgattatctggtcgccctgcgcggcggtgaaatgattgctcagggaacgcctgcggaaattatgcgcggcgaaaccctcgaaatgatttatggcatcccgatgggtattttgccgcatccggcgggtgctgcacctgtgagttttgtttattgatgagcggcttacctcttatttcgcgccgtcgactgttaacggcgatggcgctttctccgttgttatggcagatgaataccgcccacgcggcggctattgatcccaatcgtattgtggcgctggagtggttgccggtggaattactgctggcgctcggcatcgtgccttacggcgtggcggataccatcaactatcgcctgtgggtcagcgaaccaccattgccggactcagtgatcgacgtcggtttgcgcacagaacctaaccttgaactgctgaccgaaatgaaaccatcgtttatggtctggtcggcaggatatggcccttcaccagaaatgctggctcgtattgcgccgggtcgcggatttaacttcagtgacggcaaacagccgttggcgatggcgcgtaaatcgctgacggaaatggcagatttacttaacctgcaaagcgcagcggaaacgcatttagcgcaatatgaagactttatccgcagcatgaaaccccgctttgtgaagcgtggtgcgcgtccgttattgctgacgacgcttatcgatccgcgccatatgctggtcttcggtccaaacagcttgttccaggaaattcttgatgagtacggcatcccaaatgcctggcaaggggaaaccaacttctggggcagtaccgccgtcagtatcgatcgtctggcggcgtataaagacgttgatgtgctctgttttgatcacgacaacagcaaagacatggatgcgctaatggcaacgccgctgtggcaggccatgccgtttgtccgcgccggacgctttcagcgcgtacctgcagtctggttttatggtgcgacgctctcggcaatgcactttgtgcgcgttctggataacgccatcggaggtaaagcgtgagtaaacgaattgcgcttttcccggcgttattgctggcgctgttagtgattgtcgctacggcgctcacctggatgaacttctcgcaggcgctgccgcgtagccagtgggcgcaggctgcctggtcgccggatattgacgtcatcgagcagatgatttttcactacagcttgttgccgcgtctggcgatttcgctgctggtgggcgcgggtctggggctggtgggcgtgctgtttcagcaagtgctgcgtaacccgctggcggagccgacgacgcttggcgttgctacaggcgcgcaactggggattaccgtcactacgctctgggcgatccctggtgcgatggcgagccagtttgctgcgcaggcaggggcttgtgttgttggcttaattgtctttggcgtcgcgtgggggaaacggctgtcgccggtaacgctgattctcgcggggttggtagtgagcctttattgcggcgcaatcaatcagttactggttatcttccatcatgaccaactgcaaagcatgtttctgtggagcactggaacgctgacgcaaaccgactggggcggcgttgagcgtttatggccgcagctgctgggcggtgtgatgctgacgttgctgctacttcgtccgttaaccctgatggggcttgatgatggcgtggcgcgcaatctcgggctggccttgtcgcttgcgcgtctggcagcgctgtcgctggcgattgtcatcagtgcgctgctggtgaacgctgtggggattatcggctttatcgggttgttcgcgccgctgctggcaaaaatgctgggggcgcggcgtctgctgccacgactgatgctggcgtcgttgattggtgcgctgatcctctggctttccgatcaaatcatcctctggctgactcgcgtgtggatggaagtgtccaccggttcggtcactgcgttgatcggtgcgccgctgctactgtggctgttgccgcgtttacgcagcattagcgcgccggatatgaaggtcaacgatcgtgtcgcggctgaacgccaacatgtgctggcgtttgccctcgcgggcggcgtgctgctgttgatggctgtggtggtggcgctgtcgtttggtcgtgatgcgcacggctggacgtgggcgagcggggcgttgctcgaggatttaatgccctggcgctggccgcgaattatggcggcgctgtttgcgggcgtcatgctggcggtggcgggctgtattattcagcgactgaccggaaacccgatggcaagcccggaagtgctggggattagctccggcgcggcgtttggcgtggtgttgatgctgtttctggtgccgggtaatgcctttggctggctgttacctgcaggcagtctcggcgcggcggtgacgctgttgatcattatgatcgccgccggccgcggtggattttccccacaccgtatgttactggcggggatggcgttaagcaccgcgttcaccatgcttttgatgatgttgcaggcaagtggtgacccgcgaatggcgcaagtgctgacctggatttccggttcgacctacaacgcgaccgatgcgcaggtctggcgcaccggaattgtgatggtgattttgctggcgattaccccgctgtgccgccgctggctgaccattttaccgctgggtggtgataccgcccgagccgtaggaatggcgctgacgccgacgcgaattgcgctgctgctgttagcggcttgcctgacggcgaccgcgacgatgactattggaccgttgagttttgttggtttaatggcaccgcatattgcgcggatgatgggctttcgacggacgatgccacacatcgtaatttcggcgctggtgggtggtttactgctggtgttcgctgactggtgtgggcggatggtgctgtttccattccagatcccggcggggctgctgtcaacctttatcggcgcgccatattttatctatttgttgagaaagcagagccgttaatttttccatataacggccctgtacgcctggacggataaagcgtttacgcgacaacggatgcccgatgcgacgctggcgcgtcttatcgggcctacaaacggccccgaatcgtaggtcggataaggcgttcacgccgcatccgacaaaccatgctggatcacaacttcgcaaacacccgacgtgcagcatcgatggtgttattgatatcttccatgctgtgcgccacggacataaagcccgcttcaaacgctgacggtgccaggtaaacaccttcgtccagcatcatatggaagaaacgcttaaagcgttccacgtcacaggccatcacatcctgatagcacgtcacggactcggcgtcggtaaagaaaataccgaacatgccgccaacgtggttaacgaccagcggaattccggcttcttctgccgcttccagcagaccttctgccagacgtgttgtcagctcatccagcgtttcgtgaacgcccggctgcgcgacttcattcagacaggcgaaacccgctgccatcgcaatcgggttaccggaaagcgtacccgcctgatagaccggacccgtcggggccagcgcatccattacatcacgacgaccaccgaatgcgcctaccggcattccaccgccgatgattttgccgaggcaggttaaatctggcactacgccgtaataatcctgtgcgccagctagcgctacgcggaaaccggtcatcacttcatcgatgatcagcaacgcgccaaattcgtcgcacagcgcgcgcagacctggcaggaactctggcagcggcggaacacagttcatattgcctgccaccggctcgacgataatacaggcaatctcttgcgggtattgctcaaatgcggcgcgtacagaagccagatcattataagtacaggttaaggtatatttggcgaaatctgccggaacgcccggcgagtttggctggcctaacgtgagtgcgccagaaccggctttcaccagcaggcagtcagcgtgaccatggtaacacccttcaaatttaataattttgtcgcgaccggtaaaaccacgggccaggcggatggcgctcatggtcgcttcagtgccggagttcaccatgcgcaccatatccatggtcgggaccagttcggtcaccagttgcgccattttcacttccatttcggttggtgcaccaaagcttaaaccacgctcggcggcttcaatcacggcattgcggattgccggatggttatggcccagcaccatcggcccccaggaaccgacataatcgatataggctttgccatcaacatcgtacagataagcgccgtccgctttttcgataaacagtggagtgccgcccacgccagtaaaggcgcgaacaggggagttcacaccgccagggatcagctcgcgcgctgcgctgtaaagattttcagacttactcatggagggttcctgattcgtagaaaaagtgaatggctgctattctatgttattcataacaagttaaatactcgtcaaacatcaggctgcttgtactggtgcaatcctgatttcttagagtataaaagttttgtgcatttgaaacattacgctttgcaaaggattttcatggaacgtgcgagtaaaatgccgtcatcttatttgtatgaccaataagtgatcattggatgaaaactgatactccctctttagaaacaccgcaggccgcgcgcctgcgacgcagacaactgattcgccaacttcttgagcgcgataaaaccccgttagccattttgtttatggcggcagtcgtcggcacgcttgttgggctggcagcggttgcttttgacaaaggtgtcgcctggttgcagaaccaacgtatgggggcgctggtacatactgctgataattatccgcttctgttaaccgtcgcttttctctgttcggcggtgctggcgatgtttggctactttttggtgcgcaaatacgcgccggaagcaggtggttcggggatcccggaaattgaaggggcgctggaagatcaacgtcccgttcgctggtggcgtgtattgccggtgaagttctttggcgggctggggacactcggcggaggcatggtgttggggcgcgaagggccaaccgtgcagatcggcggtaacattggccgtatggtgcttgatattttccgcctgaaaggtgacgaagctcgccatacgctgctggcaaccggtgctgctgcggggctggctgcggcctttaacgcgccgctggcgggtattttgtttattatcgaagagatgcgtccgcagtttcgctatacgttaatttcgattaaagcggtatttattggtgtcattatgtcgaccattatgtaccggatttttaatcatgaagttgcgttgattgacgtcggtaaactttctgatgcgccgcttaatacgctgtggctttatctgatcctcggtattatttttggcattttcggccctatttttaataaatgggtgctggggatgcaggatttgctgcaccgtgtgcacggcggcaatattaccaaatgggtgctaatgggcggtgcgattggcggtctgtgtggattgctggggtttgtggcaccagcaacgtcgggcggcggttttaacctgattcctatcgctaccgcggggaatttcagcatgggaatgctggtgtttatcttcgtcgcgcgggtcattaccaccttactctgcttctcttccggcgcgccgggcggtatttttgccccgatgctggcgctgggtactgtgctgggaaccgctttcggaatggttgccgttgagctgtttccgcaatatcaccttgaggcggggacgtttgctattgccggaatgggggcattactggcggcatctattcgcgcgccgttaacggggatcattctggttctggagatgaccgataactaccagctcattttgccaatgattattaccggtcttggcgcaacactattagcgcaatttaccggcgggaaaccgctatactcggcgattcttgcgcgcacgctggcaaaacaggaagctgagcaactggcgcgaagcaaggccgcatcagccagcgagaatacttgaacgaaataccagggtattagataatggcgattattattgggttagaatttgcccaattgccgatgtcgtttggagcaaaatatgagtgatgacgtagcactgccgctggagtttaccgacgcagcagccaacaaagttaaaagcctgatcgctgacgaagataacccgaatctgaaattacgcgtgtatatcaccggtggcggttgcagcggcttccagtatggtttcacctttgatgatcaggtgaacgaaggcgatatgaccatcgaaaaacagggcgttggcctggtggttgatccgatgagcctgcaatatctggtcggcggttccgttgattataccgaaggtctggaaggttctcgtttcatcgtgaccaacccgaacgcgaaaagcacctgcggttgcggttcttcctttagtatctaatctgttgttcatgtgccggataaactatccggcacatcttctctcttcaacgcccattctcatccagcgcaaacgtcggtagcttaagatgccaacgaatagccgccagccgaatcaatagcgtcacgaccatgcccatcatactggctgtttccagtggtacggaaaatgtgtaataagccgtagcgtggacaataccgccgataatacaggcagttgcgtagatttctgtacgtaaaatcatggggatttcgcgggccagaacatcacgaatgatcccgccgccaacgccagtaatgacgcccatacaaaccgcgattaacggaccggcttccgcattaaaggctttattcacgccaatgccgacaaacaccgccagaccaacggcgtccagcaccggcaacatccattttggtaagcgtcttggctggcgcaccagcacgatggtcagcatgctggtgaccattgcaacgaccagatcggtgggatctttcacccaaaataccgggccgtgatccagcgccatgtcgcgaattgtcccgccgcctactgcggttaccacgcccagtaccagaacaccaaaagggtccatacgcaattttccggctaacaaaacgccggagatggcaaataccgctgtgccgactatatccagccaatagacgagcattgttcaatccccactgagcacctgaaaaggtcaggcgctaatctacctgtgaaagcgcattacagagctgttgtgcagcgaggataatacgtgggcttgcacgttcaaaccagtcactcgtgagaggaataacgggaattttgagctgttcaccccagtattgtttgattttaggaatttggtccggtccgcctgtaatgacaatcgcctgtggcgagcgtgctaacacctgttcgcggctaacttgcggccagggaacccggctgtctttaaagatgttttctccgccacaaacttcgagtacctggttctgaatcgactcttttccactggtaaatggcggattaatgccgaattgcagaaaaacacgttttttaggtttatcagcatattgcgctttcaattgcgcgtactgatccagcagggattgcgcggcttgttcggccttgtctggttgcggactccagggggccagttgacgtaacgcattggcaatttgttcaatgcttgtcgcatcgacccacatcacttttattcccagcgaagccagctggtcaacctgccgctcggcattacctccacgccaggcaatcaccagatcgggtttcagcgcgacaatgcgttccagattcatcccctgccaggtggaaacctgctcaatcttttgcgcttgtggaggatagtcggaatagctgctgaccccaaccggcgtgatcccggcggcaaaggcaagttcagtgttggcgggagaaagcgtgatgacgcgcggcgcggcgttgagccacagtggcgcaagaaaagacagggcgaccagcgccctgaacagtgacttagccatgtgcaagtttctgcaccagtgactcaaccatcaggctggactgtttagcggcaacagccaggaactcatcgaagctaagatgagactgttgatcggccacgtcggagatggcgcgtacgacaacaaacgggacgttgaaattgtggcagacatgggcgattgccgtcgcttccatctctacagcaatggcctgtgggaagttgtggcggattttcgccagaccaacagaaccgttgatgaaagcgtcgccgctaacaatcaggccacgtacagcgttaagattcagttcggcaatgcaggcctcagcggcagcgatcagtttatcgtcagctttaaagcctgccggacagcctggtaactgaccgtattcataaccaaatgccgtgacatccgcgtcgtgataacgtgcttcgtccgagacaacgatatcgcccactttcaacgttggtgccaggccaccggcagaaccggtgttaataatcacatctggcttgcagtgttccaacagcaaagtggcacccagcgccgcagcgactttaccgatgcccgatttcagaagcgcaacctcggttccattcagttggccggtatagatttcgcaaccgccgagactgatagtttgacggttttcgattttgtcacgcagcagcgtaacttcttcttccattgcaccaatgatgccgattttcatagatttactcgcgataagcccgatttgaaggcatagtttaccatgcgcttacggggaagcgtatttctcacgcgggagaggacatggcacagattgatttccgaaaaaaaataaactggcatcgtcgttaccgttcaccgcagggcgttaaaaccgaacatgagatcctgcggatcttcgagagcgatcgcgggcgtatcatcaactctccggcaattcgtcgtctgcaacaaaagacccaggtttttccactggagcgcaatgccgccgtgcgcacgcgtcttacccactcgatggaagtccagcaggtggggcgctacatcgccaaagaaattttaagccgtctgaaagagcttaaattactggaagcatacggcctggatgaactgaccggtccctttgaaagcattgttgagatgtcatgcctgatgcacgatatcggcaatccgccgtttggtcattttggcgaagcggcgataaatgactggtttcgccaacgtttgcacccggaagatgccgaaagccagcctctgactgacgatcgctgcagcgtggcggcactacgtttacgggacggggaagaaccgcttaacgagctgcggcgcaagattcgtcaggacttatgtcattttgaggggaatgcacaaggcattcgcctggtgcatacattgatgcggatgaatctcacctgggcacaggttggcggtattttaaaatatacccgtccggcgtggtggcgtggcgaaacgcctgagacacatcactatttaatgaaaaagccgggttattatctttctgaagaagcctatattgcccggttgcgtaaagaacttaatttggcgctttacagtcgttttccattaacgtggattatggaagctgccgacgacatctcctattgtgtggcagaccttgaagatgcggtagagaaaagaatatttaccgttgagcagctttatcatcatttgcacgaagcgtggggccagcatgagaaaggttcgctcttttcgctggtggttgaaaatgcctgggaaaaatcacgctcaaatagtttaagccgcagtacggaagatcagttttttatgtatttacgggtaaacaccctaaataaactggtaccctacgcggcacaacgatttattgataatctgcctgcgattttcgccggaacgtttaatcatgcattattggaagatgccagcgaatgcagcgatcttcttaagctatataaaaatgtcgctgtaaaacatgtgtttagccatccagatgtcgagcggcttgaattgcagggctatcgggtcattagcggattattagagatttatcgtcctttattaagcctgtcgttatcagactttactgaactggtagaaaaagaacgggtgaaacgtttccctattgaatcgcgcttattccacaaactctcgacgcgccatcggctggcctatgtcgaggctgtcagtaaattaccgtcagattctcctgagtttccgctatgggaatattattaccgttgccgcctgctgcaggattatatcagcggtatgaccgacctctatgcgtgggatgaataccgacgtctgatggccgtagaacaataaccaggcttttgtaaagacgaacaataaatttttaccttttgcagaaactttagttcggaacttcaggctataaaacgaatctgaagaacacagcaattttgcgttatctgttaatcgagactgaaatacatgaaaaaaaccacattagcactgagtgcactggctctgagtttaggtttggcgttatctccgctctctgcaacggcggctgagacttcttcagcaacgacagcccagcagatgccaagccttgcaccgatgctcgaaaaggtgatgccttcagtggtcagcattaacgtagaaggtagcacaaccgttaatacgccgcgtatgccgcgtaatttccagcagttcttcggtgatgattctccgttctgccaggaaggttctccgttccagagctctccgttctgccagggtggccagggcggtaatggtggcggccagcaacagaaattcatggcgctgggttccggcgtcatcattgatgccgataaaggctatgtcgtcaccaacaaccacgttgttgataacgcgacggtcattaaagttcaactgagcgatggccgtaagttcgacgcgaagatggttggcaaagatccgcgctctgatatcgcgctgatccaaatccagaacccgaaaaacctgaccgcaattaagatggcggattctgatgcactgcgcgtgggtgattacaccgtagcgattggtaacccgtttggtctgggcgagacggtaacttccgggattgtctctgcgctggggcgtagcggcctgaatgccgaaaactacgaaaacttcatccagaccgatgcagcgatcaaccgtggtaactccggtggtgcgctggttaacctgaacggcgaactgatcggtatcaacaccgcgatcctcgcaccggacggcggcaacatcggtatcggttttgctatcccgagtaacatggtgaaaaacctgacctcgcagatggtggaatacggccaggtgaaacgcggtgagctgggtattatggggactgagctgaactccgaactggcgaaagcgatgaaagttgacgcccagcgcggtgctttcgtaagccaggttctgcctaattcctccgctgcaaaagcgggcattaaagcgggtgatgtgatcacctcactgaacggtaagccgatcagcagctttgccgcactgcgtgctcaggtgggtactatgccggtaggcagcaaactgaccctgggcttactgcgcgacggtaagcaggttaacgtgaacctggaactgcagcagagcagccagaatcaggttgattccagctccatcttcaacggcattgaaggcgctgagatgagcaacaaaggcaaagatcagggcgtggtagtgaacaacgtgaaaacgggcactccggctgcgcagatcggcctgaagaaaggtgatgtgattattggcgcgaaccagcaggcagtgaaaaacatcgctgaactgcgtaaagttctcgacagcaaaccgtctgtgctggcactcaacattcagcgcggcgacagcaccatctacctgttaatgcagtaatctccctcaaccccttcctgaaaacgggaaggggttctccttacaatctgtgaacttcaccacaactccatacatcttcatcatcctttaggcatttgcacaatgccgtacgttacgtacttccttatgctaagccgtgcataacggaggacttatggctggctggcatcttgataccaaaatggcgcaggatatcgtggcacgtaccatgcgcatcatcgataccaatatcaacgtaatggatgcccgtgggcgaattatcggcagcggcgatcgtgagcgtattggtgaattgcacgaaggtgcattgctggtactttcacagggacgagtcgtcgatatcgatgacgcggtagcacgtcatctgcacggtgtgcggcaggggattaatctaccgttacggctggaaggtgaaattgtcggcgtaattggcctgacaggtgaaccagagaatctgcgtaaatatggcgaactggtctgcatgacggctgaaatgatgctggaacagtcgcggttgatgcacttgttggcgcaggatagccgtttgcgggaagaactggtgatgaacctgattcaggcagaggagaatactcccgcacttactgaatgggcgcaacggctggggatcgatctcaatcaaccgcgagtggtggctattgttgaggtcgacagcggtcagcttggcgtggacagcgcaatggcggagttacaacaactgcaaaacgcgctgactacgcccgagcgtaataatctggtggcgattgtctcgctaaccgaaatggtggtgttgaaaccggcgttgaactcttttgggcgctgggatgcagaagatcatcgtaagcgagttgaacaactgattacccgcatgaaagagtacggccagctgcgttttcgcgtttcactgggcaactattttaccggtcctggcagtattgcccgatcctatcgtacggcgaaaacgacgatggtggtgggtaaacagcggatgccagaaagtcgctgctatttttatcaggatctgatgttacctgtgttactcgacagtttgcgtggcgactggcaggccaacgaactggcgcgaccgctggcgcggctgaaaacgatggacaataacggcttgctgcgacgaacgctggcggcgtggtttcgccacaatgtgcaaccgctggcaacgtcaaaggcgttgtttattcatcgtaataccctggagtatcggcttaatcgtatatcggaactgaccgggcttgatttgggcaattttgatgacaggttgctgctgtatgtggcgttacaactggatgaagagcggtaggttatgcgttaaggttgaggcggcgctggctcattcccctcagcccgaagggtagaggggaatgcccgaattaaccgtcagttcgggattatttacgcgttagtttttccagatcggcttcaatctcgctgatcttattggttacgactgactccaggtgacgtaagtcgtcgaggatcttacgcttaagatcaacttcgctgcggtcacgctggcagatttgatcaagctcatcaatgatataccgtagattcgggctgatttcctggacttctttataaccctgacccacaccatcagcgacgaccgttttacgctgacgcggatatttaaacttaacgctcttggcgaaaaactcgcctttgtctttctggaaatagattttcagaatatcgttgttggcttcctgccggaggctgtaacgatcaatttcttcaggattggtaatacccagacttttcagattgtcgtacatagcgttacctcaaaatgagtcagtaaattgtgcttattttagcatttggcctggcccgcccggctcgactgtgatcgcagaaagcctttttcttccagacttctatcatggcgtaaaaatcaaaaaattacctgctttattctggtgataaaattcacgatctacaccagttccagcatcgttacttccgggcggcagttcagacgcaaaccatacaaactgcccacgccacgggttgtgtagatgtgtctttcgccaaaggcatttaatccggcgacgtaacgtttatcttcgacaggggcaaaaggttcaccaaccaacggtacgcgcagttgcccgccgtgagtatggccgcacagcatcagatcccagggttcatcacgcatgacttctttgctgtcgggattatgcgccagcaccagtcttggcagattggcttcgctggcgggaggcggtttgcattgtccggcccataagtcaccagtgcctaccagttcgaattgcctgttcggcgtggcgatcaccgtagcctggttaaacaacaccgtgatgcccgctgatttcaacgtctcgccaattaagtgatttttttctgtaccaacagggcgatcgtggttgccgaagcaggcaaacgtcggcgcacattcggcaaggggggagagtacgtcactaaacgccgaaaaattcagcgacatatcaaataatacgtaatcgccgcccagtaatatcaaatcgggcttttgttctatgccaagagcaatcgcgtcagaaatcaggcttaaaggaacaaaacgagagtaatggagatcggccagaaaaagaattttgaatggtgctgcgttgtctttaaaaaaggcgaggcggtgacggattaattcaaaccagcctggctcacagtaatgcatataaccgaaacctgagctcgtggctatcgtcgcggcagtagcctgcaaaaatcggcggcgtgaaatcatcgctcatccctgcaaaaaaatcgggcagcgtcgtgctgcccgtgtgcatacttttagtcgatggtacgcagcagttcgttaatgccgactttgccgcgagttttcgcgtcaactttcttaacgataaccgcacagtagaggctgtatttgccatcttttgacggcagattacctgaaacaaccacagaccccgccggaacgcgaccgtagtggatttcgccggtttcacggtcgtaaatacgggtgctctgaccaatgtatacgcccatggaaatgacggaaccttcttcgacaatcaccccttcaaccacttcagagcgcgcgccgatgaagcaattatcttcaatgatggttgggttagcctgcagcggttccagcacgccgccgatgcccacgccaccggaaaggtggacgtttttaccaatctgcgcacaagaaccgacggtcgcccaggtatcaaccatggtgccttcatcaacatatgcgccgatgttgacgtaagacggcatcagcacggtgttacgggcaataaacgcaccctgacgtaccgccgctggtggcacaacgcggaagccttctttctggaaacgtgcttcgtcgtagtcggcgaatttcatcggcactttgtcgaagtagcggctttctgccccttcgatcacctgattatcattaatacggaaagagagcagcaccgcttttttcaaccactgatgcgtcacccactgaccgtcaattttttccgctacacgcagtgcgccggaatccagcagggcgatcacctgatttaccgcttcgcgggtaacggtgtctgcattggctggcgtgatctcggcacggcgttcaaaagcggtttcaataatgttctgtaactgctgcattgttaaactcttttcatatcagtaaacacatcaccctttatcgtttggattgagggcctctgtcaaccgctgatgcacttcctgctgcaactcgttattaagcgcacgccggtcagcggtggcaattatgaataaatcttctactcgctcgccaatggttgtaattcgggcaccatgaagcgaaattcccagatcggcaaaaattttcccgactcgcgccagcagtccaggttggtcgagggcgatcagttcgaggaacgatttgcggtcggtatgggtcggcaaaaacgttacttcggtttcaacagtaaaatggcgtaatttggcgggttggcgacggggctgcggtggctgccagctactttgcgtcagtacttgctccagaccaaaccgaataacctcatgacgatctgcggacagcgggttgccatcgggttccagcacgataaaggtatccatcgccataccgtcgcgagtggtgaaaatttgtgcgtcgtgaacacttaaattgcggcggtctaattcggcacagacggcggcaaacagataagggcggtccgggctccagataaaaatctcggtgcctccacgcgtagcctgcgggctaagcaataccagcggtttgcttaaatcatgctgtaataaatggcgggcatgccaggccagttgatttgggctatggcggacaaaatagttagcacgacagcgtgaccaaatttggtgcagcgcctcttcgtcgatgttatccatgcgcagtagtgccagtgcctggagttggtgatggcgaacccgttcgcgcatatccggcgtgttttgcattccgcgtcgtagctgcttttcggtggcaaagtagagctcacgcaacagactttgcttccagctattccacagcgtttcgttggtggcgcaaatgtcagccacagtcaggcataccagatagcgcagacgattttccgtttgcacttcttcggcaaactgcttgatgacttccgggtcctgaatatcgcggcgttgggcggtcaccgacatcaacaggtgctggcgaaccagccaggcgaccagctgtgtttcgcgtgagttcagcccgtggagttcggcaaaatgcactacatcctgagcaccgagaatggagtggtcgccgccgcgtcctttggcgatatcgtgaaacagcgcggcgatgaaaatcagctcagttgacggcaggcgcggccagacgtccacacacaacggatggcgctggcgcgtttcttcactggcaaaactctccagtttcagcatcacgcggatagtatgttcatccaccgtgtaggcgtggaacagatcaaactgcatctgcccgacgatatgcgaccattgcggcatatacgcgccgagcacgctatggcgatgcattggcaatagcccgcgccgcaccgctccggggtgacgcagaatgctcaaaaacagttttcgtgcttccggaatattacacagcggttgttgcagatggcgacgggcatggcgtaactggcgcagcgtggtggagtaaatgccggtgatcgcactgttgtgcaccatggtgtagaacatacgcaagatggcttccggctggcgcataaatagtgtttcatcacgcaggtcgattagcgtaccgcgtagctgaaactcatcgtcgattggacgtggtttttcgtcggcgggaagggcgaggatggcttcatcgaacagttgcagcagcatctggttgagttcactgacgcggcgtgtaacgcggaagtaatccttcatcatccgctcgaccggttcgttaccttcaccactgtaattcagacgctgggcgacgctaagctggcgatcgaataacaggcgattatcgtaacggctgacgaccagatgcagggcaaagcgaatacgccacaatatatgcagacattcgtttaattccgcccgctccgctgaggttaagaagccaaacccgaccatttcatccagcgatgttgcgccaaaatgacggcgggccacccattgcagagtgtggatatcgcgcaagccgccagggctgcttttgatgtctggttcaaggttgtagctggtgccatggtaacgctgatggcgctggttctgttcttcaactttcgccgcgtagaacttgtcggaaggccagaatccttcgctgaaaatatgtttttgcagttcgaggaacagcgcaacatcgccaattaataagcgggattcgattaaattggtggcgacggttaaatccgataacccttccagcatgcactcttcaagcgtgcgcacgctatgaccgacttccagctttacatcccagagcagcgttaacagctcgcccactttttgcgcctgatcgtccgggagctttttacggcttaaaatcagtaaatcgacgtctgaaagtggatgcagctcgccacgaccgtagccaccgacggcgaccaatgccaggtcggcaatctggctgaatcccgcttcaatccataatcgttgcaggagctggtcgataaactcggtgcgcgcctcaatcaactgttctgcagagatcccattgtcaaaggcatcacccagccaacgctggaaagtatcgatatgggcttttatcccaccgacggttaattcatcacggggccagacgcatggattttgcggttgaccgggcagggtggggagagcggtgtttgcgtactgttctggaagggtattcattgtgcgccacccataagattaaattatcgcattaaaaaagccggcattcgccggcttcatcttattcgtcgtgcgagattatcgccgggatggtgtcatccttgcgtagcgtcagaatttcgcagccgttatcagtcaccacaatagtatgctcatattgtgcagacaagctgcgatctttggtttttaccgtccagccatctttcatggtgcggatctcttttttacccgcgttgaccattggctcgatggtgaacgtcatcccaggtttcagtacgacgttggtttcacgggagtcatagtgcagcacctgcggttcttcatggaagccgcgaccaataccgtgtccgcaatattcacgaacgacggagaagccttctgcttcgacaaatttctgaatcgccgcaccgatttcgcgcagattaatgcctggttttaccatgcgtagcgccaggtacaggctttcttgcgtgatgcggcacagacgttcgcccatgatggtcggcttaccgacgataaacattttcgaggtatcgccgtggaaaccatctttgattacggtgacatcaatgttaacgatatcgccatctttcagcagcttagcatcgtccgggataccgtggcacaccacttcattaatagagatgcaaacggatttcggatagccgtgatagccgaggcaggcagaaaccgcgtgttgttcattaacaatgtaatcattacagatgcgatccagctcgccggtgctgacgcccggtttaacatacggttcgatcatctccagcacttcggcagccagtcggccagcgacgcgcattttttcgatatcttctggggtcttgattgagatagccattaattctgtccatcagcgtcggtgataccgacaatatatatgtaagtgccgtcaatggtatcacacccgggcaaattgagaatcattctgaatttcgccaaacgtgccactgaaggttttctataatagaaaattcgacgtctgatgctgtacacagcgccaacaattattggtgtccacgacgtatttgtggtataaagcgcgccggacttccgatccatttcgtatacacagactggacggaagcgacaatctcactttgtgtaacaacacacacgtatcggcacatattccggggtgccctttggggtcggtaatatgggatacgtggaggcataaccccaacttttatatagaggttttaatcatggcaactgtttccatgcgcgacatgctcaaggctggtgttcacttcggtcaccagacccgttactggaacccgaaaatgaagccgttcatcttcggtgcgcgtaacaaagttcacatcatcaaccttgagaaaactgtaccgatgttcaacgaagctctggctgaactgaacaagattgcttctcgcaaaggtaaaatccttttcgttggtactaaacgcgctgcaagcgaagcggtgaaagacgctgctctgagctgcgaccagttcttcgtgaaccatcgctggctgggcggtatgctgactaactggaaaaccgttcgtcagtccatcaaacgtctgaaagacctggaaactcagtctcaggacggtactttcgacaagctgaccaagaaagaagcgctgatgcgcactcgtgagctggagaaactggaaaacagcctgggcggtatcaaagacatgggcggtctgccggacgctctgtttgtaatcgatgctgaccacgaacacattgctatcaaagaagcaaacaacctgggtattccggtatttgctatcgttgataccaactctgatccggacggtgttgacttcgttatcccgggtaacgacgacgcaatccgtgctgtgaccctgtacctgggcgctgttgctgcaaccgtacgtgaaggccgttctcaggatctggcttcccaggcggaagaaagcttcgtagaagctgagtaataaggcttgataactcccccaaaatagttcgagttgcagaaaggcggcaagctcgagaattcccgggagcttacatcagtaagtgaccgggatgagcgagcgaagataacgcatctgcggcgcgaaatatgaagggggagagcccttatagaccaggtagtacacgtttggttagggggcctgcatatggccccctttttcacttttatatctgtgcggtttaatgccgggcagatcacatctccgaggattttagaatggctgaaattaccgcatccctggtaaaagagctgcgtgagcgtactggcgcaggcatgatggattgcaaaaaagcactgactgaagctaacggcgacatcgagctggcaatcgaaaacatgcgtaagtccggtgctattaaagcagcgaaaaaagcaggcaacgttgctgctgacggcgtgatcaaaaccaaaatcgacggcaactacggcatcattctggaagttaactgccagactgacttcgttgcaaaagacgctggtttccaggcgttcgcagacaaagttctggacgcagctgttgctggcaaaatcactgacgttgaagttctgaaagcacagttcgaagaagaacgtgttgcgctggtagcgaaaattggtgaaaacatcaacattcgccgcgttgctgcgctggaaggcgacgttctgggttcttatcagcacggtgcgcgtatcggcgttctggttgctgctaaaggcgctgacgaagagctggttaaacacatcgctatgcacgttgctgcaagcaagccagaattcatcaaaccggaagacgtatccgctgaagtggtagaaaaagaataccaggtacagctggatatcgcgatgcagtctggtaagccgaaagaaatcgcagagaaaatggttgaaggccgcatgaagaaattcaccggcgaagtttctctgaccggtcagccgttcgttatggaaccaagcaaaactgttggtcagctgctgaaagagcataacgctgaagtgactggcttcatccgcttcgaagtgggtgaaggcatcgagaaagttgagactgactttgcagcagaagttgctgcgatgtccaagcagtcttaattatcaaaaaggagccgcctgagggcggcttctttttgtgcccatcttgtaaattcagctaacccttgtggggctgcgctgaaaagcgacgtacaatgtcgctagtattaattcatttcaatcgttgacagtctcaggaaagaaacatggctaccaatgcaaaacccgtctataaacgcattctgcttaagttgagtggcgaagctctgcagggcactgaaggcttcggtattgatgcaagcatactggatcgtatggctcaggaaatcaaagaactggttgaactgggtattcaggttggtgtggtgattggtgggggtaacctgttccgtggcgctggtctggcgaaagcgggtatgaaccgcgttgtgggcgaccacatggggatgctggcgaccgtaatgaacggcctggcaatgcgtgatgcactgcaccgcgcctatgtgaacgctcgtctgatgtccgctattccattgaatggcgtgtgcgacagctacagctgggcagaagctatcagcctgttgcgcaacaaccgtgtggtgatcctctccgccggtacaggtaacccgttctttaccaccgactcagcagcttgcctgcgtggtatcgaaattgaagccgatgtggtgctgaaagcaaccaaagttgacggcgtgtttaccgctgatccggcgaaagatccaaccgcaaccatgtacgagcaactgacttacagcgaagtgctggaaaaagagctgaaagtcatggacctggcggccttcacgctggctcgtgaccataaattaccgattcgtgttttcaatatgaacaaaccgggtgcgctgcgccgtgtggtaatgggtgaaaaagaagggactttaatcacggaataattcccgtgatggataaataagggtaagattccgcgtaagtatcgcgggggcgtaagtctggttataaggcgttattgttgcaggcagtttggtcacggccagcgcgcagcaaccggagcgtacaaaagtacgtgaggatggcgagcactgcccggggccaaaatggcaaataaaatagcctaataatccagacgattacccgtaatatgtttaatcagggctatacttagcacacttccactgtgtgtgactgtctggtctgactgagacaagttttcaaggattcgtaacgtgattagcgatatcagaaaagatgctgaagtacgcatggacaaatgcgtagaagcgttcaaaacccaaatcagcaaaatacgcacgggtcgtgcttctcccagcctgctggatggcattgtcgtggaatattacggcacgccgacgccgctgcgtcagctggcaagcgtaacggtagaagattcccgtacactgaaaatcaacgtgtttgatcgttcaatgtctccggccgttgaaaaagcgattatggcgtccgatcttggcctgaacccgaactctgcgggtagcgacatccgtgttccgctgccgccgctgacggaagaacgtcgtaaagatctgaccaaaatcgttcgtggtgaagcagaacaagcgcgtgttgcagtacgtaacgtgcgtcgtgacgcgaacgacaaagtgaaagcactgttgaaagataaagagatcagcgaagacgacgatcgccgttctcaggacgatgtacagaaactgactgatgctgcaatcaagaaaattgaagcggcgctggcagacaaagaagcagaactgatgcagttctgatttcttgaacgacaaaaacgccgctcagtagatccttgcggatcggctggcggcgttttgctttttattctgtctcaactctggatgtttcatgaagcaactcaccattctgggctcgaccggctcgattggttgcagcacgctggacgtggtgcgccataatcccgaacacttccgcgtagttgcgctggtggcaggcaaaaatgtcactcgcatggtagaacagtgcctggaattctctccccgctatgccgtaatggacgatgaagcgagtgcgaaacttcttaaaacgatgctacagcaacagggtagccgcaccgaagtcttaagtgggcaacaagccgcttgcgatatggcagcgcttgaggatgttgatcaggtgatggcagccattgttggcgctgctgggctgttacctacgcttgctgcgatccgcgcgggtaaaaccattttgctggccaataaagaatcactggttacctgcggacgtctgtttatggacgccgtaaagcagagcaaagcgcaattgttaccggtcgatagcgaacataacgccatttttcagagtttaccgcaacctatccagcataatctgggatacgctgaccttgagcaaaatggcgtggtgtccattttacttaccgggtctggtggccctttccgtgagacgccattgcgcgatttggcaacaatgacgccggatcaagcctgccgtcatccgaactggtcgatggggcgtaaaatttctgtcgattcggctaccatgatgaacaaaggtctggaatacattgaagcgcgttggctgtttaacgccagcgccagccagatggaagtgctgattcacccgcagtcagtgattcactcaatggtgcgctatcaggacggcagtgttctggcgcagctgggggaaccggatatgcgtacgccaattgcccacaccatggcatggccgaatcgcgtgaactctggcgtgaagccgctcgatttttgcaaactaagtgcgttgacatttgccgcaccggattatgatcgttatccatgcctgaaactggcgatggaggcgttcgaacaaggccaggcagcgacgacagcattgaatgccgcaaacgaaatcaccgttgctgcttttcttgcgcaacaaatccgctttacggatatcgctgcgttgaatttatccgtactggaaaaaatggatatgcgcgaaccacaatgtgtggacgatgtgttatctgttgatgcgaacgcgcgtgaagtcgccagaaaagaggtgatgcgtctcgcaagctgaggataatccggctacagagagtcgcgctatttgttagcgtagggcttcagtgatatagtctgcgccatctgatcgtaagtagttggctttataaggtcagatatgccgtggttttacacggcttttttttgtataggcttcagtattcctgagtaccgtaaaccctgtcagggaataaaaaacgcgtgatgttgtctgctactcaaccacttagcgaaaaattgccagcgcatggctgccgtcatgttgcgatcattatggacggcaatggccgctgggcaaaaaagcaagggaagattcgtgcctttgggcataaagccggggcaaaatccgtccgccgggctgtctcttttgcggccaacaacggtattgaggcgttaacgctgtatgcctttagtagtgaaaactggaaccgaccagcgcaggaagtcagtgcgttaatggaactgtttgtgtgggcgctcgatagcgaagtaaaaagtctgcaccgacataacgtgcgtctgcgtattattggcgataccagtcgctttaactcgcgtttgcaagaacgtattcgtaaatctgaagcgctaacagccgggaataccggtctgacgctgaatattgcggcgaactacggtggacgttgggatatagtccagggagtcaggcaactggctgaaaaggtgcagcaaggaaacctgcaaccagatcagatagatgaagagatgctaaaccagcatgtctgtatgcatgaactggcccctgtagatttagtaattaggactgggggggagcatcgcattagtaactttttgctttggcaaattgcctatgccgaactttactttacagatgttctctggcccgatttcgatgaacaagactttgaaggggcgttaaatgcctttgctaatcgagagcgtcgtttcggcggcaccgagcccggtgatgaaacagcctgatgggggtcgcttttgctgaagtatcgcctgatatctgcttttgtgttaatacccgtcgtcatcgcggcgttgtttctgttgccgccggtggggttcgccattgtaacgctggtggtctgcatgctggcagcgtgggaatggggacagcttagcggttttaccactcgttcgcagcgagtatggttggcggtgttatgcgggttattgttggcgctgatgctttttctgttgccggaatatcaccgaaatattcatcaaccgctggttgaaatctcactttgggcttcgctgggttggtggattgtcgcgctattgctggtgctgttttacccaggttccgcagcaatctggcgtaactctaaaacattgcgccttatttttggcgtgctaaccattgttcccttcttctggggcatgctggcgttacgggcctggcactatgacgagaatcattacagtggcgcaatatggctgctctatgtcatgatcctggtatggggcgctgactccggcgcatatatgtttggcaaattgtttggtaaacataagctggcaccgaaggtttctccgggtaaaacctggcaaggctttatcggtggactcgctactgcagcggtaatctcatggggttatggcatgtgggcgaatctcgacgtcgctcccgtcaccttactcatttgctctattgtcgcagcgttagcctcagtgctcggcgatctgaccgagagtatgtttaagcgtgaagcaggaattaaggacagcggtcatttaattccaggacacggtggtattttagatcgtattgatagcctgacggctgcggtaccggtctttgcttgcttgttgttactggtattcaggacgctttaacggaaggtaatatgctgagttttctctgggatttggcttcgttcatcgttgcactgggtgtacttatcaccgtgcatgaatttggtcatttctgggttgcccggcgttgtggtgttcgcgttgagcgtttctcaatagggtttggtaaggcgctctggcggcgaactgataagctcggcaccgaatatgttatcgccctgatcccgttgggcggttatgtcaaaatgctggatgagcgcgcagaaccggtcgttccggaactccgccaccatgccttcaataataaatctgtcggccaacgagcggcgattattgccgcaggtccggttgcaaacttcatttttgctatctttgcctactggctggtttttattattggtgtgcctggcgtacgtccggtggttggcgaaatagcagccaattcgatagctgcggaagcacaaattgcaccaggtacggaactaaaagccgtagatggtatcgaaacgcctgattgggatgccgtgcgtttgcagttggtcgataaaattggcgatgaaagcaccaccattacagtagcgccatttggcagcgaccaacggcgggatgtaaagctcgatttacgtcactgggcgtttgagcctgataaagaagatccggtatcttcgctggggattcgtcctcgtgggccgcaaattgaacctgtactggaaaatgtgcagccaaactcggcggcaagcaaggcaggtttgcaagcaggcgacaggatcgttaaagtcgatggtcagcccttaacgcagtgggtgacctttgtgatgcttgtccgggataacccgggtaaatccttagcgttagaaatcgaaaggcaggggagtcccttgtctttgacattaatcccggagagtaaaccgggtaatggtaaagcgattggttttgtcggtattgagccgaaagtcattcctttgccagatgagtataaagttgtacgccagtatgggccgttcaacgccatcgtcgaagccacggacaaaacgtggcagctgatgaagctgacggtcagtatgctgggaaaattgatcaccggtgatgtgaaactgaacaacctcagtgggccgatctctatcgccaagggggctgggatgacagcggaactcggggttgtttattacctgccgtttcttgcgcttattagcgtgaacttagggataattaacctgtttccgttgcccgtacttgacggggggcatctgctgttccttgcgatcgaaaagatcaagggcggaccggtatccgagcgggttcaagacttttgttatcgcattggctcgattctgctggtgctgttaatggggcttgcacttttcaatgatttctctcggttatgagagttagttaggaagaacgcataataacgatggcgatgaaaaagttgctcatagcgtcgctgctgtttagcagcgccaccgtatacggtgctgaagggttcgtagtgaaagatattcatttcgaaggccttcagcgtgtcgccgttggtgcggccctcctcagtatgccggtgcgcacaggcgacacggttaatgatgaagatatcagtaataccattcgcgctctgtttgctaccggcaactttgaggatgttcgcgtccttcgtgatggtgatacccttctggttcaggtaaaagaacgtccgaccattgccagcattactttctccggtaacaaatcggtgaaagatgacatgctgaagcaaaacctcgaggcttctggtgtgcgtgtgggcgaatccctcgatcgcaccaccattgccgatatcgagaaaggtctggaagacttctactacagcgtcggtaaatatagcgccagcgtaaaagctgtcgtgaccccgctgccgcgcaaccgtgttgacctaaaactggtgttccaggaaggtgtgtcagctgaaatccagcaaattaacattgttggtaaccatgctttcaccaccgacgaactgatctctcatttccaactgcgtgacgaagtgccgtggtggaacgtggtaggcgatcgtaaataccagaaacagaaactggcgggcgaccttgaaaccctgcgcagctactatctggatcgcggttatgcccgtttcaacatcgactctacccaggtcagtctgacgccagataaaaaaggtatttacgtcacggtgaacatcaccgaaggcgatcagtacaagctttctggcgttgaagtgagcggcaaccttgccgggcactccgctgaaattgagcagctgactaagatcgagccgggtgagctgtataacggcaccaaagtgaccaagatggaagatgacatcaaaaagcttctcggtcgctatggttatgcctatccgcgcgtacagtcgatgcccgaaattaacgatgccgacaaaaccgttaaattacgtgtgaacgttgatgcgggtaaccgtttctacgtgcgtaagatccgttttgaaggtaacgatacctcgaaagatgccgtcctgcgtcgcgaaatgcgtcagatggaaggtgcatggctggggagcgatctggtcgatcagggtaaggagcgtctgaatcgtctgggcttctttgaaactgtcgataccgatacccaacgtgttccgggtagcccggaccaggttgatgtcgtctacaaggtaaaagagcgcaacaccggtagcttcaactttggtattggttacggtactgaaagtggcgtgagcttccaggctggtgtgcagcaggataactggttaggtacaggttatgctgttggtatcaacgggaccaaaaacgattaccagacctatgctgaactgtcggtaaccaacccgtacttcaccgtagatggcgtaagcctcggtggtcgtctcttctataatgacttccaggcagatgacgccgacctgtccgactataccaacaagagttatggtacagacgtgacgttgggcttcccgattaacgaatataactcgctgcgtgcaggtctgggttatgtacataactccctgtccaacatgcagcctcaggttgcgatgtggcgttatctgtactctatgggtgaacatccgagcacctctgatcaggataacagcttcaaaacggacgacttcacgttcaactatggttggacctataacaagcttgaccgtggttacttcccgacagatggttcacgtgtcaacctgaccggtaaagtgaccattcctggatcggataacgaatactacaaagtgacgttagacacggcgacttatgtgccgatcgatgacgatcacaaatgggttgttctggggcgtacccgctggggttatggtgatggtttaggcggcaaagagatgccgttctacgagaacttctatgccggtggttccagcaccgtgcgtggcttccagtccaataccattggtccgaaagcagtttacttcccgcatcaggccagtaattatgatccggactatgattacgaatgtgcgactcaggacggcgcgaaagacctgtgtaaatcggatgatgctgtaggcggtaacgccatggcggttgccagcctcgagttcatcaccccgacgccgtttattagcgataagtatgctaactcggttcgtacttccttcttctgggatatgggtaccgtttgggatacaaactgggattccagccaatattctggatatccggactatagtgatccaagcaatatccgtatgtctgcgggtatcgcattacaatggatgtccccattggggccgttggtgttctcctacgcccagccgttcaaaaagtacgatggagacaaggcagaacagttccagtttaacatcggtaaaacctggtaagtgttctccacaaaggaatgtagtggtagtgtagcgatgactttaggcgatcaatataagatcgccgggccacgcaaagaactgcaccctccggtgcaaatgggatggtaaggagtttattgtgaaaaagtggttattagctgcaggtctcggtttagcactggcaacttctgctcaggcggctgacaaaattgcaatcgtcaacatgggcagcctgttccagcaggtagcgcagaaaaccggtgtttctaacacgctggaaaatgagttcaaaggccgtgccagcgaactgcagcgtatggaaaccgatctgcaggctaaaatgaaaaagctgcagtccatgaaagcgggcagcgatcgcactaagctggaaaaagacgtgatggctcagcgccagacttttgctcagaaagcgcaggcttttgagcaggatcgcgcacgtcgttccaacgaagaacgcggcaaactggttactcgtatccagactgctgtgaaatccgttgccaacagccaggatatcgatctggttgttgatgcaaacgccgttgcttacaacagcagcgatgtaaaagacatcactgccgacgtactgaaacaggttaaataagtaatgccttcaattcgactggctgatttagcgcagcagttggatgcagaactacacggtgatggcgatatcgtcatcaccggcgttgcgtccatgcaatctgcacaaacaggtcacattacgttcatggttaacccaaaataccgtgagcatttaggcttgtgccaggcgtccgcggttgtcatgacccaggacgatcttcctttcgcgaaaagtgccgcactggtagtgaagaatccctacctgacttacgcgcgcatggcgcaaattttagataccacgccgcagcccgcgcagaacattgcacccagtgcggtgatcgacgcgacggcgaagctgggtaacaacgtatcgattggcgctaacgcggtgattgagtccggcgttgaactgggcgataacgtgattatcggtgccggttgcttcgtaggtaaaaacagcaaaatcggtgcaggttcgcgtctctgggcgaacgtaaccatttaccatgagatccagatcggtcagaattgcctgatccagtccggaacagtggtaggcgcagacggctttggttatgccaacgatcgtggtaactgggtgaagatcccacagattggtcgcgtaattattggcgatcgcgtggagatcggtgcctgcacaaccatcgatcgcggcgcgctggatgacactattattggcaatggcgtgatcattgataaccagtgccagattgcacataacgtcgtgattggcgacaatacggcggttgccggtggcgtcattatggcgggcagcctgaaaattggtcgttactgcatgatcggcggagccagcgtaatcaacgggcatatggaaatatgcgacaaagtgacggttacgggcatgggtatggtgatgcgtcccatcactgaaccaggcgtctattcctcaggcattccgctgcaacccaacaaagtctggcgcaaaaccgctgcactggtgatgaacattgatgacatgagcaagcgtctgaaatcgcttgagcgcaaggttaatcaacaagactaacgttccatcttttgttcgccaaactttacggcctgtctcattcttacgattgcggcaggccgtgttattattgtcgtttcttatattttgacaggaagagtatcttgactactaacactcatactctgcagattgaagagattttagaacttctgccgcaccgtttcccgttcttactggtggatcgcgtgctggattttgaagaaggtcgttttctgcgcgcagtaaaaaatgtctctgtcaatgagccattcttccagggccatttccctggaaaaccgattttcccgggtgtgctgattctggaagcaatggcacaggcaacaggtattctggcgtttaaaagcgtaggaaaactggaaccgggtgagctgtactacttcgctggtattgacgaagcgcgcttcaagcgcccggtcgtgcctggcgatcaaatgatcatggaagtcactttcgaaaaaacgcgccgcggcctgacccgttttaaaggggttgctctggtcgatggtaaagtagtttgcgaagcaacgatgatgtgtgctcgtagccgggaggcctgatacgtgattgataaatccgcctttgtgcatccaaccgccattgtggaagagggcgcgtcaattggcgcgaacgcacacattggtcctttttgtatcgttggaccccatgtcgaaattggtgagggtaccgtactgaaatctcacgttgtcgtgaatggtcatactaaaattggccgcgataatgagatttatcagttcgcctccatcggcgaagttaaccaggatctgaaatatgctggcgaaccgacccgtgtggaaatcggcgatcgtaaccgcattcgcgaaagcgtcaccattcatcgtggcacagtccagggcggtggattgacgaaggtgggcagcgacaacttactgatgatcaacgcgcacattgcgcacgattgtacggtaggtaaccgctgtattctcgccaacaacgcaacgctggcgggtcacgtatcggttgacgacttcgcgatcatcggcggcatgaccgcagtccatcagttctgcatcattggtgcgcacgtgatggttggcggctgctccggtgtggcgcaggacgtccctccttatgtcattgcgcagggtaaccacgcaacgccgttcggtgtcaatatcgaagggctgaagcgccgcggattcagccgtgaggcgattaccgctatccgcaatgcgtataagctgatttatcgtagcggtaaaacgctcgatgaagtgaaaccggaaattgctgaactggcggaaacatatccggaagtgaaagcctttaccgatttctttgcacgctcaacgcgcggtctgattcgttaatgactgaacagcgtccattaacgattgccctggtcgccggagaaacctccggcgatatcctgggggccggtttaatccgcgctctgaaagaacatgtgcccaacgcccgctttgttggtgttgccgggccacgaatgcaggctgaaggctgcgaagcctggtacgaaatggaagaactggcggtgatgggcattgttgaagtgctcggtcgtctgcgtcgcttactgcatattcgtgccgatctgacaaagcgttttggcgaactgaagccagatgtttttgttggtattgatgcgcctgacttcaatattactcttgaaggtaacctcaaaaagcagggtatcaaaaccattcattacgtcagtccgtcagtctgggcgtggcgacagaaacgtgttttcaaaataggcagagccaccgatctggtgctcgcatttctgcctttcgaaaaagcgttttatgacaaatacaacgtaccgtgccgctttatcggtcataccatggctgatgccatgccattagatccagataaaaatgccgcccgtgatgtgctggggatccctcacgatgcccactgcctggcgttgctaccggggagccgtggtgcagaagttgaaatgcttagtgccgatttcctgaaaacggcccagcttttgcgccagacatatccggatctcgaaatcgtggtgccactggtgaatgccaaacgccgcgagcagtttgaacgcatcaaagctgaagtcgcgccagacctttcagttcatttgctggatgggatgggccgtgaggcgatggtcgccagcgatgcggcgctactggcgtcgggtacggcagccctggagtgtatgctggcgaaatgcccgatggtggtgggatatcgcatgaagccttttaccttctggttggcgaagcggctggtgaaaactgattatgtctcgctgccaaatctgctggcgggcagagagttagtcaaagaattattgcaggaagagtgtgagccgcaaaaactggctgcggcgctgttaccgctgttggcgaacgggaaaaccagccacgcgatgcacgataccttccgtgaactgcatcagcagatccgctgcaatgccgatgagcaggcggcacaagccgttctggagttagcacaatgatcgaatttgtttatccgcacacgcagctggttgcgggtgtggatgaagtcggacgcgggccgttagttggcgcggtcgtcaccgctgcggtgatccttgacccggcgcgcccgattgccgggctgaatgattccaaaaagctgagcgaaaaacgccgtctggcgctctatgaagagatcaaagagaaagcgttgagctggagtctgggccgcgcggaaccccacgaaatcgacgagctgaacattcttcatgcgaccatgctggcgatgcagcgtgccgtcgctgggctgcatattgcgccggaatatgtgttgattgatggtaaccgctgcccgaaattaccgatgcctgcgatggctgtggtgaaaggcgatagccgcgtaccggaaatcagtgccgcgtctatcctggcgaaagtgacgcgtgacgccgaaatggcggcgctggatattgttttcccgcaatatggttttgcccaacacaaagggtacccaaccgcttttcatctggaaaaactggctgaacacggcgcgaccgaacaccatcggcgcagctttgggcctgtcaaacgcgcactgggacttgcgtcctgattcttgtgtcgagattaagtaaaccggaatctgaagatgtctgaaccacgtttcgtacacctgcgggtgcacagcgactactcgatgatcgatggcctggccaaaaccgcaccgttggtaaaaaaggcggcggcgttgggtatgccagcactggcgatcaccgatttcaccaacctttgtggtctggtgaagttctacggagcgggacatggcgcagggattaagcctatcgtcggggcagattttaacgtccagtgcgacctgctgggtgatgagttaacccacctgacggtactggcggcgaacaataccggctatcagaatctgacgttgctgatctcaaaagcgtatcagcgcgggtacggtgccgccgggccgatcatcgatcgcgactggcttatcgaattaaacgaagggttgatccttctttccggcggacgcatgggcgacgtcggacgcagtcttttgcgtggtaacagcgcgctggtagatgagtgtgtcgcgttttatgaagaacacttcccggatcgctattttctcgagctgatccgcaccggcaggccggatgaagaaagctatctgcacgcggcggtggaactggcggaagcgcgcggtttgcccgtcgtggcgaccaacgacgtgcgctttatcgacagcagcgactttgacgcacacgaaatccgcgtcgcgatccacgacggctttaccctcgacgatcctaaacgcccgcgtaactattcgccgcagcaatatatgcgtagcgaagaggagatgtgtgagctgtttgccgacatccccgaagcccttgccaacaccgttgagatcgccaaacgctgtaacgtaaccgtgcgtcttggtgaatacttcctgccgcagttcccgaccggggacatgagcaccgaagattatctggtcaagcgtgcaaaagagggcctggaagagcgtctggcctttttattccctgatgaggaagaacgtcttaagcgccgcccggaatatgacgaacgtctggagactgaacttcaggttatcaaccagatgggcttcccgggctacttcctcatcgttatggaatttatccagtggtcgaaagataacggcgtaccggtagggccaggccgtggctccggtgcgggttcactggtggcctacgcgctgaaaatcaccgacctcgatccgctggaatttgacctgctgttcgaacgtttccttaacccggaacgtgtctccatgcctgacttcgacgttgacttctgtatggagaaacgcgatcaggttatcgagcacgtagcggacatgtacggtcgtgatgcggtatcgcagatcatcaccttcggtacaatggcggcgaaagcggtgatccgcgacgtaggccgcgtgctggggcatccgtacggctttgtcgatcgtatctcgaaactgatcccgcccgatccggggatgacgctggcgaaagcgtttgaagccgagccgcagctgccggaaatctacgaagcggatgaagaagttaaggcgctgatcgacatggcgcgcaaactggaaggggtcacccgtaacgccggtaagcacgccggtggggtggttatcgcgccgaccaaaattaccgattttgcgccgctttactgcgatgaagagggcaaacatccggtcacccagtttgataaaagcgacgttgaatacgccggactggtgaagttcgacttccttggtttgcgtacgctcaccatcatcaactgggcgctggagatgatcaacaagcggcgggcgaagaatggcgagccgccgctggatatcgctgcgatcccgctggatgataagaaaagcttcgacatgctgcaacgctcggaaaccacggcggtattccagcttgaatcgcgcggcatgaaggacctgatcaagcgtctacaacctgactgcttcgaagatatgatcgccctagtggcactgttccgccccggtccgttgcaatcagggatggtggataactttatcgaccgtaaacatggtcgtgaagagatctcctatccggacgtacagtggcagcatgaaagcctgaaaccggtactggagccaacctacggcattatcctgtatcaggaacaggtcatgcagattgcgcaggtgctttctggttataccctcggtggcgcggatatgctgcgtcgtgcgatgggtaagaaaaagccggaagagatggctaagcaacgttctgtatttgctgaaggtgcagaaaagaacggaatcaacgctgaactggcgatgaaaatcttcgacctggtggagaaattcgctggttacggatttaacaaatcgcactctgcggcctatgctttggtgtcatatcaaacgttatggctgaaagcgcactatcctgcggagtttatggcggcggtaatgaccgccgatatggacaacaccgagaaggtggtgggtctggtggatgagtgctggcggatggggctgaaaatcctgccaccagatataaactccggtctttaccatttccacgtcaacgacgacggcgaaatcgtgtatggtattggcgcgatcaaaggggtcggtgaaggtccgattgaggccatcatcgaagcccgtaataaaggcggctacttccgcgaactgtttgatctctgcgcccgtaccgacaccaaaaagttgaaccgtcgcgtgctggaaaaactgatcatgtccggggcgtttgaccgtcttgggccacatcgcgcagcgctgatgaactcgctgggcgatgcgttaaaagcggcagatcaacacgcgaaagcggaagctatcggtcaggccgatatgttcggcgtgctggccgaagagccggaacaaattgaacaatcctacgccagctgccaaccgtggccggagcaggtggtattagatggggaacgtgaaacgttaggcctgtacctgaccggacaccctatcaaccagtatttaaaagagattgagcgttatgtcggaggcgtaaggctgaaagacatgcacccgacagaacgtggtaaagtcatcacggctgcggggctcgttgttgccgcgcgggttatggtcaccaagcgcggcaatcgtatcggtatctgcacgctggatgaccgttccgggcggctggaagtgatgttgtttactgacgccctggataaataccagcaattgctggaaaaagaccgcatacttatcgtcagcggacaggtcagctttgatgacttcagcggtgggcttaaaatgaccgctcgcgaagtgatggatattgacgaagcccgggaaaaatatgctcgcgggcttgctatctcgctgacggacaggcaaattgatgaccagcttttaaaccgactccgtcagtctctggaaccccaccgctctgggacaattccagtacatctctactatcagagggcggatgcacgcgcgcggttgcgttttggcgcgacgtggcgtgtctctccgagcgatcgtttattaaacgatctccgtggcctcattggttcggagcaggtggaactggagtttgactaatacaggaatactatgagtctgaatttccttgattttgaacagccgattgcagagctggaagcgaaaatcgattctctgactgcggttagccgtcaggatgagaaactggatattaacatcgatgaagaagtgcatcgtctgcgtgaaaaaagcgtagaactgacacgtaaaatcttcgccgatctcggtgcatggcagattgcgcaactggcacgccatccacagcgtccttataccctggattacgttcgcctggcatttgatgaatttgacgaactggctggcgaccgcgcgtatgcagacgataaagctatcgtcggtggtatcgcccgtctcgatggtcgtccggtgatgatcattggtcatcaaaaaggtcgtgaaaccaaagaaaaaattcgccgtaactttggtatgccagcgccagaaggttaccgcaaagcactgcgtctgatgcaaatggctgaacgctttaagatgcctatcatcacctttatcgacaccccgggggcttatcctggcgtgggcgcagaagagcgtggtcagtctgaagccattgcacgcaacctgcgtgaaatgtctcgcctcggcgtaccggtagtttgtacggttatcggtgaaggtggttctggcggtgcgctggcgattggcgtgggcgataaagtgaatatgctgcaatacagcacctattccgttatctcgccggaaggttgtgcgtccattctgtggaagagcgccgacaaagcgccgctggcggctgaagcgatgggtatcattgctccgcgtctgaaagaactgaaactgatcgactccatcatcccggaaccactgggtggtgctcaccgtaacccggaagcgatggcggcatcgttgaaagcgcaactgctggcggatctggccgatctcgacgtgttaagcactgaagatttaaaaaatcgtcgttatcagcgcctgatgagctacggttacgcgtaattcgcaaaagttctgaaaaagggtcacttcggtggcccttttttatcgccacggtttgagcaggctatgattaaggaaggattttccaggaggaacacatgaacatcattgccattatgggaccgcatggcgtcttttataaagatgagcccatcaaagaactggagtcggcgctggtggcgcaaggctttcagattatctggccacaaaacagcgttgatttgctgaaatttatcgagcataaccctcgaatttgcggcgtgatttttgactgggatgagtacagtctcgatttatgtagcgatatcaatcagcttaatgaatatctcccgctttatgccttcatcaacacccactcgacgatggatgtcagcgtgcaggatatgcggatggcgctctggttttttgaatatgcgctggggcaggcggaagatatcgccattcgtatgcgtcagtacaccgacgaatatcttgataacattacaccgccgttcacgaaagccttgtttacctacgtcaaagagcggaagtacaccttttgtacgccggggcatatgggcggcaccgcatatcaaaaaagcccggttggctgtctgttttatgattttttcggcgggaatactcttaaggctgatgtctctatttcggtcaccgagcttggttcgttgctcgaccacaccgggccacacctggaagcggaagagtacatcgcgcggacttttggcgcggaacagagttatatcgttaccaacggaacatcgacgtcgaacaaaattgtgggtatgtacgccgcgccatccggcagtacgctgttgatcgaccgcaattgtcataaatcgctggcgcatctgttgatgatgaacgatgtagtgccagtctggctgaaaccgacgcgtaatgcgttggggattcttggtgggatcccgcgccgtgaatttactcgcgacagcatcgaagagaaagtcgctgctaccacgcaagcacaatggccggttcatgcggtgatcaccaactccacctatgatggcttgctctacaacaccgactggatcaaacagacgctggatgtcccgtcgattcacttcgattctgcctgggtgccgtacacccattttcatccgatctaccagggtaaaagtggtatgagcggcgagcgtgttgcgggaaaagtgatcttcgaaacgcaatcgacccacaaaatgctggcggcgttatcgcaggcttcgctgatccacattaaaggcgagtatgacgaagaggcctttaacgaagcctttatgatgcataccaccacctcgcccagttatcccattgttgcttcggttgagacggcggcggcgatgctgcgtggtaatccgggcaaacggctgattaaccgttcagtagaacgagctctgcattttcgcaaagaggtccagcggctgcgggaagagtctgacggttggtttttcgatatctggcaaccgccgcaggtggatgaagccgaatgctggcccgttgcgcctggcgaacagtggcacggctttaacgatgcggatgccgatcatatgtttctcgatccggttaaagtcactattttgacaccggggatggacgagcagggcaatatgagcgaggaggggatcccggcggcgctggtagcaaaattcctcgacgaacgtgggatcgtagtagagaaaaccggcccttataacctgctgtttctctttagtattggcatcgataaaaccaaagcaatgggattattgcgtgggttgacggaattcaaacgctcttacgatctcaacctgcggatcaaaaatatgctacccgatctctatgcagaagatcccgatttctaccgcaatatgcgtattcaggatctggcacaagggatccataagctgattcgtaaacacgatcttcccggtttgatgttgcgggcattcgatactttgccggagatgatcatgacgccacatcaggcatggcaacgacaaattaaaggcgaagtagaaaccattgcgctggaacaactggtcggtagagtatcggcaaatatgatcctgccttatccaccgggcgtaccgctgttgatgcctggagaaatgctgaccaaagagagccgcacagtactcgattttctactgatgctttgttccgtcgggcaacattaccccggttttgaaacggatattcacggcgcgaaacaggacgaagacggcgtttaccgcgtacgagtcctaaaaatggcgggataacttgccagagcggcttccgggcgagtaacgtgctgttaacaaataaaggagacgttatgctgggtttaaaacaggttcaccatattgcgattattgcgacggattatgcggtgagcaaagctttctactgcgatattcttggtttcacgctgcaaagcgaagtctatcgcgaagcgcgcgactcatggaaaggggatttggcgcttaatgggcaatatgtgattgagcttttctcatttccgttcccgccggaacgacccagccgaccggaagcttgcggtctgcgtcatctggcttttagcgttgatgacatcgatgcggcagtggcgcaccttgaaagccataacgtgaagtgtgaaaccatccgtgtcgatccatacacgcaaaaacgcttcaccttctttaacgatccggacgggctgccgttggaactgtatgagcagtaaggcttgtcatcgccgcatttgcccggtaacgtgccgggcattgctactgtaaaatcgcaccatcatgacactcacgctcaatagacaacttctcacctcacgccagattctggtggcctttagcggcgggcttgactccaccgttctgctgcatcagttggtgcagtggcggacggaaaatccgggtgtcgctctgcgcgctattcatgtgcatcacggtttaagtgccaatgccgatgcctgggttacgcattgcgaaaacgtctgccaacagtggcaggtgccgctggtggtcgaacgcgtacaacttgcgcaagaaggactgggcattgaggcccaggcgcggcaggcacgttatcaggcatttgcccgcaccttgttgcccggtgaagtgctggtcaccgcgcaacatctcgacgatcaatgtgaaacctttctgctggcgctaaaacgcggcagtggccctgccgggctttcggctatggcggaagtctcggagtttgccggaacgcggcttattcgcccgttgctcgcccgcacgcggggggaactggtgcagtgggcgcgtcagtatgatttacgctggattgaagacgaaagtaatcaggacgactcatacgatcgtaactttctgcgcctgcgcgtagtgccgttattgcagcagcgttggccgcattttgccgaagcaacggcccgcagcgccgcactttgtgctgaacaagagagcctgctggatgaactgctggcagatgatttagcacactgtcaatcgccgcaggggacgctgcagattgtgccaatgctggcgatgagtgatgcccgccgcgcggcgattatccgccgctggctggcagggcagaatgcaccgatgccttcccgcgacgcgttggtgaggatctggcaggaagtggcgctggcgcgggaagatgcctcaccctgtttacgtttgggcgcgtttgaaatccgacgctatcagtcgcaactgtggtggattaaatccgtcaccgggcaaagcgaaaacattgtgccgtggcagacgtggcttcaaccgctggaattaccggcggggctgggaagtgtacagcttaatgcgggaggcgatattcgccctccgcgtgcagacgaagcggtcagcgtgcgtttcaaagcgccaggattgctgcatattgtcgggcgtaacggcggacgtaagctaaagaaaatctggcaagagctgggcgtgccgccgtggctacgtgacaccacgccactgctgttttatggcgaaacgctgattgcggcggcaggggtatttgtgacgcaagaaggtgtggctgaaggtgagaatggcgtaagttttgtctggcagaaaacgcttagttaagtgaaagccggataagacgcatcaaacgtcgcatccggcgaaagtcaatcaggattcgcttaccaccaccgtaccgatttccgggtggctaaagctggtaattttatccagacgcagctcgcgggtttcgccagcggcctcgacgaccaggtactccacatttttgcgggagactaaatcactggcttttgcctgcaatttttcgccatctttcagctcaagtgtcagcattaaatgatgctggcaggcgagctcaagattatcgtaatcatcacaattgattggttgatacgtatcattcattgacataatcgctcaccagtaagtttgccgcagcgtatgctgctttttccctgacagcctcagaaagggcgtcgtcggcagccatttcattcagcactttcaaaacgcagcccagcgcgtccggaacgtatcctaagtctccgctggcgatttccgcgtaccgcttgcgtattaactcacaatatttttccacatgccctcctgtcagcactctgacttaaccgtggatgcaagtctaagcctacgaagataaactctgtttcgcaaggtgactataccacactcatttctgcaatatcagcgccgcaactgcacgtattccgttacaatggcctcctgattcgaaaggagttttcttatggcgcttaaagcgacaatttataaagcgacggttaatgtggccgatctcgaccgcaaccagtttctcgatgcctctctgacgctggcgcgccatccttcagaaacccaggagcgtatgatgctgcgcttgctggcgtggctgaaatatgctgatgaacgtctgcaatttacccgtggtttgtgtgccgatgatgagccggaagcgtggctgcgtaacgatcacctgggcattgatttgtggattgagctggggctgccggatgagcggcggattaagaaagcctgcacccaggccgcagaagtggcgctgtttacctataatagtcgggcggcgcaaatctggtggcagcaaaatcagagcaaatgtgtgcagtttgccaatctttccgtctggtatctggacgatgaacaactggcgaaagtaagcgcctttgccgatcgtaccatgacgctgcaggcaacgattcaggatggcgtgatctggttatcggatgataagaataatctggaagtgaacttaaccgcctggcaacaaccttcatgattgtgatttcccgacatgttgctattcccgatggtgagcttgagatcaccgccattcgtgcgcagggcgcgggcgggcagcatgttaataagacctcaacggctattcatctgcgttttgacattcgggcgtccagcctgccagagtattacaaagagcgtctgctcgccgccagccatcatttgatcagcagtgatggcgtgattgtcattaaggcacaggaataccgcagtcaggaactgaaccgcgaagcagctctggcccggctggtggctatgattaaagaattaacaacagaaaaaaaagcccgacgacccacgcggcccacccgtgcatcgaaagagcgcaggctggcatcgaaagcacaaaaatcaagcgtgaaggcgatgcgcggcaaagtgcgcagcggtcgggaataaaaagaaggaatggatggtgaaaaaagcgatagtgacagcgatggctgtaatcagcctctttactctgatgggatgtaataatcgggccgaagtcgatacgctttctccggcgcaggctgccgaactgaaaccgatgccgcaaagttggcgcggcgtgctgccgtgtgccgattgcgaaggaatcgaaacctctctgttcctcgaaaaagacggaacatgggtgatgaatgagcgttatctcggtgctcgtgaagaaccttcctccttcgcttcctacggtacatgggcgcgaaccgctgacaagctggtattaaccgacagcaaaggtgaaaagtcatattatcgggcgaaaggcgatgcgctggagatgctcgatcgtgaaggcaatccgattgaatcgcagttcaactatacgctggaagcggcacaatccagtttacctatgacgccgatgaccctgcggggcatgtatttttatatggctgatgcggcgaccttcactgattgcgcgaccggaaaacgtttcatggtagcgaataacgcagagctggagcgtagctacctggctgcgcgcggtcacagtgaaaaaccggtgttactgtcagtagaaggtcactttacgcttgagggtaatccggataccggtgcgccgactaaagtattggcacccgatacggcagggaaattttaccccaaccaggattgcagtagtttggggcagtaacccgtcttgagacagaaacaaacgcaaaacaggccagaaggatatatttcaacattttgaatttgcacgttttttgtaggccggataaggcgtttacgccgcatccggcaatggtgctcaacgcctgatgcgacgctggcgcgtcttatcatgcctacaacccccctcataccttaaggcggataaggcatttactttatcaccgggtcaaaccaacaaagcgacccgccttgatataaatcccaggcttcaggtgcccaacatactgtaactgcgtttctggcttaaacgcagagacatcaccaatacgcatatgcatcagatcggcagggctaatccagcccgattgcgccagtgtaagtggatgcccggctttggcaaaggcatccgtgacaaattccgaacaaaaccacgactttttgtctccttcgcccacactgcttaactgcgctttcgccaggccgctgacgcactgttggcgaaaatcctcggagaacggattcagtgagcacatctggcgagtcaccataaagggaataaattcgacaatgccgcgatagttataaccgctatctttgattttattggcaaacgcggtgatatctgtggcttgttgcggggtaagatccgggactcgtaagacgaaaagcttatcactatgcttcatcgcttttttaagggaaacgatctggacgccagcgcctgtcgcttctgcaacgttattatcacccagaaagattgcaacgtgactcacagaggaagtgctgaagacgcggattccaaatgaggttaccccaaggcttgaggagaacagcaaatcgccgggtttgagatcaggtgccgttatttcttttattgattgttcggtgaaagagctttgatgctggaatttgacagcccatgtttttgcctcggcatctactgctgtggctgatgggtctggctggctgatatcaacggtacaagccgaaagtaaaagaaagctggggagaaacaggcggcagtacgcctttggtttatccattttatacaatccatgtaaaaaaagggccctgaaattcaggaccctttctggcatcagcctttaatctgtttcaccagatattcgacgatgtcaccagtcttaattaactgtttctcgccgttgcgacgatatttatattcgatatcgtcgttgtcgaggttacggtcgcccagcacaatagtgtgcggaataccgatcagttccatatcagcaaacatcacgcccggacgctctttgcggtcatccagcagcacttcgataccttgtgcacgcagttcgctgtacagtttctcagcaagctcttgtacgcggaaggatttgtgcatgttcatcggcagaatcgccacctggaacggcgcgatagcgtcaggccatacgatgcctcgttcgtcgtagttctgctcaatcgccgcagctaccacacgcgttaccccgataccgtagcaacccatcgtcaggatttggttacggccatcttcaccctgtacggaggctttcagtgcttcggagtacttggtacccagctggaagatgtgaccaacttcgataccacgtttgatcagcagcctaccctggccatccgggcttggatcgccagccaccacgttacggatatctgcaacttccggggtagcgacatcgcgatcccagttgatgccgaagtagtgtttaccatcgatgttagcaccagcagcgaaatcactcatcgccgcaacggtacggtcaatcaccaccggaatcggcatgtttaccggacccagtgaacccggaccggctttaaccacggcacgaatttcttcttcggtcgcgaaagtcagcgggcttgcaacctgcggcagtttttctgctttaacttcgttcagctcgtgatcaccgcgcaccagcagcgcaacctgcgggaagctgctgccttcaaccgctttaaccagcagagtcttaaccgttttctcaatcggcagattgaactgttcaaccagttccgcgatggttttcgcgttcggcgtatcaaccagcgtcatttcctgggtagcagcagcgcgcggttctttcggcgcgatagcttctgccagttcaatgttcgctgcatagtcagaggtgtcggagaagaccacatcgtcttcaccgctctgcgccagcacctggaattcgtgagaggcgctgccgccgatagaaccggtgtcggcttgtacggcgcggaaatccagccccatgcggctgaagattttgctgtaggccgcatacattgcatcgtaggtttcctgcagggattcctgagaagtatggaaagagtaagcatctttcatcaggaattcgcgggaacgcatgacgccgaaacgcggacgcacttcgtcgcggaacttggtctggatctgatagaagttcagcggcagctgtttgtaagagctaagctcgttacgaatcaggtcagtgataacttcttcatgagttgggccgagtacgaacggacgctcgccacggtcaacaaaacgcagcagttccggaccgtactgttcccaacgaccactctcttgccacaaatcggctggctgaaccaccggcatcgacacctcgatcgcaccggcgttgttcatctcttcacgcacgatgttttcgacttttttcagaacgcgcacgccggtcggcagccaggtatataacccggaggccagcttgcggatcatcccggcgcgcagcatcagctgatggctgatcacctcggcgtcggcaggtgtctccttgagagtggagagcaggtattggctagtacgcatgttgttacggttccagttggaaggtagaacaggctcaaggcgagcctgggacaaaaaaaagtgatttagtttaccagtgcaaaagaaatgtcaaaagagaagggcgtgaatttaacgcggttccagcgcaaagacttcaaaacctgcgtcggtgacgcgccagcgaacgttaaaatcatgtagccagacggcataggttttgcccgtttcctcacctttacgataggccgggcgcgggtcctgcgccagtacttcgcggataaacagcgttaactgcggataacgcttctccagcgtcaaaagctgcttttcgacctctgcggtaaaactcaccgccatctctgcagctggcgcactttgcgcatagctggcactggcatcgggaagcgattcggcaaaggggagatacggtttgatatccactaccggcgtaccatcgaccagatccagactgccgagcttcagaatcacgctgtctttatggcaaacaacctctttcagctctaccagcgacatgccaattgggttagggcggaaagtagagcgtgttgcgaaaacccccattctggcgttaccgccgaggcgcggtggacgcacagtcggacgccagccgccttccatcgtttgatgaaagacgaaaaggatccataaatggctgaacgcttccaggccgcgaacggcgtcggcctggttgtagggagcaatgagatgcagttcgccgttggcgctttttaccagacctggctggcgcggaacggcgaacttttctttatagggcgagcgaataacgcctatttgctcgaactggaaactgctcatttcgccgtaatgttaagcgcagaaccgatacatacagcctgacgatagcagcctggcgtaccgctggtgacttcgcagctatgcagtaatacagcattggctttcattttagaggcgttgatttgcatccgcttacgtgcggttggaatgctcggcggagagtcctgattagaggcctggcaagagtcgccactgacttcaccgagatcgcggaacggtttgccgactaattcttctgcattggtataaattcggaccggcgtggcgcgcggcgctttcggttttgcaggctccgctttcggctggggtgcagtgctttgaacgggttcgacaggggatctgcttaacatggaacagccgcttagcatgagtgctactaaacagatcggtaaagcacgcatagtatttcctcaatgtatgatcaaaacgtcaatattgaatcaggagcttgtaaaaatgacaagacgggcaagcgcccgtcctgaatgatattacaaattgtggaaacagcctaaaaattaccagcctttaacagctccgccgttaaacactttgtttgctgcttcgtaaacttcgtcagactgataagcctggacgaatttcttcacgttctcggcgtctttgttatcttcacgcgtcacgatcaggtttacgtacggggactctttatcttcaacaaagataccgtctttcgccggagtcaggccaatctggctggcataggtggtattgataactgccagagcgatttgcgcgtcgtccagagaacgcggcagttgcggtgcttccagttcaacaattttcagatttttggggttctcaacaacatcaagaacggtcggcagcaggccaacgccatctttcagtttgatcaagcccactttttgcagcagcagcagtgaacgaccaaggttagttgggtcgtttggcacggcaacctgcgaaccatcctgcagttcatccagtgatttgattttcttggagtaaccagcaatcggataaacaaaagtgttgcctactgcgaccagtttgtagccacgatctttcagttgctgatcaaggtacggtttatgctggaaggcgttggcgtcgatatcgcctttgctcaatgcttcgtttggcagaacatagtcgttgaaggttaccagctcaacgtccaggccatatttgtctttcgcaactttctgcgcgacttctgcaacctgctgttcggcaccaacaatcacgccgactttaatgtggtttggatctttttcatcctgaccgcagcctaccagtgccagtgatccgatcagggctcccactgccgcaaaggttttgaatttgaacgccataccttattccttcttcaattatttatgttgtgttgaacgttacttgcgagtgacagcccggacgatgcggtcgcctgcgaactgaattaaataaaccagaatgaccagcaataccagtaccgtattcatcaccgtcgcgttatagccgatgtagccatactgatagccaatctgacctaaaccaccggcaccgactgcaccacccatcgcggaataaccgaccagggtaatcagggtgatagttgccgcattcaccagacccggcagcgcttccggtaacagcaccttacggacgatctgcatcggcgtggcacccattgcgcgggaagcttcaattaacccggttgggatctccagcagagcgttctcgaccatacgggcaataaacggtgctgcaccaacggttaacggaacaatcgctgcctgcaaaccaatcgatgtaccgacaataacgcgggtaaacggaatcatccatacaagcaagataatgaacgggatggaacggaaaatgttcacaatcgcagaaacggtacgatacagcttcgcgttagcaataatttgccccggacgcgtgacataaagcagaacgccaaccggcagaccaatcacaaagccaaaaaaaccggatacgaaggtcattgccagcgtttcccatacgccacgaaccagcagccacatcatcggctcagacataacccagtacctctacttttacatggtgttcctgcagccaggcaatggcggcttgcgtatcttgttgtgtgccgtgcatttcagtcagcatgatgccgaacttaacgccaccggcgtaatccatctgcgcgctaataatgttgttgttgacgttgaaacgacgcgcggtttcagaaagcagtggggcatcgaccgattgaccggtaaactccagacgcagcatcggcacgcagtcagtaaatggctccgcttgcagacgttcctggtaatcttccgggatatccagatgcagggtcgactgaataaacttctgcgccagcggcgttttcggatgcgagaacacttcacttaccgtgtcctgctcgatcagttctccattgctgatgaccgccacgcaatcacaaatgcgcttcacaacgtccatttcgtgggtgatcaacagaatcgtcaaccccagacggcggttgatgtctttcagcagttcgagaatagaacgtgtcgttgccgggtccagcgcgctggtggcttcatcacacagcaatactttgggattgctggctaacgcacgggcaattgccacacgttgtttctgcccaccggaaagattcgacgggtagctatcatgcttatcgccaagaccaaccaatgacagcaattccgtcacgcgacgtttgacctcgtctttcggtgtgttgtccagctccagcggcagagccacgttgccaaaaacagtacgcgaagagagcaggttaaaatgctggaaaatcataccaatctggcggcgagctttggtcaactcggattctgacagcgtggtcagttcctggccatcgaccagcacgctaccctcggttgggcgctccagcaggtttacacaacgtataagcgtactcttacccgcgcctgaggcaccgataacgccataaatttgtccagctggcacatgcaggctgacgttgttcaacgcctggatggtgcgggtgccctggtggaacactttggtgatattcgaaagttttatcattgattatttattatcgtcattaagttagtcgtggcatctcgaatgcctgaaacgggcaacgccgtcaatgaaatggatgttaaggcatccagacgtctaaatcaatcaggtttatgcgaagagcactttcttgcaggtcgaaacatgcgatactagcgtcacatgccttattaaggagctataaaaggtggcgaagagcgtacccgcaatttttcttgaccgtgatggcaccattaatgtcgatcacggctatgtccatgagatcgacaactttgaatttatcgacggtgttattgacgccatgcgcgagctaaaaaaaatgggctttgcgctggtggtagtaaccaaccagtctggcattgctcgcggtaaatttaccgaagcacagtttgaaacgctgaccgagtggatggactggtcgctggcggaccgagatgtcgatctggatggtatctattattgcccgcatcatccgcagggtagtgttgaagagtttcgccaggtctgcgattgccgcaaaccacatccggggatgcttttgtcagcacgcgattatttgcatattgatatggccgcttcttatatggtgggcgataaattagaagatatgcaggcagcggttgcggcgaacgtgggaacaaaagtgctggtgcgtacgggtaaacctattacgcctgaagcagaaaacgcggcggattgggtgttaaatagcctggcagacctgccgcaagcgataaaaaagcagcaaaaaccggcacaatgattaaaagatgagcggttgaaataaaaatgcatttttccgcttgtcttcctgagccgactccctataatgcgcctccatcgacacggcggatgtgaatcacttcacacaaacagccggttcggttgaagagaaaaatcctgaaattcagggttgactctgaaagaggaaagcgtaatatacgccacctcgcgacagtgagctgaaagccgcgtcgcaactgctctttaacaatttatcagacaatctgtgtgggcactcgaagatacggattcttaacgtcgcaagacgaaaaatgaataccaagtctcaagagtgaacacgtaattcattacaaagtttaattctttgagcatcaaacttttaaattgaagagtttgatcatggctcagattgaacgctggcggcaggcctaacacatgcaagtcgaacggtaacaggaagaagcttgcttctttgctgacgagtggcggacgggtgagtaatgtctgggaaactgcctgatggagggggataactactggaaacggtagctaataccgcataacgtcgcaagaccaaagagggggaccttcgggcctcttgccatcggatgtgcccagatgggattagctagtaggtggggtaacggctcacctaggcgacgatccctagctggtctgagaggatgaccagccacactggaactgagacacggtccagactcctacgggaggcagcagtggggaatattgcacaatgggcgcaagcctgatgcagccatgccgcgtgtatgaagaaggccttcgggttgtaaagtactttcagcggggaggaagggagtaaagttaatacctttgctcattgacgttacccgcagaagaagcaccggctaactccgtgccagcagccgcggtaatacggagggtgcaagcgttaatcggaattactgggcgtaaagcgcacgcaggcggtttgttaagtcagatgtgaaatccccgggctcaacctgggaactgcatctgatactggcaagcttgagtctcgtagaggggggtagaattccaggtgtagcggtgaaatgcgtagagatctggaggaataccggtggcgaaggcggccccctggacgaagactgacgctcaggtgcgaaagcgtggggagcaaacaggattagataccctggtagtccacgccgtaaacgatgtcgacttggaggttgtgcccttgaggcgtggcttccggagctaacgcgttaagtcgaccgcctggggagtacggccgcaaggttaaaactcaaatgaattgacgggggcccgcacaagcggtggagcatgtggtttaattcgatgcaacgcgaagaaccttacctggtcttgacatccacagaactttccagagatggattggtgccttcgggaactgtgagacaggtgctgcatggctgtcgtcagctcgtgttgtgaaatgttgggttaagtcccgcaacgagcgcaacccttatcttttgttgccagcggtccggccgggaactcaaaggagactgccagtgataaactggaggaaggtggggatgacgtcaagtcatcatggcccttacgaccagggctacacacgtgctacaatggcgcatacaaagagaagcgacctcgcgagagcaagcggacctcataaagtgcgtcgtagtccggattggagtctgcaactcgactccatgaagtcggaatcgctagtaatcgtggatcagaatgccacggtgaatacgttcccgggccttgtacacaccgcccgtcacaccatgggagtgggttgcaaaagaagtaggtagcttaaccttcgggagggcgcttaccactttgtgattcatgactggggtgaagtcgtaacaaggtaaccgtaggggaacctgcggttggatcacctccttaccttaaagaagcgtactttgcagtgctcacacagattgtctgatgaaaatgagcagtaaaacctctacaggcttgtagctcaggtggttagagcgcacccctgataagggtgaggtcggtggttcaagtccactcaggcctaccaaatttgcacggcaaatttgaagaggttttaactacatgttatggggctatagctcagctgggagagcgcctgctttgcacgcaggaggtctgcggttcgatcccgcatagctccaccatctctgtagtggttaaataaaaaatacttcagagtgtacctgcaaaggttcactgcgaagttttgctctttaaaaatctggatcaagctgaaaattgaaacactgaacaatgaaagttgttcgtgagtctctcaaattttcgcaacacgatgatggatcgcaagaaacatcttcgggttgtgaggttaagcgactaagcgtacacggtggatgccctggcagtcagaggcgatgaaggacgtgctaatctgcgataagcgtcggtaaggtgatatgaaccgttataaccggcgatttccgaatggggaaacccagtgtgtttcgacacactatcattaactgaatccataggttaatgaggcgaaccgggggaactgaaacatctaagtaccccgaggaaaagaaatcaaccgagattcccccagtagcggcgagcgaacggggaggagcccagagcctgaatcagtgtgtgtgttagtggaagcgtctggaaaggcgcgcgatacagggtgacagccccgtacacaaaaatgcacatgctgtgagctcgatgagtagggcgggacacgtggtatcctgtctgaatatggggggaccatcctccaaggctaaatactcctgactgaccgatagtgaaccagtaccgtgagggaaaggcgaaaagaaccccggcgaggggagtgaaaaagaacctgaaaccgtgtacgtacaagcagtgggagcatgcttaggcgtgtgactgcgtaccttttgtataatgggtcagcgacttatattctgtagcaaggttaaccgaataggggagccgaagggaaaccgagtcttaactgggcgttaagttgcagggtatagacccgaaacccggtgatctagccatgggcaggttgaaggttgggtaacactaactggaggaccgaaccgactaatgttgaaaaattagcggatgacttgtggctgggggtgaaaggccaatcaaaccgggagatagctggttctccccgaaagctatttaggtagcgcctcgtgaactcatctccgggggtagagcactgtttcggcaagggggtcatcccgacttaccaacccgatgcaaactgcgaataccggagaatgttatcacgggagacacacggcgggtgctaacgtccgtcgtgaagagggaaacaacccagaccgccagctaaggtcccaaagtcatggttaagtgggaaacgatgtgggaaggcccagacagccaggatgttggcttagaagcagccatcatttaaagaaagcgtaatagctcactggtcgagtcggcctgcgcggaagatgtaacggggctaaaccatgcaccgaagctgcggcagcgacgcttatgcgttgttgggtaggggagcgttctgtaagcctgtgaaggtgtactgtgaggtatgctggaggtatcagaagtgcgaatgctgacataagtaacgataaagcgggtgaaaagcccgctcgccggaagaccaagggttcctgtccaacgttaatcggggcagggtgagtcgacccctaaggcgaggccgaaaggcgtagtcgatgggaaacaggttaatattcctgtacttggtgttactgcgaaggggggacggagaaggctatgttggccgggcgacggttgtcccggtttaagcgtgtaggctggttttccaggcaaatccggaaaatcaaggctgaggcgtgatgacgaggcactacggtgctgaagcaacaaatgccctgcttccaggaaaagcctctaagcatcaggtaacatcaaatcgtaccccaaaccgacacaggtggtcaggtagagaataccaaggcgcttgagagaactcgggtgaaggaactaggcaaaatggtgccgtaacttcgggagaaggcacgctgatatgtaggtgaagcgacttgctcgtggagctgaaatcagtcgaagataccagctggctgcaactgtttattaaaaacacagcactgtgcaaacacgaaagtggacgtatacggtgtgacgcctgcccggtgccggaaggttaattgatggggttagcgcaagcgaagctcttgatcgaagccccggtaaacggcggccgtaactataacggtcctaaggtagcgaaattccttgtcgggtaagttccgacctgcacgaatggcgtaatgatggccaggctgtctccacccgagactcagtgaaattgaactcgctgtgaagatgcagtgtacccgcggcaagacggaaagaccccgtgaacctttactatagcttgacactgaacattgagccttgatgtgtaggataggtgggaggctttgaagtgtggacgccagtctgcatggagccgaccttgaaataccaccctttaatgtttgatgttctaacgttgacccgtaatccgggttgcggacagtgtctggtgggtagtttgactggggcggtctcctcctaaagagtaacggaggagcacgaaggttggctaatcctggtcggacatcaggaggttagtgcaatggcataagccagcttgactgcgagcgtgacggcgcgagcaggtgcgaaagcaggtcatagtgatccggtggttctgaatggaagggccatcgctcaacggataaaaggtactccggggataacaggctgataccgcccaagagttcatatcgacggcggtgtttggcacctcgatgtcggctcatcacatcctggggctgaagtaggtcccaagggtatggctgttcgccatttaaagtggtacgcgagctgggtttagaacgtcgtgagacagttcggtccctatctgccgtgggcgctggagaactgaggggggctgctcctagtacgagaggaccggagtggacgcatcactggtgttcgggttgtcatgccaatggcactgcccggtagctaaatgcggaagagataagtgctgaaagcatctaagcacgaaacttgccccgagatgagttctccctgactccttgagagtcctgaaggaacgttgaagacgacgacgttgataggccgggtgtgtaagcgcagcgatgcgttgagctaaccggtactaatgaaccgtgaggcttaaccttacaacgccgaagctgttttggcggattgagagaagattttcagcctgatacagattaaatcagaacgcagaagcggtctgataaaacagaatttgcctggcggccgtagcgcggtggtcccacctgaccccatgccgaactcagaagtgaaacgccgtagcgccgatggtagtgtggggtctccccatgcgagagtagggaactgccaggcatcaaattaagcagtaagccggtcataaaaccggtggttgtaaaagaattcggtggagcggtagttcagtcggttagaatacctgcctgtcacgcagggggtcgcgggttcgagtcccgtccgttccgccacttattaagaagcctcgagttaacgctcgaggttttttttcgtctgtatatctattattgccagaatcgcaaaaatcctctgcattttacgctctttttcctcaacagtctgaagcccataatcacctcagttaacgaaaatagcattaaaagaggcatattatggctatccctgcatttggtttaggtactttccgtctgaaagacgacgttgttatttcatctgtgataacggcgcttgaacttggttatcgcgcaattgataccgcacaaatctatgataacgaagccgcagtaggtcaggcgattgcagaaagtggcgtgccacgtcatgaactctacatcaccactaaaatctggattgaaaatctcagcaaagacaaattgatcccaagtctgaaagagagcctgcaaaaattgcgtaccgattatgttgatctgacgctaatccactggccgtcaccaaacgatgaagtctctgttgaagagtttatgcaggcgctgctggaagccaaaaaacaagggctgacgcgtgagatcggtatttccaacttcacgatcccgttgatggaaaaagcgattgctgctgttggtgctgaaaacatcgctactaaccagattgaactctctccttatctgcaaaaccgtaaagtggttgcctgggctaaacagcacggcatccatattacttcctatatgacgctggcgtatggtaaggccctgaaagatgaggttattgctcgtatcgcagctaaacacaatgcgactccggcacaagtgattctggcgtgggctatgggggaaggttactcagtaattccttcttctactaaacgtaaaaacctggaaagtaatcttaaggcacaaaatttacagcttgatgccgaagataaaaaagcgatcgccgcactggattgcaacgaccgcctggttagcccggaaggtctggctcctgaatgggattaagcctctctgacagctcctccgggagctgtttttacatgctcgctaaggaaatcgataaaagcccggatgcgcgtacttaccgcacggtcgctgtaatagacggcactgaatggcatttccactggcaacactttatctgccattaactccaccaattctccgcgagcgatttctttgtcgatcatgtagtcggacaaacacgcaatcccgttgccactcaggcaaagctgtttcagtgtttccccactattggatgacaaaccgtacttcacctcatgtaattgtccatcgctacgggctatcggccaggtattgagggaagcgggttcagtgaatcccaggcaaatatgttgctttaaatcgtcgatcgtttctggcttcccgtagcgggaaatataatcgggggaggcgataatttttcgataactgttaaataacggcctggcacgtaagctggaatccgttaacgtaccagcgcgtatcgcgacatccacttttctttcgatcaaattaataatcgtttcggaggagactagcgacaaagtgacttccggatagcgttcacggaaaggcttaattaacggcatcagaaagtgcagcaccactggagttgcggcatcgatccgtaacagtccacgcggtgtattacgcgtctccataatttctgattctgccgctgccatctcctgcaaaattgactgtacgcgacgaaaataacgctcgccttcttccgtcaggctaagttgtcgcgtggtccgattaagcaggctaacgccaagtttcatctccagctttttcaccgcccggcttaccgctgagtttgcttgccctaattgttccgctgcccggctaaagctgccgctttcgacgaccgaaacaaaaatggcgagttcttccgacgtggctttcatttttgctcctgttgcaaaatagaagagatattttgaatttatttgtcattaaaccatcaggatgcgtgatatgtcatgcgatttaatgttctccataatgagcaaaattctgaccggtgtaagcacttgcttacataacaatatacaattgctcgttgaaagagtgagctaaaatccctataacagtagaaccctcccgagtgcggaagggttgacgtaatagaggtttcaaagtcaaaagtgcgaaaaaacacctatgccatgcgctatgttgccggacaacctgcggaaaggatcttaccgccggggtcttttgcgagcatcggccaggcattaccacctggggaaccgttaagtaccgaagagcgtattcggatcctggtgtggaacatatacaaacagcaacgcgctgaatggttgtcggtattaaagaactacggcaaagatgcacatctggtgttattgcaggaagcgcagacaacgccagagttagtacagtttgcgaccgctaactatcttgccgccgatcaggtacccgctttcgtgctgccacaacatccttctggcgtaatgaccctttcggcggcacatccagtgtattgctgcccgttacgtgaacgagaacccattttgcgtctggcgaagtcggcactggtgacggtctatccattacctgacacccgcctgttgatggtggttaatatacacgccgtcaacttcagtctgggcgtggatgtctatagtaagcagttacttcctattggcgatcagatagctcaccacagcggcccggtcattatggcgggagatttcaatgcctggagccgtagaaggatgaacgcgttatatcgctttgcgcgggaaatgtcgctgcgccaggtgcgttttaccgatgatcagcgccgtcgggcgtttggtcgcccgctcgattttgttttctaccgtggtctgaacgtcagtgaagcttctgtactggttacgcgcgcttccgatcacaatccgctactcgttgaattcagtcccggcaagcctgataaataaggtatgtcaggtctgccacagggcagaccaacgtttggcgctgcgcaaaacgtgagcgcggtggtggcgtatgacttatctgcccacatgctggatgtcgtggcacaagctgccgaagcccggcaactgaaaaatatcaccacccgccagggatatgccgaaagtctgccatttgccgataacgcatttgatattgttatcagccgttattctgcccatcactggcatgatgttggtgcagcactgcgagaagtgaataggatattgaaacctggcggtaggctgattgtgatggacgtaatgtctccgggtcacccagtgcgcgacatctggttacagacggtagaagcattacgcgatacctctcacgtacgaaactacgccagcggtgagtggttgacgttaatcaatgaagccaatctgatagttgataatttaattacagataagttaccgctggaattttcttcatgggtcgcgagaatgcgtacgccagaagcgttagtagacgctattcgcatttaccaacagagcgcatcgacagaggtgagaacgtattttgccttgcagaatgatggctttttcaccagtgatatcatcatggtagatgcacataaagcggcataaataaaaaaggcaccgggggaatcggtgcctttttattatctggtttgtcaggaatctggcatgttgttgtttttcacaaacaacgtcagcttatcgcctggttgcagattcgcagtgtcgctgttccagcgcatcacatctttgatgttcacgccgtggcgtttagcaatgcttgaaagcgaatcgcctttgcgcacacgatacgtaatgctatcgctgttgtttgccagtcgctgtgcgctactgcctgcaccaatcgtcaaactttggcctggcttcagcttagatccgcgcagtttgttccactgctgcaaatctttggtgcttacgccgagacgtgaagcgatacttgaaagcgtgtcgccagagcgtacggtgtaaacacggctgttaagcggcgtattgtcggcaaccagcgtcgactgtacagcagcaatttcgcctgaagccagagattcacgcagttgatctgcatgcttctttggcaccatcacgtactgcgggccacttgcgcccagcgtggagccttttacgccagcgttgaatgtcttcagcttgctgacggaaatccccgccatatctgctaccttcgccatttcaaccgggctgctcaggtgcacacgcgccagagcacggctttcatcggtcgttggcagacgtacgccataacgcttgctgtttttgagaatatcactcaatgccagcattttaggcacgtactgcttcgtttcctgcggcaacggtaacgaccagaagtccgtggatttcccacgcgctttgttcgttttaattgccttcatgacccgaccttcgccgctgttataagccgctacggtcagaagccagtcgccgtcaaacattttgttcagacgctgcatcatattcagcgcggcagttgttgaagcaacaacatcgcgacgcgcgtcataattgcgggtctgtttcaaaccataattgcgccccgtgctcggaatgatctgccagatgcctgcggcattggcgccagacgttgcgtgaggatcaaaagcgctctccactatgggtagtagtaccagttccataggcatgttacgttttttaacttgccctgctatccagtacatatacggctctgcccgtaaagttacatcgtggagatagctcttattgcgtaaatatttctgtttctgttcgcgaatccggtcattttccggaattcccatctttagctcgtcgccaatgaaagcccacaagtcaccatctggcgcgatagacgtcccatcgtccatccatcgtgcctgacttgtaaactttgctgcttccccttgaccagctgcagaaaggctctgtgcgtgctgttgaacgttgccggtactctggcaacccacgagcaggacagaggcgagtaatatcgcttttgccttcatgtgtgtgtcaatagttgcttaaaagacgaccgatcataacggcgaacggagccgatgacaagaaagttttatcagaacctatctttctttgaccttaaccatgcaaaacgctcttcaggttgttgcaataatgtttcttcattaattacattaattaaatcaatatcttccgttcttaaaaaaacattaatttgccgctcatttttcagaattacgggtagtgttatttgattttttgcccgtaactccttaactttacgataataatcatttatggacaaatcgtgcggaagaatactcaaagcaaacttcatatttgataaggtatattcatgagcacaacataccaatgtatcgtcaggtaacgcacttaactttttaagtgattgatacatttgtgatgctgtcccttcaaacaaccgaccacacccaccagaaaacagtgtgtcgccgcaaaatagataaggtttactgaagtaacagatatgtcctaaagtgtgacccggcgtagcaattacactaaattcatgccccaaaacgaaggcagtttcgccatctttgactacctgtgttgttcccttatcttgtgtctcttgtggaccatacaccacaatttgtggaaacttttccaccagttcttttacgccgccaacgtgatcgtggtgatggtgggtgagaaatatggcctccggttgccagttattggcggcaatggcgtttaatactggctctgcgtctccgggatcgacaatcaggcagcgacctgcttcatcattcaaaacccagatgtaattgtcatcaaaggcgggaatactgttaagattcatagattacctctcagtgtgaaacggaaggttgtgatgaaaccggcaagagtccctcaaactgtcgtggctcctgattgctggggcgatttgccctggggaaagctttatcgcaaggcgctggagcgccagctcaacccgtggttcactaaaatgtatggttttcatctgcttaagattggcaatttaagcgcagaaatcaattgcgaagcgtgcgcggtttctcatcaagtgaatgtttctgcgcaaggaatgcccgtccaggtacaggcggacccacttcatcttccttttgccgataaatccgttgatgtttgtctactggcacatacattgccgtggtgcaccgatccgcatcgtttattgcgtgaagccgatcgggtattgattgatgatggctggctggtcattagtggcttcaatcccatcagttttatgggattacgcaaacttgtgccggtattgcgcaaaacctcgccctataacagccggatgtttactctgatgcggcagctggactggctctctttgttgaattttgaagtgctacacgccagccgtttccacgttctcccgtggaacaaacacggaggaaaactattgaatgcgcatattcctgcgcttggttgcttacaacttattgttgcccggaaacggactattcctttaacgctaaatccgatgaaacagagtaaaaacaagccacgaattcgccaggcggttggagccacccggcaatgtcgtaaaccacaggcttaaacttcaacttggtagcctgtatcttccagtgtgggattcatcgccgcggcacgagccagttcatcacagcgttcgttttccgggtgtccggcatggcctttaacccattcccatttgatttgatgctgccccaatgcagcatcaagacgttgccagagatcgacattttttactggttttttgtctgcggttttccagccacgttttttccagttatggatccactgggtgataccctggcggacatactggctgtcggtactcaaaatgacttcgcaatgttcttttaacgcctccagcgcgacaatagcggccatcaactccatacggttgttggtggtgcgggtgtagccagcgctaaaggttttctcgcgtccgcgatagcgtaaaatagcgccgtaacccccaggtcctggattgcccagacacgaaccatcggtgaaaatttctacctgtttaagcatctctggtagacttcctgtaattgaatcgaactgtaaaacgacaagtctgacataaatgaccgctatgagcactgcaattacacgccagatcgttctcgataccgaaaccaccggtatgaaccagattggtgcgcactatgaaggccacaagatcattgagattggtgccgttgaagtggtgaaccgtcgcctgacgggcaataacttccatgtttatctcaaacccgatcggctggtggatccggaagcctttggcgtacatggtattgccgatgaatttttgctcgataagcccacgtttgccgaagtagccgatgagttcatggactatattcgcggcgcggagttggtgatccataacgcagcgttcgatatcggctttatggactacgagttttcgttgcttaagcgcgatattccgaagaccaatactttctgtaaggtcaccgatagccttgcggtggcgaggaaaatgtttcccggtaagcgcaacagcctcgatgcgttatgtgctcgctacgaaatagataacagtaaacgaacgctgcacggggcattactcgatgcccagatccttgcggaagtttatctggcgatgaccggtggtcaaacgtcgatggcttttgcgatggaaggagagacacaacagcaacaaggtgaagcaacaattcagcgcattgtacgtcaggcaagtaagttacgcgttgtttttgcgacagatgaagagattgcagctcatgaagcccgtctcgatctggtgcagaagaaaggcggaagttgcctctggcgagcataaatacctgtgaaaggcgctaaaaatagcgacttgggcgatttttgcagcaaacgattcaaaagatgagaaaaaccgttgacgaaggtcgaggcaatccgtaatattcgcctcgttcccaacggaacacaacgcggagcggtagttcagtcggttagaatacctgcctgtcacgcagggggtcgcgggttcgagtcccgtccgttccgccactattcactcatgaaaatgagttcagagagccgcaagatttttaattttgcggtttttttgtatttgaattccaccatttctctgttcaatgattttactctggcgtaggtgcgtgattctcgcttgttgtctcattcattaaaattcaataatgatatcgaaccattcagcttaaatatatttctagagaataaatttatattgattaaatgaatgtatatttcaaattgattttgtttgttattatttaagtgaggtatataattagagtccgttatcaatgctaaatattctaatcattatgacaggcgagggagtgtccaattatgaattcaaaaaagctttgttgcatatgtgtgttattctcgctgcttgcaggatgtgcctctgaatcttctattgatgaaaagaagaaaaaagctcaagtcacacaaagtaatattaataaaaacactccccagcaactgacagacaaagatttattcggtaatgaaaccactctggccgtatccgaagaggatattcaagctgcgcttgatggagatgagttccgcgttccccttaattctcctgtaatacttgttcaatccggcaaccgcgcaccggaaaccattatgcaggaggagatgcgaaaatattatactgtttccacattctctggtatcccggacaggcaaaagcctctgacttgtaacaaaaacaaagataaaaatgagaacgaggatgttgccagtgctgagaatatgaactggatgcaggcactgcgttttgtggctgcaaaaggacatcagaaagcgattattgtttaccaggatatgttgcagacaggaaaatatgactctgcgctgaaatcaacagtatggtccgactataaaaatgacaaactcactgacgctatctccctgcgctacctggtacgtttcacgctggtggatgtggcaacaggtgagtgggctacctggtcgccggtgaattatgaatataaagtgcttccaccattgcccgacaagaatgaagccagtacgactgatatgacagagcagcaaatcatgcaacttaagcaaaagacctataaagcgatggtaaaagatttggttaaccgctatcaataataaattatatctgccgccaggaatttctggcggcaataatacaaaattctttgcataagaaatttttcttgacaaagacagtgcaagaaaggacatggaatccggagttaaaaactgtttgttttagaatatttaattatttaactgctgaatcttccttgcgagaaatatatccattattacatttcatgccatttttaatatagattgctcctgggaaaattcccgtattattaccgcaggggtgataattagtattgacatatcctgtgacaaaaggagctattaaaggtgctattacgatagctattagtaaaaatataagagttagctgtattgttatgtctgtggcgaaattgactaccttcgtttttttgattaagaatgattttattatcgtaagtaaaattacatgaatatttaaaaaggaaaacgacatgaaaccgaagcacagaatcaacattctccaatcataaaatatttccgtggagcattttattattgaatatagaggtttaactccggtaaaaaacaaagaagcattgaatgcagggaaaaataatatggccataaaaaacatcgaaagaaactcttttaatttaacatgtaaacgcatggttaatcctcatatcacgggtggagtgttaagaacatacataaatggagtcatgttttcccttttccatttatcaagttcctgttgccgttttagtccatctctaattgcatattttaatttttctgataaatggcattgagcatcgatttcatttaaaacaactgtacacactatccctgtcagtaaaattgctcctccgacaagaattactggaaagccaaagctaacacaggcaaaagaagccagacttccaatagcggttgcaacaccaccggctataactgctttggccacatccattgaaaaatcgccaagaaaattaaccagatctcgctctgaactcataataaattctatggttctgctgatttaaccgcagagaagttcgccacagcaatccgaaaccactggcacgtggagaataagctgcacaggcgtctggacgtggtaatgaatgaagacgactacaaaataagaagaggaaacgcagcagaattattttcagggatacggcacattgctattaatattttgacgaatgagaaggtattcaaggcagggttaagacgtaagatgcgaaaagcagccatggacagaaactacctggcgtcagtccttgcggggagcgggctttcgtagtaataccccgactctccccgtccttaaacacaacccccactcaccacaacctaaactcatccgcatcctgccatgccggaaacttttctctatattcccgcaatgctgccatcgacagctccgcatcaatgcgcgttgcctgatgcgcgtcggcagtagcgataatctctccttgcggattaatcacccggctgtcaccgcgataatggcagccgttgccatcgctgccgacgcgattgcatcccgccacatacgcctgattctcaatcgcgcgggccgtcagcaatgcctgccagtgcagagagcgcggagcaggccagttggcgacgtacagggcgaggtcataatcgttgagattgcgcgaccacacaggaaaacgtaagtcgtagcacaccagcggcaaaatacgccagccgcgccattccacaatcactcgcgcattgcccgctttataatgtagatgctcatctgccatgcggaacagatgacgcttatcataaaaatgtaccgtgccgcccggctcaaccagcaaaaagcggttaaccgaaccagactccgtttgtaatgcaacactgcctgcaatcagcgcattgcactgctgcgccttagctgtcatccagttcactacgtcatcttgtgctagcgacgaagctgccgcttccatggcaaagccgctggtaaacatctccggtagaacgatcacatcgcgcccggtaataccttccagttgacgatcaaaatgacgcaggttggcaggaccatccatccacaccagtggttgctgcaaaagcgtaatcttcaaaccaggcacggtgtacaactcctttatgcgaagggttttataactttaacaccttatcaggcagttgccttagcgcagaataaattgataacaaatgctgatattggaaatatctgatttgcaaattatcgtgttatcgccaggctttaggaggttaataacatgggcaggataagctcgggaggaatgatgtttaaggcaataacgacagtcgccgctctggtcatcgccaccagtgcaatggcgcaggatgatttaaccattagcagccttgcaaagggcgaaaccaccaaagctgcatttaatcagatggtacaagggcataagctgcctgcctgggtgatgaaaggcggtacttatactcccgcacaaaccgtaacgttgggagatgagacgtatcaggtgatgagcgcgtgcaaaccgcatgactgtggctcgcaacgtatcgctgtgatgtggtccgagaaatctaatcagatgacggggctgttctcgactattgatgagaaaacgtcgcaagagaaactcacctggctgaatgtgaacgatgcgctttcgattgatggtaaaacggtgttgttcgcggcgttgaccggcagcctggaaaaccatccggatggctttaattttaaataattagcggataaagaaacggagcctttcggctccgttattcatttacgcggcttcaactttccgcactttctccggcaactttaccggcttcgtcgccagctcttccggatcaaagtcatcaacgttaatactgcgcagacggctttcttcagctttcaccagaatagcggcttcatctttatcaatcagccccttcaccagcgcgttgtgcgccagttcatccagacgggtaaacggcaggtttttacccagctctttacagatccgctgatgaattgggtcggcggcaatcacatccaccagcgcctcttccagcaagccaaccggattatgctcgctcggcgtcaggtactgaccgcgaccaatgcgggaacgggtggcgttcggcacttgtaaaatcttcgccactttatgatccagcttgtcagaaggtgccagataatgacgtccggtcgggaagatcaccacattcagcagcccggcaaccacgcggttcgggaagttttgcagtaaatcatccatcgcctgttcagcctgatacagcgcatcttgtacgccccagtgcaccagcggcaggtcggcttcattacggccttcgtcgtcataacgcttcagcacggcagaggcgaggtagagctggcttaaaatatcccccagacgggccgagatgcgctcgcgacgtttcaggctgccgcccagcactgccatcgagacatcagaaagcagggcgaggttggcgctcaggcggttcaggtgctgatagtagcgtttagtggcatcgccggttggcgtgctgctggttaaaccgcgcgtcaggcccagccagaagctgcgaactttgttgctaccgacgtgaccgatatgtttgaacaacagtttatcgaacgcgttgacgtcattgttcttcgccgcttccatctcttccagcacgtacggatggcaacgaatcgctccttgtccgaagatcatcatgctgcgggtcagaatgttagccccttcaacggtgatggcaatcggtgcgccctggtaagcacgcgccaggaagttgctttgcccgagcataatgcctttaccgccggtaatatccatcgcatcaataatcgactgctgcccgcggtgggtacagtgatacttaacgatagccgacagcacggcaggtttttcgccgagcataatgccgtaggtaatcagcgatgccgcagcatccatcacgtaggcattaccggcaatacgcgccagcggctcttcaatcccttccatcttaccaatagagattttgaactgacggcgaatgtgagcatacgcgccggttgccagcgctaccgatttcacgccgccggttgagttggaaggcagggtgatgccgcggcctaccgagaggcactccaccagcatccgccagccttgcccggccattttcggcccgccgatgatgtaatcgatcggcacgaagacatctttaccgcgcgtcggtccgttctggaacggtacgttcagcgggaagtggcgacgaccaatttccacgcccggcgtggtggttgggatcagcgcacaggtaatgcctaaatcttctgcaccgccgagtaatttttccgggtcggagagtttaaacgccagcccaagcacggtcgcaatcggtgccagcgtaatgtagcgtttgttccaggtcagacgcatccccagcacctgctggccctgccattcgcccatgcagacaatcccggtgtccggaatcgcgcccgcatcggaacccgcttccgggctggtcagtgcaaagcaggggatctcctgaccacgcgccagacgcggcagatagtgatctttctgctcgtcagtgccgtaatgttgcaacagttcgcccgggcctaatgagtttggcacgccgacggtaatcgccaggatcccgctcacgccggagagtttttgcagcacgcgagactgggcataagccgagaactccagcccgccgtactcttttttgatgatcatcgcgaagaaacgatgctctttaaggtacgcccacaactccggcggcagatccgccagctcatgggtgatctggaaatcattcgccatccggcaggcttcttctaccgggccgtcgagaaacgcttgctcttcggcggtcaggcgcggctgcggatagttatgcagctttttccagtccggcttgccctggaacaagtcgccctcccaccaggtggtgcccgcatcaatcgcttctttctcagtgcgcgacatcggcggcatcaccttacggaaaccgcgaaataccggcgcggaaatcatcgacttacgcataggcgcaaagttaaatggcacgaggataatggccagaggcaccagtacccacgccgaccacagaccagcaacgccgagggcggctgtccaggcgagcaaaatcagactgctgataaataagctcacgcggtgatagaacaacgcgccgagcaggacaaccgtagcgagaatactcaaaatcatcataacgaaaagccccttacttgtaggaggtctgaccacttgtgatgatatggttgtagtggatgtaaaaacatttagcaatatgtttacaatataattacaacaaagctcacattgttgctgtttttatccgcacttcaggtcaaaaagtcctggtcatagcacctgcccgtacttctcgcttttggcggtatccggtacactgcattttgtctattacatttatgctgaaggatatcctcatgtaccaggatcttattcgtaacgaactgaacgaagcggcggaaacgctggctaactttttaaaagatgacgccaatattcacgccattcagcgcgcggcggtcctgttagcagacagctttaaagccggtggcaaagtgctttcctgcggcaacggcggttcccattgcgacgctatgcactttgccgaagagttgaccggtcgctaccgtgaaaaccgtccgggctacccggcgattgctatttctgacgttagtcatatttcctgcgtcggtaatgatttcggtttcaatgatattttctcccgctacgttgaagcggtaggtcgcgaaggcgatgtactgctggggatctccacctccggtaactctgcaaacgtgatcaaagcgatcgcagcggcgcgtgagaagggaatgaaagtgatcaccctgaccggtaaagacggcggcaaaatggctggcacggcggatatcgaaattcgcgtaccgcactttggttatgccgaccgcattcaggagattcacattaaagtgatccatatcctgatccagttgattgaaaaagagatggttaagtaagtctggcgtaggccggataagacgtttacgccgcatccggcatttgtgcgctgatgcctgatgcgacgctgacgcgtcttatcatgcctacaaatctgtacgcgaaccgtaggccgaataatgcgttcacgccgcatccgacctgaaaattcttaaatcaatcttcgccgggggccatgcgctcccgctgttgtggaggttacccatgtgcgaattgctcgggatgagcgccaacgtccctaccgatatctgctttagtttcaccgggcttgtacagcgtggtggtggaaccgggccacataaagatggctggggcattaccttttacgaaggtaaaggctgtcgcacatttaaagatccacaacccagctttaattcccccatcgccaaacttgtccaggactacccgataaaatcctgttcggtggtggctcatattcgccaggctaatcggggcgaggtggcgctggaaaatactcacccatttacccgcgagttatgggggcgtaactggacttatgcccataacggacaactgacgggctacaaatcactggaaaccggcaacttccgcccggtaggcgaaaccgacagcgaaaaagccttctgctggctcctgcataaattaacgcagcgttacccgcgcacaccgggcaacatggcggcggtatttaaatatatcgcctcactggcggatgaactgcggcagaagggcgttttcaacatgctgctttcggacgggcgctatgtaatggcgtattgctcgactaatttacactggatcacccgccgcgcgccgtttggcgtggcaacgttgctggatcaggatgtggaaatcgacttcagctcgcagaccacaccgaatgatgtggtcacggtgattgcaacacagccgctgacgggcaatgaaacctggcaaaagattatgccaggcgaatggcgcttattttgcctcggggagcgtgtagtttgatgccagttgtggctgcacaacttcgtggcttaacggcttgctgaccacgtaacgaccattgaccacagaaacggttggtggcttacgggtttgctcaaagtagtcgtaacccggcttcagttgctcccagaagtccttaaagttggaatatttatggcgcttcatattggcgtcggtcatgcggaacgggtaaatactcacttgcacgctcggctgaccaaacaccagcgcaccagtaacgaactggaatatctcatcaataccctgattggtcattgcgtagcagccgatggaaacacaatcgccgtggatcatcaggtatttcccttcataaccatgcgcacggtcataggcattggggaaaccaatattaatcgctttgtagtaacggctgtctggttttaactgattacgctggacgctataaaacccttccgggcttttgaaatcgccctgacgctgttttggccctaagccgccggaatatttacagattttatagctgtcgagcagttgatattgctcgcccattttgacgtagagatcgagcgtacgttcttccttgaagatctggatgtagacaggggatcccatcaactgctgcttatactctttgctcacaggcgtggtagagctactgctgcccagcaaaccggcaaatgaaacgcacgggatcaacaacatcgcaagaattaatgcgattttacgcatactgcttattccttgataaaacggttacacacgccaggacggcaaaatggatcccaaatcggaatagtctggatttggaaggctcacattatcaccaaaagagttttacgcaagcctgtcggcgcagggtttacaaatttcatcggaagcgggctttacccaaagagcgccgcgtgagttccagttctctcaaatcgtaaaagtttatcggtaagtttgtaaatcaggatccagtccggttcgacatgagcatcgcgataacctttccatgaaccttgcagcgggtggtctttataaacagctggaagcggtaaagtattattgataagaagcgtcataagatatttcaatttattcatatccttatgacgcttttgtgcaagttttacatcctttgaatattgtcccgagtattcaatatccctttgaatcatatttaaattcctaatttatcaaataaatcatcggcgtctttggccttatgaacatcaatgccagcttcgctgtttttgattgattgaatggttaattgattaggctcgcgtaaatcaaacggcaatgccttttcacgcgcgacctttgtgagggttatgcgaaccaggtcagagatggtcagccccatcccggccagtacgtccgctgcctgattcttcagatcttcatcgattcgggcgcgaacaaacgcgttagcagccattggggtatctcctgtgctgtatatttattcagcttgaattgtagctcaaatgagcaacagcgacaatccatgagtaatttaataaacggatgtttttacataattaactgaaatatatatgttaattttataataatggtttattaagtttgttcagaaacgatccgggatacactgcaacattaaagcatgaccagccattattgagtatgtccttgccgtcgattccatcctttgtattgtcgggattactgttgatttgtttgccgttttcttcatttgccagcgccaccacatcacatatctctttcagctacgccgcccgccagcggatgcaaaaccgtgcgcgtttattaaaacagtaccaaactcatctgaaaaagcaggccagctatattgtggaaggcaatgccgaaagcaaaagggcgctacgccagcacaaccgggagcagataaaacagcatccagaatggtttcctgctccgctcaaggcgagtgacagacgctggcaggcgctggcggaaaacaaccactttttaagcagcgaccatctgcataacattaccgaagtggcgattcaccgcctggagcagcagcttggcaagccttacgtctggggcggtacgcggcctgataaaggctttgactgtagcgggttggttttttatgcctacaacaagatccttgaggctaagctcccgcgcacggccaatgagatgtaccactatcgccgggcaacgattgtggcgaacaacgacctgcgccggggagatttgctgtttttccatatccacagccgcgagatagccgatcatatgggcgtgtatttgggcgatgggcaatttatcgagtcgccacgtaccggcgaaaccattcggataagccgattagccgaacctttctggcaggaccattttttgggcgcgcgcaggattttgacggaagagacgattttgtaggacggataaggcgtttacgccgcatccggcagttgtacgcaggtgcctgatgcgacgctggcgcgtcttatcatgcctacgagcccgcgaatatttgcgagccgctttcccgatataaaacaacctcattgccaacctttccttttcttcttaccgttgagaaaaaggagtcgccatgtctgaatatcgtcgttattacatcaaggggggaacatggtttttcacggtgaatttacgaaatcgtcgaagccaacttttgaccacccagtaccagatgctccgtcacgccattattaaagttaagcgagacaggccttttgaaatcaacgcctgggtcgttttgccagagcatatgcactgtatctggacattacctgaaggcgatgatgatttttcctcgcgctggcgggaaattaaaaagcaatttacccatgcttgtggattgaaaaatatctggcaaccacgtttttgggagcacgccatccgcaataccaaagattataggcatcatgttgattatatttatataaatccagtaaagcatggttgggtaaagcaagtgagtgattggccattctcaacgttccatcgcgatgtcgcgcgagggttatatcccatcgattgggcgggggacgtaacggattttagtgccggggagcgtatcatttcataattgtgcgcagatgcctgatgcgacgctagcgcgtcttatcatgcctacaaacttgtgccggatcggtaggccggataaggcgtttatgccgcatccggcagttatgcgcagatgcctgatgcgacgctggcgcgtcttatcatgcctacaaacttgtgcctgaacggtaggacggataaggcgttcacgccgcatccggcagttgtgcaccaatgctggatacttacatcaacgcccccataatcttcaactccagctcatccggcacttcgttatacgacagcacatgcagccccggcgcaaacaaccttgcataacgcgccagcaaagggcgcagctgcggtggcaccagcagcaccgggtctttccccgccgctttcatctgctctttcacctgtggcatcgtactctggaactggttgagcatattcggatcgaccggcacgctgtcgagcatcactttcccgccctgttgcgcctgattcaccacgttggtcagcagattttccagctcattattcagcgtatacaccgtcagctcctgcttgcgaacgaacggatgggtaatgctgcgccgcaatgccaggcgcacatcggccgccagcagaatatgatctttcgtcaccgtgctactggcgaccagcacggtggcgatggtgacgatatcgcgcagggaaacgccttcggtcagcagcgcccggtacactttcagcaactggctgtaattgagcgccgcgctcaaatcttccgccagacgcggtgccgtcgacgataaacggttatgcaactgcgtaatatcatcatagttaaacaaatcaggaatatagctgcgcacaatcttatttacatgggtagcgatcacgctggcgctgtcgatcacctgataccccatattcagcgccttcgctttctgcgccgcctggatccaggtgaccggcatcccgtacgccgggtcgttcccctgcacgccgtcaatctcgccgtaggtttcgctggagggcagggccatcagtttatccgccggaatatccgcttcatcagcctttatgccgttgatgaaaatggcgtactgactgggcttaaggcggaagttttcccgaatgcggatctccggcagcagcacgccgttgccgtcagaaatcacctgccgcacgccgcgaatccgctgggtgagcgggttaccctgtgctttgtccaccagcgccaccagtttgtaaccgaggcttaaactgataggctcgatcagcggaatggtttcccaactgacctgctgctcgctggtttcggtgatggtgcgggtcagcgtttcgaggcttttctcttccgcctccgccgccagcggctgtttgctcatccgccagccggtaaaaccaagcagggcgctgaacagcaaaaacggcaggtgcggcattcccggtaccaccgccagcacgaacataatcccggtggcggtgtagagcaccgacgggcttgccagcagctggttacgcacgtcatgggcgatatcgccgttgtcgctgacgcgggtgacgataatcgccgccgcggtggagagcagcagggaagggatctgcgccaccaggccgtcgccgatggtcatcagcacatactgctggaaggcagcatcggcgctcaggttgtatttgaagatcccgatacagacgccgccgatcaggttgatcgccagaatcatcatcccggcgatggcgtccccgcgcacaaacttcgatgccccgtccatcgcgccgtagaaatcggcctcgctggcaacatctttacgccgggtttgcgcctgcgcctggttgatcaatccggcgttaagatcggcgtcaatcgccatctgtttgccgggcatcgcgtctaaggtaaagcgggcagaaacctcggaaatacgctcggcccctttggtgacgacaataaagttgattgtcaacagcgtcagtaaatccgagcgtgaaagcattatcgccgcgctgcacgggcagtcgatttttaacggtggtgggctgtcgccgttaaataaaatcagcccgtctcatccgccaaaacctgccaccgtggcggtgccggaagagacggagaaaaaagcgcgtgatgtgaatgagaaaacggcgctgctgaagaagaaatccgccaccgagcttggtgagctggcaaccagtatcaacaccattgcccgtgatgcgcatatggaagcgaatctggagatggagattgttccccagggattacgcgtgctgattaaagacgaccagaaccgcaatatgtttgaacgcggcagcgcgaagattatgccgttctttaaaacgctgctggtggagctcgcgccagtgttcgactcgctcgataataaaattattattaccgggcataccgatgcgatggcctacaaaaacaatatctacaacaactggaacctttcgggtgaccgcgcgctttcggctcgtcgggtgctggaagaggccggaatgccggaagataaagtgatgcaggtaagcgcaatggcggaccagatgctgctggattccaaaaatccgcaaagcgcgggcaaccggcgcattgagattatggtgctgaccaaaagtgcgtccgatacgctgtatcaatactttggtcagcatggggataaagtggtgcagccgctggtgcaaaagctggataagcagcaggtgctttcgcagcgaacgcgttaaatgctgaatctttacgcatttctcaaaccctgaaatcactgtatactttaccagtgttgagaggtgagcaatgcgtaaaatcattcatgtggatatggactgctttttcgccgcagtggagatgcgcgacaatcccgccctgcgcgatatccctattgctattggcggcagccgcgaacgtcggggggtgatcagcaccgccaattatcccgcgcgtaaatttggcgtacgtagcgctatgccgacagggatggcgctcaaattatgcccacatctcaccttgcttccggggcgctttgacgcctacaaagaagcctcaaatcatatccgtgaaatcttctcgcgctacacctcgcgcattgaaccgttgtcactggatgaggcttatctcgatgtcaccgatagcgtccattgccacggttctgcgaccctcatcgcccaggaaatccgccagacaatcttcaacgagctgcaactgacggcgtctgcgggcgtggcaccagtaaagtttctcgccaaaatcgcctccgacatgaataaacccaacggccagtttgtgattacgccggcagaagttccggcatttttacaaaccttaccgctggcaaaaatccccggcgtcggcaaagtctcagcggcaaaactggaagcgatggggctgcggacctgcggtgatgtacaaaagtgtgatctggtgatgctgcttaaacgctttggcaaatttggccgcattttgtgggagcgtagtcaggggattgacgaacgcgatgttaacagcgaacggttgcgaaaatccgtcggcgtggaacgcacgatggcggaagatattcatcactggtctgaatgtgaagcgattatcgagcggctgtatccggaacttgaacgccgtctggcaaaggtaaaacctgatttactgattgctcgccagggggtgaaattaaagttcgacgattttcagcaaaccacccaggagcacgtctggccgcggctgaataaagctgatctaatcgccaccgcgcgtaaaacctgggatgaacgccgcggcgggcgcggtgtgcgtctggtggggctgcatgtgacgttgcttgacccgcaaatggaaagacaactggtgctgggattatgatgtatactattatgtatattctggtgtgcattattatgagggtatcactgtatgcatcgaattctcgctgaaaaatcggtcaatatcactgagttacgtaaaaacccagctaaatactttattgatcaaccggttgcggttctttctaataatcgccccgcaggatatctcttaagtgccagcgcattcgaagcgttaatggacatgcttgctgaacaagaggagaaaaagcccataaaggcgcgcttccgtccaagtgctgcaagattagaggaaattacacgccgcgctgaacaatatcttaatgatatgacggatgatgatttcaatgactttaaggaataaggatgcgggtattcaaaacaaaacttattcgcctgcaacttacagcagaggaacttgatgcgttaacggcggattttatttcctataagcgtgacggtgttttgccagatatatttggtcgcgatgcactctacgacgactcctttacctggccattaatcaaatttgagcgagttgctcatattcatctggcaaatgagaataatccatttccgccacagttgcgccaattcagcagaacgaatgacgaagcgcatttggtatattgtcagggggcgtttgatgagcaagcatggttgctcattgccattctgaaacctgaacctcataaactggctcgagataacaaccaaatgcataaaattgggaaaatggcagaagcgtttcgcatgcgtttttgaatttatattatgaataacatacaaataagaaactatcagcctggcgattttcagcaactatgcgctattttcattagagcggttacgatgaccgccagtcagcattattcaccacaacaaatttccgcctgggcgcagattgacgaatctcgctggaaggagaaactcgcgaaatcacaagtgtgggttgcgatcattaatgcacaaccggttggttttatttcccgcattgaacattatatcgatatgttatttgttgaccctgaatacacccgccgtggggttgccagcgctttgttaaaacctttgattaagtctgaatccgaacttacggtggacgcaagcataaccgcaaaacccttttttgaacgttatggttttcagacagttaagcagcagcgcgttgaatgccggggagcgtggtttactaatttttatatgcgatataaaccgcaacattaaatccagcttgcaatgaaaataacgcccgcctggtatgtgcgcgttttctgattccacaaactgcaaggaggtaaatcatgacaaatcctttatcaatgactctttgcagacctttccaggattaattctttttttcttgccctggattcgtctgccatttcctgatttttatatttatatactctaaataattcgagttgcaggaaggcgacaagcgagtgaatcgccaggagcttacataagtaagtgactggggtgaacgaacgcagtcgcagtacatgcaacttgaagtatgacgagtataaatggaatggtacatgggcaaatatattcgtcccttatccgatgcggtatttaccatcgcatctgatgacctgtggatcgagagtttagcgatccaacaattacacaccacggcaaatttacccaacatgcagcgcgtagtggggatgccagatttacaccccggacgcggctacccgattggcgcagcgttcttctctgttggtcgtttttacccggcaagacgtcgcggtaacggtgctggaaacagaaacgggccgctactctgacacactgcgttcggcgctggtttctctcgatggcgataacgcatgggcattaagcgaaagctggtgtggcactattcagtggatttgtccgagtccgtatcggcctcatcatgggcgcaaaaactggtttctgggcattgggcgttttaccgctgatgagcaggaacaatcggatgcaatccgttatgagacgctgcgttcgtcggggccgggcggtcaacatgtcaataaaaccgactcggcggtacgcgccacgcatttggcatccggtattagcgtgaaggttcagtcagagcgtagtcagcatgctaacaagcggctggcacgattgctgattgcctggaagctggagcaacagcaacaggaaaatagcgcggcgctgaaatcgcagcggcgaatgttccatcaccagattgaacgtggcaacccgcgacggacatttacagggatggcttttatcgaaggataatgaaggatgaaactgccggaaggcgattaaacgccatccggcagcaaatcaaataattacttcgccggaatttctttcagcagttcagtcagcagtgtccagtaatgacctacgctttcgatgtgaacttgctcatccggagagtgtggaccggtgatagttggcccgatagaaaccatgtccatttccggatacggttttttgaacagaccacattccaggcccgcgtggataatctggatgttcggcgtcttgttgaacaggcgctgataggtttcacgtaccagatgcatcaccggagaattagcgtccggctgccagccaggatatgcgcctttcgcttcggttttcgcgccagccagtttacccagcgaatccagcatgctcaccacgtagtctttaccgctgtcgatcagtgaacggatcaggcagtgaatttctacgttattgtcagtcatggtcaccacaccgacgttcagggaggtttcaaccacacctttggctacatcggagttacgaatcacaccgttcggggtggcgttcagcagacgaataaaggtatcgcgagatttcgcaatcagggcagctttatcgttcgctacagagtccagcaacaaggccagatttttctctttttctgccagctcgtttttcaggatctcctgataggtattcaccagagatttcaggacgtcgactttatcagctgcgacagcaatggtcgcaaaggcttcacgcgggatggcgttacgcagtgtgccgccgttgaaatcgataaggcgcagatccagttcttccgcatgacccgccaggaagcgcaccagcagtttgttggcattacccagcccaacgtggatttccccgccggagtgaccgcctttcagaccttttaaggttaacttgaaggtttcaaaaccagctggaaccgcttcacgatctaaatgcaggttggaggtgaagtcgataccccccgcacaacccatgtagatttcaccttcttcttcggagtcggtgttaatcagaatatcagcctgcaaccagttgccctgtaagccgaacgcaccgtccataccggcttcttcggtcatggtcagcagcacttccagcgggccgtgaaccacgttttcgtcagccagaaccgccagcgcagaggccataccaatgccgttatccgcacccagcgtggtgccgcgcgctttaacccattcgccatcaatataaggctggataggatctttcgtgaagtcatgcacggtgtcgttatttttctgcggcaccatatcgaggtgggcctgtaagacgaccggtttacgattttccatacctgcggtagcaggtttacgaatcaggatattacctacctgatcgcgttcgacatggaaacctttctcttttgcccaaccaacaatgtattcagcgagttgctcttcatgataggacgggtgaggaatagaacagattttggcaaaaatatcccacagcggctgtggagataattgagacagttcagacacgttaagtctccttgtcgatcacccgcaaaacagtattgcaggtcacagggttagcagaaaatgttgtcaacacaagacaggcttgcgagatatgtttgagaataccactttatcccgcgtcagggagaggcagtgcgtaaaaagacgcggactcatgtgaaatactggtttttagtgcgccagatctctataatctcgcgcaacctattttcccctcgaacactttttaagccgtagataaacaggctgggacacttcacatgagcgaaaaatacatcgtcacctgggacatgttgcagatccatgcacgtaaactcgcaagccgactgatgccttctgaacaatggaaaggcattattgccgtaagccgtggcggtctggtaccgggtgcgttactggcgcgtgaactgggtattcgtcatgtcgataccgtttgtatttccagctacgatcacgacaaccagcgcgagcttaaagtgctgaaacgcgcagaaggcgatggcgaaggcttcatcgttattgatgacctggtggataccggtggtactgcggttgcgattcgtgaaatgtatccaaaagcgcactttgtcaccatcttcgcaaaaccggctggtcgtccgctggttgatgactatgttgttgatatcccgcaagatacctggattgaacagccgtgggatatgggcgtcgtattcgtcccgccaatctccggtcgctaatcttttcaacgcctggcactgccgggcgttgttctttttaacttcaggcgggttacaatagtttccagtaagtattctggaggctgcatccatgacacaggcaaacctgagcgaaaccctgttcaaaccccgctttaaacatcctgaaacctcgacgctagtccgccgctttaatcacggcgcacaaccgcctgtgcagtcggcccttgatggtaaaaccatccctcactggtatcgcatgattaaccgtctgatgtggatctggcgcggcattgacccacgcgaaatcctcgacgtccaggcacgtattgtgatgagcgatgccgaacgtaccgacgatgatttatacgatacggtgattggctaccgtggcggcaactggatttatgagtgggccacccaggcgatggtgtggcaacaaaaagcctgtgcggaagacgatccgcaactcagtggtcgtcactggctgcatgcggctacgttgtacaacattgccgcctatcctcatctgaaaggagatgacctggccgagcaagcgcaggctttgtcaaaccgcgcctatgaagaggccgctcagcgtctaccgggcacgatgcggcagatggagtttaccgtacccggcggtgcgcccatcaccggctttttgcatatgccgaaaggcgatggcccgttcccgacggtattaatgtgtggtggtctggatgcgatgcagacggactattacagcctgtatgaacgttattttgcgccgcgcggcattgcgatgctgactattgatatgccgtcggtgggcttttcttcaaaatggaagctcacccaggactccagcctgttgcatcagcacgtcttaaaggcgctgcctaacgtaccgtgggtggatcacactcgcgtcgcggcctttggtttccgtttcggcgctaacgttgccgtgcgtctggcataccttgaatcgccgcgtctgaaagcggttgcctgtcttggtccggtagttcataccctgttgagtgattttaagtgccagcaacaggtgccggaaatgtatcttgacgttctggccagtcgtttggggatgcatgatgcttccgatgaagcgttgcgcgtggagctgaatcgctattcattaaaagtgcaaggattgctgggacgtcgctgcccaacgccaatgttatcaggctactggaagaacgatccgttcagcccggaagaggactcacgcttaatcacctcatcatctgctgacggtaaattattagagatcccatttaacccggtgtatcggaattttgacaaaggtcttcaggaaatcaccgactggatcgaaaaacgcttgtgttaaaaatttgctaaattttgccaatttggtaaaacagttgcatcacaacaggagatagcaatgacgttaccgagtggacacccgaagagcagattgatcaaaaaatttaccgcactaggcccgtatattcgtgaaggtaagtgcaaagataatcgattctttttcgattgtctggctgtatgcgtcaacgtgaaaccggcaccggaagtgcgtgaattctggggctggtggatggagctggaagcgcaggaatcccgttttacctacagttaccagtttggtctgttcgataaagcaggcgactggaagagtgttccggtaaaagacactgaagtggttgaacgactggagcacaccctgcgtgagtttcacgagaagctgcgtgaactgctgacgacgctgaatctgaagctggaaccggcggatgattttcgtgacgagccggtgaagttaacggcgtgagtgaaatgtgccggatgcatcacatccggcaatattcattaaaactgatacgtcatgccaaccgcgacaatatcatcattattaatattcaatttgttatcgctatccagttggttgattttataatcaacaaacgctgacatatttttgttgaaataatacgtagcaccgacgtcgatataattgaccagatcttcatcaccgataccttcaatatctttccctttcgataagacataacccagcgatggacgcagaccaaagtcaaactggtattgagcgaccgcttcaaagttctgtgtcttattggcaaagccgccagttattggcgtcattttgcgtgtttcagaatagaaagttgccagataaatattattggcatcgtatttcagacctgttgcccatgcttctgcacgcttgcctgtgccacggctttgcaggttctgctcgttggtgcgatctgagttggtataggccccactaatggcgaaatcgctgccgccaaagtcatatgtcaatgacgtgccgaagccatcgccgttttgctttttaacgtcgcggttttcgtttttcccttgatattgcagggttaagttcaggccatcgataacgccgaagaagtcggtgttccgatacgtcgccagaccgctggcgcgtttggtcataaagttgtcggtctgcgccgaggaatcgccaccaaattccgggaacatatcggtccaggcttccacgtcatacaacgcccccaggttacgaccataatcgaaagaacccaaatctttatatttcaacccggcaaaagcgagacgcgttttttgctgtgcagtatcactctctgctttattaccggcaaactctgcttcccaacgaccataaccagtcagttgatcgttaatttgtgtttcgcctttgaaaccaaaacggatataactctggtcgccatctttactggcgttatcactcatataatgcatggctttaactttgccatagacatccagtttattaccgtctttattatatatttctgcagcctgtacagatgcagatgccacaatgcccatcaccactaatgccagagtgctctttttcattttcattcctgattttaattaacgcgcgaatattcagcgggagagtcccgttgaaaacaggaaagtttttaacctgagattgttaaagatatattacagattaataatattcttaaaatgtggtaatttattaaatctgtaataaaagcgtaaacaactgccgctaggcttgctgatcccgcgcaacaaaacgccatgctttgctcgcagatggttggcaaccgacgacagtcctgctaaaacgttcgtttgatatcatttttcctaaaattgaatggcagagaatcatgagtgacagccagacgctggtggtaaaactcggcaccagtgtgctaacaggcggatcgcgccgtctgaaccgtgcccatatcgttgaacttgttcgccagtgcgcgcagttacatgccgccgggcatcggattgttattgtgacgtcgggcgcgatcgccgccggacgtgagcacctgggttacccggaactgccagcgaccatcgcctcgaaacaactgctggcggcggtagggcagagtcgactgattcaactgtgggaacagctgttttcgatttatggcattcacgtcgggcaaatgctgctgacccgtgctgatatggaagaccgtgaacgcttcctgaacgcccgcgacaccctgcgagcgttgctcgataacaatatcgttccggtaatcaatgagaacgatgctgtcgctacggcagagattaaggtcggcgataacgataacctttctgcgctggcggcgattcttgcgggtgccgataaactgttgctgctgaccgatcaaaaaggtttgtataccgctgacccgcgcagcaatccgcaggcagaactgattaaagatgtttacggcattgatgacgcactgcgcgcgattgccggtgacagcgtttcaggcctcggaactggcggcatgagtaccaaattgcaggccgctgacgtggcttgccgtgcgggtatcgacaccattattgccgcgggcagcaagccgggcgttattggtgatgtgatggaaggcatttccgtcggtacgctgttccatgcccaggcgactccgcttgaaaaccgtaaacgctggattttcggtgcgccgccggcgggtgaaatcacggtagatgaaggggcaactgccgccattctggaacgcggcagctccctgttgccgaaaggcattaaaagcgtgactggcaatttctcgcgtggtgaagtcatccgcatttgcaacctcgaaggccgcgatatcgcccacggcgtcagtcgttacaacagcgatgcattacgccgtattgccggacaccactcgcaagaaattgatgcaatactgggatatgaatacggcccggttgccgttcaccgtgatgacatgattacccgttaaggagcaggctgatgctggaacaaatgggcattgccgcgaagcaagcctcgtataaattagcgcaactctccagccgcgaaaaaaatcgcgtgctggaaaaaatcgccgatgaactggaagcacaaagcgaaatcatcctcaacgctaacgcccaggatgttgctgacgcgcgagccaatggccttagcgaagcgatgcttgaccgtctggcactgacgcccgcacggctgaaaggcattgccgacgatgtacgtcaggtgtgcaacctcgccgatccggtggggcaggtaatcgatggcggcgtactggacagcggcctgcgtcttgagcgtcgtcgcgtaccgctgggggttattggcgtgatttatgaagcgcgcccgaacgtgacggttgatgtcgcttcgctgtgcctgaaaaccggtaatgcggtgatcctgcgcggtggcaaagaaacgtgtcgcactaacgctgcaacggtggcggtgattcaggacgccctgaaatcctgcggcttaccggcgggtgccgtgcaggcgattgataatcctgaccgtgcgctggtcagtgaaatgctgcgtatggataaatacatcgacatgctgatcccgcgtggtggcgctggtttgcataaactgtgccgtgaacagtcgacaatcccggtgatcacaggtggtataggcgtatgccatatttacgttgatgaaagtgtagagatcgctgaagcattaaaagtgatcgtcaacgcgaaaactcagcgtccgagcacatgtaatacggttgaaacgttgctggtgaataaaaacatcgccgatagcttcctgcccgcattaagcaaacaaatggcggaaagcggcgtgacattacacgcagatgcagctgcactggcgcagttgcaggcaggccctgcgaaggtggttgctgttaaagccgaagagtatgacgatgagtttctgtcattagatttgaacgtcaaaatcgtcagcgatcttgacgatgccatcgcccatattcgtgaacacggcacacaacactccgatgcgatcctgacccgcgatatgcgcaacgcccagcgttttgttaacgaagtggattcgtccgctgtttacgttaacgcctctacgcgttttaccgacggcggccagtttggtctgggtgcggaagtggcggtaagcacacaaaaactccacgcgcgtggcccaatggggctggaagcactgaccacttacaagtggatcggcattggtgattacaccattcgtgcgtaaataaaaccgggtgatgcaaaagtagccatttgattcacaaggccattgacgcatcgcccggttagttttaaccttgtccaccgtgattcacgttcgtgaacatgtcctttcagggccgatatagctcagttggtagagcagcgcattcgtaatgcgaaggtcgtaggttcgactcctattatcggcaccattaaaatcaaattgttacgtaagatcttatcattctcccaccaaaaaattatcttaatgtaacagctggtgtaagtaaattctatcaacgaagatcaatcttatctactgaccaaaaaggcctgatagggcttcgctcactatacatccttggctgcaggtttagttgtacaccactcctaaatttaatgtgttggcaatgtgttcaataaagctcgaacaaattagctcattatgatcggttaatacttcaacttctggttgcatgattgtttgtccgtaaaaagataacgcgcctgccgggtagtagcaggcgcattacgcaataggtaaacaagggaggaagttcagaaatgtaaatcgggaaggttgtacgcaatgttcatcgtactacgttgttacggctttgccgcaacaagccagttgcctgccgcgctcgcagaatgtctgcagcccggagataaggagattgttcctgccagctaaatcccttcctgtcgatacgaaccagctcgtatttttctaccagaaaattcacggcatcggctagggtgataccggcatcgatgtgttccttaatcacagcctcattgcagaatggcgtgtcgtttattgtcagaccatagtgctgttccagcagacgtgtcagtaacatttgccagacagccacgggtgacaggcagggcttcaccgcccgctgagttattgcaggtaaagttttcatgtttgctctcgtgtaggtaattaacgctgagtggggtaaatggcgatgtatacgtagccgcaactgccaagggtgtcggcttcgcaggttaaatcgttgtggtacagggtaacgcagtgggcatggtgggggctgagttcaccggtggtcagcatcgattccatctggaggataaagtgcgggaatgtttcatccagcttccggcattcgatgtcactgaacttgccggtgatgctggcccggtcagccagataatgcagtcggttgccttcctgcaccagacgggctcccaggcgcagtgtaatctcccgctgcaggcccctggtagggttgctcattacagttctccactattgtcagttcagggtgatgctcatcaggcaggtatagggcccattgcggtcctggcggcgttcggcgtataccgcgaggactccggcgatatccggaacgtccctgccggtgtaatgacagacgctaccgtgccactggtatttgccggtgcagtagcgaaagattcgggactcaggatgctggcggtatatcgtcattgccctgcgtttactgataattttcatgtaatacctcaaagcagaccgtgttctgcgaacgaatagatttgcctgccaccgacaatcagatggtcagggacacggatatccaccagctgaagcacctgaaccagtcgctgcgtgagggttttgtcggcctggctaggtgtcgtctcgccggaaggatggttatgcgcgagtatcaccgccgccgcgttgaagtgcagagcacgtttgaccacctcccggggatgcacctcggtgcggttaatcgtgccggtgaagagcgtttcatgggcaatcaactgattctggttgtccagatacaacacccggaactcttcccgctcaagcgcggccatatgcagtcgcagccattcacgtacggcgtgggtagaggtgaaggctacgccgggctcatgcaggtggcggtccagagccctgagcgcccgctgaatgagacgccggtcctgtggcgtcatctcgccgggtaaaaaggaaagctgtttcatctgttgctccttcggtcagtcgataatacgcagaatggcgtgagcctctggatgttgcatggcatactcccgcaggcggtaatagtgtgcggtcatcgcgtcacattctgtacggcaggcatggtggctatacgcaatcaggcagacagcaatacctgctgcttctgcactcatttgggcatcgttaccgttcaggcagttaaacagacgccatgtctcatcgttgtcaggctcgggggacataaatgcgccgccattgctgagggtgtagaacgaccagataccaccgctgtagccctcacagaagcggtccatccaggcgaagatatgcggctccaggagtagccactgcgggatagcgccaaagtactgtggccagaaatcgatacgctgttcatcggggaccggcgtgacggtcagttcaaattcgggttggttagcgggtgcgaggtcgtgctgcgtctgtgttgtcatgggtatgtctccgtcaataaaaacgccagcggcgatggctggcgtatggggatataaagtgtgttcggggaggtgaatgcgggtaaatgcttcgcgatcagcgggtggccgtgtctgtacggatgcctgaggtgcggatatagcggttaagaccttcaccggcatccggctcaaagttccatgcccgccagaccatccggccttcagtatcacgaaccaccagacggaagtgactgccctggtcgtcttcgagtgtgatattgctgtacgtggtagtgaccgcttgcgcttgtctccgggtgaaaggccccggtggcagcaacacggattgggtcattttcgggctcctgataaaagaaaaccccggcagcctgctagctgtcggggtgaatttgctggggaagatactactatcagtcgttgctgcagtctccgagagtggacagaactttctcagcgttcttccggtccgcagtgaaggtccctgctttgtggtcattgacgtagacgtcgaactgcccggcctcagagatattgctgatgaagtcaaaccaggcgttatcgccgttacgccagcccaggctggacggaataatgtactgctggtgatccatcactacggtgatagtagtgtcgtcatcgtgcgaactgaccatcttgtcatcggcaagggtaagaaagactgaatgctgatagaaaccattctggtccgggttccctgtgcagttgatggtaaacgtctttccgctggcttcggtcacgctgtattccgtattgccctgaccgtaaccctgctgccagaaccccgggatagcagaggcattaaagctcgcgagcagtacacccgccagcataaaccgacttagtgaaagtattgtcattcttgtctcctttgtcgttgttttattcctgattgtcagggttcgagggtatcagtagctgccccatcagtttgccgtcatgggcgtactcaaagtatttttctttggtatacgggtccgtcacctcctggtattccagtttgatgttatcggcaatacacagcgcattcatcagtggctggacggttttttcctgcatatccacgaggtagtagtaactgccatcctcgcagccatcgggcgactggcgggtacgtaaaacctgcaaggtgggaccggataagtagtcaacctgtgaccattcttcgctgacatcatcctggtggctgaccacatcactgaaacgcggtggggtgaggtccttaaatttactgatggccttcaggtcatcacttctgtcatcgcatgcgatgagaaacagagtggtggcaaccagcgccagcagaggcagtgttttacgtttcattatttttttcctgaaatcagacgaaccactttggcaaagacataaatgcccacgaaaatacccaccggcacgccgacgaacggtgtcagcgcgacactggcagcaccggctgcgccacctcccgtcagcagtgcggcaacagtggcaagggtcagggccgcgagactgtcggacaccccggttttgttcagaatgatgacgatgacaacaatggcgataatggcaatatccggactgatactccaggtccagatacatcagccgctcacgaaaatcacgccgcagcgtgcgcaccgacacaccaaactcagcggcaagcttacgcacactcagcgtttcccctgccaccagacggctgattatcagtgacagcctgacagccagccggtcatggcggcgttctgcctgtgtcatgagacgttctccgtgaaagttaactgactgaaaatgatgtgattactttaaagagggggtcggacagggtatggacaccacagaaactatttttcatttctgcaaaagccagaggcagcgggggttacaggccttccctcggtgagtgaggaccgtcagcacggtgcgatgcggacaggtggtgtccgatattaacaaagcagcaacattaaacggtcactgcagttgcgtgagcagggcttccgccatcacccacagtgcccggttaagtttcacgtccccgtcgataccgcgaacggcacgggtatgtgaccgtcctcctttggcattacggccactgagcccgcccttaatcaggttctcctgaatacgctggtacgtggtccacaggtcattgctctcatcctgccagcggcgaggggagaggatctgcgattcagtcaccggctggtggtcttcaccaaagcggtatgtgagggcggcttttgccagtgcctgctgtgccgggggtggcaacagcaacgactgcatggcatcccgtttctcctccacccggtcaaaaatccccagcacctcatacgcgccttcaatcacctgactcaccacgtcccccttgtgtggcacccgcacctcgccaaacgactcaccgcagacgagcccgttctgacaaaccgcacgaaatagtcccggcaacatctgatacgaactggttccatcgtgagagttgagtagaataatttccggcacctgtttaccggtgatctgcccttcccgccgcagacgcagcatatgctttgtatgttcacgacgacccgggtcacgcacgcgggtctgacaggcaaagaatggctggaagccttctcgctgtaggctgtcgagcagggagatggtgggtatataggtataacgctcactacgggactcgtgtttgtcctcactgaatacactgggcactacgcgaaacagctcttcacgggttaacggacggtcgcgacggataaggtttgctgcgccaaagcgcgaagccagacgggtcataagcagactcctcataacgggaaaacaaataaaagggatccccgtcgcatcggcgacaggggcagggaagtaacagggatgggttaaatactcagaagaagaaatcccagacggcgcgggccactgacaccaccgtggtgcgcacggcctgaatgacggcccgcaccggggcgggtatcaggggaaaggcactgatgctatcgagtacggccccgacggtttcaccaaaatcgctacgagcctgttcccggactaccgtcgtgcgaaaggaaggatggagttgcgacaccaccgggctggtggcctcacgtggcaggcacttaatcatccgctcggccatcaccttaagcccccattgtagacggaccgacacagcacacaccggatggacgggctggaacagctcatgcagcaggcagattttgcggctgatattctgcttctgcgccgtggacaactgtcccccaccgctggtaggttcggccttatccgactggctgataacaaacagcaccttatgccggtatacctctccaatcacctgatgataaaaatgttcatccaccgtcagcgcccggtcatcggccttaatcagccacagtaccaggtcgaggcgaggaagctgttcgcggtacagcgcagcatactcggtatcgcgagcgccactttcgcccacgccgggcagatccatcagcgttatatagcggtcgccgacttgcaggcgaaagcgcagtggctcacgtgtacaggccgccacatcgctgaccggtgatatatctccggcaaacagggcattgcacagactgctcttcccaacaccggttttacccataatgccgatcactggctcgtagttagttaactggttaatttgctgcagaagccgctctgatacccattgcggcagatcagcaagcgattgctgaaacgacttcaaaccttcagaattattcatcactactcctctgaaaaataataaaaaacggtagaatcgtgagattccgccgttaattgcgtatgttcagagtgatgatatatatctgaagattttttcaatcctctgcgcttgaggcagctgcgcgactgctggctcaggcaatgaatgagttataatagcagcatttactaacagggatttattgagagtatgagccgccgtgatacaccttaaaatctcaacccagcaaagtttcggagccgcgagcaaaagtgagagccttcacaaaataatgcttagtaataaagttactttgaattcagagccccgattaatgtgaacatgatcaacgaattttacccagattgagttcattcagtagccaggttttgaacacatcaagcgcagaatgcatgtgttggtgctgggggaaaaccaaataatgaccgatgtaatgtatttcgctggtactgtttacaagtgggcataccagtttaccgctagcgatttcacgttcagccagtagttttgattcaagcacaactcccaagccgtcaactgcggcagcaatcgccataaagctacggtcaaatcgaaggccataattattgggtggcgtcatcttattcgcctcaaaccatcctttccactggtacaactgcacatcgcactgaatcaatgtcaacgcatagagatcctctggtttctttagccgctcagccagttggggagaacacagtggcgtaagttcttcaacagcaagcgggatcttctcatagggtgatgggcggggttcaccgtagactatatcgagatcaaaatcatcctgttcaaaacgtgcatattctgtgctggctgaaagtcgcagatcgatgcttgggttctcacgtatgaacttaccaagacgtggtaaaagccattgatgggcaaaactcggtgcagtatgaaggcgcaaaggcctggattcatcagccgtcactaatgccaacccctgctgtaattcgttaaatccccgctgtatgtgctcaagcagtatttcaccttctttcgtcagcgtaatttctcgcgtactgcgctgaaaaaggcgtacatcaagcaagttttccagtttgcggatggcatggctgatcgcactgggtgacagttccaactcagaggcggccaacgcaaaagctccggtacgaccagccgcttcaaaggcgcgtaacagatttagaggtgcttttgctaagagcttcattcatgaatccttttcactagggatgaagtggtttactgaatttggccacctgaacagaggtgatatgctcacctcagaacaacacaggtgtcataatgaaaaaaagaaatttcagcgcagagtttaaacgcgaatccgctcaactggtcgttgaccagaactacaccgtggcagatgcagccagcgctatggatgtcggcctttccacaatgacgcgatgggtgaaacaattacgtgatgaacggcagggcaaaacaccaaaagcctcccccattaccccggaacaaattgaaatccgtgagctcaggaaaaagctacaacgtattgaaatggaaaatgaaatattaaaaaaggctactgtagattcaattggtcaacgcaacagttatgtgaaaacatggggttgcggaggttttttgaatgagacgaacatttacagcagaggaaaaagcctctgtttttgaactatggaagaacggaacaggcttcagtgaaatagcgaatatcctgggttcaaaacccggaacgatcttcactatgttaagggatactggcggcataaaaccccatgagcgtaagcgggctgtagctcacctgacactgtctgagcgcgaggagatacgagctggtttgtcagccaaaatgagcattcgtgcgatagctactgcgctgaatcgcagtccttcgacgatctcacgtgaagttcagcgtaatcggggcagacgctattacaaagctgttgatgctaataaccgagccaacagaatggcgaaaaggccaaaaccgtgcttactggatcaaaatttaccattgcgaaagcttgttctggaaaagctggagatgaaatggtctccagagcaaatatcaggatggttaaggcgaacaaaaccacgtcaaaaaacgctgcgaatatcacctgagacaatttataaaacgctgtactttcgtagccgtgaagcgctacaccacctgaatatacagcatctgcgacggtcgcatagccttcgccatggcaggcgtcatacccgcaaaggcgaaagaggtacgattaacatagtgaacggaacaccaattcacgaacgttcccgaaatatcgataacagacgctctctggggcattgggagggcgatttagtctcaggtacaaaaaactctcatatagccacacttgtagaccgaaaatcacgttatacgatcatcgttagactcaggggcaaagattctgtctcagtaaatcaggctcttaccgacaaattcctgagtttaccgtcagaactcagaaaatcactgacatgggacagaggaatggaactggccagacatctagaatttactgtcagcaccggcgttaaagtttacttctgcgatcctcagagtccttggcagcggggaacaaatgagaatacaaatgggctaattcggcagtactttcctaaaaagacatgtcttgcccaatatactcaacatgaactagatctggttgctgctcagctaaacaacagaccgagaaagacactgaagttcaaaacaccgaaagagataattgaaaggggtgttgcattgacagattgaatctacaaccgcgctcttgatgtcagactccctgaacagttctcgataatcgggaaactcagggcgcgttatcctgtggccactctctgccatgtgttcggggttcatcgcagcagctacaaatactggaaaaaccgtcctgaaaagccagacggcagacgggctgtattacgcagtcaggtacttgaactgcatggcatcagccacggctctgccggagcaagaagcatcgccacaatggcaacccagagaggataccagatggggcgctggcttgctggcagactcatgaaagagctggggctggtcagttgccagcagccgactcaccggtataagcgtggcggtcatgagcacgttgctatcccgaatcatcttgagcgacagttcgccgtaacggaaccaaatcaggtgtggtgcggtgatgtgacctatagtgtgcccggagttcagggcgggcatggatgcttaaatgaaccgcgagtctgtctggaatattgaaccggtaactcacgatgagaaacccaacaatcccaccgggtgtgacggtggagaacctgagcggcagtgacctgcggcatgcccgcagggtgatgtaacccgctgacaacggggattgaggcgagatcactaagccgagatgatcctcaaggttaagtactgaaaggttgaagaacatgaacccgttaatccgcctctgtgggttgaaaacgtcaccacggcctacgtgatctgacaggccgtgcaggaggaactggcagtgatacgtaagcactgccggtcgaaggtgttttgacatgtatgcgaaacaccggggcagcagcgtctatcacgcttgcgttgctgacttctgccaacttgcggcaagcaaggataaagagtgcgacgggcagcctcctcagtatgcctgagtccaggcaggtaaaccggggaaggtcagcgacggatgttaagggggcatggctccgatgacgcgctggctggcggagcttccgtagtagtccgcgatggggaaagcccattacatggcgaagggaagcagtttgaatgtgtttgcgacgtgaattaactgacctaacgaggtgaagacctttgataatcagcgaaatgcaacgcaagcttgccacatgggcagccaccgatccgtccctacggattcaacggctgctgcgtctgataacacaaccagaatggctggctgaagcggcgcggatcacgctttcatcaaagggggcccatacccccggcgttgatggcgtgaacaaaacaatgctacaggccagactggctgttgagctgcaaatcctcagggatgaattactctcaggccactaccagcccttgcccgccagacgggtttacatccctaaaagcaacggcaaactgcgaccactgggtatccccgcgttgcgggatcgtattgttcagcgggccatgctgatggcgatggagccgatatgggagagtgattttcatacgctctcatatggcttccggcctgagcgcagtgtccaccacgcgatccgcacggtgaaattacagctcacagactgtggtgaaacccggggacgctgggtgattgaaggcgacctgtccagttacttcgacaccgtacatcatcgactgctgatgaaggctgtacgccgcaggatcagtgacgcacgtttcatgactctgctgtggaaaaccatcaaggcgggacatatcgatgtcggtctctttcgggcggccagtgaaggtgtgccacagggcggtgttatatcgccgctattatcgaacatcatgctgaatgagttcgatcaatacctgcatgagcgctacctgagcgggaaagccagaaaagatcggtggtactggaataacagtatccaacggggccgaagtacggcggtcagagaaaactggcagtggaaacccgcggtggcgtactgccgctatgccgatgattttgtcctcatcgtcaaaggcaccaaagcacaggtggaagccatcagggaggagtgtcggggtgtgctcgaaggcagtctgaaactcaggctgaacatggataagactaaaatcccccatgttaatgacggctttatctttctggggcacaggctcattcgcaaacgcagtcgttatggcgagatgcgagtggtctcaacgatcccgcaggagaaagccagaaacttcgccgcatcgctgacagcactgttatggaaggtgcgaataagcggggaaattcttctcggctgactcagtcatttcatttcttcatgtttgagccgattttttctcccgtaaatgccttgaatcagcctatttagaccgtttcttcgccatttaaggcgttatccccagtttttagtgagatctctcccactgacgtatcatttggtccgcccgaaacaggttggccagcgtgaataacatcgccagttggttatcgtttttcagcaaccccttgtatctggctttcacgaagccgaactgtcgcttgatgatgcgaaatgggtgctccaccctggcccggatgctggctttcatgtattcgatgttgatggccgttttgttcttgcgtggatgctgtttcaaggttcttaccttgccggggcgctcggcgatcagccagtccacatccacctcggccagctcctcgcgctgtggcgccccttggtagccggcatcggctgagacaaattgctcctctccatgcagcagattacccagctgattgaggtcatgctcgttggccgcggtggtgaccaggctgtgggtcaggccactcttggcatcgacaccaatgtgggccttcatgccaaagtgccactgattgcctttcttggtctgatgcatctccggatcgcgttgctgctctttgttcttggtcgagctgggtgcctcaatgatggtggcatcgaccaaggtgccttgagtcatcatgacgcctgcttcggccagccagcgattgatggtcttgaacaattggcgggccagttgatgctgctccagcaggtggcggaaattcatgatggtggtgcggtccggcaaggcgctatccagggataaccgggcaaacagacgcatggaggcgatttcgtacagagcatcttccatcgcgccatcgctcaggttgtaccaatgctgcatgcagtgaatgcgtagcatggtttccagcggataaggtcgccggccattaccagccttggggtaaaacggctcgatgacttccaccatgttttgccatggcagaatctgctccatgcgggacaagaaaatctcttttctggtctgacggcgcttactgctgaattcactgtcggcgaaggtaagttgatgactcatgatgaaccctgttctatggctccagatgacaaacatgatctcatatcagggacttgttcgcaccttccggaggcgttatgagctggcggccctttttgtatctgattattaatccccacccgctattaagcgcccggcgcgggcatctgcgtctggtgcagggttgactttgcattctgttaacaaacgcggtataacaaaccttctttggatgtttagatgtccatacgtttagaaggttatatgcaaacaacacaacaaaatgcgccactgaagcgcacaatgaaaacgcgtcacctgattatgctttccttgggcggcgtgattggcacaggattattcttcaataccgggtacatcatttccaccactggagcggcgggaacgctgctggcctatctgattggtgcgctggtggtctggctggttatgcagtgtctgggcgagctgtcggtcgcgatgccggagaccggagcgtttcacgtttatgccgcgcgctatcttggtccggctaccgggtataccgtggcctggctttactggctgacctggaccgtggcgctgggttcgagctttaccgccgctggattctgtatgcagtactggtttccacaggtgccggtatgggtctggtgcgtggtgttctgcgcgattatttttggtctgaatgttatctccacgcgcttttttgccgaaggggagttctggttctcgctggtcaaagtggtcactatcatcgcctttatcatcctcggtggggcggcgattttcggctttattccgatgcaggatggctcgcccgcgccggggctgagtaatatcacggcagaaggctggttcccgcacggtggcttaccgattttgatgactatggtggcagtgaactttgctttttcgggtaccgagcttatcggcattgccgccggtgaaacggaaaacccgcgcaaagttatcccggtagcgattcgtactaccatcgcgcgactgattattttctttatcggcaccgtgtttgtgctggcagcgctgatcccgatgcagcaggtgggcgtggagaaaagcccgtttgtgctggtatttgagaaagtagggatcccgtacgccgctgatatttttaacttcgtgatcctgacggctattctttctgcagcgaactccgggttatatgcctccgggcgcatgctgtggtcgttgtcgaatgaacgtacgctaccggcctgttttgcgcgagtaacgaaaaacggcgtgccactgacggcgctgtcggtcagtatgctcggtggtgtgctggcgctgttttccagcgtggtggccccggacacggtatttgttgcgctgtcggcaatctccgggtttgcggtggtagcggtgtggctgagtatctgcgcctcgcattttgtttttcgtcgccgtcatctgcaacaaggtaaggcattgagtgaattacattatcgcgcgccgtggtatccgctggtgccagtattaggttttgtgctgtgcctggtggcctgtgttgggctggcattcgatccagcgcagagaattgcgttgtggtgcgggttaccgtttgttgcgttgtgctatggtgcttatttccttactcaaccccgaaacgcaaaacaggagccagaacatgtcgcagaataatccgttacgcgctcttcttgataaacaggatatcctgctgctggatggcgcgatggcgacggagctggaagcgcgagggtgtaacttagccgacagcctgtggtcagccaaagtgctggtagaaaacccggagcttatccgcgaagtgcatcttgattactaccgggcgggggcgcaatgcgcgatcactgccagctatcaggcgacgccggcgggcttcgccgcgcgaggtctggatgaagcgcagtcgaaagcgctgattggcaaaagcgtggagctggcgcgtaaagcccgtgaagcgtatctggcagagaacccgcaggcgggaacgcttctggtggcgggatccgtcgggccttacggcgcgtatctggcggatggctctgaataccgtggcgattatcattgtagcgttgaggcatttcaggcgtttcatcgcccgcgcgtggaagccttgctggatgccggggccgatctgctggcctgcgaaaccctgccgaatttttccgagattgaggcgttggccgagctgttgaccgcatatccgcgtgcgcgggcgtggttctcatttaccctgcgcgacagcgaacacctgagcgacggtacgccgctgcgtgacgtggttgcgttgctggcgggttatccgcaggtggtggcgctaggcattaactgtattgcgctggaaaacaccaccgctgcgttgcagcatttacacggtttaacggtgctgccgctggtggtgtatccgaactcgggcgagcattacgatgccgtgagcaaaacctggcatcatcacggtgaacattgcgcgcagctggcggattatctgccgcagtggcaggccgctggcgcacggttgattggcgggtgctgtcgcaccacgcctgcggatatcgccgcgttaaaagcgcgaagctgagggtttatcgggtctacatcgttcattgtaggcctgataagcgcagcgcatcaggcattgccggatggcggcacaagcgccttatccggcctacaaaaccacaaaacgttatgccgcatccgccagaacaaacatgccgtacggatggatttcaagataatactgctcgccgacgtccggttgcagacgcgtagcgttgacctgcaataatatctcctgcccgtgccattccaccgtcacttcatactgcggccccatataggcgacatggcggatcacgcagcgctggctctcttcgccgcgatcgctgagcgtgatcgcttccgggcgcacaccgaccatcccttcaccctgtgtaccaaagtgcagcgggcgcggcagatgatagccgtagatatcaacgtatccgtcgctgaaggttgccgggaacaggttggcatcgcccataaagctcgccataaagcgggaggcgggctggcggtaaagatcctgcggtgagccgatctgcatgatgtgtcccttgttcatcaccagcacagtatcagaaaccgcaaaggcttcgctctgatcgtgggtgacgtacagcgaggtgatatcaaactgcttttgcaactcgcggatcttgtcgcgcatgctgcgacgcaggttggcgtcgaggttactcaacggctcatcaaacagcagcactttcggcttgaggatcagcgcgcgggccagcgccacgcgctgctgctgcccgccggagatctgatcgacaaagcggtcttcgaatccttccagatccaccatcgccaacgcctctttgacgcgggctttcagctctgcgcgcggtacgccgagcattttcaggccataaccgacattctctcccagcgacatatgcgggaacagggcataggactgaaacaccatacagatatcgcgctgctgaatagagcgatgggtgacgtcttcgccatcaatgaaaatttgcccttcgctcggtttttccagcccggcaaccaggcgcaaaatagtggttttgccgcagccggacgggccgagcagcgtcaccatttgcccctgcgggatggtgaggttgatattgtcgattaccgtattactgccaaatcgtttagtgacgttgcgcagttcaacgaaatttttctgagtcatagtgcgctccattacgcctggtttttggcttttgaacgggaggtacgtgattcaccgatcagccagtcaaagatgaaaataatcgccagcatcaccacgatcagaatggaaccgtaggcaatcgctacaccgtattcgccatcttccacgcggttgaggatgtaagccgtcgctacgcgggtatccggcgtgacgaggaacacaatggcgctgacggtggtaatggcgcgcacaaagctgtaaatcagcgccgagaggatcgccgggcgcagcagcggcagcaggatgtgcgtaatggtacgcagggaaccggcgcgcaggctgagtgaggcttcatcgagcgatttatcgatttggcccggtaatgactccaacttattgatagtgttttatgttcagataatgcccgatgactttgtcatgctgctccaccgattttgagaacgacagcgacttccgtcccagccgtgccaggtgctgcctcagattcaggttatgccgctcaattcgctgcgtatatcgcttgctgattacgtgcagctttcccttcaggcgggattcatacagcggccagccatccgtcatccatatcaccacgtcaaagggtgacagcaggctcataagacgccccagcgtcgccatagtgcgttcaccgaatacgtgcgcaacaaccgtcttccggagcctgtcatacgcgtaaaacagccagcgctggcgcgatttagccccgacgtatccccactgttcgtccatttccgcgcagacgatgacgtcactgcccggctgtatgcgcgaggttaccgactgcggcctgagttttttaaatggcggaaaatcgtgttgaggccaacgcccataatgcgggcggttgcccggcatccaacgccattcatggccatatcaatgattttctggtgcgtaccgggttgagaagcggtgtaagtgaactgcagttgccatgttttacggcagtgagagcagagatagcgctgatgtccggcagtgcttttgccgttacgcaccaccccgtcagtagctgaacaggagggacagctgatagaaacagaagccactggagcacctcaaaaacaccatcatacactaaatcagtaagttggcagcatcaccgagaacacaaatgggctaattcggcagtactttcctaaaaagacatgtcttgcccaatatactcaacatgaactagatctggttgctgctcagctaaacaacagaccgagaaagacactgaagttcaaaacaccgaaagagataattgaaaggggtgttgcattgacagattgaatctacagcagctttttttaatatgtcccgttcgtcggtaacccgtttcagctctttctggagacggcggatctcggcctgagcatctgactgttctttattagtggaagaatccggaccgtacttctttatccaggcataaaggctgtgggtggtgatatcgagacgtgttgcaacgctggcaacagaataaccgagatcaacaacctgtttgactgcttcagttttaaactcttcgggataacgcttaccgctcatgggcacctctctttaagccattttaaatgactcggaggtgtctgttaaacccgtggcgattcaaaattgcgatatatacatacccatgactgcccagcgtatcggcttcaccagtcagcccgttacggtacagtgtgacacagtgcgcgtacctgggattcagctcacaggagagcagcatcagctccagatgtgcgacaaaatgcgggaaggcttcatccagttgtagagtctgcacctcactgaatgagccggtgaatccagcccggtcagccagaaaatgcagacgatgaccttcctgcaccagtcgtgctccgaaacacggtgtgatatctcgtttaagcccccaagtttgagtagagtctttattcataattttattcctgttaaagaagaccatgttcggcgaatgagaatatttgcctgccgccgacaatcaggtggtcggggacatggtgaacactttttaacatcctttacccatggtgatcgactttttcttcaggtcgatcacccccactttcgtgctgtaccaccacacctcgtagctgccgtcttcctgcatctccttcagcccgacccgttctcccctgaacgccttgcctgcgctcagacttacccctttcacgctcagctttccgctgatatccactttcctgaccatcaccccttcatcgtattccgggggcgttgtgttgccgctgtactgccgcgctgacggctgataccgcgagcccggtaccgccatatccagcgcctcgtgcgggcgttcaaggttatagaccgtccgccagtggtcgaaggcgcgctgcagttcaccgctgtctgcgaaccattttccctgcagcacttccgccttcaggctgcggtgaaaacgctccagcttcccctgcgtctgcggatgataaggccgggagtgccccacccggatacccaggcgcatcagccacagctccagcgccgtccaggtgccggtggtgtcgccccacggtgagccgttatccatggtcatccggtccggcaggccgtaacgctcaaacacgctgaccagctgctgctgcacggtctcgcgccgttcatcggtacagtgcgccaggcacagggaaaaacgggagtggtcgtccagcagggtgagcggatggcagcgtccaccgccaaaaggaaagtggcccttaaaatccatctgccagaggcggttcggcgcgtcgtgttcgaaccggcccgtggcgggaatgcccggtgaagcgcccggcagcaggccatggcgggccatcaggttatggacggtgctgaaggcgggcatggtgtgcccctggtcctcgagccagcgcttaatcttgcgggctccccagcgttcatgacggtcatgggccatacgcagcagggccgtgatgtcgtcagatgagcggttcggggaatggtgcggaatgcgcgggcggtcctgaagaccggcggcaccttcctgagcccagcgctggagccacttgtagccggtggcaggtgaaatgccgaagcgacggcagagggaacggatgttcgccccgtcctgcgaggcgaacaaaacaaactcagtacgtaatgacatggtatctctcgcatcccagggcataagcgactccataaacgggttcttatgccttagttgtaagtgtctaccatgtccccgaacaagtgttcactatgtccccggaccgtacaccccaaaggggagaggggactgcaccgagccatcttttccccctcgcccctttggggagagggccggggtgaggggcaatatgtgatccagcttaaatttcccgcactccctcttcccttccgatttacctctccttgttctgcgtcatagtatgatcgttaaataaacgaacgctgttctataatgtagaacaaaatgattcagcaaggagatctcatgccgcagtccgcgttgttcacgggaatcattccccctgtctccaccatttttaccgccgacggccagctcgataagccgggcaccgccgcgctgatcgacgatctgatcaaagcaggcgttgacggcctgttcttcctgggcagcggtggcgagttctcccagctcggcgccgaagagcgtaaagccattgcccgctttgctatcgatcatgtcgatcgtcgcgtgccggtgctgatcggcaccggcggcaccaacgcccgggaaaccatcgaactcagccagcacgcgcagcaggcgggcgcggacggcatcgtggtgatcaacccctactactggaaagtgtcggaagcgaacctgatccgctatttcgagcaggtggccgacagcgtcacgctgccggtgatgctctataacttcccggcgctgaccgggcaggatctgactccggcgctggtgaaaaccctcgccgactcgcgcagcaatattatcggcatcaaagacaccatcgactccgtcgcccacctgcgcagcatgatccataccgtcaaaggtgcccatccgcacttcaccgtgctctgcggctacgacgatcatctgttcaataccctgctgctcggcggcgacggggcgatatcggcgagcggcaactttgccccgcaggtgtcggtgaatcttctgaaagcctggcgcgacggggacgtggcgaaagcggccgggtatcatcagaccttgctgcaaattccgcagatgtatcagctggatacgccgtttgtgaacgtgattaaagaggcgatcgtgctctgcggtcgtcctgtctccacgcacgtgctgccgcccgcctcgccgctggacgagccgcgcaaggcgcagctgaaaaccctgctgcaacagctcaagctttgctgagccggacgataacgatgaccattgagaaaattttcaccccgcaggacgacgcgttttatgcggtgatcacccacgcggcggggccgcagggcgctctgccgctgaccccgcagatgctgatggaatctcccagcggcaacctgttcggcatgacgcagaacgccgggatgggctgggacgccaacaagctcaccggcaaagaggtgctgattatcggcactcagggcggcatccgcgccggagacggacgcccaatcgcgctgggctaccacaccgggcattgggagatcggcatgcagatgcaggcggcggcgaaggagatcacccgcaatggcgggatcccgttcgcggccttcgtcagcgatccgtgcgacgggcgctcgcagggcacgcacggtatgttcgattccctgccgtaccgcaacgacgcggcgatcgtgtttcgccgcctgatccgctccctgccgacgcggcgggcggtgatcggcgtagcgacctgcgataaagggctgcccgccaccatgattgcgctggccgcgatgcacgacctgccgactattctggtgccgggcggggcgacgctgccgccgaccgtcggggaagacgcgggcaaggtgcagaccatcggcgcgcgtttcgccaaccacgaactctccctgcaggaggccgccgaactgggctgtcgcgcctgcgcctcgccgggcggcgggtgtcagttcctcggcacggcgggcacctcgcaggtggtcgcggaggcgctgggtctggcgctgccgcactccgcgctggcgccgtccgggcaggcggtgtggctggagatcgcccgccagtcggcgcgcgcggtcagcgagctggatagccgcggcatcaccacgcgggatatcctctccgataaagccatcgaaaacgcgatggtgatccacgcggcgttcggcggctccaccaatttactgctgcacattccggccatcgcccacgcggcgggctgcacgatcccggacgttgagcactggacgcgcatcaaccgtaaagtgccgcgtctggtgagcgtgctgcccaacggcccggactatcacccgaccgtgcgcgccttcctcgcgggcggcgtgccggaggtgatgctccacctgcgcgacctcggcctgctgcatctggacgccatgaccgtgaccggccagacggtgggcgagaaccttgaatggtggcaggcgtccgagcgccgggcgcgcttccgccagtgcctgcgcgagcaggacggcgtagagccggatgacgtgatcctgccgccggagaaggcaaaagcgaaagggctgacctcgacggtctgcttcccgacgggcaacatcgctccggaaggttcggtgatcaaggccacggcgatcgacccgtcggtggtgggcgaagatggcgtataccaccacaccggccgggtgcgggtgtttgtctcggaagcgcaggcgatcaaggcgatcaagcgggaagagattgtgcagggcgatatcatggtggtgatcggcggcgggccgtccggcaccggcatggaagagacctaccagctcacctccgcgctaaagcatatctcgtggggcaagacggtgtcgctcatcaccgatgcgcgcttctcgggcgtgtcgacgggcgcctgcttcggccacgtgtcgccggaggcgctggcgggcgggccgattggcaagctgcgcgataacgacatcatcgagattgccgtggatcgtctgacgttaactggcagcgtgaacttcatcggcaccgcggacaacccgctgacgccggaagagggcgcgcgcgagctggcgcggcggcagacgcacccggacctgcacgcccacgactttttgccggacgacacccggctgtgggcggcactgcagtcggtgagcggcggcacctggaaaggctgtatttatgacaccgataaaattatcgaggtaattaacgccggtaaaaaagcgctcggaatttaattattttaagagataaaaccgtctgcggaatatttcccgcagacggctttgttgtttttgaaatttattaatttaaacaattagttgagatatatcgttggcgtcacaaaagcaaaataacgtaattcggaaataagatatgaccattgctggttaattgaatagctcattacactccattaacacgatgttgtaattcggcacactacataagggtgtaattctgatgacgcaattaaccatgaaagacaaaattggctacgggctgggagacaccgcctgcggcttcgtctggcaggccacgatgttcctgctggcctatttctacaccgacgtcttcggcctgtcggcggggattatgggcacgctgtttttggtctcccgcgtgctcgacgccgtcaccgacccgctgatggggctgctggtagaccgcacccgcacgcggcacggccagttccgcccgttcctgctgtggggggccatcccgttcggcatcgtctgcgtgctgaccttctacacgccggacttctccgcacagggcaagatcatctacgcctgcgtgacctacattctcctgaccctggtctacaccttcgttaacgtgccgtactgcgccatgccgggcgtcatcaccgccgacccgaaagagcgtcacgccctgcagtcctggcgcttcttcctggcggcggcgggctcgctcgctatcagcggcatcgcgctgccgctggtgagcatcatcggcaaaggggacgagcaggtgggctacttcggcgccatgtgcgtgctggggctgagcggcgtggtgctgctctacgtctgcttcttcacgaccaaagagcgctacacctttgaggtgcagccgggctcgtcggtggcgaaagaccttaagctgctgctgggcaacagccagtggcgcatcatgtgcgcgttcaagatgatggcgacctgctccaacgtggtgcgcggcggggcgacgctctacttcgtgaaatacgtgatggatcacccggagttggcgacccagtttttactttacggcagcctcgccaccatgttcggctcgctttgctcctcacgcctgctgggccgcttcgaccgcgtcaccgccttcaagtggatcatcgtcgcctactcgctgatcagcctgctgattttcgtcaccccggcggagcacatcgcgctcatttttgccctcaacatcctgttcctgttcgtctttaataccaccacgccgctgcagtggctgatggcttctgacgtggtggactacgaggagagccgcagcggtcgccgcctcgacgggctggtgttctccacctacctgttcagcctgaagattggcctggcgattggcggggcggtggtgggctggatcctggcgtacgtcaactattccgccagcagcagcgtgcagccggttgaggtgctcaccaccatcaaaattctgttctgcgtggtgccggtggtgctctacgcgggcatgttcatcatgctgtcgctctacaagctcaccgatgcccgcgtggaggccatcagccggcagctgattaagcaccgcgcggcgcagggcgaggccgttcccgacgccgcgacagccgcatcccattaaccggaggcaatatggaaatcactaacccgatactcaccggcttcaacccggacccgtccctgtgccgccagggcgaggactactacatcgccacctcgaccttcgagtggttcccgggcgtgcgcatctaccactcccgtgacctgaaaaactggtcgctggtcagcaccccgttggaccgcgtgtcgatgctggacatgaagggcaacccggactccggcggcatctgggcgccgtgcctgagctacgccgacggtaaattctggctgctctacaccgacgtgaagattgtcgactcgccgtggaaaaacggccgcaacttcctcgtcaccgcgccctccatcgaggggccatggagcgagccaatcccgatgggcaacggcgggtttgacccgtccctgttccacgacgacgatggccgcaaatactatatctaccgcccgtgggggccgcgccaccacagcaacccgcacaacaccatcgtgttacaggcgtttgacccgcagaccggcacgctctcgcccgagcgcaaaacgctgtttaccggcacgccgctctgctacaccgaaggcgcgcacctgtatcgccacgcgggatggtactacctgatggccgccgagggcggcaccagctacgagcacgccgtcgtggtgctgcgttccaaaaatatcgacgggccgtacgagctgcacccggacgtaacgatgatgaccagctggcacctgccggagaacccgctgcagaagagcggccacggctcgctgctgcagacgcatacgggtgaatggtacatggcctacctcaccagccgcccgctgcgcctgcccggcgtgccgctgctggcctccggcggacgcggctactgcccgctggggcgcgagaccggcatcgcccgcattgaatggcgcgacggctggccgtacgtggaaggcggcaagcacgcgcagctgaccgtgaaaggcccgcaagtagccgagcagcctgcagccgttccgggcaactggcgggacgatttcgacgccagttcgcttgacccggagctgcagaccctgcgcattccgttcgacgacaccctcggctcgctcaccgcgcgcccgggcttcttacggctctatggcaacgactcgctcaattcgaccttcacccaatcgaccgtggcgcgccgctggcagcacttcgccttccgggcagaaacgcggatggagttctcgccggtgcacttccagcagagcgcggggctgacctgctactacaacagcaaaaactggagctactgctttgtggactacgaggagggacagggtagaaccatcaaagttatccagctcgaccacaacgtgccgtcgtggccgctgcacgagcagcccattccggtgccggaacatgcggagagcgtctggctgcgggtggacgtggatacgctggtctaccgctacagctactcgtttgatggcgagacgtggcacaccgtgccggtgacgtatgaggcgtggaagctgtcggacgactacatcggcgggcgcggcttcttcaccggcgcgtttgtgggcctgcactgcgaggacatcagcggcgacggctgctacgcggacttcgactacttcacctacgagccggtctaacggctcaggccgggtagcccagcgcgcgcgagagcgcgagcccggcctgctgaagctgctcgcggaaattagccagctccgcgtcgtccacgcgggaggtcagcgtcgacaggctcagggcggcgatgacgcgggactcgtggttccacaccggcaccgccacgcagcgcacgccctgctcgttctcttcgctgtccagggcgtagccttgctcgcgggtctgcgccagggcgctcattaaggcttcgcgagacgcgagggtggcgggcgtaaaggtagtgtactgatagccctccagcagggcgttcagctcggcctcgcccagccaggcaatcaacaccttgccgatggcggtggcgtgcaccggcaggcggcggccgatgcgtgaataggcgatggcggccagcttgccttcaatcttctcgatatagaccccttcacgcccgtccaggatccccagatgggtggtctgcccggtccgccgggacagctccgtcagccagccttttgccttctgccgaatatcgatggagcccacgacaaaatggccgcgctcgaccagcttcatgccgaggcgatacttgccgttctccgggttctgatcgatatagccgtgaagctgcagggtttttagcagcgagtggagggtactcttgctcagccccatcagtttgctgatgtcggtgatcttaagctcggtggcctgctcgttgaacaggtcgaggatctgcaacgcacgttcaacagactgaataatcggcataatgctggcatgtccacgctggaattaaggcgaaaacgtacctttttcgggatgaaaaatcaatgaaatggagccggtgttctccctctccctgtgggagagggccggggtgagggcaccaacgcgcagcggacccaatcactccccaagcgttgccatcatcaccgccttaatcgtatgcatccggttttccgcctggtcgaacacgatgctcgccgccgactcaaacacctcgtccgtcacctccatcccgccgtgcagatcgaactccttcgccatctgcttgccgagcgtagtctggtcgtcatggaacgccggcagacagtgcaggaacttcacgttcgggttgtcggtcagcgccatcatctgcgcgttcacctgatacccgcgcagcagcgcaatccgctctgcccacttctctttggcctcgcccatcgacacccacacgtcggtatagataaagtccgcgcccttaacgcctgccgccacgtcttccgtcagagtaattttcccgccgtgcttctccgccagcgcgctgcactccgccaccaggctctcttccggccagcaggctttcggggccaacaggcgcagatccagcccggtcagcgccgccgcttccagcatcgagttgcccatgttgttgcgcgcatcgcccgcgtagaccagcgtcatctcgttaaacgccttgcccggcaggtgctcctgcatggtcatcaggtccgccagcagctgggtcgggtggaactcgttggtcagcccgttccacaccggcacgcccgcatactgcgccagcgtttcgaccacttcctggccgtgaccgcgatactgaatgccgtcatacatccgcccgagaacccgcgcggtgtccttaattgactctttatgcccaatctggctgccgctcggccctaaataggtaacgcgcgcgccctggtcaaatgcggcaacttcgaaagagcaacgggtacgagtcgagtctttttcgaagatgagcgcgatgtttttaccggtaagcttctgtacttccttgccattttttttatcggctttgagctgtgcggcaagggtcagcagagaagtgaactgtgcaggggtaaagtcgagcagtttcagaaagtgttttttgtataaatcggacattttatcctcgcatggcgaacgccacttattgaattaaaattcactttatatgtgtaattattcatttgcaaccccatttcacaattctttcttacaaaggtggaggcaaacccgtccgtgtgtgaaaataatcgtatctgcctccgattctctgcagaagcagaaagacattggatcgaattctacaaccaggtcgagtcagaaatgagaatgattggccttctttatgattttaaggattatgcttctaaaatggcggagaacatggcgaggcttgctgccttacttcattacttcagcggtgatggaggcgatatatctgttaccgggtaatgactccaacttattgatagtgttttatgttcagataatgcccgatgactttgtcatgctgctccaccgattttgagaacgacagcgacttccgtcccagccgtgccaggtgctgcctcagattcaggttatgccgctcaattcgctgcgtatatcgcttgctgattacgtgcagctttcccttcaggcgggattcatacagcggccagccatccgtcatccatatcaccacgtcaaagggtgacagcaggctcataagacgccccagcgtcgccatagtgcgttcaccgaatacgtgcgcaacaaccgtcttccggagcctgtcatacgcgtaaaacagccagcgctggcgcgatttagccccgacgtatccccactgttcgtccatttccgcgcagacgatgacgtcactgcccggctgtatgcgcgaggttaccgactgcggcctgagttttttaaatggcggaaaatcgtgttgaggccaacgcccataatgcgggcggttgcccggcatccaacgccattcatggccatatcaatgattttctggtgcgtaccgggttgagaagcggtgtaagtgaactgcagttgccatgttttacggcagtgagagcagagatagcgctgatgtccggcagtgcttttgccgttacgcaccaccccgtcagtagctgaacaggagggacagctgatagaaacagaagccactggagcacctcaaaaacaccatcatacactaaatcagtaagttggcagcatcaccgaattttcagcccggatgtttcacgtacctatgtcgaatatctggccgataaggttgcggatcgagaagaggatgcagaggaatatctggaagcaatcatggaggctcgtgttaccgttgctggcatggggctggtgatggaggtgcaggattacttcgatggcgaggccgatagactggcgaaggcgtggctggccgagtacacaccgcaaatcaagtcgttgaaagatgagcgtaaagaggcctatcgtcaaatcgtcgaaatgagtaccgaaccgcaggatgtggatctggtcaggccggcgaacaagtttgaaatgaccagggtgcgtgaaggtgaaaaggaagctgaccttccagtctggaaacaccatttgttgtgtgacgaaagcgggaactatccggctctgttgaaccattgggaaaccaaggtttttgagatcgaaaccaaacgtgaaggatttgctttctggtatcgtaatccacagtacacagggcagtcgtcactgggaatcgcttatgttgaagctgaacagtacaagattgttcgtcccgatttcctgttctttgccgaacaggatggcaaaatggttgtggacctggtagatccacatagcctacatctggctgatgctttgcccaaactggaaggacttgcgctatatgccgaacatcattctgatgcttacaggcgaatcgaatctgtcgccgaagtaaagggtaaattacgagtgttagatttgaaacggcaggatgtgcaggatgctgttgctaccgctgaaaatgcagaaacgttatttagtagcggacttgctgatgactatcagtaatctatagaaaattgcgtaacgaaactgcattttagtaattttttgaaacaatacaaataaggccttctcactgagaaggccattaccgacttacagttcgatttggctacagccgaagttacggtctccttcaccaaacactttgctttcaactttggtcaggtagtccagtcgggttaacagcgcctggtagttctgctggaagtcagtactattggtgtctagcacatacttacagttttcaggaaaatggaccagaccagggtgatcgtctctctccagtctcagggcgctgtaccaggctcctgtgatcatccctctaaggttatcgtcctgatcgtaatccccgaggtggtagtaagcgtctttgttgaacaacaggcaaatgtgatagtggcatttacctgattcagaatactctttcgcccatataataaataaagggcaacggtaaatgcgtttatcctcacgcaccttacgggtacggtcagcctccagcttagctctgagggattcacgcatccgggatatcaccccaggttccaggttagggaagcaacagatattgtcaccgttatcaactattttgggatagtggagatcgacacgtacagcaattaacctaggataccggttagtcaaataacataataatttattaatcttactctgatattcgaggatatgtactccatgagtaccttgatatgttttcataatatatacctgtatttggtcctacggtctatagcagaccgtacagggatgccatacaggcagggctattcctggtcactgttgtcggtatatactggtatcagattttagtacggacatactgatctgattactactcttactggtgaatacaggtagtaagagtacacaatgccattatataatacctatccaacatctaaatttgagacgaaggtagccccagcctgtgatggctgttaaaaagttactctgcaattagcttctggaattaaccgatgattccgttattccagtgccgcttcacagtcgataaactgatactcaatttctttgcaatctcagcctgagtaaatccacctttcttaagtattgtgatatcacgtcggtatttgcttccctcctttcgtcctaattttttcttaacatgtcgatatcggcttttagttgatttcagattgtgaatgtcaatcgtatcctgacgagcaatcaaaaaagacaagcaactttcagcagaaggctctatccttgaagctggatggtagctgtagataaacatttctttttgaaggcaaaaaaataaaatattctgtaagtcctccacagttctgccaagacagcttagatctggaatgacaagcgtgtcctgccggttcatttcatgatgaatcaattgtctgagtaaacgttgctctgaaacaacctctttaatatctacctgctcgatcacaacatgttcaggtagaatattaaatttttggcatatctcagcaagtgagtgatgatctgtaatgctttcttgctgttcgctactgcatatggtgtaaaaaaatgaacgcatctgatgcactccggtgtcataaattattttttgatacctgaataatgtcattttgcataaaaaacaaccaaaaatagagagtgattgccagcgatactttaactggtaaagtagtattttacctctcataattgtttgtccttctttgttacctcttaggttctgctctcttgtgagtatgggtttataatgatgtcatccggtacattaacacggttggaaacatctgttttgcggagcactggcagcataaccaccatttcattgacatggtaaatatcaatccaacaaacaaccggataaggcataacaatcccctttcttctaagaacttcatttatcccgaatataatcaattgggatgttgacaagagtagagcctgcccggcatcaaagtaataaccctcaaaggttgttctatgaataagaataatgtttgaatatcctgagacactttgatgctttacatcaaaatgtctttgattgtaaatgtaaatggctttttccatatcgtaattttcccttagcgaggatagcctttcacgtataactgttttttcatctttccccatgaattcatcattagcgttcagttgaaagtaatctgcaatggggatttttaatggactcatgatgttcgttttccagattaacgaacagtactcttccagagttacttctgttttacctcggcttcgattgatgctttcttttatagagaactttaacaggtcattttttatttcatttattgaccagttatgacgattgcatttttctaatatagggatagccaaatccacaacttccgctattacggaagagtgagatttatttgttagtctggcataatgatcaattactcctaatgaagattgatttttgaacgtgactgagtgtttttttatgggagtagtctgtactacctgtgactcattgtttttgccttgacaaggtttttttcctggtagaacgctgctcatctcaaaattagtaacactattagacatttttaaggaaacctctttgttatctcaatataaaactactatctgaaatttctcagtgttgccccatttttctcggggcaacatcgctataaatcaataaaattaaatctgtaatttattacagactttctcgtacagaaaatgtatctataaaatcgaggacatctttacgtaaccagtaatggcggccattgatttgttttgggcgaggtagcccctcaggcaatttgtcctgacaaagccatttacgaatggtttgagatttgtagctaatgattttagctaactcagctgttgaaatgagctgtgattgagatgtatccgggagtttgaatgcgctcattttgccacctcagtgattgagatattggcaaagaaagctttaagcattattgaattagtaggggtagtaatgaaggcagaaggaaacgtttcgggctcggggtcggggtcactaccatcacctgaatctgatgataaggcacttttagctgatttagccgtactgtgatgcgatctggatgcctgatttttacatgacatcagacgcgcgagaaagttagtagcattttgcattctttgtttaagatgtaaaattttcagtttggcgcatgcgacagacttgcgaagagctgagtatgttcctttgagatactcgacaacctcttccatggacgcaggatcgttaaaggattgagttgttttacttgaattaatacaccagcgagctctgatagctgccagagtgggttctatggatacagttgctggggttgccattggcttatctcctgtgtagttgctgtatcattgactaaactgtgtattacgatacatgaaaatctatcttgatcaatagttgatgatattttgtaatatgttgatttttaatggaatcaacgcatatcaacgttgttttttatggtaatacctgcttcatttaagatccatgtctcaattttctcgtgccattttcgtaacagatctaacggacgacggcgatagtgtttttcggcaagagcgctgggtttgtgtcccataatttgagcaacaataccagtgggaacttcaacccactcggccaaagtaccaaaactacgacgtaaaccgtgaaggctgatatgtggtaactcagccagcactaatgctctgttgtgcgctgaacgcggctcaataattttgccacttttactgttacttctgaaaacccaaccctccttatttacgtcagaatttggggattgcgctagtacatttaacaattcagaaacataaggagtgagagggatgatacgttcaccttcgatcttgtctttaattcgcatgcttgaccatttgaaatctacgtctgaccagcgaagcgacgcaatttcttcacgccgagcaccagtgagcaaaagtacttggagataggccgatgcaataggattattgaggctacgcacggcactaaaccagctttttagttgttccttttgcaggcaatcatcagctttactcgctgacacgggaaccatttttcttacgttgtaatcttgtgccagatcgccaggaatgatcccttgatattttttctgataattactccatttgatgaaagcacgtagtaggcgataagcgtgagcagtgacggtaggtctattttgcctttctgtactcagccacgctgctatgtaatctggggttagttccgataacggcaggttgagcaaactagccaatggtccagccgaagtcgggccttggcctctttttttactttcgcctccacgactggacaagttaatgtgatcggcaatgtatcgagtagaatatgggcgtttagtttttgcactgataccggttctcaattcttgaagatagtcttcccaggcgacggagaaagtcacttttgttttacgtgattctgcctgcagggattctgcttctgcgatttttacagccttagcaattcgtggatctatccctgtatcgatcaatgtttgtaaccgtcttgcctcggctctcgcatcatcaatcttccagtcgttaatgttgccaatagtcatgcgaagggttttccccgcatatacgctttggaatacaaaggcttttgctccgctagttgctcggcatgccagggttgttacatctgcatcccaaagaaaagtttgttttttcccttccggtaaggtgaatctgcgaagtctttcgaaggtaaatttttgtcttgaaagcgccatttttcggctccagttgagaattgctgtcttacaataatgtaactgctggtgtaagtaaatggagggaataaacatcaacttttgttaatttcaatcaacgggtttattgctataacttggtgttttataatataaagtatgttgttttgattgattgctcaagtagttaaaaatgcattaacatcgcattcgtaatgcgaaggtcgtaggttcgactcctattatcggcaccattaaaatcaaagagttaccccatatttaaatacaccacgtttcctcctgtgccgtatttgtgccattgtaaccttggcaattcatcaaaatactgttctgacatcaggcagtgcaggtgcagacatttaagccaattgctgccgccattctttgacgtagtcaatcagggcgcggagctttggtgcaatattgcgacgctgtgggaaatacagatagaagcccggaaattgtggaagaaagtcatcaagcagcgatacaagcttaccgctttcaatatatggcctgaaagtttcctgagtggcaattgttattcctccgccggcaagagccagcctcaacatcagacgcagatcattagtcgtaatctgcggttcaatcgcaaggtcgaaagttctcccgttttcttcaaatggccagcgataaggcgcaacctccggggactgacgccagccgatacacttatgggtatttcccccggaggcgagaaagcactctccacgcccggccgcaaggatcaggacgacgggggcaggcatgaatcctcctcctgatggagacgtacagaggcgacttctgccagcacggagagtgccagagtatgcgcatcccgggctttggggaatatcccgacgggtgcccggatttgcgttgtttcctccctggaccatcccagctcgtggagcttttgcagacgtaacgtgtgggttcgatagctgcccaatgcgccgagataaaagggttttgcttctcgcgcggcctgcaacactggcagctcccggttgagatcatggcacagcaaaatgaccgccgtatcggtatcgatctgagcgctggctgaggccggaaaaagatcgaagatatggctgtcatagcctgtggctgctgcaagactcgcggttgcctgcgcctcaagagaacgtccgtaaatcatcagcctgacgcatggcctgaaccccacctcaaagccattgagattccagcccgtccgggtttgcgtgggcaggcacaccagcgattgtgcttgcggatcgtagcgcagccccaccggttttctctgttccaggcggttcagcacggcgagcagaggctgtgccgagcgtagtttatggagcgtcagcgtgatcccaccgccgcagggcagaacgatgtcaaaccacggcgaaccttcgccatagcgaatttcgcgatcgcggcctgagcccatcatctccagcgcttcaaaagcggcagcggcctccacgcagccgccagagacaaaaccgcagtaacgaccatcttcgcgcaccaccatctgcgccccgagcgggcgcgccgcgccgccgcgtatctccaccagcgtcaccagcaccgctcctttaccggacattagcgcctctacggcgaagcgcagaatggtccggtggtcatcggtgagaaacgcctgctctggcttatgccagtgttcgtctttgtcaaaaagcgggtatgacattgttcctccttaaaccacatccggcagcttatcgagcagcttatccagagtgatgggataatcccgtacccgaataccggtggcgttatacaccgcgttggcgatagccgcgctcacgccgcacaggcccagctcaccgacacctttggccttcatcggggaggatatggggtcggtatcatccaggaaaatcacctcctgttttgggatatccgcatgaaccggcacctcataccccgccatatcgtgattaacgaagtagcccaaacggtcatccaccgccagctcctccatcagtgccgcgcccatgcccatagtcattgcgccaatgacctggctgcgcgcagttttcggattcaggatgcgtcctgcagcacacacagcgagcatacgccggacccgaacttctcccgtcgcgctatgcacgccgacctccacaaaatgcccggcaaaggtcgactgctggtactctttgctcagtgttccgaattcaatgctctcttccgctgtcagtctgccgcctgcggtggcttcatgtagcgtggcgcttcgggtaccgttggtaatcttgccgtcggcaaactgcgactgctcaggatcaaacccgactgccgaggcaatcatttcgcgaagcttcatacaggcggcgtaaacgccggaggtggaggtattcgcgccccattgtccaccagaacccgcagaaaccgggaaactggaatcgccgaggtgaaccgcaacctgctccagcggtacgccaagcatttccgctgccgtctgggccagaatggtgtagctgccggtgccaatgtcggtcatgtccgtttctacggtaacggtgccgttttgttcgaggtgaacccgagcacccgatttttccagcagattattgcgaaagcccgccgcaacaccgtggccgactagccactccccgtcgcgcacctgtccgggtgtggcgttgcgctgcttccagccaaatttatccgctccggtgcgcaagcactcgataagctgacggcgagagaagcagcgcgtcgggtcggcggggtcaacctgagtgtcattcaggatgcgaaactcgacgggatcgatgcccgctttttccgccagttcgtcgatcgcgatttcgagcgccatcagaccgggggcttcgccgggcgcacgcatggcgttcccttccggcaaatcaagcgtggcgagccgcaggccggtatgacgattcgccccggcgtagagtaattcgctttgctgtaccgccgtttccggcgtgccgccgggcaggtttccagaccagctttcatgtgagatagcggtgattttcccgctctggtcggcaccgatacgcaagtgctgaagggtggcggggcggtgcgtggtgttattgggaatagaggggcgggggagcatcactttaaccggacgtttcaccgctcgggcggcgagggccgccagcagcgcatcgcttctcaggaacagcttgccgccaaaccctccgccgatatacggggagataatacgcacattctccacgggaactttcagcgtttttgccagatcggtgcggcaccagtcaatcatctgatttgaggtccagagggtaagcttatttccatcccagacggccatcgaggcatgcggctccatcgccatatggctctggtccggggtcgtgtaggtagcatcaatcttcaccgcagcggaggtgaaagccccgtcaaagtcaccgacgtttttgtcgggcgtgtcttccggcggctgattgacggcctgtttttcgtccgccagggagtaagctcctttattacggcgatagtgtgcctgcaccagcgaggccgccgctcgcgcctgttcgaaggtctcggccactaccagcgcaatggcctgatgatagtgctcaatagtggggccgcctaacagcctggcggtgtttttgtcgcctttgccgagtgccccggcgttactggcggtaatgacagccagtacgcccggcgctttttgcgcggcgtccgtatcaagggcggtgaggcgtcctttggcaatggcggaaccgacgatatagccataggcggcgttgggggcttcttcatgccattcgtaggcgtagcgtgccgtgccggtagttttcagcggtccgtcgatgcggtcatggggacgaccgacaaccttcagctgatcgatcgggttttcccctgcgggtttatcaaatttcatgcctgtgccctcgcttcagccagtacggaggcaagcgttcgcttcgccaacaggagtttaaaggtgttttcagcggtgggatgggcgctggcgaacagcgtgtcatatacggcctgcgccccctgggatagctgagcatccgcagcctcaatgcgccagggcttatgtgctactccgcccagcgcgacgcgcccgctgccgtcaggctgaataatcgccgcgaccgataccagggcaaaggcgtaggaggcgcgatcgcgcaccttacggtagatatgttttccgccgagcggtggaggtaacgtcaccgcaacgataagctcaccgggaagcagggcggtttcaatgtgcggcgtttttcccggagggtgataaaaatcagccagtgtgatactgcgagtctttccctccggcgtgatggtttccaccaccgcatccagcaaccgcattgcgaccgccatatcgctcggatgggtggcaatgcaggcttcgcttacgcctaccaccgcgtgctgacggctaaagccttcaagcgccgcgcagccgctcccgggcaggcgcttattgcagggctgattggtgtcgtaaaaataggggcagcgcgtgcgctggagcagattacctgcggtggttgcctgattacgtaactgaccagacgcgccagcgagcagggcgcgggagagtaccgcgtaatcacgacgcacgcgctcgtgagccgccaggtcggtgttccgtaccagtgcgccgatgcgcagcccacccgcgtcggtcacttcaatcttatcgagcccgaggccgttcacatcgataaggtgggtgggcgtttcaatttccagcttcatcaggtccagcagattggtcccgcccgcgataaattttgcgccgggtacgcgctgagcgctaagtgccgcctcggctggggtattcactcgttcataggtaaacgccttcatgattttatctcccccgcagcatcttcaatggcggcaaggatgttagcgtatgcaccacagcgacagatgttgccgctcatacgttcacggatctcatcggcagttgtttctggagcggaaaccaaatcgaccgtgacgtgactgggaatgccgtcctgaatctcttttagcaccgctactgatgagcaaatttgcccggaggtgcagtagccgcactggaagccatcatgcttgataaaggccgcctgcatggggtgaagattatctggcgaacccaggccttcaatggtggtgatctcggccccctgatgcatgactgcaagcgtcaggcaggcattaagcctgcgaccattgaccagcacggtacaggctccgcactgtccgtgatcgcaacctttcttggtaccgatcaaatgcagattttcacgcaaagtgtccagtagcgtggttcgggtatccacctcaagctgctcggttttgccgttcaccttcagtgtcaggggcattatctctggcgcgggtgtagctgccggaacgcttgccgccagcgtagaatgaggataaaccacggcggtcgccgctgttgcggcgctcactttaatcagatcgcgacgggtcaaacttaaatcgtgcggctcgtgcttcccaacccgattatcttcggggtattcgccttggttgctcataccaggcctccggtattctaaaggggaaaataagagtgcgttgcgagagtgctgatgcttttttaaacgttaagcatagtcggcgacagcaggaggattattcttaaaacgcgaatgcagctatgagcccggctaataaattcatgttcgccgggatgttgatgatgatgggagctggtttattgctttagttgtacgatgcaaaaaccaataaggaaacctgtgattttcagctctacatcaccctgcaaatctctgtcacttctaatataaaaatagggagaaatgatggagcttatattcattggcgattaggaaactatcttgttatacaaaacaatacagttctttacatttgccttgttttatgaatactcctgaagaggtgtataacataatggtacaagcagggtagatatgaatatatttgaacaaactccaccgaaccgcagacgttatggtcttgctgcattcattgggctgattgctggcgttgtttccgcattcgtgaagtggggggctgaagttccattgccgccacgtagcccggtggatatgtttaatgcagcgtgtggcccggaatcattaatcagggctgcaggccaaattgattgctcgcgtaattttctcaatccaccgtatatttttcttcgagactggttggggctgacagatcccaatgcggctgtttatacctttgccgggcatgtctttaactgggttggtgttacgcacattatcttttcgatagtgtttgctgtcggttattgtgtggtcgctgaagtatttccaaaaattaaactctggcagggcttactggcaggtgctttagcccaactttttgttcatatgatttcattccctctcatgggactgacgccacctctgtttgatctcccgtggtatgagaatgtttctgaaatttttggacatttagtctggttctggtctattgaaattattcgcagagatttacgaaacagaattactcatgagccagaccctgagatccctttaggctcaaacagataatgcattgaatgataaaaatggcgcaaatacagcgccatttttataggttaaaaacattgctttttatattctgatgcagatagtcagtgagtatatcgcgctacttcaggatgatgtagatccgaagaacgctacagaagagaggcattgttgctggcaaatagaagaagtatcgggttttgttacccctgaaaaacgaagccccgctattatcgctggcggggcagtgcaattaattattgtatgtttataacggtgtcagcccgtatttagcccttgcacgattgcaagcctcattgacgactccgttctcaccagacatggcgaattctctgcatgtggacgatcgatttttatatatcgtgcagcaggcatttttgcccggggttcctgcaagggcaatacatcgggggtttttctgattggtaccgctcatgcatcggtgaaaaggggatatttgttcagtgagcctggcgggaatagtaccgccagcatcgtcggcttcggcccagtaaaaagagacgcggaaaaatgcacaacaggcaccacacgtcatgcatggattcagattgctcataattcaccagtacagctaaaaatcgtaaagagaacagcggtacatcgtatgtaagaacgtaccgcggttggctggggaactttcgatagtgtgagtattgaatgatttccagccgttaccgattttacgtactaattcgtgattaaaccactcgttagcaggctgcctgatacctttccgtgtctcctgaacactatggtgtgcatatgagaaagcccatcgttacaggtgatattgacgatcgcttccacatcatttaaacgatttttggggctctgaggtggaattcttccctcgaccgatggataagtcttagtccgccgaagggggcttagccggacaggaatcgctaatcttaatgaatttgtcgttatagaccagatagtgattccccggctgacgtaactcaggctgatgaaccacgtctcccggacgtagataccaggcatcgccttcctcttcggtcgaatcacatcctggcttaatcagtagcttaaaccatgtgttgccagtgttacttaccgttcctgtcaccttgtcgaaggaccatttaaactgaacctgacgtggtcgtactaccagaatggtatccatcaccaccaccggctccgtgctgaccacgccgccggttgggctgcgtcttgtatggttacgagtggggacctcgcgaaatgagacccggtagtagcgctcgcggttatcccgtggaccatgatagtaaaatttaaaatactcgctctcaccagcctgcaacgccagctggcggggggcgaaaagcagttcaccatccaccggtcgggtgcgcaattcactgctgcccgggctatcaatagcactgatggcaatacggtatatccgtgcgcttttgttgttattcactacacgtttgctgacaaagtcagtctcggacggcagcgaaaatgtcagattgccgaccgaaatcgcctgtgtcaaaggtgccgccagcatacagaccgctgtcagcagggccttagttaatgttacgccacgtcgcctgaacatgaatctctcctgaagcgctgacttcgccaaaccagccgttatcatctaccgtacgcagcgaaatggcgttatccattggaatcgaaaatttgactgtggtcttatccatctgccccacttcgccagagatatcagtccacggtgtggtcaaccacagcgcatcggtcatatcccgccagctatcatcgcacccggcatcgtaggtttttgtagctccgttgcgggtaataaaggaaagtgtcgccgggaacggtactttcgccttaccgtcatcggagctgaagacacaataggagcgcccgccaatcacctgcgcgggtccggtcaccttgatcagcacttcgtcggcagctgttttaccgctggtggttacgatatagccgaaatcgagtgccgactcgccgctgccaacatatccctcccgcgacggtgtctgagtatattcatcggagataatactgatgctgaaatcacggggtttgataatcagcgtgttggaggtagaaaattcataccagccagactccggtgatgtggtgttctgaaagcgaaagttgaatagatctttggtgttgatatcgctgatcccgaggttcaccatctgcttaaagaagttgctcgagaagaaaacatagatcgagtctgcgctcttcatctcgttgaaggtgtagtaataggcggtattgctcaccggtttccatgaactgccattcagactgaactgcatatcgtacgccccgacggccgaggctaacgacgagttggcgatcgccgggaatatatggattgaggtgttgctgagtccgtttgtttgcagggtatagttaaccatcttacaacttaatcctgaacggctgccgatggtttgcgtccggcagtcggcgttcccttcgcccagagtcggtactccgtcgctgttgataaatacttccgccagcgagtgggtatttatcaaccgtagatttgctgctttcgtatgggtgacgttgcgaacataccagttgccggaggcctgatccttacagcgtgcgccgctgctggcgtcatagttcacagaggtctggcaggcattgatggtcattgtaaagctgctgccgacgggcatttgttgcatatactggtaaaacgcgtctgacaacatgccgtgcatccacttcgcgccgccgctggtcaccgtcgcgccataaaatccactggcgtcggtggtttgcggcaggataagactggtggtcatattacacccagcgtaccagttgatgcagcgcaagccagttaaaggagatgaaactggtgaattttccagccacatatcaaacttccagttggtataaaggccggtgttgtaaccgttatcaatgtagccgaggctttgctgatagatggttcctgaaccagtgtattttaaaccggtccagcggttggcaccggtcaggcgcggatccagcgccccgccaggagtgacgaaaaagttgtcgtctgagttgttttcgacaaacacaaactcgcgtgccggtgcatccgcccaggttgttttgctcactgccgctctgagcgcagttactggccagattagcgcgaaaattatcatcgttattagtaggttaactctcattctcttctcctgtctgcgtcaccgccgcccacgatgagaggccgctgcagaccacatcaccgacccagacggcaccgcgcgcctggttgagttccagagccacttcgcaggttttattgccactgtagcgaaaatcgatagtggggtatttcttatccacgtccatgacaaactcgccgttttcatcggttcgggttcggccgatatggttgttaatccgtgcgttagccagcagtgtgccgtcttccgcacggatacgaccggagacggtaaccatctgcttcacctctggctcaatgacagcgacattgcctggatagagagtcagacgacttttgcggccgctgacgatatcgtaactgtcgagtgagtttttgctgttctgtaactccacctcatatcttccatagggagagagcgggagatagttacgcttgccgttaagcgggaaaatccgcccgttgattttggcgctgatctgaccgtcgtcctccagcccggtgttgaatatcaccccagcgttgccatcagtccgcccgctggcagcaatgtttttaccctgccagccgacgctgccattggcggtcaagttggtattgacgtagccgtccgccgcgctattgacgttcagcgttccgctggcgtaacgagcgtcgaattgtgcatacgccccgccgctgagggttttgtcatcaccggtatcgccggagatggcacgtgacagattggcaccaacagtgcgaatggttccttcatcaaactgtttgcgtgctgacaggtttgccatggtgtagccgttttgatgagtcatccctgcgctaaaccagttgcccagtggtagcgagagatcgagagcgatatattttcctgtattggcgttgctgtcgccgttgttatagcgctgaataccggcccgcaggccaagcgaaccaaaggtaccgctgtagacattttgatagtaatctgccgtgtaataatggctgttgtaacggcggtcatcattgtagctgatgctgaatgtgcccagcttcgaccacagtgagttcaggttgagtgtgccgccgattgcacggttgtcggcatcgctacgtcgcaattgattgccaatgcgggttttttcctgattaacccacagcgaactaaagcctcccggtagagtggcgctgatgctgccgatgctgctccatgagctgtcactggccagcatattttgcaggttaacgttgatcgcccccccaagcggcagcgtcagacgggtttcacccaccgcctgattatcgtatccatatcccgttgccgcccagctaagcgtactcaatgagccggaggtcgaggcacctgctagccaactctctttagctggtcgcgtctttttcccgttttccgaccagcgatccatatgaaagctaccgccccatacctgccacgccagtggtgcaccgacgccgcgcccccggctaaacagcttattgacccgctgggtgcgtttgctgatcacgcgaccgttaacgatcacctcaacttccacatcgtaaatcccgtacggtagaccccgggtatccacttcatgattgcccatagtgaagttctgaacgcttagtagccgcccatcacgggtgagatgtacttcgcccgccgccggtaaaaaggcgatcactggcgtggctgactggctgctgtcgaagatggtggagctggcctggtttccccaggaaaggccgtaaatcttccctgctgaaatggcggtcatcggccctaaggactgcaagttccaggtgtcgagcattccaccggcaaatcggtgaccggcaaaatcgcgttcatacatcgctttatataattcactgtcctgttgaccgctaccgatcccgtacagcgagccgtcgagcaccacatgatgttcgcgcagtgcagtaacgttattcagcgacagatagctggatgtgttgctcccgccgttacgcaactggttgttatagacgcccaagttatagctcagattactgctgagggtgttaacactggactgcccgatgtcttcgctacgtgagcgtagtacggtgcccagcgcttcgcgcttgaccactagctgcagcagcagttggcgcaagctgagatccagctgcgcgttgtcagtcagggggatggtaagggcctcattgaacggggcgttggccagagccatcagctgctgtcgagtttgttcgctgacactggcgttatcttcactctcttccagctgtattttccggatgcgtagctgtccatcgtccagccagataaaagcgctgccgattcgctgatcgtcctggcgaccctggctaccggcgagatgaatatagagcgggacgctcatgccgtcctgaagcgcctgactgaaggcctgcggaataatcaccccacctatttgctgcgcacttatgtcagcagcgctggcatcgggctgaacgaacaaaaagaccatgccgaaggcaaactgggctttcagtcctggggagaaccgtcgtaaaggcattgtcgttatccatctgcacagctatctatttcacgggaatgaacttatcaccctgccaaagtgcaacccgtcctttgttatccgcagtgtccacgcgggtaaaacgacgcgacttgcccggcatcaggtagtaattctctttacactccttaccgttggcggctttcaggcaaggtccgtaggcgaggatccgcagcgtcgcatttcctgtatttgtcagggagccgttggcgtactgaaagtggtagttcgcctgacgaggggcgacgaccagaatggtgccgatgcgggcggaagcagtggccacagcgctgcggttggcattatcgcgctgcgcatcactgagggcctgatcaaaccagacaatgcggtagtagcgctctttttcatctgcgggtcccttatagaagaagcggatcacttcgctggcttgggcgggtagcagcaagctggcgggagtgagtagcaactcatccggcttgtccattgagataacctgcccgtcgtcaagcggtgaagagagccgttcgagacggatattgataaggcgaccactgtcggtactgtttttgatcgttttgctcagcgtgctgctgtcactgttcataaacgatgatatatcgccgacatccagcgcctgggccggagatattccggaaaacagcagagcgagaggcagaaggtgctttttcataacaattccgtccaggaataaagcaggggggctacccctgctggtacatcagagagattaactggtccaggtcgcgtcgaactgtacgctaacgtcgccgctccagatgccttccggtagagtgctgtaatctgttactgcggtggtaccattggtggtaccgctgatgatggagaaggtgaaaccatcctgtgcggtggtacgattgctggcattgtaaccgttagccagcgggctaaggttgccgcccagtacgccgttggcggtatcgatcatcacggtatcgccagttttttcgactgccgcgccgttataatccacgcccacattcagtgtggaacctgaggtatccaactgggttaatgtgttggtgataagacgtgaggtcagtttaaaggcggtagccgttgagtcaccctcgatagccacgtcaaatagacctttctgtgagttaaaacctttaatgccttcggcatactggaacgccaggctaccgagtggcgtcacaaccagcttactggtggtgtcttttttggctgttgccgaccaggtcgctacagcctgagctgttacgtcagcagcctgcgccacacccatgccggtaaacaccgttaccagagctattgccagaaccttttttttcattgcatttcttcccgagttgaattgaggacgtgatgtcccagtgagtcattttttaaaactaacttgcctggagtttactgaaccaacttatatatttttgagtacagcttggcctcagcattacgccgatgggtatacactgtcttcacactacaattttcaattctggcaatcgatttaggttgcattccctgggccgtcatgcggataatttccatttcccggtccgtgattttatctttcttaatatcttttctcaggaacctgccattaatcacatagaccagttcttttctaatatcacgactcagtccagcgtataccacgcccctaatattgctattgtaataccaataatttgctaaggcctctgactttctggccgcaatcaatacgacctgtttcccctttaccgcggataaccattcattatcacggtttataaattcagataaagaatccgtactgagattgataaacacgaaatcttttctaattttctccaacgatagataaattaatctgtcgatatccacaatcagttcagatagtcctttatagaagtaggcgtcatggggagaccagatgtatttatcagaacggttttgacattccatatggtttttaacctcatagtccctactgtaatcactttgccatgtcactactttccaaacctgtaatttttacaggtgcattcagtttccttagtaaaccggaagtaaataagatacgtagtacatatcaataaaggttaaacgagattaagtttaattattttcgattgggcttaaatttatgttttttttcccgatgagtgtcaatatgtgaacggaaaaggaattcaatggttaagtcaatatttagaaaaactgaaaatattgcttttttgataagaagaaaaagacatttggtttcataaggttattggcaatataacgttcaattcttacttgcattttatattggtcaggaactttgccctgaagtgttaggaatagtcttaatgcgctgtgtgatggactagtaaaaaaacaagttttaagggtaagggatagaatataaaactatgatgagctgtcattgaagatgatttgccaatcagtaagatattttaatggattaacatgccgcacaaaatggttacaggtgttcattccaataagtaatggaaaattgaacgggcgtatgtacgtcatctgttcggtaagcccccaagagccagattaagtgaagttaaacgaaggctgccagctgtcacaggaacgatggcctttttgtcagggcactgcattcagttatctgtgcgcgttactctaactggcactcgaacgtcggcgacggggttaccggtggatcagactgttcctgtggcgtaaacgtttttatgttagtaccaacagatttaccacatttatcatcttaacagtttgagtgaaaatgcaggctgcgccgcaaagggaggagactgagtggcgtgttcagtctaaaagagggttgatgccagcatacaggggcgaagctggtcaacaagtcaacattaagataatggaatattcggagagaaacgtcaggcagttggcctcaaatgaacaggaagaatatatccccaggaaaattaatgttggtgttataaacacaccaacattaatccgatctgattattaatcagacaaatatcgttaatccgtcgaattttgaatcaacgttttttcttacgaccctgaacggccttaaaacgtggattagatttacaaatcacatatagccgtccttttcgcttcacaatctgacagtctggatggcgttcttttgcggtacgcagagagttaagaactttcatcacgccccctttttcgtgctaacaaaacgaccaaaacgttgggtgaatcgtgcaacatttccttctgatgccactgttctcagcttccctgtatagaacgggtgcgatttagaagagacatcaattgtcacgtatggatacgttacgccatccagctcaatctcacggtctgttttgatagtcgagccgattttaaagtactcatcaacactggtgtcgtggaacaccacagtacgatactcaggatggatattgggcttcatcatttttacctgttatgttataacataaccataaagatacatgctcatccggatcatttcaacactcaatccctgtgactctttgtggatgtggaattttcgcaacggggaactctggcattgttagcagccattggtgacgctcccataaacgcctggatgagtgattgatgatggttttgctgagagtatggatttttcgagaatggaggttatctccactttactggccgataatttatcgcagtatgattgattacctgacagcgtgtattcctctcccacggatataataattacttacaaaaaagggagaggatgcatattttaaatatcactgaagtgaacagtttatttccgttattaatagaaatggagaaataaataggcgtattctacaattgcgacaaaaacaacgatattaatcagtttatgactgatttgctgtactttattctctttcattggtacttcctcgctttaaaaaagagtgcacttcgtaagtgcccttatataaataacgagtttggtcaaccaattttttgacatgtatcacaaatttgaatagatgtattacatcaactatcttttattgcaccaacgtcattgatatatgtcgcctgaagtcagttccgggaatgagtctgatctcaagactggcccagtccgggcgttgattggtgctgaggagcatatcgcatctcatcataatgtcgtatctcctggggtgttatacaagatatcgttgttggtgacctgggagaggaattgagttctattaaaccgtcaactatgccggatacatactggattacactgcaggcacgccttatgagagaacgtgccgcagtgacgggttaattatctgaaagaatttgtgaggctgtatcggttactcattgatttgatagttttactctcgggagaataatagatatttaatccattaacggaaaccagccagttcctttcgatgcctgaatttgatcccatagtttatccggaatggttaattcatgaacaagttgtgttatcgttcatgagaagcataacgtaaagggaaaagctcgattagacggcagaatttgtcaggggttatgaacgaaattcataaatctgtttgagtgttgcgatgggtagtgcaagttcgatatctccgcaatttacagtccgatgaaggaaaatgaatatccataaaaaatatattggtttatcctggcatatatacctatttcgacgtatttccaatagttttaattaaaggcaggtcattgttattcactctgaatagtgaattattcactgtccgcagagtaagaaatataacttaggtatctatttaatgacttgcacaaaaagctaaattttcccccataaataaaaatataatcccgcgcccaaccacctgatgagtggctataggcactggatatattaggtggcggtgcactttcttacataaaggtatttccttttctgcggaaaaggaaatcgggaaatccccggtttttctgacaagcagacgccattatttgtgtctgcctatgttcgttaattcgttcatcaggaaattatctcaatgtcacattataaaacaggtcataaacaaccacgatttcgttattcagttctggcccgctgcgtggcgtgggcaaatatctctgttcaggttctttttccactcgctgtcacctttaccccagtaatggcggcacgtgcgcagcatgcggttcagccacggttgagcatgggaaatactacggtaactgctgataataacgtggagaaaaatgtcgcgtcgtttgccgcaaatgccgggacatttttaagcagtcagccagatagcgatgcgacacgtaactttattaccggaatggccacagctaaagctaaccaggaaatacaggagtggctcgggaaatatggtactgcgcgcgtcaaactgaatgtcgataaagatttctcgctgaaggattcttcgctggaaatgctttatccgatttatgatacgccgacaaatatgttgttcactcagggggcaatacatcgtacagacgatcgtactcagtcaaatattggttttggctggcgtcatttttcaggaaatgactggatggcgggggtgaatacttttatcgatcatgatttatcccgtagtcatacccgcattggtgttggtgcggaatactggcgcgattatctgaaactgagcgccaatggttatattcgggcttctggctggaaaaaatcgccggatattgaggattatcaggaacgcccggcgaatggctgggatattcgtgctgagggctatttacccgcctggccgcagcttggcgcaagcctgatgtatgaacagtattatggcgatgaagtcgggctgtttggtaaagataagcgccagaaagacccgcatgctatttctgccgaggtgacctatacgccagtgcctcttacccagcaatagtggacacgcggctaagtgagtaaactctcagtcagaggtgactcacatgacaaaaacagtatcaaccagtaaaaaaccccgtaaacagcattcgcctgaatttcgcagtgaagccctgaagcttgctgaacgcatcggtgttactgccgcagcccgtgaactcagcctgtatgaatcacaactctacaactggcgcagtaaacagcaaaatcagcagacgtcttctgaacgtgaactggagatgtctaccgagattgcacgtctcaaacgccagctggcagaacgggatgaagagctggctatcctccaaaaggccgcgacatacttcgcgaagcgcctgaaatgaagtatgtctttattgaaaaacatcaggctgagttcagcatcaaagcaatgtgccgcgtgctccgggtggcccgcagcggctggtatacgtggtgtcagcggcggacaaggataagcacgcgtcagcagttccgccaacactgcgacagcgttgtcctcgcggcttttacccggtcaaaacagcgttacggtgccccacgcctgacggatgaactgcgtgctcagggttacccctttaacgtaaaaaccgtggcggcaagcctgcgccgtcagggactgagggcaaaggcctcccggaagttcagcccggtcagctaccgcgcacacggcctgcctgtgtcagaaaatctgttggagcaggatttttacgccagtggcccgaaccagaagtgggcaggagacatcacgtacttacgtacagatgaaggctggctgtatctggcagtggtcattgacctgtggtcacgtgccgttattggctggtcaatgtcgccacgcatgacggcgcaactggcctgcgatgccctgcagatggcgctgtggcggcgtaagaggccccggaacgttatcgttcacacggaccgtggaggccagtactgttcagcagattatcaggcgcaactgaagcggcataatctgcgtggaagtatgagcgcaaaaggttgctgctacgataatgcctgcgtggaaagcttctttcattcgctgaaagtggaatgtatccatggagaacactttatcagccgggaaataatgcgggcaacggtgtttaattatatcgaatgtgattacaatcggtggcggcggcacagttggtgtggcggcctcagtccggaacaatttgaaaacaagaacctcgcttaggcctgtgtccatattacgtgggtaggatcataaagtcctcgggtcgttgtccactcttttggcatgtcagcatattcacataccgtaccagcaaaagtttcaaccgtgagcaaatcgaccgattttgttgacggttcaaacgtggaaacgaaatagatatccgtcttaaaattcttcatacatctggctaaatgatgacgtcgtagtttgacttcttcatccggtgatttattcgacacttcaatgtcatatttaaatgagttgccaaaaataggtgtctcaggaaagttgattaatctacactccgtcttttgctgttgacgtattaaaaaagaagggaagatatttgcgagatcccaataatcacggtggcggtattcacggggagagcagccgaataactttttaaattcgcggctgaatgactgctgtgaatcaaaatgcaaagagagtgcaatatcaagcatagatttcgcggtgagccggacaagaatggcggcacgacaaagccttcgtttgcgaatgtattctcccaaaggcacatgcatgaaatttcggaacagaagctggatgttgcgtctgctgtagccagatttctgtgcgatatcttcgattgaaatagggtgctcaagattgcactcaatccactccaggagctgctgtagaatcttctgcctgatcatctcattctccgttaattctttgtcatatcgcacattttcgttataccctgggccctaagtgtatcaaaaatagcaagggcgaaggcaaaagcactggtagcgtctgcttcgttgtccccgaaaatagagaggtttcagtcctacattattaatgaattttttgcataagtgatatcaaaatccacatactactttgaggttacgttttaacgtagactcattgttcatgcctaatggagggactgacagtggaattttccgtatagtctgcttcagagtattgcagatgcccatcaaaaatcgatttctcactgacagataaagaaatggcacaaattagttcgcttgatttgggttatgttggggagtcggtaaaacattttaatcctgaatttgttcgtggttgtcttgctgtaaaaatacatgattgatattaatcatgtattttacctaagacgacaaaaaccttttaacagggagtgatattgatcttcactctgtcatatctccggtaatatggcgtcaggcttcatcatcagaaagggggcctgacgcctgaaaaagtgaacaacagacagtgttcggattatcaatattcagtttttaacgttgaactggattcattactgcgttgtttaagaatttcccgcgccgaatctgccattatcatgactgcacctgccagcatcagagtatctttcaataccaggcgaccagcaccggataaataagggaaaccatgatgagcgtcacccaatgcgggtacccatgcctccggggtggtgattaaaaatgagagtgttaccagcggcgtggtaaatgccatcagtcctcccaataaacctaaccagcgattgacaggattagccaaaaccagcagagcaataatcacctccacgacgccaagaccgttggaaaaaccataggtattattggccgtttgccatgcccttgcttctggtttgtattcgccttcgtgagtcagatactgtttatagtcttccgggtgttcataaaagaacgacattagtggactgtttgcgacgaatggtgtaatgctgtctgcctcgtaagggacaaactttaataacccaatccacataaaaacaattgcaatactcagacgaatcaatgtcaggccaattttatctccccgacttaacaggtgcaggtatttttccattgtgaacatccttatttatacaatactgctgttgcggttgaattattatcaattcgcatcgatgtgactttccaggatgaagcattatattttctggctatatcagcaatggtatcctccagaactgtcggtgatgctgatactgacgagacgctgatatgtttcagaattattttatcatctgcattggtggaaaatgccataacgccagataatagtgttgcaaataaaacagattttttaaacatataaaataccatcaatgaagtgattaagaagttatagagtaacagagaattaataagattcttttctctgagacgccagaatatttgttctggcgtctgattttgagtttatttgactaatgaaaatagatcattgagtgattcgctcatcgacggatgagtaaatatctgatcgcgtaatatgctataaggcagcccggcatccatcaccattttcactatattgatcatctcgtgggagtcaacacacagcagtgatgcccctaacatacgttgggttttattatcaacaatcgcttttaataccccacgagtatcattcatcactctggcacgcggaattgcagctacaggcaatgtcaccacctgaatatcagcaccactctctctggcttgttcttctgtcataccaaccctggacaggggcggtgtcataaatacggaataaggcacatttttccgatcatcagtactacgtttgccttcacccagtaactcatcacgtacaatgcggtaatcatccagtgatatgtaagtaaattgcagcccgccggtaacatctcccatcgcccaaatattgtctgcggtggtatgtaatcgcttgtcaacgacaattgccccgcgctcgtttactgcgataccggcattttctggatgtaacgaagcggtagccggttgacgaccggaagctattaacagtgcatccaccgccagttgggcgtgctcgctatgcacttgcacttgattttcatggtgactgattcgctccacatgggcattgaggataatatcgacgccctgatcgcgtaaaatcgtcgcgatattatcagcaatatcccgatcttcccgaggcaaaaacagcgaagctgcttctaaaatggttaccttgctgccaaaattagcgaacatagaggcgaactcaacgccaatatatccgccgcccaaaatacctaaatgcccaggcaattcttttagattaagtaatccggtgctgtcatatactcctggcgtggtggtaattccaggaattggcggaaccacggtttgtgcaccggtattaataaaaattttctcgccatgaatttccagatttccctcaggccgatgaacacgcaggctatgattattgataaactccgcctggccgtcgatcacgtcgatattgggcatatccgcaagattatgaaaattcttattacgtaaaaaattaaccacttcatttttacgctgtatggcacggacaaaatctgtgtgctgctgtgcgtcatgaaccaatgttttggttgggatgcagccgatattaatacaggtcccgccatacattgcatttgattgttcgatgagagccactcgccaacctgcttttgccagcgtgacggctaatgtttttccagccttgccaaaaccaataatcactgcctgatatttattcatgatgatttcctgtcgaaacgcgttcatttgacatcatgactatagacgcaaaagagcaaataacatttcttcacaacgcttgatattttgtcttatcgtctgatattttctttttcttaatcagaatcacaaaacaaaaatcatgattaactatttgatggtattagattagttatttactaagattgttggtgtttgtaatcaaaaaccactcaggagtctgatatggatgcccttagccgtttgttgatgcttaacgctccacaaggaacgatcgataagaattgcgtgttaggaagtgactggcagcttccacatggtgccggggaattatcggttattcgttggcatgcgttaacgcaaggagcggcgaagctggaaatgccgacgggggagatttttacattacgcccgggaaatgtggtcctgctaccacaaaattcagctcatcgcctgagtcatgtcgataatgaatcgacctgtattgtctgcggcactcttcggttgcaacattcggcgcgttattttttaacgtctttgccggaaacgctgtttttagcaccggttaaccacagcgtggaatataactggctgagggaggcgatcccgtttttacaacaggaatccagatcggcaatgccgggagtggatgcactgtgtagccagatctgcgctacattctttaccctcgcggtgcgtgagtggattgcacaggttaatactgagaaaaacattctcagtttgcttctgcatccacgtcttggtgcggtaatacagcaaatgctggaaatgccaggacacgcctggaccgtcgaatcgctggccagcatcgctcacatgtcccgggcaagttttgcccagcttttccgtgatgtttccggaaccacgccgctggctgtattaacaaagttgcgtctacaaatagcggcccagatgttttcccgggaaacgctccctgttgtggtgatcgctgagtcagtaggctatgccagtgaatcatcttttcacaaggcgtttgtccgcgagtttggttgtaccccgggagaatatcgggaaagggtcagacagcttgcaccctgaataaaaccgccagaaatcagggcaaagataatccgcattccgggagttgtgagcctttcaactatttctatttccaacggtggtttgggctttatatattttttctgatggactctagctcagtttttaaataaaaatgcaaactaaattgcttcaattaaataaaatcccgactattacttgatacgtgattattgtcggtgatttttttgtacaccatcagtgtatatctcaataacccctgaataagtagctctgaataggtataagggatgtagccatttttaaatggatttcttatgccaaaaatgatcgtcgatttccccataaaatgtgagcgatgccgaaagaaataaaattagttattgcatttgacgtttggatgaaagattatcatttgtcatacaaatgaggggtggtatgttgctagccaattaaaaaagaacgccatatttattgatgattgatcccccggtgggggggaaacatcgggcataaatgggcatgaagtaatggagtattagttgtgaatgtcaatttctttgtcacctgtattggtgacgccctgaaatcaagaatggcacgagactccgtgctgctactggaaaaactcggctgtcgcgtaaatttcccggagaaacagggatgctgcggtcagcctgcgatcaatagcggttatatcaaagaagcgattccagggatgaaaaatctgatcgccgcactggaggataacgacgatcccattatttcaccggctggctcttgcacctatgccgtaaaaagttacccgacgtatctggcggatgaacctgaatgggcatcacgtgccgcaaaggttgccgcgcgtatgcaggatctcacctcttttattgttaataaattaggggtagtcgatgtaggtgccagtttgcaagggagagcggtgtatcacccatcttgtagcctggcccgtaagctgggagtgaaggacgagccacttacgctgctgaaaaatgtgcgtggactggagctgttgacctttgctgaacaggatacctgctgcggatttggcggcacgttctcggtcaaaatggccgaaatatccggcgagatggtgaaagaaaaggttgcgcacctgatggaagtccgccctgagtatttaattggtgctgacgtgagttgcctgctaaacatcagtgggcgattacaacgggaagggcagaaagtcaaagtgatgcatattgctgaagtgttgatgagccgctgaggatataaagatgtcgatcaaaaccagtaatacagattttaagacacgcatccgtcagcaaattgaagatccgatcatgcgcaaagcggtggcaaacgcgcagcagcgtattggggcaaatcggcaaaaaatggtcgatgaattggggcactgggaggagtggcgcgatcgggccgcccagatacgtgatcatgttctgagtaatctcgacgcttatctgtaccagctctcagaaaaagtgacgcaaaacggcggtcacgtctattttgcaagaaccaaagaagacgctacccgctacattttacaggttgcccaacgcaaaaatgcccggaaggtggtgaaatctaaatcgatggtgaccgaagagattggtgtcaatcatgtgttgcaggatgctggcattcaggtgattgaaaccgatctgggtgaatatattctccagctggatcaagatccgccatctcatgttgtggtcccggcaattcataaagatcgccatcagatccgtcgagtgctacacgaacgtctgggctatgaggggccggaaacgcctgaagcgatgaccttattcatccggcaaaaaatccgcgaagatttcctcagtgctgaaataggtattaccggctgtaatttcgcggtggcagagaccggttcggtatgcctggtgaccaatgaaggtaatgcgcgaatgtgtaccacgctgcctaaaacgcatattgcagtgatgggaatggagcgtattgcccccacgtttgccgaggtagatgtattgatcaccatgctggcgcgcagtgccgttggtgcacgtttgacgggatacaacacctggctgacaggaccgcgcgaagctgggcacgttgatggtcctgaagagtttcatctggttattgtcgataacgggcgttctgaggtgctggcctctgaatttcgggatgtgctgcgctgtattcgctgcggggcttgtatgaatacttgtccggcatatcgccatattggcggtcatggatatggctctatttatccagggccaattggtgcggtgatttctccgctacttggcggctataaagattttaaagatttaccctacgcctgctctttatgcacagcttgtgacaacgtgtgtccggtgcgtattccgctgtcaaaactgattttgcgtcatcgtcgggtgatggctgaaaaagggatcaccgcaaaagcagagcaacgggcgataaaaatgttcgcttatgccaatagtcatccaggattgtggaaagtcgggatgatggccggtgctcatgcggcaagctggtttatcaatggcggcaaaacaccactcaaatttggcgcgattagcgactggatggaagcacgcgatcttcctgaagctgacggagagagtttccgtagttggtttaagaaacatcaggcgcaggagaaaaagaatggataatcgaggcgaatttttgaataacgttgctcaggcactgggtcgcccgctgcgacttgaaccgcaagcagaagatgcgccgcttaacaactatgctaacgagcggcttacccaacttaaccaacagcagcgctgtgacgcgtttattcagtttgccagcgatgttatgttgacgcgctgtgagctgaccagcgaggcgaaggcggcagaagctgcaatacgtctgtgtaaagagctgggagatcagtcggtcgtgattagcggtgacacgaggctggaggaattggggattagcgaacgtttgcagcaggaatgcaatgccgttgtttgggatccggcgaaaggtgccgagaatatctcgcaggcagagcaggctaaagtgggtgttgtgtatgctgaatatggtttaaccgaatcgggaggcgtggttcttttttccgccgccgagcgcgggcgttcattgagcctgctcccggaatattctctttttatcctgcgtaaaagcactatcctgccgcgtgtagcgcaactcgcagaaaaattgcatcagaaagcgcaggccggtgaacgaatgccttcctgcattaacatcattagcggccccagttcaacggcggatattgagcttatcaaagtcgtcggagttcatggcccggtgaaagcggtgtatctgattattgaggattgttgagagagatatgaagtctggacataaacctgaagaaggcatacgaggttgaaaatagcgtttaggacaacctgacttaaccccgttccgtcatggttatgctgctcttctgtaaatatcctggtattaccaatgccaggatatttacagtgaaaaagacaggcatccattcctgaaaacgggttcccttcccggtcattgtcacttcagctttatacaggcactctctatcagaatgttgtttattactgcccagagttttgttggtattcatctaccatttttttgacaaggcaaaacattacagaaattacaatgcttagaaaaaatcccagagccaggcaaatggcagcagggtatttattttttatttctggtgagcttatagttacacagccatcaccgttcggatacaatgaccagttcctggtcaggtatatcatttttgtataaagctcactgttaattgctgaaggcgtttgtatctcatcgagaacttgcctgccattatgatattctgacgcataccatttgataatagaggcctgcacgcgagatatttcctcttcagcagttggtaaagctctcttatctcctgaccattccagccttatttctctgttcttgacatctgggctggtgtgaaaaaatgtagtaattcgctgaataacatcttcagtcattgtagtctgacaggcaaaattattattgctatcacagctaacaagtatacctggcgttgtctggtttatttttaggctgtaaatcacttttatattgtctttattgatatacagaaacaacagcaccatagccatacatatagccataataaaaaggataacacgaatctttttcttcagataaaataaaatctcaatcagatcgatatcctgtttgatttgttcacgcataatatatccagagaataaaatctgtcgcagataaggttgtattaatagtctgtatcaggaatgttcgggttaaatatcagcaaaaagcccgcatcatgaatactggatatgaagcatgagagttacctcagtgtttatataaggattcggtccccctctctggaacggtaactctcaatctgatcggttcctgcgttagttcacatcacgactcattttttcgctctcaccggcatcccatttgccacaaaatatcccgccgtgctcctcggcagcgcttcctgtccacgaatcatatccgctattttctcgccaatcataattgtcgtggcgttcaaattcccggtgataatctgcggcataatcgacgcatccaccacacgcaggccttctaacccgtgtacgcggccttcgccgtcaaccacggacatctcgtcgtaacccattttgcaggtaccgcacggatggaaggcggtttcggcgtggttacgcacgaactcatcgagctgttcatccgtctggcattcgacaccggggctgatttcgcggccacgatactgatccagcgcgggttgatgcatgatctcgcgggtgatgcgaattgcgtcgcggaactcctgccagtcctgctcgtgcgacatgtagttaaacagaatcgccggatgctggtgcgggtcgcgggatttaatccgcacatgcccacggcttggcgagcgcattgagccgacgtggcactggaaaccgtgctctttcactgcattcgagccgttatagttaatcgctactggcaggaaatggtactgaatattcggccacgcaaattcctcacggctgcgaataaatccacctgcttcaaagtggttgctggcaccaacgccagtgccgccaaacagccactccgcaccgattttcggctggttccaccactgcagggcagggtagagggaaaccggttctttgcactcatattgcagatacatctccagatgatcctgaagattttcgccgacgccgggtaattcatgcaccagcggaatatcaaactccgccagcagttcagcgttgccgacgccggagcgttgcaggatctgcggtgaggcaatcgcgcctgcacataacagcacttctttgttggccgttgcgcgggttgggatggtgctgtcgccttccagccattcgacgcccaccgcgcgtttgccgtcaaaaatgatgtgatcggtcatagcgtgagtacgaatggtcaggttaggacgcgatttggcctgatcgagatagccacgcgcggtgctggcgcgacggccctgcggcgtgacggtgcgatccatcggaccaaaaccttcctgctgataaccgttgagatcgtccgtgcgcgggtagcccgcctgcacgcccgcttcaatcatcgcttcaaacagcggattgacgccgggtttggaggtagtgacgctcaccgggccatcaccgccgtgatagtcgttttcacccatatcgcgagtctcggccttgcggtagtagggcaggcagtcgaggtagctccagttctccagaccgggttcttgcgcccagttatcgagatccagcgcattgccacggatgtagcacatgccgttgatcagcgacgatccacccagacctttaccgcgtccgcactccatgcggcggttattcataaacggttcaggttccgtttcataggcccagttgtagcgtttaccctgtagcgggaatgccagggcagcgggcatctgggtgcggaagtcaaagcgatagtccgggccgcccgcttcaagcagcagcacggaggtattcggatcttcagtcagacgggtagcgagaacgttgccggctgagccggcaccaataatgatgtagtcaaattgcaaataaacctcctggttagaatatggactggaatttagccatctcaacctggatggacttcacctgggtgtaactctggagcgtcatcacgccgttctcgcgaccaatgccggagtgtttgtagccgccaacgggcatctctgccggggattcgccccaggtgttgatccagcaaatacccgcttccagctgatgaatgacgcgatgcgcgcggttcaggtccgctgtcacgatgcccgccgccaggccgtagtcggtatcgttagcgcggcgaatgacttcgtcttccgactcgtaggtcagaatggacatcactggcccgaagatctcttcacgcacgatggtcatatcgtcgctgcaatcggtgaacactgtcggtgcaacccatgcgccgttatcgaagccatcgcctttcagtacatcgccgccgcacagtacgcgcgcgccttcctctttgcctttggcgatatagcgcagcacgttatcgcgatgcgggaagctgaccagcgggccgaagttagtttgcggatcgaaaacgtcgcccgcgcgaatgcgctcaacgcgcgccagaattttctgctcaaatgcggctttgcatttcgccggaacgaagacgcgggtgccattggtacacacctgaccggagctgaagaagtttgccatcatggcgatatcggcggcgagatcgagatccgcatcatcgaaaacgatcagcggtgatttaccgcccagttccatggtcacttctttcagggaagaggccgccgagttagccatcacttttttgccgctggcgacaccgccggtaaatgacactttggcaatgcccggatgctcggtcagatattgcccggtctccgcgcccacgcccggcaacacgttaaatacgccgtccggcaggcccgcttcgctgtaaatttcagccagctttaacgcggtaagcggggtaacttcgctcggtttgaaaatcattgcgttgcctgccgccagcgccggggcggatttccacagggcaatctggatcgggtagttccatgcgccaatccctgccactacgcccagcggttcgcggcgggtatacacaaaggacgtttcacgcaacgggatctggctgccttccagcgccgggatcagcccggcgtagtactccagcacgtccgcaccggtaacgatatcgacggttgaggtttccgaatatgcttttccggtgtcgagggtttccagttttgcgagttcgtcattgcgttcacgcagaatatcaacggcccgacgcagaatacgcgagcgctccatggcggtcatcgacgcccagattttttgcccctgctgggcgcttttcacggcgcgatcgacatcctcgcgcccggcggcctgcacggtcgccagcacgttaccgttggccgggttaatggtctcgaaggtgcgaccgctggtggcggaggtataaccaccatgtatataaagctgctgttctgccattcgggacatcacgtctcctcggttaatcggtgggtagatgctgagtgataaagtggcgggtcagggaattagcgcgggttttatccagcggtttgccgctcagagccgcgcgcagccataatccatcaatcagcgcggccaggccgtagcccgcttcctgtgcctgttcgcgcggcaattcgcgacgaaactcgctcaccagattcgacagcaagcggcggctgctgacctgctgtaaacgatagagcatcggctgatgcatactgctggcccagaacgccagccaggctttcatcgccgcactgctcacctgcgtttcatcgaagtttccgccaacaatcgcctgtaatcgctgctctgcactgccctgcggaagtgcatgtaatcgattcaaaaccgcgtcacgcagctgactggtgatatcgcgcatggttgcttccagcagaccatttttgtccctgaaatagtggctgatgatccccgtagaaacgcctgcacggcgggcgatctgcgcgatcgttgcatcgtgcatgcccacttcatttattgcttccagtgtggcgtcgatcagttgtctgcgccggatcgactgcatccccaatttgggcattttcgccactccattcatcagcggtgtttatctattaaagcggttattgattggacgttcaatataaaatgtgtcttaattgttacgaatttgattttaaatagtaacaataacagtggggatactggatgacagacctttcacacagcagggaaaaggacaaaatcaatccggtggtgttttacacctccgccggactgattttgttgttttccctgacaacgatcctgtttcgcgacttctcggccctgtggattggccgcacgctggactgggtttctaaaaccttcggttggtactatctgctggcggcaacgctctatattgtctttgtggtctgtatcgcttgttcgcgttttggttcggtgaagctcgggccagaacaatccaaaccggaattcagcctgctgagttgggcggcgatgctgtttgctgccgggatcggtatcgacctgatgttcttctccgtagccgaaccggtaacgcagtatatgcagccgccggaaggcgcgggacagacgattgaggccgcgcgtcaggcgatggtctggacgctgtttcactacggcttaaccggctggtcgatgtatgcgctgatgggcatggcgctcggatactttagctatcgttataatttgccgctcaccatccgctcggcgctgtacccgatcttcggtaaacggattaacgggccgataggtcactcagtggatattgcagcggtgatcggcactatcttcggtattgccactacgctcggtatcggtgtggtgcagcttaactatggcttgagcgtactgtttgatattcccgattcgatggcggcgaaagcggcactgatcgccttgtcggtgataatcgccacgatctctgtcacctccggtgtcgataagggcattcgcgtgttatcggagcttaatgtcgcgctggcgctgggattgatcctgttcgtattgtttatgggcgacacttcgttcctgcttaatgcactggtgctgaatgttggcgactatgtgaatcgctttatgggcatgacgctcaacagttttgccttcgaccgtccggttgagtggatgaataactggacgctcttcttctgggcatggtgggtggcatggtcgccgtttgtcggcttgttcctggcgcgtatctcgcgtgggcgtaccattcgccagttcgtgctgggcacgttgattattccgtttaccttcacgctgttatggctctcggtgttcggcaatagcgcgctgtatgaaatcatccacggcggcgcggcatttgccgaggaagcgatggtccatccggagcgcggcttctacagcctgctggcgcagtatccggcgtttacctttagcgcctccgtcgccaccattactggcctgctgttttatgtgacctcggcggactccggggcgctggtgctggggaatttcacctcgcagcttaaagatatcaacagcgacgcccccggctggctgcgcgtcttctggtcggtggcgattggcctgctgacgctcggcatgctgatgactaacgggatatccgcgctgcaaaacaccacggtgattatggggctgccgttcagctttgtgatcttcttcgtgatggcggggttgtataaatctctgaaggtagaagattaccgccgtgaaagtgccaaccgcgataccgcaccgcgaccgctggggcttcaggatcgcctgagctggaaaaaacgtctctcgcgcctgatgaattatccgggcacgcgttacactaaacagatgatggagacggtctgttacccggcaatggaagaagtggcgcaggagttgcggttgcgcggcgcgtacgtggagctaaaaagcctgccaccggaagagggacagcagttgggtcatctggatttgttggtgcatatgggcgaagagcaaaactttgtctatcagatttggccgcagcaatattcggtgccgggctttacctaccgcgcacgcagcggtaaatcgacctactaccggctggaaaccttcctgttagaaggcagccagggcaacgacctgatggactacagcaaagagcaggtgatcaccgatattcttgaccagtacgagcggcaccttaactttattcatctccatcgtgaagcgccgggccatagcgtgatgttcccggacgcgtgattgttattgcataaaaccgcgccatgtctgcatatggcgctgtttctcctacctcttgatacgttatatctatacggttaagcccttagtatctattgatgattaccagacaacagataataaaaaagaaaagaactattgcagcccaaaacctacatttgggctgttgcgaatgttcaataagtttagtcttatttaatgtaaatattgctgatcatttgaaatgacgcattattcatgagaaatgtgtatcgtaaatcaactgaaattaacgcaaccatttgttatttaaggtttaattatctgtgtgtgatattttattgaatgttttaaatattgtttttattggcattgctataatattggttatcatttgctgaatggattcagtcttaatgagtgggtttttaagggacaggcatagagtaatgatacgtatgcataaccaacatctttactcattatgtcattgaatgttgacgctatgtgtttatgagggagaggtattttcagttgatctggattgttaaattcatataatgcgcctttgctcatgaatggatgccagtatgtagtgggaaattataaatattgaaatagtccaactacttctttattaccaaaaatgagtatctgaattttaatattgcattcttgcgtgattatctcctgagtttgacttgtgattacctttttaaggtatttagcgtaactgtttttgagcgagcatcagaggtaaagataatcttcttgatagtgatgtgggatgttatacgtatggcatcgctgatgtttatggttaccccttatgtgtgctcaggaatcgacaggtaatcactcatactgaacagcgataaaagataaaggtgtgttcatgaattcatgtgattttcgtgtttttctgcaagagttcggtacaacggttcatttgtcattgcctggtagcgtatccgagaaagaacgactgctactcaagctgctgatgcagggaatgtctgtaacagaaatatcacagtacagaaatcgcagtgcaaagacaatttcacatcaaaagaaacagctctttgagaaactggggattcagagcgatattactttctggcgcgatattttctttcagtacaatccggagatcatatccgccacggggagtaatagtcacagatatattaatgataatcactatcaccatatcgtcacgcctgaagccatcagtctggcgttggaaaaccacgaattcaaaccgtggatccaaccggttttctgcgcgcagactggcgtactgacgggctgtgaggtgcttgtccgctgggaacatccacaaacgggaattatcccaccggatcagtttattcctctggcggagtcatccggtcttattgtcataatgacccgccaactgatgaaacagactgcggatattctgatgccggtaaaacatttgctgccggacaatttccatattggcatcaacgtctcggcgggttgttttttggcagcgggatttgaaaaagagtgtctgaacctggttaataaattaggtaacgataaaatcaagctggttctcgagctaacggaacgtaaccctattccggtaacgccagaagccagagcgatatttgacagccttcatcagcacaacattacctttgcgctggatgactttggtacgggttatgcgacctatcgttacttgcaggcgttcccggtcgattttattaagatcgataagtcatttgtgcaaatggcgagtgtcgacgaaatctccggtcatattgtggacaatattgtcgaactagcgcgtaagcctggtctgagtatcgtggcggaaggggtagaaacccaggagcaggcggatttaatgatcggtaaaggcgttcactttttgcagggctatttgtactctccgccagtaccgggtaataaatttatctctgaatgggtaatgaaagcaggtggttgatgtaaaccgctattcacagcgcatcgggaggttggcagcgattaattctcccgatgcagtaaatcctgatagatccccgttaatatgccatttggcgcaaattgttttttaatccactgcgtcacctgacccgtagcagaatgctgagtcgccagtaacatgcgcgaatcctggcgcggattatggatttgtcgggtaaccagcagggattgcgtcatcgcctcacggaccatgtaatccggcaaaaaaccaattccttcacctaaaatctggcactgacatttggtgttgaaatctggcaccagaattgactcctgcccgtgcagcaaccagcccacttttttattaatcgtatgcgcggtgtcctccaccataatattagggtagagacgcagttggctttcggcgatgggttccggcacaaaggctaacgggtgatccggggcgatagcaaaagcccagcgaatcgcgccaatttcagtgtaatcaataccgccgccgtccagtagtgtatcgggtgcgccgatggcgatattggcctgattattaataatcgcatcccagacgccgttatacacttcggtggtgacggtaatctggcaggtaggaaactgctttttcagcacctgtaacaagcgtgcggtgtgtttgggcgtataaagcagctgattaatacaaatgcgcacacgcgcttctatgccctgcgaaatagtatcgattctgcgtttgatggcataaaaatcattcagcaggtcggtagctttgcggaaaaaataacgcccggactccgttaactcaatgctgcgggtactgcgagtgaacagcaccacatccagccccgtctccatacgcttaatggtgtagctaatggcggaagtggttaaacccaactcttctgcggctttactgaagctgccaaaacgcgcagcggtagtaaatgccaacagattctcttcggtaaaaattgagttcattaaaccattctcgccattatctactatgaatttctccagctatgactgtagaggtatcggttaaagatagataatcatttttgaataacttttaatacccgtcgcgtttagtcgtcgcttcgcttaatttttgtccaccatattctgaaattacccccacgcagttacccgccagaaaacccagtaacgtcaccgtccagttcatcccgctggcaaaaaacagcgtcatgccgagaaagccaccgggaataaaggacagtaaccagaaacgcccttgccagaccactaccgccgagaagggtacggtagtaattacgctcgcccagaacgcggacagtccacttacagaggccagccaaccagcagtcagcgcggcgaaaaacgcccacaccatcccggaataattaaccgccagacttctgataaaccccgatttaccgccgcctgcggcataaaaactgcaaaaggcgacgaagccaatggttcctaataattcccatccttgagagagcccgacatgtgaagacactaactgccaaagccctgcacaaataccgacggtgacacccgttgccgtgagtccgttcatcttgttcccctctggttagacatggacgaaagctactcttacatgtgcagactatagagaaataaaacctgattgagtgaaagggtatcgggtcaaagaaacaaatattgcactaccgcacactgcgaaaagattgttgaatattattcaacaaaaaggcgagatacggcgaattaaatttaagcgggttcttttatcagattatcgttgctattctcaattcatcgaaaacagccacaaaaaccaggggaatgtgaatgagtataaaaaatctacctgccgactatttattggctgcacaacagggtgatatcgataaagtaaaaacctgccttgcgctgggtgtcgatattaatacctgcgatcgtcaggggaaaacggcaattacgctggcaagtttatatcagcaatatgcttgcgttcaggcattaattgatgccggagcggatattaataagcaagatcatacctgtttaaatccttttttaattagctgtctgaacgatgatttaacgctactacgaattattttaccggctaaacccgatcttaattgcgtaacccgttttggcggtgtcggcctgacgcctgcctgtgaaaaaggccatttaagtattgtaaaagagcttttggcgcatacggagattaacgttaaccagaccaaccatgtaggctggacgccgctactggaagcgattgtgcttaatgatggtggtattaaacagcaggcgattgtgcagttattgctggaacacggtgccagcccgcatctgaccgataaatatggcaaaacgccactggaactggcgcgggaacggggctttgaagagattgcgcagttactgattgccgcaggtgcataaaccgggaggcttgctatcaacacaccagaaagacggtgtgtgtgggcgctaactgcggatgcggattttctggcgcagcgggggcaaggacaggttgaacaggtctttgccagagcggtaaatatcgcactcccggctcgccagcagttgctgacgctgctttgtgaagagtacgacaatgcgccaaacagttgtcggttggcactcactcactttgatgatctgttccggcatggtgataaggttcagtttgacgatcaaggtattacggttggtcaacatcttcatatagagatgagtcgttgtcggcgttggctgtccccaaccttgcaaatgaccgctgtgaattttcaccttatcgcctggctacagtggcacgacattattcatcagcacctgggggaaaatgaaaccctgtttaattatcgcggcgataatccgttttatcaggcgttaaataaagaattacatattaaacgacgggcagttattcaggccgtaaacgataaacaaaatatcgcctcagcggtcgccagtatgatggggttagggattggccttacgccatcagccgacgattatttaacaggtctggcgcttattttatttattcccgggcatccggcggaaaaatacaaagaggaattttatctcggtctgcaacgcggcaaaaataataccacattattaagtgccataacgctggaagccgcattacaacaacgctgccgggaaaatattcatcgttttattcacaacattatttatgacatccctgggaacgcaactcaggcaatagaaaaaattaaacatattggctccagttccggctgcgacatgctgtatggcatggccgatggttgtgcgctgagccaaacctacggagggaattatgtcagttaaaatagtcattaaaccgaatacctattttgattctgtctcgctgatgtctatctccacgcgtgcaaataaactcgacggcgtcgagcaggcatttgtggcgatggcgaccgaaatgaataaaggcgtgctgaagaatttaggactgctgacgccggagctggagcaggcgaaaaacggcgacctgatgattgtcatcaatggtaaatcgggtgcggacaacgagcagttactggtggagattgaagaactgttcaacaccaaagcgcaaagcggctcgcacgaggcgcgttacgccactattggcagcgccaaaaagcatatcccggaaagtaacctggcggtgatttcggtcaacggtctgtttgccgctcgcgaagcgcgtcaggcgctgcaaaacgatctcaacgtgatgctgttttccgataacgtctcagttgaagatgaactggcgctcaagcaactggcccacgaaaaagggctgctgatgatggggccagactgtggcacggcgattatcaacggcgcggcgctctgttttggtaacgccgtgcgtcgcggcaacatcggtattgttggcgcatccggcaccggcagtcaggagttgagcgtccgcattcatgaatttggcggcggcgtttcgcaactgattggcaccggcgggcgcgacctgagcgagaaaatcggcggcctgatgatgctcgacgccatcgggatgctggaaaacgatccgcaaactgaaatcattgcgcttatctccaaaccgcctgcgcctgcggtggcccgcaaagtgctggaacgtgcgcgcgcctgccgcaagccggtggtcgtctgcttcctcgatcgtggcgaaacgccagtggatgagcaggggctacagtttgcccgcggcaccaaagaggcagcgctaaaagcggtgatgctctccggcgtgaaacaggaaaatctcgacctgcatacgcttaaccagccgttgattgcggatgtgcgtgcgcgtctgcaaccgcagcagaaatacattcgtggcctgttctgcggcggcacgctgtgcgacgaaaccatgttcgcggtgatggaaaaacatggcgatgtctacagcaacattcagcccgatccggaattccgcctgaaagatatcaaccgcagcatcaaacacaccttcctcgactttggcgatgacgacttcaccaatggcaagccgcacccgatgattgaccccaccaaccgcatcagtcgcttgatcgaagaggcgcgcgatccagaagtggcggtgatcgtgatggattttgtgctcggatttggatcgcatgaagatccggtcggctccaccatcgagacgatcaaagaagcgaaagcgatcgccgctgccgaaggacgcgagttgatcattctcgcctatgtgctgggtaccgatcttgatacgccatcgttagaacaacaaagccagatgctgcttgatgccggagtgattctggcgagcagcagcaccaataccggattgctggcgcgtgaatttatctgcaaaggggaggaagcctgatgagccagtcactgtttagccaaccattgaacgttattaacgtcggcatcgccatgtttagcgatgacctgaaaaagcagcatgtagaagtgactcaactcgactggacgccgccggggcagggcaatatgcaggtggtgcaggcgctggataacattgccgattcgccgctggcggacaaaatcgccgccgctaaccagcaggcgctggagcgtattatccagtcgcatccggtgctgattggttttgatcaggcgattaacgtggtgccgggcatgacggcgaaaaccattcttcacgccgggccgccgatcacctgggaaaaaatgtgcggcgcgatgaaaggcgcggtcaccggagcgctggtgttcgaaggactggcgaaagatctcgacgaggcggctgaactggcggcttccggggagatcaccttctcgccgtgtcacgagcacgactgcgtgggatcgatggcgggtgttacctcggcctcgatgtttatgcacatcgtaaaaaacaaaacctacggcaacatcgcttataccaacatgagcgagcagatggcgaagattttgcgtatgggcgctaacgaccagagcgtgattgaccgcctgaactggatgcgtgatgtgcagggaccaatactgcgcgacgcgatgaaaattatcggcgaaatcgatctgcgcttaatgctggcgcaggcgctgcatatgggcgatgagtgccataaccgcaataacgccgggacgacactgctgattcaggcgctgacgccggggattattcaggcgggttattccgtcgagcaacagcgcgaagtgtttgagtttgtcgccagcagcgactacttctccggcccgacgtggatggcgatgtgtaaagcggcgatggatgcggcgcatggcatcgaatacagcaccgtggtcaccaccatggcgcgtaacggcgtcgagttcggcctgcgggtcagcggcctgccggggcaatggtttaccggcccggcgcagcaggtgatcggcccgatgtttgccggttataagccggaagattcggggctggatatcggcgacagcgccatcaccgaaacctacggtattggcggatttgctatggcgaccgcgcccgctatcgtcgcgctggtgggcggcacggtggaagaagctattgatttctcccgtcagatgcgcgaaatcaccctcggtgaaaaccccaacgtcaccattccgctgctcggttttatgggcgtgccgtcggcaatcgacatcacccgcgtgggtagcagcggcattctgccggtgatcaacaccgccatcgcccataaagatgcgggcgtcggcatgattggcgcgggcattgtgcatccaccttttgcctgcttcgagaaagccattcttggctggtgcgaacgttacggcgtctgacctacatgttcatgccggatgcggcgtgaacgccttatccggcctacgaatggcgcaagaatctgtaggcctgataagcgtagcgcatcaggcatttgtcaccattgccggatgcggcgtgaacgccttatccggcctacgaatggcgcaagaatctgtaggcctgataagcgtagcgcatcaggcatttgccaccactgccggatgcggcgtggacgccttatccggcctacgagtggcgcgagaatctgtaggcctgataagcgtagcgcatcaggcatttgtcaccattgccggatgcggcgtgaacgccttatccggcctacgagtggcgcgagaattgtaggcctgataagcgtagcgcatcaggcagtctggcgttggtcataaccccatcaccctctgtagcggacataacaacatgaaagagcttgtggtcgttgccattggtggcaacagcattatcaaagataacgccagccagtcgattgagcatcaggcggaggcggtgaaagccgtcgccgatacggtgctggaaatgctggcttccgattacgacattgtgctgacccacggcaacgggccgcaggtcgggctggatttacgccgtgcggagattgcccacaagcgcgaagggctgcccttaacgccgctggcgaactgtgtggcagatacgcagggcggcatcggctatctgatccaacaggcgctgaataaccggctggcgcgtcacggcgagaagaaagccgtcaccgtggtgactcaggtggaagtggataaaaacgatccaggttttgcccatcccaccaagcccatcggcgcattctttagtgacagccagcgtgacgaattacaaaaggcaaaccctgactggtgttttgttgaagatgccgggcggggctatcgccgcgtggtcgcctcgccggaaccgaaacgtattgtcgaagcacctgccattaaagcgctgatccaacaaggttttgtcgtaattggcgcgggcggcggtggaattccggtagtgcgtactgacgcgggagattaccaaagcgtggacgcggttatcgacaaagatctctctaccgcgctgctggcccgtgaaattcacgccgacattcttgtgatcaccactggcgtcgaaaaagtgtgtattcactttggcaaaccgcagcagcaggcgctcgatcgggtggatattgccaccatgacccgctatatgcaggaagggcatttcccgcccggcagcatgttgccaaaaatcatcgccagcctgacatttttagaacaaggcggcaaagaagtgattatcaccacgccggaatgcctgcctgcggcgctgcgcggcgaaacgggcactcatattattaaaacgtaaggacgtaagatgaaagaaagcaatagccgccgtgaatttctgagccagagcggtaagatggtcaccgccgccgcgctgtttggtacctctgtgccgctcgcccatgcggcggtagctggcaccctaaactgcgaagcgaacaacaccatgaaaatcactgacccgcattactatctcgataacgtgctgctggaaaccggttttgactacgaaaatggcgtggcggtgcagacccgcacggcgcgccagaccgtggagattcaggacggcaaaattgtcgccctgcgcgagaacaagctgcatccggacgccacgctgccgcactatgacgctggcggtaagctgatgctgcccaccacccgcgacatgcatattcatctcgacaaaaccttttacggcgggccgtggcgctcgctcaatcgtccggcaggcaccaccatccaggacatgatcaaactcgagcagaaaatgctgccggaactgcaaccgtacactcaggagcgggcagaaaaactgattgatttattgcagtcgaaaggcaccaccattgcccgcagccactgcaatatcgaaccggtttccggcctgaaaaatctgcaaaatttgcaggcggtgctggcgcgacgtcaggcgggctttgagtgtgaaatcgtcgccttcccgcagcacggtttgctgctgtcgaaatctgaacctttaatgcgtgaagcgatgcaggcgggggcgcattacgtcggcggcctggacccgaccagtgttgatggcgcgatggaaaaatccctcgacaccatgttccagattgcgctggactacgacaaaggcgtcgatattcacctgcacgaaaccactccggcaggcgtggcagccatcaattatatggttgaaacggtagagaaaacgccacagctgaagggcaagctgaccatcagtcacgcctttgcgctggcaacgctcaacgagcaacaggtagatgaactggcgaaccggatggtggtgcaacaaatttctatcgcctcgacggtgccgattggcacgctgcatatgccgctcaaacagttgcacgacaaaggcgtaaaagtgatgactggcactgacagcgttatcgaccactggtcgccttatggtctgggcgacatgctggaaaaagccaatctgtacgcgcagctctatattcgtcctaacgaacagaacctctcccgctcgctgtttttagccactggcgatgtattgccgctgaatgaaaaaggcgagcgtgtatggccaaaagcgcaggatgacgccagctttgtgctggtggacgcctcctgttccgccgaggcggtggcgcgtatctcgccgagaaccgcaacgttccataaagggcaactggtgtgggggagtgtggcaggttgatgcgcatttgaaacgcctgcaacggtgaatagtaagagatttaagccccagggagtggggcaatctgaatatgagtgtgtcggcagaaatggacattatctttgaggaatatgcccttattgacgttgtgtagataactatttgtctacgtgaaaagatcatcagttttgccgattttagtcttttacagatagcaaatatcacacttacaggcgctcgccttatggggaacgttgctgctctgtttcattcaggctcgcggcatgttggggctggatcgggtggtttaaatattggctatattcaatggacgcgttttgccgcgatgacatatcaggcgttgccaaatacacatagctaatcaggagtaaacacaatgaagatcaaagctgttggtgcatattccgctaaacaaccacttgaaccgatggatatcacccggcgtgaaccgggaccgaatgatgtcaaaatcgaaatcgcttactgtggcgtttgccattccgatctccaccaggtccgttccgagtgggcggggacggtttacccctgcgtgccgggtcatgaaattgtggggcgtgtggtagccgttggtgatcaggtagaaaaatatgcgccgggcgatctggtcggtgtcggctgcattgtcgacagttgtaaacattgcgaagagtgtgaagacgggttggaaaactactgtgatcacatgaccggcacctataactcgccgacgccggacgaaccgggccatactctgggcggctactcacaacagatcgtcgttcatgagcgatatgttctgcgtattcgtcacccgcaagagcagctggcggcggtggctcctttgttgtgtgcagggatcaccacgtattcgccgctacgtcactggcaggccgggccgggtaaaaaagtgggcgtggtcggcatcggcggtctgggacatatggggattaagctggcccacgcgatgggggcacatgtggtggcatttaccacttctgaggcaaaacgcgaagcggcaaaagccctgggggccgatgaagttgttaactcacgcaatgccgatgagatggcggctcatctgaagagtttcgatttcattttgaatacagtagctgcgccacataatctcgacgattttaccaccttgctgaagcgtgatggcaccatgacgctggttggtgcgcctgcgacaccgcataaatcgccggaagttttcaacctgatcatgaaacgccgtgcgatagccggttctatgattggcggcattccagaaactcaggagatgctcgatttttgcgccgaacatggcatcgtggctgatatagagatgattcgggccgatcaaattaatgaagcctatgagcgaatgctgcgcggtgatgtgaaatatcgttttgttatcgataatcgcacactaacagactgaaaaaattaataaataccctgtggtttaacatattaacttcgctctccacttaactttttagttaaggagagcgaaataatatcaaagtagcagtaaaacctataacgtaaatttaaattgttaaattaacgccctccagtacacaatacttcacacgttagttatgagcgatttctgatagtgcctggtttaatcagagctttattatctgcgacgtttatttttatttaagagagatcgcgatgatatcattaaaagctccgcacaataatttgatgccatatacgcaacaaagcatacttaatacggttaaaaacaatcagttaccagaggatatcaaaagctccctggtttcctgtgtcgatatattcaaggttttgattaaacaatattatgattatccttatgattgtcgtgatgatttagtcgatgacgacaaactcattcatctcatggctgccgtacgagactgtgagtggtcagacgataacgcactcaccataaatgtgcagtttaatgatttccctggattttatgactggatggattaccctgatcacccggttaagtttgtttttcacatacttgaaaatcaaaaagggacagtttgggtatatgaccaggatgatgcgtttcttgatattaaagcaaacgtgcaggctggacgctttaccgggcttaagaaattagtgcagtttatcgattcagtgcgaacagattgcaaatgtattcttcttgaataccatatgcctttgctgagaattttccctaaagggaaagagtgtatgcatgtggaaaaatggcttcgcgaaatgtcgtctattccggagacagacgcgcccattaagcaggcgcttgcgcatggattattattacacttaaaaaatatctaccctgtttttcctgaatcactggtgatgttattgctctctgttctggacgtaaaaacatacagagatgatgcgcgattaaatgaatggatatctaatagagtgcaggaattaggtgacagatattatcctgtaaataagcacgttaaaatccgctacactctttagttcagaaagggttccacctgcaagttgttattccacctgagagtgaatcgcaatgcaggtaatcatttcatctgtatatctgtatgccaactggcattccatctcttttttcgccgatattttgttgtgatcggcgacacttcgcttaaaaaagcaccagtagtggtttcgcagccatgcggtgtataaaaaatgatctcatgcagatgttttgtgaatgtgttggttgacattcatatgaaaaaaatcataattccatcatgtttgtgtggggtcttttctgtatcttacgcatcgcactcaagcctgacagaaaatatgctgtaaggctcatatcaaaaaccgccattagctcatcaggaagagcagacgacaaccaggattgttgtatggtacggggttcgaggcctcgatggcggtccaacttttcaaaactcttctgaatcagatccccttattatcatccctgcaaagtggaacattgccattgtttggctattcaggatggggcagaccaatgaaaaaagcccacacaggggagagtgggctgaaatgggaagctaaagactcaagtaaacttatcggaaataaggaccacgcattacgggggctatcatcgccgatggccgtgattcggcaaatcaggttgattacgtagagagtaaattatctgctcaccgctgcgtcaccccttcgtaaatcaggcgtagcgcgaatacaccaataattgcaccaataacccgactggcaacgcgttgcatacgcccataagcacgacgcacagcgggcaaagaaaacgcctgactaagaaaaactcgccagataattgatgcgagcacaatccccgcccaggccattaaacgtgcccatgttggtgtttcggcatttaatgttactgagaaaatactgataaaaaataaaacggtttgcgggttagagagatcggtaattaatccgcggcgaaaaaagacataccagggggcgctaatcggttgttgtagtgtgctcatttgcggtgttgactggcggcgcatgctgcaccacgcaaaccataagagataagcgccgccgacgattctgataagcgaaaaaatctcctcacactgcgtaattagcgttgcaagaccaaacaaacccaacccggaataaaatgcatcgcccagcgccacgcccagcccggtcagcacccctgcgcgtcgaccggaagccaggctggtttgtactaccacaaagagattggctcccggattaaaaaaagtaatcacgaacagtcctacggtcaggtaaacggcatgcaaaggatccatagtgatttcatccataaataagtgaactaactgcatcatatttctaccaaaaataatcgggtgcgagagagatcacaaagtgtcttatttccggttactggcgtttatgccctgactgaactaattattaatcaacccaataatgtgggtgggtgatagtgtgataacaactctggagccgtaatatgaaaataatctctaaaatgttagtcggtgcgttagcgttagccgttaccaatgtctatgccgctgaattgatgaccaaagcggaatttgaaaaagttgaatcgcagtatgaaaaaataggtgatatttcaaccagcaatgaaatgtcgactgcagatgcaaaagaagatttgatcaaaaaagcggatgaaaaaggggctgatgtgttggtactgacctccggtcaaactgacaataagatccacggcacggcaaatatttataagaagaagtaattctgaatcctatgtaaacatctccgatgcgtaagtttatcggtgatcatctattgaaatttatgccggataaagcgttcgcgctgcattcggcagttcagcttttcagccgccgccagaacgtcgtccggctgatgcctaaataattcgccgctgctgttttatcgccattaaatttctccagtgcctgttgtggtgtcagtaagcgtggagcgggagttttcgccgactcgcgcgccagttccggcagtagcagttgcataaactgcggcgttaaatccggcgtcggttccacacttaaaaacagcgccagtcgttccatcatattgcgcagttcacgaatattgcctggccagtcgtagtgcagcagcacagtttcacttgcctgtaacccctggcgtaatgcagcagaaaatggggcggagagcgccgccagagacactttcaaaaagctttccgccagcggaagaatatccgccacccgctcgcgcagtggtggcaattgcagacgcaaaatactcagccgataaaacagatcacggcgaaaacgtccttgctgcatatcttcttccagattgcagtgagtggcgctaatgacccgtacatctaccggaacaggctgatgcccgccgacgcgggtgacctctttttcttccagcacccgcagcagccgggtctgcaaaggtagcggcatttcgccaatctcatccagaaacagcgtaccgccgtgggcaatttcgaacagcccggcgcgacctccgcgtcgcgagccggtaaacgccccttcctcatagccaaacagttctgcttccagcagcgattcggcaatcgccccgcagttgacggcaacaaacggatgcgactttttgccctgtcgcgcatcgtggcgggcaaaatattcccgatgaatcgcctgggccgccagctctttgcccgtccccgtttccccctcaatcaacaccgccgcactggagcgggcatacagcaaaatagtctgccgtacttgttccatctgtggtgattgaccgagcatatcgcccagcacgtaacgagtacgcagggcgttgcgggtggcatcgtgagtgttatggcgtaacgacatgcgcgtcatatccagcgcatcgctgaacgcctggcgcacggtggcggcggaatagataaaaattccggtcattccggcttcttctgccaaatcggtaatcagccctgcgccgaccaccgcttcggtgccgttagcttttagctcgttaatctgcccgcgtgcgtcttcctcggtaatgtagctacgttggtcgaggcgcaaattaaaggttttttgaaacgccaccagcgctggaatggtttcctgataggtgacaacgccgatagaagaggtgagttttccggcttttgccagtgcctgtaacacatcgtagccgctcggtttaatcaaaataactggcactgacaggcggcttttcaggtacgcgccgttagagccagccgcgatgatggcgtcacagcgttcgtttgccagtttcttgcggatgtaggtcactgctttttcaaagccaagctgaataggggtaatgttcgccaggtgatcaaactcgaggctgatatcgcgaaacagctcgaacaggcgcgttacagataccgtccagataaccggtttgtcgtcattaagccgtggtggatgtgccatagcgcaccgcaaagttaagaaaccgaatattgggtttagtcttgtttcataattgttgcaatgaaacgcggtgaaacattgcctgaaacgttaactgaaacgcatatttgcggattagttcatgactttatctctaacaaattgaaattaaacatttaattttattaaggcaattgtggcacaccccttgctttgtctttatcaacgcaaataacaagttgataacaaaggatgggctatgtctctacactctccaggtaaagcgtttcgcgctgcactgactaaagaaaatccattgcagattgttggcaccatcaacgctaatcatgcgctgttggcgcagcgtgccggatatcaggcaatttatctttctggcggtggcgtggcggcaggttcgctggggctgcccgatctcggtatttctacccttgatgatgtgctgaccgacattcgccgtatcaccgacgtttgttcgctgccgctgctggtggatgcggatatcggttttggttcttcggcctttaacgtggcgcgcaccgtgaaatcgatgattaaagccggtgcggcaggattgcatattgaagatcaggttggtgcgaaacgctgcggtcatcgtccgaataaagcgatcgtctcgaaagaagagatggtggatcggatccgcgcggcggtggatgcgaaaaccgatcctgattttgtgatcatggcgcgcaccgatgctctggcggtagaggggctggatgcggcgatcgagcgtgcgcaggcctatgttgaagcgggtgccgagatgttgttcccggaggcgattaccgaactcgccatgtaccgccagtttgccgatgcggtgcaggtgccgatcctcgccaacatcaccgaatttggtgccacgccgctgtttaccaccgacgaattacgcagcgcccatgtcgcaatggcgctgtacccactttcagcgttccgcgccatgaaccgcgccgctgaacatgtctacaacgtcctgcgccaggaaggcacgcagaaaagcgtcatcgacaccatgcagacccgcaacgagctgtacgaaagcatcaactactaccagtacgaagagaagctcgacaacctgtttgcccgtagccaggtgaaataaaaaacgcccgttgattgtattcgacagccgatgcctgatgcgtcgctgacgcgacttatcaggcctacgaggtgcactgaactgtaggtcggataagacggatggcgtcgcatccgacaaccgatgcctgatgcgccgctgacgtgacttatcaggcctacggggtgcactgaactgtaggtcggataagacgcatagcgtcgcatccgacaaccgatgcctgatgcgccgctgacgcgacttatcaggcctacggggtgcactgaactgtaggtcggataagacgcatagcgtcgcatccgacaaccgatgcctgatgcgccgctgacgcgacttatcaggcctacggggtgaactgaactgtaggtcggataagacgcatagcgtcgcatccgacaacaatctcgaccctacaaatgataacaatgacgaggacaacatgagcgacacaacgatcctgcaaaacagtacccatgtcattaaaccgaaaaaatctgtggcactttctggcgttccggcgggcaatacggcgctctgcaccgtgggtaaaagtggcaatgacctgcattaccgcggctacgatattcttgatctggcgaaacattgcgaatttgaagaagtggcgcatctgctgatccacggcaaactgccgacccgtgacgaactcgccgcttacaaaacgaaactgaaagccctgcgcggtttaccggctaacgtgcgtaccgtgctggaagccttaccggcggcgtcgcacccgatggatgttatgcgcaccggtgtttccgcgctcggctgcacgctgccagaaaaagaggggcataccgtctctggcgcgcgggatattgccgacaaactgctggcgtcgcttagctcgattctcctttattggtatcactacagccacaacggcgaacgcatccaaccggaaaccgatgacgactccatcggcggtcacttcctgcatctgctgcacggcgaaaagccatcgcaaagctgggaaaaggcgatgcatatctcgctggtgctgtacgccgaacacgagtttaacgcctccacctttaccagtcgggtgattgcgggcaccggctctgatatgtattccgcgattattggcgcgattggcgcactgcgcgggccaaaacacggcggggcgaatgaagtgtcgctggagatccagcaacgctacgaaacgccggacgaagccgaagcagatatccgcaagcgcgtggaaaacaaagaagtggtcattggttttggtcatccggtttacaccatcgctgacccgcgccaccaggtgattaaacgtgtggcgaagcagctctcgcaggaaggcggctcgctgaagatgtacaacatcgccgatcgcctggaaacggtgatgtgggagagcaaaaagatgttccccaatctcgactggttctctgctgtttcctacaacatgatgggcgttcccaccgagatgttcacaccactgtttgttatcgcccgcgtcaccggctgggcggcgcacattatcgaacaacgtcaggacaacaaaattatccgtccttccgccaattatgttggaccggaagaccgcccgtttgtcgcgctggataagcgccagtaaacctctacgaataacaataaggaaacgtacccaatgtcagctcaaatcaacaacatccgcccggaatttgatcgtgaaatcgttgatatcgtcgattacgtcatgaactacgaaatcagctctaaagtggcctacgacaccgcacattactgcctgctcgacacgctcggctgcggtctggaagctctcgaatacccggcctgtaaaaaactgctggggccaattgttcccggcaccgtcgtacccaacggcgtgcgcgtccccggaactcagttccagctcgaccccgtccaggcggcatttaacatcggcgcgatgatccgctggctcgatttcaacgatacctggctggcggcggagtggggccatccttccgacaacctcggcggcattctggcaacggcggactggctttcgcgcaacgcggtcgccagcggcaaagcgccgttgaccatgaaacaggtgctgaccgcaatgatcaaagcccatgaaattcagggctgcatcgcgctggaaaactcctttaaccgcgtcggcctcgaccacgttctgttagtgaaagtggcttccaccgccgtggtcgccgaaatgctcggcctgacccgcgaggaaattctcaacgccgtttcgctggcgtgggtggacggtcagtcgctgcgcacctatcgccatgcgccgaacaccggcacgcgtaaatcctgggcggcgggcgatgccacttcccgcgcggtacgtctggcactgatggcgaaaacgggcgaaatgggttacccgtcagccctgactgcgccggtgtggggcttctacgacgtctcctttaaaggtgaatcgttccgcttccagcgcccgtacggttcctacgttatggaaaatgtgctgttcaaaatctccttcccggcggagttccactcccagacggcagttgaagcagcgatgacgctctatgaacagatgcaggcagcaggcaaaacggcggcggatatcgaaaaagtgaccattcgcacccacgaagcctgtattcgcatcatcgacaaaaaagggccgctcaataacccggcagaccgcgatcactgcattcagtacatggtggcgatcccgctgctattcgggcgcttaacggcggcagattacgaggacaacgttgcgcaagataaacgcattgacgccctgcgcgagaagatcaattgctttgaagatccggcatttaccgctgactaccacgacccggaaaaacgcgccatcgccaatgccattacccttgagttcaccgacggcacacgatttgaagaagtggtggtggagtaccccattggtcatgctcgccgccgtcaggatggtattccgaaactggtcgataaattcaaaatcaatctcgcgcgccagttcccgactcgccaacagcagcgcattctggaggtttctctcgacagagctcgcctggaacagatgccggtcaatgagtatctcgacctgtacgtcatttaagtaaacggcggtaaggcgtaagttcaacaggagagcattatgtcttttagcgaattttatcagcgttcgattaacgaaccggagcagttctgggccgagcaggcccggcgtattgactggcagacgccctttacgcaaacgctcgatcacagcaatccgccgtttgcccgttggttttgtgaaggccgaaccaacttgtgccacaacgccatcgaccgctggctggagaaacagccagaggcgctggcgctgattgccgtctcttcggaaacagaagaagagcgcacctttacctttcgtcagctgcatgacgaagtgaacgcggtggcctcaatgttgcgttcattgggtgtgcagcgcggcgatcgggtgctggtgtatatgccgatgattgccgaagcgcatattactctgctggcctgcgcgcgcattggcgctattcactcggtggtgtttggtggatttgcctcgcacagcgtggcggcgcgaattgatgacgctaaaccggtgctgattgtctcggctgatgccggagcgcgcggtggcaaaatcattccctataaaaaattgctcgacgatgcgataagtcaggcgcagcaccagccacgccatgttttgctggtggatcgcgggctggcgaaaatggcgcgcgtcagcgggcgggatgtcgatttcgcgtcgttgcgccatcaacacatcggcgcgcgggtaccggtggcgtggctggaatccaacgaaacctcctgcattctctacacttccggcacgaccggcaaacctaaaggcgtgcagcgtgacgtcggcggatatgcggtggcgctggcgacctcgatggacaccatttttggcggcaaagcgggcagcgtgttcttttgcgcatcggatatcggctgggtggtggggcattcgtatatcgtttacgcgccgctgctggcggggatggcgactatcgtttacgaaggattgccgacctggccggactgcggcgtgtggtggacaatcgtcgagaaatatcaggttagccggatgttctcagcgccgaccgccattcgcgtgctgaaaaaattccctaccgctgaaattcgcaaacacgatctctcgtcgctggaagtgctctatctggctggagaaccgctggacgagccgaccgccagttgggtgagcaatacgctggatgtgccggtcatcgacaactactggcagaccgaatccggctggccgattatggcgattgctcgcggtctggacgacaggccgacgcgtctgggaagccccggtgtgccgatgtatggctataacgtgcagttgcttaatgaagtcaccggcgaaccgtgtggcgtcaacgagaaagggatgctggtggtggaagggccgctgccgccggggtgtattcagaccatctggggcgacgacggccgctttgtgaagacttactggtcgctgttttcccgcccggtgtacgccacctttgactggggcatccgtgacgctgacggttatcactttattctcgggcgcactgacgatgtaattaacgttgccgggcatcggctggggacgcgcgagattgaagagagtatctccagccatccgggcgttgccgaagtggcggtggttggggtgaaagatgcgctgaaagggcaggtggcggtggcgtttgtcattccgaaagagagcgacagtctggaagatcgtgatgtggcgcactcgcaagagaaggcgattatggcgctggtggacagccagattggcaactttggccgcccggcgcacgtctggtttgtctcgcaattgccaaaaacgcgatccggaaaaatgctgcgccgcacgatccaggcgatttgcgaaggacgcgatcctggagatctgacgaccattgatgatcctgcgtcgttggatcagatccgccaggcgatggaagagtaggttattgtcggatgcgtcgcgcggtgcatccggcactgtgtgccgatgcctgatgcgacgctgacgcgttttatcatgcctacggacctgaaccgtaggtcggataaggcgctcgcgtcgcatccgacaccatgctcagatgcctgatgcgacgctgacgcgtcttatcaggcctacccactgtttttacaccgataatttttcccccacctttttgcactcattcatataaaaaatatatttccccacgaaaacgattgctttttatcttcagatgaatagaatgcggcggattttttgggtttcaaacagcaaaaagggggaatttcgtgtcgcaagataacaactttagccaggggccagtcccgcagtcggcgcggaaaggggtattggcattgacgttcgtcatgctgggattaaccttcttttccgccagtatgtggaccggcggcactctcggaaccggtcttagctatcatgatttcttcctcgcagttctcatcggtaatcttctcctcggtatttacacttcatttctcggttacattggcgcaaaaaccggcctgaccactcatcttcttgctcgcttctcgtttggtgttaaaggctcatggctgccttcactgctactgggcggaactcaggttggctggtttggcgtcggtgtggcgatgtttgccattccggtgggtaaggcaaccgggctggatattaatttgctgattgccgtttccggtttactgatgaccgtcaccgtcttttttggcatttcggcgctgacggttctttcggtgattgcggttccggctatcgcctgcctgggcggttattccgtgtggctggctgttaacggcatgggcggcctggacgcattaaaagcggtcgttcccgcacaaccgttagatttcaatgtcgcgctggcgctggttgtggggtcatttatcagtgcgggtacgctcaccgctgactttgtccggtttggtcgcaatgccaaactggcggtgctggtggcgatggtggcctttttcctcggcaactcgttgatgtttattttcggtgcagcgggcgctgcggcactgggcatggcggatatctctgatgtgatgattgctcagggcctgctgctgcctgcgattgtggtgctggggctgaatatctggaccaccaacgataacgcactctatgcgtcgggtttaggtttcgccaacattaccgggatgtcgagcaaaaccctttcggtaatcaacggtattatcggtacggtctgcgcattatggctgtataacaattttgtcggctggttgaccttcctttcggcagctattcctccagtgggtggcgtgatcatcgccgactatctgatgaaccgtcgccgctatgagcactttgcgaccacgcgtatgatgagtgtcaattgggtggcgattctggcggtcgccttggggattgctgcaggccactggttaccgggaattgttccggtcaacgcggtattaggtggcgcgctgagctatctgatccttaacccgattttgaatcgtaaaacgacagcagcaatgacgcatgtggaggctaacagtgtcgaataacgctttacaaacaattattaacgcccggttaccaggcgaagaggggctgtggcagattcatctgcaggacggaaaaatcagcgccattgatgcgcaatccggcgtgatgcccataactgaaaacagcctggatgccgaacaaggtttagttataccgccgtttgtggagccacatattcacctggacaccacgcaaaccgccggacaaccgaactggaatcagtccggcacgctgtttgaaggcattgaacgctgggccgagcgcaaagcgttattaacccatgacgatgtgaaacaacgcgcatggcaaacgctgaaatggcagattgccaacggcattcagcatgtgcgtacccatgtcgatgtttcggatgcaacgctaactgcgctgaaagcaatgctggaagtgaagcaggaagtcgcgccgtggattgatctgcaaatcgtcgccttccctcaggaagggattttgtcgtatcccaacggtgaagcgttgctggaagaggcgttacgcttaggggcagatgtagtgggggcgattccgcattttgaatttacccgtgaatacggcgtggagtcgctgcataaaaccttcgccctggcgcaaaaatacgaccgtctcatcgacgttcactgtgatgagatcgatgacgagcagtcgcgctttgtcgaaaccgttgctgccctggcgcaccatgaaggcatgggcgcgcgagtcaccgccagccacaccacggcaatgcactcctataacggggcgtatacctcacgcctgttccgcttgctgaaaatgtccggtattaactttgtcgccaacccgctggtcaatattcatctgcaaggacgtttcgatacgtatccaaaacgtcgcggcatcacgcgcgttaaagagatgctggagtccggcattaacgtctgctttggtcacgatgatgtcttcgatccgtggtatccgctgggaacggcgaatatgctgcaagtgctgcatatggggctgcatgtttgccagttgatgggctacgggcagattaacgatggcctgaatttaatcacccaccacagcgcaaggacgttgaatttgcaggattacggcattgccgccggaaacagcgccaacctgattatcctgccggctgaaaatgggtttgatgcgctgcgccgtcaggttccggtacgttattcggtacgtggcggcaaggtgattgccagcacacaaccggcacaaaccaccgtatatctggagcagccagaagccatcgattacaaacgttgaacgactgggttacagcgagcttagtttatgccggatgcggcgtgaacgccttatccggcctacgtagagcactgaactcgtaggcctgataagcgtagcgcatcaggcaattccagccgctgatctgtgtcagcggctaccgtgattcattcccgccaacaaccgcgcattcctccaacgccatgtgcaaaaatgccttcgcagcggctgtctgccagctgtagtttatgccggatgcggcgtgaacgccttatccggcctacgtagagcactgaactcgtaggcctgataagcgtagcgcatcaggcaattccagccgcagacctgtgtcagcggctaccgtgattcatttccgccaacaaccgcgcatttatccaacgccatgtgcaaaaatgccttcgcggcggctgtctgccagctatttttccgccgcaacaaaaccgccgttctctccagtagtggcggggcaagagaaatagctttaagcccgtcatgttgtgtggcaatcgctgctggtaacaatgtggaaagggaagtgcggcgaatcagctccagaaccgcgctaattgagttcgcctcaatgaccacctgtggatgtagccccgctttctcgcagtagtggtcaatttgctctctggtggcaaattccgcgctgagcaggaccagtttttcatcatgcaagcgactcaacgccacctgttcatggacggccagcggatgatgttgcgccacgactaacgctaaactttctgtcagtaaaggaattgcctccagctccggcgaatgcacaggcgcgaaggcaatcccaacgtccaactcgtcgcggcaaagcatatcctcgattttctcctgcgacatttcctgtagctggagcgtgatgctgggatagcgcgcatagaaatccgccattaaggggccgataaagtagctcgtaaaggtgggggtgacggcgatacgcagcgatcctcgcgtcagatcggcaacatcatgaatcgcccgtttacccgcccccagttcctgtaacgcccggctggcgtactgtcgccagacttctcctgcatcagtgagacgaatcgttcgcccgctacggtcaaacagcggcacgcctaaactctcctctaactggcgaatctgctgggaaagcgcaggttgggagacgtgcaacgcactggcggcacgggtgaagctgccatgttcagccacggcaagaaaataattgatatgtcgagagagcattcgcaacctataagtaaatccaatggaactcatcataaatgagacttttaccttatgacaatcggcgagtagtctgcctctcattccagagacagacagaggttaacggtgaaagagattattgatggattccttaaattccagcgcgaggcatttccgaagcgggaagccttgtttaaacagctggcgacacagcaaagcccgcgcacactttttatctcctgctccgacagccgtctggtccctgagctggtgacgcaacgtgagcctggcgatctgttcgttattcgcaacgcgggcaatatcgtcccttcctacgggccggaacccggtggcgtttctgcttcggtggagtatgccgtcgctgcgcttcgggtatctgacattgtgatttgtggtcattccaactgtggcgcgatgaccgccattgccagctgtcagtgcatggaccatatgcctgccgtctcccactggctgcgttatgccgattcagcccgcgtcgttaatgaggcgcgcccgcattccgatttaccgtcaaaagctgcggcgatggtacgtgaaaacgtcattgctcagttggctaatttgcaaactcatccatcggtgcgcctggcgctcgaagaggggcggatcgccctgcacggctgggtctacgacattgaaagcggcagcatcgcagcttttgacggcgcaacccgccagtttgtgccactggccgctaatcctcgcgtttgtgccataccgctacgccaaccgaccgcagcgtaaccttatttttaaaccatcaggagttccaccatgattcagtcacaaattaaccgcaatattcgtcttgatcttgccgatgccattttgctcagcaaagctaaaaaagatctctcatttgccgagattgccgacggcaccggtctggcagaagcctttgtaaccgcggctttgctgggtcagcaggcgcttcctgccgacgccgcccgcctggtcggggcgaagctggatctcgacgaagactccattctactgttgcagatgattccactgcgtggctgcattgatgaccgtattccaactgacccaacgatgtatcgtttctatgaaatgttgcaggtgtacggtacaaccctgaaagcgttggttcatgagaaatttggcgatggcattattagcgcgattaacttcaaactcgacgttaagaaagtggcggacccggaaggtggcgaacgtgcggtcatcaccttagatggtaaatatctgccgaccaaaccgttctgacagccatgcgcaaccatcaaaagacgttcacgatgctgctggtactggtgctgattggtcttaatatgcgaccactgctcacctccgtcgggccactgctaccgcaattgcgccaggcgagcggaatgagctttagcgtggctgccctgttgaccgctctgccggtggttaccatgggcgggctggcgctggccggaagctggcttcatcagcatgtcagcgaacgtcgcagtgtcgccatcagtctgttgctgattgccgtcggtgcattgatgcgtgagctttacccgcaaagtgcgctgctgcttagcagcgcactgcttggtggggtggggatcggcatcattcaggcggtgatgccttcggtgattaaacggcggtttcagcagcgcacgccactggtgatggggctgtggtccgcggctctgatgggcggcggtgggcttggtgccgccataacgccctggttagttcaacatagcgaaacctggtatcaaacactcgcctggtgggcgctgcctgccgttgttgcgctctttgcctggtggtggcaaagcgcccgcgaggtcgcctcttcccacaagacaacaaccactccggttcgcgtggtattcactccccgcgcgtggacgctgggtgtttacttcggtctgattaacggcggttacgccagcctgattgcctggttacccgctttctatattgagattggtgccagcgcgcagtacagcggttccttactggcattgatgacgcttgggcaagccgcaggagctttgctgatgcctgctatggctcgccatcaggatcggcgcaaactgttaatgctggcgctggtgttacaactggtggggttctgcggctttatctggctgccgatgcaattgccggtattgtgggcgatggtgtgtgggttaggtctgggcggcgcgtttccgctctgtttgctgctggcgctcgatcactctgtgcaaccggctattgctggcaagctggtggcgtttatgcagggaatcggttttatcatcgccgggcttgccccgtggttttctggcgtgctgcgtagtatcagcggcaattacctgatggactgggcatttcatgcgctgtgcgtcgttgggctgatgatcataaccctgcgttttgcaccagtacgttttccgcagctgtgggtcaaagaggcatgatgcgacgcttgttcctgcgctttgttcatgccggatgcggctaatgtagatcgctgaacttgtaggcctgataagcgcagcgtatcaggcaatttttataatttaaactgacgattcaactttataatctttgaaataatagtgcttatcccggtcgtttatttcgcgaataacccgacaaggaacgccagccgccacgacgtttggtggaatgtcttttgtgacgatactacccgcgccaataacagaattatccccgatggtgacgcctggattaataaccacatgacttccgatccagacgttattgccaatcgttatcggaaaagagtacatctcgccgttttttctcaattcatggtgtacagggtgtcccgtaacggaaagagtaacgttgggtgcaatcagtacgttatcaccgattgttaccgtgtagtcatcgacaatggttaaattgaaatttgcataaaaattgcggcctatatggatgttggaaccgtaagagaaatagacaggcggttctacccaggcgttttcccctaccgtggcaaacatttctttaatcaggctttctcttttttcaacttctgatggatgcgagtgattaaactcatacattaacgttttcccacgaagtcttttttccggtaagccttcgcacatatcggtaaatagcttgcctgctcttattctttcggtcattggcatgttcaatgcgatcactccgttatgatatgttggtcggataaggcgctcgcgccgcatccgacattgattgcttaagcgacttcattcacctgacgacgcagcagggaaagcgggccggggccgctaagcgtgaacacggaaattaaggtgaagcccagcgccaccagacccagcaccagataagcgccctggaaaccgatgctttcatacatattgcccgccagtacagacataaaaatcatcgccagttgcttaaagaagcagaaacagaccagataaatcgtcgctgaaaaacgcacttcaaactggctggtaatatatttaaagcagcccaccagcaggaacggtacttcaaacatatgcagcgttttcagaataaccacttccagcgctgaggtggcgaacgatgagccaataatacgtacagacataatagtgccagccagcagcagggcgtttttcccaccgatgcgattaatgatcagtggcgcaaagaacataatcgaggcgttaagtaattcgcccattgtcgttacgtagccaaatacccgcgtaccctgttcaccggtagcaaagaacgaagtaaagaaattagcaaactgttggtcaaaaacatcgtaggtgcaggaaacgccaataacatacagtgacaaaaaccacagttttggctgtctgaacagttccagtgccagcttaaggctaaatgccgaatggttggcacctaccgcattggcaaccgtggcagaagagggcgcatccgttttggcgaaaaagagtaaaacggcgaggatgagtgcacagccagagcccagccagaaaacaaactgattattgatggtgaacatgatgccgacaatcgaggcacacagcgcccagccaacacagccaaacatccgcgcgcgaccaaattcgaaattactgcgacggctgactttctcaataaatgcctctactgctggcgcaccggcgttaaaacaaaagcctagataaataccaccaacaatcgatcctactaaaatgttgtattgtaacagtggcccgaagataaaaataaagaacggcgcaaacatcactaacatgccggtaataatccacagcaggtatttgcgcagcccgagtttgtcagaaagcagaccaaacagcggttggaataatagcgagaacagagaaatagcggcaaaaataatacccgtatcacttttgctgatatggttgatgtcatgtagccaaatcgggaaaaacgggaagtaggctcccatgataaaaaagtaaaagaaaaagaataaaccgaacatccaaaagtttgtgttttttaaatagtacataatggatttccttacgcgaaatacgggcagacatggcctgcccggttattattatttttgacaccagaccaactggtaatggtagcgaccggcgctcagctggaattccgccgatactgacgggctccaggagtcgtcgccaccaatccccatatggaaaccgtcgatattcagccatgtgccttcttccgcgtgcagcagatggcgatggctggtttccatcagttgctgttgactgtagcggctgatgttgaactggaagtcgccgcgccactggtgtgggccataattcaattcgcgcgtcccgcagcgcagaccgttttcgctcgggaagacgtacggggtatacatgtctgacaatggcagatcccagcggtcaaaacaggcggcagtaaggcggtcgggatagttttcttgcggccctaatccgagccagtttacccgctctgctacctgcgccagctggcagttcaggccaatccgcgccggatgcggtgtatcgctcgccacttcaacatcaacggtaatcgccatttgaccactaccatcaatccggtaggttttccggctgataaataaggttttcccctgatgctgccacgcgtgagcggtcgtaatcagcaccgcatcagcaagtgtatctgccgtgcactgcaacaacgctgcttcggcctggtaatggcccgccgccttccagcgttcgacccaggcgttagggtcaatgcgggtcgcttcacttacgccaatgtcgttatccagcggtgcacgggtgaactgatcgcgcagcggcgtcagcagttgttttttatcgccaatccacatctgtgaaagaaagcctgactggcggttaaattgccaacgcttattacccagctcgatgcaaaaatccatttcgctggtggtcagatgcgggatggcgtgggacgcggcggggagcgtcacactgaggttttccgccagacgccactgctgccaggcgctgatgtgcccggcttctgaccatgcggtcgcgttcggttgcactacgcgtactgtgagccagagttgcccggcgctctccggctgcggtagttcaggcagttcaatcaactgtttaccttgtggagcgacatccagaggcacttcaccgcttgccagcggcttaccatccagcgccaccatccagtgcaggagctcgttatcgctatgacggaacaggtattcgctggtcacttcgatggtttgcccggataaacggaactggaaaaactgctgctggtgttttgcttccgtcagcgctggatgcggcgtgcggtcggcaaagaccagaccgttcatacagaactggcgatcgttcggcgtatcgccaaaatcaccgccgtaagccgaccacgggttgccgttttcatcatatttaatcagcgactgatccacccagtcccagacgaagccgccctgtaaacggggatactgacgaaacgcctgccagtatttagcgaaaccgccaagactgttacccatcgcgtgggcgtattcgcaaaggatcagcgggcgcgtctctccaggtagcgaaagccattttttgatggaccatttcggcacagccgggaagggctggtcttcatccacgcgcgcgtacatcgggcaaataatatcggtggccgtggtgtcggctccgccgccttcatactgcaccgggcgggaaggatcgacagatttgatccagcgatacagcgcgtcgtgattagcgccgtggcctgattcattccccagcgaccagatgatcacactcgggtgattacgatcgcgctgcaccattcgcgttacgcgttcgctcatcgccggtagccagcgcggatcatcggtcagacgattcattggcaccatgccgtgggtttcaatattggcttcatccaccacatacaggccgtagcggtcgcacagcgtgtaccacagcggatggttcggataatgcgaacagcgcacggcgttaaagttgttctgcttcatcagcaggatatcctgcaccatcgtctgctcatccatgacctgaccatgcagaggatgatgctcgtgacggttaacgcctcgaatcagcaacggcttgccgttcagcagcagcagaccattttcaatccgcacctcgcggaaaccgacatcgcaggcttctgcttcaatcagcgtgccgtcggcggtgtgcagttcaaccaccgcacgatagagattcgggatttcggcgctccacagtttcgggttttcgacgttcagacgtagtgtgacgcgatcggcataaccaccacgctcatcgataatttcaccgccgaaaggcgcggtgccgctggcgacctgcgtttcaccctgccataaagaaactgttacccgtaggtagtcacgcaactcgccgcacatctgaacttcagcctccagtacagcgcggctgaaatcatcattaaagcgagtggcaacatggaaatcgctgatttgtgtagtcggtttatgcagcaacgagacgtcacggaaaatgccgctcatccgccacatatcctgatcttccagataactgccgtcactccagcgcagcaccatcaccgcgaggcggttttctccggcgcgtaaaaatgcgctcaggtcaaattcagacggcaaacgactgtcctggccgtaaccgacccagcgcccgttgcaccacagatgaaacgccgagttaacgccatcaaaaataattcgcgtctggccttcctgtagccagctttcatcaacattaaatgtgagcgagtaacaacccgtcggattctccgtgggaacaaacggcggattgaccgtaatgggataggtcacgttggtgtagatgggcgcatcgtaaccgtgcatctgccagtttgaggggacgacgacagtatcggcctcaggaagatcgcactccagccagctttccggcaccgcttctggtgccggaaaccaggcaaagcgccattcgccattcaggctgcgcaactgttgggaagggcgatcggtgcgggcctcttcgctattacgccagctggcgaaagggggatgtgctgcaaggcgattaagttgggtaacgccagggttttcccagtcacgacgttgtaaaacgacggccagtgaatccgtaatcatggtcatagctgtttcctgtgtgaaattgttatccgctcacaattccacacaacatacgagccggaagcataaagtgtaaagcctggggtgcctaatgagtgagctaactcacattaattgcgttgcgctcactgcccgctttccagtcgggaaacctgtcgtgccagctgcattaatgaatcggccaacgcgcggggagaggcggtttgcgtattgggcgccagggtggtttttcttttcaccagtgagacgggcaacagctgattgcccttcaccgcctggccctgagagagttgcagcaagcggtccacgctggtttgccccagcaggcgaaaatcctgtttgatggtggttaacggcgggatataacatgagctgtcttcggtatcgtcgtatcccactaccgagatatccgcaccaacgcgcagcccggactcggtaatggcgcgcattgcgcccagcgccatctgatcgttggcaaccagcatcgcagtgggaacgatgccctcattcagcatttgcatggtttgttgaaaaccggacatggcactccagtcgccttcccgttccgctatcggctgaatttgattgcgagtgagatatttatgccagccagccagacgcagacgcgccgagacagaacttaatgggcccgctaacagcgcgatttgctggtgacccaatgcgaccagatgctccacgcccagtcgcgtaccgtcttcatgggagaaaataatactgttgatgggtgtctggtcagagacatcaagaaataacgccggaacattagtgcaggcagcttccacagcaatggcatcctggtcatccagcggatagttaatgatcagcccactgacgcgttgcgcgagaagattgtgcaccgccgctttacaggcttcgacgccgcttcgttctaccatcgacaccaccacgctggcacccagttgatcggcgcgagatttaatcgccgcgacaatttgcgacggcgcgtgcagggccagactggaggtggcaacgccaatcagcaacgactgtttgcccgccagttgttgtgccacgcggttgggaatgtaattcagctccgccatcgccgcttccactttttcccgcgttttcgcagaaacgtggctggcctggttcaccacgcgggaaacggtctgataagagacaccggcatactctgcgacatcgtataacgttactggtttcacattcaccaccctgaattgactctcttccgggcgctatcatgccataccgcgaaaggttttgcgccattcgatggtgtcaacgtaaatgcatgccgcttcgccttccggccaccagaatagcctgcgattcaaccccttcttcgatctgttttgctacccgttgtagcgccggaagatgcttttccgctgcctgttcaatggtcattgcgctcgccatatacaccagattcagacagccaatcacccgttgttcactgcgcagcggtacggcgatagaggcgatcttctcctcctgatcccagccgcggtagttctgtccgtaaccctctttgcgcgcgcgcgccagaatggcttccagctttaacggttcccgtgccagttgatagtcatcaccggggcgggaggctaacatttcgattaattccttgcggtcttgttccgggcaaaaggccagccaggtcaggcccgaggcggttttcagaagcggcaaacgtcgcccgaccattgcccggtgaaaggataagcggctgaaacggtgagtggtttcgcgtaccaccattgcatcaacatccagcgtggacacatctgtcggccataccacttcgcgcaacagatcgcccagcagtggggccgccagtgcagaaatccactgttcgtcacgaaatccttcgcttaattgccgcactttgatggtcagtcgaaaactatcatcggaggggctacggcggacatatccctcttcctgcagcgtctccagcagtcgccgcacagtggtgcgatgcaggccgctgagttccgccagcagcccgacgctggcaccgccatcaagtttatttaacatatttaataacattagaccgcgggttaagccgcgcacggttttgtattccgtctgctcattgttctgcatattaattgacatttctatagttaaaacaacgtggtgcacctggtgcacattcgggcatgttttgattgtagccgaaaacacccttcctatactgagcgcacaataaaaaatcatttacatgtttttaacaaaataagttgcgctgtactgtgcgcgcaacgacattttgtccgagtcgtgaggtactgaaatggcaatacaacaccctgacatccagcctgctgttaaccatagcgttcaggtggcgatcgctggtgccggcccggttgggctgatgatggcgaactatctcggccagatgggcattgacgtgctggtggtggagaaactcgataagttgatcgactacccgcgtgcgattggtattgatgacgaggcgctgcgcaccatgcagtcggtcggcctggtcgatgatgttctgccgcacactacgccgtggcacgcgatgcgttttctcaccccgaaaggccgctgttttgctgatattcagccaatgaccgatgaatttggctggccgcgccgtaacgcctttattcagccgcaggtcgatgcggtgatgctggaaggggtgtcgcgttttccgaatgtgcgctgcttgttttcccgcgagctggaggccttcagtcagcaagatgacgaagtgaccttgcacctgaaaacggcagaagggcagcgggaaatagtcaaagcccagtggctggtagcctgtgacggtggagcaagttttgtccgtcgcactctgaatgtgccgtttgaaggtaaaactgcgccaaatcagtggattgtggtagatatcgccaacgatccgttaagtacgccgcatatctatttgtgttgcgatccggtgcgcccgtatgtttctgccgcgctgcctcatgcggtacgtcgctttgaatttatggtgatgccgggagaaaccgaagagcagctgcgtgagccgcaaaatatgcgcaagctgttaagcaaagtgctgcctaatccggacaatgttgaattgattcgccagcgtgtctacacccacaacgcgcgactggcgcaacgtttccgtattgatcgcgtactgctggcgggcgatgccgcgcacatcatgccggtatggcaggggcagggctataacagtggtatgcgcgacgcctttaacctcgcatggaaactggcgttggttatccaggggaaagcccgcgatgcgctgctcgatacctatcaacaagaacgtcgcgatcacgccaaagcgatgattgacctgtccgtgacggcgggcaacgtgctggctccgccgaaacgctggcagggtacgttacgtgacggcgtttcctggctgttgaattatctgccgccagtaaaacgctacttcctcgaaatgcgcttcaagccgatgccgcaatattacggcggtgcgctgatgcgtgagggcgaagcgaagcactctccggtcggcaagatgtttattcagccgaaagtcacgctggaaaacggcgacgtgacgctgctcgataacgcgatcggcgcgaacttcgcggtaattggctggggatgcaatccactgtgggggatgagcgacgagcaaatccagcagtggcgcgcgttgggcacacgcttcattcaggtggtgccggaagtgcaaattcataccgcacaggataaccacgacggcgtactacgcgtgggcgatacgcaaggtcgcctgcgtagctggttcgcgcaacacaatgcttcgctggtggtgatgcgcccggatcgctttgttgccgccaccgccattccgcaaaccctgggcaagaccctgaataaactggcgtcggtgatgacgctgacccgccctgatgccgacgtttctgtcgaaaaggtagcctgatatgcacgcttatcttcactgtctttcccactcgccgctggtggggtatgtcgacccggcgcaagaggtgctcgatgaggtcaatggcgtgattgccagcgcccgcgagcgtattgcggcattctcccctgaactggtggtgctgtttgcgccagatcactacaacggctttttctatgacgtgatgccaccgttctgtttaggcgttggagcgacggcaattggtgatttcggcagtgcggcaggagagctgcccgtgcctgtggagctggcggaggcctgtgcgcatgccgtcatgaagagcgggatcgatcttgccgtttcttactgtatgcaggtggaccacgggttcgcccagccgctggagttcctgctcggtgggctggataaggtgccagttctgcctgtgttcatcaacggtgtcgccacgccgctgcccggtttccagcgtacccgcatgttgggtgaagccattggacgtttcaccagcactctcaataaacgcgtgctgttcctgggttccggtgggctttcccatcagccgccggtgcccgaactggcgaaagccgatgcccatatgcgcgaccgtctgttggggagcgggaaagatttacccgccagtgagcgcgaattgcgtcagcaacgggtgattagcgccgctgagaagtttgttgaggatcagagaacgctgcatccgctcaacccgatttgggataaccagttcatgactttgctggagcagggacgcatacaggaactggatgccgtcagtaacgaagagctttccgccattgccggaaagtcgacacatgaaatcaaaacctgggtcgccgcttttgccgctatttctgcgtttggcaactggcgtagcgaagggcgttattaccgcccaatcccggagtggattgccggatttggctcgttaagcgccagaacagagaactgaatatgcaggagaagatgatgagttatcagccacaaaccgaagccgccaccagccgttttctgaatgtagaagaagcgggtaaaacgctgcgcatccattttaatgactgcggacaaggcgacgaaaccgttgtcctgctgcatggttccggcccgggtgctactggctgggcgaacttcagccgcaatatcgatccgctggtagaggcgggctatcgggtgatcctgctggattgtccgggttggggcaagagcgattcggtcgttaatagtggttcgcgatcggatcttaatgcacgaatcctgaaaagcgtggtggatcaactggatatcgccaaaatccacctgctgggcaactcgatggggggccatagttctgtggcgttcacccttaaatggccggagcgcgtcggcaaactggtgctgatgggcggcggtacgggcggcatgagtttgtttacgccgatgccaaccgaaggtattaagcgactgaatcagctttatcgtcagccgactatcgaaaacctgaagctgatgatggatatcttcgtttttgataccagcgatttgaccgacgccctgtttgaagcgcgcctgaataatatgctgtcgcgccgcgatcacctggaaaacttcgttaagagcctggaagctaatccgaaacagttcccggattttggcccacgtctggcggaaatcaaagcgcaaaccctgattgtctgggggcgcaacgaccgctttgtgccgatggatgcgggtctgcgtctgctgtccggcattgccggttctgaactgcatatcttccgcgactgtggtcactgggcgcagtgggaacatgccgacgctttcaatcaactggtgctgaatttcctcgcacgcccttaaggaatggtcatgacgaagcatactcttgagcaactggcggcggatttacgccgcgccgcagagcagggcgaagcgattgcaccgctgcgcgatctgattggtatcgataacgctgaagcggcttacgccattcagcacataaatgtgcaacatgacgttgcgcaggggcgtcgcgtggtagggcgtaaagtgggcctgacacatccgaaagtgcaacaacaactgggcgttgatcaaccggattttgggacgttatttgccgacatgtgttatggcgataacgaaatcattcctttttcccgtgttctgcaaccccgcattgaagcggagatcgcactggtgttgaaccgcgatttgcccgcaaccgatatcaccttcgacgaattgtataacgccattgaatgggtacttccggcgctggaagtggtggggagccgcattcgcgactggtcgattcagtttgtcgataccgtggcagataacgcctcctgtggggtgtatgtcatcggcggtccggcgcaacgtccggcggggttagacctgaaaaactgcgccatgaagatgacgcgtaataacgaagaggtttctagcgggcgcggcagcgaatgcctgggacatccgcttaatgcggccgtctggctggcacgcaaaatggccagtctgggtgaaccgctgcgcaccggagatatcattcttaccggggcattaggtccgatggtggcggtgaatgcgggcgatcgttttgaagcccatattgaaggcataggttcagttgctgcgacattttcaagcgcagccccaaaaggaagtctgtcatgagtaagcgtaaagtcgccattatcggttctggcaacattggtaccgatctgatgattaaaattttgcgtcacggtcagcatctggagatggcggtgatggttggcattgatcctcagtccgacggtctggcgcgcgccagacgtatgggcgtcgccaccacccatgaaggggtgatcggactgatgaacatgcctgaatttgctgatatcgacattgtatttgatgcgaccagcgccggtgctcatgtgaaaaacgatgccgctttacgcgaagcgaaaccggatattcgcttaattgacctgacgcctgctgccatcggcccttactgcgtgccggtggttaacctcgaggcgaacgtcgatcaactgaacgtcaacatggtcacctgcggcggccaggccaccattccaatggtggcggcagtttcacgcgtggcgcgtgttcattacgccgaaattatcgcttctatcgccagtaaatctgccggacctggcacgcgtgccaatatcgatgaatttacggaaaccacttcccgagccattgaagtggtgggcggcgcggcaaaagggaaggcgattattgtgcttaacccagcagagccaccgttgatgatgcgtgacacggtgtatgtattgagcgacgaagcttcacaagatgatatcgaagcctcaatcaatgaaatggctgaggcggtgcaggcttacgtaccgggttatcgcctgaaacagcgcgtgcagtttgaagttatcccgcaggataaaccggtcaatttaccgggcgtggggcaattctccggactgaaaacagcggtctggctggaagtcgaaggcgcagcgcattatctgcctgcctatgcgggcaacctcgacattatgacttccagtgcgctggcgacagcggaaaaaatggcccagtcactggcgcgcaaggcaggagaagcggcatgaacggtaaaaaactttatatctcggacgtcacattgcgtgacggtatgcacgccattcgtcatcagtattcgctggaaaacgttcgccagattgccaaagcactggacgatgcccgcgtggattcgattgaagtggcccacggcgacggtttgcaaggttccagctttaactatggtttcggcgcacatagcgaccttgaatggattgaagcggcggcggatgtggtgaagcacgccaaaatcgcgacgttgttgctgccaggaatcggcactattcacgatctgaaaaatgcctggcaggctggcgcgcgggtggttcgtgtggcaacgcactgtaccgaagctgatgtttccgcccagcatattcagtatgcccgcgagctcggaatggacaccgttggttttctgatgatgagccatatgaccacgccggagaatctcgccaagcaggcaaagctgatggaaggctacggtgcgacctgtatttatgtggtggattctggcggtgcgatgaacatgagcgatatccgtgaccgtttccgcgccctgaaagcagagctgaaaccagaaacgcaaactggcatgcacgctcaccataacctgagtcttggcgtggcgaactctatcgcggcggtggaagagggctgcgaccgaatcgacgccagcctcgcgggaatgggcgcgggcgcaggtaacgcaccgctggaagtgtttattgccgccgcggataaactgggctggcagcatgggaccgatctctatgcgttaatggatgccgccgacgacctggtgcgtccgttgcaggatcgaccggtacgagtcgatcgcgaaacgctggcgctgggatacgctggtgtttactcgagcttcctgcgtcactgtgaaacggcggcggcgcgttatggcttaagtgcggtggatattctcgttgagctgggcaaacgccggatggttggcggccaggaggatatgatcgttgacgtggcgctggatctgcgcaacaacaaataatgatgactgccgagaacgtgcattttgtatgcccatcccagcacgactgccggatgcggcgtgaacgccttatccggcctacggatggcgtgagaatttgtaggtctgataagacgcgttagcgtcgcatcaggcatctgcgcacgactgccggatgcggcgtgaacgccttatccggcctacggatggcgcgggaatttgtaggcctgataagacgcgttagcgtcgcatcaggcatctgcgcacgactgccggatgcggcgtgaacgccttatccggcctacgggtggcgcgagaatttgtaggcctgataagacgcgttagcgtcgcatcaggcatctgcgcacgactgccggatgcggcgtaaacgccttatccggcctacggatggcgcgggaatttgtaggcctgataagacgcgttagcgtcgcatcaggcatctgcacacgactgccggatgcgataaacgtcttgtccggcctacatttcgcccgtaggcagtcattaaatagttctgattacgcggctggcaatgtatcagtcgcgattcacctgcactcgcaacgaggttcatcttatgtcgactcgtaccccttcatcatcttcatcccgcctgatgctgaccatcgggctttgttttttggtcgctctgatggaagggctggatcttcaggcggctggcattgcggcgggtggcatcgcccaggctttcgcactcgataaaatgcaaatgggctggatatttagcgccggaatactcggtttgctacccggcgcgttggttggcggaatgctggcggaccgttatggtcgcaagcgcattttgattggctcagttgcgctgtttggtttgttctcactggcaacggcgattgcctgggatttcccctcactggtctttgcgcggctgatgaccggtgtcgggctgggggcggcgttgccgaatcttatcgccctgacgtctgaagccgcgggtccacgttttcgtgggacggcagtgagcctgatgtattgcggtgttcccattggcgcggcgctggcggcgacactgggtttcgcgggggcaaacttagcatggcaaacggtgttttgggtaggtggtgtggtgccgttgattctggtgccgctattaatgcgctggctgccggagtcggcggttttcgctggcgaaaaacagtctgcgccaccactgcgtgccttatttgcgccagaaacggcaaccgcgacgctgctgctgtggttgtgttatttcttcactctgctggtggtctacatgttgatcaactggctaccgctacttttggtggagcaaggattccagccatcgcaggcggcaggggtgatgtttgccctgcaaatgggggcggcaagcgggacgttaatgttgggcgcattgatggataagctgcgtccagtaaccatgtcgctactgatttatagcggcatgttagcttcgctgctggcgcttggaacggtgtcgtcatttaacggtatgttgctggcgggatttgtcgcggggttgtttgcgacaggtgggcaaagcgttttgtatgccctggcaccgttgttttacagttcgcagatccgcgcaacaggtgtgggaacagccgtggcggtagggcgtctgggggctatgagcggtccgttactggccgggaaaatgctggcattaggcactggcacggtcggcgtaatggccgcttctgcaccgggtattcttgttgctgggttggcggtgtttattttgatgagccggagatcacgaatacagccgtgcgccgatgcctgacgtgccttattaggcaggggcgaaagggacttcaccccaatacacctacggcgtttacaggtatactcgctaaaaattattcagcgggtttggaaacaaagatggcaaaacttaccttacaagagcagttgctcaaagcaggattagtcaccagcaaaaaagcggcgaaggtggagagaacggcgaaaaaatcgcgcgttcaggcgcgtgaagctcgggcggcggtagaagaaaataaaaaggcacagcttgagcgtgataaacagcttagcgaacagcaaaaacaagcggcgttggcgaaagaatataaagctcaggtgaagcagcttattgaaatgaaccgaatcaccattgccaatggcgatattggttttaacttcactgacggcaatctgattaagaagatttttgtcgataagctcacacaggcgcagttgattaatggtcgtctggcgattgcccgcttgttggtcgataacaatagcgaaggtgaatacgccattattcccgccagcgttgccgataaaattgctcagcgcgatgccagcagtatagtgttgcacagcgcgctcagcgccgaagagcaggatgaagacgacccgtatgccgacttcaaagtgcctgatgatttgatgtggtaaacatagataagtcgtgcgcagatgcctgatgcgacgctatgcgcgtcttatcaggcctacggtttatgggcgaagtgtagaccggataaggcgttcacgccgcatccggcagtcgtgcgccatgcctgatgcgacgctttgcgcgtcttatcaggcctacggcttacgggcgaagtgtaggccggataaggcgttcacgccgcatccggcagtcgtgctattatcaacgcatattcagtttattggcgtggtaggcaatatgctcgccaataaaactggagacaaaataatagctgtgatcataaccctcgtgataacggattaacgtcttgatattcatctcctggcagatcttttcaagatttggagtccgcagctgttctgcgtaaaaatcatcactcaacccctgatcaaccatgatttccgcaacgcgttgaccttgtgaaataagactcaccgggtcgtaatccaaccaggcatctttattttcagcaagatatgcagcaaaggcttgctgtccccacggcacttgcgatggggagacaatgggcgaaaacgccgagacgctgacatattcatctgggttacgtaacgccagcaccagcgcgcccagcccgcccatagaatgaccagagatagactttttggccgttgccggaaaatgatgcatcactaaatccggcagctcgttgcggatatagtcatacattttgtaatgttcattccacggcgcttgcgtcgcgttcaggtaaaacccggcaccttgcccgagatcgtaacggtcagcatctgcgacatgactgcctcgcggactggtgtccggcgcaacaacaataatgttgtgctcagccgcgtaacgctgcatccccgatttagtaatgaaattctgctcgttgcaggtcaggcctgaaagccagtacagcaccggcaatttttcattcgcggcttttggtgggagatagacgccgacattcatttcacatttcagtgattgggaataatgccgatacatattttgccagccgccaaagctgacatgtttttcaatgagttccatcagtcattatctcagggttaatcccccggacggctgcccggggagagtattaagaacccccgcctgaagtggacggggtaaacctgcgggaaatcagtaacgaattacggttcgaatggatttgccttcatgcatcaggtcgaaggcgtcattaatttcatccaggctcatggtatgcgtgacaaacggttccagatcgatatcacctttcatcgcatcttcaaccatgcccggtaactgggaacgacctttcacgccgccaaacgcggaacctttccatacgcgaccagtgaccaactggaatggacgggtggagatttcctgaccggcaaccgcgaccccgatgatcaccgactgaccccagccgcggtgcgcactttccagcgccgcacgcatcacgttgacgttaccgatgcattcaaaggtatggtcgataccccatttgttgatatccaacaggacatcttttatcggtttgtcgtagtcattcgggttaatgcagtcggtagcaccgaagcgacgcgccagatcgaatttcttcgggttggtatcgatagcgataatccgacccgctttcgcctgacgcgcgccctgaaccactgccagaccaatcgcgccaagaccaaacacggcaacagaatcacctggctggactttagctgtgttgtgtaccgcgccaataccggtggtcacgccacagcccagcaggcagacgtgttcatggtttgcttctggattaatttttgccagagacacttccgcgactacggtgtattcactgaatgtagagcaccccatgtagtgataaagcggctgcccgttgtaagaaaaacgggtggtgccgtctggcatcaggcctttaccctgggtttcgcgaaccgcaacacagaggttagttttgccagaacgacagaactcacactcgccgcactccgcggtgtaaagcgggatcacatggtcgccaggtttgacgctggttacgccttcaccgacttcaaccacaacgccggccccttcgtgaccgagaaccaccgggaatacaccttccgggtcatcgccggagagggtaaatgcgtcggtatggcaaacgccggtatgggtgactttaattagcacttcaccttttttcggtggtgcaacgtcaatttcaacgatttccagcggtttaccgggagcaaatgcaacggcagcacgtgatttcatctctcgctcttcctcaatatggtaatagattcagctatttaagataggcacgaaccagttcaatagtgtcgtcaacggattggctgacttcgcggctgtagcagtcatttcggtcaaacgtttcccggatatggctttcaagcacttctgccatcagcccattagccgcgccccgaacggcagcgatctgttggagtatggcacggcattcggcatcaccctccagcgaccgttccagagcatcaatctgcccccgaatacgacgaactcgagtaaggacctttttcttctcttccggagtactgggcatttcgcacctcatcatctgcatgcaatatactataggggggtattctatatgtcaatgcatacccccctatagtatataacactggagaataaaatttatccggtgaatgtggtcggaaaacaaagaggaaaggggggggggctaatcggcagggaaggccgccccggatagcgggcggcagaaggaatcagaatttccaggtcagacgggctgcaagttgcagaccgttaaaatcatcggttggggtgtcgtaccacactttacctgccgtcagcccgagattaagttgctcagtcagcggttgaatacgttgcagactgacgctcttcatgctgccgtagcgtgtttctggcgtccagtcataggtgtaagcacctgttccgcggcttagccatagttgcgtataaccagtgccgcgcgggtcattcagacgcacggaaatcatattgctataactaccacctgcatcgctggagtcataatgggtatagcggtagctggtgatcaccgggccagtatagagtgatacgccgccttgccaggcatcgacttcgacatcatcgtaatatttagtgtagcgataaccggtcgtgaaaagcgtttttggtaacagggccaggttaatatcctgacgaaaatcctggcgggcaaagaccggcgtattatccgcaaaggcaatacccgttcgggttgtcagccagttattccatttataccagaccgcaccctgaccgcgagtggcattgaaatgttcagtttcataatcacgacgcccctgggaaagattaaaaagcagcgttgcgttttcaactttcgccaccagttcagcatacgctaaattacggttgccatgatcgccagaataatcggtaaaatcgtagcccgcggtaatggaagttaacccggcataagcgggcaatgcgctaaaaatggccgccgctaataacgtccgttttatcattttaatctcctgtacggataagttcttgtcggagtgaataagttccggtaggtaaattacgttctacaatcacgcgcgggccaagttgcgtgttcggggaaataattcgcccaggcaaaataataacttgtacgccaaggcgtgaacgctgcccgatataacaacctaatttatcgcatccggtagcgataattccctctggagttcgaacagacacgggctgttcatccagacgatgattactggtacgtacttgtgcgcctaaatatgcctggtttgcaactaccgagtcggcaataaaacattgcggaccaatcgttgcttccgcttcaataaccgcatttttaatctcggtggcaaaaccaatttttacgccattgctgattattgtgccaggacgaataaacgcataattactagactggccccctgaatctccagacaaccaatatcacttaaataagtgatagtcttaatactagtttttagactagtcattggagaacagatgattgatgtcttagggccggagaaacgcagacggcgtaccacacaggaaaagatcgcaattgttcagcagagctttgaaccggggatgacggtctccctcgttgcccggcaacatggtgtagcagccagccagttatttctctggcgtaagcaataccaggaaggaagtcttactgctgtcgccgccggagaacaggttgttcctgcctctgaacttgctgccgccatgaagcagattaaagaactccagcgcctgctcggcaagaaaacgatggaaaatgaactcctcaaagaagccgttgaatatggacgggcaaaaaagtggatagcgcacgcgcccttattgcccggggatggggagtaagcttagtcagccgttgtctccgggtgtcgcgtgcgcagttgcacgtcattctcagacgaaccgatgactggatggatggccgccgcagtcgtcacactgatgatacggatgtgcttctccgtatacaccatgttatcggagagctgccaacgtatggttatcgtcgggtatgggcgctgcttcgcagacaggcagaacttgatggtatgcctgcgatcaatgccaaacgtgtttaccggatcatgcgccagaatgcgctgttgcttgagcgaaaacctgctgtaccgccatcgaaacgggcacatacaggcagagtggccgtgaaagaaagcaatcagcgatggtgctctgacgggttcgagttctgctgtgataacggagagagactgcgtgtcacgttcgcgctggactgctgtgatcgtgaggcactgcactgggcggtcactaccggcggcttcaacagtgaaacagtacaggacgtcatgctgggagcggtggaacgccgcttcggcaacgatcttccgtcgtctccagtggagtggctgacggataatggttcatgctaccgggctaatgaaacacgccagttcgcccggatgttgggacttgaaccgaagaacacggcggtgcggagtccggagagtaacggaatagcagagagcttcgtgaaaacgataaagcgtgactacatcagtatcatgcccaaaccagacgggttaacggcagcaaagaaccttgcagaggcgttcgagcattataacgaatggcatccgcatagtgcgctgggttatcgctcgccacgggaatatctgcggcagcgggcttgtaatgggttaagtgataacagatgtctggaaatataggggcaaatccaattacctatcaggcagtttgcgccaatcactaccggaccctgaataacggcaccatgacaaatacgggtattcgcgccgataacaacttcacctgcagtttcatcaataattacctggtctgcaatctgaatatttttctctttaacattaagcttcagatagtttttcagttcctgtgacagaaggttgggaataagcggttgacgcttccaccagtgcggaatagcgggtgggtttgtcgcgctgaggttcgcgtccagtaaaaaaggcaataagtccataaataatccagatggcataagctaataatacatacacaacggaaagcggcgctaaaggcaccaacaaccagcaacgatgaaaccaggcgctaaaagcaccaataacacaaactacgccgacccagataagcggaaacattgccaacaccactccatgcggcccggtggtgatgaattcattaaaccaggtagtgagataaatcccaacgccataaagcacaaccaacagcataggaaatatactgaagataccgaagcggctaaataaaagtcttttatgcaggcgcatacagaccgcgtatcccacaatccaacgccgccagcgacgccactcctcacgcgggctgttgcattcctgtgggtatacgatgcagcgattcgcctgccgaatacggtagccgtttgccaccaatgtccaggtgagatcaaggtcttcgactttagtacgatccgagaaaccgaacttacgcaatacatcagtacggaacatcccgcaggcaccgctgataataaacggtgcgccacccaggagctgctgtagcgtgcgcttcataacaatcatcggcaactttacggtcgcgcggatgtgcggtaacagacccgcgcctttcaacgcagtagagggaatgccgcctacggcatcggcaccgcgctcaatttctgccagcatatagcccattccgtcttgatcgggcggaacataggtgtcggcatcacttaaaaaaacctggtcgcaggtggcgtaattgaggccattcatcagcgcaccacctttaccggtatttttttgcgtgacggcaacaaagcggtcgccccatttgcgtttgacttccgccatgaccgcttcggtattgtccgtggagccgtcgttaacgcaaattacccggcaaaaataagggttacgcagtagattatccagtgactgcgccagacacgggccttcgttatacgcaggtataatggcgtcaatacagcctttcttttgactgggtttacgtcttagcgtacttaaaaaccatagcaacattgctatggacatacagataaatatccaggttttcatgcaatttgctcaaagaatcattttatgaattacaaagccttcacccagatcgctattgacctgttgtccgcgaaattgtgcaactgcacgcaggcgatcatgacgcatataatcgcgtcgttcctagcttttatgtttttttaatgcagcaagtttgactgtgaaatattcttctttaacggattcaaaaacctgaggcataaatgaaagccaggtacttggggtttcgtagccgagaatttgcggaatagttcggcaggcaaccattgaagcttgataaacagcaagatgatcctgatggcggtcggcatcatgcatggtatatacccgcatgatttcaacatcagaaggaatttgatttttaatgatgtcttccagggcggaaatcatatcattgagctgtaaatgagcgcgggtgtcagcaaaattaagatgaatagtttggtggcaccctaatatctttagggcgttgcgcgattcttcatggcgatcgattattccatctgtgccagagttgccggtagtcatcaccacggctgcgatataaattcctttttgcgcaagacgagcaagcgatgcgccacagcctaattctatatcgtcaggatgtgcgccaatagcaaggataccctttcttttatttgccgaagaaaggagggctgaatctaaaaccttatccacttaatgacactccattttatttattatactacaagcacaacgatgcactcagagacgtaatctctggcgcagccagatgttaatttataaatgttaaatgttgctaataactgaaaagcaagggctttcagacccgtgggttcgactgggtaatgtttctatgcaattcatatgttaagtgtttgtatgtttggtatgtatagttattttgttttatacattgtatttagatgtgatttagtttgtcaattaattgcatttaaaaaatatgttctgtgaacaagcattgtttatatacattatgtgaatgtaatatgcgagtgattgagaatgatacagtgatatatacaatgcgaatataatagttttattatatgtattgatattgatagaaataatgaagtaataaatctcgtaatgtggttgtttatgcatcactaaaatgaagtgtagtaattttcccaattgttagaacggagtaattgcatatttaatctttccttagccgtttttttgctaagaataaaatcatctgtgcgataacgactaattcttttaatgaatgtttttattcctgaatactgctcccataacaagacaggggagcagacaatcatggcaatttcatcgcgtaacacacttcttgccgcactggcattcatcgcttttcaggcacaggcggtgaacgtcaccgtggcgtatcaaacctcagccgaaccggcgaaagtggctcaggccgacaacacctttgctaaagaaagcggagcaaccgtggactggcgtaagtttgacagcggagccagcatcgtgcgggcgctggcttcaggcgacgtgcaaatcggcaacctcggttccagcccgttagcggttgcagccagccaacaggtgccgattgaagtcttcttgctggcgtcaaaactgggtaactccgaagcgctggtggtaaagaaaactatcagcaaaccggaagatctgattggcaaacgcatcgccgtaccgtttatctccaccacccactacagcctgctggcggcactgaaacactggggcattaaacccgggcaagtggagattgtgaacctgcagccgcccgcgattatcgctgcctggcagcggggagatattgatggtgcttatgtctgggcaccggcggttaacgccctggaaaaagacggcaaggtgttgaccgattctgaacaggtcgggcagtggggcgcgccaacgctggacgtctgggtggtgcgcaaagattttgccgagaaacatcctgaggtcgtgaaagcgttcgctaaaagcgccatcgatgctcagcaaccgtacattgctaacccagacgtgtggctgaaacagccggaaaacatcagcaaactggcgcgtttaagcggcgtgcctgaaggtgacgttccggggctggtgaaggggaatacctatctgacgccgcagcaacaaacggcagaactgaccggaccggtgaacaaagcgatcatcgacaccgcgcagtttttgaaagagcagggcaaggtcccggctgtagcgaatgattacagccagtacgttacctcgcgcttcgtgcaataaaaggaggcgcagatgctgcaaatctctcatctttacgccgattatggcggcaaaccggcactggaagatatcaacctgacgctggaaagcggcgagctactggtggtgctggggccgtccggctgcggtaaaaccaccctgctgaatctgattgccggttttgtgccttatcagcatggcagcattcaactggcgggtaagcgtattgagggaccgggagcagagcgtggcgtagtttttcagaatgaagggctactaccgtggcgcaatgtacaggacaacgtggcgttcggcctgcaattggcaggtatagagaaaatgcagcgactggaaatcgcgcaccagatgctgaaaaaagtggggctggaaggcgcagaaaaacgctacatctggcagctttccggtggtcaacgtcagcgggtggggattgctcgtgcgctggcggcgaatccccagctgttattactcgacgaaccgtttggtgcgctggacgccttcacccgcgaccagatgcaaaccctgctgctgaaactctggcaggagacgggcaagcaggtgctgttgattacccacgatatagaagaagcggtgtttatggcgactgaactggttctgctttcatccggccctggccgtgtgctggagcggctgccgctcaactttgctcgccgctttgttgcgggagagtcgagccgcagcatcaagtccgatccacaattcatcgccatgcgcgaatatgttttaagccgcgtatttgagcaacgggaggcgttctcatgagtgtgctcattaatgaaaaactgcattcgcggcggctgaaatggcgctggccgctctcgcgtcaggtgaccttaagcattggcacgttagcggttttactcaccgtatggtggacggtggcgacgctgcaactgattagcccgctatttttgccgccgccgcaacaggtactggaaaaactactcaccattgccggaccgcaaggctttatggacgccacgctgtggcagcatctggcagccagtctgacgcgcattatgctggcgctatttgcagcggtgttgttcggtattccggtcgggatcgcgatgggacttagccctacggtacgcggcattctggatccgataatcgagctttatcgtccggtgccgccgctggcttatttgccgctgatggtgatctggtttggtattggtgaaacctcgaagatcttactgatctatttagcgatttttgcaccggtggcgatgtcggcgctggcgggggtgaaaagcgtgcagcaggttcgcattcgtgccgcccagtcgctgggtgccagccgtgcgcaggtgctgtggtttgtcattttgcccggtgcgctgccggaaatcctcaccggattacgtattggtctgggggtgggctggtctacgctggtggcggcggagctgattgccgcgacgcgcggtttaggatttatggttcagtcagcgggtgaatttctcgcaactgacgtggtgctggcggggatcgcggtgattgcgattatcgcctttcttttagaactgggtctgcgcgcgttacagcgccgcctgacgccctggcatggagaagtacaatgagtgaacgtctgagcattaccccgctggggccgtatatcggcgcacaaatttcgggtgccgacctgacgcgcccgttaagcgataatcagtttgaacagctttaccatgcggtgctgcgccatcaggtggtgtttctacgcgatcaagctattacgccgcagcagcaacgcgcgctggcccagcgttttggcgaattgcatattcaccctgtttacccgcatgccgaaggggttgacgagatcatcgtgctggatacccataacgataatccgccagataacgacaactggcataccgatgtgacatttattgaaacgccacccgcaggggcgattctggcagctaaagagttaccttcgaccggcggtgatacgctctggaccagcggtattgcggcctatgaggcgctctctgttcccttccgccagctgctgagtgggctgcgtgcggagcatgatttccgtaaatcgttcccggaatacaaataccgcaaaaccgaggaggaacatcaacgctggcgcgaggcggtcgcgaaaaacccgccgttgctacatccggtggtgcgaacgcatccggtgagcggtaaacaggcgctgtttgtgaatgaaggctttactacgcgaattgttgatgtgagcgagaaagagagcgaagccttgttaagttttttgtttgcccatatcaccaaaccggagtttcaggtgcgctggcgctggcaaccaaatgatattgcgatttgggataaccgcgtgacccagcactatgccaatgccgattacctgccacagcgacggataatgcatcgggcgacgatccttggggataaaccgttttatcgggcggggtaatacgagagtggacggtcccctcgcccccttggggagagggttagggtgagggggcgttcaccgtactttcaacaggttaactccccctttctgagaggaaacaaaattaacgcagaatcttcttctcagccaaatccagcgcaaagtagctgaaaatcagatccgcacccgcacgcttaatcgaacctaagctttcgagcacgactttctcttcatctatagcacccgccagcgcggcgaacttaatcatcgcatactcaccgctcacctgatacgcgccaatcggcaattcagtacgttcacgcagctcacgcacgatgtcgaggtacgctccagcaggtttaaccatcaggcagtctgcgccctgggcttcatccagcagtgattcacgaatcgcctcacgacggttcattgggttcatctgatagcttttgcggtcgccttttaatgcgcttccggcagcttcacggaacgggccataaaaggaggaggcgaacttggtcgaatacgacataatcgccgtatctttaaatcccgcagcgtccagcgcctgacgaatcgcctgtacctggccgtccatcgcggcggaaggggcgatgaagtctgcacctgcagcagctgcaaccacggcttgcttgcctaaattttccagagtcgcgtcgttgtcgacgccatgctcgcacagcacaccgcagtgaccgtgagaagtgtattcacagaagcaggtgtctgacataacgatcatttctggcacggtctgcttgcagatgcgcgacatacgcgccaccagtccatcttcccgccaggcatcgctgccggtttcatcggtatggtgagagatgccaaaagtcatcacggaacgaataccggcgttggcgatgcgttcaatttcgcgtgccagatgtttctctggaatgcgcatcacgcctggcatggcttcaacggctttgtagtcgtcaatttcttcttcaacaaagatcggcaacaccaggtcgttaaggctaagtgttgtctcttcaaacatagcgcgcagcgcaggagatttgcgcaggcgacgagggcgttggattaagtctgtcatggtctgcctgatgtttgtggaatcgaggggcatagtatacctgaagcagggtagggatgttttacgaaagttgtcgcgatgttgacaagaagagaatggaagagaggccaggacatctttttaatagaaacagcaataattttatattcactgaaaatatttttaatctttatttatagctgttggttattattttttggagtttggttgcgctgctataaattgaataattaaaactttgttgcatattcataggatatttatctggtttgtgtttgtgatatttattatgcgtatgcttcaaaaacaaaattatctgcaacatgttgaaatactgtgcttttatgaatttgatgcgtgtttttctccataaattatatatgtccacattcggacttaggggaaagaataattgaaccattcgtctgtaacgcagcataatcgttagcgcgaaacataatatgttttctatgcattgataattgatggatcaacttattacgtccctgaggagggatgacaaatgcactcctggaaaaagaaacttgtagtatcacaattagcattggcttgcactctggctatcacctctcaggctaatgcagcaaactatgatacctggacttatatcgataatcccgttacagcacttgattgggatcatatggataaggcaggcactgtagatggcaactatgtaaactatagtggttttgtctattacaacaacaccaatggtgatttcgatcagtcctttaacggcgataccgttaacggcacgatctcaacctattatttgaaccatgattatgcagacagtactgctaatcagcttgatatcagtaattcagtgattcacggttcgattacttctatgctgcctggcggttattatgatcgttttgatgcagatggtaataatctgggtggatatgatttttacactgatgcggttgttgatacacactggcgtgatggtgatgttttcactttgaacattgctaacactactattgatgatgattatgaagctctttacttcactgattcttataaagatggtgatgtaaccaagcacacaaatgagacatttgatacaagtgaaggcgttgctgttaatcttgatgtagaaagtaacatcaatatttccaataactcccgcgttgcaggtattgcattatctcaaggtaatacttacaacgaaacctacactaccgaatctcatacttgggataacaatatctctgtaaaagattccacagtgacttcgggttcaaattatatcctggatagcaatacttatggcaaaactggtcactttggcaattctgatgaaccgagtgattatgctggcccgggtgatgttgcaatgtcctttactgcttcaggttccgactatgcgatgaagaacaatgtattcctcagcaattcaacgctgatgggtgatgttgcctttaccagcacctggaatagtaattttgatccgaatggtcatgattccaacggtgacggggtgaaagataccaacgggggttggactgatgatagcctcaacgttgatgaactaaatctcactctcgataacggaagcaagtgggttggtcaggcaatttataacgttgctgaaacgtcagcaatgtatgatgttgctacaaacagccttactcctgatgcaacatatgaaaacaatgactggaaacgtgttgttgatgacaaggtcttccagagcggtgtatttaacgtagcgttgaataacggttctgaatgggatactacaggtcgttccatcgttgataccttgacagttaataatggttctcaggttaatgtttcggaatctaaattaacttcagatactatcgatttaactaacggttcttcgctgaacattggtgaagatggctacgttgataccgatcatctgactattaactcctacagtactgttgcgttgaccgaatctactgggtggggggctgattgatcctacccacgtaatatggacacaggcctaagcgaggttcttgttttcaaattgttccggactgaggccgccacaccaactgtgccgccgccaccgattgtaatcacattcgatataattaaacaccgttgcccgcattatttcccggctgataaagtgttctccatggatacattccactttcagcgaatgaaagaagctttccacgcaggcattatcgtagcagcaaccttttgcgctcatacttccacgcagattatgccgcttcagttgcgcctgataatctgctgaacagtactggcctccacggtccgtgtgaacgataacgttccggggcctcttacgccgccacagcgccatctgcagggcatcgcaggccagttgcgccgtcatgcgtggcgacattgaccagccaataacggcacgtgaccacaggtcaatgaccactgccagatacagccagccttcatctgtacgtaagtacgtgatgtctcctgcccacttctggttcgggccactggcgtaaaaatcctgctccaacagattttctgacacaggcaggccgtgtgcgcggtagctgaccgggctgaacttccgggaggcctttgccctcagtccctgacggcgcaggcttgccgccacggtttttacgttaaaggggtaaccctgagcacgcagttcatccgtcaggcgtggggcaccgtaacgctgttttgaccgggtaaaagccgcgaggacaacgctgtcgcagtgttggcggaactgctgacgcgtgcttatccttgtccgccgctgacaccacgtataccagccgctgcgggccacccggagcacgcggcacattgctttgatgctgaactcagcctgatgtttttcaataaagacatacttcatttcaggcgcttcgcgaagtatgtcgcggccttttggaggatagccagctcttcatcccgttctgccagctggcgtttgagacgtgcaatctcggtagacatctccagttcacgttcagaagacgtctgctgattttgctgtttactgcgccagttgtagagttgtgattcatacaggctgagttcacgggctgcggcagtaacaccgatgcgttcagcaagcttcagggcttcactgcgaaattcaggcgaatgctgtttacggggttttttactggttgatactgtttttgtcatgtgagtcacctctgactgagagtttactcacttagccgcgtgtccactattgctgggtaagatcagattacaacctgtacgccaatactatcaccgtaactaacggcggtgtattggatgtgaacgttgatcagttcgatactgaagctttccgtactgacaaactggaactgaccagcggcaacatcgctgaccataacggtaacgtagtatctggtgtgttcgatatccatagcagcgattacgttctgaacgctgatctggtgaacgaccgtacctgggatacttccaagtctaactacggttacggtattgttgctatgaactctgatggtcacctgactatcaacggtaacggcgacgtagacaacggtactgaactggataacagctctgtagacaatgttgttgctgcaaccggtaactacaaagttcgtatcgacaacgcaactggcgctggcgctatcgctgattacaaagataaagaaattatctacgtaaacgacgtcaacagcaacgcgaccttctctgctgctaacaaagctgacctgggtgcatacacctatcaggctgaacagcgcggtaacaccgttgttctgcaacagatggagctgaccgactacgctaacatggcgctgagcatcccgtctgcgaacaccaatatctggaacctggaacaagacaccgttggtactcgtctgaccaactctcgtcatggcctggctgataacggcggcgcatgggtaagctacttcggtggtaacttcaacggcgacaacggcaccatcaactatgatcaggatgttaacggcatcatggtcggtgttgataccaaaattgacggtaacaacgctaagtggatcgtcggtgcggctgcaggcttcgctaaaggtgacatgaatgaccgttctggtcaggtggatcaagacagccagactgcctacatctactcttctgctcacttcgcgaacaacgtctttgttgatggtagcttgagctactctcacttcaacaacgacctgtctgcaaccatgagcaacggtacttacgttgacggtagcaccaactccgacgcttggggcttcggtttgaaagccggttacgacttcaaactgggtgatgctggttacgtgactccttacggcagcgtttctggtctgttccagtctggtgatgactaccagctgagcaacgacatgaaagttgacggtcagtcttacgacagcatgcgttatgaactgggtgtagatgcaggttataccttcacctacagcgaagatcaggctctgactccgtacttcaaactggcttacgtctacgacgactctaacaacgataacgatgtgaacggcgattccatcgataacggtactgaagggtctgcggtacgtgttggtctgggtactcagtttagcttcaccaagaacttcagcgcctataccgatgctaactacctcggtggtggtgacgtagatcaagactggtccgcgaacgtgggtgttaaatatacctggtaatattcttcactccgaagaaatactggtaatttaatctaaataatgcccgtcaaggatttgacgggcattactgcaaaggacgcgcaaatgttatctgtagttaaacctcttcaggaatttggtaagctcgataaatgtttgtccagatacggtacgcgcttcgagtttaataatgaaaagcaagttatattttccagtgatgtcaataacgaagatactttcgttattttagagggagttatctctctgcgtagagaagaaaacgtacttatcggtattacccaggctccttatattatggggctggctgatggtttaatgaaaaacgatataccatacaaattaatatcagaaggaaattgtacgggatatcatctaccagccaaacaaaccattacgcttattgaacaaaatcaactctggcgagacgctttttactggttagcctggcaaaatagaattctggaattacgcgacgtgcagctcattgggcataattcctacgaacaaatccgcgcaacattattatcaatgattgactggaatgaagaattgcgatcacgtattggtgtgatgaattatatccatcaacgtacacgcatatcgcgttctgtcgtcgcagaagttctcgctgctttgcgtaaaggcggctatatcgaaatgaataaaggcaaactggtcgctatcaaccgtttgccttcagagtattaatcaggacgcggggataaccaacggtttattcccgcttagctcggtcaccaggtcattgatgccatcgctcatatttttaaagcgcgtcaacggcgaacgagtgaccaccacaaacgcgccaatattcttctgcgggatcatcgccatataggtaatgaaaccgccaccaccgcctgtcttctgaataatccccggacgaccctctttcggggccatatatacccaacctaaaccaagcgcatccgctttgccggggacatccatgccaatcactttcgtaaactgcgcgcgctgataaatcaacgtctgcatgcgatctgcctggttactgcgctgataaaaatcagatgacaaatactgctgcatccagcgcatcatatcgccaggcgtggaatagacgccgccgctgccaattgccgccagcgtgttattgcacggactggcaccgcgctcagcaaccattaaacggcggcactgatccggtgagggggtgtaggtggtgtctttcatccccaatggacgggtaatctgctcttcaaacaactgggtataaggcttgccggacgcattcgccagtgcatctgccagcaggtcgaacgcaaggttagagtacgccgcctgactgcctggcgcggctttcagcttcgccgtagaaaggtatttccagcgttgctcgcgcgttggccagacaaacaccggacgatgtgccgcgccaccgggctgttcacggggcagggcgctggtatgggttgccagattgaccagcgtaatgggcgtcccattgtaggttggcacgcgtgcgcctggcggagcatatttacttagcggatcgtttaacttcacggtcccctggtcgagcaatttcaccagcatctcactggtcattagcttggtgagggaagcaatacgcacgaccgaatccagctgcgggcgaacgttattaccaggtcgcgtttcgccataactgcgaaagacgcgctggttaccgtcgataacaaccagagccatccccgtggcaccgctgccgtaaaaaatatgatcggcataacgatcgacaatatcagaggcaaactccggttcagtgatcggctgcgccgcatggacggaggtcaatgacgccgcacacagcacggcagaaaaaagcagactacgtttcaacggtggtgtccatagattgaatgaaggtaactgagcgtatttatactactcattgatagattgcaaagggcgaattagtgcaataatagtgttaaaaacgtaacggcgcgtaaacacgatctttttcctgctcaccaatgcctgcatttgtgatcctgcgcgtgttaatccgcttatgtaaacaatctttggtttgtgaaatccgtcgaaacaattcttatggtcaggctggcgaactaagcgccttgctatgggtcacaatgggcggtttcatttggctgacgctttgtagcggtcatgcggttaatacacagcagttgttaaaacgataagaagttagcaggagtgcatatgtttaagtcttttttcccaaagccgggaacgttttttctctcggccttcgtttgggcattgattgccgttatcttctggcaagccggtgggggtgactgggtggcgcgtatcaccggcgcttccgggcagatcccgattagcgccgcgcgtttctggtcgttggatttcctgattttttacgcttactacattgtttgcgtaggactttttgcattgttctggtttatctacagcccgcatcgttggcaatactggtcaatactcggtactgcactgatcatcttcgtcacctggtttttggtggaagtcggggtcgccgtcaacgcctggtatgcgccgttctatgatctgattcaaaccgcgctaagttcgccgcataaagtcaccatcgaacaattttaccgcgaagtgggcgtctttctggggattgcgctgatcgctgtggtgatcagtgtgctgaacaacttctttgtcagtcactacgtgttccgctggcgtacagcgatgaacgaatattacatggcgaactggcaacaactgcgtcatatcgaaggggccgcacagcgtgtgcaggaagacaccatgcgttttgcttcaacgctggagaatatgggcgtcagttttatcaacgccatcatgacgttgatcgccttcctgccggtgctggtaacgctctccgcgcatgtgccggagctgccgattatcgggcacattccgtatggtctggtgattgccgcaatcgtctggtcgctgatggggaccggattgctggcagtggtagggatcaaactgccggggctggagtttaaaaaccagcgtgtagaggctgcctaccgtaaagagctggtttatggtgaagacgatgccacgcgcgcgacgccgcctacggtacgcgagctgtttagcgccgtacggaaaaactatttccgcctctattttcactatatgtatttcaacatcgcccgcattctctatttgcaggtcgataacgttttcggtttgttcttgctgtttccgtcaattgttgccggtacgattacgctcggcctgatgacgcagattaccaacgtttttggtcaggttcgcggtgctttccagtacctgattaactcatggaccacactggttgagttgatgtctatctacaaacgtctgcgcagctttgaacatgagctggatggtgacaaaattcaggaagtaacccataccttgagctaaaaaggagaagtaatgtcgcgcgtcaatcctctatcttcgctgtcattgttggcggttctggttttagcggggtgtagtagtcaggctccgcaaccgttgaaaaagggcgaaaaagcgatagatgtagcgagcgtcgtgcggcagaagatgcctgcgagcgtgaaagaccgcgatgcctgggcgaaagatctcgccaccacctttgaaagtcaggggctggcaccgacgctggaaaacgtctgctcggtgctggcggtggcgcagcaggagtcaaattatcaggcagatccggccgttccgggcttaagcaagatcgcctggcaagagattgaccgtcgtgctgaacggatgcacattcctgcttttctggttcataccgcgctaaaaatcaaatcgccaaacggcaaaagttatagcgaacggttagattcggtgcgtacagaaaagcaattgagcgcgatttttgacgatctgatcaacatggtgccaatggggcagacgctgtttggttcgctcaatccggtgcgcaccggtgggccgatgcaggtcagcattgcttttgccgaacagcataccaaagggtatccgtggaaaatggacggtacagtccgtcaggaagtcttcagtcgccgcggcgggttgtggtttggtacttaccatttactgaattatcccgccagttatagcgcaccgatataccgttttgctgattttaacgctggctggtacgccagccgtaatgccgcgtttcagaacgcggtcagtaaggccagcggcgtgaagctggcactggacggtgatttaattcgttacgacagtaaagaacccgggaaaaccgaactggcaacgcgcaaactggctgcaaaactggggatgagcgacagcgaaattcgccgtcagttagagaaaggtgacagcttctcttttgaggagacggcgctgtacaagaaagtttatcaacttgccgaaacgaaaacgggtaaatcactcccccgcgaaatgttgcctggcattcaactggaaagcccgaaaatcacccgcaacctgactacggcctggtttgcgaagcgcgtagacgaacggcgggcgcgttgtatgaaacagtgatcaaacaggaatgtcaggccagataaggcgtttcaggccgcatctgacaatgtaaaacttactggcggcgatgtcgccagtgcagccatagcgccaccactgcaaaaatgaggcagcctactaaaaacgggatcagcccgaaaatggtgccgacacctaaaccaatttccacccgtgggcgacctgtttcctggacctgcattaaacgctcatagacgccgggcgcatgcactaacaggttcagcaattgcgccccagcccaaaagcaaaacagcacaaacaacgcataggcaatgttgccaggcgttgaagaggcattgcgatattttccgctaaacagcgattttgacagggtgaaatcagccataaaaacctccggaagtcatctgcttctcttctggtgtgataccagcggcttatggcaagtctgacaggtcatttagattgtcaatatcagaatcatggtaaattgatgttgggaatattcccgaagcgtgaatcttcgttgtgagtcacaaaatggcaaccttaagttaaatttattaacaattacgaaaatgttgtctacaccacagacggttgttgcagaatatgcaaggatgttgtttttcgttaacggagctgccatgaatctgcctgtaaaaatccgccgtgactggcactactatgcgttcgccattggccttatattcattcttaatggcgtggtggggttactgggatttgaagcaaaaggttggcagacctatgccgtcggtctggtgacgtgggtgattagtttctggctggcggggttgattattcgtcgtcgcgatgaagaaactgaaaacgcccaataagaatattatcgggcgttaaaatattacattgtggttttcaatgcgttatccgcagcgtgacgctccagcgccagttcaatcaaacgtgtgatcagatcggtgtaacccagaccgctggcttgccacagcttcggatacatactgatattagtgaagccaggcagggtgttgatctcgttgatcaccacttcgttctctggggttaaaaacacgtctacacgcgccatgcctgcgcatcccaacgtttgataagcctgaacggcaatcgcccggatcttatcgttgatttctggcgcaatggctgccggaactaccactttcgcgccatcttcgtcaatgtacttggtgtcgtaggcatagaaatcgctggtgagtacgatctctccacaggtgctggcttgcggattgtcgttgcccagaactgcgcattcgatctcacgacctttgatcccttgctcaacgatcactttatgatcgaactcgaacgccagatcgacggcaattgcgtactgttcttcactggttactttgctgacaccaacagaagagccctgattagccggttttacaaacagtggtaaccccagtttagactccacttcggcaaaactaatgttgtgacgattggcgcgcgtcagggtaataaatggcgcaatgttcagcccggcatcgcgtagcagacgtttggtgacatctttgtccatacaggctgctgaagccagaacatcagaacctacaaacggtaaattggcgacccgcagcattccctgcaaggaaccatcttcgcccagcgtaccgtggacaatcgggaaaatgacatccaccgtcggcaacggctgaccgttttgcgcgtcgataagctgatgctcatgtttacctggcacctgcgcaaggctggtcgccgaagggcgcaacgcaatatgggcaggatcgtctgcatttagcagataattgctggcatcgctgacgtgccattgcccttgtttatcaatgcccagcagcacaacgtcgaagcgacttttatcaatggcatcgacaatgttttttgccgattgcagagacacttcatgttccgctgatttaccaccaaaaacgattcctacccgcagtttttccatcttaaaaacctatcccgtctaacacaaagtgcatacattaccacgacaaaacgggggattcgcggccttctgaaagattgttgcaatcttctgctgacaaagcgtgcaacgtactggtgaagaaagtgcgttatctcaaagatgtgcgcaagatcacaaaaatgatgaacgggaagctaatttattcctggcttaaatggccatgcggtgagtttttttctcttaattataagttaacgaagagaatatatttcataacttttatttataataaaggttgataattaaaagcctatattttgtgtgggtaattatttaaataagagaaacgtttcgctggtaatcaaacaaaaaatatttgcgcaaagtatttcctttgtcataaaaataatacttccagacactatgaagttgtgaaacataatgttaacttctccatactttggataaggaaatacagacatgaaaaatctcattgctgagttgttatttaagcttgcccaaaaagaagaagagtcgaaagaactgtgtgcgcaggtagaagctttggagattatcgtcactgcaatgcttcgcaatatggcgcaaaatgaccaacagcggttgattgatcaggtagagggggcgctgtacgaggtaaagcccgatgccagcattcctgacgacgatacggagctgctgcgcgattacgtaaagaagttattgaagcatcctcgtcagtaaaaagttaatcttttcaacagctgtcataaagttgtcacggccgagacttatagtcgctttgtttttattttttaatgtatttgtacatggagaaaataaagtgaaacaaagcactattgcactggcactcttaccgttactgtttacccctgtgacaaaagcccggacaccagaaatgcctgttctggaaaaccgggctgctcagggcgatattactgcacccggcggtgctcgccgtttaacgggtgatcagactgccgctctgcgtgattctcttagcgataaacctgcaaaaaatattattttgctgattggcgatgggatgggggactcggaaattactgccgcacgtaattatgccgaaggtgcgggcggcttttttaaaggtatagatgccttaccgcttaccgggcaatacactcactatgcgctgaataaaaaaaccggcaaaccggactacgtcaccgactcggctgcatcagcaaccgcctggtcaaccggtgtcaaaacctataacggcgcgctgggcgtcgatattcacgaaaaagatcacccaacgattctggaaatggcaaaagccgcaggtctggcgaccggtaacgtttctaccgcagagttgcaggatgccacgcccgctgcgctggtggcacatgtgacctcgcgcaaatgctacggtccgagcgcgaccagtgaaaaatgtccgggtaacgctctggaaaaaggcggaaaaggatcgattaccgaacagctgcttaacgctcgtgccgacgttacgcttggcggcggcgcaaaaacctttgctgaaacggcaaccgctggtgaatggcagggaaaaacgctgcgtgaacaggcacaggcgcgtggttatcagttggtgagcgatgctgcctcactgaattcggtgacggaagcgaatcagcaaaaacccctgcttggcctgtttgctgacggcaatatgccagtgcgctggctaggaccgaaagcaacgtaccatggcaatatcgataagcccgcagtcacctgtacgccaaatccgcaacgtaatgacagtgtaccaaccctggcgcagatgaccgacaaagccattgaattgttgagtaaaaatgagaaaggctttttcctgcaagttgaaggtgcgtcaatcgataaacaggatcatgctgcgaatccttgtgggcaaattggcgagacggtcgatctcgatgaagccgtacaacgggcgctggaattcgctaaaaaggagggtaacacgctggtcatagtcaccgctgatcacgcccacgccagccagattgttgcgccggataccaaagctccgggcctcacccaggcgctaaataccaaagatggcgcagtgatggtgatgagttacgggaactccgaagaggattcacaagaacataccggcagtcagttgcgtattgcggcgtatggcccgcatgccgccaatgttgttggactgaccgaccagaccgatctcttctacaccatgaaagccgctctggggctgaaataaaaccgcgcccggcagtgaattttcgctgccgggtggtttttttgctgttagcaaccagacttaatggcagatcacgggcgcatacgctcatggttaaaacatgaagagggatggtgctatgaaaataacattactggttaccttgcttttcggtctggtttttttaaccaccgtcggcgctgccgagagaactttaaccccacaacaacagcgtatgacctcctgtaatcagcaggcgacggcgcaggcgttgaaaggggatgctcgtaagacctacatgagtgattgcctgaagaacagcaagtctgcgcctggcgaaaaaagtttgacgccacagcagcaaaagatgcgcgaatgcaataatcaagcaacacaacaatctctgaaaggtgatgatcgtaataagtttatgagtgcctgcctcaagaaagccgcctgatacctgatagtgctaacgggtgagctacgaaaatggctcacccgaaatatcatacttctgcctttagctccgtctctataatttgggaaaattgtttctgaatgttcccaaaaataatgaatgatgaaaactttttcaaaaaagcggcggcgcacggggaggaacctcctttaactcctcaaaacgaacatcagcggtccgggctgcgcttcgcccgtcgcgtcagactaccccgtgcggttggcctggctggcatgttcttaccgattgcttcaacgctggtttcacacccgccgccgggctggtggtggctggtgttggtcggctgggcgttcgtctggccgcatttagcctggcagatagcgagcagggccgtcgatccgcttagccgggaaatttacaacttaaaaaccgatgcagtattagcgggaatgtgggtaggcgtaatgggcgtaaacgtgctgccttccaccgcgatgttgatgattatgtgtctgaatttgatgggggcaggcggcccccgtctgtttgtcgcgggtctggtgttgatggtggtttcctgccttgtcaccctcgagctgacgggcattaccgtgtcgttcaatagtgcgccgctggaatggtggctctcccttcccattattgtcatttatcctctgctgtttggctgggtcagctaccagacggcaaccaaactggcggaacataaacgcaggttgcaggtcatgagtacccgcgacggcatgacgggcgtgtataaccgacgtcattgggaaactatgttacgcaatgaatttgataactgtcggcggcataatcgcgatgcaacgttactgattatcgatatcgaccatttcaagagcatcaacgatacctggggccatgatgtgggcgatgaagcgattgtggcgcttacccgacagttacaaattaccctgcgcggtagcgatgtgattggtcggtttggcggcgatgagtttgcagtaatcatgtccggtacgccagctgagagcgccattaccgccatgttacgggtgcatgaagggctaaatacattacgtttgccgaatacgccacaggtaactttacggattagtgtgggggttgcgccgctgaacccacaaatgagtcactatcgtgagtggttgaaatcggcagatttggcgctttacaaagcaaagaaagccggacgtaaccgcaccgaagtggcggcctgacgtccggcgaaagtcatcaggatttgctgagtttttctgatttttccatacacttcgtcatcgcttcgatcactgcagcacggaagcctttctcttccagtacgcgtaccgcttcaatggtggtgcctcccggtgagcagaccatatctttcagtgcccccggatgttctcccgtttccagcaccatttttgcggaacccattaccgcctgagcggcaaatttatacgcctgggcgcgtggcatcccgcccagcacggcggcgtcggccatcgcttcgataaacataaatacgtaggctggcgaagaaccgctcacaccgaccaccgggtggatcatcggctcagcaattacttccgcttcgccaaagcagcggaaaatattcagcacatcagcggtatcttctggggttaccagcgcgtttggcgttacggaggtcatcccggcattaaccagtgcgggagtgttcggcatggcgcggataattttccggtcatggcccagcgcgcgggcaagctggtcgagcgtgacacctgcagcaatagaaacgaccagagagtctttattcaggctggaggtgatttcgctaagcactttaatcatgatgccaggtttaacggcagcaaaaatgatgtcggcgatttgcgccacttcttgcgccgattctgcggcgttgatgccgaactggtcatgcagggcggcgactttatccggggagggggtgtatacccagatttgccctggaagcacctgaccgctggcaatcagaccgccgagaatggcttttcccatattgccgcagccaataaaaccgattttcttttccattgcctcactcctgccgtgaaattcattgttttgataatcgctggcagaagcataaacagaactatgccggaaggcaaaagcgcgacacaatagaggattacccaacaaaggatgactttatgacaatttgggtggatgccgacgcgtgtcccaatgtaattaaagagattttgtatcgcgcggcggaacgtatgcagatgccgctggtactggtagcaaaccagagtttacgcgtgccgccatcgcgatttattcgtacgctgcgcgtcgcggcaggtttcgacgttgccgataacgaaattgtccggcagtgtgaagcgggcgatttggtgatcaccgcagatatacctttggctgctgaagccatcgagaaaggcgctgcggcgcttaatccgcgcggcgaacgttacacgccagcgaccattcgtgagcgcctgacgatgcgcgattttatggataccttacgtgccagtgggatccagaccggcggaccagatagcctttcacaacgtgaccgccaggcctttgccgcggagctggagaagtggtggctggaagtgcaacgtagtcgtggctaaatgtaatttattatttacacttcattcttgaatatttattggtatagtaaggggtgtattgagattttcactttaagtggaattttttctttacaatcgaaattgtactagtttgatggtatgatcgctattctcatgacaccggctttcgccgcattgcgacctattggggaaaacccacgatgacacaacctctttttctgatcgggcctcggggctgtggtaaaacaacggtcggaatggcccttgccgattcgcttaaccgtcggtttgtcgataccgatcagtggttgcaatcacagctcaatatgacggtcgcggagatcgtcgaaagggaagagtgggcgggatttcgcgccagagaaacggcggcgctggaagcggtaactgcgccatccaccgttatcgctacaggcggcggcattattctgacggaatttaatcgtcacttcatgcaaaataacgggatcgtggtttatttgtgtgcgccagtatcagtcctggttaaccgactgcaagctgcaccggaagaagatttacggccaaccttaacgggaaaaccgctgagcgaagaagttcaggaagtgctggaagaacgcgatgcgctatatcgcgaagttgcgcatattatcatcgacgcaacaaacgaacccagccaggtgatttctgaaattcgcagcgccctggcacagacgatcaattgttgattttcgagcgcctatacttaacgttcatcccgtgaaataaggaagaacgatgccaacgaaaccgccttatcctcgtgaagcatatatagtgacgattgaaaaaggaaagccaggacagacggtaacctggtaccaactcagagccgatcatcctaaaccagactcgttgatcagtgaacatccgaccgctcaggaagcgatggatgcgaaaaaacgctatgaggaccctgacaaagagtgaccgcatcagactgctcggaagggattctgagtgccactacaagggatctgcgtcacatttttcataattcatgtttttctaataattagaatattaaacaataacaatccattactggaatcatttggaatctttacattatgccgtgcacgtctgctgctacgctttttgtcatttgtagcacaagtaagtgtcagcagtggtgcttcacacttgcccggtaattaacgacgaaagaaaagtaaggtggatgaacaatgagtgcgtcgttggcgatcctgaccatcggcattgtacctatgcaggaagttttgccgctcctgacggaatacattgacgaagataatatttcccatcatagcctgctggggaagttaagtcgtgaagaagtgatggcggagtacgcgccagaagcaggcgaagacaccattctcacattattaaatgacaaccagctggcccatgtttcgcgtcgcaaagtggagcgtgacctgcaaggtgtggttgaagtgctcgataatcagggttatgacgtcattttattaatgagtacagcaaacattagtagtatgactgcgcgtaatacgatctttcttgagccgtcgcgaatattgcctccactggtttcctctattgttgaagatcatcaggtgggggttatcgttccggttgaggagatgctgcccgttcaggcgcaaaaatggcaaattttgcagaaatcgccggtattttcattgggtaaccccattcatgattcagaacaaaaaatcattgatgccgggaaagaattactggcaaaaggggctgatgtcatcatgctggattgtttaggatttcaccaacgtcatcgcgatttactgcaaaaacagctcgatgttcctgtcttgctgtctaacgtattgattgcacggctggctgcggaattactggtgtaattttgcgtgacagccagcgcctctggcccctatagtgaagtagatgttcaactaccaaacagggccagtttatgcttcaaagtaatgagtacttttccggcaaagtgaaatcaatcggcttttccagcagcagcactggtcgcgccagcgtgggtgttatggttgaaggcgaatacaccttcagcaccgctgagccggaagagatgacggtaatcagtggcgcgctgaatgtgttactgcctgacgcgaccgactggcaggtgtatgaagccggttcggtgtttaatgttcccggtcacagtgagtttcatctgcaagttgccgaacccacctcttatctgtgccgctatctgtaattcctcgccttccccttgaacgggagggcatttttctgaaatatcctttctttagcccataataatatttcctttgctgcgattttttcaatttccgatatattcataatttatcaaggttgatataaatatcagtgaagatctccagatattgttgcggaactggctacgataaaagataaatcagatgatgaatggtggcgtgcattgctgcaaagtcgcaatgatcatttacgccaaacggcattgcgcaacgcacataccccggcgttgttgttaacgacattgactgagcctcaggatcggtcgctggctattaataatccacagctggctgccgatgtgaaaacggcgtggttaaaagaggatccatcattactcttatttgtcgaacaacccgatctttcgctgttacgtgatttagtgaaaaccggggcaacgcggaaaattcgcagtgaagcgcgtcaccggcttgaggaaaaacaatgacacaacgtccatggagcaagttacagcgtaaaacgcataatattgctgcgctaaaaattattgctcgccgtagcgaataattatatgcctggtgtggcttcgtacgccggataagacgcggcaggcgtcgcatccggcattaaaggaaaatcagcaattaacgttgtgcttcgccacctaatccttcaatcaggttttgaattaacgctgccagttcaccagtcatcaggatgaaatcggcatcaaaacgctgggcgaaatcttcacggtcgatatcttcgttttgatcgcgcagctcgtcgcagaacttcagacgcttgagcgaaccatcgtcgcacatcacaaactgaatgcgctgctgccagtcgagcgccagtttagtcaccacttttccggcttcaatgtgattggtgatctcttcgctggtcagatcttgtttcttcgcgcggatcacgccgccatcttccagcaacgatttcagctcggcttcatcaagcagctggaagccctgtgccgcactaccggagcgaacccattcggtcagcgtcagttcaatcgggttttccatgctcaatggtacaaccggtaacgaccccaggcttttacgcagtaatgccagcgtatcttccgcttttttggcactggcgcagtccaccataatcaaaccgttaaccgtgtcgatccacatcattgtctggctaaaacggctgaaagcacgcggcagcagagagtgcagcacttcgtctttcagcgaatctttttcggttttcttcagcttacgcgcctgttccgcttccagtttggcgattttcgcttccagcgcctgtttaatcaccggagacgggaggattttttcttctttgcgcgcgcagataacaatttgaccattggcaacgtgcgttaacgcatcgctgtgcgatcccatcggaggaacccagcccatcttcgccatgtcctggctgccgcatggggtaaatgccatcgaggctagctgtttttccatctcttctgcacgcagcgaaatctcgcggctaagacggtaaaccattaaatttttgaaccacagcatgataatttccacggccttgtcgttaaatttagcgggcatgataacgaattgtcggcggccttgcattgccaatccggttgtccgtctctacgctattgatattgaaaaaaataaggagagtaccgtgcgtataggtatcgatttaggcggcaccaaaactgaagtgattgcactgggcgatgcaggggagcagttgtaccgccatcgtctgcccacgccgcgtgatgattaccggcagactattgaaacgatcgccacgttggttgatatggcggagcaggcgacggggcagcgcggaacggtaggtatgggcattcctggctcaatttcgccttacaccggtgtggtgaagaatgccaattcaacctggctcaacggtcagccattcgataaagacttaagcgcgaggttgcagcgggaagtgcggctggcaaatgacgctaactgtctggcggtttcagaagcagtagatggcgcggcagcgggagcgcagacggtatttgccgtgattatcggcacgggatgcggcgcgggcgtggcattcaatgggcgggcgcatatcggcggcaatggcacggcaggtgagtggggacacaatccgctaccgtggatggacgaagacgaactgcgttatcgcgaggaagtcccttgttattgcggtaaacaaggttgtattgaaacctttatttcgggcacgggattcgcgatggattatcgtcgtttgagcggacatgcgctgaaaggcagtgaaattatccgcctggttgaagaaagcgatccggtagcggaactggcattgcgtcgctacgagctgcggctggcaaaatcgctggcacatgtcgtgaatattctcgatccggatgtgattgtcctggggggcgggatgagcaatgtagaccgtttatatcaaacggttgggcagttgattaaacaatttgtcttcggcggcgaatgtgaaacgccggtgcgtaaggcgaagcacggtgattccagcggcgtacgcggcgctgcgtggttatggccacaagagtaaaaaacgtaggcaattggcgcatcatgcctgatgcgacgcttgccgcgtcttatcaggcctacaaaaggtgccagaaccgtaggccggataaggcgttcacgccgcatccggcaataagtgctccgatgcctgatgcgacgcttgccgcgtcttatcaggcctgcaaaatgtgccagaaccgcgtagggcggataaggcgttcacgccgcatccggcaataagtaatgagcaccgagactataacctaccccagtggtttcgccagcaccggagtatccgccgcttgctggcgcttatagcgaccatacagcagcaacgacgacatcgcagcaaacgaaagcagggcggcaggcagcgccacgtaattatatgccagccccagcgtcagcatcatacctccgcaatatgcgccgacggcgctaccgaggttaaacgctatttgcccacctgcggcacctaataactctccgcctttggcgttttgtagtaacaatatttgtagcggtgctgaaagggcaaataatcccgcgcaacaaataaaagcaaaaataagcgacgttgttttcatgccgccgcagaaaaagagcatcagcagtgccagtacaattataaagtcagtcactgctgcaatgcgcagtggtgaataacgtcctgaaatcctgccacttagcatatttcccagcaccatccctagcccaactaacatcataataaaggtcatcgccgtttccgaaaaaccggaaataaacatcatgtatggctttacgtagctgaaccaggcaaacacacctgcgttgccaaacatcgtggcggcgaaaattaaccacggggccgggctgcgcaaaaagtgaaattgttcgcgcagatttcctttcgcctcgtcgcgaatatctggcacccaaaaatagaccgatgccatcaccgcaatattaaaaacagcgatcaataaaaaggtgtaacgccagctaaattcctgacttaaatacgttcccagcggaatgcccagcaaattggcgactgtcatcccggaaaccatccccgccacggcggcggtgacttttccgggtttgataatttttgataacacgatcgctccgacgccaaaaaatgcgccatgcggaaagccggataccagccgaccaatggcgagcatcaggtaagacgaagagagcgtgaacatggcgttgccaatgacgcacaacgccaccagaaacaacaagatatgtttgagtgagtagcggctggaaaagagtgcgatgattggcgcaccgaccaccacccccagtgcataatacgagatcatatgcccggcggcaggaatcgaaattcctacgttatgcgccagctccgtgagcacgcccataatgccaaattcggccatccccaaaccaaacgtgcccagagccaaagataaaatgacttttttcataccaccatcacaaccaccagaacggctaccaatcaccgtagccaataaagtgatagcttgcaggataacgaccagcaaggccaagagataattcgcccctctgtattcattatcctgctgaatagttatttcactgcaaacgtactttccagtttgctgtagcccaggccgttgatctttttcactttgatctgcaccggaatacgctctttcatcgcttctacgtggctaatcacaccgatggttttgccactggcgttcagggcatccagcgcatcaagggcggtatccagcgtttcgctatccagcgtgccaaaaccttcatcaaggaacagcgagtcaatacgtgttttatggctgaccagatccgaaagcgccagcgccagcgccagactaacgaggaaactttcgccgccggaaagggtacgggtatcgcgtaccgcatctgcctgccaggtatcaacaacctcgacttccagcgcctcgctggctttgcgctgtaacagatagcgcccgtgcagccgggtaagttgctgattagcgagatggactaaattatccagcgtcagcccctgggcaaacttgcggaatttatcgccctctttggaacctattagcgaattcagatatccccagtcctcaacctgctgcgtcatttgagcaatttgctgcattaaggtttgttgttgctgacggttatctgcatcctgcttcagctgctggcgaatctcgccttgactcgtggtgttttcacgcaacttttggtgagtttgcgctaactcttgctgaatctgctccaccgtcacagtgagagccaacccgtcgtcaggtcggtgttgttgatgctgtgccagcgtttctgctgtctgagtgaccagagtttgcgcctgacggcgctggttttccagattctgcttgagctgttccagctgcgttagtgtttgttcatccattagcgccgcaaggaacgcctgctgatcgtcaaagacgctggcctgtagcgcggtgtcaaactgcgcctgggctttttgcagactttgcgccgccagaacatcctgttgctgtaacgtctgctgctggctgtgtaatgcgagacattgttcatgtacctgccgccagttttccaataccacagtttcttcgcagtgcgggagttcatcactttgcggcaacgtttccagaatcggcgtcagctgctgaatacggttttgcagcgcggttaattcgttctggcgttgctgccagctctgcgcttcttgctgacgtgtcgccaaccagctctcttcttcatcttcctgtggcaatgtcagtgcataacccgtcaatgtcgttaaaagtagttgctggcgttgttcaatttgctgttgatactggataatttgctgattatgcgcggcaatctgcccttgtaattcatgccgttggctgagtaaccgcagctggcgttcgtgctcatcttgtgcatccagccacggttgaatatcgtccagtggctgcaaggtgatattgaggctggccgtgacggcttgccattgttgagtaagtgcttgctcatcttgtcggaggctttgcgcttcgttttcatcacgctgaagctgctttgttatggcgtccagttgcccacgtagcgtcgcaccttcttcaccgagctttttaacttcgttttccagcgccagtaatcgagactgattaacgccaggctccagcgcctgatacgcctcgaccgccgggtggctggtggaaccacaaagtgggcaaggctgacccgcctgtaactgtgcacgttgagcttccagcgttttgatgcgcgcttcctgctcgcaaatggttttcacatcggcaagttgctgcgtcttttctttataacgctggcgcatttcgttaagtgcggcgttacgttgcgtctgttcttgcgtgacattctggatagcgacctgtaactgcgccagacgtttttgttggggaacaatctgtccatgcagcgcgaccaggtgctgacgcagtgggcgttgctcagcatgttgcgccagggcggtagcaacttcatcggcggttaacgtcaacgtgatcgccgcaagcgcattaagtttttgctcagcatgggttaactgttgctgccattgccgcagatgctcgcgatcgctggtttgttgggagaactgcgcacgccaacccgccggttcgttgttccactgacggaagcggtcgtgttcctgtaaccaggtattcaggctttgttgctgctgctgtaattctgctgactgcttcgccgcgtggtggcgaatgctcgcgcgaagcgccattgtgctctgtaagcgagtatttacttcttcaatctgctggcgaatatgcgccagcgccgcgctgtgttctgcgatgcgttcccagtgtggacgaagatttcgtgccggttgtgccagactaagcgccgccagttgaggttgcgctttttcttcttcggctaacgcctgttgcaaggcctgctgacggcggctggcttcttgctgcaattcgtcctgacgcgttaaccagtttagcgattgttgttcttgctgctgcgcggtaattaactgtttttcttcgtcagtaagtacctgcaaactcgctgtcagcgattgcacttgttccggcgtgagcaacgtgacgccgctggcctgcgcttgcagcttctccagctctgtgcgggccgatttgtgctgctcaaaaaccatcgccgagatttgcccgtagatttcagtgccggttaactcctcgagcaattccgcgcgttctttgggtttggcattcaggaaggcagcaaattgcccctgcgaaagcagcatcgaacgggtgaagcgcccgtaatccagcccggttaacgtcgctgtcagttccagcttatctttcactttgtcggcgagaattttgccgtcggcgcagcgcgccagctctacgcgtggcacctgcaaattaccgtcgggttggttacgcgcccgattctggctccagaatgcacggtacgcttcacctttcacttcaaactccacctccgccagacattcggcggtatcgcgggtcatgagatcattttgcgattgtgaaacgttagagagacgcggagtttcgtgatacagcgccagacaaatggcgtccagcagggtggttttccccgcacctgttgggccggtaatagcaaacagcccgttgctggcgaacggctcgcgggtgaaatcaatcttccattcgccttttaatgagttcaggtttttcaggcgcaggctgagaattttcatgcttcgtgttctccggcgagggtatgcaacgtcgtggtgaaaagatgctgcagacgttgctgctgcgattcatccagttcttccagtgccagacggcgattgaacacctcttcgacgctgagttcgctgagggtttcacgctgttggctggctaacacacgctcgcgctgttcacgactccgacgtaccagcaatacttcgacaggcaatgattcggttaatgcctggattttgcgctgaatatcatgcagatactcatcagtagtgatttcgatatccagccagacaggtggctcctgcgatacatcgcgccactgttccagctgtgcggtaatcgacgccagatcgcctttcagcactgccatgggttgcgttaccggtacgttcaggttttccacgctctctaatttgccgtttgaaaatgtcaccagatggacatatttactcttaccgcattcatcaaaactcagtggaatgggggagccgcaatagcgaacatgttccatgccgccaataatctgtgcgcggtgaatatgcccgagcgcgatgtagtcggctggtggaaagttttgtgccggaaacgcgtccagcgtgccaatataaatgtcacgcacggcgtcacttttactggcccccacggtcgttaaatgtcccgtggcgatgatgggcagaggctgatcgccgcgcagtttgcaggcatcggcatagtgttgttggtaataatcggtaatcgctgccagtaaatgctgctgtttttcaataccgttaagccccgcctggctggtaataatgtcacgcggacgtaaaaacggaatggggcacagcactgcgcctggcgtcccgtcgcgacgaggcaagatttgcggcgcatgtccggcgctggcgaccacggtagtattgaggaacgccatgatatcgcgcgattcattcagcgtggcgaccgagtcatggtttcctgccagtaccaccagatgacagccagtttgctgtaaattgacaacaaaacggttgtataacgtgcgggcgtaactgggcggcgagccggtatcgaaaacatcaccggcaacaataatcgcatccacctgatgggtttgtgctgtctccagcagccagtcaagaaaagcctgatgttcagcttcgcggcttttactgtagaagttctggccgagatgccagtctgaggtgtgaaggatgcgcataacggttccctggcgaaaaagcatgggcgcgattatacccaaacagatgtgccatttgcttttttctgcgccacggaaatcaataacctgaagatatgtgcgacgagcttttcataaatctgtcataaatctgacgcataatgacgtcgcattaatgatcgcaacctatttattacaacagggcaaatcatggcgagacgtattctggtcgtagaagatgaagctccaattcgcgaaatggtctgcttcgtgctcgaacaaaatggctttcagccggtcgaagcggaagattatgacagtgctgtgaatcaactgaatgaaccctggccggatttaattctcctcgactggatgttacctggcggctccggtatccagttcatcaaacacctcaagcgcgagtcgatgacccgggatattccagtggtgatgttgaccgccagaggggaagaagaagatcgcgtgcgcggccttgaaaccggcgcggatgactatatcaccaagccgttttcgccgaaggagctggtggcgcgaatcaaagcggtaatgcgccgtatttcgccaatggcggtggaagaggtgattgagatgcagggattaagtctcgacccgacatctcaccgagtgatggcgggcgaagagccgctggagatggggccgacagaatttaaactgctgcacttttttatgacgcatcctgagcgcgtgtacagccgcgagcagctgttaaaccacgtctggggaactaacgtgtatgtggaagaccgcacggtcgatgtccacattcgtcgcctgcgtaaagcactggagcccggcgggcatgaccgcatggtgcagaccgtgcgcggtacaggatatcgtttttcaacccgcttttaacgccttgctcatcggacgcagagcagggcttatgatttcttaactggagtatcttacgtgctggaacggctgtcgtggaaaaggctggtgctggagctgctactttgctgcctcccggctttcatcctgggtgcattttttggttacctgccctggtttttgctggcatcggtaacaggactgcttatctggcatttctggaatttattgcgcctttcatggtggctgtgggtggatcgcagtatgaccccgccaccggggcgtggtagctgggaaccgctactatacggcttacaccagatgcagctgcgaaataaaaaacgccgccgtgaactgggcaatctgattaaacgctttcgtagcggcgcggagtcgctgcccgacgcggtggtgctgaccacggaagagggcggtattttctggtgtaacggtctggcgcaacaaattcttggtttgcgctggccggaagataacgggcagaacatccttaacctactgcgttacccggagtttacgcaatatctgaaaacgcgtgatttttctcgcccgctcaatctggtgctcaacaccgggcggcatctggaaattcgcgtcatgccttatacccacaaacagttgctgatggtggcgcgtgatgtcacgcaaatgcatcaactggaaggggcgcggcgtaacttttttgccaacgtgagccatgagttacgtacgccattgaccgtgttacagggttacctggagatgatgaatgagcagccgctggaaggcgcggtacgcgaaaaagcgttgcacaccatgcgcgagcagacccagcggatggaaggactggtgaagcaattgctgacgctgtcgaaaatagaagccgcaccgacgcatttgctcaatgaaaaggttgatgtgccgatgatgctgcgcgttgttgagcgcgaggctcagactctgagtcagaaaaaacagacatttacctttgagatagataacggcctcaaggtgtctggcaacgaagatcagctacgcagtgcgatttcgaacctggtctataacgccgtgaatcatacgccggaaggcacgcatatcaccgtacgctggcagcgagtgccgcacggtgccgaatttagcgttgaagataacggaccgggcattgcaccggagcatattccgcgcctgaccgagcgtttttatcgcgttgataaagcgcgttcccggcaaaccggcggtagcggattagggttagcgatcgtgaaacatgctgtgaatcatcacgaaagtcgcctgaatattgagagtacagtaggaaaaggaacacgtttcagttttgttatcccggaacgtttaattgccaaaaacagcgattaatccgcctttgtcatcttttattgccataagccagtcgatgctggcttattttctttgcagtcaaaatacgggcgttagattttacaacgattggtgattttttgttcgcatgattagccatgtctttttcacggaaatagtgttttatactggttggtgatttcttatcgctatatacctctggtttttagatccctccttgctttaaaacgttataagcgtttaaattgcgcttcaggtgctgtcatactgactgcattaacgcggtaaatcgaaaaactattcttcgccgcgcctggttgggagtatttcccgctaaaattgtttaaatataccgctgtatcatccccagggattggcacaaaaatttaacgttacaacaccacatccacaggcagtatgatttatgacccatcaattaagatcgcgcgatatcatcgctctgggctttatgacatttgcgttgttcgtcggcgcaggtaacattattttccctccaatggtcggcttacaggcaggcgaacacgtctggactgcggcattcggcttcctcattactgccgttggcctgccggtattaacggtagtggcgctggcaaaagttggcggcggtgttgacagcctcagcacgccaatcggtaaagtcgctggcgtactgctggcaacggtttgttacctggcggtggggccgcttttcgctacgccgcgtacagctaccgtttcctttgaagtggggattgcgccgctgacgggtgattccgcgctgccgctgtttatctacagcctggtctatttcgctatcgttattctggtttcgctctatccgggcaagctgctggataccgtgggcaacttccttgcgccgctgaaaattatcgcgctggtcatcctgtctgttgccgctattgtctggccggcgggttctatcagcacggcgactgaggcttatcaaaacgctgcgttttctaacggcttcgttaacggctatctgaccatggatacgctgggcgcaatggtgtttggtatcgttattgttaacgcggcgcgttctcgtggcgttaccgaagcgcgtctgctgacccgttataccgtctgggctggcctgatggcgggtgttggtctgactctgctgtacctggcgctgttccgtctggggtcagacagcgcgtcgctggtcgatcagtctgcaaacggcgctgctattctgcatgcttacgttcagcacacctttggcggcggcggtagcttcctgctggcggcgttaatcttcatcgcctgcctggtaacggcagttggcctgacctgtgcttgtgcagaattctttgcccagtacgtaccgctctcttatcgtacgctggtgtttatcctcggcggcttctcgatggtggtttctaacctcggcttaagccagctgatccagatctccgtaccggtgctgaccgctatttatccgccgtgtatcgcactggttgtattaagttttacacgctcatggtggcataattcgtcccgcgtgattgctccgccgatgtttatcagcctgctttttggtattctcgacgggatcaaagcatctgcattcagcgatatcttaccgtcctgggcgcagcgtttaccgctggccgaacaaggtctggcgtggttaatgccaacagtggtgatggtggttctggccattatctgggatcgcgcggcaggtcgtcaggtgacctccagcgctcactaaatcactgaacatttgttttaaccacggggctgcgatgccccgtggttttttattgtgttgatgggttaggaattgatggaaagtaagaacaagctaaagcgtgggctaagtacccgccacatacgctttatggcactgggttcagcaattggcaccgggctgttttacggttcggcagacgccatcaaaatggccggtccgagcgtgttgttggcctatattatcggtggtatcgcggcgtatatcattatgcgtgcgctgggggaaatgtcggtacataacccggccgccagctctttctcgcgttatgcgcaggaaaacctcggcccgctggcaggttacattaccggctggacctactgctttgaaatccttattgtcgccatcgccgatgtgaccgcttttggtatctatatgggtgtctggttcccgacggtgccgcactggatttgggtactgagcgtggtgctgatcatttgcgccgtaaacctgatgagcgtgaaggtattcggtgagctggaattctggttctcgttctttaaagtcgccaccatcatcatcatgattgtcgccggtttcggcatcatcatctgggggattggcaacggcgggcaaccgaccggtattcataacctgtggagcaacggcggcttcttcagtaacggctggcttggcatggtaatgtcgttgcaaatggtgatgtttgcttacggtgggatcgaaattatcgggattaccgccggtgaagcgaaagatcctgagaaatcgataccgcgtgcgattaactccgtgccgatgcgtattctggtgttctacgtcggtacgctgttcgtcattatgtctatctacccgtggaatcaggttggcactgccggtagcccgttcgtgctgacgttccagcatatgggcattacctttgccgccagcattcttaactttgttgtgctgactgcttcgctgtcggcaattaacagtgatgtatttggcgtaggccgtatgctccacggtatggcagagcagggcagcgcgccgaaaattttcagcaaaacgtcgcgtcgcggtattccgtgggttacggtgctggtgatgactaccgcgctgctgtttgcggtgtatctgaactacatcatgccggaaaacgtcttcctggtgatcgcttcgctggcaaccttcgccacggtgtgggtgtggattatgatcctgctgtcgcaaattgccttccgtcgccgtttgccgccagaagaagttaaggcgctgaaatttaaagtgccgggtggggtagcaacgaccatcggcgggctgattttcctgctctttattatcgggttgattggttatcacccggatacgcgtatctcgctgtatgtcggtttcgcgtggattgttgtgctgttgattggctggatgtttaaacgccgccacgatcgtcagctggctgaaaaccagtaatccttgcgttctgtaagccggttcaggaggaaatcctgatccggctattccgaaagttatccgcccccgtcctcctcccccaaatatccttcagatgatgagtgatcctgcattaggctatggcaaggtgatcagattttcatcacaggggaattatgatgttaaatgcatggcacctgccggtgcccccatttgttaaacaaagcaaagatcaactgctcattacactgtggctgacgggcgaagacccaccgcagcgcattatgctgcgtacagaacacgataacgaagaaatgtcagtaccgatgcataagcagcgcagtcagccgcagcctggcgtcaccgcatggcgtgcggcgattgatctctccagcggacaaccccggcggcgttacagtttcaaactgctgtggcacgatcgccagcgttggtttacaccgcagggcttcagccgaatgccgccggcacgactggagcagtttgccgtcgatgtaccggatatcggcccacaatgggctgcggatcagattttttatcagatcttccctgatcgttttgcgcgtagtcttcctcgtgaagctgaacaggatcatgtctattaccatcatgcagccggacaagagatcatcttgcgtgactgggatgaaccggtcacggcgcaggcgggcggatcaacgttctatggcggcgatctggacgggataagcgaaaaactgccgtatctgaaaaagcttggcgtgacagcgctgtatctcaatccggtgtttaaagctcccagcgtacataaatacgataccgaggattatcgccatgtcgatccgcagtttggcggtgatggggcgttgctgcgtttgcgacacaatacgcagcagctgggaatgcggctggtgctggacggcgtgtttaaccacagtggcgattcccatgcctggtttgacaggcataatcgtggcacgggtggtgcttgtcacaaccccgaatcgccctggcgcgactggtactcgtttagtgatgatggcacggcgctcgactggcttggctatgccagcttgccgaagctggattatcagtcggaaagtctggtgaatgaaatttatcgcggggaagacagtattgtccgccactggctgaaagcgccgtggaatatggacggctggcggctggatgtggtgcatatgctgggggaggcgggtggggcgcgcaataatatgcagcacgttgccgggatcaccgaagcggcgaaagaaacccagccggaagcgtatattgtcggcgaacattttggcgatgcacggcaatggttacaggccgatgtggaagatgccgccatgaactatcgtggcttcacattcccgttgtggggatttcttgccaataccgatatctcttacgatccgcagcaaattgatgcccaaacctgtatggcctggatggataattaccgcgcagggctttctcatcaacaacaattacgtatgtttaatcagctcgacagccacgatactgcgcgatttaaaacgctgctcggtcgggatattgcgcgcctgccgctggcggtggtctggctgttcacctggcctggtgtaccgtgcatttattacggtgatgaagtaggactggatggcaaaaacgatccgttttgccgtaaaccgttcccctggcaggtggaaaagcaggatacggcgttattcgcgctgtaccagcgaatgattgcgctgcgtaagaaaagtcaggcgctacgtcatggcggctgtcaggtgctgtatgcggaagataacgtggtggtatttgtccgcgtgctgaatcagcaacgtgtactggtggcaatcaaccgtggcgaggcctgtgaagtggtgctacccgcgtcaccgtttctcaatgccgtgcaatggcaatgcaaagaagggcatgggcaactgactgacgggattctggctttgcctgccatttcggctacggtatggatgaactaacgttttataacgccttgcgtgacgcctgcgccatcatccgcggataaaactgccagaagcgggtttcgagggcgtcataatgagcgtctaaatcgtaccaggagtcacgcagggcatccagacgtgggcggcggcttgccatgccgtttaacacgttctggatgaaatccatatcgcgatagcgcaccagccactgctctgaccacaagtaattgttcagattgataaaacgtggcggtgagtccggcaaaatcgtcatcacttgctcgcgggcataacagacaaattcctgtagcggaaagtccggcgacagctgcgaccagtggcgggaaagaaagtgatcccacatgacatccagcgtaataggcgcaacgcggcgcgtttcactacgaaaccactcccgtgcttcgcggacttccggcagattgtcagtcaatacgtcgatacgtcgatgcatatgaatgccagccacgacgtcgggcggaaaactttcttcaggatttccgcgtacgaaatcagccagtaaattgccggaaagcgagctttccgcgagatgggctaaatgcaggtgagctaaaaaattcatcgattatattctatccaaaagggggtaaaggttgcagggagagcgccccggcactagactacccgcctcttattttagtctgagtcagtgtcatgcgcgttaccgatttctcctttgaattgcccgaatccctgattgcccactatcccatgcctgaacgcagtagctgtcgtttactgtcgctggacgggccgacgggcgcgctgacgcacggtactttcaccgatttacttgataagctcaaccccggcgatcttctggtttttaataatacccgcgtgatcccggcgcgcctgtttgggcgtaaagccagcggcggcaagattgaagtgctggttgaacggatgctcgacgacaaacgcattcttgcgcatattcgcgcctcgaaagcgccaaaacctggcgcagaactgctgctgggcgatgacgaaagtattaacgcaacaatgaccgcgcgccacggcgcactgtttgaagtcgaatttaatgatgaacgctcggtgctggatattctcaacagcatcggccatatgccgctgccgccgtatatcgaccgtccggacgaagacgctgaccgcgaactttatcaaaccgtttatagcgaaaaaccgggcgcggttgcagccccgaccgcaggtctgcattttgacgagcctttgctggaaaaattgcgcgccaaaggcgtggagatggcgtttgtgacgttgcacgttggtgcgggcaccttccagccggtgcgcgtcgacaccattgaagatcacatcatgcactcggaatacgctgaagtaccgcaggatgtggtagacgcggtactggcggcgaaagcgcgcggtaaccgggtgattgcggttggcaccacttcagtacgttcgctggaaagcgcggctcaggcagcgaaaaacgatctcattgaaccgttcttcgacgatacccaaatctttatctatccgggcttccagtacaaagtggtcgatgcgctggtgacgaacttccacttgccagagtcgacgctgattatgctggtttcggcctttgccggttatcaacacaccatgaacgcctataaagcagcggtagaagagaaatatcgcttttttagttacggtgatgcgatgtttatcacgtacaatccgcaggcaattaatgagcgcgtcggggagtaattccgcggcgctggtttaaaacgttggactgtttttctgacgtagtggagaaaaaatgaaatttgaactggacaccaccgacggtcgcgcacgccgtggccgcctggtctttgatcgtggcgtagtggaaacgccttgttttatgcctgttggcacctacggcaccgtaaaagggatgacgccggaagaagttgaagccactggcgcgcaaattatcctcggcaacaccttccacctgtggctgcgcccgggccaggaaatcatgaaactgcacggcgatctgcacgattttatgcagtggaaggggccgatcctcaccgactccggcggcttccaggtcttcagccttggcgatattcgtaaaatcaccgaacagggcgtgcacttccgtaacccgatcaacggcgatccgattttcctcgatcctgaaaaatcaatggagattcagtacgatcttggttcggatatcgtcatgatctttgatgagtgtacgccgtatcctgctgactgggattacgcaaaacgctccatggagatgtctctgcgttgggcgaagcgtagccgtgagcgttttgacagtctcggaaacaaaaatgcgctgtttggtatcatccagggcagcgtttacgaagatttacgtgatatttctgttaaaggtctggtagatatcggttttgatggctacgctgtcggcggtctggctgtgggtgagccgaaagcagatatgcaccgcattctggagcatgtatgcccgcaaattccggcagacaaaccgcgttacctgatgggcgttggtaaaccagaagacctggttgaaggcgtacgtcgtggtatcgatatgtttgactgcgtaatgccaacccgcaacgcccgaaatggtcatttgttcgtgaccgatggcgtggtgaaaatccgcaatgcgaagtataagagcgatactggcccactcgatcctgagtgtgattgctacacctgtcgcaattattcacgcgcttacttgcatcatcttgaccgttgcaacgaaatattaggcgcgcgactcaacaccattcataaccttcgttactaccagcgtttgatggcgggtttacgcaaggctattgaagagggtaaattagagagcttcgtaactgatttttaccagcgtcaggggcgagaagtaccacctttgaacgttgattaatattaataatgagggaaatttaatgagcttttttatttctgatgcggtagcggcaacgggtgcaccggcgcaaggtagcccgatgtctttgattttgatgctggtggtattcggtctgattttctatttcatgatcctgcgtccacagcagaagcgcaccaaagaacacaaaaagctgatggactccattgccaaaggtgatgaagttctgacgaacggtggcctggttggtcgcgtaaccaaagtagcggaaaacggctacattgctatcgcgctgaatgacaccactgaagtagttattaaacgtgacttcgtagctgccgtcctgccgaaaggcaccatgaaggcgctgtaattaaaatttttccctaagggaattgccgtgttaaaccgttatcctttgtggaagtacgtcatgctgatcgtggtgattgtcatcggtctgctgtatgcgcttcccaacctgtttggtgaggatccggctgttcagatcactggtgcgcgcggagtcgccgccagtgagcaaacgctgatccaggtccagaaaacgttacaagaagaaaaaataactgctaagtctgtggcactggaagagggcgctattcttgcgcgcttcgactccactgacacccagttgcgcgctcgtgaagcattaatgggcgttatgggtgacaaatacgtcgtggcgcttaaccttgccccggcaacgccgcgctggctggcagctattcacgctgagccgatgaagctcggccttgacctgcgtggcggcgttcacttcctgatggaagtggatatggacaccgcgcttggcaaactccaggaacaaaatatcgatagcctacgcagtgacctgcgcgaaaagggcatcccgtataccactgttcgtaaagaaaacaactacggcctgagcatcactttccgcgatgctaaagctcgtgatgaagccattgcgtatctgagcaagcgccatccggacctggtgattagcagccagggcagcaaccagctgcgtgcggtaatgagcgatgctcgtctgagtgaagcgcgtgaatatgcggtgcagcagaacattaatatcctgcgtaaccgtgtaaaccaacttggcgtggcggagccggtggttcagcgtcagggtgctgaccgtatcgttgttgaactgccaggtattcaggacactgcgcgtgcgaaagagattctgggtgcgacggcaacgctggaattccgtctggtaaacaccaacgttgaccaggccgctgcggcatccggtcgcgtaccgggcgactctgaagtgaaacagacccgcgaaggtcagccagttgtgctgtacaaacgcgtaattctgaccggtgaccatatcaccgactccacttccagccaggacgaatacaaccaaccgcaggttaacatctcgctcgatagcgctggtggtaacatcatgtctaacttcactaaggacaacatcggcaaaccgatggcaaccctgtttgtggagtacaaagacagcggtaagaaagatgcaaatggtcgtgcggttctggtgaaacaggaagaggtgattaacatcgccaacatccagtctcgtctgggtaacagcttccgtatcaccggcatcaacaacccgaacgaagcccgtcagctgtcactgctgctgcgtgccggtgcgttgatcgcgccgattcagattgttgaagaacgtaccattggcccaaccctgggtatgcagaacattgaacaggggctggaggcttgccttgccggtctgctggtttctattctgttcatgatcatcttctataagaagtttggtctgattgcgaccagtgctctgattgccaacttgatcttaatcgtcggcattatgtcgctgttgccaggcgcaacgctgagtatgccaggtatcgcgggtatcgtcttaacccttgcggtggcggtcgatgcgaacgtactgatcaacgaacgtattaaagaagagttgagcaacggacgtactgttcaacaggcaattgatgaaggttatcgtggcgcattcagttctatcttcgatgcgaacatcaccacgctgattaaagtcatcatcctgtacgcagtgggtaccggggcaattaaagggttcgcgattactaccggtatcggtgtggcgacgtcgatgtttaccgcgattgtcggtacgcgtgccatcgtaaacctgctatatggcggcaagcgcgtcaagaagctgtcaatctgaggagtgcgatgtggcacaggaatatactgttgaacaactaaaccacggccgtaaagtctatgactttatgcgctgggactactgggctttcggcatctctggtctgctgttaatcgctgctatcgttattatgggcgtgcgcggctttaactgggggctggatttcaccggtggtacggttattgaaattacgctcgaaaaaccggctgaaattgacgtaatgcgtgatgcattgcaaaaagccggttttgaagagccgatgctgcaaaactttggtagcagccatgacatcatggtccgtatgccgcctgctgaaggcgaaaccggcggtcaggtgttgggcagccaggttctgaaggtgattaacgaatccaccaatcagaatgcagcagtgaagcgtattgagttcgtcggtccgagcgtgggggcagaccttgcgcaaaccggtgcgatggcgttgatggcagcgctgctgtctatcctcgtgtacgtaggtttccgctttgagtggcgactggcggcaggggtggttattgcgctggcgcacgacgttatcattacgctgggtattttgtcgttattccatatcgagattgacctgaccattgtggcatcgttgatgtcggttatcggttactcgcttaacgacagtatcgtggtatcggaccgtattcgtgaaaacttccgcaagatccgtcgcggtacgccttacgaaatctttaacgtgtccttgacccagacgctgcaccgtaccttgatcacatccggtactaccttgatggttatcctgatgctgtacctcttcggtggtccggtactggaaggcttctcgctgaccatgcttatcggtgtttccatcggtactgcatcttccatctatgtggcatctgcgttggctctgaaactgggtatgaagcgcgaacacatgttgcagcagaaagtggaaaaagaaggggcggatcagccgtcaattctgccgtaatcaagttcccgttgatgttgaaaatcccggtcagaagatcgggattttttttgatgtatggagattgcgaaaatccccgcatcttgggaaactgcgcgtaaccctacatttcatccaggtaacttttcatggctatcatcccaaaaaactatgcgcggttagaaagcggctatcgcgaaaaagcattaaaaatctatccgtgggtctgcggtcgctgttcccgcgagtttgtttattccaacctgcgtgaacttaccgttcaccacattgatcacgaccataccaataacccggaagatggcagtaactgggaattgttgtgtctctattgccacgatcatgagcattcgaaatataccgaagcggatcagtatggtacgaccgttatcgcaggggaagatgcgcagaaagatgtcggtgaagcgaagtacaacccattcgctgacctgaaagcgatgatgaacaagaagaagtgattaaaacgtaaaattgcctgatgcgctacgcttatcaggcctacgttatttcagcaatatattgaatttacgtgcttttgttggccggacaaagcgtttacgccgcatccggcatgaacaaagcacacgttgttaacaatcagaaatgccgggaataaatcccggcattttcataatcagaagttgtaacctactaccaggtaaccaccccagccggtagagcgaacgttgaagttgccgttgccgaagttcagttctgcatcgtcgttccactgaccaccgtcgtgccagtaacgagctacgacagagtagtgccagtgatcgtagttcagagccagaatatggctggaagcgatagagttattagtacgggtcttaataccgttgattgcgttaccgctgtcatcccctaaatcggaaccccagtcgaagttggtgaagccgatgtagctcagctgaccgccccacagatcggtaatcggcacaaagtatttaattttgaaacggtaaccgtcccactcgttttcgttcgctgcgccatagttctgccactggtatttcgcatagacgttcatggacaggctcatcggcaggccagtgtcgatatcggtacccagacccatgtaccaggtgctctggcgaccatctttattacgacccatgtcgtaaatgtagttgttcgcgaagtaccactctttgaacggaccgaagctaaggtcagtattggtcagcttgtcgatggagaaacgtggttcgatttccataaacagcggagaaccgtggttccagatacctttagcatcggagttaccgccgaagaataccggcgcatccgcataaccatagaagtcgaaccagtcttttttagcgaatgcttcgtactcaaggtaggtatcgttgcggatctgcggtccgaaacgggtgtgatagcttccgacaacgttaacgctctggtgccaccagtcggaaagatactgcggtttgtcgttttcagctgcgttgacagtaaaagacgaagagagcgccagtaccgcaccggctgccagtaatgtttttttcatatgtatgccactgtttgaaaatcccttgcgggagtgaaaaaggcgcaaattgcgtttctaaatatttcgtatacagaggagcctattataaaaatcattgctcacaaaaatatgtttcgtttcacagttctatcatttacgtaatcgattgcgttcacgtttacacacattcgggcggggattgtactgactttcgcccttgttgcaaacttttactatcaatccaggtgatgtaagcagagtaacaaaatgacggggaaagatgttgcgggacgcacaaaatcgtcccgaaatacgtttactgcataacaggttgaatgtcgtggatacgtacaaagcctaactgatccacagaaatcccctttaactgtaacggaatatcaacatcgctgggggcgaggacgctggcaggggcattaatcaattgattctgcacattgatttcctgaaagttgtctattgttccctgaatttgcccatattcaacagttccgctgaatgcgggcaagggatcattcgactcaccctgaatacgtagtgtaagggtggtgccatctgcatcaggcgtaatattcaccagcgacatacgtaaagtaccgatctggctttccagtcttgccggtgttttcgctccaggcagaaggtaaaccccactgctggattttgcattcagcctgttttgctgagtgattttgactgtttcttgattgagttgcgtcatctcctggttcagcgtgctgacgctgtgtttcatctgtcgcacttcactttgctgcacacaggcgctaaggctgaacaggcttcccagcaggagcagtcgaaaaacgttagtattcataggtcgtccctttctcgtcgcaattagcctaatggtagagggtaaaagcagcgaaagcatcgatcctttatctcaaaagcgttgcgcctttgttgtatcgtcagttcagggtaaaatagatttccgttaaccacctggtcaggacgccgtatgcattgcccattctgtttcgccgtggacactaaggtaattgactctcgtctcgtgggcgagggttcatccgtacgccgccgtcggcagtgtctggtgtgtaatgaacgtttcaccacctttgaagtggcggagctggttatgccgcgtgttgtaaaaagcaacgacgtgcgtgaaccgtttaatgaagagaaattgcgtagcggaatgctgcgggcgctggaaaaacgtccggtgagttccgatgacgtcgaaatggcaatcaatcatattaaatcgcagctgcgcgccaccggtgagcgcgaagtgccgagcaagatgattggcaatctggtgatggagcaattgaaaaagctcgataaagtcgcctatatccgttttgcctctgtctaccgcagtttcgaagatatcaaagaatttggcgaagagatcgcgcgcctggaggactaagccgtgcaggacgagtattacatggcgcgggcgctaaagctggcgcaacgaggacgttttaccacgcatcccaacccgaatgtcgggtgcgtcattgtcaaagatggcgaaattgtcggtgaaggttaccaccaacgtgcgggtgaaccacatgccgaagtacacgcgttgcgtatggcgggtgaaaaagccaaaggtgcgaccgcctatgtcacactcgaaccctgtagccatcatggtcgtacgccaccgtgctgtgacgcactcatcgccgctggcgtagcgcgcgtggttgcctcgatgcaagatcctaacccgcaggtcgctgggcgtggactttaccgtctgcaacaggctggcattgacgtcagccacggcctgatgatgagtgaagccgagcaattgaataaaggctttctcaagcggatgcgcaccggctttccttatattcagttaaaacttggcgcatcgcttgatggtcgcacggcgatggcgagcggcgaaagccagtggatcacttcgccccaggcgcggcgtgatgtacaactactgcgcgcgcaaagtcatgccattttaaccagcagcgccacggtgctggcggatgatcctgccttaacggtgcgttggtctgaactggatgaacaaactcaggcgctctatccgcaacaaaatctccgtcagccgatacgtattgtgattgatagccaaaatcgcgtgacgccggtacatcgcattgtgcagcagcccggcgaaacctggttcgcgcgtacgcaggaagattctcgtgagtggccggaaacggtgcgtaccttgctgattccagagcataaaggtcatctggatctggttgtactgatgatgcaactgggtaaacagcaaattaacagcatctgggtggaagcggggccaacgctcgctggcgcattgctgcaggcgggtttagtcgatgagctgattgtctatatcgcacctaaactattaggcagcgacgcccgcggattatgcacgctgccagggcttgagaaattagccgacgccccccaatttaaattcaaagagatacgtcatgtaggcccggatgtttgcctgcatttagtgggtgcatgatctcccggctcgaaagggaagcagcgcacgaaatattatgctaaaatccgcccccctgcggggccatactcgaacccgaaggaagaaaatgaacattattgaagctaacgttgctaccccggacgctcgcgtcgccatcaccatcgcgcgtttcaacaactttatcaatgacagcctgctggaaggtgcaattgacgcactgaaacgtatcggtcaggtaaaagatgaaaacattaccgttgtttgggtgcctggtgcctatgagctgccgctggcggcgggtgcactggctaaaaccggtaaatacgacgcggtgattgcgctgggtacggttattcgtggtggcactgcccactttgaatatgtcgctggtggtgcaagcaacggcctggcgcatgttgcccaggacagcgaaattccggttgcttttggggttctgaccactgaaagcattgaacaagcgatcgaacgtgctggcaccaaagctggcaacaaaggtgcagaagctgcactgaccgcgcttgaaatgattaatgtattgaaagccatcaaggcctgaaattagtaaggggaaatccgtgaaacctgctgctcgtcgccgcgctcgtgagtgtgccgtccaggcgctctactcctggcagttgtcccagaacgacatcgctgatgttgaataccagttcctggctgaacaggatgtaaaagacgttgacgtcctgtacttccgtgagctgctggccggggtggcgactaataccgcatacctcgacggactgatgaagccatacctgtcccgcctgctggaagaactgggacaggtagaaaaagcagtactgcgcattgcgctgtacgaactgtctaaacgtagcgatgtgccatacaaagtggccattaacgaagcgatcgaactggcgaaatcgttcggcgcagaagacagccataagttcgtcaacggcgtactcgataaagcagcacctgtgattcgccctaacaaaaagtgatatccaggccggtagattcacggaagaccgttccatgatcgccggccttttcttttttacctgctgaggcataacgtatggcatgtggcgagttctccctgattgcccgttattttgaccgtgtaagaagttctcgtcttgatgtcgaactgggcatcggcgacgattgcgcacttctcaatatccccgagaaacagaccctggcgatcagcactgatacgctggtggcgggtaaccatttcctccctgatatcgatcctgctgatctggcttataaagcactggcggtgaacctaagcgatctggcagcgatgggggccgatccggcctggctgacgctggcattaaccttaccggacgtagacgaagcgtggcttgagtccttcagcgacagtttgtttgatcttctcaattattacgatatgcaactcattggcggcgataccacgcgtgggccattatcaatgacgttgggtatccacggctttgttccgatgggacgagccttaacgcgctctggggcgaaaccgggtgactggatctatgtgaccggtacaccgggcgatagcgccgccgggctggcgattttgcaaaaccgtttgcaggttgccgatgctaaagatgcggactacttgatcaaacgtcatctccgtccatcgccgcgtattttacaggggcaggcactgcgcgatctggcaaattcagccatcgatctctctgacggtttgatttccgatctcgggcatatcgtgaaagccagcgactgcggcgcacgtattgacctggcattgctgccgttttctgatgcgctttctcgccatgttgaaccggaacaggcgctgcgctgggcgctctctggcggtgaagattacgagttgtgtttcactgtgccggaactgaaccgtggcgcgctggatgtggctctcggacacctgggcgtaccgtttacctgtatcgggcaaatgaccgccgatatcgaagggctttgttttattcgtgacggcgaacctgttacattagactggaaaggatatgaccattttgccacgccataaagatgtcgcgaaaagtcgcctgaagatgagtaatccgtggcatctacttgctgtcggattcggaagtggattaagcccgatcgttcctgggacgatgggctcgctggcagcgattccgttctggtatctgatgacctttttgccctggcagctctactcgctggtggtgatgctggggatctgtatcggcgtctatctttgtcatcaaacggcgaaagacatgggtgtgcacgatcatggcagcattgtctgggacgaatttattggtatgtggatcacgctcatggcgctgccgaccaatgactggcagtgggttgccgccgggtttgtgattttccgtattctggatatgtggaagccgtggccgatccgctggtttgatcgcaatgtgcatggcggcatggggatcatgatcgacgatattgtcgccggggtgatttccgcaggcatcctgtattttatcggtcatcactggccgctgggtattctgtcgtagttgtgcaccgatgcctgatgtgacgcttgtcacgtctcatcaggcctggactcttatttaaatcctacgacaggatgcggtttatacggcgtttccagttcggcaatctgttccggcttcaaagtgatatccaccgcgttcaatagctcatcaagctgttcttcgcgcgaagttccgataatcggtgcggcaatgcccggtttactcaacaaccaggccagcgcaacttgtgctcgtgtcgcccccagttcttcactgacgcctgttaaccgctctgcgatctgcgcgtcattttcatcgctttctttatagagatttttccccacctcatcagacaccagtcgtgcggtagtttctccccacggacgcgtcagacggccccttgccagcgggctccatggaattaccgccacgccctcctgataacacagtggtagcatctcgcgctcttcttcacgataaatcagattgtagtgatcctgcatactgacaaactgcgcccagccgtgctgtttttggagttccagtgcctgagcaaactgcgaagcgtgcattgatgacgcgccgatataacgcgctttcccggcttttaccacgtcgttgagggcttccagcgtctcttcgatcggcgtgttgtaatcccagcgatgaatttgcaggatatcgacataatccatgccgagacgtcgcaggctgtcgtcgatagagcgcaaaatttgcgcacgggataatccttccggtaaatcaccaacgcgatggaacactttggtcgcaacgaccacgtcttcacgacgggcgaaatcccgcagtgcgcgaccgacgatctcttcgctgctgccgtcagaataactgttggcggtatcaaagaaatttatgccgccttccagtgcacgtttaattatgggacggctgctttcttccggcagtgtccatgcgtgattaccgcgatctggctcgccaaaggtcatacagccgaggcaaagtcgggaaacgcgaaggtcggtttttcctaaggggttgtattgcatgctgccactcctgctatactcgtcatacttcaagttgcatgtgctgcggctgcattcgttcaccccagtcacttacttatgtaagctcctggggcttcactcgtttgccgccttcctgcaactcgaattatttagagtctatgaataatttcttaagcatagcaggagtggagtagggattatgccagccaggccttgattttggcttccataccagcggcatcgaggccgagttcggcgcgcatttcttcctgagttccttgcggaataaagaagtccggcaggccaatgttcagcacgggtactggtttacgatgggccatcagcacttcgttcacgccgctgcctgcgccgcccataatggcgttttcttctacggtgaccagcgcttcatggctggcggccatttccagaattaacgcttcatcaagcggtttcacaaaacgcatatcgaccagcgtggcgttcagcgattcggcgactttcgccgcttctggcatcagcgtaccaaagttaaggatcgccagtttctcgccacgacgcttcacaatgcctttgccaattggtagtttttccagcggcgtcagttccacgccgaccgcgttgccacgcgggtagcgcaccgctgacgggccatcgttatagtgatagccggtatagagcatctggcgacattcgttttcatcgctcggggtcataatgaccatttccggtatgcagcgcaggtaagagagatcaaaagcaccctgatgggtttgaccgtcagcaccaacaatgcccgcgcggtcgatggcgaacaggaccggaagcttttgaatcgccacgtcatgcagcacctgatcataggcgcgttgcaggaaagtggagtaaatcgcgacaatgggtttgtacccaccaatcgccagacccgcagcaaaggtcaccgcgtgttgctcggcaattgccacgtcgaagtagcgatccgggaatttacgtgaaaactcgaccatgccggaaccttcacgcatcgccggagtaatcgccatcagcttgttgtctttcgctgccgtttcgcacaaccagtcgccaaagatttttgaatagctcggcaaaccgccgctacttttcggcaaacaaccgctggagggatcaaatttaggcacggcgtggaaagtgatcgggtctttttctgccggttcataaccacgaccttttttggtcatgatatgcaggaactgcgggcctttcaggtcgcgcatgttctttagcgtggtgataagccccagcacatcgtgaccgtccaccgggccgatgtagttaaagcccagctcttcaaacaacgtgccaggcactaccatgcctttaatatgttcttcggtgcgtttgagcagctctttaattggcggcacgccagagaaaacttttttcccgccttcgcgcagtgaagagtaaagcttaccggaaagcagctgtgccagatggttgttgagcgcgccgacattttcggaaatcgacatttcattgtcgttgagaatcaccagcatatcaggacggatatcgcccgcgtgattcatcgcttcaaacgccatgcctgcggtaatcgcgccatcgccaatgacacagacggtgcggcgatttttgccttctttttcggcagcaaccgcaataccaattccggcactgatggaggttgatgaatgcccgacgcttaatacgtcatattcgctttcgccgcgccacgggaacgggtgcagaccgcctttctgacggatggtgccgattttgtcgcggcgtccggtcaaaattttatgcggataagcctgatgccccacatcccaaatcaattggtcaaacggggtgttgtagacatagtgcagcgccacggtcagttcgaccgtgcccagcccggaggcgaagtgcccgctggaacggctcacgctgtcgagtaaatagcggcgcagttcgtcgcagagtttcggtaaactctctttcggcaacagtcgtaactcctgggtggagtcgaccagtgccagggtcgggtatttggcaatatcaaaactcatcaggggcctattaatacttattgtttatttattacgctggatgatgtagtccgctagcgcttccagtgccgaggtatcgagtgactgttcagccagttgtttcagcgactgacgggcatcgtcgatcagatcccgggctttcttccgggcttgctcaagacccagaagtgcagggtaggtacttttaccaagttgctggtcggcaccctggcgttttcccaacgttgcagtatctcccaccacatccaggatgtcatcctgaacctggaaggcaaggccgatgctctctgcatacttgtcgagtaccggcagagcacgacgtcctttatctccggcgcttaatgcaccaaggcgaacggcggcgcgaatcaatgcgccggttttatgacgatgaatacgctcaagcgcgtccagaggtacgtgtttgccttccgcgtctaaatctaatgcctgaccaccgcacattccggcaataccactggcgctcgccagttcagaaatcatcgaaattctgtcgcggtccgacacttccggcatatcggcatcgcttaaaatcgagaacgccagcgtttgtaaagcgtcgccagcgagaatcgcgtttgcttcgccaaacttcacatggcaggttggcaaaccgcgacgcagatcgtcatcatccattgccggtaaatcatcatgaattaatgagtaagcgtggatacactcaacggcggcagcgggtgcgtccagcgtgtttgtgctaacgccgaacatatgaccggtggcataaaccaggaaaggtcgcaggcgcttaccacctaataatgcgccatactgcatggtttcgaccacgggagtgttctgaaagggcagtggggcgataaaacggctcagcgcctggttggcctgcttaacgcaggcttcgagttgctgcggaaagtccattactcattgtccggtgtaaaaggggttagagaggcgtcttcattgtcagacagcagaatttgtacgcgctgttcggcttgttgtaatttggcctgcccctgacgtgccagctgcacgccgcgttcgaactcgttcagcgcctcttccagcggcaggtcgccactttccagacgggttacaatctgttccagctcgctcagcgccttttcaaagctggcgggcgcctcatttttcttcggcataatgaatgtctgactctcaatatttttcgccccgtcatggtaacggactcagggcaaatagcaaataacgcgcaatggtaaggtgatgtgcacagcaaagcgatgttagtggtatacttccgcgcctggatgcagccgcaggtgtgggctgctgtatttttccctatacaagtcgcttaaggcttgccaacgaaccattgccgccatgaagtttatcattaaattgttcccggaaatcaccatcaaaagccaatctgtgcgcttgcgctttataaaaatccttaccgggaacattcgtaacgttttaaagcactatgatgagacgctcgctgtcgtccgccactgggataacatcgaagttcgcgcaaaagatgaaaaccagcgtctggctattcgcgacgctctgacccgtattccgggtatccaccatattctcgaagtcgaagacgtgccgtttaccgacatgcacgatattttcgagaaagcgttggttcagtatcgcgatcagctggaaggcaaaaccttctgcgtacgcgtgaagcgccgtggcaaacatgattttagctcgattgatgtggaacgttacgtcggcggcggtttaaatcagcatattgaatccgcgcgcgtgaagctgaccaatccggatgtgactgtccatctggaagtggaagacgatcgtctcctgctgattaaaggccgctacgaaggtattggcggtttcccgatcggcacccaggaagatgtgctgtcgctcatttccggtggtttcgactccggtgtttccagttatatgttgatgcgtcgcggctgccgcgtgcattactgcttctttaacctcggcggcgcggcgcatgaaattggcgtgcgtcaggtggcgcattatctgtggaaccgctttggcagctcccaccgcgtgcgttttgtcgctattaatttcgaaccggtcgtcggggaaattctcgagaaaatcgacgacggtcagatgggcgttatcctcaaacgtatgatggtgcgtgccgcatctaaagtggctgaacgttacggcgtacaggcgctggtcaccggcgaagcgctcggccaggtgtccagccagacgctgaccaacctgcgcctgattgataacgtctccgacacgctgatcctgcgtccgctgatctcttacgacaaagagcacatcatcaacctggcccgccagattggcaccgaagactttgctcgcacgatgccggaatattgtggtgtgatctccaaaagcccgacggtgaaagcagttaaatcgaagattgaagcggaagaagagaagttcgacttcagcattctcgataaagtggttgaggaagcgaataacgttgatatccgcgaaatcgcccagcagaccgagcaggaagtggtggaagtggaaaccgtcaatggcttcggcccgaacgacgtgatcctcgatatccgttctatcgatgaacaggaagataagccactgaaagtcgaagggattgatgtggtttctctgccgttctataaactgagcaccaaatttggcgatctcgaccagaacaaaacctggctgctgtggtgtgagcgcggggtgatgagccgtctgcaggcgctctatctgcgcgagcagggctttaacaatgtgaaggtatatcgcccgtaatttgtggtttttacgtcgcatctggtcagatgcgacgtttgccgcatccgacactactcgtaataattataaatccctgccgccatcaccagttgtgatgccacttcatgggctttttcacgcccaaccaacaggtcgataattttcagaccaaagtcgatagctgtacccggcccctggctggtcagcaattttacccgtgcatcccagacgacgcgcttgtccagccattgttcggcgggaattttgtctttcagcgtcgggaagccggtcatattaccaatcgggaagatatcgtgcggcaccagcacggtggctggcgcggcgcaaatagccgcgacgatacgcccggaacggtggaactgtttaacggtttcaaccagcagagtgctatcgcgaaaacactccgcgcctttaatgccaccaggcagcacgatcacgtcatattcgccatcagccacttcgaccagcggcgcatccgccagcagcttcacgccgcgcgagcaggtaatcgccaggttaccatcgctggcgacgctggcagtggtgactttgataccgccgcgaaccagcagatcgatagtggtgacggcttcagtctcttcactaccaggggcgaggcaaaccagtgccgatgcgctcatattcactctcctttctttttaccatttcaaacaggcgggtgttttccggtacggcaatcccatgcgcgcgggcgcggcgtaagagaaaaccattgatatagtcgatttcagtgtggcgcagcgcgcggatatcctgcaacatcgacgagatattttccgctgtggcatcaatcacctgcatcacgtaatcacgcaaatcttctgctgaagtatgatgcccttcgcgttcgatcaccgccgcgacttcttcgcatatctgcataatttcttgcggatgatgacgtaattcaccgttcgggcaattccagatggcagtcagtggattaatcacgcagttgactgccagcttgcgccacagctcggcgcgaatattgttatgccaggcaacgtcaggcaacacggtttgcaaaatatccgccagataactgtaatccccgtcctgttgccgtgccgggccaatatgcgtgataccgtttgccacatgaataatgacattgccgtcgcggcgggctgcatgggtggtggtgcccatcagtaatggctgctgaatgttttgcaactcttcgatggtgcccatgccgttgtgaattaacagtattggcgtagttacaggcagtgtggacgcgaggcttttgacggcatcggaaacctgccatgctttcagcgtcaccaggagcagatcgctggtggcgagaaaatcgggatcgttggcggtcagcgattcgttaaatatcgaaccatctgtctcaaccagattcacgctacaataaggttgcggtacgcgcagccagccctgaacttcatgaccctgtttgcaaagtgctgtaagccataattgccctaaggcaccgcatcccaatacggtaattttcattgttcctcctcacccgcaaccactccgggtgttcaataaggctatcccttaattgtgcatgctgttgcgactatgcacaattaagggatacgtcctggtgcaggactgtcggttatttaactttgcgggtattatgcttcgcatcaaaaatgaagggagaggaaaagatgccatctttcgatattgtctctgaagttgatcttcaggaagcacgtaacgcggtcgataacgcgagccgcgaagtggagtcccgttttgacttccgtaacgttgaagcctcatttgagctgaacgacgccagcaaaaccatcaaagtgttgagcgagtccgatttccaggtcaatcagttgctggatattctgcgtgccaagctgctgaagcgcggcattgaaggcagttcgctggatgtaccggagaatatcgttcatagcggtaaaacctggtttgtggaagcgaaactgaaacagggcattgagagcgcgacccagaagaaaatcgtcaagatgatcaaagacagcaaactgaaagtgcaggcgcaaattcagggcgatgaaatccgcgtaacgggcaaatctcgtgatgatttgcaggctgtcatggcgatggtacgtggtggcgatctcggtcagccgttccagttcaaaaacttccgcgattaatcgcgactatgtgcgttttgttcatgtcagatgcggcatgaacgcctgattcggcctacaaaggtttgtaattcagaaactttgtaggcctgataagcgtagcgcagcaggcaattcgccgcgttttttatgcctgacgaattgcctgttctatctcaaagcgattcgtcactttgctgtcgattttcacataagctgaatgttcttcttctgcaatcaacacttctttgatgccttcagtttctagcaaacgcacttttaacgcctcgtttgcggcaatgttcgccgggatttcaatgcgcaaactgctgacatacggcggttctttcatggtactggcgactgtcagccacactgcggccagcattgcgccagcgagaaataccccctgaccgtcaaacatgccgttaatccagccgcccagcgaaccgccaatcgccacgccaagaaactggctggtggagtaaacacccatcgccgtacctttgtaacctgctggcgactctttactgataagtgagggcaggagggcttccatcaaattaaacgccacaaagaaaagctgcacgccgaccaccagttgccagaactgcgtttgcgcgttccacaacacaatttccgcaaccacgatcaacccgacgcagaagacaaagacttgcttcattttgcgcttaacttcagcgtagataatgaaaggcacgaccgagccaaaggcgattagcattgtcgccagatagaccttccagtgttcagccgccgggaaccctgcatcagccagttgtccgggcagggcaacaaacgtcgacatcagcaaaatatgcagacacataatgccaaagttgagtttcagcagccgcggttccgccagcactttactgaaactgcctttcaccattccggactcacgattaagtacgtgagtgctactgttgggcacaacccaaatggtcaacgcaatgccggtcgttgccagaatagcgatcatccagaacagcgcgtgcagcccaagtttgtgagtgatgatcgggccaagcaccatcgcaatggcaaaggtaatgccaaagctcacgccgataaacgccatcgctttggtgcggttttgttcgcgcgtgagatcggaaagcagcgccataacggcggcggcaattgctccagagccttgtagcgcccggcccagaataattccccagatggagtcggaaagcgcagcgataacgctaccggcggcaaacaccgccagcccaccgacaattaatggtttgcgaccaatgcggtcggaaagcaggccaaacggaatctgaaaaacggcctgagtcagaccataaataccaatggcaataccgattaatgcttcgctggcaccttgcagagccatgccgtacgtggtcagaaccggcagaaccataaacatgcccagcatgcgcaacgagaatacggtccctaaaccccaggtcgcgcgcctctcacctggcgtcattttataatcgttcattaccacctctgttttaaattcgcgactagtgtaaagcggcaaacgaatggggtaaacatgcggattttttagtaaatatttcgagagggatatgtttctaatgctaagaaaaaaggtgccgtagcacctttttaatagagaggttttgttaccacacagcagccagcagcgtatgcgagtccggtaccataaaatcaacggacatcatcaccgagagggcagtgatggcgatgatagagaagccgaacagcttgcgcgcccagattctgtcatcagcaactttataaccgcgcagagccatacctaaccaccagacgctaaccgccgcggcgaccaccagatatttatacccagcgtaaccgccaagagagagcatcagcgtggcaacggcaaaggcgatgatatacagcgtgatgtgattcttcgccaccgaaatgccttttaccactggcaataccggaatgtttgccgcctggtaatccttaaagcggaaaatggcgatggcataggagtgaggcatctgccacaggctgaagatagccagcaggatcgctgcgccgctatcgaactcaccggttaccgcacagtagccgatcaccggcggcgcagcgccggagagcgaaccaatcaacgtgccgtagacagagtggcgtttcatgtacaggctataaacgccgacataaaccacaaagcccatcacccccagccagcaggccagcggattcgcgccaaaccacagcagcataaagccagcaatacccagcaacgtggcgtacaccagcgagacagcaggagagatcaggcctttcaccagcacccgattcttcgtcctttccatctttctgtcgatatccctgtcgatgtagttgttaaacacacaacccgacgccacaaccagtgacaccccaaccagcgtgtagataaacaggggataatcaatgctgccctttgaggccagcaggaatcccccaatcaccgagatcaggttgccaaagatgatgcctggtttcgttacttgcaggtattgcttaaacatcataaccgccgctcttagtgcatcatcatgttgtagttgaggttccacataatccagatggagcctacaaccaggatagcgatgattagcacggtgaagacaaacgccgtcatgttccagccttcatctgatttggtattcatgtgcaggaagcacaccagatgcaccagaacctgtaccactgccattgccaggattgttcccagaattacggccggagaggcagctcctgtcatcaccatccagaacggaatcaccgtcagaatgatcgacaggataaagcctgtcatgtaggtttttacgctgccatgggacgcgccgctgtgatcggtagaatgactcattacatcgcccccatcagataaacaacagtgaacacacagatccaaaccacatccaggaagtgccagaacaggctcaggcacatgatgcgggtacggttagtgctggtcaggccgcgacgggcgatttgcaccatcagcaccgccatccagataagaccagaagtgacgtgcagaccgtgcgtgccgaccagcgcaaagaacgctgacaggaagccgctgcgatccggacccatgccgttaacaatcaggtgatggaattcatagatttccatcccgataaatccggcaccaaacaaccaggtcaacgccagccaggagataacctggcttttgttgtttttgtacatggcgatagccgccatgccgtaggtgatggagctgaacaacagcaagaaagtttcaaccagaacgaacggcagttcgaaaatgtccttacctgtcgggccgcctgcggtgccgttcaccagaacggcataggtagcaaacaagatagagaacagaatgcagtcgctcatcaggtagatccaaaatccgaagattttggttccgcctgcatcgtggtgcccgtgttcgtgcgcgtgggcagtcgcgtgcgtcaaagtatcagttgccatttttcagccctgccttagtaatctcatcgaaatgctggttttccagtttttcgatttctgccaccggcacgtagtaatccacgtcctcgtcgaagcttttcacgatccaggtgatgatcatgcctgcgaagccaacaatcgccagccaccagatatgccagatcatggcgaaaccgaagatggtggagaaagctgcaatgacgatacctgcaccgctgtttttcggcatatgaatttcttcatagtggtcaggctttttatacgcttcgcctttctctttcatttcccagaatgcatcacgttcgtgaacgtgcggcactacggcaaagttatagaacggaggcggggaagaggttgcccactccagcgtacggccaccccacgggtcgccagtcaggtcacggttctggtcgcggtcgcgaatagaaacgtacatctgaataacgaggcagagaatacccagcgcaatcagtactgcaccgctggctgcaatcatcagcatggtgtggaactgcgggtcaatctgctggctcaaacgacgggtcatgcccatgaagcccagcgcatacagtggcataaaggcaacgaagaagccgatgatccagaaccagaacgcgcgtttaccccaggtttcgttcagtttgaaaccgaacgctttaggccaccagtaggtcatccctgcgaagcagccgaagaccacgccgccgatgatcacgttatggaagtgcgcaatcaggaacaggctgttatgcagaacgaagtccgcgcccggtacggccagcagcacgccagtcatcccgcccaccgagaaggtgacgataaaaccgatggtccacagcatcgcagaatggaacacgatgcggccctgatacatggtgaacagccagttgaagatcttcaccccggtcgggatggcgataatcattgtggtgataccaaagaaggcgtttacgttcgcgcccgcacccatcgtaaagaagtggtgcagccaaacgatgaacgacagcacggtgatacagacggttgcccataccagcgaggtataaccaaacagacgtttacgcgagaaggttgccgcaatttcggagaacacaccgaaaacaggcaggatcaggatgtaaacttccgggtggccccaggcccaaatcaggttgatgtacatcatcatgttgccacccatatcgttggtaaagaaatgggtgcccagatagcgatccagggtcaacaacgcgacggtaaccgtcagaattgggaaggaagcaataatcagtacgttcgcgcacagtgatgcccaggtaaatactggcatcttgaacatggtcatgcccggtgcgcgcatcttcagaatggtaacgaagaagttgataccggtaagcgtcgtacctataccggatagctggagactccatatccagtaatcgacaccgactcccggactgtactctattcccgatagcggtggataggccagccagccggtctgcgcaaattcgcccacgccgagagaaacgttaaccagaatcacaccaacaacggtaaaccagaagcttaagttgttgaggaacgggaacgcaacgtcacgcgcgccgatctgcagcggaaccaccaggttcatcagaccgataacgaaaggcatcgccacgaagaagatcataatcacgccgtgcgcggtaaagatctgatcgtagtggtgaggtggcaggaagcccgcttcgcccgccgaggcaagagcctgctggctacgcatcataatggcgtcagcaaaaccacgcagcaacatcacaatcgccacgatgatatacatgataccgaggcgtttatggtcgacggaggtcagccactctttccacaggtaggtccacttaccgaagtaagtgatcaggccaacgagcgccagacctcccaaaataatgccagcgatcgtaaccatgacgataggttcatggaacgggactgcatcaagtgataattttccgaacatctttattcttcctcaacccctttaatgggcggattccgcgtggctcatgtccatgccttccataccttcgtgtgcgctgtgctcaccttctggctgggtcatgtccatgctcttaccgtgagccataaacttgttaattacatcggcaaacaagtctggtttcacgttggagaaatattccacctggttgtattcgctaggcgcggccagtttttcgaacgcagccatgtcagacatggtgttcggcgactgcttcgcttttgcgacccactggtcgaatgcggcgcgatccggtgttgcaatagctttgaacttcatgcctgagaagcccgggccgctgtagctggcggagataccgtcataagtgccgggttcgttggcgatcagatgcaggcgagtctgcataccggccatggcataaatctggctacccagacgcggaatgaagaaggagttcatcacggagttggaggtcactttgaagtacaccggagtgttcgccgggaaagcgatttcattcacggtagcaatgccctgttccgggtagatgaagaaccatttccagtccatggaaaccacttcgatggtaatgggcttctcgtcgtgtgccagcggcttgctaggctcaagagcgtgagtggttttccaggtcagtactgcaaggaagatgatgattaagataggtaccgtccagaccacagcttccactttattggagtgtgaccagttcgggctgtacttagcatctttattgctcgcacggtacttccaggcgaaaccaacagccatcaagattgcgggaataacgacaatcaacatcaggccaaatgccgtcagtatcagtgaacgttgctccagaccaatctgtcctttgggatctaacagcgcagaattacagccactgagcaatacagtgcctgcaaataatgacaaccatcccaaacttttattgtatttcctgagtctcatttaacgacctcaattccacgggatctggtggcgtttaaagtgtgtgggcattttacgggaaggttacattactgtaaacatgattaaattcctgttacttggatttggctgccaggtcacatatgttgcaaaacatatcaggttgattttaagaagctgttgcaaaagggcgttataacaaaaggggagtgctgaaggagtctgggcgggcaattggtataaccaatgtgaaataaaacaattatttaacaaataattatcattagagtgacaactgggtgatgagaaaataaagactcattagctgaatcgtgtaagaaaaatagaatttataaatggcgccaataatttccaaacgctaagccgcacaaaagaacaaatattaataagcgatactgatgtttatttagccgtaataattacggcgagtgattactacagctaaataatatttacagattacgtcagatgcgtttttcgtagcgccagataatccagcaaaccaccaagcacgacgccagaaagggcgactaaaaccccgacttccagcagagcaggcaggaaagagaagtgcgtcaaatccagcgcgtccatcgtcaatagcagtaaccacacggccaacaggctgacgcccgccgccagtgtccacatggcaaaggcataacctgccggatatgcggtacgggagataaagttgtcatttactcgtgtatattcaagcgtctggcggcaaaccagcagcaaaataagccctggtacggcagcggcgacggagaatagatagaatgtcgaccagccgtgtgcttcaacaaaccaacccgccacggggccgacataaactcgccctacagcagaaagcgctgagagcagggcaaattgagtagcggaaaatgacttattacatagcgtcattaacagcgcgacaaaggctgatgtgcccatcccgccacagaggttttcgaaaaagacggctgcgcccatgctgtagagatgcttatcagtaatcgacagcagccagtaaccggcgttagacgcaccttgtaaaatgccgaaaatcagcagtgcccggaacagtgacaggcgctgcatcaaaatcccaccgtacaatgcgccaacaatggtcgctagtaagccaagcgttttgttaaccacgcctacttcacccgcatcaaacccgacgccgcgaatcaaaaacgtggttgtcaggctcatggcgaatgcgtcgcccagcttatacagcacgataagaagcaaaataagccaggcattattgcgaccaaagaaatctcgcagaggtgcaacaaccgcttgttccagcgttttgggcacaggaatggtgtcggttggttctggtgcaagcaacgtcgcgataatacaggggatcaacagtgccgccattaaccagtacatgccctgccagcccagccatttatctgccagccacagggctaggccgccggaaaccagcatccctaaacggtaacccagcacgctgattgccgcgcccgcaccacgttcttctgccggaagcacatcggttttccacgcatcgaagactatatcctgggaagcagagcaaaaagcgatcaccactgccagcgccgccatccagcggagttgggtgcctggttcgagaaaacccatcgccgcaatggcgactaataacaggatttgcgtggcgagcagccaaccgcgccgccgcccaaaaaatggaggcgtgtagcggtccatcagcggtgaccagaggaatttaaaaacgtaagcctggcctaccagagagaagaaaccaatggttttgagatcgatattctcgaccgtcatccaggcctgtaaggtaccggatgtcagggcgagcggtagcccggaagcaaaacccaggatcagcaatatggctgaacgcggctgttgaaaaatacgtaaatattgactggacatgggcgtctacaggcccggcttgcaccgggccagagggcagaaattaacgcgcgttctgcttgatgaattcgtggatgctggtgtcctgagacatatcagcgatggtatcggtcagcacactgttaaccgcatcggcgatatttttgttggaggcctggaacgcaccttcaacgttgtagctggcacgatagtttttggtcattttgttgccattctgcgcggtagcgatgatggcgatatccgctttggtcgcgatgttgtagcgcacgttgccctgggacacgtcagcatacagttggctaacgatgatttgcagattaaccgggccattcggaccaaccatgtaaccacgcgcggtcatctgtttttccagcacttcttgcagcaggaaacgcagatcgcgggaggcggtcagggtaacgatttgattatcgcgggtgacttttgccagcgcctgatcggtacgctgatcggcaccattaatgcttacggtgacgcccatcaggcttggatcctgctgtggcagtgtaatcgtcggggaaacttcaatagttgttggcggttttgcgcatcctgcaagcataaacagagcaactaacgggaagaggatttttttgaacatgttcgggctctcagagactcttaagcgtgtttggtaaaaattcccgccatcataacattgccaacggcgaggggaagtgggtaaggcatgtaaattcatcatgttgacgaaataatcgcccctggtaaaagaaacactgatgcgaggcctgtgtttcaatctttaaatcagtaaacttcatacgcttgacggaaaaaccaggacgaaacctaaatatttgttgttaagctgcaatggaaacggtaaaagcggctagtatttaaagggatggatgacatctcagcgttgtcggaggagatatttcatgatgatacgtgagcggatagaagaaaaattaagggcggcgttccaacccgtattcctcgaagtagtggatgaaagctatcgtcacaatgtcccagccggctctgaaagccattttaaagttgtgctggtcagcgatcgttttacgggtgaacgttttctgaatcgtcatcgaatgatttacagtactttagcggaggaactctctactaccgttcatgcgctggctctgcatacttacactattaaggagtgggaagggttgcaggacaccgtctttgcctctcctccctgtcgtggagcaggaagcatcgcgtaaaaacgcatttgcaactgtcggcgcttttccagtatgttgctaaagattttatgaaaaacggcctgcgggccgttttgttttgtctggattttgcgctttttgcccagcattcagacgaaaattgcccgggaattgtgaaaaaatacgcgacagcgcgcaataaccgttctcgactcataaaagtgatgccgctataatgccgcgtcctatttgaatgctttcgggatgattctggtaacagggaatgtgattgattataagaacatcccggttccgcgaagccaacaacctgtgcttgcggggtaagagttgaccgagcactgtgattttttgaggtaacaagatgcaagtttcagttgaaaccactcaaggccttggccgccgtgtaacgattactatcgctgctgacagcatcgagaccgctgttaaaagcgagctggtcaacgttgcgaaaaaagtacgtattgacggcttccgcaaaggcaaagtgccaatgaatatcgttgctcagcgttatggcgcgtctgtacgccaggacgttctgggtgacctgatgagccgtaacttcattgacgccatcattaaagaaaaaatcaatccggctggcgcaccgacttatgttccgggcgaatacaagctgggtgaagacttcacttactctgtagagtttgaagtttatccggaagttgaactgcagggtctggaagcgatcgaagttgaaaaaccgatcgttgaagtgaccgacgctgacgttgacggcatgctggatactctgcgtaaacagcaggcgacctggaaagaaaaagacggcgctgttgaagcagaagaccgcgtaaccatcgacttcaccggttctgtagacggcgaagagttcgaaggcggtaaagcgtctgatttcgtactggcgatgggccagggtcgtatgatcccgggctttgaagacggtatcaaaggccacaaagctggcgaagagttcaccatcgacgtgaccttcccggaagaataccacgcagaaaacctgaaaggtaaagcagcgaaattcgctatcaacctgaagaaagttgaagagcgtgaactgccggaactgactgcagaattcatcaaacgtttcggcgttgaagatggttccgtagaaggtctgcgcgctgaagtgcgtaaaaacatggagcgcgagctgaagagcgccatccgtaaccgcgttaagtctcaggcgatcgaaggtctggtaaaagctaacgacatcgacgtaccggctgcgctgatcgacagcgaaatcgacgttctgcgtcgccaggctgcacagcgtttcggtggcaacgaaaaacaagctctggaactgccgcgcgaactgttcgaagaacaggctaaacgccgcgtagttgttggcctgctgctgggcgaagttatccgcaccaacgagctgaaagctgacgaagagcgcgtgaaaggcctgatcgaagagatggcttctgcgtacgaagatccgaaagaagttatcgagttctacagcaaaaacaaagaactgatggacaacatgcgcaatgttgctctggaagaacaggctgttgaagctgtactggcgaaagcgaaagtgactgaaaaagaaaccactttcaacgagctgatgaaccagcaggcgtaatttacgcagcataacgcgctaaattcgcacaaaggcccgtcaccgccaggtggtgggcttttttttgtcatgaattttgcatggaaccgtgcgaaaagcctctttcggtgttagcgtaacaacaaaagattgttatgcttgaaatatggtgatgccgtacccataacacagggactagctgataatccgtccataaggttacaatcggtacagcaggttttttcaattttatccaggagacggaaatgtcatacagcggcgaacgagataactttgcaccccatatggcgctggtgccgatggtcattgaacagacctcacgcggtgagcgctcttttgatatctattctcgtctacttaaggaacgcgtcatttttctgactggccaggttgaagaccacatggctaacctgattgtggcgcagatgctgttcctggaagcggaaaacccagaaaaagatatctatctgtacattaactccccaggcggggtgatcactgccgggatgtctatctatgacaccatgcagtttatcaagcctgatgtcagcaccatctgtatgggccaggcggcctcgatgggcgctttcttgctgaccgcaggggcaaaaggtaaacgtttttgcctgccgaattcgcgcgtgatgattcaccaaccgttgggcggctaccagggccaggcgaccgatatcgaaattcatgcccgtgaaattctgaaagttaaagggcgcatgaatgaacttatggcgcttcatacgggtcaatcattagaacagattgaacgtgataccgagcgcgatcgcttcctttccgcccctgaagcggtggaatacggtctggtcgattcgattctgacccatcgtaattgatgccagaggcgcaactgtgccgctatacttatccagggcggcacaacgctgtaagcggcttgcgcctgagaatggcatttgcgtcgtcgtgtgcggcacaaagaacaaagaagaggttttgacccatgacagataaacgcaaagatggctcaggcaaattgctgtattgctctttttgcggcaaaagccagcatgaagtgcgcaagctgattgccggtccatccgtgtatatctgcgacgaatgtgttgatttatgtaacgacatcattcgcgaagagattaaagaagttgcaccgcatcgtgaacgcagtgcgctaccgacgccgcatgaaattcgcaaccacctggacgattacgttatcggccaggaacaggcgaaaaaagtgctggcggtcgcggtatacaaccattacaaacgtctgcgcaacggcgataccagcaatggcgtcgagttgggcaaaagtaacattctgctgatcggtccgaccggttccggtaaaacgctgctggctgaaacgctggcgcgcctgctggatgttccgttcaccatggccgacgcgactacactgaccgaagccggttatgtgggtgaagacgttgaaaacatcattcagaagctgttgcagaaatgcgactacgatgtccagaaagcacagcgtggtattgtctacatcgatgaaatcgacaagatttctcgtaagtcagacaacccgtccattacccgagacgtttccggtgaaggcgtacagcaggcactgttgaaactgatcgaaggtacggtagctgctgttccaccgcaaggtgggcgtaaacatccgcagcaggaattcttgcaggttgatacctctaagatcctgtttatttgtggcggtgcgtttgccggtctggataaagtgatttcccaccgtgtagaaaccggctccggcattggttttggcgcgacggtaaaagcgaagtccgacaaagcaagcgaaggcgagctgctggcgcaggttgaaccggaagatctgatcaagtttggtcttatccctgagtttattggtcgtctgccggttgtcgcaacgttgaatgaactgagcgaagaagctctgattcagatcctcaaagagccgaaaaacgccctgaccaagcagtatcaggcgctgtttaatctggaaggcgtggatctggaattccgtgacgaggcgctggatgctatcgctaagaaagcgatggcgcgtaaaaccggtgcccgtggcctgcgttccatcgtagaagccgcactgctcgataccatgtacgatctgccgtccatggaagacgtcgaaaaagtggttatcgacgagtcggtaattgatggtcaaagcaaaccgttgctgatttatggcaagccggaagcgcaacaggcatctggtgaataattaaccattcccatacaattagttaaccaaaaaggggggattttatctcccctttaatttttcctctattctcggcgttgaatgtgggggaaacatccccatatactgacgtacatgttaatagatggcgtgaagcacagtcgtgtcatctgattacctggcggaaattaaactaagagagagctctatgaatcctgagcgttctgaacgcattgaaatccccgtattgccgctgcgcgatgtggtggtttatccgcacatggtcatccccttatttgtcgggcgggaaaaatctatccgttgtctggaagcggcgatggaccatgataaaaaaattatgctggtcgcgcagaaagaagcttcaacggatgagccgggtgtaaacgatcttttcaccgtcgggaccgtggcctctatattgcagatgctgaaactgcctgacggcaccgtcaaagtgctggtcgaggggttacagcgcgcgcgtatttctgcgctctctgacaatggcgaacacttttctgcgaaggcggagtatctggagtcgccgaccattgatgagcgggaacaggaagtgctggtgcgtactgcaatcagccagttcgaaggctacatcaagctgaacaaaaaaatcccaccagaagtgctgacgtcgctgaatagcatcgacgatccggcgcgtctggcggataccattgctgcacatatgccgctgaaactggctgacaaacagtctgttctggagatgtccgacgttaacgaacgtctggaatatctgatggcaatgatggaatcggaaatcgatctgctgcaggttgagaaacgcattcgcaaccgcgttaaaaagcagatggagaaatcccagcgtgagtactatctgaacgagcaaatgaaagctattcagaaagaactcggtgaaatggacgacgcgccggacgaaaacgaagccctgaagcgcaaaatcgacgcggcgaagatgccgaaagaggcaaaagagaaagcggaagcagagttgcagaagctgaaaatgatgtctccgatgtcggcagaagcgaccgtagtgcgtggttatatcgactggatggtacaggtgccgtggaatgcgcgtagcaaggtcaaaaaagacctgcgtcaggcgcaggaaatccttgataccgaccattatggtctggagcgcgtgaaagatcgaatccttgagtatcttgcggttcaaagccgtgtcaacaaaatcaagggaccgatcctctgcctggtagggccgccgggggtaggtaaaacctctcttggtcagtccattgccaaagccaccgggcgtaaatatgtccgtatggcgctgggcggcgtgcgtgatgaagcggaaatccgtggtcaccgccgtacttacatcggttctatgccgggtaaactgatccagaaaatggcgaaagtgggcgtgaaaaacccgctgttcctgctcgatgagatcgacaaaatgtcttctgacatgcgtggcgatccggcctctgcactgcttgaagtgctggatccagagcagaacgtagcgttcagcgaccactacctggaagtggattacgatctcagcgacgtgatgtttgtcgcgacgtcgaactccatgaacattccggcaccgctgctggatcgtatggaagtgattcgcctctccggttataccgaagatgaaaaactgaacatcgccaaacgtcacctgctgccgaagcagattgaacgtaatgcactgaaaaaaggtgagctgaccgtcgacgatagcgccattatcggcattattcgttactacacccgtgaggcgggcgtgcgtggtctggagcgtgaaatctccaaactgtgtcgcaaagcggttaagcagttactgctcgataagtcattaaaacatatcgaaattaacggcgataacctgcatgactatctcggtgttcagcgtttcgactatggtcgcgcggataacgaaaaccgtgtcggtcaggtaaccggtctggcgtggacggaagtgggcggtgacttgctgaccattgaaaccgcatgtgttccgggtaaaggcaaactgacctataccggttcgctcggcgaagtgatgcaggagtccattcaggcggcgttaacggtggttcgtgcgcgtgcggaaaaactggggatcaaccctgatttttacgaaaaacgtgacatccacgtccacgtaccggaaggtgcgacgccgaaagatggtccgagtgccggtattgctatgtgcaccgcgctggtttcttgcctgaccggtaacccggttcgtgccgatgtggcaatgaccggtgagatcactctgcgtggtcaggtactgccgatcggtggtttgaaagaaaaactcctggcagcgcatcgcggcgggattaaaacagtgctaattccgttcgaaaataaacgcgatctggaagagattcctgacaacgtaattgccgatctggacattcatcctgtgaagcgcattgaggaagttctgactctggcgctgcaaaatgaaccgtctggtatgcaggttgtgactgcaaaatagtgacctcgcgcaaaatgcactaataaaaacagggctggcaggctaattcgggcttgccagcctttttttgtctcgctaagttagatggcggatcgggcttgcccttattaaggggtgttgtaaggggatggctggcctgatataactgctgcgcgttcgtaccttgaaggattcaagtgcgatataaattataaagaggaagagaagagtgaataaatctcaattgatcgacaagattgctgcaggggctgatatctctaaagctgcggctggccgtgcgttagatgctattattgcttccgtaactgaatctctgaaagaaggggatgatgtagcactggtaggttttggtacttttgccgttaaagagcgtgctgcccgtactggccgcaacccgcagaccggtaaagagatcaccatcgctgctgctaaagtaccgagcttccgtgcaggtaaagcactgaaagacgcggtaaactaagcgttgtccccagtggggatgtgacgaagttcaagggcgcatctactgatgtgccttttttatttgtattcggtgactttctgcgtcttgtgggctgacaattgcccccgtttcttgtcacaataggcctttgcgcgcatcgatacgttgcgtgaggtacacagtcatctacagcggagtgttgttacaccatgatggacagcttacgcacggctgcaaacagtctcgtgctcaagattattttcggtatcattatcgtgtcgttcatattgaccggcgtgagtggttacctgattggcggaggcaataactacgccgcaaaagtgaatgaccaggaaatcagccgtgggcaattcgagaacgccttcaacagcgagcgtaatcgcatgcagcaacagctgggcgatcaatactccgagctggcagcgaacgaaggctatatgaaaaccctgcgtcaacaggtgctgaatcgtctgatcgacgaggcgctgctggatcagtacgcacgtgagctgaaactgggtatcagcgatgagcaggttaaacaggcgattttcgcgaccccagccttccaggttgacggcaaatttgataacagccgctataacggtatcctcaaccagatggggatgaccgccgatcagtacgcccaggcgctgcgtaaccagctcactacccaacagctgattaacggcgttgccggtaccgattttatgctgaaaggtgaaaccgacgagctggcggcactggtcgcgcaacaacgcgtggtgcgtgaggcgactatcgatgttaacgcgctggcggcgaagcagcctgtgaccgaacaggagattgccagctactacgaacaaaacaaaaacaatttcatgacgccggaacaattccgcgtgagttacatcaagctggatgccgcaacgatgcagcaaccggttagcgatgcggatatccagagctactacgaccagcatcaggatcaattcacccagccgcagcgtacccgctacagcatcatccagaccaaaactgaagatgaagcgaaagcggtacttgatgagctgaataaaggcggtgattttgctgcattagccaaagaaaaatctgccgatattatctctgctcgtaacggcggcgatatgggttggttagaagatgccactatcccggacgaactgaaaaatgctggtctgaaagaaaaaggccaactgtctggtgtcatcaaatcttcggtcggtttcctgattgtacgtctggacgacattcagccagcgaaagtgaaatcgttagacgaagtacgtgacgacattgcggcgaaagtgaaacacgaaaaagccctcgatgcgtactacgcgctgcagcagaaagtgagcgatgcggcaagcaacgacaccgagtctctggccggtgcagagcaagctgccggcgttaaagccactcagacgggttggttcagcaaagataacctgccggaagagttgaacttcaagccggttgccgacgctatctttaacggcggtctggtaggtgaaaacggcgcgccgggcatcaactctgacatcatcaccgtagacggcgaccgcgcattcgtgctgcgcatcagcgagcacaaaccggaagcggtgaaaccgttggcagatgttcaggaacaagttaaggcattggttcagcacaacaaagctgaacaacaggcgaaagtggatgctgagaaactgctggttgatttgaaagccggcaaaggtgcggaagctatgcaggctgccggtctgaaatttggcgagccgaaaaccttaagccgttccggtcgtgacccgattagccaggcggcgtttgcactgccactgccagcgaaagacaaaccgagctacggtatggcgaccgatatgcaaggtaatgtggttctgctggcgctggatgaagtgaaacaaggttcaatgccggaagatcagaaaaaagcgatggtgcagggtatcacccagaacaacgcacaaatcgtctttgaagctctgatgagtaacctgcgtaaagaggcgaaaatcaaaattggcgatgcgctggaacagcaataatcctgaagccgcctcgcaaaaaaatgcgttgcagctgtaacaagaaaaggtcgctttcgcggccttttccatttctgaacattgccatttgtttactgttttcactgccgttaaggtgattccactgttaacaaacaaggagaaaacagtatgaaacacggaattaaagcactgctcattaccctgtccctggcctgtgccggaatgtctcatagcgcgctggcggcagcttctgtggcgaaaccgacggcggtagaaaccaaagcggaagctcctgcagcacaaagtaaagcagcagtaccggcgaaagccagtgacgaagaaggcacccgggtcagcattaataatgccagcgcggaagagctagcccgcgcgatgaatggcgttggcctgaagaaagcgcaggcgattgtcagttatcgcgaagagtacggtccgtttaaaactgtggaggatctaaagcaggtgccggggatgggcaattcgctggtggaacgtaatctggcggtattaaccctgtaattaatttgcatagtggcaattttttgccagactgaagaggtcataccagttatgacctctgtacttataacaacaacgtaaggttattgcgctatgcaaacacaaatcaaagttcgtggatatcatctcgacgtttaccagcacgtcaacaacgcccgctaccttgaatttctcgaagaagcccgctgggatgggttggaaaatagcgacagttttcagtggatgacggcccataacatcgccttcgtcgtggtcaatatcaatattaactatcgtcgcccagcggtattaagtgacctgttaactattaccagtcagttgcagcaattaaacggtaaaagcggcatcttaagccaggtcattacactggagccggaagggcaggtggtagcggatgcgcttattacgtttgtttgtattgatcttaaaacgcagaaagcattagctctggaaggggaattgcgcgaaaagctggagcagatggttaagtaaacgttttgtggtgccggatgctcaagccgcatccggcgacacccggaataattacctcaacccggttttctgcttcatcgctgccatcaccgtcggtttatcggccagataatgattcaaaccgttggcgcgtaaattacatgccgcacaatgaccgcaaccgtcgcctttaaagccgttatagcaggtcaacgtttcgttacggactaaatccagtttgccgtaataatctgccagcgcccaggtttccgctttatcaatccacatcagcggcgtttcaaaacgaatatctttcgccatgcccaaactgacggcatggtttagtgctttcacaaactcatcgcggcaatccgggtagccggagaaatccgtttcgcagacgccagtaattacggcttctgcttttacctgatacgcatatattgccgccagcgtcaggaacaaaatattacgccctgggacaaacgtattcgggataccatcggcttcaggttcataatcaggcaccggaatgctgtcacgcgtcaggctactgaccgccagctcgttgagcagggtgacatccagcaccttatgcgcgcgtgcccccagtttcagcgccagttcgcgtgccacgtcgatttctgcgcgatgccgctgaccgtaatcgaacgtcacgcaatggacttcatcatattgttgtaatgcctgcaccagacaggtggtggaatcctgacctccactgaacacaacgacagcacgtttcatagataatcctgcttgaacaataaaagcgttatggtaacgcctgcgattaacccggaccagctattcattgcgatggcgcgggaagccaggcttcggtaaattcaaaccagccgcgcggtgtcagtcgcacaccgttcacgccgggaggggcactaatgcgatagtgatagttgaacagcggcgtcagcgtcgcatctgtcattaactggctaaaaaccgctttcagggcattaaatcggttttcttcatcaggcattatttgcacggcatccagtgtcgattgtagatgtgcgtatgctggagcgtcgaaaacatgtggccacagcggatcgcagcgcagccattgctccagagtatattccggtgcttcgccaattaatctgtcgcccatcatgaggtctgcgtgtgcctgtagggtcgtgtcgtcccagttttttgcgttatgaaaaataattgtgagttcacagccttccgctgccagtgtcgcctgtaggcgttctgccatggtatgaagttctatcggtaggtgataaaccagcgtcaaggttttcggtagtttgacttcatccggtacctgccaatgcggaatagtccagcctggcagtaatgcatgactggcggtgatcaggttttctccgacttctaacgtttgtaataaaccggattgatgaataatggagatcacttttcgcgcctgccagagggagagtcggggacttttgcgcaacgtcaaatagcaaaaacctaaactgatgccgctactgacctggctgacccgttgcagctcctccggtttgccgatggtgatttgcacgggatgccgacaactggttcccaaatctttttcgaaaagcggcggagttatccagtactcaaccgctttaagcagcggatgacgtaaatggtaataatcatggctttccaggcgcaccagctctgctgtgaattgtgttaagcgaaaaggacccgtgccgatcagtgggaattgcggatgcgccagatggctgcaatagctcgccagccggtgcgcaagccagtaatcagggcgatgtaaaaagaaggtcagacactgcggatgggtgacttcaatacgcttcacgctaataaataattgatccagtgctggcagttgtaacagcatcaataatcgctggtgtaagtgtgaggcttttactgcatcgccgttatgccagtgtagggttgaacgaagataaaagtcccagcgtaacccgtcagtagaggtttcccagtgatgcgctaaatcgccaatcgggcgctgagtattattatcgaagcgggtcaggccggaaaatatctgcccggcgagatgctgctcggcacggccgggcaaaaagcctggttgtagcggttcgagcgggcgatagtagggaatacgcaacgtgggtgtatcgttttgccattgtccgcccataaacggctgtaacagagtgcgcagctcacctggggccagttgcgccagctccagcacatcttgctgctttccggtttccagtgcctgttccatcatcgcattgcgtagcgattccggcgtgaccagaaagcgtaattgtccgcgctttccgcgtcctgactgcgcctgccactccagccatcccgcctcctgtgcctgacgcaacagcgtacgaacatggcgttcgctgcaaaaacagcgttcggccagttcgctgacggtgacggtttgcggctttccggcggaaggttgccacagacgttgatactggttaagacggttgagcaatcgcatataaacccggaacaatattatttaactattcactattacttccgtatatatcaggtgatactcaatcaccattaaccgtgtcacagagtggagaaagaaatggctcgtctggcagcatttgatatggatggcactttattgatgcccgaccatcatttaggtgagaaaaccctctctactttggcgcgactgcgtgaacgcgacattaccctcacttttgccacggggcgtcatgcgctggagatgcagcatattctcggggcgctatcgctggatgcgtatttgattaccggcaacggaacgcgcgtgcattctctggaaggtgaacttttacatcgtgatgatttacctgcggatgtcgcggagctggtgctgtatcagcaatgggatacccgagccagcatgcatatcttcaatgacgacggttggtttaccgggaaagagatccctgcgttgttgcaggcatttgtctatagcggttttcgttatcagataatcgatgtcaaaaaaatgccactcggcagcgtcaccaagatctgcttctgtggcgatcacgacgatcttacacgcttgcagatccagctatacgaagcattaggcgagcgtgcacatttgtgtttttccgccacggattgcctcgaagtgctgccggtgggctgcaataaaggcgctgcattgacggtgctgacccaacatttaggtttatcgttgcgcgattgcatggcctttggtgatgcgatgaacgatcgcgaaatgttagtcagcgtcggtagcggatttattatgggcaatgcgatgccgcaactgcgcgcggagctcccgcatttaccggtgattggacattgccgaaatcaggctgtctctcactatttgacgcactggctggactatccacatctaccttattcccccgaataacgagatcccttccagcaccgggcaattgcccggttttttttgcgttgaatttgtcattttgtgccgtggtgtttaaaccgcacagaataaattgtcgtgatttcacctttaaaataaaattaaaagagaaaaaaattctctgtggaagggctatgttagataaaattgaccgtaagctgctggccttactgcagcaggattgcaccctctctttgcaggcactggctgaagccgttaatctgacaaccaccccttgctggaagcgcctgaaacggctggaggacgacggtatccttatcggcaaagtcgccctgctggatccggaaaaaataggcctcggcctgaccgcttttgtgctgataaaaacgcaacatcacagcagcgaatggtattgccgctttgtcacggtggttaccgaaatgccagaagtgctggggttctggcgcatggctggtgaatacgattatctgatgcgcgtccaggttgccgacatgaaacgctacgacgagttttataagcgtctggtaaacagcgtgccggggctgtcggacgtcacttccagcttcgcgatggaacagattaaatacaccacttctttacccatcgaataaatatccagaatcaggtcaggacacaacgcgtgcgattatttgctcaattaagctggtatttccgtcgggaatggcgtcgctatctcggggctgtcgccttgcttgtcattatcgcgatgctgcaactggttccgccaaaagtggttggtattgttgtcgatggcgtgacagaacaacactttactaccgggcagatcctgatgtggatcgccaccatggtgctgattgccgttgtggtttatctcctgcgttacgtctggcgggtattgctgtttggtgcgtcttatcaactggctgttgaactgcgtgaagattattaccgtcagctaagccggcagcatcctgagttttacctgcgtcatcgcaccggtgacctcatggctcgtgcgaccaatgacgtcgatcgcgtcgtgtttgccgccggagaaggggtgctgacgctggtggattcactggtgatgggctgcgctgtgttgattatgatgtctacgcaaattagctggcagttgaccttattttccctgttgccgatgccagtgatggcgatcatgattaagcgcaacggcgatgctttgcatgaacgctttaagctggcacaggcggcgttttccagtcttaatgaccgcacccaggaaagcctcaccagtatccgcatgatcaaagcctttggtctggaagatcgccagtcggcgttatttgccgcggatgccgaagataccggcaaaaaaaacatgcgggtggcgcgtattgatgctcgtttcgacccgaccatctatatcgcgattggtatggcgaacttgctggcgattggcggcggtagttggatggtggtgcagggcagtttaacgctgggccagctcaccagttttatgatgtatttaggtctgatgatttggccaatgctggcgctggcatggatgtttaacattgtggaacgtggtagtgctgcgtacagccgtattcgcgcgatgctggcggaagcgccggtggtgaacgatggtagcgaacccgtgccggaagggcgtggcgaactggatgtaaatattcaccagttcacgtatccgcagactgaccatcctgcgctggaaaacgtcaatttcgccctgaaacccggtcagatgctgggtatctgcgggccgactggttccggcaaaagtaccctgttgtcgctcattcagcgtcatttcgacgtcagcgagggggatattcgctttcatgatattcctctgacgaagttacaactcgatagctggcgtagccgcctggcggtagttagccagacgccattccttttttctgacactgtggcgaataacatcgcgctgggttgcccgaatgccacccagcaagagattgagcatgtcgcgcggttagccagcgtacatgacgatattttgcgtctaccgcaaggttacgatacagaggtgggcgagcgcggtgtgatgctttccggcgggcaaaaacagcgtatctccattgctcgtgcgttattagtcaacgcggaaatcctcatccttgatgatgcgctttcggcggtggacggacgcactgagcaccagatcctgcataacctgcgtcagtgggggcagggaagaacggtaatcatcagtgcccatcgcctttctgcactgacggaagccagtgaaattattgtgatgcagcacggacatatcgcccagcgtggcaatcatgatgtgctggcacaacaaagcggctggtatcgcgatatgtatcgctatcaacaactggaggcggcgctcgacgacgctccggaaaatcgcgaggaggccgtcgatgcgtagttttagccaactgtggccgactctcaagcgcctgttagcgtacggttcgccgtggcgtaaaccgctggggattgcggtcctgatgatgtgggttgcggcggcggcagaagtcagtgggccgctgcttatcagctattttatcgacaatatggtagcgaaaaataacctgccgttgaaagtggttgcagggctggctgcggcgtatgttgggctgcaactgtttgccgccgggctacattacgcgcagtcgctgctgtttaatcgggcggcagtaggcgtagtgcaacagttgcgtaccgacgtgatggatgctgcgttacgccagccattaagcgagtttgatacccaacccgtcgggcaggtgatttcccgcgtcactaatgacactgaagtgatccgcgatctctacgttaccgtagtggcaactgtcctgcgcagtgccgcgctggtgggcgcgatgctggtggcgatgttcagcctcgactggcgaatggcactggtggcgataatgattttcccggtggtgctggtggtaatggtgatataccagcgttacagcacgccgattgtccgtcgtgtgcgcgcctatttggcggatatcaacgacggctttaacgaaatcatcaatggcatgagcgttatccagcagtttcgtcagcaggcgcgatttggcgaacgtatgggggaggccagtcgttcacactatatggcgaggatgcaaaccctgcgcctcgacggttttctgctgcgtccgctgctgagtctgttttcatcgctcattctttgtggcttgttgatgctgtttggcttctccgccagcggcaccattgaagtgggcgtgctgtatgcgtttatcagctatcttgggcgacttaacgaaccattaatcgaactgaccacgcaacaggcgatgctgcaacaggctgttgttgctggtgagcgcgtgtttgaactgatggacggaccgcgccagcaatatggcaatgatgatcgcccgttacagagtggcaccatcgaagtcgataacgtgtcatttgcttatcgcgatgacaatctggtgctaaagaacattaatctctctgtgccttcgcgcaattttgtggcgctggtcgggcataccggcagtggcaaaagcaccctcgccagtttattgatgggctattacccgctaacggaaggtgagattcgccttgatggtcgtccattaagttcgctaagtcacagcgcgctgcgccagggcgtggcaatggtgcagcaagatccggtggtgctggcggataccttcctcgccaacgtgacgctggggcgggatatctccgaagaacgcgtctggcaggcgctggaaaccgtgcaactggcggagctggcgcgtagcatgagcgacggtatttacacgccgctgggcgagcaggggaataatctctcagttgggcaaaagcaactgctggcactggcgcgcgtgctggtcgagacgccgcaaatcctgatccttgatgaggcaaccgccagcattgactccggtactgaacaggcgattcaacatgctctggcggcggtgcgtgaacataccacgctggtagtgattgctcaccgcttatcgaccattgttgatgccgacaccattctggtgcttcatcgtgggcaagccgtggagcagggcactcaccagcaactgctggcggcccagggacgctactggcagatgtatcaactgcaacttgcgggcgaagagctggcagccagcgtgcgtgaagaggaatcattgagcgcctgaatagcgcaatatttcatcgttggtgcaaaaatgtaacgcactgtgcactgtcatagtgcgttttcattttcaaacttcttaacttcctgctctctttctcgtttttcatttctggcacaccgcttgcaataccttcttcgtgtagcagaaccattaccgaattctgaccggaggggatctatgaagctggtgaccgtgataatcaaaccattcaagctggaagacgttcgtgaagcgttatcttccattggtattcagggcctgaccgtcaccgaagtgaaaggtttcgggcgtcagaaagggcatgccgagctgtaccggggggcggaatacagcgtcaatttcctgccaaaagtaaaaattgatgtggcgattgctgatgaccaactcgatgaagtgatcgatatcgtcagtaaggcggcttacaccggaaaaattggcgacggcaaaatcttcgtcgctgaattgcaacgcgtcattcgtattcgtaccggcgaagccgacgaagcggcgctgtaatctctggcacacagcaacaggaacgaaaaatgaagatagcgacgataaaaactgggcttgcttcactggcgatgcttccgggactggtaatggctgcacctgcggtggccgataaagccgacaatgcgtttatgatgatttgtactgcgctggtgctgtttatgactattccggggattgccctgttttacggtgggttgattcgcggcaaaaacgtgctgtcgatgctgacgcaggtgacggtgacatttgcactggtctgtattctctgggtggtttacggttactcgctggcgtttggtgagggcaacaacttcttcggcaacattaactggttgatgctgaaaaacatcgaactgacggcggtgatgggcagcatttatcagtatatccacgtggcgtttcagggatcgtttgcctgcattaccgtcggcttgatagttggggcgctggcggaacgaatccgcttctcagctgtgttgattttcgtggtggtatggctgacgctctcttacattccgattgcgcatatggtgtggggcggtggtttgctggcttctcacggtgcgctggatttcgcgggtggcaccgtggtgcacattaacgccgcaatcgccggtctggtgggcgcgtatctgataggaaaacgcgtgggcttcggtaaagaggcgtttaaaccgcacaacctgccgatggtcttcaccgggactgccattctctatatcggttggtttggctttaacgccgggtcagcgggcacggcgaatgaaatcgcggcactggcatttgtgaatactgtggtcgcaacggcggcggcaattcttggctggatcttcggtgaatgggcgctgcgtggtaagccttcactgctgggggcgtgttctggcgcgattgccggtctggtcggcgtgacgccagcctgcggctacattggggttggcggcgcgttgattatcggcgtggtagctggtctggcgggcttgtggggcgttaccatgctcaaacgcttgctgcgggtggatgatccctgcgatgtcttcggtgtgcacggcgtttgtggcattgtcggctgtatcatgaccgggatttttgccgccagctcgctgggcggcgtgggcttcgctgaaggtgtgacgatgggccatcagttgctggtacagctggaaagcatcgccattacgatcgtctggtccggtgttgtggcatttatcggctacaaattggcggatctgacggttggtctgcgtgtaccggaagagcaggagcgagaagggctggatgtcaacagccacggcgagaatgcctataacgcgtaacaagcactgcaaaaaacagccggacggttttcacctccggctatttttttaattgtgattacgcatcaccccttcctgaacggtcgaggcaaccagtacgccgtcttgggtataaaactcaccgcgcacaaagccacgtgcgctggacgccgaggtgctctccacgctatacagcagccattcattcaaattaaacgggcgatggaaccacatggaatggtcaatggtggcaatctgaatccccggttcgagaaaaccgatgccgtgcggctgtagagctaccggcaggaagttaagatcagaagcgtaaccgagcagatactgatgaacgcgcaggtcatccggcacgctaccatttgcgcggatccacacctgacgatgtggttctgcgacgtgacctttcagtgggttatgaaactccaccggacggacttccagcggacgatcgcagatgaatttatctttcagcactggcggcagcaggtgcgccagcgattgggcgatttgcgtttccgaagggaggccatcaggcgctggcgcggacggcattgttttttgatgttcgaaacccgcttctggtgcctggaaagaggcagtcatataaaaaatcggtttgccgttttgaatagcagcaacccggcgggcgctgaagctgttaccgtcacgcagcgtttcgacatcataaataatcggcttcttactatcgccagggcgaagaaagtagctgtgaaacgaatgtaccagccgctcttcagggacggtctcttttgcagcatacaaggcctgacccacgacctggccgccaaacacctggcgtaaacctaaatcttcactctggccgcgaaagagtccttcctcaattttttccagatttaacaatgtcagtaaattttttagcgcctgactcatataactctccagtaacaaagctgccgcagcaagccaaagtgagttgagtataacgcaaatttgctactggtccgatgggtgcaatggtctgaattacgggctaattacaggcagaaatgcgtgatgtgtgccacacttgttgacgttactattttgttaaccactcttccggcgaggaaagttagcccgctggtgcattgataataaggagaaatgaatgaaactcgtgcacatggccagtggtttagcggttgcgattgcgttggcggcttgcgcagataaaagcgcggatattcagacgccagcaccggctgcaaatacgtctatttcagcaacacaacaaccagctatccagcaaccgaatgtctccggtaccgtctggatccgtcagaaagtcgcactgccgcctgatgctgtgctgaccgtgacactttctgacgcgtcgttagccgatgcaccgtcaaaagtgctggcgcagaaagcggtgcgtactgaaggtaaacagtcaccattcagctttgttctgtcatttaacccggcagatgttcagccgaacgcgcgtattctgttgagtgcggcgattaccgtgaatgacaaactggtatttatcaccgataccgttcagccggtgatcaaccagggcggaactaaagccgacctgacattggtgccggtacagcaaaccgccgtgccggttcaggccagcggtggcgcaacgactaccgtaccttcgacttcaccaactcaggtgaatccgtcttcggcagttccagctcctacgcaatattaagcgacgttaaccctctccgcccggagagggttagtagttccagcgataacgctgcaagtcgatttgcccgcttcccgataccatcacaccttctgccagtaatgcctgtcgctgacgctgtaaatccggtccggttagcgaaattgtgccgtggcgattaaccacccggtgccagggtaaggtgctgccttcagggagacgctttaacacaccgcccacctggcgcgcggcgcggggcgatcccgccagtttcgccacatcaccgtaagtggtgacatagccttcgggaatagcggcgacgatttgccagacgcgttggggaaatgaatcttctttttccatcttttcttcctgaggtaatttttcagcataatctggaaaaacgcccgagtgaagtcgcattgcgcaagaaaccagcatctggcacgcgatgggttgcaattagccggggcagcagtgataatgcgcctgcgcgttggttctcaacgctctcaatgggggctctgttggttctcccgcaacgctactctgtttaccaggtcaggtccggaaggaagcagccaaggcagatgacgcgtgtgccgggatgtagctggcagggcccccacccatttctgcctcccaccgtttcgtcaaaaaatcccaacatggctaaactttaaccacaactgacgtcgcaagaattgtctggctgcgcagtacgcttcggaggtatgtctgatgaagtatgttgatggttttgtggttgccgttcctgccgataaaaaggatgcctatcgggaaatggccgctaaggctgcgccattgtttaaagagtttggcgcgcttcgtattgtcgaatgctgggccagcgatgtaccggatggcaaagtgaccgattttcgtatggcggtgaaagcggaagagaatgaagaggttgtctttagctggattgaatacccttcaaaagaggtccgcgacgctgctaatcaaaagatgatgtcggacccacggatgaaagagttcggcgagtccatgccgtttgacggcaagcgaatgatctatggcggattcgagtcaatcatcgacgaataggtagcgtgacgggctgtgcggcgtgccgtcagcccaaaaattcacaaatgttgctcggcccagcgtaagaaatcttctttcggtaatgccttgctgtagagccagccctgaccgtagtgcacgccatgctggcgtaaccactcttcttgtttactggtttcgattccctccgctaccattttcagtttcagtgtttttgccatttcgatgatatgcggcgtgacatttttatattccagcgcatcaacgaaagatttatcgatcttcagaatgtcgacatccagatcctgtaaataacttaaacttgaataccccgtaccaaaatcatcaagataaatttcatggcccgcctcccggtagcgagaaattatcggggcgctggttttcggatcggcaaactcgcgttcagtgagttcaagcgcgatctgtctgggattaacctgatagtgattgatcatgtcacgcagcaattgcgggattttttccgaggtgagcacgggggattcaagattgatcgaaatatgctgctgtggatgctgacgcagccagtcgcccatatcttcaaagacgcttcttataatcagtagcgtcaatggctcagaaaggcccgtttgctgtgccagcggaataaaactatctggtgacaaccaactaccgtctgtctgcggccagcgcgccagtgcctcagcaccgacaattttgccattggctaaggagacaatcggctgatagtgcacgcaaatatcacgattttcgatagcatcctgcagccgatgatgcggtgactgaatacggcgcaaaatacgcagcacaaacatcgctgccagcaggccaatcaccaacccgagcggtaaccaaataaagacttgccgatgccagcctttctgcaacattttcgttgaagcccatgtgatgatcgaaatattcatctccggtaagggcaggatatcgtaaatgattccattattttcgatatgctcaccgggtgttttttgtagcctggtaataattccctgagcaatttcatcgctgctggttatgacaacgttatgggcattgccaataatggcggcatcaatttgccatgagctatagggaatgacatcaataaaggaagcggggtcgatcatgacgacataatgtgccgttcccatggcgaccatgtaacggataatgcctaaatcgttatgcgatgttaaccagacacgataaccatctttcgaaattttacctggctcggggaaggtatcgggcggactttcatgctccagagacgaacactggggaacgttgttatcgatataagccacttcctgaatatagcgataactgtaagatacccgacgcatttccatgagatgggcttcgctacaggcagcgccttgccatctttccagctcctgcagcgcatctttcccttgtgtcgccaccttattggctcgaatagcgacgcgggaggaataggtatccagctcttcaataaacgatgtttctacctgctgatgggccagccagatgcttaagccgacaggcagcaatactgaaagaatcagtactcccgaaataaggccgaccagatgtcgtgttctcaccagcatatccttattaacacagtgtagggaaagtatatctgattgtggaaaaaggctggctggagataaggaggtagagctggtatttcatgaagtgatgggtggaaacgatcattgtcatttgaccaggcgcagagctttacgcctggtatgtaaccctaacttaagatgttgattcggcgcgagcgagggtaaaaatatcgtaaaaagacagttcacctttacggacgatcattttttgcagttgttccttatgaacatccgcgacacgcggagagttcaagatggcttcaaccagcgcggcaggtacaaagcgcgtgttgtaccattcgccgttatagcaaacgcggaaatccagcacgtcgatatcttcatagcggtagcgtgggtagacatcgaaaaagaagaaaccattaagcaggataaataatacaaccagtagccagacagagcctgacagcgtttcggactgcaacatcaccgccagggtggcaaaaaaagcaacgtacataccgataaacagccccggatgtttacggataaaactgatactaaagcggggtttgttgtcgcgtttttcgcgggtattcagagactcaatcgtttcggtcagcaggcgttgtatttcggtcatcgtttgccttcgtggtatctgcaactttccagggaacaccctattttaacgtgggaatagtagaggggaagtaacagatctaccacaattttgcataacagttgcgaaaaaccgattacaattttttaattattctggctggattaccgcccacgacaacgttgtccgggacatcttttgtgacaactgcacctgaggctaccacgacgttatcaccaatggtcacaccagggttaatgaccgcgcgtccgccaatccagacgttattaccgatggtgacgggtttccccagttcagcaccgctattacgtgctacagggtcgatgggatgtgttgccgtgtagatatgaacgcctggtgccaacatacagttatcaccgatgcgaatagggcagacatcaagcatcacgcaatcgaagttggcgaaaaaattattaccgagaaaaatgttatagccatagtcacagcgaaacgttggctcaatataagcctctgtcacctgaccgaatagatcagcgagaatttgctggcgtaatgtgtgctcttccgccagggaatgattgtatcggtgaataagctgacgagcgcgcaggcgatcgcgagataacgtctcatctgccgagcgatacaactcaccagcaatcatcttttctttttctgtgctcattactgacctccggttgctgaaaatgcggcaacacagtaagacgaaaagtcagtgaagagaacgttcccattacatctgtgtgataaagatcacatagggtatgtcttcatggcgaaaaagtataaaattcttaataaacagccggttatagctccgaaagcgaattatttattagcgaataaatttccatactgaggaagggatcttgtcgtacagtttattcatggtcaattcggcgaggcggtgatctgcggctgagtaaaataccgccagttcattatctgataattcgtatttatttttctcgataacacgctccagcgtgtcaattgtctggcaacgacgtaaacgcattaaataatcggttttcgttaaaggtttttcggacatacttctacctatggttgtaataattctaacaagataaactcgcaggattctctttcgtcgcattgacaaaacaacggaatagtcgattacctgacttccgccatttctgaagatcctgcatattaataccataactactgaacaacataaaggtgtcatccagatattcgtcgatctgctcaatgagcttattgtcttcattatacttaattttgtaattaagtgcgaaggtcgcaatatgctcaatcagttcattcaactggaggttgatcgccgaggttgggtcgtttacccagccatgattgctttcttcaaggtttgcaaggcagtcatgatacagggtttcacagagaaacttaagctgtgcgatatcatgtcttttgggtgagtattcatccataacgcgtccccttcttagcggttgaactaacggacacctttcgggatggaaaaaacttactgacctggacttgccctctcgtttgttagcttaactataagccactctttgcaggttttcatcgcattattacgaaaaattacaattaggaaggaagcgggacaggactcactttttcatactagcactaacccgcagcaggtaaaagcagtttgctcgaactattcataacatttcaggattatcgccagatgaaattggtgacactaataccaggattgctctgaatatgacgtaataaccgaggaatgaataaagaattaccgcaaataattaagaatagcctctaaatgattatggattattaaatctattagcgctacttaatataaattaactaacaatcagtattttttatgaattttatccgtggttaatactggttttcgtatgagatcctgagttggtggttcaattactccttaatgttcgtaggttatgcataaaaaaggccgcttacgcggccttagtgattacacgttgtatcaatgatgatcgacagtatggctgtgctcgatatcttcattcttgcggctaaagcggcggcgaaccaccacaaagaataccggaacgaagaagattgccagtaccgttgcggtcaccatcccgcccattacaccggtacctactgcgttctgcgcgccggaaccagcaccagtactgataaccagcggcataacgccgaggataaacgccagcgaggtcatcaggatcggacgtaaacgcatccgcaccgcatcaagcgtcgcttcaatcagacctttaccttctttatccatcaagtctttggcgaattcgacgataaggatcgcgttcttcgccgacaacccaatggttgtgagcaggcctacctggaagtaaacgtcattggtcaggccacggaaggtggcagccagcaacgcaccgataacccccagcggaacgaccagcataacggagaacggaatcgaccagctctcgtacagcgccgccagacacaggaacacgacaatcaacgaaatcgcgtacagtgaaggtgcctggttgccggagagacgttcctgataggacatccccgtccagtcatagccaacaccggtaggcagtttgctcgccagttgttccatcagctccattgcttcaccggtacttttacccggtgccgcctggcctaagatttccatggatggcaggccgttgtaacgttccagacgcggcgaaccgtactcccaacgagaagaggagaacgccgagaatggcaccatctgaccatcagcagcacgaacataccagtcgccgatatcatccggcagcatacggtatttcgcttctgacatgacataaactttcttcacacgaccgcggtcgataaagtcgttcacatagctgccgccccatgcagcgcccagagtggtgttaatgtcgttgatagaaacacccagcgcctgcgctttttcctggtcgatatcaatcttaaactgcggggtatcttccagaccgtttggacgtacgctggtcaacatatcagggtgcttcgctgcttctgcaagcaactggttacgcgcctgagtcagtttttcgtgaccaaggccagcctggtcaatcagctcaaagtcaaagccggttgcagtacccagttccacgattgcgggcaggttaaaggcgaaaaccatcgcatctttgatttgcgagaaagcgcgtgttgcacgcatggtaatcgcttcaactttgttttcttcgcccggacgatcggcccagtccttcaaggaaacgaacgcaataccggtattctgaccacgtcccgcaaagccgaagccgttaacggcgaacaccgactcaacgttgttcttttctttggtcagatagtaatgcgttacctcattgagcactttctgtgtacgttcctgcgttgcacctgctggcagctgaaccatggtcataaacacgccctggtcctcatctggcaagaaggagcttggcagacgcacgaacagataggccatgccgaccacgatgatcagatacagcaccaggtaacgccccgtactgcgcagaataccgcctacgctgtcggtgtagtggtgcgtgctcttctcgaacatgcggttaaaccagccgaagaagccttttttaccttccccgtgatcgcctttggcaatcggtttcagcatggtggcacaaagagctggagtcaggatcaacgccaccagtaccgacagcgccattgctgaaacaatggtaatagagaactgacgatagatagcaccagtagaaccgccaaagaaggccatcggtacgaataccgccgacagtaccatcgcgataccgaccagagcgccctgaatctgccccatcgacttacgggtagcttcttttggcggcaaaccttcttccgccataacacgctcaacgttttctaccacaacgatggcgtcatccaccaacaggccgatggcgagcaccatcccgaacattgttagcgtgtttatcgagaagccaaaggcggcaaggacggcaaaggtcccgagcaataccaccggtacggcaatggtcggaatcaacgtcgcgcggaagttctgcaggaacagatacataaccaggaacacgaggatgatcgcttcgaccagcgttttaaccacttcgtgaatagagattttcacgaacggcgtggtgtcgtatgggtaaacaattttcagacccgacgggaagaacggttccatcttcgccagttcagcacggattgccgcagcggtatccagcgcgtttgcaccggtcgccagcttgatccccagaccggaagccggttggccgttaaactctgcgatgatgtcgtagttctcaccacccagctcaatcttcgcgacgtcacgcagcagcacgcgggaaccatcctgattcactttcagcaggattttgccgaactcttcagtagaggtcagacgcgtctgagcaataatagaggcgttaagctgttggcctttcaccggcggcgtaccaccgagctgacccgccgcaacctgggcgttctgcgctttgatggcggtaatgacatcaaccggcgttagctggaatttgttcagctcattcgggttcatccagatacgcatcgcgtactgtgaaccgaacaactgaacatcacccacgcccgacgtacggctgatggcatctttcatattcgccgccacgtagtcggagatatcctcctgcgtcatggtgccatcggtgttgataacgccgacaaccatcaggaagctgctggatgatttctcaacgctcaccccttgctgctgaacttcttgcggcagcaacggcatcgccagctgcagtttgttctgcacctgaacctgcgcgatatccgcatcagtaccagactcaaaggtcagggtgatctgcacggtacccgtggagtcactgttagaggacatgtacatcaggttatcgataccgttcatattctgttcgataacctgtgtcaccgtgtcctgcactgttttcgcatcagcgccggggtaggaggcggagatcgttactgccggcggtgcaatcgtaggatattgcgccaccggcagtttgaggatcgccagcccccctgccaacatgatgataatggcgatcacccacgcaaaaatcgggcgatcgataaagaaattaggcatgtcttaacggctcctgtttaagttaagacttggactgttcaggctgagcaccgcttgcggcttgctggttattatcagcggtaacttcttgtgcttttacctggacaccaggacgcactttctgcagcccacttattactacgcgatcgcctgctttcagaccttctgtcaccagccacttatcgccaatagcctggcttgcaacgatcggacgggtttccactttgtcatccgcgccaactaccagtacggtggcatcgccacgcggcgtacgggttacgccctgttgcgggactaaaatagcgtttggattaagcccttcttccagacgtgcgcgcacgaacatacccggcagcagagtgtgatccgggttcgggaagatagcgcgtagggtgatagacccagtggtctgatcaacggtaacgtcagagaattccagcgtaccgtcctgcgggaacttaatgccgtcactggtgatcagtgacactttggctttgccgttctcttgtttcagcgtgccattcgccagttcctgtttcaggcgcaggaagtcgttgctggactgggtcacatcaacgtagatcggatcaagttgctgcacggttgccagcgcagtcgcctgaccgttctgtaccaatgcgccttccgtcacgttcgacttaccaatgcgaccgctaatcggagaggtgactttggtgtaagccagattgatccgcgcagtttcaacggcagctttcgccgcagttaccgcagcattcgcctgttgcgcatcagccagagcctgatcgtactcttgcttactgatgtactgagtaccgagcagtttctgataacgattcaccgtcaattgcgcgatattggctgcagcctgggctttcgccagatcacctttcgcactgtcgtatgtcgcctgataggtcgcaggatcaatctgatagagagagacacctgcttcgatgtcgctaccttctttgaaattacgcttcaggataatcccgctaacttgaggacgaacttctgcgatccggtaggcactggtgcgacccggaagctcggttgtgatctgcagaggttcagttttgactgttactacgccaacggcgggcatctgctggccaccttgttgggcctgtttgtcgtcacatcctgttagggctaagctgcctgagagcatcagaacgaccgccagaggcgtaaaccctctgtttttgttcatatgtaaacctcgagtgtccgatttcaaattggtcaatggtcaaaagttaataaacccattgctgcgtttatattatcgtcgtgctatggtacatacattcacaaatgtatgtaaatctaacgcctgtaaattcacgaacatatggcacgaaaaaccaaacaagaagcgcaagaaacgcgccaacacatcctcgatgtggctctacgtcttttctcacagcagggggtatcatccacctcgctgggcgagattgcaaaagcagctggcgttacgcgcggtgcaatctactggcattttaaagacaagtcggatttgttcagtgagatctgggaactgtcagaatccaatattggtgaactagagcttgagtatcaggcaaaattccctggcgatccactctcagtattaagagagatattaattcatgttcttgaatccacggtgacagaagaacggcgtcgattattgatggagattatattccacaaatgcgaatttgtcggagaaatggctgttgtgcaacaggcacaacgtaatctctgtctggaaagttatgaccgtatagaacaaacgttaaaacattgtattgaagcgaaaatgttgcctgcggatttaatgacgcgtcgcgcagcaattattatgcgcggctatatttccggcctgatggaaaactggctctttgccccgcaatcttttgatcttaaaaaagaagcccgcgattacgttgccatcttactggagatgtatctcctgtgccccacgcttcgtaatcctgccactaacgaataaccctgaatctgactccaggatttttcctggacattttcgtcgttgctattctggttcactgcgtcgtgatattcttgcggtttgactttttcaggtcgttcttcaggttcagaaaccttcattcatcatgactatgttccagtattacaaacgatcacggcattttgttttttcagcatttattgcttttgtttttgtcttgttatgccagaacacggcgtttgcgcgggcgtcatcgaatggtgatctgccgacaaaagcggacctgcaggcgcaacttgactcactaaataaacaaaaagatctttctgctcaggacaaactggtgcagcaggatctgacagatacattagccaccctcgataaaatcgatcgcataaaagaagagacagttcagctacggcaaaaagtcgctgaagcgccggaaaaaatgcgccaggcgaccgcggcgttaacagcacttagcgatgtcgataacgacgaagaaacgcgcaaaattctgagcacgctgtcgttgcgccagctggaaactcgcgttgcccaggcgctggacgatttgcaaaacgcacaaaacgatctggcgtcttataacagccagctggtttcgttacagacgcagcccgaacgcgtgcaaaatgcgatgtataacgcttcgcagcagctgcaacaaattcgcagtcgtctggatgggactgatgtcggcgagacagccttacgtcccagccagaaagtgttaatgcaggcccagcaggcgttgctgaatgcggagattgaccagcagcgtaaaagcctggaagggaacaccgtcttgcaggataccttgcaaaagcaacgtgattacgtgacggcgaacagcgctcgtctggagcaccagttacaactgttgcaagaagcggtaaacagcaagcgcctgactttaaccgaaaaaacggcgcaggaagccgtctccccggatgaagccgcgcgtattcaggctaatccgctggtgaagcaggaactggaaattaaccagcagttaagtcagcgtctgattaccgcgactgaaaacggtaatcagttgatgcagcaaaacattaaagtcaaaaactggctggagcgggcgctgcaatcggaacgcaatattaaagagcagattgccgtcctgaagggcagcctgctgttgtctcgtatcctttaccagcaacaacaaacgctgccctcggcggatgaactggaaaacatgaccaaccgcatcgcggatttgcgtctcgaacagtttgaagttaaccagcagcgtgatgcactcttccagagcgatgcgttcgtcaacaaactggaagaaggtcacaccaacgaagtcaacagcgaagttcacgatgcgttattgcaagtggttgatatgcgtcgcgaattgctggatcaactcaacaaacagttgggtaaccagctgatgatggccattaacctgcaaatcaaccagcagcagttaatgagtgtgtcgaaaaacctgaaatccatcctgactcagcaaatcttttgggtgaacagtaaccgtccaatggactgggactggatcaaagcgttcccgcaaagcctgaaagatgaatttaagtcgatgaaaatcacggtgaactggcaaaaagcctggcccgccgtttttatcgctttcctcgctggtttgccgctgctgttgattgccgggctgatccactggcgtctgggctggctgaaagcgtatcaacaaaaactggcttccgctgtgggttccctgcgtaacgacagccagctcaacacaccaaaagcgatccttatcgacctgatccgtgcgctgccggtgtgcctgattattctcgcggttggcctgattctgttgaccatgcagctcaacatcagcgaactgctatggtcgttcagcaaaaaactggcgatattctggctggtgtttggcctgtgctggaaggtactggagaaaaacggcgttgccgtacgtcacttcggcatgccggaacagcagaccagccactggcgtcggcaaattgtccgcatcagtctcgcattgctgcctatccatttctggtctgtggtggcagaactttccccgctgcatctgatggatgatgtgctggggcaagcgatgattttcttcaacctgctgctgattgccttcctggtatggccgatgtgccgcgaaagctggcgtgataaagagtcgcacaccatgcgactggtcaccattaccgtgctgtcgataatcccgattgcgctgatggtgctgactgctacaggctacttctacactacgctgcgtctggcaggacgctggattgaaaccgtttatctggtgatcatctggaacctgctgtaccagacggtactgcgtggcttaagcgtagcggcgcggcgtatcgcctggcgtcgtgcgctggcgcgtcggcagaatctggtgaaagagggcgcagaaggtgctgaaccgccggaagaacccaccattgcactggagcaagttaaccagcagacgctgcgtattaccatgttgctgatgtttgcgctgttcggtgtcatgttctgggcaatttggtccgatttgatcaccgtgttcagctatctcgacagcatcacgctctggcattacaacggcactgaagctggcgctgcggtggtgaaaaacgtcaccatgggcagtctgttgtttgcgattatcgcctcaatggtggcctgggcgttgattcgcaacctgcctggtttactggaagtgctggtgctctcgcgactgaatatgcgccagggcgcgtcgtatgccattactaccatccttaactacatcattattgctgttggtgcgatgacggtgttcggatcgctgggcgtctcttgggataaactccagtggctggccgcagcattatccgtaggtcttggttttggtttacaagaaattttcggtaacttcgtctccggtttgatcattctattcgaacgtccggtgcgtattggcgatacggtaaccattggtagcttctcggggacggtaagtaagatccgtattcgtgcgacaacgattaccgatttcgatcgcaaagaagtgatcatcccgaacaaagcgtttgttaccgagcgtctgatcaactggtcgttgactgacactactacgcgtctggtgatccgtctcggcgtggcctatggctccgatctggaaaaagtgcgtaaagtgttactgaaggcggcgactgagcacccaagggtgatgcacgaaccaatgccggaagtcttctttacggcatttggtgccagcacgttggatcatgagctgcgtctgtatgtgcgtgaactgcgtgaccgtagtcgtactgtcgatgagctgaaccgtactatcgatcagctgtgccgtgaaaacgacatcaacattgcctttaaccagcttgaagtgcatctgcacaacgagaagggcgatgaggtgacggaagtaaaacgcgactacaaaggcgatgacccgacgccagcggtagggtaaaaacgaaagggggcaacatttagttgccccgagattgctaacaaagtgcgcgttgttcatgccggatgcggcgtgaccgccttatccggcctacgaaaccgcaagaattcaatatattgcaggagcggtgtaggcctgataagcgtagcgcatcaggcagttttgcgtttgcccgcaaccttaggggacatttagcgaccccatttatttctcacttttccgcctcatcatcgcgcgttaatttcttttcataatcacgctttacaatatccagcgcgcgcagcacggtactggcagggatctgattttcctccagcagcacaatcaaatcgacagccagtttgacatcgtcaggggcattttccagtgacatattctctccattgctagcgggttaaacgcgctaacctgttttcgattttttccagcgcatggcggcagcgtgccaggcgcgcttcataggcttccacttcacgatgcagcgtttgctgttccacgagatcggtcacccgcgccagacgggctctgcgttcggcaaccatctcacgtagccgccgctcaaaatcctgatgctgaatacgtttacgctgccagcgggcaattttcggtggtgcactgtcccactcgcgcaatgaccaggcggaggcttcacgcgcgatggcttccagttgtgccgccagatgttccgccagccaggccacttgcggcagctgttgctgctcaactgcatgacgaagcgcagccagattatcgcccgcctcgtcgagacaagcctgtagtgttgtcgcacgagtctgaaaaagatgcctgtcgaaacgagcacttagcgtggcgaactgtgacaccggggcacaacgctgacgcagcgtagcgagctgtccttccagtttttccagcagcagggcggttttcacgataagacctcaatgaaaatgataattgttatgctaaagtagccactctgtaagctgacaacactcaatatgcaacgaatcattttaatcatcattggctggctggcggtagtgctgggtacgctgggcgtggtattaccggtattaccgacgacgccgtttatcctgctggcggcctggtgctttgcccgttcttccccgcgctttcacgcctggttgctgtaccgctcatggtttggcagctatctacgtttctggcagaaacatcatgcgatgccgcgcggcgtcaaaccgcgggcgattttgcttattttgctcacgtttgccatttctctgtggttcgtccagatgccatgggtgcgcatcatgttgctggtaattctcgcctgtttgcttttctatatgtggcgaattccggtgattgatgaaaagcaagaaaagcactgaagcacaacaatcgcagttgcaattattgcgtacagccagtacattctggcgttttcgagcacaggcgcaggcggtcaaaggttaaacaactgttacttttgatacgtttaaaacgcgccgtgagtaccaccgtaacaagcaggcatacacttatgaccgcgactgcacagcagcttgagtatctcaaaaatagcatcaaaagcattcaggactacccaaaacccggcattcttttccgcgatgtcaccagcttactggaagacccgaaagcttacgctctcagcatcgacttgctggttgagcgttacaaaaatgcgggcattaccaaagttgtcggcaccgaagcgcgtggcttcttgtttggcgctccggtagctctgggtctgggcgttggctttgtaccggtccgtaaaccgggcaaactgccgcgtgaaaccatcagtgaaacttacgacctggaatacggcaccgatcagctggagatccacgttgatgccatcaaaccgggcgacaaagttctggtggtggacgacctgctggcaaccggcggcactatcgaagcgaccgttaaactgatccgtcgtctgggtggtgaagtggctgacgctgcgttcattatcaacctgttcgatctcggcggcgaacagcgtctcgaaaaacagggcattaccagctacagccttgtcccgttcccgggccattaattatcgccagtcttgtgctgcccacgctacggacagcacaagatgtgcattcagcctcgccgttctgacggggctgtgttagcattaccccttcgtgaatccaccttccagcgtttcagagcctgccaatgagttatcaggtcttagcccgaaaatggcgcccacaaacctttgctgacgtcgtcggccaggaacatgtgctgaccgcactggcgaacggcttgtcgttagggcgtattcatcatgcttatcttttttccggcacccgtggcgtcggaaaaacctctatcgcccgactgctggcgaaggggctaaactgcgaaaccggcattaccgcgacgccgtgcggcgtgtgcgataactgtcgtgaaatcgagcaggggcgctttgtcgatctgattgaaatcgacgccgcctcgcgcaccaaagttgaagatacccgcgacctgctggataacgtccagtacgctccggcgcgtggtcgtttcaaagtttatctgatcgacgaagtgcatatgctgtcgcgccacagctttaacgcactgttaaaaacccttgaagagccgccggagcacgttaagtttctgctggcgacgaccgatccacagaaattgccggtgacgattttgtcacgctgtctgcaatttcatctcaaggcgctggatgtcgagcaaattcgccatcagcttgagcacatcctcaacgaagaacatatcgctcacgagccgcgggcgctgcaattgctggcacgcgccgctgaaggcagcctgcgagatgccttaagtctgaccgaccaggcgattgccagcggtgacggccaggtttcaacccaggcggtcagtgcgatgctgggtacgcttgacgacgatcaggcgctgtcgctggttgaagcgatggtcgaggccaacggcgagcgcgtaatggcgctgattaatgaagccgctgcccgtggtatcgagtgggaagcgttgctggtggaaatgctcggcctgttgcatcgtattgcgatggtacaactttcgcctgctgcacttggcaacgacatggccgccatcgagctgcggatgcgtgaactggcgcgcaccataccgccgacggatattcagctttactatcagacgctgttgattggtcgcaaagaattaccgtatgcgccggaccgtcgcatgggcgttgagatgacgctgctgcgcgcgctggcattccatccgcgtatgccgctgcctgagccagaagtgccacgacagtcctttgcacccgtcgcgccaacggcagtaatgacgccaacccaggtgccgccgcaaccgcaatcagcgccgcagcaggcaccgactgtaccgctcccggaaaccaccagccaggtgctggcggcgcgccagcagttgcagcgcgtgcagggagcaaccaaagcaaaaaagagtgaaccggcagccgctacccgcgcgcggccggtgaataacgctgcgctggaaagactggcttcggtcaccgatcgcgttcaggcgcgtccggtgccatcggcgctggaaaaagcgccagccaaaaaagaagcgtatcgctggaaggcgaccactccggtgatgcagcaaaaagaagtggtcgccacgccgaaggcgctgaaaaaagcgctggaacatgaaaaaacgccggaactggcggcgaagctagcggcagaagccattgagcgcgacccgtgggcggcacaggtgagccaactttcgctaccaaaactggtcgaacaggtggcgttaaatgcctggaaagaggagagcgacaacgcagtatgtctgcatttgcgctcctctcagcggcatttgaacaaccgcggtgcacagcaaaaactggctgaagcgttgagcatgttaaaaggttcaacggttgaactgactatcgttgaagatgataatcccgcggtgcgtacgccgctggagtggcgtcaggcgatatacgaagaaaaacttgcgcaggcgcgcgagtccattattgcggataataatattcagaccctgcgtcggttcttcgatgcggagctggatgaagaaagtatccgccccatttgatcgtaagcacagcttacgttcgtcatccttaacgtgattgagagagaaacctatgtttggtaaaggcggtctgggtaacctgatgaagcaagcccagcagatgcaagaaaaaatgcagaaaatgcaggaagagatcgcgcagctggaagtcaccggcgaatctggcgcaggtctggtaaaagtgaccatcaacggtgcacacaactgccgtcgcgtagagatcgacccgagcctgctggaagacgacaaagagatgctggaagacctggtggctgcagcattcaacgacgcagcacgtcgtattgaagaaacgcagaaagaaaaaatggcctctgtatcctccggaatgcagctgccgcctggctttaagatgccgttctgatgcaaaccagcccgctgttaacacagcttatggaagcactgcgctgtctgccgggcgttggcccgaagtcggcgcagcgtatggcgttcacgctgcttcagcgcgatcgtagcggcgggatgcgtctggcgcaggcgctcacccgggcgatgtcggaaatcggccactgcgccgattgccgcactttcaccgaacaggaagtctgtaacatctgttcgaatccgcgtcgtcaggaaaacggtcaaatctgcgtggtggagagtccggcggacatctacgccattgagcagacggggcagttttcaggtcgttattttgtgttgatggggcatctgtcaccgctggacggcatcggtccggatgatatcgggcttgatcgtctggaacagcgtctggcagaggaaaaaatcactgaagtgatcctcgccaccaaccccacggttgaaggtgaagctaccgctaactacattgccgagctttgcgcgcaatatgacgtggaagccagccgaatcgctcatggcgttccggttggcggcgagctggaaatggtcgacggcaccacgttgtcacactcccttgccgggcgtcataagattcgtttttaagcaaacgagagcaggatcacctgctctcgcttgaaattattctcccttgtccccatctctcccacatcctgtttttaaccttaaaatggcattattgaggtagacctacatgaaaggacaagaaactcgtggttttcagtcagaagtgaaacagcttctgcacctgatgatccattctctctattccaataaagaaatcttcctgcgtgagcttatctctaacgcctccgatgcggcggacaagctgcgtttccgtgcgctctctaacccggacctgtacgaaggtgatggcgaactacgcgttcgtgtctctttcgataaagacaagcgtacgctgaccatctccgataacggcgtggggatgacccgcgacgaagtgattgaccatctggggactatcgctaaatccggtaccaaatcattcctcgaatccctgggttctgaccaggcgaaagacagccagctgatcggtcagtttggtgttggtttctactctgcgtttatcgtggccgacaaagtgaccgtgcgtactcgcgcggcaggcgaaaaaccagaaaatggcgtcttctgggaatcggctggcgaaggtgaatacaccgttgccgacatcaccaaagaagatcgtggtactgaaatcaccctgcatctgcgtgaaggcgaagacgagttcctcgatgactggcgcgtgcgttccatcatcagcaaatactccgaccatatcgcgctgccggtagagatcgaaaaacgcgaagagaaagacggcgaaaccgttatctcctgggagaaaatcaacaaagcgcaggcgctgtggactcgtaacaagtcggaaatcaccgatgaagagtacaaagagttctacaaacacatcgcccacgactttaatgatccgctgacctggagccacaaccgtgttgaaggtaagcaggagtacaccagcctgctgtacatcccgtcccaggctccgtgggatatgtggaaccgcgatcataaacacggcctgaaactgtatgttcagcgtgtgttcatcatggacgacgcagaacagttcatgccgaactatctgcgcttcgtgcgtggtctgattgactccagcgatctgccgctgaacgtttcccgtgaaatcctccaggacagcacggtaacgcgtaacctgcgcaatgcgctgaccaagcgtgtgctgcaaatgctggaaaaactggcgaaagacgacgcggaaaaataccagaccttctggcaacagtttggcctggtactgaaagaaggtccggcggaagatttcgctaaccaggaagcgatcgccaaactgctgcgttttgcttctacccataccgattcttctgcgcagaccgtatctctggaagactacgtttcccgcatgaaagaagggcaggagaaaatctactacatcaccgcagacagctatgcggcagcgaagagcagcccgcacctggaactgctgcgtaagaaaggcatcgaagttctgctgctttccgaccgcatcgatgagtggatgatgaactatctgactgagttcgacggtaaaccgttccagtcggtgtctaaagttgacgagtcgcttgaaaaactggctgacgaagttgatgagagcgcgaaagaagcggagaaagcactgactccgttcatcgaccgtgtgaaagccctgctcggcgagcgcgtgaaagatgtccgtctgactcaccgtctgaccgatacgccagcgatcgtttcgaccgacgcggacgaaatgagcactcagatggcgaaactgttcgctgcggcgggccagaaagtgccagaagtgaaatacatcttcgaactgaacccggatcacgtactggtgaaacgtgcggcagatactgaagatgaagcgaagttcagcgagtgggtagaactgctgctggatcaggcgctgctggcagaacgcggcacgctggaagatccgaacctgtttattcgtcgtatgaaccagctgctggtttcctgatgtaatgccggatgaccttcgtgtcatccggcatttttcttttcatcatctgcactttccgcaaattatctcgccattaaccgtttcagccccaggtgcctttcttgaggcaatcgcctgttggtggtatcgtttatcgctttttcaaaaaattcgacacattttaaggggattttcgcaatgcgtatcattctgcttggcgctccgggcgcggggaaagggactcaggctcagttcatcatggagaaatatggtattccgcaaatctccactggcgatatgctgcgtgctgcggtcaaatctggctccgagctgggtaaacaagcaaaagacattatggatgctggcaaactggtcaccgacgaactggtgatcgcgctggttaaagagcgcattgctcaggaagactgccgtaatggtttcctgttggacggcttcccgcgtaccattccgcaggcagacgcgatgaaagaagcgggcatcaatgttgattacgttctggaattcgacgtaccggacgaactgatcgttgaccgtatcgtcggtcgccgcgttcatgcgccgtctggtcgtgtttatcacgttaaattcaatccgccgaaagtagaaggcaaagacgacgttaccggtgaagaactgactacccgtaaagatgatcaggaagagaccgtacgtaaacgtctggttgaataccatcagatgacagcaccgctgatcggctactactccaaagaagcagaagcgggtaataccaaatacgcgaaagttgacggcaccaagccggttgctgaagttcgcgctgatctggaaaaaatcctcggctaattcgaaagcgcgcacggacagtcccctcgccccctcggggagagggttagggtgaggggaacaggcccgcacaagcaaacttatcagcaatctcaggccggatattcattcggccttttacaaaaacctcaatctgcgctattcctttttctgatttgacctctcacagcaattagttcttcttcctcacttttccgctacaattatcaacaagttgaatcgataagaggcggtaatgcgtcagactaaaaccggtatcctgctggcaaacctgggtacgcccgatgcccccacacctgaagcggtaaaacgctatctgaaacaatttttaagcgacagacgcgtggttgatacctcacggttgttatggtggccattgctgcgcggcgtgattttgccgctgcgctcgccgcgtgtggcgaagctgtatgcctctgtctggatggaaggtggctcgccgctgatggtttacagccgccagcaacagcaggcgctggcacaacgtttaccggagatgcccgtagcgctgggaatgagctacggctcgccatcactggaaagcgccgtagatgaactcctggcagagcatgtagatcatattgtggtgctgccgctttatccgcaattctcctgttctacggtcggtgcggtatgggatgaactggcacgcattctggcgcgcaaacgtagcattccggggatatcgtttatacgtgattacgccgataaccacgattacattaatgcactggcgaacagcgtacgcgcttcttttgccaaacatggcgaaccggatctgctactgctctcttatcatggcattccccagcgttatgcagatgaaggcgatgattacccgcaacgttgccgcacaacgactcgtgaactggcttccgcattggggatggcaccggaaaaagtgatgatgacctttcagtcgcgctttggtcgggaaccctggctgatgccttataccgacgaaacgctgaaaatgctcggagaaaaaggcgtaggtcatattcaggtgatgtgcccgggctttgctgcggattgtctggagacgctggaagagattgccgagcaaaaccgtgaggtcttcctcggtgccggcgggaaaaaatatgaatatattccggcgcttaatgccacgccggaacatatcgaaatgatggctaatcttgttgccgcgtatcgctaaagctgagcggtaaagaactgagcgccgtcgcgaagagcctcgtcggcggttttcatcatccgtgaataatgcaaaaaggcgtgcagcgtgcctgggtagagtttgaactcacagggctgctgatgcgccgctaacgtctggtaaagcagacggctgtcatccagcagcggatcgaactccgccccggcaataaaacagggcggaacttcgcgagtgagatcattattaaacagacagtaatacggcgactcgcggtccgcgtcgttgcttaaatatgcctcttcgtacatctgcaaatcctgttgcgttaagccatcccagacaccgcccaacagacgacgagtcacggaatcccgtaatccgtaaagcccataccacagcaaaacgcccgcaactttaccgcaatcgatctgtttatcacgcaaccacaacgcactggcgagcgccagcatggcacctgcggaatcaccggcaaagccaatgcgggacatattgatttgataatcctccgcctgctggtggaaataacaacaagcagccacaatttcctctatcgcttgcggaaaacgcgcttcaggtgaaagggtgtaatcaataccaatcaccgtacattggctgtagcttgccagcaggcgcatgatgcgatcgtgggtatcgagattgccgagaataaaaccgcctccatgcaaataaaatagcgtcgctgggctatctggctgcggacaaaagagacgtgtttccacctgcccatattttgttggaaccatgtaagctctggttgccatttctggagcgcccgcattccagaatcggcgctcaagcgtgtaatactgtcgttgctcagcaatcgttcccgttgcgggccagggcggtaaatccggctgaagagtattcacaacggtcttcatttcagcagaaataaggtccagaacaggtagtttgttttccggcttcatacaaaaactcctttcaaattacgtcattgtaaggaaccactgccatgaaaatgcgatcccgcctgctgatattgaaactggctgcgtctcgcgcgctcccgtcagattgtgttaacattcgccgctcagttaaccacccgtaaaaacaaccatgaaatttcccggtaaacgtaaatccaaacattacttccccgtaaacgcacgcgatccgctgcttcagcaattccagccagaaaacgaaaccagcgctgcctgggtagtgggtatcgatcaaacgctggtcgatattgaagcgaaagtggatgatgaatttattgagcgttatggattaagcgccgggcattcactggtgattgaggatgatgtagccgaagcgctttatcaggaactaaaacagaaaaacctgattacccatcagtttgcgggtggcaccattggtaacaccatgcacaactactcggtgctcgcggacgaccgttcggtgctgctgggcgtcatgtgcagcaatattgaaattggcagttatgcctatcgttacctgtgtaacacttccagccgtaccgatcttaactatctacaaggcgtggatggcccgattggtcgttgctttacgctgattggcgagtccggggaacgtacctttgctatcagtccaggccacatgaaccagctgcgggctgaaagcattccggaagatgtgattgccggagcctcggcactggttctcacctcatatctggtgcgttgcaagccgggtgaacccatgccggaagcaaccatgaaagccattgagtacgcgaagaaatataacgtaccggtggtgctgacgctgggcaccaagtttgtcattgccgagaatccgcagtggtggcagcaattcctcaaagatcacgtctctatccttgcgatgaacgaagatgaagccgaagcgttgaccggagaaagcgatccgttgttggcatctgacaaggcgctggactgggtagatctggtgctgtgcaccgccgggccaatcggcttgtatatggcgggctttaccgaagacgaagcgaaacgtaaaacccagcatccgctgctgccgggcgctatagcggaattcaaccagtatgagtttagccgcgccatgcgccacaaggattgccagaatccgctgcgtgtatattcgcacattgcgccgtacatgggcgggccggaaaaaatcatgaacactaatggagcgggggatggcgcattggcagcgttgctgcatgacattaccgccaacagctaccatcgtagcaacgtaccaaactccagcaaacataaattcacctggttaacttattcatcgttagcgcaggtgtgtaaatatgctaaccgtgtgagctatcaggtactgaaccagcattcacctcgtttaacgcgcggcttgccggagcgtgaagacagcctggaagagtcttactgggatcgttaagttatcgtcggttcgtaggccagataaggcgttcacgccgcatctggcatttggctctcgatgcctgatgcgacgctggcgcgtcttatcatgcctacatatttttcatattttacatccggcaaccaccgtttaccccgtcaccacctcacccgccggtggcgtttccagcagttccagcatggtacgggcgatttcacgctcgcccatcactacctgattcgcaccacgttcggtgatatacgccacttcatcgtcataatgggcgcgggcaataatctcaatatccggatttttcgcgcgggcagatgccacaatctcacccgcttcataaccgttgggaatcgtcaggatcagccattttgcacattccagatgcgccagttgcataatttcttcgttcgccgcattgcccaatactgcgcggaccccgcgctctcgcagctcatcaacacgggttcgtgacgtctcaatcaccaccagcggaatatcagaggcgagcaatttctcccccagcaggctgcctacacgaccgtaacccaccagtagcgcatggttgcaaatatccactgggatctgcttctcttcttcgattgcctcttccagcgtctgctcttccagcgtttcggtcttcgccagatatttctccagtagtgcgaacagtaccgggttgagcataatcgacaggatcgcccctgccagtaccaggttttgtccggcctgcggcagtaaattcaatgccattcccagtcccgccaggataaacgcgaactcaccaatctgcgccaggctggcggcgatggttaatgccgtacgttgggagtgaccaaacagtcgcaccaggaaaaatgcggctaacgacttaccaaacagaataatcgccagcgtcgccagcactgccagcggttgctgaatcagaattaacggatcaaacaacatcccgacggagacaaaaaacagcaccgcaaacgcgtcgcgcaatggcagcgtatcgtgggcggcacggtgactcagttcagactcgttcagtaccatcccggcaaagaacgcaccgagtgcaaaggagacatcaaacagctctaccgcaccaaaggcaacccctaacgccagcgccagcaccgacagggtaaacagctcgcgagaaccggttgccgcgctgcgtgccataatccacggcaccagacggcgacctaccagcatcataatggcgataaatgcgatcactttgccgatggtgatccccatatcgactgcaagagtggcaaagcccacatcgccctgttccatcattcctgccactgcgggcagcaacaccagcgtcagaaccattaccaggtcttccacaatcaaccaaccgatggcgatttgcccacgctgactgtcaattaattgccgttcttcaagtgcgcgcagtaacaccacggtactggcggtggaaagacataaaccgaacacgataccggtcattaacgaccagcccagcacggcagagagcgccatacccagcagcgtcgccacggctatctgggcgatcgcaccgggaatggcgatggcctttaccgccatcaaatccttcagcgaaaagtgcaaaccgacgccaaacatcaacagaatgacgcccagttcagccagttccggggcaagcttggtatcggcaacaaagcccggagtgaatggtcctgccagcacacccgctaacagatatcccaccagaggagaaatacgtagtttattggccagcatgccgaggataaaggcgagcacaaggccgccaacaatggtggtgataagcggggtggcgtgatgcattccgtctccttttcctggtggttattgtccatttttggccgggaaaaccaaaattacaggtaatagtttatgacaatttcattgatgatgttcatgaataattattgaattttgcagaaaaatggaattagctgcaaaaaaagcacggatcggaaaacagaaggcggtttaacagaggaaaggcttatggcgactgtaaaacgatgcagccaaagtttgcctttggctgcaatgaaatcagtctttatgccggttatcaggcaggaatatggtcaacatccccaatagtggcaggaaagcacagattttatagactaactcgatgctggtgtgatcggcgataagccccagaactgccgctcccagacctcccatgccaaaagcaaaaccgaaaaagagtccagaaaccataccgatacgtcctggaagcagctcctgagcgtagaccagaatggcagagaatgccgaagcgaggataaatccaataatcaccgttaaaacccccgtccagtgcaggctggcgtagggtaaaatcagcgtaaacggcgcaacgccgaggatagagccccaaatcacatatttccgcccaattttatcccctacaggcccgccgatcaccgtacctgccgcaacggcaaacaggaaggcaaacagatgaagctgagcattctggatagataatccgaatttttgcatcagataaaaggtgtaatagctgctgatgctcgccatatagaaatatttcgagaaaatgaggattaacagaatgctgaccgccagtacaactttattgcgcggcagtggattgataatcgtcgctttgggttttcctttattcattcggtgctgtgccgagtaccaacggctgatttgcgccaacaccacgatcgccagcagtgccgcaagcacaaaccaggcaacgttgcctttgccataaggcgcgataatcaccgccgccagcaagggtcccagggaactgccaaagttgccgccgacctgaaagatagattgcgccaggccatgccgcccgccggaagccatacgggccacgcgagaagattccggatgaaagaccgatgaaccggtaccgaccagcgccgccgccagcagaactgcgccaaaactgcccgccagcgcaagcagcaccagaccgcttaaggtaaagcacatgccaattggcaacgaccatggcatcggatatttatcggtccagtagccgaccactggttgcagtagcgaagaggcgagctggaaggtgagggttatcatgccaatctgcataaatgtcagagaaaattctgactgaagcagcggataaatcgccagaatcagcgattggatcatgtcgttcagcagatgtgagaggctgatagcacctaaaataccaaacgatgttcgggccttggtcgttgacgcagccgcgcccgccacaggctggggttgttcactcattgccataggaaagtcactttttcagggttgcgatgtaaagaatgatcttatttgtgattattaccagactaacatacctgtatgcgtcgtctgaaggaagtctcaacgccgaatacagaatttctaatctggatgcagatttatcttcaccggacgcagacttgtctatgatgtcgcgtcatactatttttcaacacgttgaaatcaggtcagggagagaagtatgaaattattgcagcggggcgtggcgttagcgctgttaaccacatttacactggcgagtgaaactgctctggcgtatgagcaggataaaacctacaaaattacagttctgcataccaatgatcatcatgggcatttttggcgcaatgaatatggcgaatatggtctggcggcgcaaaaaacgctggtggatggtatccgcaaagaggttgcggctgaaggcggtagcgtgctgctactttccggtggcgacattaacactggcgtgcccgagtctgacttacaggatgccgaacctgattttcgcggtatgaatctggtgggctatgacgcgatggcgatcggtaatcatgaatttgataatccgctcaccgtattacgccagcaggaaaagtgggccaagttcccgttgctttccgcgaatatctaccagaaaagtactggcgagcgcctgtttaaaccgtgggcgctgtttaagcgtcaggatctgaaaattgccgttattgggctgacaaccgatgacacagcaaaaattggtaacccggaatacttcactgatatcgaatttcgtaagcccgccgatgaagcgaagctggtgattcaggagctgcaacagacagaaaagccagacattattatcgcggcgacccatatggggcattacgataatggtgagcacggctctaacgcaccgggcgatgtggagatggcacgcgcgctgcctgccggatcgctggcgatgatcgtcggtggtcactcgcaagatccggtctgcatggcggcagaaaacaaaaaacaggtcgattacgtgccgggtacgccatgcaaaccagatcaacaaaacggcatctggattgtgcaggcgcatgagtggggcaaatacgtgggacgggctgattttgagtttcgtaatggcgaaatgaaaatggttaactaccagctgattccggtgaacctgaagaagaaagtgacctgggaagacgggaaaagcgagcgcgtgctttacactcctgaaatcgctgaaaaccagcaaatgatctcgctgttatcaccgttccagaacaaaggcaaagcgcagctggaagtgaaaataggcgaaaccaatggtcgtctggaaggcgatcgtgacaaagtgcgttttgtacagaccaatatggggcggttgattctggcagcccaaatggatcgcactggtgccgactttgcggtgatgagcggaggcggaattcgtgattctatcgaagcaggcgatatcagctataaaaacgtgctgaaagtgcagccattcggcaatgtggtggtgtatgccgacatgaccggtaaagaggtgattgattacctgaccgccgtcgcgcagatgaagccagattcaggtgcctacccgcaatttgccaacgttagctttgtggcgaaagacggcaaactgaacgaccttaaaatcaaaggcgaaccggtcgatccggcgaaaacttaccgtatggcgacattaaacttcaatgccaccggcggtgatggatatccgcgccttgataacaaaccgggctatgtgaataccggctttattgatgccgaagtgctgaaagcgtatatccagaaaagctcgccgctggatgtgagtgtttatgaaccgaaaggtgaggtgagctggcagtaatccgaaagtgccggatgtttgcatccggcacaatgcttaatcgcggcgggcgatatcagcaaatttggcatcgaggatctttgccagatcgcctgccgccagttcgatatccagtccgcgcttgccgccggaaacataaatagtggcaaattcttgtgcgggggcgtcgataatcgttggcagacgttttttctgccccagtgggctaatccccccaaccaggtatcccgtcgaacgctgcgcgaccatcggatcggccatctcaactttcttggcacccagcgcttttgctacttttttaagatccagttgacctgcgaccggcgtaacggccacggcaaggtgtttcatatcaccgttcactgccaccagcagcgttttgtagacctgatccggattcaaacctaattttttgacgacttcatcgccaaaattggtttcagccggatcgtgctcgtaggtatggatttgaaacgaaatcttgtttttttcgagtaatttaactgcgggtgtcatggtaattttcctgccttaaacaaaaaaacgaagcaagcatacgcctgatggcggtccaaaaaaaagagtcatcttgcctaagagtattggcaggatggtgagattgagcgacaatcgagttacaccgtcgcttaaagtgacggcataataataaaaaaatgaaattcctctttgacgggccaatagcgatattggccatttttttagcgcaacatttgcggcaaattcccttctccatacaggtgtagtgcaccgaccgcgaccacatatcgccccggcggcatggcgcgtaatttatcccgccaggcgagatttcgctgatgcatcagcacatcgtacagcgactgactgaacgtattgggcagcgttatatcattattttgcggcggtgcattcagccaccagctcatcatttgttgcagcaaccgtgcgttggtatgccagtgggtcagcgtatcgtccagcagcgccagtcctttgtcagggagctggagcaacatggcaatctggttttcagccccttccagttcaatcacgggtttatgttgttgcttcgccgcctgcaatagctggtaatcgataccgtattctgcccgcagccccagtttttgtgcctgcgtcgcctgaagaaccatcgcgatttgccacagcggttgggtagaaaagagtgagggagaaatgcccatctcctggctaatgtgctgcaggttttggagttgctcctcgctaatgcgctcttccagcgcctcgcaggcaggcaaattagcaaaaggcgtatcgctggtggaaacatccgcctcgacgatcagcgcatcggcgtttttgagctttttgagcaaacgggtgggcaggggagccatatcgtggctacccatatgaatactgccaatcagatgaaaatggcgattgccggggagggtgatatcgatggcaggccaggtgtaatgattaccgcgcagcgcggcccaaagcgtttttacccggtacaacagatccatacgacctccctttgtgaaatatcatgctagcgcgcggtgagggatggcgcaaatggagttggagacttgtttaatgtgtttgtatgattcagtatgttcttgcatcgctattcacaaggaagcaacagttaaaaaccatgaaacaggcaacaagaaaaccgacgacacccggagatattcttctctatgaatatctggaaccgctcgatttgaaaatcaatgagttagcagagttgctgcatgttcatcgtaatagcgtcagtgcactgatcaataacaatcgtaaactcactactgagatggcatttcgtctggcgaaagtttttgataccacagtcgatttttggctaaacctccaggcggcggttgatctttgggaagttgaaaacaacatgcgcacccaggaagaattgggacggattgaaacagtggctgaatatttggcacgccgtgaagagcgtgcaaaaaaggtcgcgtaaggccaaaacatcgcttcatctcgtaggccggataaggcgttcacgccgcatccggcatccgagcaccattgcctgatgcgacgcttacccgtcttatcaggcctacaaacttgtgcctgaaccgtaggccggataaggcgtttacgccgcatccggcatccgagcaccattgcctgatgcgacgcttacgcgtcttatcaggcctacaaacctgtgcctgaaccgtaggccggataaggcgtttacgccgcatccggcagtcatgcgtcgatgccaaatgcgccaccctaaagcagcgcatccgcaatgatgtacttattccttcggtttaaaccgcagcaaccggttggcgttactcactacggtaatcgacgagagcgccattgccgctccggcaactaccgggttaagcagtgttccagtgaacggccacaaaataccggcggcgaccggaataccgatactgttgtagataaacgcaccgagcaggttctgcttcatgttgtgcagcgttgcgcgggaaatagcgagcgcatccgcaacgcccatcaggctatggcgcatcagggtaatcgccgcggtttcaatggcaacatcactgccgccacccatcgcaatgccgacatccgcctgagccagcgctggcgcgtcgttaatgccgtcgcccaccattgccacctgacgtccttcactttgcagatgtttgatcgcttcggctttaccgtccggcagcaccccggcgatcacctcatcaatccctgcttctttggcgatcgcattggcggtggttgggttatccccggtcaacatcaccagacgatatcccgctttatgcaggcgttgcagcgccgccacgctatcactacgcaacggatcgcgtactgccagcagggctaccgctttcccgtcaaccgccagcagcacaggcgttgccccttgcgatgcctgagcagtaatctccgcttcgatagctttggtaccaacctgttgctcatttaacagcgcctgattgcccagcaataacgcatgaccttcagcttcaccgctcacgcccagcccgcgcaatgtgcggaaaccgttgacctgcggtagctgcatatcacctgctttatcgaggatcgctcgtgccagcggatggctggaaccttgctccagtgccgccgccagacgcaatgcctgcgcttcatcaacatcagcaaatgttttcactgcgacaacctgcggcttcccttcagtcagcgtcccggttttatcgaacactacagtgtcgagtgtactggcgcgttgcagcgcgtcagcgtcccgcaccagcacgccaaactcagccgcccgcccgacgccggaaataatcgacatcggcgtcgccagccccagcgcacacggacaggcaataatcagtaccgtggtggcaatcaccagggtatagacaatctgcggtgccggaccaaagaaataccagattgccgcactgacaagcgcaataaccaccactaccggcacaaatacggctgagattttatccgccagctgaccgatttctggcttgctgctctgggcctggcgcaccatgcgaatgattcgtgacagcgtagtatggctgccaaccgcactggcacgaaacagcacactgccgtcctgtaccactgtcccggcatggacgctatcgccttcgcctttttgctgcgggattggttcgcccgtcagcatcgcttcatccagccatgcttcgccctgggtaatctcgccatctaccggcacgcgatcgccggtcgtcaggcgcagcaacatacctggctgcacttctgccagaggcacgcttttttcaccttcgtcagtaaccaggcgtgccgtcggcggggttaaatcgagtaacttttccagcgccttagaagaacgctggcgtgcgcgcgcttccagcatatggccgagattgatcagaccgataatcatcgcgctggcttcgtaataaagatgtcgcgcttccatcgggaaccactgcggccacaggttgacgctcatcgaatagagccacgccacgccagtacccagcgccaccagcgtatccatcgtcgccgcaccgttcagcaggcttttccatgcactgcggtaaaaatggccgccggcgaaaaccatcactgccagggttatcaggccgataaccaaccacaggctgcggttgtcagcggtgaccatcatgttatcgccgatcatcccccagaccatcaccgggatacccaccgccagtgcgacaattgcctgccagcggaagcgcttcatcgtagcgacggcggtttcttgctggcgctcgcggcgtttagcgtcatcttcaatcgcttccgcgccgtagcccgctttttccaccgcctgcactaaatcttgtggggaggcactgcccatcaccagcgcagtacgctccgccaggtttacccgtgcctgagtgacgcccggtacgctttgcagcgcattttgtacgcgggtgacacagctggcgcagctcatgccgctcagcagcaactgctggctgtcatcgtcatcggcggtcgctgccggaagcgcctcagaaaccgctgtcagtgcttccgacgggattgatgactccgccagcggtttagcctttgggtggcttacagatgcgtcataacccgcttgtttgatggtttcgatcagctgttctgcactggcagtcccggtaacgtgcgcttcagtgatagacacatccgcctgctcaacatccggacgctgttcaagactttctttcacgcgtttaacgcagtgaccgcaggacaggccgtccagggtcaggtcgatagtttgtgacataaaacactcctttaagacagttttgactggctgtgataaaggttaaaccttccagcaaggggaaggtcaagaaattaataaaccaggcgggtaaaagtccgtaaagattaaaaaatcggctcgatttgcatcaggattagacatttatctctttgttttcctgtagttaagttgcgggtgctaagttaaatcaggatgcctgaaaatcggcaccggggtgaggaattacctcccgcatctataaaaaggagttaacaaaagatgttagatgcaaacaaattacagcaggcagtggatcaggcttacacccaatttcactcacttaacggcggacaaaatgccgattacattccctttctggcgaatgtaccaggtcaactggcggcagtggctatcgtgacctgcgatggcaacgtctatagtgcgggtgacagtgattaccgctttgcactggaatccatctcgaaagtctgtacgttagcccttgcgttagaagatgtcggcccgcaggcggtacaggacaaaattggcgctgacccgaccggattgccctttaactcagttatcgccttagagttgcatggcggcaaaccgctttcgccactggtaaatgctggcgctattgccaccaccagcctgattaacgctgaaaatgttgaacaacgctggcagcgaattttacatatccaacagcaactggctggcgagcaggtagcgctctctgacgaagtcaaccagtcggaacaaacaaccaacttccataaccgggccatagcctggctgctgtactccgccggatatctctattgtgatgcaatggaagcctgtgacgtgtatacccgtcagtgctccacgctcctcaatactattgaactggcaacgcttggcgcgacgctggcggcaggtggtgtgaatccgttgacgcataaacgcgttcttcaggccgacaacgtgccgtacattctggccgaaatgatgatggaagggctgtatggtcgctccggtgactgggcgtatcgtgttggtttaccgggcaaaagcggtgtaggtggcggtattctggcggtcgtccctggagtgatgggaattgccgcgttctcaccaccgctggacgaagatggcaacagtgttcgcggtcaaaaaatggtggcatcggtcgctaagcaactcggctataacgtgtttaagggctgatcatgatgaacacggaaggtaataacggtaacaaacctctcggtctatggaacgtcgtttccatcggcattggggcaatggtgggggcggggatcttcgcgctgctggggcaggctgcattgctaatggaagcctcgacctgggtcgcctttgcttttggcggtattgtggcgatgttttccggttatgcctatgcgcgtctgggggcgagctatcccagcaatggcggcattatcgacttctttcgtcgcggattaggcaacggcgtcttttcgctggcgctctcgttactgtacctgttgacgctggcggtgagcatcgccatggtcgcccgtgcttttggcgcttatgccgtgcagtttttgcatgaaggcagccaggaggagcaccttattttgctctacgcgttggggatcattgcggtgatgacgcttttcaactccttaagcaaccatgcggtagggcggctggaagtgatcctcgtcggcattaaaatgatgatcctgttattgctgattattgccggtgtctggtcgctgcaaccggcgcatatttccgtctctgcgccccccagctccggtgcgttcttctcctgtattgggataactttccttgcctatgcgggctttggcatgatggcgaacgcggcggataaagtgaaagatccgcaggtcattatgccacgggcgtttctggtggcgattggcgttaccacgttgctttatatctcgctggcactggttttgcttagcgatgtatcggcattagagttagaaaaatatgccgataccgccgtagcgcaggctgcttctccgctgctcgggcatgtgggttatgtgatcgtcgtcatcggcgctttactggcgacggcttcagccattaacgcgaacctgttcgccgtgtttaacatcatggacaacatgggcagcgaacgcgaactgccgaagctaatgaataaatccctgtggcggcagagtacctggggcaacattattgtcgtggtgttgattatgctgatgacggcggcactgaatttaggctcactcgccagcgttgccagcgccacctttttgatttgctacctggcggtgtttgtggtggcgatccgcctgcgtcatgatattcacgcctcgttgccgattcttatcgttggtacgttggtgatgttgttggtgatcgttggctttatctacagtctgtggtcccagggtagccgtgcgttgatatggattattggctcactcttactcagccttattgtggcaatggtcatgaagcgcaataaaaccgtataacatctctctgtgcgcagtacttcctgtattattgtggtggcggtcgatattcgcactggcaaaaaaacgtgcttgaatatctgttgaaaccctttaacaaagcacaggaggcgttgcgcgaacgatgaacatcagcgatgtagcaaaaattaccggcctgaccagcaaagccattcgcttctatgaagagaaggggctggtgacgccgccgatgcgcagcgaaaacggttatcgcacctacacgcagcagcatctcaacgaactgaccttactgcgccaggcacggcaggtgggctttaacctggaagagagcggcgagctggtgaatctgtttaacgacccgcagcggcacagcgccgacgtcaaacggcgcacgctggagaaggtggcggagatcgaacgacacattgaggagctgcaatccatgcgcgaccagctgctggcactggcgaatgcctgccctggcgatgacagcgccgactgcccgattatcgaaaatctctccggctgctgtcatcatcgggcagggtgattaagacgagacggctcggatatgtagggttatcccttctatcgcaatgacttcaacatgcgtacctgcaccgagatcctcgctggcgctgacaggccatgaactgtcaccgacgcgcatatgaccgcgcccgttgaccagcggagattccagcacaaaacgtcggccaatcagctgctgcccgcgctggtttaaatgactatcgctgtgcttttgttcgcgcacccgccgcgacaaccatttccaccacagccaggcggcgagcagcgtcaggatggcaaacattaccccttgccactcccaacccagcggcaccagccagaccaccaggccggtaatcaccgctgccacgccgctccacaacaaataaccatttccgcccagcatctcggctgccagcagcaaaccgccgagactgagccagaaaatatgtggatgaacgaccattaactccatcatggctgagtccgtttgttggcgctgtctttcaccagctcggcaatcccggcaatcgaccccatcaggctgctggcctctaatggcatcatcactactttgctgttactggaggaaccgatctgctgtaacgcttcggtgtatttctgcgctacgaagtagttcaccgcctgaatatcaccggaggcgatagcttcagacaccattttggtggcgcgggcttctgcttcggcggaacgttcacgcgcttcagcctgtaaaaacgccgactgacgttcgccttccgctttcaggatttgcgactgtttttcaccttcggctttgaggatttccgcctgacggatcccttccgcttcaagaatgtaagcgcgtttggtacgttccgctttcatctgcgcgttcattgaagagataagctctgccggtgggcgcacgtcgcgaatttcaatacgggtgactttaatcccccacgggttggtggcttcatcgacaatacgcagcaggcgtgagttgatgctgtcgcgctgagagagcatttcgtcaagttccattgaacccagcacggtacggatgttagtcatggtcaggttgatgatcgccagctccagattgctgacttcataagccgcgcgcggcgcgtcaatcacctgaataaagcacacggcgtcgatggtaacgttggcgttatctttcgagataacttcctgggaagggatatcgagcacttgctccatcatattgatcttgcgaccaatgcgatccataaacggcaccaccagactgagccccggctgtaacgttttggtatagcgaccaaagcgttctactgtccactgatagccctgcggtacgattttgacacccgcgccgacaatgaccagcgcgacaaaaatgagaatcgggataaagataagcatcggaaaaacctcctgttgtaccgtccataatcagcaaaattgctgcttgattaaacaaattatacctgattactgaaagagagttcccccttattcctgcgaaggataaactgtttttagtaaaaatcagaaaaagggaacagcgatgcaggaaaatagtcctttgcttcagctacaaaacgtaggatatctggcgggtgatgcgaagattcttaataacatcaatttttcgctgcgtgctggcgaatttaagttaattaccggtccttctggttgtggcaaaagtacgctgctaaaaatagttgcttcattgatcagcccaaccagcggaacgttactgtttgaaggtgaggatgtcagcacactaaagccagaaatctaccgccaacaagtctcttactgcgcccagacaccgacgctgtttggcgatacggtatacgataatctgatctttccctggcagatccgtaaccggcagcctgacccagccatttttctcgattttctcgaacgcttcgccttgccggacagcattttgacgaagaatatcgccgagctatctggtggtgaaaaacaacgcatctcattgattcgtaacctgcaatttatgccgaaggttttattgctggatgaaataaccagtgcgctggatgaaagtaataaacataacgtcaatgagatgatccatcgttatgtgcgcgagcaaaatattgccgtgctgtgggtgacacacgataaagacgaaattaatcatgcggataaagtgattacactgcaaccgcatgccggagaaatgcaggaagcacgctatgaactcgcataatattactaacgaatcattagcactggcattaatgctggtggtggtggcaatcttaattagccataaagaaaaactggcgctggagaaagatattctctggagcgtcgggcgagcgataattcagctgattattgtcggctatgtgctgaagtatattttcagcgtggatgatgccagcctgacattattgatggtgttatttatctgctttaatgcggcgtggaacgcgcaaaaacgcagtaaatatattgctaaagcttttatctcatcgtttattgccattacggtcggggcgggaattaccctggcggtgctgattctctcagggtcgattgaatttatcccgatgcaggtgatccctatcgccgggatgattgccggtaacgccatggtagcggtggggttgtgttacaacaatttagggcaacgggtcattagcgaacagcaacagattcaggagaaactgagtcttggtgcgacgccgaagcaggcttcagcgatattgattcgcgacagtattcgcgcggctttaattccgacggtcgattcagcaaaaacggttggcttagtgagtttaccaggaatgatgtccgggctgatatttgccgggattgatccggtgaaggcgattaaatatcagattatggtgacctttatgctgctctcaaccgccagcttgtcgaccattattgcctgctatttaacctatcgtaagttttataattcgcgccaccagttggtggtgacgcaattgaagaagaaatgatgcgatgccggatgcgcagcatcgcatccggcgttgtggttcatgtgccgatcaacggaatatcaatacaacaatgcatacagctggcggcgatacttcgacgccagtgcatcacccgtacccagcgcagcgaggatctcctggaacgttttacgcgtctgaccgtctgcggcggtgagatctttacgcagatgcccgaacagcaactccagcgcctcttcattgcgcccaacctgatgcagttgcagcgccagttgcgtcgccagtgcggcatcttctggattctccgccacctgctgttgcaactgttgaatttccggcgtatcagccgcctgcttcagcagttcgatttgcgccaccagcccctggtagcgggtgtcctgatcctgcaacggaatggttttcagcaccgcttccgcatcttcagaacggttcagcgcaatcagcgtttctgccagcagcaggccgatctccccgttctgattcgacaactgccaggcgtctttcagcaatggcagggcatcggtgtaattgctttcctgcatcagttgcatcgcctgctgcgctttcagctcttcttcgcgcggcagcactttatccagcagggcgcggatcgcctcttccggttgcggcccctggaagccatctaccggttgcccgttctggaacagatacacggtcggaatcgcacgcagaccaaactgcgcggcaatcatctgctccgcgtcgcagtccagcttcgccagaataaattgcccgttgtactgcgccgcgaggctttccagaattggggttaactgcaaacagtgctggctacgttcagaccaaaaatagaacagcaccggagtggtcatcgactgttcaagaacctgttgcaggttagattcgttaatgttgacaatattttctacggacatggagtcgctctctgttgtcgatattttctttgacatgggggcttaagcgcgcgcttcaactcacccctgcaatattttgtccatcacgcgccccggcagcaggcgcttaagcaccattaccgcccaggtcaccagcgtcaccggatagcgcatcttcggcttctcgctaataaaagcatggcgtactttgtccaccaccgcttccggtcccaacgtaaagcgggcggcgatgccgggattttcgactggtttatcactttgcgtctggttgacgttgtcggtgaagcgagtacgaatgggaccgggttcgatcaggctgactttaattccgctgtggcgcagctccatgcgcagtgcatctgaccacgcctccagcgcatatttactggccgcgtaagcgccacgacccggcgtggagattaatcccatcaccgatgatgtcatcacaatacgcccttcaccgtgcggtaacatcgcgggtaacaggcgcatggtgagctggtgtgcgccgaaaaagttggcggaaaactgctgttccatctgcgcacggctgatggtggaaagggggccatacatgccgaatccggcattgttaaagatcccatacagacaattatcggtcagggcgatcacctcgtcggctgcgcgatcaacactttctggtgaatccagatcgatcaacacgccggtaaatcccatgctgttcatgcgctcaacatcatccggtttccggcaacctgccagcacatgaaaaccctggcgttttaattcgagcgcgctttccaggccaattccactggaacatccggtaattaagaccgatttttgcataactttacctgtcaggatctccgttgctttatgagtcatgatttactaaaggctgcaactgcttcgccatccagtcggcaataaacggctgggcgtcgcggttgggatgaataccgtcatcctgcatccattgtggcttgaggtagacctcttccataaaaaagggcagcagcggaacatcaaactctttggcgagtttggggtaaatggcgctaaaggcttcattataacggcgaccatagtttgcaggcagacgtatttgcattaacaatggttcagcgttggcggctttgacatcctgcaaaatctggcgcagcgtttgctcggtttgctgtggctgaaaaccacgcaaaccgtcattgccgcccagttcaaccagcacccaacgcggctgatgctgtttcagcagagccggaaggcgcgccagtccttgttgcgaggtgtcgccgctgatgctggcattaactaccgacgttttactctgccacttatcattcaacaaggcaggccaggccgcgctggcagacattcgatacccggcgctcaggctatcacccagaatcaataacgtgtccgctgcggcggcacggaaggttaacaggaccaggaacaggaagggcaaatgccagcggaaaacattgttgaagttcatcatcttaagaagtccgtcggtcagggggagcatgaactctccatcctcaccggagttgagctggttgtcaaacgtggcgagaccatcgcactggtgggcgagtcgggatcgggtaagtcaaccttgctggcgatcctcgccgggcttgatgacggcagcagtggcgaagtgagtctggtgggacaaccgctacataatatggacgaagaagcgcgggcaaagttgcgcgcgaagcacgtcggctttgtttttcagtcatttatgttaattcctacccttaacgcgctggaaaacgtcgagcttccggctctgctgcgcggtgagagtagcgcggaaagtcgtaacggggcgaaagcgttgctcgaacagttagggctgggtaaacgtctggatcatcttccggcacagctttccggcggtgaacagcaacgagtggcgctggcacgagcctttaatggtcgacctgatgtgctgtttgccgacgaacccaccggcaaccttgaccgccagacgggcgataaaattgccgacctgctgttttccctcaaccgtgaacatggcaccacgttgattatggtgacccacgacctgcaactggcggcacgctgcgaccgctgcttacggctggtgaacgggcagttgcaggaggaagcatgattgcacgttggttctggcgcgaatggcgttcgccgtcgctattaattgtctggctggcgctaagcctggcggtggcctgcgtgctggcgctgggcaatatcagcgatcgcatggagaagggcttaagccagcaaagccgtgagtttatggcgggcgatcgggcgttgcgcagttcacgcgaagtgccgcaagcgtggctggaggaagcgcaaaagcgcggcctgaaagtcggcaagcagctgactttcgccacaatgacctttgcaggcgacacaccgcagctggcgaacgtcaaagcggtggatgatatctacccgatgtatggcgatctgcaaactaatccccctggcctgaaaccgcaggcgggcagcgtattgctggccccacgcctgatggcactgcttaacctgaaaacgggcgacaccattgacgtgggcgatgccaccttgcggattgccggagaagtgattcaggaaccggattccggttttaaccccttccagatggctccgcgtctgatgatgaatctggcggatgtcgataaaaccggagccgtgcagccggggagtcgggtcacctggcgttataaattcggcggcaacgagaaccagctcgacggctatgagaaatggttgttacctcagcttaaacccgaacaacgctggtacggtctggaacaggacgaaggcgcgctggggcgatcgatggaacgctcgcaacagttcctgctgctttcggcgcttctgaccttgctgctggcagtggcagcggtggcggtagcgatgaatcattactgtcgcagtcgctacgatctggtggcgatcctcaaaacgctgggggcagggcgagcgcaactgcgtaagctaatcgtcggtcagtggttgatggtgctgacgctttcagccgttaccggtggggccataggcctgttgttcgaaaacgtgttgatggtgctgctcaagcccgttctgcctgctgcactaccgccagccagcctctggccgtggctgtgggcgcttggcaccatgacggtcatctcgctgctggtggggctacgaccatatcgcttgttgctggcaacgcagcctttacgcgtattacgtaatgatgtggtagcgaacgtctggccgctgaagttttatctgccgattgtcagtgtggtggttgtgctgctgctcgccggattaatgggtggcagcatgctgctttgggcggtgctggcgggcgcggtagtactggctttgctgtgcggtgtgctgggctggatgctgctgaatgtacttcgccgcatgacgctgaaatcgctgcctctgcgcctggcggttagccgcctgttacgtcagccgtggtcaacgttaagtcagctttcggcattttcgctctcctttatgctgctggcactgctgctggtgttgcgtggcgatctgctcgaccgctggcagcagcagctacctccagaaagcccgaactactttttaattaacatcgccacagaacaggtagcaccgctaaaagcgttcctcgcggaacatcagatagtcccggaatcgttttatccggtggtgcgggcgcggctgacggcgattaacgataagccgacagaaggtaatgaagatgaggcgcttaaccgcgaactcaatcttacctggcaaaatacgcggcccgatcataatccgattgtcgccggtaactggccgccaaaagccgatgaagtgtcgatggaagaggggctggcgaaacgcttaaacgttgccctcggtgataccgtgacttttatgggcgatacccaggagttccgcgctaaagtgaccagcctgcgcaaagtggactgggaaagtctgcggcctaatttctattttattttccctgaaggggcattagacgggcaaccgcagagctggcttaccagtttccgctgggagaatggcaacggcatgttgacacaactcaaccgccagttcccgaccattagcctgttagatattggcgcgattttaaaacaggtcggtcaggtgctggagcaggtaagtcgggcgctggaagtgatggtggtactggtcaccgcctgcggtatgttgctgttgctggcacaggtgcaggtgggaatgcgtcagcgtcatcaggagctggtggtgtggcgcacactcggtgcggggaaaaaactgctgcgtaccacgttgtggtgtgagttcgccatgcttgggtttgtttccggcctggtggccgcaattggtgcggaaacggcgctggcagtgttgcaggcgaaagtgtttgattttccgtgggagccagactggcgattgtggattgttctgccgtgcagcggagcgctgctgctgtcgcttttcggcggctggctgggtgcgcgactggttaagggtaaggcgctgttcaggcagtttgcggggtgatgagagtaaataaggggcgttctggttgaatggaacgccttgtttaaattaattctacaatatgtttcattgatgatgttattgaattggtgatttcctatctttctattgctgatattaatctgaatcggtggagtttattgattttaaatatagccctacaaaaataactcagactaataaaatcataaatcatatgcgttgaatggatattatccatatagtgaatttgttgatgatgaattcatctgtgctaaaaatgttagtttaataaaatattgaaagtgacctgtaataacagttgttgttgattgagaacaaataagtttatgtgaaaaatatataaatacattagctggtcttgtgtgtcattttatttttttttgttgctaacacagggatatgaacaataactaaaagggcactttatatgagcggaaaaccagcggcgcgtcagggagatatgactcagtatggcggtcccattgtccagggttcggcaggtgtaagaattggcgcgcccaccggcgtggcgtgctcggtgtgtccgggcgggatgacttcgggcaacccggtaaatccgctgctgggggcgaaggtgctgcccggcgagacggaccttgcgctgcccggcccgctgccgttcattctctcccgcacctacagcagctaccggacgaagacgcctgcaccggtgggcgttttcggccccggctggaaagcgccttctgatatccgcttacagctacgtgatgacggactgatactcaacgacaacggcgggcggagcattcactttgagccgctgctgccgggggaggcggtgtacagccgcagtgagtcaatgtggctggtgcgcggtggtaaggcagcacagccggacggccatacgctggcgcggctgtggggggcgctgccgccggatatccggttaagcccgcatctttacctggcgaccaacagcgcacaggggccgtggtggatactggggtggtctgagcgggtgccgggtgctgaggacgtactgccagcgccgctgccgccgtaccgggtgcttaccgggatggcggaccgcttcgggcggacgctgacgtaccggcgtgaggccgccggtgacctggccggggaaatcaccggcgtgacggacggtgccgggcgggagttccgtctggtgctgaccacgcaggcgcagcgtgcggaagaggcccgcacctcttcgctatcttcttctgacagttcccgccctctctcagcctcagcgttccccgacacactgcccggtaccgaatacggccccgacaggggtatccgcctttcggcggtgtggctgatgcacgacccggcatacccggagagcctgcccgctgcgccactggtgcggtacacgtatacggaagccggtgaactgctggcggtatatgaccgcagcaatacgcaggtgcgcgctttcacgtatgacgcgcagcacccgggccggatggtggcgcaccgttacgcgggaaggccggagatgcgctaccgctacgacgatacggggcgggtggtggagcaactgaacccggcagggttaagctaccgctatctttatgagcaggaccgcatcaccgtcaccgacagcctgaaccggcgtgaggtgctgcatacagaaggcggggccgggctgaaacgggtggtgaaaaaagaactggcggacggcagcgtcacgcgcagcgggtatgacgcggcaggaaggctcacggcgcagacggacgcggcgggacggaggacagagtacggtctgaatgtggtgtccggcgatatcacggacatcaccacaccggacgggcgggagacgaaattttactataacgacgggaaccagctgacggcggtggtgtccccggacgggctggagagccgccgggaatatgatgaaccgggcaggctggtatcggagacatcgcgcagcggggagacagtacgctaccgctacgatgacgcgcacagtgagttaccggcgacgacaacggatgcgacgggcagcacccggcagatgacctggagccgctacgggcagttgctggcgttcaccgactgctcgggctaccagacccgttatgaatacgaccgcttcggccagatgacggcggtccaccgcgaggaaggcatcagcctttaccgccgctatgacaaccgtggccggttaacctcggtgaaagacgcacagggccgtgaaacgcggtatgaatacaacgccgcaggcgacctgactgccgttatcaccccggacggcaaccggagcgagacacagtacgatgcgtggggaaaggcggtcagcaccacgcagggcgggctgacgcgcagtatggagtacgatgctgccggacgtgtcatcagcctgaccaacgagaacggcagccacagcgtcttcagttacgatgcgctggaccggctggtacagcagggcggctttgacgggcggacgcaacgttatcattatgacctgaccggaaaactcacacagagtgaggatgagggacttgtcatcctctggtactacgatgaatcggaccgtatcactcaccgcacggtgaacggcgaaccggcagagcagtggcagtatgatggccacggctggctgacagacatcagccacctgagcgaaggccaccgtgttgccgtccactatggctatgacgataaaggccgcctgaccggcgaatgccagacggtggagaacccggagacgggggaactgctgtggcagcatgagacgaaacacgcatacaacgagcaggggctggcaaaccgcgtcacgccggacagcctgccgccggtggagtggctgacgtatggcagcggttacctggcgggaatgaagctgggcgggacgccgctggtcgagtatacgcgggacaggctgcaccgtgagacggtgcgcagcttcggcagcatggcaggcagtaatgccgcatacgaactgaccagcacatacacccccgcaggccagttacagagccagcacctgaacagcctggtatatgaccgtgactacgggtggagtgacaacggcgacctggtgcgcatcagcggcccgcgacagacgcgggaatacggctacagcgccacgggcaggctggagagtgtgcgcaccctcgcaccagacctggacatccgcatcccgtatgccacggacccggcgggcaaccggctgccggacccggagctgcacccggacagtacactcacagtgtggccggataaccgcatcgcggaggatgcgcactatgtctaccgccacgatgaatacggcaggctgacggagaagacggaccgcatcccggcgggtgtgatacggacggacgacgagcggacccaccactaccactacgacagccagcaccgcctggtgttctacacgcggatacagcatggcgagccactggtcgagagccgctacctctacgacccgctgggacggcgaatggcaaaacgggtctggcggcgggagcgtgacctgacggggtggatgtcgctgtcgcgtaaaccggaggtgacgtggtatggctgggacggagacaggctgacgacggtgcagactgacaccacacgtatccagacggtatacgagccgggaagcttcacgccgctcatccgggtcgagacagagaacggcgagcgggaaaaagcgcagcggcgcagcctggcagagacgctccagcaggaagggagtgagaacggccacggcgtggtgttcccggctgaactggtgcggctgctggacaggctggaggaagaaatccgggcagaccgcgtgagcagtgaaagccgggcgtggcttgcgcagtgcgggctgacggtggagcaactggccagacaggtggagccggaatacacaccggcgcgaaaagctcatctttatcactgcgaccaccggggactgccgctggcgcttatcagcgaagacggcaatacggcgtggagcgcggaatatgatgaatggggcaaccagcttaatgaggagaacccgcatcatgtgtatcagccgtaccgtctgccagggcagcagcatgatgaggaatcagggctgtactataaccgtcaccggtactacgatccgttgcaggggcggtatattactcaggacccgatggggttgaaagggggatggaatttatatcagtatcctttaaatccactacaacaaattgaccctatgggattattgcagacttgggatgatgccagatctggagcatgtacggggggagtttgtggtgttctttcacgtataataggaccaagtaaatttgatagtactgcagatgctgcgttagatgctttgaaagaaacgcagaatagatctctatgtaatgatatggaatactctggtattgtctgtaaagatactaatggaaaatattttgcatctaaggcagaaactgataatttaagaaaggagtcatatcctctgaaaagaaaatgtcccacaggtacagatagagttgctgcttatcatactcacggtgcagatagtcatggcgattatgttgatgaatttttttcaagtagcgataaaaatcttgtaagaagtaaagataataatcttgaagcattttatctcgcaacacctgatggacgatttgaggcgcttaataataaaggagaatatatttttatcagaaatagtgtcccgggattgagttcagtatgcataccgtatcatgattaattttagtgcttttattagtggggcctataaggagattcaatgaaatatagttcaatattttcgatgctttcattttttatactatttgcctgtaatgagacagctgtttacggttctgatgaaaacattatttttatgaggtatgtggaaaaattacatttagataaatactctgttaaaaatacggtaaaaactgaaacaatggcgatacaattagctgaaatatatgttaggtatcgctatggcgaacggattgcagaagaagaaaaaccatatttaattacggaactaccagatagttgggttgttgagggagcaaagttaccttatgaagttgcgggtggtgtatttattatagaaattaataagaaaaatggatgtgttttgaatttcctacatagtaaataatgctggcgctgatggatgcggatggaaacattgcgtggagcggggagtatgatgagtggggcaaccagctgaatgaagagaacccgcatcacctgcaccagccgtaccggctgccggggcagcagtatgataaggagtcggggctgtactacaaccggaaccggtactacgatccgttgcaggggcggtatatcactcaggacccgatagggctggaggggggatggagtctgtatgcgtatccgctgaatccggtgaatggtattgatccattagggttaagtcccgcagatgtagcgctaataagaagaaaagatcaactaaaccatcaaagagcatgggatatattatctgatacttatgaagatatgaagagattaaatttaggtgggactgatcaatttttccattgtatggcattttgtcgagtgtctaaattaaatgacgctggtgttagccgatcggcgaaagggctgggttatgaaaaagagattagagattacgggttaaatctgttcggtatgtacggcagaaaagtaaagctatcccattctgaaatgattgaagataataaaaaagacttggctgtaaatgaccatgggttgacatgtccatcaacaacagattgctcagatagatgtagtgattatattaatccagagcataaaaaaacgataaaggctttacaagatgctggctatctcaagtaatctatcaaagatgataatatttatttttgctattataatcattgttgttttatgcgtaattacttatctttatttatacaaagatgaatctcttgtaagtaaacattacataaactatatggcaataccagaaaatgatggagtttttacatggctcccagatttttttccgcacgtagcggtggatatatcaatatacacaaatgtagaagatgattatttttttcttatttttccctaacaaatgatgatgggggtaggtttaagaaaacattgacagtgagggccagggaacaagtggcgaaaatcgtatcaaagaatgatccagatacaaaaaaagtgtggtgtaaatatggtaagataccagggcaaggggatggtgtaaaccttttttttgttggtgaaattaatgttacgcattattttataacaaatattggagctggattgcctgatgcttgtgcagagtaattgcttgaattaagagtctatcccatatcgaagtcgtcaacttcgtagtgaggaaaagtaaaattcctgactgagaaaagacatgtcggctattgtgtaaagccatatagctcagacgatgaatatctactcgtattcagttgtttattgagggtgagttccgaccctgaaacaacaaataaaatgaacagtcagagagtttacatagaattgcactggtcttttacgatatctgacattgtgtaatacatattcagccatgcattaattaaaatgttacgtgtttaatgtgagtccctatctgaaaataaataatccttccggattaaaataaattcttgccgggaaagaaagaggaaataaaccattagcggaaaaccagcggcacgccagggtgacatgccccagtacggcggcccgatagtccagggttcagcgggggtactgatagtcgcgccgactgcatcgagaactccatacaactttttacggaacgtcacctgataaaatttgttcagtatcgtcttttgagattctcaaggttatggagtaaccagacagaacggacaccactgtcggagataaaaaccccctgtttacgcagctcgttgctggcccggtgctgaccatgtgtcgggaaagcgacggcgtaatcaacaacagcctgttcagttgcctcatcggtacggttcttaaggttaggagcgcggcgactacgattaatctgcgcatccacaccgccttcagcgaccagttcgcggtaacgataaaacgtatcacgcgaaacgcccatgattttacaggcttttgatacgttgctgagttcttcagccagattgagcaaaccggctttgtgtttgatgacgggattggcagtatgaagcatgagagttacctcttgttttggataaggattcgacactcatatcaaaaccggtaactctcaacctttcaaggccatgtgtcagatcaagtcgcgactaatacaaatacgtccctcattaccgcgccttaacccattccgccacttccgcccactcaccgcgaaagacaactttttccgcttttttctcaagctgatagcgatacatcgggtcgtaatattcttcaagtaacggcaccagccaggccagatgaccgtcggtgctgccggtggtgagttgcgttgtcagtgctgcatccagccttgcagccagttcgttatagcgctgtagccccagccgacgcttaatcgccgaaagtccgtgatgcaggtattcgcaatactcctgccagccctgttcgtcgccgtacgcgtgggtaaaatcatgatgcatacgcaagaaatactcttcgttcaggcgctcaagacggatctcaaacggatcttctaccaccgcaatcgccgcctgagtcattcgctcgcgcaggcattccggcaggtgattcgaaccgatcatccggctttcgtcttccagcacccacaggcgcaaattctgacgggcgtcggtttttagcatttcggcagccagcaggttttcaaaactcgcctggctaagttgtggttgtaacgtgcgaccaaacgccgaaccgcgatgacgcgccaacccttccagatcaacaccgttcggctgttgctgcactaacagcgttttaccgctgccggtacaaccgccaatcagcactatcggtttttgtgccagttcaatagtcgcctgaatcgcggtctggcgcagtgccttataaccgccttccaccagcggataatcaatccccgctgcatgcaaccagctttgcacaatatgtgagcgctgaccgccacgggcgcagcagagaataccttgcggattttgcaggcacgctgcccgccaggcgtccatgcgctgctgacgaatttcacccgccaccagtttatgtcccagcgccagcgctgcgtctgagccttgctgtttatagcaggtgccaacggcggcgcgttcatcgttattcattaacggcagattgatagcggcgggcattgcgccgtgctcaaactcgataggggcgcgaacatcaataatgggcgtatcagcaatcagcagggcacgatagtcctgttccgtgtgtctctcttgcatagttaaaagtgaacctcaaatcagcttgcgcgctattttacgcgccaacgcgcaaggaaacttgatttttaactgcgtgggttgccgaaaatttctaaaaatccgctgatttccggcctgcgctgggtaaacaaggtcacaatatcttctaccgctttgccgctgccaaatttgcgccatgccagactcaatggcgaaggagggcgcatcgttgggattacccggctgaccagttgttgattatcgatcattgactggcaaagcgattttggcaaaaaaccaatgccaacgcccgccagatgggcggcgattttcgtttccatatcgggaacaataatctctttttgccctggcaatcgccaggcgacgcgtttggttaaggtgcgggcgctgtcttcaatattgaccgccggaaagcgccgcaactgcgcttctgttagcggctcttcaacgttcgccagcggatgatccgccgccatgacaaagcgccattgcaccgatcctaagggatcaagactaaaggtatttgccagcgcctcagttcccgtgacgccgatagccagcgaaaaaccttcgtacaatagcgagtcccagacgcccatatagatttgtcgggagatgtgaaactgggtaaaggggtaacgctcattcagccacgccagcaactgggcgacggcctgggggttgtagagcaggttgttgatgacaatattcacctggcgttccacgccatcattcacctgttgcagctcgcttggcatactttccagccagctcagccagtctctggcctgggaaagtagatgctcgccagccgctgtcaacgtcacgctgcgagtcgtacggaaaaacagcgctactccggtattctcttccagaagtttaatgcgataactgatcgtcgccgtggttttacataatcgttctgccgcttttgaaaaacttcctgtttcagcaaccgcaatgaaagtccgcaaggtttctggatcgaacatcttcaggtatccccttttaaatccgcaagttgcgtgattttcttatcctctgatttatcagtatttttacatgataaccctgttcaatttgtggactaaatctagttttggaaaaatattccaacttttgtattgatgttgttctcttaaggttttagattgcctgttattgaaaccaagctgaccggtcggcggtggttgaacggaattatgttacaaggacaaaaagatgaaacttcaggtattaccgttaagtcaggaagcctttagtgcttatggcgacgtaatcgaaacgcagcaacgggattttttccatattaacaatggcctggtggagcgttaccacgatttggcgctggttgagattcttgagcaagactgtacgcttatcagcattaaccgcgcgcaaccggcgaatctgccgctgaccattcacgaactcgaacgtcatccgctgggtactcaggcctttatcccgatgaaaggtgaggtgtttgtggtggtcgtggcgttaggtgacgacaaaccagacctgtcaacgctgcgggcgtttatcaccaacggcgaacagggagtgaattaccatcgtaacgtctggcatcacccacttttcgcctggcagcgcgtcaccgattttctgaccatcgatcgcggcggcagtgacaactgtgatgttgaaagtattcctgaacaggaactctgttttgcgtgacgcctgcaaccgacttgcataagataaactaattgttcattgtttatgctcacttgtaggtcggagttaacgtaggtatgacggaagttagacggcgcggcaggccaggacaggcggagcctgtggcacagaagggcgcacaggcgttagagcggggaattgcgattctgcaatatttggaaaaaagtgggggaagttcgtcggttagcgatatttctctcaatctggatttgccgctctccacgacctttcgcttgctgaaggttttacaggcagcggattttgtctatcaggacagtcaattaggctggtggcatataggattaggtgtctttaacgtcggtgcggcgtacatccataaccgcgatgtcctctccgtcgccgggccgtttatgcgccgcctgatgttactttccggcgaaacggtcaatgtcgcgatccgtaacggcaatgaagcggtattaattggtcagttagagtgtaaatcgatggtcaggatgtgtgcgccactgggcagtcgtctgccactgcatgcttccggtgcgggcaaagcgctgctttatccgctggcggaagaggagttgatgagcatcattctgcaaaccggtttgcagcagtttacgccaactacgcttgtggatatgcccaccttgctgaaggacctggaacaagcgcgtgaactgggctataccgtagataaagaagagcatgttgtaggtctgaattgcatagcttcagcaatttacgatgatgtcggtagtgttgttgccgctatctccatctccgggccttcatcaagactgacagaagatcgttttgtcagtcagggtgagctggtcagagacaccgcccgcgatatcagcacggcgttgggactgaaagcacatccataatgtctgtcgcatcccgctctgcggagcgggtttttttgacaaaatttgaaagttggaaaaattttccaataaatagaggtaggaataaaatggcaaaaatgagagccgttgacgcggcaatgtatgtgctggagaaagaaggtatcactaccgccttcggtgttccgggagctgcaatcaatccgttctactcagcgatgcgtaagcacggcggtattcgtcacattctggcgcgtcatgtggaaggtgcttcgcacatggcggaaggttatacccgcgcaacggcagggaatatcggcgtatgtctggggacttccggtcctgcgggcacggacatgatcaccgcgctctattccgcttctgctgattccattcctattctgtgcattaccggccaggcaccgcgcgcccgtctgcataaagaagattttcaggccgtagatattgaagcaattgctaaaccggtcagcaaaatggcggttacagttcgtgaagcggcgctggtgcctcgcgtgctgcaacaggcatttcacctgatgcgttctggtcgtccgggtccggtactggtggatttaccgttcgacgttcaggttgcggaaatcgagtttgatcctgacatgtacgaaccgctgccggtctacaaacctgctgccagccgtatgcagatcgaaaaagctgtagaaatgttaatccaggccgaacgtccggtgattgttgccgggggcggggtaattaatgctgacgcagctgcactgttacaacagtttgctgaactgaccagcgttccggtgatcccaacgctaatgggctggggctgtatcccggacgatcatgaactgatggccgggatggtgggtctgcaaaccgcgcatcgttacggtaacgcaacgctgctggcgtctgacatggtgtttggtatcggtaaccgttttgctaaccgtcataccggctcggtagagaaatacaccgaagggcgcaaaatcgttcatattgatattgagccgacgcaaattggtcgcgtgctgtgtccggatctcggtattgtctctgatgctaaagcggcgctgacactgctggttgaagtggcgcaggagatgcaaaaagcgggtcgtctgccgtgtcgtaaagaatgggtcgccgactgccagcagcgtaaacgcactttgctgcgcaaaacccacttcgacaacgtgccggtgaaaccgcagcgcgtgtatgaagagatgaacaaagcctttggtcgcgatgtttgttatgtcaccaccattggtctgtcacaaatcgctgcggcacaaatgctgcatgtctttaaagaccgccactggatcaactgtggtcaggctggtccgttaggctggacgattccggctgcgctaggggtttgtgccgctgatccgaaacgcaatgtggtggcgatttctggcgactttgacttccagttcctgattgaagagttagctgttggcgcgcagttcaacattccgtacatccatgtgctggtcaacaacgcttatctggggctgattcgtcagtcacaacgcgcttttgacatggactactgcgtgcaactcgctttcgagaatatcaactccagtgaagtgaatggctacggtgttgaccacgtaaaagtagcggaaggtttaggttgtaaagctattcgggtcttcaaaccggaagatattgcgccagcctttgaacaggcgaaagccttaatggcgcaatatcgggtaccggtagtcgtggaagttattctcgagcgtgtgaccaatatttcgatgggcagcgaactggataacgtcatggaatttgaagatatcgccgataacgcagcggacgcaccgactgaaacctgcttcatgcactatgaataagggagataaataatgttacgtttctctgctaatttatcgatgttatttggagaatatgattttctcgcccgttttgagaaagctgcgcagtgtggttttcgcggcgttgaatttatgtttccttatgactacgacattgaagaattaaaacatgtgctggcgagtaataaactcgaacatacgctgcacaatttaccggcgggtgactgggcggcgggggagcgcggtattgcctgtattcctggccgtgaagaagagtttcgggatggcgtagcagcagcgattcgttatgcccgtgcgctgggtaataaaaaaattaactgtctggtcggtaaaacgccggctggtttcagcagtgaacagattcacgcaacgcttgtagaaaacctgcgttatgccgcgaatatgctgatgaaagaagatattttattactgattgaacctattaaccattttgatattcctggtttccatctcaccggaactcggcaggcgctgaaattgattgatgatgttggttgctgcaatttgaaaattcagtatgacatttatcatatgcagcggatggaaggtgaattaaccaacaccatgactcagtgggctgataaaattggtcacctgcaaattgccgataatccgcatcgcggcgaaccgggaaccggagaaattaattatgattatctctttaaggtaatcgaaaattctgactacaacggttgggttgggtgtgaatataaaccccaaaccaccacggaagccggtttacgctggatggatccgtaccgttaaaacgtaacgctattcagacaatgcttttttaggccgctaagttggcaggggatcgtgttgtctgaattcaggaaaagcgaaatttaaaagaggttaattatgaaactgggatttattggcttaggcattatgggtacaccgatggccattaatctggcgcgtgccggtcatcaattacatgtcacgaccattggaccggttgctgatgaattactgtcactgggtgccgtcagtgttgaaactgctcgccaggtaacggaagcatcggacatcatttttattatggtgccggacacacctcaggttgaagaagttctgttcggtgaaaatggttgtaccaaagcctcgctgaagggcaaaaccattgttgatatgagctccatttccccgattgaaactaagcgtttcgctcgtcaggtgaatgaactgggcggcgattatctcgatgcgccagtctccggcggtgaaatcggtgcgcgtgaagggacgttgtcgattatggttggcggtgatgaagcggtatttgaacgtgttaaaccgctgtttgaactgctcggtaaaaatatcaccctcgtgggcggtaacggcgatggtcaaacctgcaaagtggcaaatcagattatcgtggcgctcaatattgaagcggtttctgaagccctgctatttgcttcaaaagccggtgcggacccggtacgtgtgcgccaggcgctgatgggcggctttgcttcctcacgtattctggaagttcatggcgagcgtatgattaaacgcacctttaatccgggcttcaaaatcgctctgcaccagaaagatctcaacctggcactgcaaagtgcgaaagcacttgcgctgaacctgccaaacactgcgacctgccaggagttatttaatacctgtgcggcaaacggtggcagccagttggatcactctgcgttagtgcaggcgctggaattaatggctaaccataaactggcctgatacccgcaataaaaatggccgatatcagaaaatgaatcggccagcaatattaaaaaagaaagcagccaaagatgttgcttcagtattaaaaataatatttttattttatttgttcctcatagctagattaaaacaacgttattcgatacgtgaaattaagagggatttatggaacatcagagaaaactattccagcaacgcggctatagcgaagatctattgccgaaaacgcaaagccagcggacctggaaaacatttaactattttaccttatggatgggttcggttcataacgttcccaattatgtgatggtcggcggcttttttattctcggcttgtctacctttagtattatgctggcaattatcctcagcgcctttttcattgccgcggtaatggtattaaacggtgctgcgggcagtaaatacggtgtgccttttgccatgatcctgcgtgcttcttacggtgtacgtggtgcactgtttcccggattattaaggggcggaattgccgccatcatgtggtttggtttgcaatgttacgcggggtcactggcctgcttgattctgattggcaaaatctggccgggatttttaactctcggtggtgatttcactctgttaggcctttctctaccgggcttaattactttcttaatcttctggctggtcaacgttggtataggttttggcggtggcaaagttttaaataaattcactgccattcttaacccgtgcatctatatcgttttcggcggtatggcgatttgggcgatttcactggtcgggatcggtccaatctttgactacattccgagcggtattcagaaagcagaaaacggtggcttcctgttcctggtggtgattaacgcggtagttgcggtctgggcggcaccggcggtgagcgcatccgactttacgcaaaacgcccactcgtttcgtgagcaggcgctggggcaaacgctgggtttagttgtggcctatattctgtttgcggtcgccggggtatgtattattgccggagccagtattcactacggcgctgatacctggaacgtgctggatattgttcagcgttgggacagcctgttcgcctcgttctttgcggtactggttattctgatgacaactatctccactaacgcgaccggtaatattattccagccggttatcagattgccgccattgcaccgacaaaactgacctataaaaacggcgtactgattgccagtattatcagcttgctgatctgcccgtggaaattaatggaaaatcaggacagcatttatcttttcctcgatattatcggcggaatgcttggtccggtaattggtgtcatgatggcgcattattttgtggtgatgcgcggacaaattaatcttgatgaactgtataccgcacctggcgattataaatattacgataacggttttaacctcactgcgttttcagtaactctggtggccgttattttatctcttggcggtaagtttattcactttatggaaccgttatcgcgtgtttcatggtttgtcggcgtcatcgtcgcctttgcggcctacgccttattaaagaaacgtacaacagcagaaaaaacaggagagcaaaaaaccataggttaattaatcccgatattgaacattgagttaaaaaccaatctgtattttacaaggagtttgttatgtcttttgatttaatcattaaaaacggcaccgttattttagaaaacgaagctcgcgttgtagatatcgccgttaaaggcggaaaaattgctgctatcggtcaggatctgggcgatgcaaaagaagttatggatgcgtctggtctggtggtttcgccgggcatggttgatgcgcacacccatatttctgaaccgggtcgtagccactgggaaggttatgaaaccggtactcgcgcagcggcaaaaggtggtatcaccaccatgatcgaaatgccgctcaaccagctgcctgcaacggttgaccgcgcttcaattgaactgaagttcgatgccgctaaaggcaagctgactattgatgcggcacaactcggtggcctggtgtcttacaacatcgaccgtctgcatgagctggatgaagtgggcgttgtcggcttcaaatgcttcgttgcgacctgtggcgatcgcggtatcgacaacgacttccgtgatgtaaacgactggcagttcttcaaaggtgcgcagaagctgggcgaactgggtcagccggtgctggtgcactgcgaaaacgcgctgatttgtgacgaactgggcgaagaagcgaagcgtgaaggtcgcgtaaccgctcatgactatgtggcttcgcgtccggtatttaccgaagtggaagcaattcgccgcgtactgtatctggcgaaagttgctggttgccgtctgcacgtttgccacgtcagcagcccggaaggtgttgaggaagtgactcgtgcacgtcaggaaggtcaggacgttacttgtgaatcctgcccgcattactttgtactggataccgatcagttcgaagaaatcggtactctggcgaagtgttcaccgccgatccgcgatctggaaaaccagaaaggcatgtgggaaaaactgtttaacggtgaaatcgactgcctggtttccgaccactctccatgcccgccggaaatgaaagccggtaacatcatgaaagcatggggcggtatcgccggtctgcaaagctgcatggacgtgatgttcgatgaagcggtacagaaacgcggtatgtctctgccaatgttcggcaaattaatggcgactaacgcagcagatattttcggtctgcagcaaaaaggccgtatcgccccaggaaaagatgccgacttcgtcttcattcagccgaatagcagctatgttcttaccaatgacgatctggaatatcgccacaaagtcagcccgtatgttggccgtaccattggcgcgcgtatcacgaaaaccatcttacgtggtgatgtgatttacgacattgaacagggcttccctgttgcgccgaaaggtcaatttatccttaaacatcagcagtaatctggcccctgcaatgcccgtccttgcggcgggcattctccggttaaggtgtgtttatgttcaattttgcagtcagccgcgaaagcctgttatcaggatttcagtggtttttctttattttttgcaacacggttgtggttcctcctacgctactttctgcttttcagttgccgcaaagtagcctgcttacgctcacgcaatatgcttttcttgctaccgcactggcctgcttcgctcaggcgttttgcggtcatcgtcgcgctattatggaagggccaggtggcctgtggtggggaaccatccttactatcacccttggtgaagcatcgcgcgggacaccgatcaacgatatcgccaccagcctggcagtggggattgcactctccggcgtgctgacgatgttgattggttttagcggattaggccatcgcctggcacggttatttacgccgtcggtgatggtcttgtttatgttgatgctgggcgcgcagctgaccactatctttttcaaaggtatgctcgggctgccgtttggcatagccgacccgaattttaaaattcagttaccgccgttcgcgctctcggtggcggtgatgtgcctggtactggcgatgattatcttcctgccgcaacgttttgcccgttatggcctgctggtcggcaccataaccggctggttgttgtggtacttttgctttccttcttcgcactcgctctccggtgagttgcactggcagtggttcccgctcggcagtggcggtgctttgtcgccgggaattattctgacggcggtgattacaggtctggtaaatatcagcaatacctacggtgcgattcggggcacggatgttttttatccgcagcagggcgcagggaatacgcgttatcgtcgtagctttgtggcgaccggatttatgacgctgataaccgtaccgctggcggtaattccattttcaccgtttgtttcatccattggtttattaacccagactggcgattacacgcggcgttcgtttatttatggcagcgttatttgcctgctggtggcgctggttcctgcactcacgcgactgttttgcagtatccctttacccgtgagtagtgcggtcatgctggtttcttatctgcctttactcttttccgcgctggtgtttagccagcaaataacgtttaccgctcgcaatatttatcgactcgcattgccgttatttgtcggcatatttttaatggcattaccgcctgtgtatctgcaagaccttccattaacgcttcgtcctctgctcagtaacggcttattggtcgggattttactggctgttcttatggataaccttattccgtgggaacgcatcgaataatttgttgaaaaaggattgataatgaagattgtcattgcgccagactcttttaaagagagcttaagtgcagaaaaatgttgtcaggcaattaaagccgggttttcgaccctctttcccgatgcgaactatatctgtttgccgatagcggatggcggcgaagggacggtggatgcgatggtcgccgcgacgggcggcaacatcgtgacgcttgaagtctgcgggccgatgggcgaaaaagtgaatgctttttatggccttaccggcgacgggaaaacggcggtgattgagatggcggcagcaagtggcctgatgctggtcgcgcctgaaaagcgtaatccgttgctggcctccagttttggtacgggggagttaattcgtcatgcgctggataacgacattcgccatattattctcggcattggcggcagtgcgacggtcgacggcggtatgggcatggcgcaggcgctcggtgtgcgtttccttgatgccgacggtcaggcgctggcggcaaacggtggtaatttagcgcgcgtggcaagcattgagatggatgaatgcgatccgcgtctggcgaattgccatattgaagtagcatgtgacgttgataacccgctggtaggggcacgcggcgcggcggcggtgtttggcccgcaaaaaggggcaacgccggagatggtcgaagaacttgaacaggggctgcaaaattacgcccgtgttttacaacagcaaactgaaattaatgtctgccagatggcgggcggcggcgctgcgggcggtatgggtattgcggcggcggtatttctcaatgcggatattaaaccgggcattgaaattgtgttgaatgcggtcaatcttgcgcaggcagtgcagggcgcagcactggtgattaccggggaagggcgcatcgactcgcaaacggcaggcggtaaagcgccgctgggtgtggcgtcggtggcgaagcagtttaatgtaccggtgattgggattgctggcgtattgggtgatggcgtggaagtggtgcaccagtacggcattgacgcggtattcagcattttgcctcgtctggcacctttagccgaagtgctcgccagcggtgaaaccaatctcttcaacagcgcgcgaaatattgcctgcgccattaaaataggtcagggaattaaaaactaacccttacctttaaagcggatgcgatttatatcgcataagagtgcagtactcatgccggatgcggcatgagtaccatatccttcctgaaaatcgcgcaaattctatatattgcagagatcatgtaggcctgataagcgaagcgcatcaggcaatgttacaaaaaaagccacggtataaaccgtggcaaaatccaacatagctaaaaataatcaggcgagtggtatgacttaaatctctacgtcgcggttacaatctttcgagtaaatatagctgaacgcttcaccacgccctacaccataaccagcctgtaaagaataagcgcccataaagatgtaatcgccttttttcaccgggatccagttattgtcgaggttataaaccccctgaccggaaagaatataggcaccgtgttcctgaacgtgtgtttcgatataaccgtggctggcacctggtgcaaaagagaggatatgcatgttcatatcaaaacctaactctttgggcagaaaatccagcagaataacatcgtccatgccttcataatgaatgcgttccagttcgctggcattgccagaaaccagccacggtgcatagccttctaccggaacatagcggcgcttatataaaaagatttggctgtcttcggcctgggcgttaacaaacgtcattaaggagcctggcgggcaataaagatagccaccttcgcttaaggcaaatgttttgccttcggctttggcagtgatatttccagagatcacatacaggaacgtttcaatgccttcgccaccgaagccctgttggttgccaccgttttgatgcagtgtgaccagataatcaacaaaagaggcacccagctttggcgtggagaggattgtcgcgtcacaattttcaaagcccggaataatattttttaccagaccatccggggttaacagtgcgaaattaccgtgtttaacaatcgcacggttagccagtaaatcttcgcggtaaccggtgacgttatttaaatatcccatttatgactccttatttctgccaggcaagttgataaagcatgagtgccaacgttttgaccccttcggcaaggtcggtaatattggtgcgttccgccgggttatggctgatcccgttgatgctggggataaaaatcatgcaggttggtacgcgaggcgcgaaaatttgcgcgtcgtgcccggcaccactgtgcatcacccggtaattcagtttttctctttcacacaattctgtcagggtggcgaccagctccttattcatcggcacgggttcttcgtccatccataaatcgatatcaataccaatgtccatttcatcgcaaatcgcccgcatgtcgttttctaactgttgggtgaaatcgcgcagcacggcagcgtcggtatgacgacaatcaatggtgaacgtggttttacccggcaccacatttaccgtattcgggcgcggctctactttgccaaaggtcagaaccagcggatcgcccatccttttcgctttttcgaccgactgatggcaaatgcgactgaaagcgtaaactgtatcacgacgataacccatcggcgtggtgcctgcatggtttgattcgccgttcagcgttaccgtataacgacgctgcccgacaattgcattcaccacgccaattgattgcccattactttccagcacacagccctgttcaatatgcagttcaacaaaggctttaatatcctgacgcggagttagtggggcgttcggaagagtaaatccgcaagccttcatcgcatcgacaaaactatttcctttggcatcacagatattccgcacgtcgtcaggattcgccagcccaaaaatatttttactgccccagaagacatacgggaagcggctgccttcttcttctgccatcgccaccacttcgaccgtacgtagcggcgcgccgtattgcgttttcagccagtcaattgccagccacgccgccagcgcgccgaattgcccgtcaaggttaccgccgttaaccacggtatcgatatgcgaaccgctcagaaccacttcctgtggatattcggtgccattcaggcgaccgtataaattccccacttcatcgaaacgtgtttccagcccgcttgctgccattctttttttaaattgctgctgggtttccagccattccggcgaataaagtaaacgggtcatcccacccgctgggtcagcgccaaaagaggaaagccagggcagcgtttcttctatagcttgacggaaatgtgtaatcataagaaagtcctgtctcaataattattgcgcaaagggatttttcgtttcgtatgacgtgttataaagcgcgtcggaaattaaatactggtaaatatcatcaacaatttcgatgccttcgacggcggctttgcgttgtttaatatcctgatcctgtccgggataataaacctgattaaaaccgggcgcgggggtaatggcatttaattcgcgcatggtctggctaagatgttgacggaataattcgctggaggagaaaaagttcggattaataactatatgtaattgccccaaattacgccctgcgtgtaaatcgtcatacatcgaactaacctgtcgcccgaacggtaagccgagtaagacgcctgagaggacgtcaatcatcatcatcaggccatacccttttggcccggcggcggggagcagagcatgtaccgcgaacggatcggttgttggtacaccgtttttatcgaccgcccaggtatccgggatagacatattacgcgagcgggcgtcgagcacttttccccatgcctgtacggtagtcgccatatcaaaggtaaggatctcgtcgccttctcccggcgcggcaaaggccagggggttagtaccgtagtaaatttccgcgccgccaaacggcaccaccattggatcggactggcacatcgaaatgccaatgaatccggcgcgggctgcctgctgcacaaaataagagattgcgccgctgtgacccatccggctgataccgaccaccgcaacgccattttgctgggcggttttgatggcatgttccatacccattttcgccgcgacctgtccggcggcattgtcggcatgtaaaattgccgagcacggcccggtttcctcaagacgaaactccggttcgcggttggtgccgccttttgaaatgcgttccgcgtagtattccacgcgcaccgcgccatgagagtggatccctctggcatcggcgtaaaccaatacttcagccacggttgcagcgtgctcacgttttaacccagcctggcagagtttattctcaattagctggtggagtgtttcccgactgattttcatctgtcttcctttttaacgacggtgtgaagcatgactgcaattaacatacagggaaaatatctggattatgtgatccagacaggcaaaaaaatatagttagaatttatttgataatccgctcacttttaacctgatttttaaaacaacaacgcttattaaaaaataatgagtaatagcctggtggttatttgaattcttttgttaataattcctgtgtgatattcatcaccttatttactcgttgtcatcgataccgtaatcgccacattaacactgctcgtgcaattgccatgggtgcaatttttaaggagttgttatgatccacgcctttattaaaaaagggtgttttcaggattcggtcagtttaatgattatttcacgaaaactcagcgaatcagaaaatgttgatgatgtttccgtaatgatgggtacgcccgccaataaagcgttattagataccacaggtttctggcatgacgattttaataacgccacgccgaacgatatttgcgtggcaattcgtagcgaagcggcggatgcggggatcgcgcaggcgattatgcagcagcttgaagaggcgctaaaacaactggcgcaggggtcaggcagcagccaggcgttgacgcaggtgcgtcgctgggacagtgcctgtcagaaattacccgatgccaatctggcgctgatttcagtggctggcgagtatgcggcggagctggcaaaccaggcgctggatcgcaacctcaacgtgatgatgttctccgataacgtcacgctggaagatgaaatccaacttaaaacccgcgcgcgggaaaaaggcttgctggtgatggggccggactgcggtacgtcgatgattgccggcacaccgctggcttttgctaacgtgatgccggaaggcaatattggcgtcattggcgcttccggtaccgggattcaggagctgtgttcgcagattgcgctggcaggggagggaattactcacgcgattggccttggcgggcgcgacctcagccgtgaagtgggcggcatcagtgcgctaacagcgctggaaatgctcagtgcagacgagaaaagcgaagtgctggcatttgtttcaaaaccacctgccgaagctgtgcgtctgaaaattgttaatgccatgaaagcaaccggcaaaccgacggtggcgctgtttttaggttataccccggcggtggcccgcgacgagaatgtctggtttgcctcctcgctggatgaggccgcacgcctggcttgcctgctttcacgcgtcacggcgcgacgtaacgcaatagcgcctgtcagcagcggatttatttgcggtttgtataccggcggtacgctggctgccgaagcggcgggattacttgccggacaccttggcgtggaagccgacgatacccatcaacatggcatgatgctggacgccgatagccaccagattattgacctcggcgatgatttctacaccgtcgggcgtccccatccgatgatcgacccaaccttacgcaaccagttaattgccgatctcggcgctaaaccgcaagtgcgcgtgttgctgcttgatgtcgtgattggcttcggtgcgaccgccgatcctgccgcctcgctggtgagcgcctggcaaaaagcctgtgccgcgcgtttagataatcaaccactgtatgccattgccacggtgacaggcactgaacgtgacccgcaatgccgctcgcagcaaatcgccacgctggaagatgcggggattgcggtcgtgagttcgctaccggaagccaccttgctggcggcagcgttaattcatccgctctcgcctgccgcacagcaacacacaccgtcattactggaaaacgtcgccgtgattaacatcggattacgcagctttgcgctggagctacaaagcgccagcaaaccggttgtgcattaccaatggtcgccagtcgccggtggcaataaaaaactggctcgtttattagaacgtttgcaataaggggttcccatgtttacatcagtggcgcaagccaatgctgcggttatcgaacaaattcgtcgcgctcgtccacactggctggatgtgcaaccggcttcttcacttatcagcgaactaaacgagggcaaaacactgcttcacgccgggccgccaatgcgctggcaggagatgaccggacccatgaaaggggcgtgcgtgggcgcatgtctgttcgaaggttgggcgaaagatgaagcgcaggcgctggcaatactggagcagggggaagtgaacttcattccttgtcaccatgtgaatgccgtcgggccaatgggcggtattacttctgccagtatgccgatgctggtggttgagaacgtgaccgacggcaaccgggcgtactgcaacctcaacgaaggtatcggcaaagtgatgcgttttggcgcttacggcgaagatgtcctgactcgccatcgctggatgcgcgatgtgttaatgccagtattaagcgcggcgctggggcgcatggagcgcggtatcgatctcacggcgatgatggcgcagggcattacgatgggcgatgagttccatcaacgcaatattgcttcctctgcactgttaatgcgtgcgctggccccacaaattgctcgcctcgatcatgataaacagcacatcgccgaagtgatggatttcctcagcgtgaccgatcagttcttcctcaacctcgcgatggcttactgcaaggcggcgatggatgctggcgcgatgatccgcgcaggcagcatcgtcacggcaatgacccgcaacggcaatatgttcgggattcgggtaagcgggctgggcgaacgctggtttactgcgcctgtaaacactccgcaaggtctgtttttcaccggcttctcgcaggagcaggcgaacccggatatgggcgatagcgcgattaccgaaacctttggtatcggaggtgcggcaatgatcgcagcgcctggcgtaacgcgctttgtcggtgcgggtggcatggaagcggcaagagcggtatctgaagagatggcggaaatttaccttgaacgcaatatgcagttgcagatcccaagctgggattttcagggcgcgtgcctggggctggacattcgtcgcgtggtagaaaccggcattacgccactcatcaataccggtatcgcccataaagaggcggggatcgggcagattggcgcaggcaccgtgcgggcaccgctggcgtgctttgaacaggcgctggaagcactggctgaaagcatgggtattggttgaggaacgcgcaatgacgatcatccatcctctgcttgccagtagtagcgcaccgaattatcgccagtcctggcggttagcgggagtgtggcggcgggcgattaacctgatgacggaaagcggcgaactgttaacgttgcatcgtcagggtagtggtttcggccccggaggatgggtgcttcgccgtgcgcaattcgatgcgttatgcggtggattatgcggcaatgaacgaccacaggttgtggctcaagggattcgcctcgggcgtttcacggttaaacagccacagcgttattgtttgctgcgtattacgccgcctgcgcatcctcaaccacttgcagctgcatggatgcaacgcgcggaggaaaccgggcttttcgggccactggcgttggcggcaagcgatccgctgcctgctgagttacgccagtttcgtcactgttttcaggccgcgctcaatggcgttaagaccgactggcggcactggctgggtaaaggccccggattaacgccgagtcatgatgacacgctgagcggaatgctgctggcggcctggtattatggcgctttagatgcgcgctccggtcgtccgttttttgcctgttccgacaatctgcaactcgttaccacagcggtgagcgtcagttatttacgttatgccgcgcaaggatatttcgcctcgccactcctgcactttgttcatgctctgagttgcccgaaacgtaccgctgttgcgattgattcgctgctggcgctggggcatacgtcaggggcagatacgctgctggggttctggcttggccaacaattattacaaggaaaaccatgaaaacactggttgtggctcttgggggcaacgccttactccagcgcggtgaggcgctgacggcagaaaatcaatatcgcaatatcgccagtgctgtacccgcgctggcacgcctggcccgttcttatcggttggcgattgttcacggcaacgggccgcaggtggggctgctggcattgcagaatctggcgtggaaagaggtagaaccgtatccgctggatgtgctggttgcggaaagccaggggatgattggctatatgctggcgcagagtttgagcgcacagccgcagatgccgcccgtgacgacggtgctgacgcgcattgaggtttcgcctgatgatccggcgtttttgcagccagagaaatttattggtccggtttatcagccagaagaacaagaggcactggaagcggcttacggctggcagatgaaacgtgatggtaaatatttgcgccgggtggtggcgtctccgcaaccgcgtaaaattctcgacagcgaagccatcgagttgttgctcaaagaggggcatgtggtgatttgcagtggcggcggcggtgtgcctgtgacggatgacggagcagggagtgaagcagtgattgataaagatctcgccgctgcgttgctcgccgagcagattaatgcagatggactggtgatcctcaccgatgctgatgcggtatatgaaaactggggaacgccgcagcaacgtgccattcgccatgccacaccggatgagttagcgccatttgccaaagccgatggttcgatggggccgaatgtaacggcggtgagtggttatgtcagaagccgtggtaaacccgcgtggattggggcgttatcgcgaattgaagagacgctggcgggcgaagcggggacctgtatttcgctgtagtcgtaggcattagacatttgtgcctgatgcgacgcttgacgcgtcttatcaggcctacaaccggtgccgcatccggcaattggtgcacaatgcctgatgcgatgcttgacgcatcttatcaggcctacaatgggtaccggatcggtaggccggataaggcgtttacgccgcatccggcaagaatagagcaccagttaaccgaacttactctgcgcccaaatcacgccgctggcatattccggcggcagcagcgggattaaggcttccagcgtcgcagtcagacgcgatgtgtcgctgtcggtcaaattcagatgccccactttacgccccggacggacttctttgtcgtaccagtgcagatgcaccagcggcagtttcagccagtcataattcacatcgctaccaatcagattgatcatcaccgacggattattcaccactggttgcggtaacggcagatcggtaatcgcccgcagatgcagctcaaactggctgatgctggcaccgttttgtgtccagtgaccgctgttatgcacacgcggtgccagttcgttgatcaacagaccttgcggggtgacaaaacactccatcgccatcacgcccacatagcccagctcctgcataatcgccgacagcatctcttcggcttgcgcctgctgctgtgcgttggcctgcggaaaagcgacgctggtgcgcaaaataccgtcctgatgcaggttatgcgtcagcggataaaacacggtgctgccatcaaagccgcgcgcgccaaccagcgacacttcaccagagaagttaatgccctgctcgacaatacattcgccgtaacactctgccggtaactgttcggtttcatttgcgcgtaaacgccattgaccgcgaccgtcataaccaccagtgcgacgcttaacaatcgccagctcacctaaacgatcaaacaccgcaggccactcgctgcgttcggcaagtaactgccacggtgcagtcggcaggtggagcttatcgaaaagctgcttctgagtcagacggtcagcaataatcgggaacacatcgcggttcacaaaggccggatggcgcgccagctcgcgggttaatgcggtttccggccagcgttctatctcagcggtaatcacgctttgttgaaaaggcaccgccgccggttcagcgtccagcccgactggccagacagcaatgcctaacggttcgcctgcctgacgcagcatacggcctaactgcccgttaccgaggacgcaaacctgtttcatgccgcacctcgcgggtccgggttttccagcacttcgtcggtctgggctttgcgccagtcattcagacgctggtgcagttctttatcatgagtcgcaagaatttgtgctgccagtaacgccgcgtttgccgcgccagctttaccaatcgccagcgtacccaccggaatgccgcgcggcatttgtacgatggagtagaggctatcgacaccgctcagtgcggcgctctgtactggcacgcccagcaccggcaccagcgttttggcggcaatcatgcctggcagatgcgctgcgccgcctgcgcccgcaataatcacctgataaccgttctcttcggcgctttcggcgaagctgaacagtttatcgggggtgcggtgagcagaaaccacttcaacgtggtgcgggacattcaggatttcgaagatttcggcggcgaactgcatggtagcccagtcgcttttggaccccatcacgatggcgacacgcgccggattattgcgggaagacatgcgtcttaaaactcctgtggtgcacaactctcggctttagagggcacagagaatagcacggaaagagagcaaggaaaacggttgcgtggctgtgaaatcagcaaagttgcgggttttttaaaacggaaaatgaatcagctcaacgtcatccgccgtgactttcaccattgaaccttccgtatgccaggcacccagtaccacgcgaaaagcaggttgctgattggcgataagttcatgcaccgccgggcgatgggtatgcccgtggatcagccattgcacctgatgtttttccatcgcactgaccaccgcgttttggttaacgtccatgatcgccagcgatttactgctgttggcttctttgctgttcgcgcgcattcgcgcggcaatgcgtttgcgcacaaacaacggcagggcgaggaatagcgtctgcagccagggtttgtggaccttggcgcgaaaagcctgataacccgcgtcatcggtgcacagcgtgtcgccatgcataatcaacacccggcgaccataaagttcgagcaccttttcttccggcaataacgtcatgccactttcacgggcaaagcgtttgccgagcagaaaatcacggttgccatgaatgaaataacagggaacgccggaatcggacaccgctttgatcgccgccgccatcttgcgatggagtgggttgggatcgtcgtcgccaatccatgcttcaaacagatcgccaagaatatacagcgcgtcggccttgcgggcttcccccgctaaaaaacgcagaaaaccggcggtgatcgccggttcttccacgcagagatgaagatctgcaataaagagtgtcgccacgattactcgctaacggtcacgctttcaatgataacgtcttcttttggcacgtcctggtgcataccgctacgaccggttgcaacacctttgattttgtctaccacgtccatgccgtcaaccacttcagcaaacacgcagtagccccaaccttgcaggctttcgccagagaagttcaggaagtcgttatcaaccacgttgatgaagaactgtgcagttgcagagtgcggagcctgagtacgtgccattgccagcgtaccacgggtatttttcaggccgttgttggcttcgtttttgatcggttctttggtggctttttgtttcatgcccggttcaaaaccgccgccctgaatcataaagccgttgataacacggtggaaaatggtgttgttgtaaaaaccttcgcggcagtagtccaggaagtttttaactgtttcaggtgctttatcgtcaaaagttttgatgacaatatcgccgtgattggtgtggaaagtaaccatttttgcatcctgttccgtttgattggtgcttcaacccagttcgggtcatatatagggtggtgttatagcataaccgcacgatcggatcatcacgcaatgtatgctgattcgcgcgggaaatatgggtattatacgcaactcaattacccacacatgtctaaacggaatcttcgatgctaaaaatcttcaatactctgacacgccaaaaagaggaatttaagcctattcacgccggggaagtcggcatgtacgtgtgtggaatcaccgtttacgatctctgtcatatcggtcacgggcgtacctttgttgcttttgacgtggttgcgcgctatctgcgtttcctcggctataaactgaagtatgtgcgcaacattaccgatatcgacgacaaaatcatcaaacgcgccaatgaaaatggcgaaagctttgtggcgatggtggatcgcatgatcgccgaaatgcacaaagattttgatgctttgaacattctgcgcccggatatggagccgcgcgcgacgcaccatatcgcagaaattattgaactcactgaacaactgatcgccaaaggtcacgcttatgtggcggacaacggcgacgtgatgttcgacgtcccgaccgatccaacttatggcgtgctgtcgcgtcaggatctcgaccagctgcaggcaggcgcgcgcgttgacgtggtcgacgacaaacgcaacccaatggacttcgttctgtggaagatgtcgaaagagggcgaaccgagctggccgtctccgtggggcgcgggtcgtcctggctggcacattgaatgttcggcaatgaactgcaagcagctgggtaaccactttgatatccacggcggcggttcagacctgatgttcccgcaccacgaaaacgaaatcgcgcagtccacctgtgcccatgatggtcagtatgtgaactactggatgcactcggggatggtgatggttgaccgcgagaagatgtccaaatcgctgggtaacttctttaccgtgcgcgatgtgctgaaatactacgacgcggaaaccgtgcgttacttcctgatgtcgggccactatcgcagccagttgaactacagcgaagagaacctgaagcaggcgcgtgcggcgctggagcgtctctacactgcgctgcgcggcacagataaaaccgttgcgcctgccggtggcgaagcgtttgaagcgcgctttattgaagcgatggacgacgatttcaacaccccggaagcctattccgtactgtttgatatggcgcgtgaagtaaaccgtctgaaagcagaagatatggcagcggcgaatgcaatggcatctcacctgcgtaaactttccgctgtattgggcctgctggagcaagaaccggaagcgttcctgcaaagcggcgcgcaggcagacgacagcgaagtggctgagattgaagcgttaattcaacagcgtctggatgcccgtaaagcgaaagactgggcggcggcggatgcggcgcgtgatcgtcttaacgagatggggatcgtgctggaagatggcccgcaagggaccacctggcgtcgtaagtaattgcgctattgccggatgcgagttttcgcatccggttatcgtctgcgccaccacaacattcccatcagtagcatccccggcaaccacacccacatcaattcagaaataatcacctgatgcccgtacggcgtggtgtaacgagacaatgcaaacggcgcgacttttatcacctgccagggagcgaaaaagcgttcatctgaccacggccacagccagccaacgcctttaccgccagtggttaccgaatccagcaagctgtgcgatagcaacgagacggttaaaaacagccagcagcgaatcagcccagccctgaaccatcggcgtccaataaacacacataacagcgggacaacaaacgcaaacaccagcgaatgggtaaacccgcgatgaccaaaaacattgccgtaagcaacgccaaatttaaacgacaatacgtcggcgtcgggcagcatcgccaggatgattccggcaaataacagacgcggagggatgactttcgaacccaaccctaaaccaatgcataggggaacggcggcgtgcgtaataacggttggcatgatggtcgcttcggcaaaatgtcgatgctatcagcatggatgaacggggcgtagagggcaaaagtctgaaaagagaaccggcctgttgatacaggccgggaaagggatcaggcaacaacctgtacgctgtgacctgcaaaactcactgtctgaccggcgacgattttgcagcgtttgcgcgtttcaaccgcaccgtcgactttcacctggccttcggcaatcgcgattttcgcctgcgcgccgctttcgctccagccttccagtttcagcaagtcgcacagctcaacgtgcggatgtttacctaaagaaaatgtcgccatgttactcatcctgtggatcatgatattcaacgcacgcctgtagcgtgttttcaatcagcgtggcaaccgtcatcgggccaacgccgccgggaacaggcgtaatgtatgaggcgcgtttagccgcgtcttcaaacacgacgtcgcccacaactttgccattttccagacggttgatgccgacatcaatcacaattgcgccttctttgatccagtcaccgggaataaagcctggcttgccaacggcaacgatcaatagatcggcattttctacgtgatgacgcagatttttagtgaagcggtgagtcactgtagtggtgcaacctgccagcagcagttccatgctcatcgggcggccaacgatattcgatgcgccaatcaccacggcgttgaggccgaaggtatcaatgttgtaacgctcaagcagcgtgacgataccgcgcggggtgcagggacgcagacgcggcgcgcgctggcacagacgaccgacgttgtaaggatggaaaccgtccacgtctttgtccggatgaatacgttccagcactttgacgttatcaatacccgccggtaacggcagttgaaccagaatgccatcgatggtgttgtcggcattcagcgtatcgataagctccagcagctccgcttcgctggtggtttccgggaggtcataagagcgggagacgaacccgacttcttcacaagccttgcgtttgcttgcgacataaatttgcgatgcagggttactacccaccagcacaacggccagtcctggtgcccgcagtccggctgcaatacgcgcctgaactttttgagcaacttcagagcgcacctgctgcgcaatcgttttaccgtcaataatctttgctgccatcagagagaggattccatctgttacgtagatcgaaggggatgcgcctattttgtcagaagcggggcgcgctgtcaggtttcgtttcagatttatcgcgtgaagcgacctcttgcgaaggtgaggcgcaccgtcgctgagactgaaagcttcatttttcgtccatgatggcgttgtaaatctggaactgatttatttccttgtctaaggattaagataatttaagaaatacctgacaatataaaaagaattttcagcctggtaatttaccgcttcaggtctatatttgtgttgaatatattttgcgcggaagtattcatctaacggggctctctattttttagaatagagtgcatattttcaattaagacattcttagaggataaaaaggaatttactactatcagtgtcttaaataaagtaatcggttatatacggatgtggagtcgataaatgagattgaaggaatatatatgaaattaagatttatttcgtctgcgctggctgccgcactattcgccgctacgggtagttatgctgccgttgtagatggcggtacaattcactttgaaggcgaactggtgaatgctgcctgttcagtgaatactgactcggcagaccaggttgtcacactcggtcaatatcgtaccgatattttcaatgctgttggtaatacctctgcattaattccattcaccattcagttgaacgactgcgatcctgttgttgccgctaatgctgccgttgcattttctggtcaggctgatgcaatcaatgataatttattggccattgcatccagtaccaatacaacaacagcaacgggtgtcggtattgaaatacttgataatacatccgcaattctcaaacctgatgggaatagcttctcaaccaaccagaacttgatccccgggaccaacgttcttcatttttctgcacgttataaaggcaccggtacaagtgcatcagcagggcaagcaaatgctgacgcgacttttattatgagatatgaataatcaaaaccacgttgttttgaattatatatcacgtcttataacaaagtaatgtaccggttgtctgaagcggtatggtggcaatgtaaatcgaaatcatgttcactttgtatcatgccgctttattaaatgaaaagggaatgatgtgttgtaagaaaccaaagcaatcatttctttatattccttatttttgccgtcaggaatacacaaggcgtattaactatgatgactaaaataaagttattgatgctcattatattttatttaatcatttcggccagcgcccatgctgccggagggatcgcattaggtgccacgcgtattatttatcccgctgatgctaaacagactgcggtatggattagaaatagccataccaatgagcgctttctggtcaattcgtggattgaaaacagcagcggtgtaaaagaaaagtcattcatcattacaccgccactgtttgttagtgaacccaaaagcgaaaatactttgcgtattatttacaccggtccaccgctggcagcagatcgtgagtctctgttctggatgaatgttaagacgatcccttcggtagataaaaatgcattgaacggcaggaatgttttgcaactggcgattttatcgcgcatgaaattatttctccgtccaattcaattacaagaattacccgcagaagcgccggacacactcaagttttcgcgatccggtaactatatcaatgttcataatccatcacctttttatgtcaccctggttaacttacaagtgggcagccaaaagttggggaatgctatggctgcacccagagttaattcacaaattcccttaccctcaggagtgcagggaaagctgaaatttcagaccgttaatgattatggttcagtaactccggtcagagaagtgaacttaaactaaccgaatcatctgacaatatcagagctaattatgaaaatacccactactacggatattccgcagaggtatacctggtgtctggccggaatttgttattcatctcttgccattttaccctcctttttaagctatgcggaaagttatttcaacccggcatttttattagagaatggcacatccgttgctgatttatcgcgctttgagagaggtaatcatcaacctgcgggcgtgtatcgggtggatctctggcgtaatgatgagttcattggttcgcaggatatcgtatttgaatcgacaacagaaaatacaggtgataaatcaggtgggttaatgccctgttttaaccaggtacttcttgaacgaattggccttaatagcagtgcatttcccgagttagcccagcagcaaaacaataaatgcatcaatttactgaaagctgtacctgatgccacaattaactttgattttgcagcgatgcgcctgaacatcactattcctcagatagcgttgttgagtagcgctcacggttacattccgcctgaagagtgggatgaaggtattcctgctttactcctgaattataatttcaccggtaacagaggtaatggtaacgatagctatttttttagtgagctcagcgggattaatattggcccgtggcgtttacgcaacaatggttcctggaactattttcgcggaaatggatatcattcagaacagtggaataatattggcacctgggtacagcgcgccattattccgctgaaaagtgaactggtaatgggagacggcaatacaggaagtgatattttcgatggcgttggatttcgtggtgtacggctttattcttctgataatatgtatcctgatagccagcaagggtttgccccaacggtacgtgggattgcccgtacggcggcccagctaacgattcggcaaaatggttttattatctatcaaagctatgtttcccccggcgcttttgaaattacagatttgcacccgacatcttcaaatggcgatctggacgtcaccatcgacgagcgcgatggcaatcagcagaattacacaattccgtattcaacagtgccaattttacaacgcgaagggcgtttcaaatttgacctgacggcgggcgattttcgtagcggtaatagtcagcaatcatcgcctttcttttttcagggtacggcactcggcggtttaccacaggaatttactgcctacggcgggacgcaattatctgccaattacaccgcctttttattagggctggggcgcaatctcgggaactggggcgcagtgtcgctggatgtaacgcatgcgcgcagtcagttagccgacgccagtcgtcatgagggggattctattcgcttcctctatgcgaaatcgatgaacaccttcggcaccaattttcagttaatgggttaccgctattcgacacaaggtttttatacccttgatgatgttgcgtatcgtcgaatggaggggtacgaatatgattacgacggtgagcatcgcgatgaaccgataatcgtgaattaccacaatttacgctttagccgtaaagaccgtttgcagttaaatgtttcacaatcacttaatgactttggctcgctttatatttctggtacccatcaaaaatactggaatacttcggattcagatacgtggtatcaggtggggtataccagcagctgggttggcatcagttattcgctctcattttcgtggaatgaatctgtagggatccccgataacgaacgtattgtcggacttaatgtttcagtgcctttcaatgttttgaccaaacgtcgctacacccgggaaaatgcgctcgaccgcgcttatgcctcctttaacgccaaccgtaacagcaacgggcaaaatagctggctggcaggtgtaggtgggaccttactggaaggccacaacctgagttatcacgtaagccagggtgatacctcgaataatgggtacacgggcagcgccacggcaaactggcaggccgcttacggtacgctggggggcgggtataactacgaccgcgatcaacatgacgttaactggcagctgtctggcggtgtggtcgggcatgaaaatggcataacgctgagccagcctttaggggataccaatgttttgattaaagcgcctggcgcaggcggtgtacgcattgaaaatcaaactggcattttaaccgactggcgcggctatgcggtgatgctgtatgccacggtttatcggtataaccgtatcgcgcttgataccaatacgatggggaattccatcgatgttgaaaaaaatattagcagcgttgtgccgacgcaaggcgcgttggttcgtgccaattttgatacccgcataggcgtgcgggcgctcattaccgttacccagggcggaaaaccggtgccgtttggatcactggtacgggaaaacagtaccggaataaccagtatggtgggtgatgacgggcaagtttatttaagtggtgcgccattgtctggtgaattactggttcagtggggagacggcgcgaactcacgctgcattgcgcactatgtattgccgaagcaaagcttacagcaagccgtcactgttatttcggcagtttgcacacatcctggctcataaaggaaattatcaataagataatctgcagattattattggcgatggcatgtttgtgtctggcaaacatatcctgggctactgtttgtgcaaatagtactggcgtagcagaagatgaacactatgatctctcaaatatctttaatagcaccaataaccagccagggcagattgttgttttaccggaaaaatccggctgggtaggtgtctcagcaatttgtccacccggtacgctggtgaattatacataccgtagttatgtcaccaactttattgttcaggaaactatcgataattataaatatatgcaattacatgattatctattaggtgcgatgagtctggttgatagtgtgatggatattcagttccccccgcaaaattatattcggatgggaacagatcctaacgtttcgcaaaaccttccattcggggtgatggattctcgtttaatatttcgtttaaaggttattcgtccctttattaacatggtggagatccccagacaggtgatgtttaccgtgtatgtgacatcaacgccttacgatccgttggttacacctgtttataccattagttttggtggccgggttgaagtaccgcaaaactgcgaattaaatgccgggcagattgttgaatttgattttggtgatatcggcgcatcgttatttagtgcggcagggccgggtaatcgacctgctggtgtcatgccgcaaaccaagagcattgcggtcaaatgtacgaatgttgctgcgcaggcttatttaacaatgcgtctggaagccagtgccgtttctggtcaggcgatggtgtcggacaatcaggatttaggttttattgtcgccgatcagaacgatacgccgatcacgcctaacgatctcaatagcgttattcctttccgtctggatgcagctgcggcagccaatgtcacacttcgcgcctggcctatcagtattaccggtcaaaaaccgaccgaagggccgtttagcgcgctggggtatttacgcgtcgattatcaatgaggtacggagaatgagaagagtactctttagctgtttctgcgggctactgtggagttccagtggatgggcagttgaccctttaggaacgattaatatcaatttgcacggtaacgttgttgatttctcctgtaccgtaaacacagcggatattgataagacggtagatttaggcagatggcctacgacacaactactgaacgctggcgataccacggcactcgtcccttttagcctgcggctggagggatgtcctccgggttcagttgcgattttatttacgggaacgccggcatccgataccaacctgctggctctggatgatcccgcaatggcacaaaccgtcgccatcgaattacgtaatagcgatcgctcccggctcgcactgggggaggcgagcccgactgaggaagtagatgcaaatggcaatgtcacactaaacttttttgccaattatcgagcgttagccagcggtgttcggccaggtgtggcgaaagcggatgcgatatttatgatcaattataattaatattatattaattcgtataatttggcgtagtcgataagctctacaattgaatgcaaacctagcttgccataaatattagatttatgcgcactaactgttttattgctaagtaataacttatcggcaatttctttattagataatccgctaaccagataacgtaatatggtcacttcacgattagatagcacagtgaccgttgaactattcgtactacatttattgctttttatatagttaagcgtttcgctgggaaaaaacgtgtatccggagaggatcatctgaacggcatgaaaaatatcattctgatcattgcatttactgacaaaaccgttagcaccagcttgtatcgctctgccagcataaaagcattctgatttcgatgataaaaataacactttcactgtgctctggatttgtttgatccttttcaggaaggtaaaaccgtctgttccgggcaagtctatatccataatgattaaatcaacaggacgggttcggagataatcgatggttatgcgataatcatccgttttcaggacaatctgcaattcactgtttttttgcaacagaacttcaatagacattctgatgataggatgagtatccataatgatcaccgacgttggtttcatagttaccagtctcataggagcggacaattttccgttaggtcgggaaattgtactttgatacatgaaaatacgggttttcttgattcagacgcgcagcggtgtgcgtttgtttgccgctatagcgaaataaatcagaaaatcagacgcggtcgttcacttgttcagcaaccagatcaaaagccattgactcagcaagggttgaccgtataattcacgcgattacaccgcattgcggtatcaacgcgcccttagctcagttggatagagcaacgaccttctaagtcgtgggccgcaggttcgaatcctgcagggcgcgccattacaattcaatcagttacgccttctttatatcctccataatttcagagtgggacatatttgggacattatcaccaaaaatgtcgtctattttcctcgcatgctctgtcaaatgattaggcgcaaggtgagcatacctacgaaccatttctatggactcccatccgcccatttcctgaagcactgataatgggacgcctgactgaatcagccagcttgcccaggtgtgtctgaggtcatggaaacggaaatcttcaattcctgcacgacgacaagctgatagccatgatgtcttgctgtcgatgcgcatcttcctgaccgcaggcgttgatgttccatctgctcgcttagccgccttggtatgtacaaacacccatttgtgatgcttgcctatttgatcacgcaacactttacaggcggtatcgttcagcgccacaccaatggcgcggtttgatttgctctcttctggattcacccaggcaactcgtcgctgcatgtcgatttgttgccattccagatttatgatgttcgactttctcagaccagttgccagcgcaaacttgacgacagatttcagtggttcggggcactcatcaataaggcgttttgcttcctccttttccagccatctgactcgcttgtttctgaccgctggtatcttgatgacaggcgctttttccagccacttccagtcgcgttctgcagcacggagaatggcctttatcatggcaagatgctttgcctttgtctgagttgatactggctttggttcataaacaggcagttctttacctttcctgatggcggcctgaactttctgtttccatatttctttcgtctttctgttatgcattctgcttacagcagagtaaatctttgcctccgagatatctttaagccttataccctcaaaatgttcaagccagaactcaatccggcttttatctgaatcgagagattttttatcagctttttcctcaagccatcttaggcaggcctcttcaaaagtgacatcaggtaaatcccctagcttttctactcgccagagttctgcttttcgcttgtcgtgcaactcctgagcttgccgtttgtcctttgtgccaagagattccttaattcgtttcccgcccgggagcgaatacgaggcataccatatttcatttctgcggaagagtgacattttctttcctctgttatgccatcacccgcgctcacctggacagtatgcagcggagactgaagcgccgcaatgcaggcttgccgtgttgtgaggtacccggatattatcgtgaggatgcgtcatcgccattgctccccaaatacaaaaccaatttcagccagtgcctcgtccattttttcgatgaactccggcaccatctcgtcaaaactcgccatgtacttttcattccgctcaatcacgacataatgcaggccttcacgcttcatgcgcgggtcatagttggcaaagtaccaggcatcttttcgcgtcacccacatgctgtactgcacctgggccatgtaagccgattttattgcctcgaaaccaccgagccggaatttcatgaaatcccgggaggtacgagtattgccggaagcgtggcctgtatccggatgcagagtcttatccgtggaaatcgaacgcgcattactggttggttaccaacttgtaccagaacatgcgggccaatgcgctggctgacgcggaattacggcgcaaggctgccgatgaactgacctgtatgacagcgcgaattaaccgtggtgagacgatacctgaaccagtaaaacaacttcctgttatgggcggtagacctctaaatcgtgcacaggctctggcgaagatcgcagaaattaaagctaagttcggactgaaaggagcaagtgtatgacgggcaaagaggcaattattcattacctggggacgcataagagcttctgtgcacaggacgttgccgcggtaacaggcgcaaccgtaatctgatcttacccagcaatagtggacacgcggctaagtgagtaaactctcagtcagaggtgactcacatgacaaaaacagtatcaaccagtaaaaaaccccgtaaacagcattcgcctgaatttcgcagtgaagccctgaagcttgctgaacgcatcggtgttactgccgcagcccgtgaactcagcctgtatgaatcacaactctacaactggcgcagtaaacagcaaaatcagcagacgtcttctgaacgtgaactggagatgtctaccgagattgcacgtctcaaacgccagctggcagaacgggatgaagagctggctatcctccaaaaggccgcgacatacttcgcgaagcgcctgaaatgaagtatgtctttattgaaaaacatcaggctgagttcagcatcaaagcaatgtgccgcgtgctccgggtggcccgcagcggctggtatacgtggtgtcagcggcggacaaggataagcacgcgtcagcagttccgccaacactgcgacagcgttgtcctcgcggcttttacccggtcaaaacagcgttacggtgccccacgcctgacggatgaactgcgtgctcagggttacccctttaacgtaaaaaccgtggcggcaagcctgcgccgtcagggactgagggcaaaggcctcccggaagttcagcccggtcagctaccgcgcacacggcctgcctgtgtcagaaaatctgttggagcaggatttttacgccagtggcccgaaccagaagtgggcaggagacatcacgtacttacgtacagatgaaggctggctgtatctggcagtggtcattgacctgtggtcacgtgccgttattggctggtcaatgtcgccacgcatgacggcgcaactggcctgcgatgccctgcagatggcgctgtggcggcgtaagaggccccggaacgttatcgttcacacggaccgtggaggccagtactgttcagcagattatcaggcgcaactgaagcggcataatctgcgtggaagtatgagcgcaaaaggttgctgctacgataatgcctgcgtggaaagcttctttcattcgctgaaagtggaatgtatccatggagaacactttatcagccgggaaataatgcgggcaacggtgtttaattatatcgaatgtgattacaatcggtggcggcggcacagttggtgtggcggcctcagtccggaacaatttgaaaacaagaacctcgcttaggcctgtgtccatattacgtgggtaggatcaaccagcataaatcaggctgcggctaaaatggcgcgggcaggaatcctggtcgttgatggtaaggtctggcgaacggtgtattaccggttcgctaccagagaagaatgggaaggaaaggtgagcacgaatctgatttttaaggagtgtcgccagagtgccgcgatgaaacgggtattgagggtatataaaagaacatcaatgggaacacaatgatgaaacaggtgagttgagttcaaactgtagtacaattctctccagtttgaacaggaaagaatatgctatgaacccttatatttatcttggtggtgcaatacttgcagaggtcattggtacaaccttaatgaagttttcagaaggttttacacggttatggccatctgttggtacaattatttgttattgtgcatcattctggttattagctcagacgctggcttatattcctacagggattgcttatgctatctggtcaggagtcggtattgtcctgattagcttactgtcatggggatttttcggccaacggctggacctgccagccattataggcatgatgttgatttgtgccggtgtgttgattattaatttattgtcacgaagcacaccacattaaaataatttgtttctaaacgactaaaatatggaggctcttatatttatatgagcctcgttttatgctttttgttaatgtctttattttttatgtattcttttgtgctttcaagattatggcgtaagaaaattgcaatacgattattgttgtatattcaagataatgtgaccttaattgtctttttaaataaaaaataaacaaaaattatatcccaccactaaggtttataaaagcatacgttagcaggtgtcaccatgaaaaaagccatagcatatatgcgattttcatcaccaggtcagatgtctggcgactcattaaaccgacagagaagacttattgctgaatggttaaaggtaaatagtgattattatcttgataccataacatatgaagatttaggattaagtgcattcaaaggaaagcatgcacaatcaggagctttttcggaatttttagatgctatagagcatggttatatattgccaggaactacattgttagttgaaagtctggacagactttcaagagaaaaagtcggtgaagcgattgaacgtctgaaattgattttgaatcacggtattgatgttataactctttgcgacaatacagtctataatattgactctttgaatgagccatattcattaataaaagccatacttatagcacaaagggcaaatgaagaaagcgagataaagtcaagtcgggttaaattatcatggaagaaaaaacggcaggatgcactggaatcaggtacgattatgacggcgtcttgtccgagatggctctccttagatgacaaaagaacggcttttgttccagaccccgacagggtgaaaactattgagctaatttttaaactcaggatggaaaggcgctcattgaatgcaatagccaagtatttaaatgatcatgctgtaaagaatttctcaggaaaagaaagtgcatggggaccttctgtaattgaaaaattattagcgaataaagctctgataggtatttgcgtaccttcatatcgtgcaagagggaaagggataagtgaaatcgctggctattatcccagagtcatatcagatgatttgttttacgctgtacaggaaattcggttggcaccttttggtattagcaatagtagcaagaatcctatgctaataaatctacttcgaacagttatgaagtgtgaggcttgtggtaataccatgattgttcatgcggtatctggaagtttgcatggctattatgtttgtccgatgagaagattacatcgatgtgacaggccatcaataaaaagagatttggttgattataatatcattaatgaattgctttttaattgtagcaaaattcaaccagttgaaaacaagaaagatgctaatgaaactttagagttaaaaattattgagcttcagatgaaaattaataatttaatcgttgcattgtctgtcgcgcctgaagttaccgctatagcagagaaaataagactattagataaggaattacgaagggcttcggtatcattgaaaactttgaagagtaaaggtgtaaattcattcagtgatttttatgctattgacttaaccagtaaaaatggacgagagttatgccgtacacttgcctataaaacattcgaaaaaatcataattaatacggataataaaacctgtgatatctattttatgaatggcattgtttttaaacactatcctttaatgaaagtaatatccgcccagcaggcgataagtgctctcaaatatatggttgatggtgagatttatttctaaataatgatctcggattttaagttatgctatggtgataaagtgcaagacagaattaattatctttgacgaaacttaatgggtaattactttgtttgctcccacaagcgagttttgtacggctgtattggggtagtaaatgagctatacaatcttaatcatttgttaggtgagaactcttggtcgcagattcaaatactgaaaatacgtgacaaattattatgagcaaaatggtgtatgtcacgtattttgaatggtaggttaaaaaataacaccgactttcgtaggtgttactaataataaagcagagtttttagatagtatcaatgtgctttgtgtatattgtggcaaataattgggttgggggtacaattgtgattgcttttgcatgaacattgcgcctttatgcataatgagataaaggaatatcaaataaaataacgataggtcataacaaagaggtttttatgaaaacacttatcgtttcaactgtattggcattcataacattttctgcgcaggctgcagcatttcaggtcactagtaatgaaataaaaacaggagagcaacttacaacgtctcatgtcttttctggatttgggtgtgaaggtggtaatacatcgccctcattaacctggtctggtgttcctgaaggtaccaaaagctttgccgtaactgtatatgatccagatgcacctacaggcagtggttggtggcattggactgttgttaatattccagcaacagtaacatatttgcccgttgatgcagggagacgtgatggaacaaaactgccgactggtgctgttcaaggccgaaatgattttggctatgctgggtttggtggcgcatgtcctcctaaaggagataaaccacatcattaccagtttaaagtatgggctctaaaaactgaaaagattcctgtagattctaactccagcggagcgttagttggttatatgcttaatgctaataaaatcgcaaccgctgagataacaccagtttatgagataaagtagggtgagagtatgctggcaagaggtaagactaacttaaagatcgaagaaatacggatgcataaacatcatgagattcatagggttaagcctcttatgccagctttgtgtcgtatccgtcagggaaagaaagttatcaattgggagacgcatactttaactgttgataataatcaaataatattatttccttgtggttatgaattttatattgagaattatcctgaagcagggctttatcttgcagaaatgctttacttacccattgatttaattgagagtttccaaaaactttatacggtaactgatcaaatacgtaacaaaacaagtttctttttacctcagaatcctgagttaatatattgttgggagcaactaaaaacatctgtttcccgaggcttctcaactaaaattcaggagcacttagcaatgggcgttctactttcgttaggagtgaatcatgttaatcatttacttttatcatatagtaaacaatcattgataagtcgttgttataacctgctgctatccgaacccggcacaaaatggacagcaaacaaggttgctcgatatctctacatttctgtttctacattacatcgccgtctagcaagcgagggggtaagtttccaaagtatactggacgatgtgaggttaaataatgcgttgtctgctatacaaacgacggtaaaacctataagcgagattgccagagaaaatggttataagtgtccttctcgttttactgaaagatttcataatcgttttaatataacaccaagagagataagaaaagcttccagagagtaaaagtgttttaagaaggagcaattctatcgattttgattttgggaaatcaacacggcataattatgtcaccggagcctgaacaactccggtgacttctgcgctaaacggggacgtttatgcgcacatacaatccaaactctcttctcccttcacagatgcagaaatgcacctgcaattctttgcatctagcgtttgacctctgcggaggggaagcgtgaacctctcacaagacggcatcaaattacatcgcggcaacttcaccgctatcggtcggcagatccagccttatctggaggagggcaaatgctttcgcatggtgcttaaaccgtggcgtgagaaacgcagtctttcccagaatgcactcagccacatgtggtacagcgaaatcagtgaatacctcatcagcaggggtaaaacgttcgccactccagcttgggtaaaagatgctctcaaacacacatatctcggttatgaaaccaaagacctggttgatgtcgtaaccggtgatatcaccactatccagtcgttacgccatacctccgatcttgataccggagagatgtatgtcttcctgtgtaaggttgaagcctgggcgatgaatattggttgccacctgactattccacagagctgcgagttccagctgctgcgcgacaagcaggaggcgtaatggctacaccgcttattcgtgtcatgaacggacacatctacagagtaccaaatcgtcgtaagcgtaaacctgagctgaagccatccgaaataccaacactgctcggatataccgccagcttggttgataaaaaatggttgcgactggcagcaaggaggagtcatggctgatttgagaaaagcagcgcgtggtcgggaatgccaggtaagaatccctggcgtatgtaatggcaaccctgaaacgtctgtactggcacatatccggctgactggattgtgcggcaccggtacgaaaccgccagacctgattgccaccattgcatgttctgcctgccacgacgaaatcgaccgccgcacgcattttgttgacgctggatatgcaaaagaatgcgcgctggaaggtatggcgagaacacaggttatctggctgaaagagggggttattaaggcgtgaatacctacagcatcacattaccctggcctccgagcaataatcgctattaccgccataatcgcgggcgcacgcacgtcagcgcagaggggcaggcataccgcgataacgtcgcccgaatcattaaaaacgcaatgctggatatcggcctggctatgcctgtgaaaatccgcattgagtgccacatgccggatcgccgtcgccgtgacctggataatctgcaaaaagccgcttttgacgcactcactaaagcaggtttctggctggatgatgctcaggtcgttgattaccgcgttgtgaagatgcctgttaccaaaggtgggaggctggaactgaccatcaccgaaatggggaatgaatgatgtttgagtttaatatggcagaacttcttcgccaccgctgggggcgtctgcgcttatatcgtttccccggttctgttttgaccgattaccgaatactgaagaattacgccaaaaccctgacaggagcaggagtatgaagtcagagataacaatcaactaatactgttttgttgatttttgcttgtaattggcgttctggtctgatttttgtggagtaagttgatgcgtgatattcagatggttcttgagcgttggggagcgtgggcggctaataatcatgaagatgtgacctggtcgtccattgccgccggttttaagggattaattacttcaaaagtaaaatctcgcccgcaatgttgtgacgatgacgcgatgatcatttgcgggtgcatggcccgtctgaaaaagaacaacagcgatttgcacgatttattagtagattattatgtagtcggtatgacattcatgtcactggcaggtaagcattgctgctctgatggttatatcgggaaaaggttacagaaggctgagggcataattgaagggatgttaatggcattagatatccggttagagatggatatcgttgttaataactctaattaatatgccaattgtttactaaaaattattaaaaatggggcgttgagacgcccccaaaaataaagggtaatatataacagaaggtttatatagttagaagcaaggttgtgcttctaaaggaagtggcttgagggagccacttatatgttggggaggcaacgcctcccgcaacatatctttttcgtaatcagattagaactggtaaaccagacctacagcaacgatgtcatcagtgcttacaccgagtgctttagggaaggtgcgaataagcggggaaattcttctcggctgactcagtcatttcatttcttcatgtttgagccgattttttctcccgtaaatgccttgaatcagcctatttagaccgtttcttcgccatttaaggcgttatccccagtttttagtgagatctctcccactgacgtatcatttggtccgcccgaaacaggttggccagcgtgaataacatcgccagttggttatcgtttttcagcaaccccttgtatctggctttcacgaagccgaactgtcgcttgatgatgcgaaatgggtgctccaccctggcccggatgctggctttcatgtattcgatgttgatggccgttttgttcttgcgtggatgctgtttcaaggttcttaccttgccggggcgctcggcgatcagccagtccacatccacctcggccagctcctcgcgctgtggcgccccttggtagccggcatcggctgagacaaattgctcctctccatgcagcagattacccagctgattgaggtcatgctcgttggccgcggtggtgaccaggctgtgggtcaggccactcttggcatcgacaccaatgtgggccttcatgccaaagtgccactgattgcctttcttggtctgatgcatctccggatcgcgttgctgctctttgttcttggtcgagctgggtgcctcaatgatggtggcatcgaccaaggtgccttgagtcatcatgacgcctgcttcggccagccagcgattgatggtcttgaacaattggcgggccagttgatgctgctccagcaggtggcggaaattcatgatggtggtgcggtccggcaaggcgctatccagggataaccgggcaaacagacgcatggaggcgatttcgtacagagcatcttccatcgcgccatcgctcaggttgtaccaatgctgcatgcagtgaatgcgtagcatggtttccagcggataaggtcgccggccattaccagccttggggtaaaacggctcgatgacttccaccatgttttgccatggcagaatctgctccatgcgggacaagaaaatctcttttctggtctgacggcgcttactgctgaattcactgtcggcgaaggtaagttgatgactcatgatgaaccctgttctatggctccagatgacaaacatgatctcatatcagggacttgttcgcaccttccttagtgaagtcatttttgtcaagcaggttgattttgtaatcaacgaaagtagacatatttttgttgaagtaataggttgcacctacatcaacatatttgactaagtcctgatcgccccatactccaagatccttacctttagattgcaggtaagcaacggacggacgcagaccgaaatcgaactgatattgtgcaacagcttcgaagttttgggctttattagcaacgaagtgatcagcaaatacagtcatattctgggtttcagaataggtagtggccaggtaaatgttgttagcgtcatatttcagacctgcggcccaaacttctgcatttttaccggaagcaaatacttcaggaagaactttccctgcattaacttgagtgtcggtacgatcagatttcgcataagttgcaccgataccgaatccttcgtattcataggtagcagagaaaccgaagccatcaccgttaccttcagtgtagttatcgaaatcgctacgatcgtttttgccttggtactgagcagcaaagttcagaccatcaaccagaccaaagaagtcgttgttacgataggttgcaacaccagttgcacgttgagtcatgaacacgtcggtttgagtccaagtgtcaccaccgaattctggcaggacgtcagtccacgcaccgatgtcgtatgctacaccgtagttacggccgtaatcgatggagccgtagtcaccgaatttcaggccagcgaaggcaagacgggttttatctttggaggaaccttgagattcagcgcggttgcctttgaattcatattcccactgaccgaaaccagtcagttgatcgttgatttgggtttcacctttgaagccaagacgggcataagtagtatcaccatcatctgcatcattagaggagaagtagtgcttagcattaactttcccgtacagatccagcttgttactgtctttattataaatttcagctgcctgagcagacatcgccattagtactgatgcagctacagcagaaattgccactgttaattttttcatcgtgagccctttttttgaactattattaaaaaatgatgtcactgcgcgataaatattcatctaatcaatgtgattatttcaagatgtaagttttggtttctcgtttgatttgtgaagtagatctctatttttatctgaacttttttctatcgaatcctattcatggctcttggctgaataaaaataaatctattagccaatttatattaacggctgttatttataagtgctctataatttgaaggttcaatttaaaccggctaaaaataacactggaaattattttttggttatttgttgagatttgcttatgtatttgtagtggtgttttcaatactcggtagcattctctcaaatatcatttagtggtttacgtacgtaaaaaattggttatgctgttaagagtggttacttcgtcacacagcttaaacccgccgtcgagcgggtttttccattttttgagtctcgatattagctgataacccaatacctgagttattcactgactccgagtctgttacgtttcgtagtattccctcaatttacacccgctttgtctgcgaggtggggttatgaaatccatggataagttaacaacgggtgtcgcctatggcacctcagcaggtagtgccgggtactggtttttacagctgctagataaagtcactccctcacagtgggcagcaataggtgtgctgggtagcctggtatttggcctgctgacgtacctgacaaacctttatttcaagattaaagaagataagcgcaaggctgcgagaggtgaataatgcctccatcattacgaaaagccgttgctgctgctattggtggcggagcaattgctatagcatcagtgttaatcactggcccaagtggtaacgatggtctggaaggtgtcagctacataccatacaaagatattgttggtgtatggactgtatgtcacggacacaccggaaaagacatcatgctcggtaaaacgtataccaaagcagaatgcaaagcactcttgaataaagaccttgccactgtcgccagacaaattaacccgtatatcaaagtcgatataccggaaacaacgcgcggcgctctttactcattcgtttacaacgtgggtgctggcaattttagaacatcgacgcttcttcgcaaaataaaccagggcgatatcaaaggcgcatgtgatcagctgcgtcgctggacatacgctggcggtaagcaatggaaaggcctgatgactcgtcgtgagattgagcgtgaagtctgtttgtgggggcaacagtgagcagagtaaccgcgattatatccgctctgattatctgcatcatcgtcagcctgtcatgggcggtcaatcattaccgtgataacgcaatcgcctacaaagtccagcgcgacaaaaatgccagagaactgaagctagcgaacgcggcaattactgacatgcagatgcgtcagcgtgatgttgctgcgctcgatgcaaaatacacgaaggagttagctgatgcgaaagctgaaaatgatgctctgcgtgatgatgttgccgctggtcgtcgtcggttgcacatcaaagcagtctgtcagtcagtgcgtgaagccaccacggcctccggcgtggataatgcagcctccccccgactggcagacaccgctgaacgggattatttcaccctcagagagaggctgatcactatgcaaaaacaactggaaggaacccagaagtatattaatgagcagtgcagatagagctgaccatatcgatgggcaactcatgcaattattttgagcaatacacacgcgcttccagcggagtataaatgcctaaagtaataaaaccgagcaatccatttacgaatgtttgctgggtttctgttttaacaacattttctgcgccgccacaaattttagctgcatcgacagttttcttctgcccaattccagaaacgaagaaatgatgggtgatggtttcctttggtgctactgctgtctgtttgttttgaacagtaaatgtctgttgagcacatcctgtaataagcagggccagcgcagtagcgagtagcatttttttcatggtgttattcccgatgctttttgaagttcgcagaatcgtatgtgtagaaaattaaacaaaccctaaacaatgagttgaaatttcatattgttaatatttattaatgtatgccaggtgcgatgaatcgtcattgtattcccggattaactatgtccacagccctgacggggaacttctctgcgggagtgtccgggaataattaaaaacgatgcacacagggtttagcgcgtacatgtattgtattatgccaacaccccggtgctgacacggaagaaaccggacgttatgatttagcgtggaaagatttgtgtagtgttctgaatgctctcagtaaatagtaatgaattatcaaaggtatagtaatatcttttatgttcgtggatatttgtaatccatcggaaaactcctgctttagcaagattttccctgtattgctgaaatgtgatttctcttgatttcaacctatcataggacgtttctataagatgcgtatttcttgagaatttaacatttacaacctttttaagtccttttattaacacggtgttatcgttttctaacacaatgtgaatattatctgtggctagatagtaaatataatgtgagacattgtgacgttttagttcagaataaaacaattcacagtttaaatcttttcgcacttgatcgaatatttctttaaaaatggcaacctgagccattggtaaaaccttccatgtgatacgagggcgcgtagtttgcattatcgtttttatcgcttcaatctggtctgacctctttgtgttttgttgatgatttatgtcaaatattaggaatgttttcaattaatagtattggttgcgtaacaaagtgcggtcctgctggcattctggagggaaatacaaccgacagatgtatgtaaggccaacgtgctcaaaccttcatacagaaagatttgaagtaatattttaaccgctagatgaagagcaagcgcatggagcgacaaaatgaataaagaacaatctgctgatgatccctccgtggatctgattcgtgtaaaaaatatgcttaatagcaccatttctatgagttaccctgatgttgtaattgcatgtatagaacataaggtgtctctggaagcattcagggcaattgaggcagcgttggtgaagcacgataataatatgaaggattattccctggtggttgactgatcaccataactgctaatcattcaaactacttaacctgtgacagagccaacacgcagtctgtcactgtcaggaaagtggtaaaactgcaactcaattactgcaatgccctcgtaattaagtgaatttacaatatcgtcctgttcggagggaagaacgcgggatgttcattcttcatcacttttaattgatgtatatgctctcttttctgacgttagcctccgacggcaggcttcaatgacccaggctgagaaattcccggaccctttttgctcaagagcgatgttaatttgttcaatcatttggttaggaaagcggatgttgcgggttgttgttctgcgggttctgttcttagttgacatgaggttgccccgtattcagtgtcgctgatttgtattgtctgaagttgtttttacgttaagttgatgcagatcaattaatacgatacctgcgtcataattgattatttgacgtggtttgatggcgtagatgcacgttgtgacatgtagatgataattattatcattttgtgggtcctttccggcgatccgacaggttacggggcggcgacctcgcgggttttcgctatttatgaaaattttccggtttaaggtgtttccgttcttcttcgtcgtaacttaatgtatttatttaaaataccccctgaaaagaaaggaaacgacaggtgctgaaagcgagctttttggcctctgtcgtttcctttctctgtttttgtccgtggaatgtgcaatggaagtcaacaaaaagcagctggctgacattttcggtgcgagtatccgtaccattcagaactggcaggaacagggaatgcccgttctgcgaggcggtggcaagggtaatgaggtgctttatgactctgccgccgtcataaaatggtatgccgaaagggatgctgaaattgagaacgaaaagctgcgccgggaggttgaagaactgctgcaggccagcgagacagatctccagccagggactattgagtacgaacgccatcgacttacgcgtgcgcaggccgatgcacaggagctgaaaaatgccagagactccgctgaagtggtggaaaccgcattctgtactttcgtgctgtcgcggatcgcaggtgaaattgccagtattctcgacgggatccccctgtcggtgcagcggcgttttccggaactggaaaaccgacatgttgatttcctgaaacgggatatcatcaaagccatgaacaaagcagccgcgctggatgaactgataccggggttgctgagtgaatatatcgaacagtcaggttaacaggctgcggcattttgtccgcgccgggcttcgctcactgttcaggccggagccacagaccgccgttgaatgggcggatgctaattactatctcccgaaagaatccgcataccaggaagggcgctgggaaacactgccctttcagcgggccatcatgaatgcgatgggcagcgactacatccgtgaggtgaatgtggtgaagtctgcccgtgtcggttattccaaaatgctgctgggtgtttatgcctactttatagagcataagcagcgcaacacccttattccagctggcttcgtggctgttttcaacagtgatgagtcatcgtggcatctcgttgaagatcatcggggtaaaacggtttatgacgtagcgtcaggggacgcgttatttatttctgaactcggtccgttaccggaaaatgttacctggttatcgccggaaggggagtttcagaagtggaacggtacagcctgggtgaaagatgcagaagcagaaaaactgttccggattcgggaggcggaagaaacaaaaaacagcctgatgcaggtagccagtgagcatattgcgccacttcaggatgctgtagatctggaaatcgcaacggaggaagaaacctcattgctggaagcctggaaaaaatatcgggtgttgctgaaccgtgttgatacatcaactgcacctgatattgagtggcctacgaaccctgtcagggagtaatcattgggattatgccgcagcacgtcttaagcaagaacatgctgcggttggatgctatttttttcctgaagcggaaaacattactacagtaccttgaaccttggttttaacattctcgaaatgctctgagagtatatgtgttaagccttcttcggaatcttttgtgtttgaaaagatgcctttctgattgtaaatgcgcatcagtttttgaccgaagctattgtgcacaactccatcgccaagaattgtggctccgtatagagttccatcgtcagttaaggcctgcgccgcattgcgtattacacagctttttgtagatatatttccaggcaggcagtgaagaaggtaagacatggaaatggaatcaaattgaccatgtaacgccgcgggataaggttcaaaaacatcatggctaattttatgtttaatttttgattccccagcccttgtagatgccgcgttcaggctagcttcgttcaaatccattaaagatatcagactactctcaggtacgtgagtaaggtaaaacccagttccaacaccaatatccagatggttgttacctaaatgttccagaaagtgtggaagaaggtgttcctttgtaggacatccccatgcaagccgatttgatactcccaaaacccaccagtcataaagctttagggtaagtggtgtgtaaattctagccccatcatctgtgtttttttattaatttcaccatgttatagttttatttgtgaattaaatcaattatggcaatgaattacaaggggttaaatgctgccgcagcatagcgatattgaaatagcctggtatgcttcaatacagcaggagccgaatggctggaagaccgtcaccacacagttctacatccaggaattcagtgagtatattgcgccactgcaggatgctgtagatctggaaatcgcaacggaggaagaaagatcgttgctggaagcctgaaaaaagtatcgggtgctgctaaaccgtgtggacacttccgtagcaccagatatcgagtggcttattcaaccataataaacagtatgtatatcataggttattaattgtgagttttttcggtgtgttatttgtttgtttgatgttatgcttttgcgccccaaaaggttgtttagatgtattttatcaattgattttcaatatcgtttaataaagaaaaattaagcaagctggatgttggttttttgttaattgaatggttctaataatgtttttttactgttgttgaatgtgacttgataagaaatgcaagtaaaaatgatactctttttattttaaattcaaacggttgacatatatatagcaagaggtttcaggtgcgttgtagtgagtttatgttaataaaaagcatagtaagcgttgaaaaatgtaactttgaaataagttagaataaaaaacaacatacatataataatttaatcttaaatgaaatttattaaaatttgcaaactataattttgtgtataaaaatataaatgcacatcatcctgattatgattgtgtatttaattggttgttatttgactactatcaacttgttttaattttatgataggtgcaagatggattatgtttgctccgtagttttcatctgtcaatcatttgatttaattataaacaggagagttatctcgttcaaaaaaaattcattgtttattgtaagcgacaaaattagaagggagttaccagtatgcccctctaaactaagaattgttgatatagataagaaaacatgtttatccttttttatcgacgtgaataatgagctgcctggcaaatttactcttgataagaatggctatattgctgaagaggaacctccattatcgcttgttttttctctgtttgaagggattaaaatagcagactcacactccctttggttaaaagaaagactatgtatatccttacttgccatgttcaaaaaacgcgaaagtgtaaattcatttatactaacaaatataaatacatttacctgtaaaattactggaataatcagttttaatattgagcggcaatggcatttaaaagatattgcggaattgatttatacgagtgaaagtttaataaaaaaaagattaagggatgaaggaacgtcatttactgaaatattgagagatactaggatgaggtatgcaaaaaaactcataacttcaaactcttattctatcaatgtcgtagcccagaaatgtggctataacagtacttcatatttcatatgtgcatttaaagattattatggtgtcacgccatctcattattttgagaaaataatcggcgtcacagatggaataaacaaaacaattgactgataatgtttattacaagttgtctacatgttaattataatattatacagcgttttttttgatgtgatattctggaaccattaatttgtaattgggttgctgtcgcctattttatacatactataattgatggttttctatgtgatttagttaataaccttctgggtttattttaagggttaattgttacattgaaatggctagttattccccggggcgattttcacctcggggaaattttagttggcgttcttaaaatgtgtacttaagaccagcagtagtgatgaagttatagttttctatacctgctccatttttgctgtagtctgaagtgttattattgtgatcataaagtgaagtattaccttttttattcgtaacccgattccatgcgccttcaacataaacttttgcgttaggtgtgacgtaataacctgcattgactgcaacagaatagtaattttggtctttgaccttactgcgataagtgattctttttcccgggtcatagtgttcatcgttatcagatgattccacccagccgctgtatttaaatgtgccaccgagttcaaaatcttcataacgataacttccagtcaagccaatgtagggcattttaaaacgttgtttgtagccgattgctctttctccattcgggaaggagccgatatcatctctgaatccctcctcagaactgtagatataggaaccacctctggctgtaaagctataacggctttcctgatatccggccatgagtcccaggcggtaattgggttcgttgaggagccagcctttgatattcagatcaaattcgttggcataattgagttgtgtatcagggtgtctactttcatccgtccaggttccggggttactggaatccatccagtcctgatcgaccatattgccacctcggctgccgagagttgtccagccagcagccccgatagatatctggggcatcaaatcccaattaattgcacctttaataattgcagcgttattgaatttccagtcgagttgactgacttttcggcctccttcttcggctagataaacacgctcttttgtttttccgctcagagttccaagactaatgtccgcatttatgttgtcaggagtaaacgataaagtctcggtagaagcaaaagagctgatcgcaataggggttgtcaggactattcccagaagtttcgcccgcataaaagttctccattcaatcgttttaatgattgaatatgtattttttatatctaacttaatgagtcaattacatattgctccactgtttatattttgtttagtattgaatgattatcacaatgcgctatctgtttttggtttaattatctgttattgtttcatatttcggttttactgtgtggtttttttatgcttttgtggtgcttttatctatttaagtgccatgcctttagaggcatataagcgaaaatagcatgaggtttatcctcaattactatgttttttagtacaaaaaagagggacaaaactgagacacataaggcctcgcaatggcttgcaaggctttacatgttttgaggtagtgggacgtgtgagcgcagagatggcgcggtaagttgttgacttaaaatgtcgttctaggaacttctaagtcgtgggccgcaggttcgaatcctgcagggcgcgccatttcttcctcatttatgcccgtcttatccgtttccgctttgcccttcaccacatcactttttgtcgctgtttggcgagataattcaacggtgtcaggccgtaaaacgccttaaaaacagagataaagtacgacgtgctgctatagccacataattgcgccacctgagtgatatttttgttatccatcaataacatctgtacggcgtaacgcatacgacactctgtgacaatctggctatagctggtattttcgttttttaatttctttttgagcaggctggggcttaaacatagcgaactggcgacaattcgcagattccagtaatgctgaatatcgctttgaataatgcggcagacgctgtcgcggacgctgctgcgtaagatatacatcagtagggcaataaaccgcgattgctcaagaaagttagacaatacggtaaaaagcaatgcgcgcgtcaactccgcttcgcagggtctgctgggttgctgcttgctgtggttggcggctagccggaacacttccggtgtacggctatgacaagcgataaccggggttgccagccgcgaccagggctttacacaggttaagttcttatttaaaaacaacagataatcgttgatgatgttacggttgatgtgggtgattaatacgtgatttaacgttgagagttcaatgacgttattgttgcacgcgaaggcggccaggtagtttttcggaagggtaaacgtagcatggttattgacgcttacctctacctctttttcggtcaggatcaccacgcaaggttcactgctgctcaattgcatttcgcactcctcagatatcagaaactccgctcaaaggatctatgcttcctgcatgagtgatcggcccgttcgccgataacgatcttctttctttagcacgctttttagcaattaatcttgatggaattctgatgagagcgaaagaggtaagccaggtcgtacccgacttacctggaggagatttaatactcgagaatgccgtgcgcgacgggcaaatagcgcagagagaaatagagagtgtctttaccgcaagaggaacgtttcgctaacagcgaggcaatttctgcgtccggtttcggtttcgctgtaaaggttttgcctttgccggcgacaaaaagttcataaacaacgccgctggcaggggcgggactttggcaatcggcgctggcctgtaaataacgttcacgctgttcagcggtcagtttatccacgccgctgccatcctgtacccagacattaacgccggttgctttaacgtgttccagcagttggcgatagccatcgggcgacatgtttccggcgaaaaaactactgatataaaccggttttgctgaaacatcgctaatcagccgctgcgcgttgtttaaccatgttagcaaaggctgacgggcggcttcgctgcgccagttcaggtcgtcaatttccgcgctgatgtaccagccatccggcgttatgccaggcgcggcgctccataatctggcttgctggagatcggcagccagcaggcgattaagatagctttccagcgctgcggacgactgtttctggtgcataaaaaattccggatcggcgttcagcccgacaataagcttcagaccagcctgttgcgcagctgcggcccgcttaaacaataacgtgcgctgttctggctgggtaaatgcatcgccgtaacgggtccattgcaaaacaagggtatcgaagccttgcaaacgtaactgactcatcagcccctgccactgggtatcggtaacctgactatctcggttttgtggttgccagataatacctttcatcgcaaaggaaaaagggctgaccaaaagcagtgtcagcaatacgaaaatgaacttacgcatttaccagtgcactccaatggtgagaaacgcgttgttgcgctctccgttacgttgattaatcgccttaaaggtatgttgatactcgacgccgagactgactttgtgcggccaggcgtcgtagtgcgtctcgccggtccagatattccagcggaccccgactccgccaagctgcgcgccctgagtgcctttatcacgatagccgttgtcctgaacgtgagcgtaaggctcaatagtctgtccgttagctaccttctgatgccagctgacgcgataatctgccgtccacgcctgaatatcctggcggatatattgcgccgcatcgaggtacaggttttgggcaaaccagcctgaaccgttcgggtgccattcgtcgctgtatttgccgccattaaagaatgaggcgctggcgcgcagcatggtatcggatgcgccattttggccgttcagcggcaactgctgttcgacggcgatgaaaaagatctgatcgcgcagcggcttccagcgcagaccggtgccggacatcggatttttcaccggcatcatcaccccgttttctccggtatcggcaaagacgcggctataaactgagagcaggtcgccttccagcagcatattgcgtccgatgcggtactcggcttccagttgtccgtagctacgatagcttttccctggcgctgcgccgccgacattattgttagcggtactcattgcgccggaacgcaagccgatggaagaatcgaaactgaacgtccagcggcgaccgacctcctcatgcaaacggcggaaattgaagcgttgttgattttgttctggggtcagtggggttatcagcgcctgattatcaatgtcatcaatcaccagccgggcgtagtgctgcgtcgcaggcatgtcatccagacgctggttcacgtaggccagttgtcggatcagtgccggatcgtccggaagccctttatgcgccggttcgagcatttcccgcgactgtgcgatatcaccgctatcccacaaggcgtaaccaagcgctgcctgggtgttgctattattcggttccagttccagcgcggcgcgcaaatcactcaccgcggccgggacattatgacgttggcgataaattgtcgcccgcgcaacgtaagcgttggcagaaggcgcaatattgattgagcgcgtgagatcgttcagtgcgagttccggctgaccaggaatgtaacgttgcgcatgcagccaccagtagagggcattgcttcccagtccacgtttttctgcctgttgtagccagcgatcgcgagccgcaccatttcctgccgcctgggcggtattggcagcagcaagcagatcctcattgctcatgtcgtgaagactgattttctgccaggccgccagtgcggtggcgtagtcctcaacctgatacgcctgataggctaccgcacgatgttgccaggcgctcggttgtcgttgttcggcctgaagccatgcatacaacgccacaccgggtagcgtgtcccgataacactttgccagacggttccaggcggcggcatcgtaggaaggcgacatatcgcccagcaagcgaactattgccgggcaattatctgcaatacccggcaactgactttgccactgacgttgctccgccagcggtaagggtttcgataaaatcgccaccttcgccggcgttgccaggtaaggatgactttccagcagagacgccagtcgcgccattaaagtctggctgacacgcgcatcgccctggaaaggatagcgttgcagcaataaatcggcagcttcgcgtgactgctcgttctgcatcagttgccaggttagttgatccaggcgggtaagatttgccggttcttgctgatacagcaatcgtgccagacgcagagcttcagccttgttacgggtcgccacgctgacagcataacgctcctcaagcatttcattggcggggagggtggcgagcagtttttgcgctgcgtcgtactgaccttcttttaacagcaccggtagcgtcgcgccaacaacatactggcggttgtcggcaaactgtaccgtataattcgccaacgcctgaacggggttagcgctgtatttagataacagatagagccaacttttctcttgtgcgtccgtggtaaatagtggcttattttcaatgagataatgctggaggcgtgctttttcgccacgataagccagcgcggtcgcgtaagtaatatatgactgaggatcggtgaagatcccctgtgattgcagtgccaggatccgatcgtccagctgcccggcaagaagcacgtcaaaccactgacggcgttctgccgcgcttaatgtgttctgctggcgtgcttcattgtatagcgtatctgcctgggaccattgtttcaggtagattgcccgttgcagcagatcggttcgcagcgtttttccttccggcgatgcagcaaacgtcgcatcgttcagttgcgctctggcgacaggtaactgtgccagccgcagggcattctgcccgacttcactgcgacaacgcagggtcggcgcagcatcgcacgctttttgctgggcaagcagttcttcaactgtcgtaacgcttttcacttcaaccggaatagccgccagactgcgctcaagtcgggcatctcctgggtgacgtttcagttgatcctcaagcaacagccgcgcccggtcatcatgaccaaaatggcgataggcttccgcaaggtataaagtcagcggaatattatccggcacctgctggtgtatatattcaaattcgcggatggcggttgcttcgtcgttatttttctgtgccttcagcgctttatcgagacggggataaataacaaaatggcgataatcgctcagccccagctcttctgcgctggtgccgatattgtctgcgagtgcgctggtactcaataaagacgtcagcagtaaaccagaccatccgatgacgcgattaaggttattctccttcattttcggactccagttgcgcaacctgttctgtgtttaaacctgctttgagtaatagtgattgcatcgaaacttgtaattcgcgttgaattgtcaggacgcgatccaacgtttcctggctgataacgccttcggtgaccaaaaacttgccgagcggcagagaactgcgttcatggcgcaataacaacacgttaattgctgaacgattaatatgaccgagcgtggtcagtatttcggcgaacaggaactgatgcggcacatattgccgccagatttcaccggcctgctgttccgtgagccactgatgctgaaccgcattgtacaacattgcccgcggatcgtgaccgcgtcggcgtgcataccagtgacgtaaccctgtgacaatttgtccccgcagaacaatgacgtaacgcactttgcgtccgactttacgcgtcagggccgccagcgaaaccgggtcaataccatcttcactgccgacaattaactcgtcattttccagacgcagcggcagtaccgcataatgcagcgccacggaggccggcatttcggcaatcagcgaggaagggatctgccaggcatcgatggattcccacgccacgccgttttgctctgccagcgcctgtgccagctgctcggcgctaatcagcccctgcatcagcattgaaccgcccaggcgtagaccttcgacgcgattacgcagtgctgtatcgagttgttcttcagtgatgacctgattttccagcagaatttgacctaacgggcgcaacgagcgggtatcgccagtcacgctggggaagtcatgcgttgttttatcccacgccacgcgacgtggatcgccgtgttgaagtacctgttttagcgcgcgccagttggccatgaagttaatcaggttgccccagaaaagacgcaggacggaaagcagcccctgcgtcaggccgtagtagccagtaacgaaaatcacccgctgcacgatgcggttaaccatcaaaccaaagtttagccacagcagggtcattaaccatgcgctgccgctgaaaatagaaaggaaatgccaggcatcgggccacaaactttcatacgccagcaacagcaaaagctggatcatcaccagcatcgcgaggaagctgacaaagttactgattgcccctttgcggtcgcgccagagaaagtagttcagcgtcaggctggaggtccatttatgggttttaaagccttggaaaacaatgccgatgatccagcgggatttttgtcgaaccgcagtcgaaaaggtatcggggaaatattcgcgcacgcagatcatgtttgatgtccgcgcgtgctgtaaaaatttacgctgctcgcgttctttggcttcgtccaccaccggaaaacggacaaaaatttccgtcatacctttttctttcaggcggaagccaatgtcgtaatcttcagtaagactctgcacgtcgaaagcaataccgtcaccgtcagctaacagtgcggtcacggcgcggcggctgaaacaggtgccgacgcctgcgctgggcacttgtccggcgagggcttcacgcaccggaacatctttgccatgcagctctgaaaactcatcaatgtaagtcatgctggtgaagtgcgtccattcgcgttcgaacggatacaccgggatctgaatcagatctttacgctcgaccagatagttgaacagacgcaattccatcggtgaaatcacatcttcggcgtcatgcagaataaaaccagcaaaagcgaaattggcgctacgctcaaattgggtgatggcgtccagcacgttgttcagacagtcggctttgctggtggggccaggacgcgcgcagactaccttatgcacattcgggaagcgagcgcacacttcgtcaacatcacgctgagtatcggggtcgttggggtaggtgccaacaaagatatgatagttttcgtagtcgagcgtggtcgccgccagctcggccatattgccgatgacgcccgtttcattccacgccggaaccataatcgctaacggtttttcatctggtttatacagttcgcggtaactcattcgcgggtagcggcgataaacactcaacttgcgtttaatgcggcgtacccagtagacgacatcaataaaaaaatcgtccagcccgctgatgaacatgatgaccgctaacgttatcgcgattacttttaagccgtagagccaggtagcaaaaacatcaagaagccagtccacacaaaaaccttacattaacgctggttatgtttagggtggcgtatattaaggttttttatgaattgtgacagctttttaccattaataggtatgactattgcggcacgttatttttacactggttataaaagttgccgtttgctgaaggattaagcgggtaatgtgataacaaaccttgtcccccgcgcatccgacgttaccgcaaccgtgcctttatgcgcgacaacaatcgatttcactatcgccaggccaataccgctaccttcaccttttcgctggcgggaggggtcaacgcgatagaaacggtcaaacaatcgcggtaagtgctcgggcgcaatgggcgtaccggggttttcgacgataacttgcaccaggtgatcgaccgtctgacagcgcactacaattgtctctccggttggcgtataacgcagggcgttcgaaagcaggttgcttagcgcccgacgcagcatcagcggatcgcccgcgacctgacacttgtcgccaacaaaccgcaactccacgccgcgatcttccgctaacgcctcgaaaaaatcgaacactttgccgacttcatccgccaggttgagcattttcttttcggggattagctggttgttatcggcctgagcgagaaacagcatatcgctgaccattttcgccattcgcgtcagctcttcgagattagagtagagcacatcttccagctccttctggctgcgcgactggctgagggcgatttcggtttgcgttatgagattcgtaattggtgtgcgaatttcgtgagcgatatccgctgagaaattggactggcgggtaaagacatcctcaatacgctcgatcatatggttgaacgacagtaccagctgttccagctcaatgggcacggtctgcgggtcgaggcgaacgtcgagatctttcgaggtaatattctggatttgacggctgacgctgcggatcggcgcgtgacctttatgtaccgccaacagtacgataaagacgatcaggatgctgattaccgatgcggtcataataagtttattcatcaaatcatttatgtaatgaagatgaaaatcgatcgaaagcgcgatgtagagcgtataaatcggtttgccgtccaccaacgggccaaccggcaagttaatcatccgccagttgctgtgttccatatgcccgtgaccgtggcctggcatcatcatcgtcgggccggaaaggagatacacctcgccaccctgagcgtctttatcgggtatggcgtcacgcgtaaactcgcggatatccggcgcaccgggggagtgatacaccgttttaccctgactatctgccagggaaatcaacacattggaataaccactgacgatatcttccagcgtcattaagcgtcgggcttgcgtttcgtcagggtgatttagtacccgttcaagggtggcgctaatctcttttaaatcattaatatcctgctcggcaaaatgaacttttactgagtggatcatgatccatgcaaaggcgaaaaacgccgcgatggtggccaggctgataaaaaaggtcaggcgggttgccagcgaaaacgggcgctgaaatggcttactgaccatccggcacctcaagcatgtaacccacgccgcgcacggtctgaattagcttcggctcaaagtcgttgtcgattttgccgcgcagccgcttcaccgccacatcaatagcattggtatcgctgtcaaaattcatgtcccatacctgcgaggcgataagcgagcggggcagcacttcgccctgatggcgaaggaagaactccagcagagtaaactctttactggtcaaagtgatgcgcgtgccgctgcgggtgactttgcggctgacgagatcgaccatcaaatcggcaacctgaaactgactttcgataatcaccgccgccccgcgccgcagtaatgtgcgcacccgcgccagcagttcagcaaaagcgaatggcttcaccaggtagtcatctgcccccaactccagccccttgacgcgatgttcaatggtgccaagcgcggtaagcaacagaatcggcatccctttattggcggagcgtaacatgcgcacgatatcccagccgttcacgtccggcagcataatatcgaggattatcagatcataatcaccggtcatcgccagatggtagccattcagcccgttgtcggccaaatcgaccacaaaaccggcttcggttaaccctttggtcaagtattctccggttttcttttcatcttcgacaatcaacagtttcatatttcctccgcatgttgcccgggcaattctagagtagcgggatcagatggcaatcgcttattggcaaaatgacaattttgtcatttttctgtcaccggaaaatcagagcctggcgagtaaagttggcggcataaaatcaccagaaattatgagcctatgtctccttgtaaacttctgccattttgtgtggcccttgcgctaaccggttgttcactggcaccggattatcagcgtccggcaatgcccgtgccgcagcagttctcactcagccagaacggcctggttaacgcagcagataactatcagaacgcgggctggcgcaccttttttgttgataatcaggtgaagacgctgattagcgaggcgctggtgaataatcgggatttgcgcatggcgacgctgaaagtgcaggaggcacgggcgcaatatcgtctgaccgatgccgaccgctacccacagctcaatggcgagggcagcggcagctggagcggtaatcttaaagggaataccgccacgacacgggagttttcgaccggccttaacgccagctttgacctcgattttttcggtcgcttaaagaacatgagcgaagccgagcgacaaaattatttagccactgaggaagctcagcgcgcggtgcatattctgctggtttctaatgtcgcgcaaagctatttcaatcagcaactggcgtatgcgcaattgcaaatagccgaagaaacgctgcgtaattatcagcagtcatatgcgtttgtcgaaaaacaactgttgacaggtagcagtaatgttctggcgctggaacaggctcgcggggtgatagaaagtacccgcagcgacatcgctaaacgtcagggggaactggcgcaggcgaataatgcattgcaactgttgctgggaagctacggcaagctgccgcaagcgcagacagtaaacagcgacagcctgcaaagcgttaaattaccggcgggattgtcgtcgcaaatcttattgcagcgcccggatattatggaagctgaacacgcgttaatggcggctaatgccaatattggcgctgcacgcgcggcattttttccgtctataagcctgaccagcggaatatcgaccgccagtagcgatctatcgtcattatttaacgccagcagcgggatgtggaattttatacccaaaattgagatccccatttttaatgccggacgcaaccaggccaatctggatatcgccgaaattcgccagcagcagtcggtggtgaattatgaacagaaaatccagaacgcctttaaagaagtggcagatgcgctggcattacgtcaaagcctgaacgatcaaattagcgcccagcagcgttatctggcatcgctgcaaattactttgcaacgggcgcgggcattatatcagcacggcgcagtaagttatctggaagtgctggatgccgagcgttctttatttgcaacccgacaaactttacttgatctgaattatgcccgtcaggttaacgaaatttctttgtataccgcacttggtggcggttgacagcaatatactcgtcatacttcaagttgcatgtgctgcgtctgcgttcgctcaccccagtcacttacttatgtaagctcctggggattcactcgcttgtcgccttcctgcaactcgaattatttagagtatgacttttaactccaggagagaataaatgaaaaaagcactgcaagtcgcaatgttcagtctgtttaccgttattggctttaatgcccaggctaacgaacatcatcatgaaaccatgagcgaagcacaaccacaggttattagcgccactggcgtggtaaagggtatcgatctggaaagcaaaaaaatcaccatccatcacgatccgattgctgccgtgaactggccggagatgaccatgcgctttaccatcaccccgcagacgaaaatgagtgaaattaaaaccggcgacaaagtggcgtttaattttgtccagcagggcaacctttctttattacaggatattaaagtcagccagtaacccaggtttaatgagatgaaaaaaatcgcgcttattatcggcagcatgatcgcgggcggtattatttctgcggcaggttttacctgggttgcaaaggcggaaccgcctgcagaaaaaacgtcgaccgcagaacgtaaaatcttattctggtacgacccaatgtatcccaatacgcggttcgataaaccaggtaaatcgccgtttatggatatggatctggtgccgaaatatgccgatgaagagagttctgcgtctggtgtgcgcattgacccgactcagacgcagaatctgggggtgaaaacggctaccgtcacgcgcggaccgctgacttttgcccagagtttcccggcgaatgtcagttacaacgagtatcagtatgccattgtgcaggctcgcgctgccgggtttatcgacaaggtgtatccgcttaccgtgggcgataaagtacaaaagggcacaccgcttctcgacctgaccattcctgactgggtggaagcgcagagtgagtatttactgctgcgcgaaaccggcggtacggcgacccagactgaaggcattcttgagcggctgcgactggcgggaatgccggaggcggatattcgccgcctgatcgccacgcaaaaaatccagactcgctttacgctcaaagcgcccattgatggcgtgatcaccgcgtttgatctgcgcgcgggaatgaatatcgccaaagataacgtggtagcgaaaattcagggtatggacccggtgtgggtcactgctgcgatcccggagtctatcgcctggctggtgaaagatgcctcgcagtttaccctcaccgttccggcgcgaccggataaaacactcaccatccgcaaatggacgctgctacctggcgtggatgccgcgacccgcacgctgcagctgcgtctggaagtcgacaacgccgacgaggcgctaaaaccgggcatgaacgcctggttgcaactcaacaccgccagcgaaccgatgctgctcattccgtcacaagcgctgattgataccggcagcgaacagcgggtgattaccgttgatgccgacgggcgctttgtaccgaaacgcgttgctgttttccaggcatcgcaaggcgtcaccgcattacgctctggtctggcggaaggtgaaaaggtggtttccagcggcctgttcctgattgattccgaagccaatatttctggcgcactggagcggatgcgctctgaaagtgctacccatgcgcattgagggaataaccaatgattgaatggattattcgtcgctcggtggcgaaccgttttttggtgctgatgggcgcgttgtttctgagcatctggggcacctggaccatcattaatacgccagtggatgcgctgccggatctctccgatgtgcaggttattattaaaaccagctatcccggtcaggcaccacaaatcgttgaaaatcaggtgacttatccgctaaccaccaccatgttgtcggtgcctggcgcgaagactgtgcgcggtttctcacagtttggcgactcttatgtgtatgtcattttcgaagatggcaccgatccgtactgggcgcgttcgcgggtgctggagtacctcaaccaggtacagggtaagctgcctgcgggagtcagcgccgagctggggccagatgccacgggtgttggctggatctatgaatatgcactggtggatcgcagcggtaagcacgatctggccgatttacgctcattacaggactggtttctcaaatatgagctgaaaaccatccctgacgttgcggaagtggcgtcggtgggcggtgtggtgaaagagtatcaggtggttatcgatccccagcgcctggcgcagtatggcatcagtctcgccgaagtaaaaagcgcgctggatgcttcaaaccaggaagcgggcggttcgtcgatcgaactggcggaagcggaatatatggtgcgcgccagcggctatctgcaaacgctcgacgactttaatcacatcgttttaaaagccagtgaaaatggcgtgcccgtttatctgcgcgatgttgcgaaggtccagattggcccggagatgcgccggggcattgccgaactaaacggcgaaggcgaagtggcgggcggggtggtgatcctgcgatccggcaaaaacgcccgagaagtgatcgccgccgtgaaggacaaactggaaacgctgaaaagtagtctgccggaaggcgtggagatagttacaacatacgatcgcagccagctcattgaccgcgccatcgacaacctcagcggcaagttgctggaagagtttattgtggtggcggtagtctgtgcgctgtttctctggcatgtgcgctcggcgctggtggcgattatttcgttgccgctggggttgtgtattgcttttattgtcatgcacttccagggactgaatgccaatattatgtcgttgggtggcattgcgattgccgtcggggcgatggtcgatgctgctatcgtcatgatcgagaatgcgcataaacggctggaagagtggcagcaccagcatcctgacgccacgctggataataaaacgcgctggcaggtgatcaccgatgcgtctgttgaagtggggccggcgctatttatcagtctgctgattatcacgttgtcgtttatcccgatcttcaccctggaagggcaggaagggcgtctgtttggcccgttggcgttcaccaaaacgtatgcgatggcgggtgcggcgctgctggcgatcgtagtgatcccgatcctgatgggctactggatccgtggcaaaattccgccggaaagcagtaacccgctcaatcgctttttgattcgtgtttatcatccgctgttgctgaaagtactgcactggccgaaaaccacgctgctggtggcggcgctttcggtgctgacggttctctggccgctcaataaagttggcggggaatttttaccgcagatcaatgaaggcgacttgttgtatatgccatcgacgctgccggggatttccgcagcagaggcggcgagtatgctgcaaaaaaccgacaagctaattatgagcgtacctgaagtggcgcgggtatttggcaaaaccgggaaagcggaaaccgccaccgattctgctccgctggagatggtagaaacgaccatccagcttaagccgcaggagcagtggcggccaggcatgacgatggacaaaatcattgaggaactggataacaccgtgcggctgccggggctggcgaatctgtgggtgccgccaattcgtaaccgtatcgatatgctctcaaccggcattaaaagccccatcggcattaaagtttccggcactgtgctggcggatatcgacgcgatggctgagcaaattgaagaagtagcgcgaacggtgccaggcgtagcttctgcgcttgccgagcggctggaaggtgggcgctatatcaacgttgagattaaccgtgaaaaagccgcacgttacggtatgacggtggcggatgtgcagttgtttgtgacttctgcggtgggcggggcgatggttggcgaaacggtggaagggattgcccgttatccaattaatctgcgttatccgcaaagctggcgcgatagtccgcaggcactgcgccagctgccgatcctgacgccgatgaagcagcaaatcaccctggcagacgtggccgacattaaagtctctaccggaccgtcgatgctgaaaaccgagaatgcgcgcccgacgagctggatttatatcgatgcccgcgatcgtgacatggtgtcggtggttcacgatttgcaaaaagcgatagctgaaaaagtgcagttaaaaccgggcaccagcgtggcattctccgggcagttcgagctactggagcgcgccaaccataagcttaaactcatggtgccgatgacgttgatgattatcttcgtgctgttgtatctggcgttccgtcgggtgggcgaagcgttgctgattatcagcagcgtaccgtttgcgctggtgggcggcatctggttgctgtggtggatgggctttcatctttccgtggcgacgggcactggctttatcgccctcgccggggtcgccgccgaatttggcgtggtgatgctgatgtatttacgtcacgccatagaggccgtgccgtcgttgaataatccacaaacattcagcgagcagaagctggatgaggcgttatatcacggcgcggtcctgcgcgtgcgcccgaaagcgatgacggtggcggtgattatcgccggtctgctgccgattctgtggggaacgggggctggttcagaggtgatgagccggattgccgcgccgatgattggcggcatgatcaccgcacctttgctgtcgctgtttattatcccggcggcgtataagctgatgtggctgcaccgacatcgggtacggaaataaaagcaggataccccgtttaaccgtgtggattgtgtcttgcgacgatgggcactaaatgttaaaaggtgcccctcaacaaaaaagacacacaggggaaaggcgtgaaaaacgcgtcaaccgtatcggaagatactgcgtcgaatcaagagccgacgcttcatcgcggattacataaccgtcatattcaactgattgcgttgggtggcgcaattggtactggtctgtttcttggcattggcccggcgattcagatggcgggtccggctgtattgctgggctacggcgtcgccgggatcatcgctttcctgattatgcgccagcttggcgaaatggtggttgaggagccggtatccggttcatttgcccactttgcctataaatactggggaccgtttgcgggcttcctctctggctggaactactgggtaatgttcgtgctggtgggaatggcagagctgaccgctgcgggcatctatatgcagtactggttcccggatgttccaacgtggatttgggctgccgccttctttattatcatcaacgccgttaacctggtgaacgtgcgcttatatggcgaaaccgagttctggtttgcgttgattaaagtgctggcaatcatcggtatgatcggctttggcctgtggctgctgttttctggtcacggcggcgagaaagccagtatcgacaacctctggcgctacggtggtttcttcgccaccggctggaatgggctgattttgtcgctggcggtaattatgttctccttcggcggtctggagctgattgggattactgccgctgaagcgcgcgatccggaaaaaagcattccaaaagcggtaaatcaggtggtgtatcgcatcctgctgttttacatcggttcactggtggttttactggcgctctatccgtgggtggaagtgaaatccaacagtagcccgtttgtgatgattttccataatctcgacagcaacgtggtagcttctgcgctgaacttcgtcattctggtagcatcgctgtcagtgtataacagcggggtttactctaacagccgcatgctgtttggcctttctgtgcagggtaatgcgccgaagtttttgactcgcgtcagccgtcgcggtgtgccgattaactcgctgatgctttccggagcgatcacttcgctggtggtgttaatcaactatctgctgccgcaaaaagcgtttggtctgctgatggcgctggtggtagcaacgctgctgttgaactggattatgatctgtctggcgcatctgcgttttcgtgcagcgatgcgacgtcaggggcgtgaaacacagtttaaggcgctgctctatccgttcggcaactatctctgcattgccttcctcggcatgattttgctgctgatgtgcacgatggatgatatgcgcttgtcagcgatcctgctgccggtgtggattgtattcctgtttatggcatttaaaacgctgcgtcggaaataaggcattcacgctacatccgacaaaacgatgtcaaccatccgaaaccgctctcatccattcgatgagagcggtttttttaattactgcttaaatgcacccgccagagagcgaatatcattgccggttggcgactgatgaagtcgcagaccaaactcttcgacaatcgcaaatatgtgatcgaatatatcagcctgaatgctttcatattccagccacaccacggtgttagtaaacgcgtagatctcgagcggtaaaccgttatcacctggagccagttggcgtaccattaaggtcatatctttacgaatccgcggatggttacgcagatattcgttcagataggcacgaaaggttccaatattggtcattcggcgcagatttaataccgactccgtagaaccttgctggcgattccactcattaatttcctgatggcggctggttaaataaggctttaacaaatgcgctttattcagacgttgcatttcgtcttcatcaagaaaacgaatactggtgacatcaatactgatactgcgcttaatacgtcgcccgccagatgctgacatcccgctccagtttttaaaggagtcagaaaccagagaccaggtgggaatagtggtaatggtattgtcccagttacgcactttgacggtggttaacccaatatcgatcaccgcgccatccgcgccgtatttcggcatctccagccagtcgcccagtttcagcatatcgttcgcggaaagctgaatacctgccaccagaccaagaatcggatctttaaataccaacatcagcacggcagccattgcaccaagaccgctgatcagaatcgctggcgactgaccaatcagcagcgagatcatcaaaatgccgaccagaatcgcgccgatcagtttaatcccctgaaatatccctttcagcggtaactgagatgctgccgggaatttctgcgccagattcaaaataacatccagcaacgagaagactgaaagcagcgcatacatcatgatccacaactgcgcgcaggtagtcagaatatctgccgcttcggtgcctttttgcagccagaataccgcctgaatattgacgataatcccctgcagggtaaaagctaaacggtggaagagtttattctgggtaatgatttgcaaccaaagccgtgaactggcgatggcacgtttttcgaaggtccgcagtaccacccaatgcaaaataatatgcaccacgacggcggtcagaaaaataataccgaaaatcatcaccatcgaggtggtgtgatcgatctcaatacccgctaaatcttcaacctgggatattaaatcctgcataacgtctcctttatacaacagcagcctatgatgacggctgaaacagggttatgcaaatcaggagaatctgagaggaaatagccgggcagatgcccggcaagagagaattacacttcggttaaggtgatgttttgcggcagacgagatttcggcagcgtagcgttaaaatcttcaacgctgtgatgacctaccggaacaaccaccagactggtgtagcctttctctttcagaccaaattctgcatcgaggatggcggcgtcaaaaccttcgatgggtaccgcgtccagacccagagccgccacgccgagcaggaagttaccgacgttgagataaacctgttttgccatccactctgcatcatcatgcagatctttacggtgcatatcagcgaagaacttgcgacctttatcgttcgcggctttcgcttccggcgtggcaaagcggccatcggcatcttcctggtcaacaaccagcttcagccagacatcgtccatcgcggtttttgcacagaacaccacgacgtgcgaggcatcaagcattttacgctcgttgaacacgtaattaccggcagcggatttggcaacacgcgctttaccttcttccgtgctggcaacaataaaatgccacggctgggagttggtgctggatgggctgtattgcagtagcgttttgatctgctcggcctgttccggggtaagttttttgctggcatcaaatgccttagtggaatgacgctttaaggcgacagaaatgatatccataaagactccatgtgaaagtaattttgcgtgccagcagattacaaggttcaacgagaaatggtaagcgagaaaaatgcgctatagatttccgctttagcctggacgcactcttttttgatcgcgtttagccagaccatcaaccaccagattccacgaatcgttgatcagatcgcgaagtaacgcttcggagatttcttcgccgggatacactgaaatccagtgctttttattcatgtgataccctggcttaatgcttgggtatatttgctgatttaacagggatttttgtggatcggacttcagattgataaaggggacgccgcgtagctccgacgacagcataaaaatcttgccgccaattttaaaaacatcgaactccgggccaaaaggccagcaaagctcgacaaagggtaactcaagggccaggcgtttcgccgtttcgtgcagtgattgcttatccataaacgttcctttaggcgaaggagaataagcaaagtatgccgcgaagtacggcgataatcgacgtttaatccgccagcgagaaccagcgtcgccagataaagcgcagaacaaaatactcaatagcgcccagcactaaaaaccacagacaaaacaataaagtgtaaagctgactaagatccatcagatggaacatggtcaccagtttttgtgccagcgccagccccagtgcgggggcgggcagcagcaggcaagagaggaaagccatcagcaaaatgcctgctgcggtggtcaaggtttctaaagggtgtttcataacattgttaaatgtaagttaaaacaccattgtcagggatattcttctgtaaggcaattcccggcttagtcaccggcccagatctcacaatgctttttcaccagcccaatcagcgagccgccatcggcgacgaaatcgcgcattagctgcgcttcattcagaccgctgacgacctggcgatgcagggcctcaatcgcgctcgatgcaccaattttatgtgcggaaggggcgattttttccagcaatcgcaaggtatcttccgttagcggtcgacgatctccagtgtgcggatcggtgatgacgccttcaagcccatagcgacaggcctggaaacggttgaatttatacagcaggtaatctttttcctgatgtttaaacgggcgttccgtcagtaaccagtgggcggtagcctgaattaatcccgccatatttactgcgtggctaagggttaacggggtatccatcacccgaacctccaccgtgccaaaatgaggactggggcgaatatcccagtgcagatctttaatgctgtcgatcatcgtggtgtaactcagacagcgaaacagggcttcaaattgttgccagttactgacccacggcatcgggccattatcaggaaaggcggaaaaaatattcggtcgtgaggaggcaaaacgcgtatccgttccctgcatatatggcgacgcggcggaaagggcgataaagtgcggcacaaatcgtgacaagccgtgcagcaaataaatggcgtcatcgccactggcgcagccaacatggacatgctgaccaaaaacggtcgcctgctgaatgagataaccaaagttttccagcgtgcgttgatagcgttcgttatcgcatacctcctgacgctgccatttctgaaacgggtgcgtgccaccgccgcaaatttccagatgatggtctgtggctgcctgcaatacgactttctgcatcgctgaaaactgcccggcagcctggttgatatcacggcaaacatccgtcgccagctccagcatactttcggtgatatcgtgctttacctctccggccgtgatcttatttttaaccgcgtcaatcagcattgaagagtcctggcttaagtcatagcccggcggattaaccacctgcatttccagttcaataccgagggtaaaaggttcagaaacatgaaaatcgggtaatggcataggtttctcttatgttggcgttttctattcagtatagaagtcggagcggctgggcgagatgcggaagttctggaatgtttcttttttttggtgatggtgaactgatggtgcctgaagcaatttggctacttttgcaatgtgacaagttatggcagtgctgactggtggcgaagaattttgacgattgagtcatgcagaaaaaaacgggttcagcttcagttgattaaatgaggagtgagaagtccgaaacaggactcactgtataaataaacagctattttgttgaggaagggtaagataacggcgggtgcctgaagctttccggtttcaggtttactctgaggtctggaaagatgaagccccaggagatatttctatcaaccctggggctgccactccaaacccgaacaatttggatggtagtcccttcttcgcatggaggcaatataaacatgctgacgaaatatgcccttgcggcagtcatagtgctgtgtttaacggtgctgggatttacgcttctggtcggagactcgctgtgtgagtttacggtgaaggaacgtaatattgagtttaaggctgttctcgcttacgaaccgaagaagtagccgttgtgcggggagtaatcccataagcgctaacttaagggttgtggtattacgcctgatatgatttaacgtgccgatgaattactctcacgataactggtcagcaattctggcccatattggtaagcccgaagaactggatacttcggcacgtaatgccggggctctaacccgccgccgcgaaattcgtgatgctgcaactctgctacgtctggggctggcttacggccccggggggatgtcattacgtgaagtcactgcatgggctcagctccatgacgttgcaacattatctgacgtggctctcctgaagcggctgcggaatgccgccgactggtttggcatacttgccgcacaaacacttgctgtacgcgccgcagttacgggttgtacaagcggaaagagattgcgtcttgtcgatggaacagcaatcagtgcgcccgggggcggcagcgctgaatggcgactacatatgggatatgatcctcatacctgtcagttcactgattttgagctaaccgacagcagagacgctgaacggctggaccgatttgcgcaaacggcagacgagatacgcattgctgaccggggattcggttcgcgtcccgaatgtatccgctcacttgcttttggagaagctgattatatcgtccgggttcactggcgaggattgcgctggttaactgcagaaggaatgcgctttgacatgatgggttttctgcgcgggctggattgcggtaagaacggtgaaaccactgtaatgataggcaattcaggtaataaaaaagccggagctccctttccggcacgtctcattgccgtatcacttcctcccgaaaaagcattaatcagtaaaacccgactgctcagcgagaatcgtcgaaaaggacgagtagttcaggcggaaacgctggaagcagcgggccatgtgctattgctaacatcattaccggaagatgaatattcagcagagcaagtggctgattgttaccgtctgcgatggcaaattgaactggcttttaagcggctcaaaagtttgctgcacctggatgctttgcgtgcaaaggaacctgaactcgcgaaagcgtggatatttgctaatctactcgccgcatttttaattgacgacataatccagccatcgctggatttcccccccagaagtgccggatccgaaaagaagaactaactcgttgtggagaataacaaaaatggtcatctggagcttacaggtggccattcgtgggacagtatccctgacagcctacaaaacgcaattgaagaacgcgaggcatcgtcttaacgaggcaccgaggcgtcgcattcttcagatggttcaacccttaagttagcgcttatgggagtaatccccgcatatccggttgtcaggtcaggatggtaaggcacctgctttacactttcgcccgtggtcagtgatggctgcgggcgaatcgtaccagatgttgtcaattaatcgtgttggcacagcgttatgactatcttttcttttatctgccagtgcacagcaaacatctcattctcacgatgaatgatgacctgctgtttattccagctaattatctgatagtccagaaaacctgcatcagtttggatctcacttgccttaaatgcgctctctttggcggaaaatgccagtgtcagcgccagagaaaaggctaaaccgcagtctgcgagtcgctcgtgttccgctggtgtaataatgttgtctgtcaattctcttgcggtttgtacagaaaaaatttcttctatatcaatgccaatcggttgacgagataccacggctaatgccgtagtcccacagtggctaatactgccgtatacctccgcaggccagacaggttggcgtagctcgccgattgcgggcacacatttatagccatattcccgcaaagcataaacagcagcgatccgtccggctaaatgctctgttttacgtttacgtccagcgtgttgcagttgtgcgtagtgcggcagccagagtaaatcctgctcacaaaaattcgccggatcgaactcaacaaaatgcagcgtatgtccggcaaaggggagggaggtatgcgtagttttcatatcgaccatattcgagactgatgacaaacgcaaaactgcctgatgcgctacgcttatcaggcctacatggtcctgcaatatattgaattggcaagatttttgtaggccggataaggcgttcacgccgcatccggcatgaacgacgcgcactttgtcaacaatctgacgttagcatcagaagtgggtgtttacgctcatataccacgtacgtcccggctcgttataggtatacgccccggcaccggcgatatagttggcccctgccaaatcgcccgtggtctgggcattacccgcacgccacaaacgtttgtcgaacagattgtccacgccgccggtcagactgacattcttcgtcacatcccaggtcgcgctcaggccaacaatgctgtaaggactaatttctttggtttccggtccaaccgctggctgacctttatagttgtacttcttcggctgctgcttgccgtaccaggtgaaggtcgtttgcatcgacaaatcttcccgtgcctgccagctcagcgttgagttcaacgtatactccgggatgatcgacaaacggtcgcccgtggttttgttttcactcttcagcatataagtgatgttattggtccacatcaccgtttcgctaaccggtacgtttaacgatccttccagaccttcaaccaccgctttcggcacgttatcccactgatagagatcggtgccgactgcgttttgccctacagccacatagcccgcttcaatcttattgcgataatcgttacggaaccaggtgacgcccgccagccacccgtcgcgtttgaactccagaccaatctctttgttgatgctggtttctgctttcaggtcatcgttaccttgcagatagcagccgcccgcgctggcatagcaaccctgacctttactgtagagaatgtagttcgggttagtctggtacaggctcggcgctttataagcacgggcgatgcccattttcagcgtgaagtcatcgcctaaaccttgcgatatgttcagcgccgggctccagttattgccgacaatactgtgatgatcgaaacgcagccccggcgttacgatggtgctgtcagtcagctccatgttgttttcggcaaacagcgagaaaatttctgcttttgaatacgggctacggtcggtggtactcacgccatcaatagcgccaccggtattcgttccggtcagtgcctgggtgttggaacttaagtccttcatccgttgctgattccactccgtacccagcgtcagcgtctggttaacgaggaaatcaatcggcaggttaacttcgctgtgcagcatcacgtcatcaagatcgatatcgacgaaatcctgtgtcgctttttcgttaaatttcccttcggtaccgcccgccagaccttccggaatacgcgagttacgggtgtgttcgtactgcacccagttgctggtggtcacgccgttatcccagccaccgttccaggtcagcgcgtagttctggcgatacagacggttggtttcatcgccatatttcgagcgggtataggaatcggagttggtattctgggtgtcgcccgcatacaggttaccctggcggctgtaacctgcttccagttccagcgattgcaatggcgcgaaatcccagcgcaccacgccattaatatctttgttgattaccccttcgcgcccggctggtaacgtcgtggcatacgttccggcacgcgcggactgatggccctggttgatatcccacgcgtcagcctgggttttgtcgaggttgccatacaaacggaagctgaattcgtcgcccagcggaccggtcaggctaaagttagtgcgtttggtggcaccttcctctttatgttctggcgcattgaaatatgcgtcccaggagccgtgccactcgccgctgccttttttggtaatgatgttaaccacgccgcccgccgcgccgttgccataacgcgcagctgccggaccacgcagaacttcaatacgttcaatcatttcaggtggcacccaggaagtatcaccacgggtatcgcgctcgccacgccagccctgacgcaccgagttacggctgcttaccggcttgccgtcaatcaaaatcagcgtgttttccggacccataccgcgaatatcaatctgtcggttattcccacgctgaccactggtggagttaccggtcaggttaacgcctggcatggtacggatgatcttcgacacatcgcgggcaaccgggtttttgcggatttcatctgcggtgatggtcgaaacgccaggcgcctgtaagttctgctcggcggcggtaacgacaatagtatcgtcatgtgaaacaggagtatcggtcggctcttgtgcctgcgctaccccataaatccccagattgaccaacaaggccagggaatgaatcttcttgttcattgttttattcctgcatttttgccacgaattgcaactgtcgggcatggtcgtcatcaacacgacgcatcccgctaccgcgaaaacctttgatcctgaaagacacgcagtgcagttggttaattaatgtccgcgcttcccacggcgcgccattacgctattgcaaatgcaaatagttatcaataatattatcaatatatttctgcaatcaatgaaaaattgcacagtaaacatggggttatggtgtgacggcgttaaaagtaggaagtgagagctggtggcagtcgaaacatggcccggaatggcagcgtctgaatgacgaaatgtttgaggtcactttctggtggcgtgatccccaaggttctgaagaatactcgacgataaagcgcgtatgggtctacatcactggtgtgaccgatcaccatcagaacagccagccccagtcgatgcagcgaattgcaggcactaacgtctggcagtggacgacacaactcaatgccaactggcgcggcagctactgctttattcccaccgaacgcgatgacattttttctgtaccatcccccgatcgcctcgaattgcgcgaaggctggcgaaaactattaccccaggcgatagccgatccgctgaacctacaaagctggaaaggcgggcgagggcacgctgtttctgcactcgaaatgccgcaagcgcctctgcaaccgggatgggattgtccgcaagcgccagaaatacctgccaaagaaattatctggaaaagtgaacggttgaaaaagtcacggcgtgtatggatttttaccaccggcgatgcaacagcagaagaacgcccgctggcagttttgctcgatggcgaattttgggcgcaaagtatgcccgtctggccagtgctgacttcgctgacccatcgtcagcaacttcctcccgccgtgtatgtgttgatcgacgctatcgacaccacgcaccgcgcccacgaactgccgtgtaatgcggatttctggctcgcagtacagcaagagttattacccctggtgaaagctattgccccttttagcgatcgtgccgatcgcaccgtggttgccgggcagagttttggtgggctttccgcgctgtatgccggactgcactggcctgaacgctttggctgtgtattaagccagtcaggatcgtactggtggccgcatcggggcgggcagcaagagggcgtgttacttgaaaagctaaaagctggtgaagttagcgccgaaggtctgcgcattgtgctggaagcgggtattcgcgagccgatgatcatgcgggccaatcaggcgctgtatgcgcaattacaccccataaaagaatccattttctggcgtcaggttgacggcggacatgatgcgctttgttggcgcggtggcttgatgcaggggctaatcgacctctggcaaccacttttccatgacaggagttgaatatggcattcagtaatcccttcgatgatccgcagggagcgttttacatattgcgcaatgcgcaggggcaattcagtctgtggccgcaacaatgcgtcttaccggcaggctgggacattgtgtgtcagccgcagtcacaggcgtcctgccagcagtggctggaagcccactggcgtactctgacaccgacgaattttacccagttgcaggaggcacaatgagccagcatttacctttggtcgccgcacagcccggcatctggatggcagaaaaactgtcagaattaccctccgcctggagcgtggcgcattacgttgagttaaccggagaggttgattcgccattactggcccgcgcggtggttgccggactagcgcaagcagatacgctgcggatgcgttttacggaagataacggcgaagtctggcagtgggtcgatgatgcgctgacgttcgaactgccagaaattatcgacctacgaaccaacattgatccgcacggtactgcgcaggcattaatgcaggcggatttgcaacaagatctgcgcgtcgatagcggtaaaccactggtctttcatcagctgatacaggtggcggataaccgctggtactggtatcagcgttatcaccatttgctggtcgatggctttagtttcccggccattacccgccagatcgccaatatttactgcacatggctgcgtggcgaaccaacgcctgcttcgccatttacgcctttcgctgatgtagtggaagagtaccagcaataccgcgaaagcgaagcctggcagcgtgatgcggcattctgggcagaacagcgtcgtcaactgccgccgcccgcgtcactttctccggcacctttaccggggcgcagcgcctcggcagatattctgcgcctgaaactggaatttaccgacggggaattccgccagctggctacgcaactttcaggtgtgcagcgtaccgatttagcccttgcgctggcagccttgtggctggggcgattgtgcaatcgtatggactacgccgccggatttatctttatgcgtcgactgggctcggcggcgctgacggctaccggacccgtgctcaacgttttgccgttgggtattcacattgcggcgcaagaaacgctgccggaactggcaacccgactggcagcacaactgaaaaaaatgcgtcgtcatcaacgttacgatgccgaacaaattgtccgtgacagcgggcgagcggcaggtgatgaaccgctgtttggtccggtactcaatatcaaggtatttgattaccaactggatattcctgatgttcaggcgcaaacccataccctggcaaccggtccggttaatgaccttgaactggccctgttcccggatgtacacggtgatttgagtattgagatcctcgccaataaacagcgttacgatgagccaacgttaatccagcatgctgaacgcctgaaaatgctgattgcccagttcgccgcggatccggcgctgttgtgcggcgatgtcgatattatgctgccaggtgagtatgcgcagctggcgcagctcaacgccactcaggttgagattccagaaaccacgcttagcgcgctggtggcagaacaagcggcaaaaacaccggatgctccggcgctggcagatgcgcgttacctgttcagctatcgggaaatgcgcgagcaggtggtggcgctggcgaatctgctgcgtgagcgcggcgttaaaccaggggacagcgtggcggtggcactaccgcgctcggtctttttgaccctggcactccatgcgatagttgaagctggagcggcctggctaccgctggataccggctatccggacgatcgcctgaaaatgatgctggaagatgcgcgtccgtcgctgttaattaccaccgacgatcaactgccgcgctttagcgatgttcccaatttaacaagcctttgctataacgccccgcttacaccgcagggcagtgcgccgctgcaactttcacaaccgcatcacacggcttatatcatctttacctctggctccaccggcaggccgaaaggggtaatggtcgggcagacggctatcgtcaaccgcctgctttggatgcaaaatcattatccgcttacaggcgaagatgtcgttgcccaaaaaacgccgtgcagttttgatgtctcggtgtgggagtttttctggccgtttatcgcaggggcaaaactggtgatggctgaaccggaagcgcaccgcgacccgctcgctatgcagcaattctttgccgaatatggcgtaacgaccacgcactttgtgccgtcgatgctggcggcatttgttgcctcgctgacgccgcaaaccgctcgccagagttgcgcgacgttgaaacaggttttctgtagtggtgaggccttaccggctgatttatgccgcgaatggcaacagttaactggcgcgccgttgcataatctatatggcccgacggaagcggcggtagatgtcagctggtatccggcttttggcgaggaactggcacaggtgcgcggcagcagtgtgccgattggttatccggtatggaatacgggtctgcgtattcttgatgcgatgatgcatccggtgccgccgggtgtggcgggtgatctctatctcactggcattcaactggcgcagggctatctcggacgccccgatctgaccgccagccgctttattgccgatccttttgccccaggtgaacggatgtaccgtaccggagacgttgcccgctggctggataacggcgcggtggagtacctcgggcgcagtgatgatcagctaaaaattcgcgggcagcgtatcgaactgggcgaaatcgatcgcgtgatgcaggcgctgccggatgtcgaacaagccgttacccacgcctgtgtgattaaccaggcggctgccaccggtggtgatgcgcgtcaattggtgggctatctggtgtcgcaatcgggcctgccgttggataccagcgcattgcaggcgcagcttcgtgaaacattgccaccacatatggtaccggtggttctgctgcaacttccacagttaccacttagcgccaacggcaagctggatcgcaaagccttaccgttgcctgaactgaaggcacaagcgccagggcgtgcgccgaaagcgggcagtgaaacgattatcgccgcggcattctcgtcgttgctggggtgtgacgtgcaggatgccgatgctgatttcttcgcgcttggcggtcattcgctactggcaatgaaactggcagcgcagttaagtcggcaggttgcccgccaggtgacgccggggcaagtgatggtcgcgtcaactgtcgccaaactggcaacgattattgatgctgaagaagacagcacccggcgtatgggattcgaaaccattctgccgttgcgtgaaggtaatggcccgacgctgttttgtttccatcctgcgtccggttttgcctggcagttcagcgtgctctcgcgttatctcgatccacaatggtcgattatcggcattcagtcaccgcgccccaatggccccatgcagacggcggcaaacctggatgaagtctgcgaagcgcatctggcaacgttacttgaacaacaaccgcatggcccttattacctgctggggtattcccttggcggtacgctggcgcagggtattgcggcgcgactgcgtgcccgtggcgaacaggtggcatttcttggcttgctggatacctggccgccagaaacgcaaaactggcaggaaaaagaagctaatggtctggacccggaagtgctggcggagattaaccgcgaacgcgaggccttcctggcagcacagcagggaagtacttcaacggagttgtttaccaccattgaaggcaactacgctgatgctgtgcgcctgctgacgactgctcatagcgtaccgtttgacggtaaagcgacgctgtttgttgctgaacgcacacttcaggaaggtatgagtcccgaacgcgcctggtcgccgtggatagcggagctggatatctatcgtcaggattgtgcgcatgtggatattatctctccagggacgtttgaaaaaattgggccgattattcgcgcaacgctaaacaggtaaattaatattatttataaacccataattacagaaaataattatgggttttttatttgtttgatttataggtttgatgaatatttctcttaaatagagtgaatgttgcattcagtggaaggaatttacaaacttcagcttcggataattatcaccaactggtaaagtgagcgccgtggagatttccccctattggactcattttcaggttataccccatgtcatcactgaatattaaacagggaagtgacgctcattttcccgattatcctctggcgtcgcccagtaataatgaaattgatttacttaatctaatctcagttttatggcgggccaaaaaaacggtcatggcggtcgtttttgcgtttgcctgcgcaggcttgctgatctctttcatcctgccgcaaaaatggaccagcgcggcggttgtcacgcctccagaacctgttcagtggcaagagttggagaaatcattcactaagcttcgtgtgctggatctggatatcaaaattgatcgtacagaagcatttaacctgtttatcaagaagtttcagtcggttagcttgctggaagagtacctgcgttcatcaccttatgtgatggaccaattaaaagaggcgaaaatcgacgaactggatttgcatcgcgcaattgtcgcattgagcgaaaaaatgaaagcggttgatgacaatgccagtaagaaaaaagatgaaccgtcactgtatacctcctggacgctaagttttaccgcgccaaccagtgaagaggcgcagaccgttttgagcgggtatatcgattatatctctacgttggtggtgaaagagtcgctagaaaacgtccgtaataaactggagatcaaaacccagtttgaaaaagaaaaactggctcaggatcgcattaaaacgaaaaatcaacttgatgcaaacattcagcgcctcaattattcactcgacattgccaacgcggcaggaattaaaaagcccgtttacagtaatggtcaggccgttaaagatgaccccgatttttctatttctctcggtgcagacggtattgaacgcaaactggaaatagaaaaagcggtcactgacgttgcggaactgaacggtgaattacgtaatcggcagtatcttgtcgagcaattaacaaaagcacatgtcaacgatgtgaattttacgccgtttaaatatcagttaagcccgtcattgccagtgaaaaaagacggtccgggtaaggcgattattgtgatcctttccgcgttgatcggcgggatggtggcttgtggtggcgtgctgttgcgctatgcgatggcatccagaaaacaggatgccatgatggcagaccacttagtttaactatttgcggttgaaggtgccgttcgtccgagcggcaccacaagcggcgttccggcaactggatcgtcaatgatcatgcagcgcagaccataaatgcgctcaatcagttcagcagtgacaatctccttcggcgctccctgagcaacaattttcccttcccgcaatgcaatcaaatggctggcgtaacgacaggcctgattaagatcgtgcagcaccgccgccagggtatagcctttttcgcggttcagttcgcttaacaactccagcaaatcaatctgatgactgatatccagccaggtcgtgggttcgtcgagcagcataattgccgtttcctgggccagcaccatcgcgatccacgctcgctggcgttgtccgccagaaagggtatccacgctttgatctgccagatgagttattcccgtggcctgcattgctttcgttaccgcttcttcatcctctttgcgccagcgggtaaacagcggttgatgcggataacgtccacgcgccaccagctcctgcacggtgatatcgcccggcgtggtagcattttgcgccaacagaccaatccggcgtgcaacctctttactggcgtaatgttgaatgtgctcgccatccagccagacatgcccatgagcaggcgtcatcaggcggcttaaggtacgcagtaacgtggatttaccgcagccatttggcccgataattgccgtgaagtgaccatcaggtatttctacagtcagattttccgcaacggtatatttgccatatcccagggttaactgttcgccgcgcaaacgggctactgattcggtcattttttgcgagactcctgaattaacaagacgataaggtaaataccgccgaggctgacggtaacgacgccaaccggaagttgatacggcataaacagttgttgggcgcagagatcggccgccagcagtaacagcgccccgcatagcgccgcctgggttagcccccagcgagcggtgccgctaatgcgtcgggcaatgtgcggtgcgactaaagcaataaaggaaatcggcccggcaagcgctgttgccgcagcggtaagcaccactgcaaccagcatcattaacagacgcgaacgttcgacgctgacgcccagcgcacacgcggtatcatcgcccatttccagcaagcgcatccggcgtaccagtaaggcggcggcaatgagcatcaatataatgatgggtgcggaaggcgaggtttttgcccacgtcaggccgttgagcgatccggcattccacaaacctgctgttagcgccgtttctaaagacgctttcagcaacagccaggtattaaaggccaccagcatggcgcgaacgccgataccgataataatcaaccgaaaggtgtcgatgccgttgcgccaggcgagcagccagaccagcagcgaagtgacaatgccgcccaccattgctgacagcgcgatagccgtcaggtcctgaccaaacagcaccatcgccaccagcacgccgctccacgccccggtgttaaagcccattacgtcagggctgccgagcgggttacgcatcagcgactgaaaaatcgcgccactgacgcccagtgctgcgccaatcaacagcgccatcagcacgcgtggtaaacgccattcggtgaccaccatcgtcatactgcgcggcgcatcgcccatcagcgcggcgaatacctgcgaggtttccagcgtgacggcaccgctgcgtaatccccagatacctgcaaccacacaggcggaaaccagcagcaaacaggtgatgagtaatcggcgagagacgtaaatcatgcaccacctcgcgttttacgtcgcacgaggaagatcagcaccggtgcaccaataaacgcactgaccacagaaacgcgcagttcgccgggcacaatcacccgcccgatgatatcggcaaacagcagcagggcaggggtagcaagtagcgtgacgggcagcgaccagcgatgatcggcacccaccagccaacgcgccatatgcggcatcatcaggccaataaaggcaatcgggccaactattgccgtcgcactaccacaaagcacggtaatcgccagcagaccaatcaactgtgtgcgcgccacgcgactgcccagcgccgtcgcggtgtcgctgccgaggctcaaactgttcagcgcgcgactcagtaatagcgcagttgctccggcgatcagcaccgggatcagcaccacttttaaggtatgtagattgcgaatatccagcgaaccggcttgccagaaacgcaactgatcgtagacgtcaggattaagcagggcgatgccgctggtcagtccttccagcaccgccgccagcgccacgcccgccagggttaaacgcaccggacttaactgcccgccgccctgactgccggtaaaggcaacaatcaatgaggccaccagcgccccggcgaaggccatcgccagttgttcctgcgcggaagagtaaccaaacagcgccgcacccagcacaatggcaaagctggctccggcgttcacgccaagcaagccggggtcggcaagtgggtttcgggtgagggtttgcattaacgccccggcaaggccaagcgcgccgcctgccagtaaaccggcaagggtacgcggcagccgcgcgtcgagcacgatggtgcagtcggcgctctggcaggtgccggagaaggcctccagcactacggaagcggggagtgattttgccccaatgagcaggcttaatgccgtcgcgataatcagtaataacagcaatccgggcacggcaatggcgcgtgtcacggcaacagaaccagacatacgaacttccatgataatgaaattaattatcgttatcgatcttatttggatatgttagcatgtgcagcctaagaataggtatttaaaatatttgatggcaaggcattgtaatgaataaacaatcctggctgcttaacctcagcctgttgaaaacgcacccggcgtttcgcgcagtattcctcgctcgtttcatctcaattgtgtctctgggtttgctcggcgtcgcggtgccggtgcagatccagatgatgacacattccacctggcaggtggggctttcggtgacgctgaccggcggcgcgatgtttgttggcctgatggtcggcggtgtgctggcggatcgctatgagcgcaaaaaagtgattttgctggcgcgcggcacctgtggcattggcttcattggactgtgccttaatgcactgctgccggagccgtcattgctggcaatctatttacttggtttatgggatggttttttcgcatcgcttggcgttacggcgctattggcggcgacaccagcactggtagggcgtgaaaacttaatgcaggccggggcgatcaccatgttgaccgtgcgtctggggtcggtgatttcgcccatgattggcggtttattgctggcgaccggtggcgtagcctggaactacgggctggcggcggcgggcacgtttattaccttgctaccgttgttaagccttccggcgttgccaccgccaccgcagccgcgtgagcatccgttgaaatcattactggcaggatttcgttttctgcttgccagcccgctggtgggcgggattgcgctgctgggtggtttattgacgatggcgagcgcggtgcgggtactgtatccggcgctggctgacaactggcagatgtcagcggcacagattggttttctctacgcggcgatcccgctcggcgcggctattggtgcgttaaccagcgggaagctggcacatagtgcgcgaccagggttattgatgctgctctccacgctgggatcgttcctcgccattggtctgtttggcctgatgccgatgtggattttaggcgtggtttgtctggcgctgttcggctggttgagtgcggtcagctcgttgctgcaatacacaatgctgcaaacgcaaaccccggaagcgatgttagggcggattaacggtttgtggacggcgcagaacgtgacgggcgatgccataggcgcggcgctgctgggtggtttgggcgcgatgatgacaccggttgcttccgcaagcgcgagcggttttggtttgttgattatcggcgtgttgttattgctggtgctggtggagttgcgacattttcgccagacgccgccgcaggtgacagcgtccgacagttaatgcttaaaacagcgccttaagcctatccagcacttgcatggcgctgtagtaatccagacggaacgtctcggttcccagcgcataaacctgcttgttttgtactgcaggcaggtgcgcgagcagcggattagcataaatagcatcggcatctttctgatcaccggcgaacaggaatagtgactcgccatttaaccctgcagccagattttccccaccaagctgaatgatgtcatggcgtttaccctgactttggctggcatttaaccctgcgggtaacttcgccagcgtaaagccgagttgttccagcatctgcccttgtgctgattctggcgtccagagattggcactgtgtgcagcggcagtatagacaatggcagtgaccggctgcggcggtaatttgatttgctctttcgccgccgccagttgcttatcaaactgcgcaatccgctctgccgcttgtttctcatgcccggtaatttcgccaagttgcgttaacagcgactgccagcttttgtcgtcgtaattgatgattaatgtcggggcgatggtggaaagctgatcatacagtgccagcgccgaatccccgccggttgcgctaattaaaatcagatccggcatttgcgcggcaacggcttcggcgctcggttcgccgatatagagccgttgcagtttgcgttctttcgccaccttgctccactggcgtaaaaagccctggtcatccgcgacgcggttattcggcgtggtcgcgccgctggcgatcaccggagcatcaatcgccagcagtgagccggtcagggtgacgctggtggaaacaatacgctgcggctggctttccagtgtatgtgtgccacggctgtcagtaatctgacgcggccagtcagcggcctgaactgcggctattcctgaaagcaaaagtcctgttaatagaagggcgttgcggtagagcggggcgagtctcacaaatcagcttcctgttattaataaggttaagggcgtaatgacaaattcgacaaagcgcacaatccgtcccctcgcccctttggggagagggttagggtgaggggaacagccagcactggtgcgaacattaaccctcaccccagccctcaccctggaagggagagggggcagaacggcgcaggacatcacattgcgcttatgcgaatccatcaataatgcttctcattttcattgtaaccacaaccagatgcaaccccgagttgcagattgcgttacctcaagagttgacatagtgcgcgtttgcttttaggttagcgaccgaaaatataaatgataatcattattaaagcctttatcattttgtggaggatgatatggatacgtcactggctgaggaagtacagcagaccatggcaacacttgcgcccaatcgctttttctttatgtcgccgtaccgcagttttacgacgtcaggatgtttcgcccgcttcgatgaaccggctgtgaacggggattcgcccgacagtcccttccagcaaaaactcgccgcgctgtttgccgatgccaaagcgcagggcatcaaaaatccggtgatggtcggggcgattcccttcgatccacgtcagccttcgtcgctgtatattcctgaatcctggcagtcgttctcccgtcaggaaaaacaagcttccgcacgccgtttcacccgcagccagtcgctgaatgtggtggaacgccaggcaattccggagcaaaccacgtttgaacagatggttgcccgcgccgccgcacttaccgccacgccgcaggtcgacaaagtggtgttgtcacggttgattgatatcaccactgacgccgccattgatagtggcgtattgctggaacggttgattgcgcaaaacccggttagttacaacttccatgttccgctggctgatggtggcgtcctgctgggggccagcccggaactgctgctacgtaaagacggcgagcgttttagctccattccgttagccggttccgcgcgtcgtcagccggatgaagtgctcgatcgcgaagcaggtaatcgtctgctggcgtcagaaaaagatcgccatgaacatgaactggtgactcaggcgatgaaagaggtactgcgcgaacgcagtagtgagttacacgttccttcttctccacagctgatcaccacgccgacgctgtggcatctcgcaactccctttgaaggtaaagcgaattcgcaagaaaacgcactgactctggcctgtctgctgcatccgacccccgcgctgagcggtttcccgcatcaggccgcgacccaggttattgctgaactggaaccgttcgaccgcgaactgtttggcggcattgtgggttggtgtgacagcgaaggtaacggcgaatgggtggtgaccatccgctgcgcgaagctgcgggaaaatcaggtgcgtctgtttgccggagcggggattgtgcctgcgtcgtcaccgttgggtgagtggcgcgaaacaggcgtcaaactttctaccatgttgaacgtttttggattgcattaaggagcgaggatgagcattccattcacccgctggccggaagagtttgcccgtcgctatcgggaaaaaggctactggcaggatttgccgctgaccgacattctgacgcgacatgctgcgagtgacagcatcgcggttatcgacggcgagcgacagttgagttatcgggagctgaatcaggcggcggataacctcgcgtgtagtttacgccgtcagggcattaaacctggtgaaaccgcgctggtacaactgggtaacgtcgctgaattgtatattacctttttcgcgctgctgaaactgggcgttgcgccggtgctggcgttgttcagccatcagcgtagtgaactgaacgcctatgccagccagattgaacccgcattgctgattgccgatcgccaacatgcgctgtttagcggggatgatttcctcaatactttcgtcacagaacattcctccattcgcgtggtgcaactgctcaacgacagcggtgagcataacttgcaggatgcgattaaccatccggctgaggattttactgccacgccatcacctgctgatgaagtggcctatttccagctttccggtggcaccaccggcacaccgaaactgatcccgcgcactcataacgactactactacagcgtgcgtcgtagcgtcgagatttgtcagttcacacaacagacacgctacctgtgcgcgatcccggcggctcataactacgccatgagttcgccaggatcgctgggcgtctttcttgccggaggaacggttgttctggcggccgatcccagcgccacgctctgtttcccattgattgaaaaacatcaggttaacgttaccgcgctggtgccacccgcagtcagcctgtggttgcaggcgctgatcgaaggcgaaagccgggcgcagcttgcctcgctgaaactgttacaggtcggcggcgcacgtctttctgccacccttgcggcgcgtattcccgctgagattggctgtcagttgcagcaggtgtttggcatggcggaagggctggtgaactacacccgacttgatgatagcgcggagaaaattatccatacccagggttacccaatgtgtccggatgacgaagtatgggttgccgatgccgaaggaaatccactgccgcaaggggaagtcggacgcctgatgacgcgcgggccgtacaccttccgcggctattacaaaagtccacagcacaatgccagcgcctttgatgccaacggtttttactgttccggcgatctgatctctattgatccagagggttacatcaccgtgcaggggcgcgagaaagatcagattaaccgtggcggcgagaagatcgctgccgaagagatcgaaaacctgctgctgcgccacccggcggtgatctacgccgcactggtgagcatggaagatgagctgatgggcgaaaaaagctgcgcttatctggtggtaaaagagccgctgcgcgcggtgcaggtgcgtcgtttcctgcgtgaacagggtattgccgaatttaaattaccggatcgcgtggagtgtgtggattcacttccgctgacggcggtcgggaaagtcgataaaaaacaattacgtcagtggctggcgtcacgcgcatcagcctgaaggagagaacacgatggctattccaaaattacaggcttacgcactgccggagtctcacgatattccgcagaataaagttgactgggcctttgaaccgcaacgtgccgcgttgttaatccatgatatgcaggactattttgtcagcttctggggcgagaactgcccgatgatggagcaggtgatcgcgaatattgctgcgctgcgcgactactgcaaacagcacaatatcccggtttattacaccgcccagccgaaagagcagagcgatgaagatcgggcgctgttgaatgatatgtgggggccgggcctgacccgctcgccggaacagcaaaaggtggtggatcgcctgacgccagatgccgacgacacggtgctggtgaagtggcgctacagcgcgtttcatcgttctccgctggagcaaatgctgaaagagagtggacgtaaccagctgattattaccggggtatatgcccacattggctgtatgaccaccgcaaccgacgcatttatgcgcgatattaaaccgtttatggtggcggatgcgctggccgatttcagccgtgacgagcatttgatgtcgctgaaatatgtggccggacgttctggccgggtggtgatgactgaagaattactgccagcacctatccccgccagcaaagcggcgctgcgtgaggtgatcctgccgttgctggacgagtccgatgaaccgttcgatgacgacaacctgatcgactacggtctggattcggtgcgcatgatggcgctggcggcgcgctggcgcaaagtgcatggtgatatcgactttgtcatgctggcgaaaaacccgaccatcgacgcctggtggaagctactctcccgcgaggtgaaataatggatttcagcggtaaaaatgtctgggtaaccggcgcaggtaaaggtatcggctacgccacggcgctggcgtttgttgaggcgggagcgaaagttacaggttttgatcaagcgttcactcaggagcaatatccctttgcgaccgaagtgatggatgttgccgacgctgcgcaggtcgcgcaagtgtgtcagcgactgttagctgaaacggagcgactggacgcgctggtcaatgcggcgggaattttacgcatgggcgcgaccgatcagctcagtaaagaggactggcagcagacttttgcggttaacgtcggcggtgcgtttaacctgttccagcaaaccatgaaccagtttcgccgtcagcggggcggggcgattgtcactgtggcgtccgacgccgcgcacacgccgcgtattggcatgagtgcttatggcgcatcgaaagcggcgctgaaaagcctggcgttgagcgtcgggctggaactggcgggtagcggcgtgcgctgtaatgtggtttcgcctggctccaccgacaccgatatgcaacgcacgctgtgggtgagcgatgacgccgaagaacagcgtattcgcggctttggcgagcagtttaaactcggcattccgctggggaaaatcgcccgtccacaagagatcgccaacacgattttgttcctcgcctctgacctcgccagccatattaccctacaggatattgtggtcgatggcggctcaacgctgggggcataagcatgatctggaaacgccatttaacgctcgacgaactgaacgccaccagcgataacacaatggtggcgcatctgggaattgtgtatacccgtctgggcgatgatgtgctggaagccgaaatgccggttgatacccgtactcatcagccgttcggtttactacatggcggcgcgtcggcggcgctggcggaaacgctgggatcgatggccggatttatgatgacccgcgacggacagtgtgtggtaggcacagaacttaatgcaacacaccatcgcccggtgtctgagggaaaggtacgcggcgtctgccagccgctgcatcttggtcggcaaaatcagagctgggaaatcgtcgttttcgatgaacaggggcggcgttgctgcacttgtcggctgggtacggcagttttgggatgaacccgacagaattagatgagattgcaggaaaactcggttaacggagtgatcgagttaacattgttaagttaaatattggtttcaactccgatttacatggttgctgtgttgttaaattgtacaaagatgttatagaaacaaaatgtaacatctctatggacacgcacacggataacaactatgaacaaatcagggaaatacctcgtctggacagtgctctctgtaatgggagcatttgctctgggatacattgctttaaatcgtggggaacagatcaacgcgctgtggattgtggtggcgtcggtctgtatctatctgatcgcttaccgtttttatgggctgtatatcgccaaaaatgtgctggcggttgacccgacgcgtatgacgccagcggtgcgccataacgacgggctggactatgtgccgacggacaagaaagtgctgttcggtcaccattttgcggccattgccggagcaggtccgctggtggggccggtactggcggcgcaaatgggctacctgccggggatgatctggctgctcgctggggtggttctcgccggtgcggtgcaggatttcatggtgctgtttgtttctacgcgccgtgacggtcgctcgctgggtgagctggtcaaagaagagatggggccaaccgccggggtgattgcgctggtggcctgctttatgatcatggtcattatccttgcagtgctggcgatgatcgtggtgaaagccctgactcatagcccgtggggaacatataccgttgcgttcaccattccgctggcgctgtttatggggatctacctgcgctatctgcgtccggggcgtattggcgaagtgtcggtcatcggtctggtattcctgattttcgccattatctctggcggctgggtggcagaaagtccgacctgggcaccgtactttgactttaccggcgtgcagttgacctggatgctggtgggttacggttttgtggcggcggtgctgccggtgtggttactgctggccccgcgtgactacctctctaccttcctgaaaatcgggactatcgtcggtctggcggtaggcattttgattatgcgcccgacgctgaccatgcctgcgctgaccaaatttgtcgatggcactggcccggtatggaccggtaacctgttcccgttcctgtttatcaccatcgcctgtggcgcggtgtctggcttccatgcgctgatctcttctgggaccacgccgaagatgctggcgaacgaagggcaggcgtgctttatcggctacggtgggatgttaatggaatccttcgtggcgattatggcgctggtttccgcctgtatcatcgatccgggcgtgtattttgccatgaacagcccgatggcggtgctggctccggcagggacggcggatgtggtcgcttctgccgcgcaggtggtgagtagctggggctttagcattacaccagatacgctaaaccagattgccagcgaagtgggtgaacagtcgatcatttcccgtgcgggcggtgcgccgacgctggcggtggggatggcctacattctgcacggcgcgctgggcggcatgatggatgtggcgttctggtatcacttcgccattttgtttgaagcactgtttattctgacggcggtggatgcaggtacgcgtgctgcgcgctttatgttgcaggatctgctgggcgtggtgtctcctggcctgaagcggaccgattcactgcctgctaacctgctggcaacagcgctgtgcgtactggcgtggggctacttcctccatcagggcgtggtcgatccgctgggcggcattaacactctgtggccgctgtttggtattgccaaccagatgctggcagggatggcgctgatgctctgtgccgtggtgttgttcaagatgaaacgtcaacgttacgcctgggtggcgctggtaccaacggcctggctgctgatttgtaccctgaccgcaggctggcagaaagcgtttagcccggatgcgaaagtcggcttcctggccattgctaataagttccaggcaatgatcgacagcggcaatattccgtcgcagtatactgagtcacagctggcgcaactggtgttcaacaaccgtctggatgccgggttaaccatcttctttatggtggtcgtggtggttctggcactgttctcgattaagacggcacttgcggcattgaaagatccgaagccaacggcgaaagaaacgccgtatgaaccaatgccggaaaatgtcgaggagatcgtggcgcaggcaaaaggcgcacactaaagtcagagtgagggggggatgttggcgaatgttggcttagtgcccagggttccctctcaccctaaccctctccccggtggggcgaggggactgaccgagcgcgttgatagcatttgtaggccggataaggcgttcacgccgcatccggcactctttcagcaacatggttagcggaggccaagatgtttgattcactggcaaaagccggaaaatatttaggtcaggcggcgaagctgatgattggtatgcctgattacgacaactatgtcgaacatatgcgggttaaccatcccgatcaaacgccgatgacctacgaagagtttttccgtgagcggcaggacgcgcgctacggtggaaaaggcggcgcgcgctgctgctaaatttgtacgtcaggctttaaacgattccacttttttgaacgctgcacgcaacgtatctggtgtcagcgtgactggcaggtaatgaatggactccaccggacgcagggtgtgggcaatcactttgtcgatctccgcctgattattgatatccacttccagctccgccagtgtagtcggcagatgaaaacgctgatacgctccagttaattgcgccagcacatcatcctgacccagcaaggcgctttgcaccagaattccgtaggcgactttggtgccgtggagaaacttctcggtttgcggcagcacggtcagaccgttatgcacggcatgagctgccgccacacgcgtaaaacgatcgcccagaccaccaaccatcccaccaccagcaataatagcatccaccacatcgcaaaatgattgcgttaactgttgattttgctgatcgctcagcgcctgttcgctactgtttaacaagacgtcgcgaatggcttgcgcattattgatccccagtcgcacggttagcggcaacgtttctggttgcggagccagcaccaccgcttcataccatttcgccagcgtgtcaccgatccccgccagcagatattgttgcggtgcattgaggataatctccggttccaccagcaccataaaattggcgtcgtcgaaaatctcataatgcagcgcctgtccggcatcattataccagacggagagcggtgtccaggcggcgcaggtggcggcgatcgtcggaacggcaacaaacggcagaccgagacggcgggcgagggctttcgcggtgtcgagcagtgcaccgccaccgacgccaatcaccacgctgcggtcgtcaccggactcagccgccagttgttgtacatcgctttcgctgcaatgaccgcgaaacaaaatatgctttgcccctggcagtccaaacgctggcggaagtttggtttgcgccgcagcaatggcgcgtttgccgtagatccacaccgcgcgagaaagttgttcatcagtgaaaaaatcgtgcaggtgattgaaacttcctggatgtgaaaagtagttagccgggccgacgaccacgcggataggattgtgaggcatgttgtgttgtccttattgttttatttagacatctaaacgtcttgattgccaaatactagcatcgtgttatagtgccttcaacacgcaacttcgtcaggtacaataaaaatgacaaataaccctctgattccacaaagcaaacttccacaacttggcaccactattttcacccagatgagcgcgctggcgcagcaacaccaggcgattaacctgtcgcaaggctttcctgattttgatggtccgcgctatttacaggagcggctggcgcaccacgttgcacagggggcaaaccaatacgcgcccatgaccggcgtgcaggccttgcgcgaggcgattgctcagaaaacggaacgtttgtatggctatcaaccagatgccgatagcgatatcaccgtaacggcaggggcgacggaagcgttatacgcggcgattaccgcactggtgcgcaatggcgatgaagtgatttgttttgatcccagctatgacagttacgcccccgccatcgcgctttctgggggaatagtgaagcgtatggcactgcaaccaccgcattttcgcgttgactggcaggaatttgccgcattattaagcgagcgcaccagactggtgatcctcaacactccgcataaccccagtgcaactgtctggcagcaggctgatttcgccgctttgtggcaggcgatcgccgggcacgagatttttgtcattagcgatgaagtctacgagcacatcaacttttcacaacagggccatgccagtgtgctggcgcatccgcagctgcgtgagcgggcagtggcggtttcttcatttggcaagacctatcatatgaccggctggaaagtgggttattgtgttgcgccagcgcccatcagcgccgaaattcgcaaggtacatcagtatctgaccttttcggtgaataccccggcacagctggcgcttgctgatatgctacgtgcagaacctgagcattatcttgcgttaccggacttttatcgccagaagcgcgatattctggtgaatgctttaaatgaaagccggctggagattttaccgtgtgaaggtacatactttttgctggtggattacagcgcggtttctaccctggatgatgttgagttttgccagtggctgacgcaggagcacggcgtagcggcgattccgctgtcggtgttttgcgccgatcccttcccacataaactgattcgtctctgttttgccaagaaggaatcgacgttgctggcagcagctgaacgcctgcgccagctttagctatttaaccgtccaggcgcgggaatattgacggtcggcaaacaactcttgcaggccgttaatttgcttcaggcgcagcacttcgtcgctgtccattcccagctctttgccaattttattatcgtcccatcccaactggctaagttcacggacgatttccgacatggcggtgatttgatggcgtccacgagcgcgattatgacgaatagtcgcggcgatgcgttgattacgcgtaccttccagacaggtcaccggcaaataaccttttaagcgtaattttaatgatgatgagcctttaccaatttcatggcggtgaaaaccatccacgatttccatggcatttttatccgtatgtgtgaccacaatgggttgggtaaaaccatctatttcaatggatttttgcagcagttttttttcgggtggtgccacgttgtttgggttgtaatcattaggcataagttggctgtttttaacccacagaacgcaatccactggctcttcacgaaaggggctaacctgatggatcgccatgcggatttcattaatcgctttgatgcgatcatcttccggcaagctggcgagaaattgcgttaaatcctgcgttaatcgttgttgcatagtatcccccattcctgacgttttccttttatccgttcgttataacgctgatagttcttcgattttgtggggctaaatgataatgcccgacaccagtaatcgttattgagtaaaactttgcatatccgccgccaggaggggatatctttcgcgccaatgtccccttgctgggtttgtggaacctcgatgccttttttctgataccagtgcaaataaatggcgattttattgcggtaatgctcagctgttttttccggcatgctattgagcagcaataatgcatattcttgccagtctaaatgttctggcttgaggattttccgatgcccatagaaatgattgtcatgtccggcgtaaatgccgccactttttaccccgctgactcgtgcgcacatagcagcccagcgatccggttcgataacgtgatagagccataatccttgtcgttgctccgggccaaaaggttcgcaaattcgcatatgacgcagaggaacgcctgcctgatacattaggttatacagtgggttgcagagactttgatgatttgcataccaggtccagatatcagccactttccagtcgtaaatggggtaaatgtaccagctatgaccgcctggtgcggccgtagtccagggtttatcgtcggcaaaacgttgtttatttaaactggcgatggcgacaaaacggttgtaggactcatccgcacggatgccgatcatcatcgccgccggacgtttttgtgaaaaccattcggcaaactcacgtacaaattgttcgaaggtcatgcctggctggtaaaagcagaaaaagtcagggtcggttatcgcatcttggggaggttgacgtacccattcgacatcaggttcccagcactgccattcgggttggtattgtgaaagggaattttgcgtcgtaagcgggagcgcaacccagtaaaactcttcgatgacatcggtgtacaactcgcgcagggactgaacatagttaatggtgcaagagaattgcgcctcccagtcgataaacaaaacgcagatttttttgcccatttgtcgggcaagttcggctgtcagatgcagcattaaaccagagtctttgccgccagaaaatgagacacaaacgcggggtagggtgttgagtgtccaggtaatacgctctcgtgcagcttccagaatattgagcggaagaggaattttataaatagacatctgaagacgctctctgaacgttacagggtgatcagtgagataagtctgttaattataaagtaaacactgtaaagcagagtgttttatttttcattcgcgctgtgaataaatagatgaaagttatagtagctgtctgtagttatatatcaaaaactctcatttagacggtcaataaatcgggagaacaccaaattatttaaagaagatttattataggaaatgtaaagctttattgaaggtaacggatgttctagttttatctcttttaagttaagaaagtcacggtaggaattataaagttcataggggactattcccagtaaatctgtaactgcaatgctattaatgattgtcagcaaagaggaaccacgaaatgagattttgcgattcataaatctctcgtctatttccatttgaatatcatcaacccctgctgatttagatattaattgggtgaactcttctgccataatttgttcataagtgctattgtcagtaattcgtggatgcctattactacaaattagagtattgcgaatcgtatgcaatggcatgcaaatgacggaacggctgatcactggcatttgggtgatcaccagatcggctttgcggtgaaccaacagttcttcagcattctctgctgacatgaggatatcatggcactcaatctcgacagaggaatcttgccgtaggcagcggatcagcatactattattagagcaagaaatgagctgagggccgtagataataaagtttttctttagttcggacttattgactatattaattgtttgttcaaggcctctgagatttttctcaagatggtgatgcagatttaaccctgttgtcgtcggcgcgataccttttcctgagcgaatgaataaagggtcattaaattgcgcacgtaagcgttgtaacgactggctcacggctgatggggtgatatatagtgattcagcagctttgctaatgcttaaatgctggtaaatacactcaaatatgacaagaagatttaagtcgaactttttcaagtcgtagagattggccatacactactccggttatatttttcttccatgatatattcacttaatcaatgttttttgcgtatatatttttattgattatgtttttttgcttaactcaggattaagtttttctaaaatagcacagccacttagggcagagcgagcaattcatgcttttttaggatggttgaaaagcagggatatagttcaaccatccatgaattaccttttatttattccccataatgatattaagcgttttctgatcgggcaaccccacggcctgttgtagcgtattttccttactcatgtaatagatagccggcgtgacatttgcccccagatcgtccatcagtttctcattgtcacttaacactttcatttgctctgtacttacgtttgcaggcacgtttagcttaagcttgccaccagaggcttcatattgttgccaggtttttgcgggatctttggaggcaagaattgccgctgctgtcgccgggctttctggcttgataaccccaaccaacaatgttcttaattgcactttgccagaatctacccacgggcgcgcctgctgccagaactgtttacaatatgggcagaacggatcggcgaagacgtagacaatgaccggcgcatcttttttaccgtcgaggagccagtgggattgttccatccgttgccacatttcgcgtccggctggtgcgtaaatttctttttcgataagtgtgttactcaggttttcacctttctcgttgtacatgtaaccagagatagcgtgcttaccatctggagtcaggtagatggtgacgcccatatcctgatactttccgagataacctttcattcctccgggggcatcgaatgttttgatgattgtaatgccctgtttttcaatcgcttttactggagcaggaagttcctctgcgaaggcgattgcaggaagcagagccagtaaaagtatcttttttaacattaatttgtccttttcagtcagtgcaaaagtcgagtaaaaggcataacctatcactgtcataggtaagagcttagatcaggtgattgccctttgtttatgagggtgttgtaatccatgtcgttgttgcatttgtaagggcaacacctcagcctgcaggcaggcactgaagataccaaagggtagttcagattacacggtcacctggaaagggggccattttactttttatcgccgctggcggtgcaaagttcacaaagttgtcttacgaaggttgtaaggtaaaacttatcgatttgataatggaaacgcattagccgaatcggcaaaaattggttaccttacatctcatcgaaaacacggaggaagtatagatgtccttgattaacaccaaaattaaaccttttaaaaaccaggcattcaaaaacggcgaattcatcgaaatcaccgaaaaagataccgaaggccgctggagcgtcttcttcttctacccggctgactttactttcgtatgcccgaccgaactgggtgacgttgctgaccactacgaagaactgcagaaactgggcgtagacgtatacgcagtatctaccgatactcacttcacccacaaagcatggcacagcagctctgaaaccatcgctaaaatcaaatatgcgatgatcggcgacccgactggcgccctgacccgtaacttcgacaacatgcgtgaagatgaaggtctggctgaccgtgcgaccttcgttgttgacccgcagggtatcatccaggcaatcgaagttaccgctgaaggcattggccgtgacgcgtctgacctgctgcgtaaaatcaaagcagcacagtacgtagcttctcacccaggtgaagtttgcccggctaaatggaaagaaggtgaagcaactctggctccgtctctggacctggttggtaaaatctaaatttccttcgtctttcacgccatagcggcgttggcgtcgcccgctcaccccggtcacttacttgtgtaagctcccggggattcacaggctagccgccttgctctgacgcgaaatacttcggaaattcacctaattcttcgggtgctgcggcacccgattttcttccccgcaccatgatgcaagctgcatccaggtagccgcagaggccgcttgcatgatgatgtttaaagcccaggagataaacatgctcgacacaaatatgaaaactcaactcaaggcttaccttgagaaattgaccaagcctgttgagttaattgccacgctggatgacagcgctaaatcggcagaaatcaaggaactgttggctgaaatcgcagaactgtcagacaaagtcacctttaaagaagataacagcttgccggtgcgtaagccgtctttcctgatcaccaacccaggttccaaccaggggccacgttttgcaggctccccgctgggccacgagttcacctcgctggtactggcgttgctgtggaccggtggtcatccgtcgaaagaagcgcagtctctgctggagcagattcgccatattgacggtgattttgaattcgaaacctattactcgctctcttgccacaactgcccggacgtggtgcaggcgctgaacctgatgagcgtactgaacccgcgcatcaagcacactgcaattgacggcggcaccttccagaacgaaatcaccgatcgcaacgtgatgggcgttccggcagtgttcgtaaacgggaaagagtttggtcagggccgcatgacgttgactgaaatcgttgccaaaattgatactggcgcggaaaaacgtgcggcagaagagctgaacaagcgtgatgcttatgacgtattaatcgtcggttccggcccggcgggtgcagcggcagcaatttactccgcacgtaaaggcatccgtaccggtctgatgggcgaacgttttggtggtcagatcctcgataccgttgatatcgaaaactacatttctgtaccgaagactgaagggcagaagctggcaggcgcactgaaagttcacgttgatgaatacgacgttgatgtgatcgacagccagagcgccagcaaactgatcccagcagcagttgaaggtggtctgcatcagattgaaacagcttctggcgcggtactgaaagcacgcagcattatcgtggcgaccggtgcaaaatggcgcaacatgaacgttccgggcgaagatcagtatcgcaccaaaggcgtgacctactgcccgcactgcgacggcccgctgtttaaaggtaaacgcgtagcggttatcggcggcggtaactccggcgtggaagcggcaattgacctggcgggtatcgttgagcacgtaacgctgctggaatttgcgccagaaatgaaagccgaccaggttctgcaggacaaactgcgcagcctgaaaaacgtcgacattattctgaatgcgcaaaccacggaagtgaaaggcgacggcagcaaagtcgttggtctggaatatcgagatcgtgtcagcggcgatattcacaacatcgaactggccggtattttcgtccagattggtctgctgccgaacaccaactggctcgaaggcgcagtcgaacgtaaccgcatgggcgagattatcattgatgcgaaatgcgaaaccaacgtgaaaggcgtgttcgcagcgggtgactgtacgacggttccgtacaagcagatcatcatcgccactggcgaaggtgccaaagcctctctgagtgcttttgactacctgattcgcaccaaaactgcataagaagaagtaagattcacctgcaattgcttagccgccggggtcaaacctggcggcttttttatggcattaaaaagccccgccgggatggctccgggcagggcgggatacttattctggcaattaacgcacaaccagcaccggcagattggcgtggcggatcacgctcgaggcgttagaacctaacagatgggtcgaaatcgatgggttgcgagaaccaataactacaacatcagcccccagttcttctgccaactcattgacttcatcccgcacgctaccaaaacggacatgttgtttaatgcgggaaggatcgatggtgaagtggctgaccatcgtttgcagacgttcttgtgcttcatgttgcagatgctcttcaaaacgacgcacatcagcggcaaaacggtgcaggctcaggctggctgacccgggtagtacgtgaagtagatgaataactccgtcatcctgggcgaggaattcagcgtggcgaacagctttgtcgctcaattccatttcaaatacatcaactggcataatgattgtcttatacataaccctttctccctgttaatcatgaacaaatcattcgccatgattataatatttatccctgatatttgtctggttctttttccttacgaactgtttctgtgatgaatatattctcactgaacaccaggaattctcccaaaacctgtggtaccgcccgttttcccgctgtgatagctacccttaaagactgactcttttttgaactgtctctggaggttgcatgaaagcattgacttatcacggcccacatcacgttcaggtagaaaatgttcccgatccgggcgttgaacaggcagatgatattattctgcgtattacggcaacggcgatctgtggctctgacctccatctttatcgaggcaaaatacctcaggttaaacatggcgatatttttggtcatgaatttatgggggaagtagttgaaaccggaaaggacgtaaaaaatttgcaaaaaggcgaccgagtggtaattccgttcgtcattgcttgtggcgactgttttttctgtcgattgcaacaatatgccgcctgcgaaaataccaatgcgggtaaaggcgctgcgctcaataaaaaacagataccagctccagcggcattgtttggttatagtcacctgtatggcggcgttcctggtgggcaggcggaatatgtccgcgtccctaaagggaatgtggggccgtttaaagtaccgcctttgctttcagatgataaagcgcttttcctttctgatattctgccaacggcatggcaggcagcaaaaaatgcgcagatccaacaaggttcaagcgttgcagtctatggtgctggtcctgtgggattgttgacaatcgcctgtgcacggttgctcggtgcggaacagatttttgttgttgatcatcatccctaccgcttgcatttcgccgccgaccgctacggcgcgatcccgattaattttgatgaagacagcgatccggcacagtcaattattgaacaaacggcaggtcaccggggcgtggatgcagtaatagacgccgtcggttttgaagcgaaaggcagcaccacggaaacggtgctgactaacctgaaactggagggcagcagcggtaaagcgttgcgtcagtgtattgcggcggtcaggcgtggcggcattgttagcgtaccgggcgtctacgctggatttattcacggtttcctgtttggcgacgcctttgataaagggttgtcgtttaaaatgggacagacccacgttcacgcatggctgggagaattattaccgttaattgagaaaggattactgaaaccagaagaaattgttacccactatatgccgtttgaagaggccgcccggggatatgagattttcgaaaaacgtgaagaggagtgccgtaaggtgattctggtacccggtgcacaaagcgcagaggcggcgcagaaggcggtttcaggtctggtgaatgcgatgccggggggaacaatatgatcgtcaggagtggttttcgaggtaaaggacagccatgacgataatcgccgccataatcagaaatcctatcaggatgtaaaatgcttctgccatggttattcccacaaacgaaacggaataattttgcagcaaaagtgaacagtgagaaccaggaaaaattgctgattttgcgtaaagaggatgcgagtgcatcctctgggcaaagcgagttatcgcttgtgcagatgggattaaagcaggtagtcgccagcagcttctggctggtattcgagttccagcacttcaaggtgggttgcaacgccgcccggaagttcccagtgaatggaatcgccaacgcgcagccccagcagtgcggcacctaccggagccataacggaaagctgagtattgctatcggtcatttttgccggatacaccagcgtgcgcacacgcacttcgccatcgctaagattgcggaatttaacccggctgttcattgtcaccacgtcgtgtggcatctcttctggcgaacacatttgggcgcgatccaactctgcgtttaacgcgtcggcgattggcaaaccagcataggcgggttgctccagcagaatatcgatgcgttcggcatccaggtcgttaatgatgatagttggtctggacatttttactccatgtcgtcggtgctgcgagtgtcgcagataaacatacccaaaagaaaaccctcaccgtcaggcggcgagggtttaactcacatgatgatactgactgttgctcactctttgaagtgatttgcgtcacattcagggaattcctcaatgcagcgcattatgtataaatcttaatcgccttggtttatggaagacgaattagcgtgttttgtaaatcagatgattaataacccgctttatcaatcacaaaggttttgccacagttacctgggtgaggttgtggcaagaatgagtttgcagaaagcggagcgttgatggcgtcagctttgatcgagatctgaatttcagtcaaatacgcagggttaccctggcacgttagcttaactgctttcacgttctcttttccccagcttttggcaaaggcggcgtcaaagtcacggcggctcactgttttaccgtaattatccgcaaggaattttccggcttcgctctctttaatttcttgattcaggcgtaccatcgtaccgaagtatgcgtccggatcaaaaccaaagcaggcaccgtgtttggcatattcgtagcgttccaggcaggaacgtccgccagctcctggcatgacttcacttagtttagcggccgtttccagtgataatccggtttccggcgatgaacacattcggctggcgcgcgcttctggtagattcgggattgggcgagtagcgcaaccgaagcgcatccagcggcgttcatcaacaccacgggcagcaaccgatttaggcaatcctggccacagaccatgtacggtcagaaaatcagctttgttggtcgtttcggtttgcaggcgacattcatctcgttcgttacgatttcgatcgtgttgactctggcaaaatccggtttgccaggagagggccaggacatagcgatcaaaatcgccatactgttttgcctgcaacgctaaggcgttggcagaagagaagggaagcagagaaaccgcgagcaacgcggcgttacgccagaatgctttcataatgggtgtggaactcatacatacactgaatactatctattaaatcataaaaaagcccgccaggtgggcttacctggcgggcgtgatgatttattcagcgtttggcgaacgtattagttccacatggcgagaatcggccagccaaccaacagcaacatagagatgtaaatcaccccgaagattgcgccaagacgccagtaatcttttgatttcacatagccacagccgtaaataatcaccccaggaccggttgcatacggcgtcagacagcccatgataccgatagacagcaccagcaggatacacagttgttccattggtacgcccggaatacctttaccgacggccagaataaccggcagcatggttgcggtgtgcgcagacaggctggcaaacaggtagtgtgcaaagtagaacaccagaaccagtacaatcaccgttgcgtttggtgagaatccttccaggtgcgtactcatggtaccggcgaaccagtcaataaaaccagaacgagtcaggccgttagccatcacaaccagagttgccaggttgaccagtgtgttccatgcgctgttatagcgggtaatgtctttccaaggcacaacgtgcagggccagcattagcgaaactgccagcagaccaaccgcagtagcattaatgacttcactgccaaatacccacaaacctaagctgagcaatacaaggccaatcagtgtccactctctgcgtgtcagcgcacccatggttttcagttcatcacccgcccaggttgccacttcttcactgtgtgtgatttccggtttgtacagcacgtaggaaagccacggcgcaatgataagcaagataaccccaaccggcaggaagcagaggaaccactgcaaccagctaatctggataccggcaattttgctgacgaactccagacccagcacgtttggtgccgcaccggtgacaaacatggacgaactcagactggtactaatgaccatcatccacatcaaatagccgccaatacgacgcgcggacggatcgttcgggaatgatttaaacaacggcggcaggtttttaatgaccggaaaaaccgtacccccggtacgcgcggtgttggaaggtgtaaacggtgccagcagaatgtcgataatgacaatcgcataacccaacgtcagcgtgcgtttgcccatgaatttcaccaggaaaagggcaatgcgacgacctaacccggaaacttcataccctaatgcaaaaataaatgcgccaaataccagccataccgtggtgctggaaaaaccagccaggccccatttcagcgcctgtttttgcgcattaaacgctgggtcagctaattctttggcatcaaagagcaggtaattactgccaataacgcaaatagtaaccgcaataaaactgatcgctgttgccggaattggctcgaggatcatgccgacaatcattgccacaaacacagcgaagtaatgccatgcctgcggcggcataccgtcggggacagggataagaaacatgacacccatcaccaccagtggggccaatagtttccatatattatcttttgctaaagacatacgggttctccgaaaattaatatttccaaatttatcaagtgcttaaataattaaatctgtgctaaaaaccaggtaaggatcagtaggtcagcactgccgcctggactgagatttcgttcgatacactccctgtcgaactgccggagataatcgagatcggcgggggttcgaatgccccctttttgcaataatgtttgcgcctcgcgctgtagccagcgcaggcccccctcgccaccgcgcgatgcaacgttggtatcgccgttgatcgccatcagtaggagcaaggtatcgagcaatgccagttcaggatctaacccctgatccagcagagtgaggtaatgcggcaaggcgtgattgatcaccagtggataacccgcttcggcttcaccgcgtgcgccggtaaggccaagctgttggtacaaccgttgacctgccgtcagttgtgaattattggtacgcagttcgcgatcggtcaggccacggcagaaacttgccgccgtagaacaaacggttgttggcgttaccggttggttgagttgaagcaaacggccaattgccgcacatagcagccctaaagaaaaaatgctgcctttatgcgtgtttacgcccgcagtggcgcggaacatatcaccttcgcaagccataccaattgggcgtaatccgtggagtaccgcttctggtgccatttccgcactacaggcaccaaattcaatgaaacggggtagccagccctgaatcgccagcgcgctgcggtggaaatcttccagcgccatatctttgtgcgcaccgcagttaatgcgatccacgaggcctggtttcggtgacagattgacttcagtcagcatggcgcgccagcccagcagggcgtactcatcgattaatgacgtcgcaagctttgtggttttagttgacgttgcaggcatcgacatcgttcagcagtgcctccatgcggttgagtaaatcggtcagttgatgggtttttccacgcgcgcagacggctgcgctttgttcgcacaacaggcagcggcgaggcggcagtgaatagtcgcggcgggagagaatttcgccttcgggcgtcaggacatcgatatcccataaccgcccgagaggatgactatgttcaagctcaatggtggcgagcttgaggtcgcgagccggggcggcaatgctcaacatgccctccggcccgctggcggaaaccagtgcagcctgctcctgaatttgccagccctgttttgcggctaaggcacgcaaggctgtcacgccatgattaaaaattcggcgtgtgacctcgctgtctttaatcggcccaggcgcaaccacggtaaaggagaccagtggaacaggatggcgcttgagccagacgtgttgccgtgcttgcctttcatcccggctgacgagcagctcgggaattgataccgcatggtggctggcgagttcaggaagcaggtgcatggcttattccttcacctgatgcacaacatcgatcaccgagccatcgcggtaacgcacaacggcaacgacgcggtctgtgaattcaatcggctgtggttcaccggtcagcagacgcgcacgttcgcgcagccactcaatggaaaccactttaatgcccgcttcctgcagacgttctgccagttccggacgtgccgggttaactgcgataccgtggtctgtgaccagaatatcgacactggagcctggggtgatgcaggtcagtacgttatccaccagagtcggaatacgaccgcgtaccagcggcgcgacgatgatggaaagcgcagaggcaatcgcggtatcgcagtgaccaccggaagcaccacgcagtacgccgtcagagccggtcagcacgttaacgttgaactgggtgtcaatttccagcgcgctcagtaccaccacgtcgagacgatcaaccgatgcgcctttcgaaccccagttagcgtactggttggcgctgatttcgatgtgattggggttacgggccagcgattgcgcagcatggctgtcaaagctctgcacatccagcagtttgcggatcagacctttttcgtgcaggtcaaccatcgtcgcggtaataccgccaagggcgaagtcggcgcgaatatcgcggctacgcattttgtcttccaggaaacgggttaccgccagcgatgcgccgccggtgccggtttgcatggagaaaccttctttgaagtagccagagttgacaatcacatccgcagcgctacgggcaataagcagttcgcgcgggttagtggtcatacgggtcgcgccagcgccgatttttgcagcatcgccaacgcggtcaactttgacgatcaaatcaacctgatcttgctcaatgcttgccggattatgcggataaggcagcagttcttcggtaagcatcacgacctgttttgcgttgtcggcatcaactattgcatagccgagggagccgcagcaggctttaccggtgtagccgttggcattaccgaattcatcacaggacgggacgccgaggaaagccacgtcgatattcagttcgccgctctgtaccagatgcacacgaccgccgtgagagtggatctgcaccggttctgccagcagaccacgggagatctcttccgccagtggaccacgcaggccggaggtataaatgcgggtaaccacgccctggcgaatgtgttctaccagcggcgcatggcaatcactcagggagctggacgccagggtcaggtttttaaagcccatcttcgcgatgacgtccatcaccatattgacggtcaggtcaccgccacggaaagcgtgatggaaggaaaccgtcatgccgtcctgtaaaccagagcgacgaatcgcttcttccaggttggcgcacagtttgcgatcgcgcgctttttcagcctggtaggtttgctttggcgagttctggaaagcggcaagatcgcattcagcgcgacgattccaggccgctacccgttcttgtcgttgagattgttcaattttctgcgtcattttgattgccttattcttcgcggatgccggaaagttctgcacgggagagcaccagacgggcgcgatcgataaccggaccgtccaccatcttgccgttcagggaaaccacgccgaggccttcgcgagcggcggcttcagcggcttctacgacgcggcgggcgtgatccacttctttctgggtcggtgcgtagaggttgtgcagcagatcaatctgacgcgggttgatcagcgatttgccgtcaaagcccagctgtttgatgtgggcggcttcttgcagaaatccggcttcgttgttagcgtcggaatagacggtatcgaacgcctgaatacccgcagagcgcgcggcctgcaaaatggaacagcgtgcgaacagcagttcagttccttccggggagcgttctgtacgcaggttgcgcacatagtcttctgcaccgagggcgataccgatcaaacgctcggaagcgtgagcgatttccactgcgcgggtaatccccagcggagattcaatcgccgccagcaggccggtgctgccgggttcacgaccacaggctttttcgatacgcaggatctctttttcaatatccagaacatcctgagcggtatcggttttcggcagacgcacaacgtccgcaccaccgcgaacgacggcttccaggtcgttaacaccccattcggaatccagcgcgttgacacgcacaatggtttcaatatcgcgatacagcggatgttgcagcgcgtggtaaaccatgcggcgggcggtgtctttttcacgcaatgctacggagtcttcgaggtcaaacatcagggcatcagccgggtagatgaaggagttgctgaccatcgcggcattggcaccaggcacaaacaacatgctgcggcgggtgcgagttttacgttgttgcagcgaagcggaaatcattggcaatcctcccatggcagagccgggataccgctggcgcgtgccagcagggcttccagtcgtgcacgtaaaatgcagtccagtgcgcctttgtcatcgacattcagctgtacgccgcgcacgttgtagcgggcgagaacgtccagaatggtggtgcgaattgcatcgccaaactgtttctcaacgctgctattgatttgcaggtcgatatcctgcgtatcgagtggggcgatgcgtatcatcacatccccagactcaagggtgcctgcaacggcgggctggtttattttcatttttcacctgtttctcatgcgggggtcttttgacgagctgccgcgtcctggcgggagtgctcaagcaggttctgcaaataatgcagcgtgactgcagggaccagcggcgcgatagccgtgagatcgtttttcgccagcagttgacgtacccgggaagcggatatcggcatctcctggtaacgcagccgctcaatttcaaccagttcgatgggcggtgcggagatagtcggcgtttccagccagtagcgcatatcctggttgtactgggcggtaacgcgacaaaagggttcagtaccgacaaagcggtgagttacacccagcgcgggagcgaggtactgacggaaaatcttcagatcaatttcggtgtaacaatggttaatgacgctctgttctttaatgaagtagcaagggaacgtagcgcgggagatgatgtattcggagccacgatgcacagtcaggcgtggaatatcggcggtgccttttaacaccaaatccagccggtcttcataggggaagcgtgaagaatcttctttgactaaaaacagatgcaaccagtcgcactgtgccgcagcctgttgaatcagataacggtgaccattcgtaaagggattggcgttcatcacaatgcagccaatcttgttccctggatgacgaaattttttcagcgattcggcatagcgtttcagtcgcgtggcgctgttttccatcagcaccatcacgccgggtacgctggtcagcgtggaaaaaccgcactggcggaacagcgcctcgtattcggttttggtataaataaacagatgcgtgctgtgccgctcataggcgaggtttatcaattcagtggctaatgtcagcgccagtccttcaccgcggacggattcactgatagcaacgcatttaataatatttccggcaattccaccgcacgcgataagcttttcatcgcgggttacggtaataaatacttcgactgtggtgtcaacgctcaaatcattttcatgcaggaattgggcgatttccgccatttttttattttctgaacgttttacgcgggtgaaaatatcattgccgaacataataaatagtatcctgaaggtgcatgttgttatcgatttgcaacgaatgttgttcaatgttgcaaactgataaccttttattttcacttgggagaaagggggtgatcgaggtatatctttttctcctttcgctatacatcctaaggagtatttcggcgtgaaattttgatttatttcacatagagttagtggttttttatttatttaatgattttaagttttttaattaatgtaattacgaaatgactcgcaggtttaagtgatttaattgatttaatgaataaaatttgccacgatcataattaatatctatgtattttgattcaacattttaattacatccgtcaaagaggctcgggacaacccgcaaggaaaacaatgttgcagcttaacgagaataaacagtttgcatttttccaaagactggcatttccgctgcgtatctttttgctgattctggtgttctcaatatttgtcattgcagccctggcgcaatattttacggccagttttgaggactatttaacgcttcatgtacgcgacatggcaatgaatcaggcgaaaattattgcctccaatgacagtgtcatctctgcggtgaaaacgcgtgactacaaacggctggcgaccatcgctaacaaattacaaagagataccgattttgattatgtggtgattggggaccggcactcgatccgcctttaccatcctaatccggagaaaattggttatcctatgcagttcaccaaacagggcgcgctggagaaaggggagagctacttcattaccgggaaagggtcaatggggatggcgatgcgcgccaaaacgccaatctttgatgacgatggaaaagtcatcggcgtggtgtcgattggctacctggtgagtaaaatcgatagctggcgggctgagtttttattaccgatggcaggtgtgtttgtcgtgctgttagggattctgatgttgctgtcgtggttcctggccgcgcatatccgtcggcagatgatgggcatggagccaaagcaaatcgcacgcgtggtccgtcagcaagaggcgctgtttagttcggtttatgaagggctgattgcggtggatccgcatggttacattaccgccatcaatcgtaacgcaagaaagatgctggggctgagttcccccggacggcaatggttgggtaaacccattgttgaagtggtcaggcccgccgatttctttaccgaacagattgatgaaaaacgtcaggatgtggtggcgaactttaacggtctgagcgttattgccaaccgggaagctattcgttcaggtgatgatttgctgggggccattatcagctttcgtagtaaagacgaaatttccaccctcaatgcgcaactgacgcaaataaaacaatacgttgagagccttcgtacattgcgacacgagcatctcaattggatgtcgacgctcaatggtctgttgcagatgaaagagtatgatcgcgtgctggcgatggtgcagggggagtctcaggcccagcaacagcttattgacagcctgcgcgaggcgtttgccgatcgccaggtggcggggctgctttttggtaaagtgcagcgcgcccgggaactggggctaaaaatgatcattgtccccggtagccagctttcgcaactgccgccaggactggatagcaccgagtttgcagccattgtgggcaatttacttgataacgccttcgaagccagcctgcgtagcgatgaaggaaacaagatcgttgaattattcctcagcgatgaaggcgatgatgtggtgattgaagtcgccgatcagggctgcggcgttccagagtctctacgagacaaaatatttgagcagggggtcagtacgcgtgctgacgagcccggtgaacatggcattgggttgtacttgattgccagctacgtaacgcgctgcggtggtgttatcactctcgaagataatgatccctgcggtaccttattttcaatctatattccgaaagtgaaacctaatgacagctccattaaccctattgatcgttgaggacgaaacgccgctggcagagatgcatgcggaatatattcgtcacattcccggattcagtcagatattactggcgggaaatctggcgcaggcccgaatgatgatcgagcgttttaagccggggctaatcttgctcgataactatcttcctgacggtagagggattaatttactgcatgaactggtgcaggcgcattatcccggcgacgtggtgtttaccactgcagccagcgatatggaaacggtgtctgaagccgtacgttgtggtgtatttgattatctcattaagcccattgcctatgaacggctggggcaaacgctaacccgtttccgccagcgtaaacatatgctggaaagtattgatagcgccagccagaagcaaattgatgagatgtttaatgcttatgctcgcggtgaacctaaggacgagctaccgaccggcattgaccccttgacgctaaacgcggtgcgaaaactgtttaaagagcctggtgtgcaacatacggcagaaacggtggcgcaggcactgaccatcagccgcaccactgccaggcgttatcttgaatattgcgccagccgccatctgattattgctgaaattgttcacggcaaagttggcagaccacaacgcatataccacagtgggtgacatgataaagccggaggaaacttgcctccggcattactatttacttgcctgtgaccgctgctgccgttcctggcaccatcagctctgtagcaacgataacaatcaccaaaccaacaagcaccggtaccgaggtgcgttttacgacttcaaacggcgagatcttcgccatcccggcaaccgcaacgactacgccagaaacgggcgaaagggtacggccaaggtttgacgcctgcagcatcgggatagtcaaatacgccgggttaatgccggaagagtgcgccagtttcgggatcatctcaacaaacgcataaaacggcgcattgcctgaaccggtcgtgactgccgccagcattgtcagaatcaccaataccagcatcaggatgatactcgccgaaccaaacgaggtagcgatagaaatcagactttgaataaagccgatggtgctaagcccctgagcgaataccccagcggcaaccagcagcatcaccacgttagcaaacgcatctgccatcccgcgataagccacttccagaccagagaaaactttctgggtattaaagctgcggaggaactccagaatggaggcaatcagcatacaaatcaccagaatagtgatgatgtgtaattgcggaccccatttaccgtcaaaaatcagtacaccgatgatcggcgtgaacggcaaaatggcataaaacgcaggagcagtggtggtgatttcactgacatctaacatttcatgagagatgtgctcttttttatccagataacgttgccagaagaagtgggcgatcgccatgccgataattgcagcaattgagataggcagcgtcgttttgaaggcgaagtcaatcagcgacatttcggaagcttgcgccgccagcaccacatcccctgaagtcggtgcgagaataatcgccgccggggaggcacaaatggcagcagctgcgccacgactgataccaacgtttaccatcaccggaaatagggttgccatcagcaaaacacccagaccggttgcggaagagacggccagagacatcagacaggcgacaaaataggcggcaatcatcagcaggtaaggggagttaatatactgcaatggttttgacgccagcttgaccaccatatcattcgcgccgatatgggtcatgtaagcggcaaatccacacagcatcataatcatcatgccgaggtcgccgccgcggctcattagtaatattttaacgtattcaacgatatccgtggcgctgtagcctgttgaagcctggctggacggtaacactttgtgccccataatggcactgataatcagcaataacaggccaccgacaaataacacaccagtggcggaataccctttaatgatgtagcgagctacacccacaataaccacaaccccaataaggagctcaatgaatgtcagcataatttttcctgtctccaggccccaaagtaaataataaaaaattcctaaagcttaaggaaaaaatatgcccaataaattggcgatgaatgctgattaaaatcaagaaaaactgccattaagacattgaagttgctgtttttatacatagataacaaaacgcatatttagcggttggcaattatcacataataatgtgtgcaaattgatggtggattgatgcaaatttgttaattgcaatggtgttagctgcggctgtgcgctcaaaaaataatctaatatgagcataggttgacgatatatattatatacttcgttaagatgattgttgtatctcgttaaaaaataaaataatttttccttgattgcattttgtcatcaaaaaagacttggtttttcttttttgactattcccatcgcagaaaacgacgcatcatctttaatcgatgcgcggaaatatttaacttgaacaagcggaaataaatagagcagctattcagattattctttatgttgggtctattaaggttatgttaattgtagctttgctatgctagtagtagatttttgataaatgttttatggtcacaaatgaacgtgagtaaatatgtcgctatcttttcctttgtttttattcagttaatcagcgttggtaaagtttttgctaacgcagatgagtggatgacaacgtttagagaaaatattgcacaaacctggcaacagcctgaacattatgatttatatattcctgccatcacctggcatgcacgtttcgcttacgacaaagaaaaaaccgatcgctataacgagcgaccgtggggtggcggttttggcctgtcgcgttgggatgaaaaaggaaactggcatggcctgtatgccatggcatttaaggactcgtggaacaaatgggaaccgattgccggatacggatgggaaagtacctggcgaccgctggcggatgaaaattttcatttaggtctgggattcaccgctggcgtaacggcacgcgataactggaattacatccctctcccggttctactgccattggcctccgtgggttatggcccagtgacttttcagatgacctacattccgggtacctacaacaatggcaatgtgtactttgcctggatgcgctttcagttttgagacaaatgaagttttagtaacttctttaaaatcaatagctaaaataagtaacatcaaaaataacgcgacttttatcactttttagtaaagttacactggacaaagcgtaccacaattggtgtactggtaaccgacacagcatttgtgtctatttttcatgtaaaggtaattttgatgtctaagattaaaggtaacgttaagtggtttaatgagtccaaaggattcggtttcattactccggaagacggcagcaaagacgtgttcgtacacttctctgcaatccagactaatggttttaaaactcttgctgaaggtcagcgcgtagagttcgaaatcactaacggtgccaaaggcccttctgctgcaaacgtaatcgctctgtaagatacgtcagcaagaattcaaaacccgcttaatcagcgggttttttttggtctttagtgtgcggttgaggccgaaaacagccagaatgccagtgcggtcatggcaaaagaccccagaaggttgacgaaaacgttcagtaatgcccagccaaagcggccctcttgtaacaaaaacaccacttctgccgaaaatgttgagaaggttgttagaccgccacaaaatccggtggtgattaatactttccacactggatcaatgttcgtcatcctgctgaaccatgcgaatcctattcctatgatgaatgccccaatcaggtttgctgtcagcgtccccaacggaatcgcctgatgcagtgggttaaatcgcatacttaacagccatctcgccacgcttcccgtaccaccgccaataaaaactgctaaaagaagttgtaacactgcaaaatcctgctatttgatttgtatgagtgataagtgtaacgccgaataatcgtcgttggcgaattttacgactctgacaggaggtggcaatgctggttgccgcaggacagtttgctgttacatctgtgtgggaaaagaacgctgagatttgtgcctcgttgatggcgcaggcggcggaaaacgacgcatcgctgtttgccctgccggaagcattgctggcgcgcgatgatcatgatgcagatctatcggttaaatcagcacagctgctggaaggcgaattcctcggactttacggcgagaaagtaaacgtaacatgatgacgacaattctgacgattcatgttccttcaacgccggggcgcgcatggaatatgctggtggcacttcaggcaggaaacatcgtcgcccgttatgccaaactgcatctctatgatgcatttgccattcaggaatcacgccgtgttgatgctggtaatgaaatcgctccgttactggaggtggaagggatgaaggtcggtctgatgacctgttatgacttacgctttccagagctggcgctggcacaggcattacagggagctgaaatcctggtacttcctgccgcctgggttcgcgggccgctcaaagagcatcactggtcaacgttgcttgccgctcgtgcgctggataccacctgttatatggtggcggcgggggagtgcgggaacaaaaatatcggtcaaagccggattatagatccctttggcgtcaccattgcggcagcgtcagaaatgcctgcactcattatggcggaagtgacgcccgaacgtgtgcgtcaggtgcgcgcgcaactgcccgtcttaaacaaccgtcgctttgcgccgccgcaattattatgatgtttttttactcggcgcttgattcaccttgttacagattgctattgtgtgcgcgcgtcgaatgaccgttaatattctctggtttttaaggcgcgttctgttgccggttatatgtcaagaaggtatctatgggtgagattagtattaccaaactgctggtagttgcggcgctggtcgttctgctgtttgggactaagaagttacgtacgctgggcggagaccttggagcggccattaaagggttcaagaaggcgatgaatgatgacgatgctgcggcgaaaaaaggcgcagacgttgatcttcaggctgaaaagctctctcataaagagtgacgtggcgagcaggacgctccctcaatatcttgttcgatacaaaaaacccgcttcaaaaagcgggttttttatcagacagatgtaagtaattattacaggattacttaacttccatccctttcgcctgcaaatcggcgtggtaagaagagcggacaaacggaccgcatgcagcatgggtaaagcccatcgccagcgcttcggctttcatttcgtcgaactcatccgggctaacgtaacgttgaaccggcaggtgatggcggcttggctgcaaatattgccccagcgttaacatcgtcacaccatgacggcgcaggtcgcgcattacctcaataatttcttcattggtttcacccagtcccaccatcagaccagacttggtcgggatttccggatgcgcttctttaaagcgttccagcagcttcagcgaccagttgtaatctgcaccaggccgtacctgacggtaaatacgcggtacgttttccaggttatggttgaacacatctggtggcgttgcagtcagaatatccagagcacgatccatacgaccgcggaaatccggcaccagagtttcaattttgatttgcgggcttttttcccgaatggcagtaatgcaatccgcaaagtgctgggcaccgccatcgcgcaggtcatcacggtcaacggaggtgataaccacataacgcagcgccatatcggcaatggtctgcgccagtttcactggttcattggcatcaggagctaccgggcgaccgtgggcaacatcacagaacggacaacggcgggtacaaatagcgccgaggatcataaacgttgctgtgccgtggttgaagcattccgccaggttagggcaggaggcttcctcgcagacagaatgcaggccatttttgcgcattgcggctttgatgccctggatacgtgtagagtccgctggaagcttgattttcatccattccggcttgcgcagcagggcttcgcgctctgttgccacgtttttaaccgggataagggccatcttatcggcatcgcggtatttaacaccgcgttccatcacaatgggtttactcatagcgtgcgtgttccagttgcgaattacgaaggaaagcgtttcaattcaatagattgttgtaattatcaactatttttgaattaacgactggcagtatatcattgaaacggacctgaaagcagccaaagcggtcgcgaaaatgtaaaattgttgttggattgtgccattttatcgttctgcgctgtgatctggctgtaacaatactttttcaaaatgcattacggataacatctattactccgtgcaggatgggatcacgcaggctgaatttgttgtagtggatagagaaatctatttgctcctcatttaaggacggaaaaggcagtttttccagcggccagcagcggctaaacaggttataaaaacggctgggaataatcgctaacatgtcactgttggcaaccagtgcagcgattgtcaaaatgttgtagctggtgaaattgatttgccggtccggaaacatttcttgaactctctgccgcagaccgctgaaattttgctcttccggtaacagaagtacatgcgcagcgttgtcgatagtctctctgtcatcttctaaagagagtagtggatttccctcgcggcaaattaacaccatattgtcggtgaacagaacatgatgttgcaccgtacgattggtgcaaaacatgttatcgatgatgagatcggtttgaaactgactgagttggttttccgcgtcgctgatgggcgggttgcgcagtaaaagctgcggatagtgagttttaatcgcccgatagatgacaggaaggaccagtgctccgaccgagggagtggtcgcaatagttatcgttcgttgcttatcatagcttccttcgatatccagcgcgccaagaatggactcaaggccctgactgatatactcatgtagatgcatcgcaaatgcggtaggagtgacaccctggcctttgcgaataaacaatgggtcagggaatataacgcgcagtttctgaatagactgactgattgccgagggggtcagattaagcactttcgctgcattaacgatccctttatgtacatatacagcttcaaaaatagtcagaaggttaagatcaatatttcgtaaggttgtaaatatttgtggtttaccttctgacgactttctgcttaaacagggttcaatttgattattactatccacgcacttactccaattttattcatggaaaaataatatttaaaaaattacaataatcttatgtctaattggaacggaacgcttttgctcaccataatcaactatttcaataggttaatcaatggggtgagttacggagcaaggcgtggcaccgcatttctgcaagtgataaagaaaatatacaaacgcgaaggagatgtaaagcattagcagatattatgagtaatgacccagtgtaaattgggccattgatgtatggaattaagcggtaatatattcgaagtccggattgtttagtagcgctaaaatattttccagtaaacgtggagcaatattattagtcgtcgcttcgggtttccattgtgatattttagccatttccattccggcatacccacaaggattaatacgtaaaaatggtgaaagatccatattgacgtttaatgccagaccgtggaatgaacaaccgcgtcgaatacgtaaacccagtgagcaaattttcttttccccaacatagacacctggcgcgtcagcccgaggatgcgcttctatacccagttcagccagggtattcaccactgtttgctcaagcaaggtcaccagttcacgcacaccgagtttacggcgtttcaggttaagcaacacatacatcacctgttgccccggcccgtgataagtcacctgcccaccgcgatcgctctggatcaccggaatatcacccggcattaaaatgtgctccgcttttcctgcctgaccttgggtgaataccggatagtgctcgaccagccagatttcatcaagggtactatcatcgcgggtatcggtgaattcatgcatagcctgggagattggctcgtaaggctgaagaccgagctggcggacaagaattttatcctgatacaaaacggcatctccgtggagaatgagtaaaagtgggggaaaagtatatcacagcgaggagaggggagttacccgaccaggagccgggtaacggagaagcgagttacagaaccatgcggacaatatcgattttgcccagttcttcatacagtgtttcaacctgctcgatatgagtggcgttgatagtgatagataccgagtggtagttgcctttgctgcttggttttaccgttggggtgtagtcacctggcgcatggcgctgtaccacttcaaccacctgatcaaccagctcaggtaacgcctgccccataactttgtaagtaaaaggagtagggaattcaagcagttcgttaagtttggttttcatgtcagctccggcgtaacgtaattaaatagcaactcccgccagaaggcgggagttttttactgatgcttagtatatggggacggaaattacactttcaagtgtttaatttttaaccaaaccagtgatggaacattaatttaatgtaatcaatgattttgccgaagaagttaccttccgggatttcttgcaacacaaccagcgggcgttgctcgatcgttttgccatcaagctggaagttgatagttccgacgacctgattcttttgcagcggcgcatgcaattcactgctgttcagcacatagctggctttcagatctttcatgcgaccacgcggaatggtcaggtacacgtctttatcaacccctaacgaagcgcgatcagaatcaccaaaccaaaccggttcagaggcgaactctttacctactttcagtgggttaacggtttcaaagaaacggaagccccaggttagcagttttttactttcggcttcacggcctttaaaagtacgtccgcccattaccgcagaaatcaagcgcatctggccttcagtcgcagaagcaacaaggttgtaacctgctttgtcagtgtgtccggttttgatgccgtcgacattcaggctgttatcccataacaggccgttacggttcagctggcgaataccgttaaacgtaaattctttttctttatagatcgagtattcattcggtacgtcacggatcaatgcctggccgatcagcgccatatctcgcgcggagctgtactgaccatcagcatccagaccatgtaccgtctggaagtgggtatttttcaggcccagtgcgttaacgtagctgttcatcaagccaacaaaagcgtcctggctaccagcggcaaaatcggccatggcgacacaagcatcgttacccgattgcaggttaataccgcggatcagctgagaaaccggaacctgcatgcccggtttgaggaacatcagcgaagaacctttaaacaccgggttaccggtggcccatgcgtcgttgccgatagtgactaaatcagtttctttaaatttaccggctttcattgcctggccgataacgtaactggtcatcattttggtcaggctggcaggatcgcggcggacatctgcgttctgttcggcgagcactttgccggagttatagtcaatcaggatgtaggactccgcatcgatctgcggtacacccgggatcatagttttgatattcaggtcatcggcatgtgcagcagagataaaggctgtgcaaagagccgtggtgagcgccaggcgcttcatgatacgagcggaaaaaatggtattcatggtctgaactacgacatccgtgatggaattaaaaaagtgccctactatagcaaatgcactaccggcaggcatctgactttccgcgtgactttgttaacgtcatttacagaaattgacacatcagatgcctgctttacgctactgcgcggtagtaataaatgactgtaattgggcttcggtttgcaaacgttgctgcaaggtactggcttcggctttgctggcgaatgggccaagctggatccgccagaccgcgccattttgagttacgcgaccggggacgccgaacttctgtcccagttgctgttggtactgttgcgcacgagcctgatcgcttacggccccgacttgcaccataaagttgccgctggcgctttgcgagacggcttgcggtgtcaccattgcaggcgaggttgcaggcgttgtcgacggagctgtaacaacgggctgtggcgcaggcgtcggttcgctgccttccagtacaccaggcgctaaggtcgttggtgcgccgaggaaaccgctactggttaccggcgcgccggtcggatcttcgctttttagcgtcgaattactgaccggaagaatgtcaccctgcgggccagacactgaacttgttcccgcgccaccgcttaaatcgggaggtgcaggcagggcgtaagtctgtttggcgactgtggtacaagccataccaggaccagaaagcgaaccatcctgggcaacaataatcggatcgatacgaactttggtgttgtttgacgtgttaagacggtcagctgccgcgcgagaaagtgaaataacgcggtcgttgccgtaagggccgcgatcattaatgcgcaccacgatcattcgcccgttagccaggttagtgattctggcgtagctggggatcggaagcgttggatgggctgccgtcagctgtgtcggatcgaatgcttcgccagaggccgtcaggttactgccgggttcggcatcatagattgccgccagtcccgcctggctaaatcgagacggatcctgcacgattttgtagcttttaccgtcgcgctggtaatcctgatttgccgtcgcgttcagtggttcgaaacgcgggtccgccccgctaatttcaactatagggccgttacataccgcaggctgcggtacacttaccgtctgttgctgaccatcatcgcttgtacatgccgcgagcattcctgccgcgatgcagatcccgagccactgcttacgcattgcgcacctcttacacgcttttcgacaacattttcctgtgggtgtggattgacattacaatcccgaacccagccatcagcacaattagcgccgatcctccataactgaccagtgggagcggaacccctacaaccggcagaataccgcttaccataccaatatttacgaagacataaacgaataatatcagcattaagccgccagccatgacgcgaccaaaggtggtttgcgctctggcggctatccacagcccgcgcatgatcagcagaatgtagagagcgagcagaatcagaatgcccactaatcccagctcttccgccagtaccgcgaagataaagtcagtatggcgttcggggagaaattcaagctgtgactgagtgccgtgcagccagcctttgccgcgtaatccgccggagccaatagcaattttagactgaataatgtgatagcccgcgccgagtgggtctgattccgggtccaggagcatcattacgcgctggcgctggtaatcatgcatcaggaagaaccacagaatcggaatgaacgccgctaccagcactactgcgacgccaatcagacgccagctaaggccagagaggaacagtacaaacagaccggaaagcgcaacgaggattgatgttcccaggtcaggctgtgcagccaccagcagcgtgggcataaatatcagcaccagcgcgatgccagtgttcttcaacgatggcgggcaaacgtcgcggttgataaagcgcgcaaccatcagtggtacggctattttggcaatttccgacggctgaaaacgaacaataccgaggtccagccagcgttgagcacctttagagatggcaccgaaagcatctaccgccaccagcaaaataatacagatgatatagagatagggggcccagccttcataaacgcgtggaggaatttgcgccatcaccaccatgatgaccagacccatcgcgatttggccgattttacgctccatcatgccaatatcctgaccgctggcgctccagataaccagggcgctgtaaaccagcaatgccagtaagatcagcagcattgtgggatcgagatggactttatcccagaatgtttttttattcggattatccgtcatgattaatggtcctccgctgcggcaaccgctggattttccgcaggcagatcggtgttgttatcacccagcataatgtggtcgaggatctggcgcatcagtgtaccaaccgccggacccgcaccaccgttctccagaatcatggcgacagccacttgcggattgttgtatggcgcaaaggcggtcatcagtttgtggtcacgtaaacgctcggcaattttgtgcgcattataggtttcgttcgctttcagaccgaagacctgagcggtaccggatttcgccgcaattttgtacggtgcgctagcaaagtatttatgcgccgtaccgttagggcggttagcaacaccgtacataccgtctttcgccagctcccagtaaccggaatgaatatcgccgacgggcggttcatgcggctgtacccatggcacctgtttgccgtcttcggcggtgctcatcagcaaatgaggaaccttcacgataccgtcattaatcaggatcatcagtgccttactcatctggattggggtcgctgtccagtaaccctgaccgataccaaccggaatggtgtcaccctgataccacggttttttaaagcgtttctgtttccattcgcgggtaggcatgttgccggaacgttcttccgccaggtcgataccggtgtaatgaccataaccgaatttacccatccattcggagaggcgatcgatccccatatcgtaggccacctgatagaagaaggtatccgcagattcttccagcgatcttgtgacattcagacgcccgtggccccattttttccagtcacgataacgtttttccgaacctggcagttgccaccagcctgggtcaaacagcgtcgtattgcgcgtgatcaccccggcgctcaatgccgaaaccgccacatagggtttaactgtagacgcgggaggataaaccccctgtgtggcgcggttcaccagcggtgtattcggatcgttcaacaaggcggaataatctttgctggagataccgtcaacaaacaagtttgggtcataactaggcgtggaaaccagcgccagcaccccacctgtacgcggatcggtgactaccacagctgcgcggctacccgccagcagcgtttcaatatattgctggagtttgagatccagcgtcaggtaaatatcgtgtccggcttgcggtggtacttcttttaactggcgaataacacgcccacggttgttaacttcaacctcttcataaccggtctgaccgtgcagcacatcttcatagtaacgctcaatgcccagcttaccgatatcatgcgttgccgcatagttggccagtttgccgtcattattcaggcgttcgacgtctttatcgttgattttcgacacatagccgatgacgtgggtcaacgccgaaccgtaaggatagtaacgacgtttatagcctttaacttcgacacccggaaaacggtactgattgacggcaaagcgagctacttgtacttcggtcaggttagttttcaccggaatagaggtgaaacggtgtgaacgtgcgcgctcttttcggaatgcagcaatatcgtcatcggtcagatctaccacgctgcgcaaagcgtccagcgtttgctgcacgttatcgactttctccggcatcatttctatctggtagatagtgcggttgagggccagagggataccgttacgatcgtagataatgccgcggctgggcgcgataggcaccagcttaatgcggttttcattagagcgggtctggtagtcggtaaagcgaacaatttgcagattatacaggttggcgataagcacgccggtcagcagcaaaatccccaaaaaggcgaccagcgcccggcgcacaaacagcgcggactctgccgtatagtcgcgaaaagagttctgtagtttcatccgctgcgttttctactcaaagctcccttatcactcacggtgataaggatggttggtggtgatgctccacgcccggtacagactctctgcgaccagcacgcgaaccagcggatgggggagggtaagcgccgacagcgaccagctctgctcagccgccgctttacaggcaggcgacaacccttcaggcccgccaatcagtagactgacgtcgcgaccatccagcttccagcgttccagctcagcggctaactgcggcgtatcccagggcttgcctggaatatcgagggtgacaatgcggtttttgcctgcggccgccaacatctgctcaccctctttgtcgagtatgcgcttgatgtccgcattcttgccgcgttttccggccggaatttcaatcagctcgaagggcatatctttcggaaaacgacgcaggtactcggtaaaaccggtttgtacccagtccggcattttcgttcccacggcgacaagttgcagcttcacgcattaactccagagtttttccagttcatacaggcgacggctctcttcctgcatgacatggacaatcacatcgcccaaatccacgacaatccagtcggcgctgttttcaccttctacgccgagcggtaacaggcccgctgcgcgagactcctgcacaacgtggtcagcaatggacataacatgacggctggacgtacccgtacagatgatcatgcagtcggtgatgctggatttgccctgaacgtctaaggcgatgatgtcctgacctttgaggtcatcaattttgtcgataacaaaatcctggagtgctttaccctgcaagttttccccctgggtgaatcaaatagataaaaatggtctgtcagtatacctgaaccagaggcgatttcgggacaattgtcgccgaatcggctttcgaaagtgggctatcatcccaccccgcgccgcagattgcatcgccatttttgtaaaacaatttctacaaagtcgtgtctggcggaaaaagtctggctgcggagaatatcagcctgcccgggtctgtcaatggtcgttgcggcttacccgtaaaaaaacagaaaagtcatgcattctcgaccccgatggcacggctattgaggacgcgtagcgtcgcgaatttttggttgatatcaatggcgctccaacacccctggtcaacgcgaaaatgccacatagcttcggcaggcatgccaattaaacgggcgattaacagactcagtacaccctgatggctgacgactaaaatattctgatagtgctgaaattcactaagccttgcgataaagcgttccacacgttgcgaaaatgcctgaaatccttcaccgttcgtggggattgcatgctgccagtcattgcaccacgcgctatagttttcggcatcttcttgcatgaggtcgcgatgatgtcgcatctcccagtcgccaaaaaacatttcgttgagttcaggtatgatttgcacggggagctggcggtcactgagaaccagtcgcgcggtatgctgtgcccgttccagttcactgcataaaaccagatcaaaggaaacaccatgtagcagcgtatgcagattttgcgcttgctcaataccgcgcgcggtcaggggggtgggcgcatgaccgctgtaaagaccatcgatattcgcttgcgtttcaccatgacgaattaaccacagtcgcatcatgccctccgtaacgacaggtatcagcgatacaagccttgttggttaatgtaagtcagtaccggttccggcaataaatcctcacatgattcaccgttttgcaaacgttcgcggatgatggtcgccgagatgttaaaccacggcgtttcagccagataaattttaccggcaggctgaaggtgaagatcttccgggttatgtgtcaaatgatcttccagccattgctggtattgcggttgcgccatttcaagtgggtaacctggacgccgacagacgatcaaatgtgcattgtcgagtatcgtttcgtattcgtaccaggtcggaaaggtcagcagtgaatcctgaccaataataaacgccagcggcacgtccggtccttgttcctgccgccactctttcagtgtttgcgcagtgtaagagggggcattgcgctttagctcgcgttcatcaagagtaaataatggcttgtcggcaatcgccagttcaagcatgtgtttacgctgcacgctgttcgcttccggctggggacgatgcggaggaacattattagggatgattgtgacccgcgtcagaccaatcaaattcgccagcgtttccacgggttttagatgaccatagtgcaccggatcaaaggtgccgccaaacagagcctgtaaagatttcatatcaaccgtcgataaatacgtccgccaggggtttatggcacaacagaagagataacccttccagctctgcccacactgactgaccgtaatcttgtttgagggtgagttccgttcgtgtcaggagttgcacggcctgacgtaactgcgtctgacttaagcgatttaacgcctcgcccatcatgccccggcggttctgccatacccgatgcttatcaaacaacgcacgcagtggcgtatgggcagactggcgtttcaggttaaccagtaacaacagttcacgttgtaatgtgcgcaacaaaataaccggttcgctgccttccagacgcagttgctgaagaatatgcaatgcgcgcttactttttcccatcaacaaagcatcaacccaatgaaaaggggtgaaatgcgcggcatcattcaccgcctgttcaacgcgcggtaatgtcaatttgccgtctggccagagcagcgataaacgctccagtgcctgagccagcgccagcaggttaccttcataacagtagcagagcacctgatttgccgcgtcatccagttctaagttgagctgttttgcgcgcgcagcaacccagcggggaagctgagcctgctccggtgtctgacaggtcacctgcacgctgcgattcgcaagcgcagtaaaccaggcggcattttcttgcgctttgcttaatttattaccgcggacgatcaacagcaggtcgtcatgcagaagtccggtgagtgtgagaagttgctcattgatcgccgcattcggtccgttttctggtaacaacagcaatagcgtttgtcgactggcaaacagactcatagcctggcataacgaaaagatcgcattccagtcagtgttgggatcaatggaaaaagtgtggtgttcttcgaatccttgtgccgcagctacctgacgaacagcgtcctggctttcctgcaataacagaggatcgttaccaagtaaaagatacgccgcgcgcagcccttcattgagctgcgcgcggagttgttccgggtacaaccgaatcatcagttacccagcgtggtggagacgcgtgcaggcgttgccggagtatccgttgtggtcgacgtctgttcttcgtcggaacgaatatccgcagcacggatgcttggcagcttacgaatcagctgttcggcagcacggtcgtacatctcttttacgatcatgtcttgttcgttatctttcgctaacgccatttgcgggttatcgaagaacgaacggaagactttggcgctaatcgggtagatatcacggccggggatcaacacggtcgcattaaccgtcatgatcatctgatactctgctgtttgaccgttacggaataccgatgcggtatctttcgcgatgctcactttacccaaacgcaaggatggaacgtccttacgcgtggtttctttatcaagcaactcgacaccattcagacgtaactggttacgcaccgcacggcttaatggcccgttcggatcgcctgagtccaggatcatgaccttcatagtggaaggaacctgcgtggtatcacgcagatgccagccacacccggcggtgattaacaccgccagagataacaacaatgttgccagatatcgcacgcttcctcccgcgcttagccaacgaccagattgaggagtttacctggtacgtaaatcactttacgtacagtaacgccatcaagatattttgctaccagatgttcctggccagcacgttcgcgaacctgttcttccgttgcgtccaccggaacggtgattttggcacggactttaccgttaacctgcaccacgaccagcgtggagtcttccaccatcgctttttcgtcagcaaccggccacggcgcgttgtcgatatcgccttcgcctttcagttcctgccacagcgtgaagcagatgtgcggggtgaacgggttaagcatacggacaacggccagcagtgcttcctgcatcagagcgcgatcctgctcgccatcggttggtgctttcgccagtttgttcatcagctccataatcgccgcaattgcggtgttgaaggtctgacgacggccgatatcatcggtcactttagcgatcgttttatgcacatcgcgacgcagcgctttctgattttcagtcagcgcatcaacgttcagtgccgcaacatcaccttttgctgtgtgctcgtaaaccagtttccagacacgtttcaggaagcggttagccccttccacaccggattcctgccattcgagagtcatatcagccggagaagcaaacatcataaacagacgaacggtgtccgcgccgtaacgttcaaccatcacctgcgggtcgataccgttgttcttcgacttggacattttgctcatgccggtataaaccagttcatggcctgccgcatctttcgctttcacgatacggcctttctcgtcacgttcaacgatagcatcaaccggggaaacccagttacgttcgccgttttcgccaacatagtagaaggcatctgccagcaccataccctgacacagcaactgtttcgctggttcgtcagagttcaccatgcctgcatcacgcatcagtttgtggaagaagcggaagtagagcaggtgcataatggcgtgttcaataccaccaatgtagatatccaccggcagccagtagttagccgcttcggaatccagcataccttctttgtactgcgggcaagtgtagcgcgcatagtaccaggaggactccataaaggtgtcgaaagtgtcggtttcacgcagtgctggcataccgttaacggtagttttcgcccactccggatctgctttaatcgggctggtaatgccgtccattaccacatcttccggcaggatcaccggcagctggtcgtccggggtcggcattacggtaccgtcttccagcgtcaccatcggaatcggcgcgccccagtaacgctgacgggaaacaccccagtcgcgcaggcggtagttcactttacgctcgccaacgcccatcgcagtcagtttatcggcgatggcgttgaaggccgcttcatggtcaagaccgttgaactcgccagagttgaacagcacgcctttttcagtcagggcttgctgagaaagatctggctcagagccgtcagctgccaggataaccggtttgatgttcaggccgtatttagaggcaaactcgtagtcgcgctggtcgtgccccggtaccgccataactgcgcccgtgccgtactccatcaatacgaagtttgctgcccaaacgggaatttcttcgcccgttaatgggtgaaccgctttaaagccagtatcgacgccttttttctccatcgtcgccatttcagcttcggcaactttggtgttacggcattcgtcaataaaggccgccagttcaggattattttccgccgctttctgcgccagcggatgacccgcagctaccgccaggtaggtacaacccataaaggtgtccgggcgggtagtgtaaacggtcagcgtgttgtcatagtcgttaacgttgaaggtgatctccacgccttcggaacgaccgatccagttacgctgcatggttttaacggtgtctggccagtgatccagtttatccagatcgttgagcagctcgtcagcgtaagcagtgattttgataaaccactgcgggatctctttacgttcaactttggtatcgcagcgccagcagcagccgtcgataacttgttcgttcgccagtacggtctggtcgttcgggcaccagttgaccgcagaagtcttcttatataccaggccttttttatacagctcggtgaagaatttctgttcccaacggtagtattccggcgtacaggttgccagctcgcggctccagtcataaccaaagcccagcattttgagctggtttttcatatacgcgatgttgtcgtacgtccacggtgccggagcggtgttgtttttcaccgccgcgccttccgcaggcagaccaaacgcgtcccagccgatcggctgcaggacgtttttgcccagcatacgctggtagcgggcgatcacgtcaccgatggtgtagttacgtacgtggcccatgtgtagtcgaccagaaggatagggaagcatagacaggcagtaatacttctctttgctctcgtcttcggttacttcaaatgtgcgcttctcatcccaatgaagctgtactttggattctatctcttccgggcggtattgctcttgcatggcagccagtggtcctgttttcaatacggctacaaatgtagcgttgaggtggtttttcagatccgcatagcatagcccaaacgtccgcgtcaaaacagcctttcgcgcactcgacgttgaaatgatgcccggattattcatacattaatttacagagtttgtgggcgtattagcaaagcaaggaacaaagaacgtctattattatagtcagttaacgacccgggagatgaaacgatgaacaaggttgctcaatattaccgtgaactggttgcgtcactgagcgaacgcctgcgcaatggcgaacgtgatatcgacgcactggtggaacaggcgcgcgagcgcgtaataaaaacaggggagttaacgcgaaccgaggtcgatgagctgacgcgagctgtcagacgtgacctggaagagttcgccatgagctatgaagagagcctgaaagaagaatctgacagcgtctttatgcgggtgattaaagaaagcttgtggcaggagctggcagacatcaccgataaaacgcagcttgaatggcgcgaagttttccaggacctcaatcatcatggggtttatcacagcggagaagtggtcgggctgggaaatctggtctgcgagaaatgtcacttccatctcccgatctacacaccggaagtgctgacgctatgcccgaaatgtggtcatgaccagttccagagacgcccgtttgagccgtaatagtctgatttcgcacagcaataaagagaatatgggccgaatgaaattccccggcccttgtttttatctctacagtaaatcttcagtctcacgaatttcctgactgacatctctggttccggatgactgaactttacgatacaggtcgagagcctgtcggagatcgacaggtcttccttctccgtagtgatacataatggccaggttataccaggcagtggcgtcattgcattcagcggctttcgtaaaccattcaaaggcagcctgataatctttctcaacgccttgtccgtgtttatacatataaccgatgttgacgtaagcgccgacgctcccctgagcggcagccttcagataccagtacatcgcttgcttatagtcctggtccaccccttcgccagcgttataatcccatgcaatttgaaactgggcgtgccgattaccctgctgtgcgcttttcaaataccagaatgcggcgagtgtcttgttttgagcaacgccttttccgtcttcataaagatcggccagattgttttgcgcgtcactatggccttgtaatgcagcttgtttgtaccagaaaaatgccagcgcatagtcttttgcgactccgttgccatttctgtacatccacccaagattattttgcgcataagacattccgctctccgcggctatctgataccagacaaccgcttctttataattgggggcttctccacgatccagtgtccagccaagggcgttggaagcgaaagtatggccttgtagggcagcttttttcagccagaagatggcttgctcattatctttatgacggcttttatcctcggtatacttttgccctaaggaatactgtgcttcacaatgaccttgctcagcggccagcttcagccagtaaaaggctttttcgtcgtccggagaatcaattgcgctatcgcgattataataaaacccaacaatatattgagcctcgcaatcgcctttttcagcacgttcgataatctcatctattgataaattatcgcagcaacttgacgtgaaaatcattatcatttccttatggttgcagataaaacatattatatttttatgtgttccatttttgcgtaagccttattttatgcgtattatgtcgcgtcagaaaagtataaataaacgagcctcgcaatgcggctaatattcatttaatgaatatttaaggataaattatatggacatggagtcgcaaaaaatattgtttgcactttccactccgatggaaatacgcaatgaatgctgtttaccttcgcattcatcacccaaaatgtatttaggtacatgcttttttgacctttcttcctcatggggaattgatgaccgtgatgacctgctgcgcacaattcaccgaatgatcgataacggtcatgccgctcggttggcagggttttatcaccgctggtttcgttattcgccatgtgaatggcgtgactatcttgctgaactaaatgagcaaggtcaggcttatgcgcaatttgtcgccagcaccgccgaatgctgtggcgaagggggaatcaaagcctgggattatgtccggatgggttttttaagccgaatgggcgtacttaataactggttgagcgaagaagaaagtctatggatccagtcgcgcattcatctacgggctctacgttattatagtaactggcggcaatactttgccggttatacctttggtcggcaatattggcagtctcccgaagatgatcatctgcctttattacgcgaattcttagcgcgtaaagaatacgacgattccggcaatgatatgttttatcaattatttgccagtgatgatgcgtattaccctaccttgtcctggcaaccattggcttactattctgcatgcccggaaacgcttaaggatatgagcgacctatgaaaaattgctggaagatcctcgatatagaggaaacgactgacgtcgatattatccgccgcgcttatctggcgctgttaccgtcctttcatccagaaaccgatccgcagggttttaaacaacttcgtcaggcgtatgaggaggcgctacggattgcgcagtcgcctgctaaatctgtttggcaaccagaagaatatgaggtagcagaacatgaaattctgctcgcctttcgtgcgttacttgcctctgatagtgaacgttttctgccctccgcctggcagcgattcattcagcaattaaattattgctcgatggaggagattgatgaattacgctggtcgctgtgcacaatcgccatgaacactgcccatttatccttcgagtgcgtggtgttattagcagaaagattgcggtggttacaggaggaaaataccggggaaatagacgaagaagaactggaatcctttttatatgccattgcgaaggggaatgtttttaacttccagaccattctgcatctgcccgttgccgtgcaaaatgacaccatcgatttttaccaaatgttcgctcggatttggtcatcgcatccacaatggctgacattgtatttagcgcaacatcgcgcagtgattatccccgatgatgcaaaactgcacagaaatttactccgctggtatagcgcaggtcgcctggatatccccgaacttctggattacgcccagtcatggcgggaaactgaacctgataatgaagatgcgccttattatgaatacgcgcaacgcgtctattgtggagaaggcgaaagcctgttggcagaactttgtgactactggcgcgagtatccctccacccaggcggatgctttaatgttgcaatggtgccgtcagcatcgggtcgattattacccattactggtgatgatgattgaagcgcgtgatctggttaacgatcagggaaaaccgctactttatgtccccggcgacagcgcccgtacgcgttttcatttatacgaaatactcagcgatgaaaaactctctgcgctggggcgttcactggtcgagatggttttgcacaaaggacgtaagccgcggatctcactcacgcgtgatacagaacataccttatggccattatatctagttgccaaacaattagtgcaggcctgccaacctacagaagaatcattaatgccgattgtgagccgccttgatgcagaaaatcgttgtccactggaagcattaattattcgtcgattattaattcaggcggcgaattttaccgagaagcaaactgttgaaccggagccgcaaccgcagccaatgcccgttgacgatggtgggccaggctgtctgggcatcattaaaattattttctatatttttatctttgctggtttgatagggaaaatactccatctgttcgggtgacagtcgacgttaatgtgcgggaagcccggcaagtaatctttccgcatttttgtaatgttgtttggcggtcagttttaaccatttttgagattcataatggttaacattaatacctgagccatttctgtagatcaaacctaaagtatattgagcatgagcatacccttgttcagctgcttccttataccagagaattgctttacgggtgtcgggtttgacccccagacctttgaggtagatccaccccagtttactttgcgcgcgtggattttcctgttccgctgattgctcataccagtatctcgcctgtgtataatccagtggtttaccgtcgctaccatgaagataaaattctccaaggcgatattgcgacgttgagtgaccatgaatcgcggaaagctccgtggctgccgtggtgaatggaagactgcccggtgagcttaaataatcaaaggcataattcaccatggctttatcacgcaacgtcgttttcttgggttggctaatacaggtaattgctgcaactataaaaattgcgaatatatacattaattttttattcatgtgtgaatgcttcgattttctttttattttgaaagcgtcaagtttatactcatcaataataaaaaagtagtcagttaatgcacttaagggattattaacaaatgaataaggaagaacaatatcttctttttgcgctttctgcgcccatggaaatacttaatcagggttgcaaacccgcgcatgactcgccaaaaatgtatactgggataaaagaattcgagctctcatcatcctggggaataaataatcgtgatgatttaattcagactatttatcagatgactgatgatggtcatgccaatgatttagctggcttatatctgacatggcatcgctcttcccctgaagagtggaaagcattaattgctggtggctcggagagagggttgatttatacccaattcgttgcccaaaccgctatgtgctgtggggaagggggaatcaaagcctgggattatgttcgaatggggtttctgtcacgggtcggtgtgctcaacaagtggctgacggaagaagagagtttatggctgcaatcgcgcgtctatgtacgagctcaccattactatcacagctggatgcactatttttccgcctattcgttaggacgtctctactggcaatcttctcagtgcgaagacaacacttcgctacgcgaggcgctaaccctgtacaaatacgatagcgccgggagtcgtatgttcgaagagctggcagcgggaagcgatcgtttctatgccacgcttccctggcagccattaactgtccagtctgaatgcccggtaacgcttaaggatgtgagcgacctatgaaaacatgttggcaaatcctcgaaattgaaagcacgacgcaaatagacattatccgccaggcttatcttgctcgcttaccgttgtgtcatcccgaaaccgatccgcaagggtttaaagcattacgccaggcctatgaagaggccctgcgactggcggtaaatcctgtcgaggaagcagatgatgaagaaaaagatgctgccgctgaacatgaaatactacgtgcattcaggacattactggattcagaaagtgatcgttttcagccttccgcctggcagaaatttattcagcaattaaatacctggaacatggaggatgtcgatcaattacgctggccgctgtgtgcaatcgccatagaagcgcgatatctttcattaaattgtgcttctttgctggcagagcgtttgaactggcattcatttaatgacagcgaaggaatggatgaggaagaaagggaggcttttcttgaggccattcaggctggtgattgtttcgatttccttagccttctggaatatcccattgcgttgcagaaccagactgttgagtattacttcgcgctggaacgttgctgccgttaccatcctgactatgtcactgcgtttttggcgatggaaggtccgtggttaattcctgatgatgcaaagttacatcgcaaactgttgcgctggtacagctcggtgcaaacaggtatggcggaactcattcctgtcgctcaacagtggcaaacggaagaaccagaaagcgaagatgcccggtattacttgtgtgcacaacgtttgtactgcggcgagggggaaagcctgcttgccgatctctgcgcgtactgggaaagttacccatctacacaagctgataatttgttgttgcagtggagcaagcgtcattgcccggattatttcgcgttattagtgatggttatcgaagcgcggagcatggtagatgcgcaaggtcaaccgctgaaatatgttcctggtgagagcgcccggacgcggctgttatgggcggagattttacatagcggaaaattatcgccgttaggtcaatcgtttattgagtcgttattcttcaagcgcaaagcatgggcgtggtggaaatcgagagtcggtagcgagacagagcaagattcaccgttcctggatttgtatcgggtagcggaacaggtagtacttgaagcgtttccgaaacaagagatgctggcccgtcttaatacaaggctggaaggcggagatgctcatccattagaggccattgtcacccggatgcttttgacgaaagtgaaactcgagccggaggatgaagatgtcgatgagccaacacctgaaaatcatgaagaaaaaaatgatgagggtgaaaaaccacagagcattaccagcattatcaaaatcagtttaacggtgctggtgataggttatgctctcggcaaaatcgcgatgttgtttagctgacgatgtgttttttgcgccgatgccggatgcagcgtttacgccgcatccggcagccgtgtttatgggatctcaatggctaaataatcgctcgcccgccgccgaacttcatccacgcgggccatatcgtttgactgcaacgccgcatcaaaatcggtgatcacccggccgatctcttctcgctcgtcacccagcgcccgcgcccacaactcttccagtttggctttaaaggtgcgattgatgagcatatcgcgcggataaattttcaatgcggataaccgcgtccgactctcttcaatctgctgcgcgctcaatgttaccgggctgtggttaatcactctggacttaacgctgccgtcttccagaagcacgtcaacttcaagcaacccgttgatatcataactaaagcgaatatcaatcgactgataagccccggttttcttcaacggcacatcgaaggattccaccagaatgttgtttttaactttgtggttttctccctgatagacgttaaccgtaattgaatcctgttccgggtgcatggttgaataagtttctacacgcgacacgggcacagtggtgtttcgttcaataatcggcgagaaaatgccggaaacgccctggcggttaacttcaacgcccaacgagtaagggcaaatatcagtgaggattacctcttcaatatcttcactgcgtaagcggcaggcggcctggattgctgcgcccagcgcgacaatggtgctcggatcgtaactttgatacggtaatttgccaaacagacgcacggcgattcgctgcaccagcggcatttgtgacgcgccgccaaccagcaccagactgtcgatttgactcggcttcagacgcgcatcgcgcaacgcctgttcaatcggcactcgcaagcgattgagcagcggcaaccacaaatcttccagttcgttctcgtaaaattcgcattcccgcgtttcttcctgatactgccagcgaatgtgcaatggcgattgattgctacattttgccgcttccacacaggcgtacaaggctgccagttcactctcgttaagcgtggtcctggcgacatccgcgcgttttaaaacctcatcgaccagcatatgggtaaaatcttcgccaccaagaaagttgtcgccagcggaggcgtgaacttcaatcaccggcgtggcgtactcaagcaccgtaacgtcaaacgtgccgccaccgagatcaaacaccagcgaacgggtattttgttgggtatgcaggccatacgccatcgcagctgctgtgggttcattaattaagcgtaccgcatttaacccggctaactccgctgctaaacgggtatgcttgcgttgttcatcgctgaaataagccggaacggagatcaccacatctttaatcggacgttgcagaaattcttcggcatcttcttttaatgagcgtaataccaaagaggacagttctggcgcgttaaatgtgtcgctgcctaaccgccagttggtattactgcccattgcacgtttaaataacgctgccgttttatccggatgcgaagtacgccgtgatacagccggttttccgactaaaatatgattattttcatccatgctaattatggatggtgttaaatattcaccgaacttatttggaattaattgcgcggcaccgtctttccagacggcaattaaactattggtagtaccgagatcgataccaatggcgagttctgcattatccattgcatttatatcttgaaagaaaaagagataaacagattaagaccacccaggtaacgcgtggtgatcttaatcaatgacgtgtgttaagcgtaaaatttcagacgatcagccagtaaatcaacaaagccctgacgatcaacatcgaccattacggtggcattcggtttattgcctgtcagataataataatcaacaaccgtcataccctgggtatatttcccctgtgtttccacgccaacccagcgctcaacagaggtaaataactccggtttcaacagccaggcgatggtgcatgggtcatgcagtggtgcgccgacaaagccccatttttcgtctttatgatattcgaggaagaaatccagcagttcggcaacaatggttgaaacagggttaccaatcgcgcggaaacgctcggtgtcttcaacgtggatttgtgctttatgagtaacatccagaccggccatcaccaccgggatccctgactggaagacaatttctgccgcttccgggtcaacgtaaatattaaattcagccgcaggcgtccagttacccagccccatagcgccacccataatcacgatacgggcaattttgctatgcagttccggatggctattgagcagcaaggcaacgttagtttgcggtccggtagacacaatggtgacaggttccgcactttcacgcagcgttttcgccatcagctctaccgccgtacagttttgcggtgcgaatgtcggttccggtaatgccgggccgtcgagaccgctttcgccgtgcacattgtccgcgataatcaactcacgcattaacggttttaccgcgccgcctgctaccggaatatcggtgcgattaagcaaggtcagcatacgcagaacattgcgtaaggttttttctggtgtctggtttccggcggaagacgtaattgctttgacatcaagctctggtgaggcgagggcgagaactattgcgatagcgtcgtcatgacctgggtcgcaatctaacagaattggcagtgccattgttgctccttgttgtgtgcttctttgcgacaagggtaacgccaggatgtaacagatacgaggggcgaaacgataaagcgtgagatggcgcgcaattgggtatgcgcgccagagtgattaatgcaggattttcgcgaggaagtcttttgcgcggtccgatttcggatcatcgaagaaagcgtctttcggcgagtcttcgacaattttaccctcgtccataaagatcacccgattcgccactttacgggcaaagcccatttcgtgggtcaccaccatcatggtcattccttcgttcgccagttccaccatcacgtccagtacttcgttgatcatctccggatccagcgccgatgtcggttcgtcaaacagcatcgcaataggatccatacacaacgcgcgagcgattgccacacgctgctgctgaccgccggaaagctgcgccggaaacttattggcgtgagcagaaagcccgacacgctccagcagtttcagggctttttcacgagccggcgctttatcgcgtttaagcactttcacctgcgccagggtcaggttttcgataatcgacagatgagggaacagctcgaaatgctggaataccatcccgacgcgggaacgcagctttgccagatcggttttcttgtcgttaaccacgataccatcgacggtgatttcaccttgctgcaccggttcgaggccgttgacggttttaatcagcgttgatttgccggaaccagacgggccgcaaaccaccaccacttcgccttttttcacttcggttgagcagtcggtcagcacctgaaagtgaccataccattttgaaacatttttcagggtaatcattatgctgtccttcttttcaagtagctgaccaacaacgacgcgctaagactaataacgaaataaacaaatccggcaaacaggatcatctcaacctgcgtaccatcacgctcaccaatggttgaggcggtacggaagaaatcggccagggataacacatacaccagtgaggtatcctggaacagtacgatgccctgagtgagcagcagcggcaccatcgcgcggaacgcctgcggcagaataatcagtttcatcgactgccagtgagtcattcccaacgccagcgcggcgctcgattgaccacgagaaatactttgaataccagcacggataatctctgaatagtaggccgcttcaaacatcgaaaacgccaccatcgccgaaattaaacggatatcattttttggcgataatcccagcacgttttgcagaaaacccggcacgatcaggtaaaaccacagcaaaaccataactaaaggaatcgagcggaatacgttaacgtaggctttggcaaaccacgccacgggcgcaaagctggataaacgcatcaccgccagcatcgtgccccacaaaataccaatcactaccgccgtgacggtgattttcagggtgatcaccagcccgtcgagcagatatggcagggaagggacaatggaactccagtcaaactcgtacattatttgccccccatgttgccaggcaggcgaactttacgttcaaccagcgtcatcaccagcatgataaaagcgttaatcaacacatacgccagcgtaatggcggtaaacgactcccaggcatgggctgagtaatcgagcaatttacccgcctgcgccgccatatccaccagaccgatagtcgaggcgatggcggagtttttcaccaggttcatcatctctgaggtcatcggcgggacgataacgcgataagcattaggcagcagtacgtatcgataagcctgcggtagcgtcaggcccatcgccagcgcggcatttttttgccctcgcggcagcgactgaatcgcggcgcgtacctgttcgcaaacacgggcggcggtaaacagccccaggcagagcatggatgaaaggaaaaactgaatattgggatccagctcggccttaaaccacatgccgattttctccggcagcagctccgggatcaccagataccaggtaaagaattgcacaatcaacggcacgttgcggaacagttcgacatacaacgtacccagaccagagagaaaacggtttggaacggtacgtaaaatgccgaaaaatgaaccgacgaggaaagcgataatccaggcgcagatcgacaaagcgatcgtcacctgaaaaccactccagatccaaccaagataggtggtgttgccgaacggggcttgttgtaaaaaaataccccagttccagtctatagacataaatctactccagaaaaaagagggtagcagcgttaactgctaccctcgaagattgttacccagcgtattgcggttttcaggcccgatggggaacgaccatcaggcgtatagtctgtccgtgctacgtaacaatcgagagggctggaatttccgcccctggttcttgtaattagttcagtgccttgtcattcggttctttgaacagtgctttcatttcgtctgacagttcgaaattcatgttcaggtttttcggcggaattggatttttgaaccacttatcaaaccatttttccgcttcaccggaggtctgcacctgagcgatggtgtcatccatcagctttttgaactgcggatcatctttacgcaacatacaaccgtaggcctcctgagactgcggcttgccgacgatttcccagttgtctggtttcttcgctttcgcacgttcaccggccagcagagcgtcatccatcataaaggcaacggcacgaccgctttccagggtgcggaaagagtcaccgtgatctttggcgctgatgatgcgcatattcattttttgctcttcattcagtttgttgagcaaaacttcagaggtagtgccggaagtgacgactacggctttgtctttcaggttggcaaaatctttgatatcgccaccctttttggtcaacaggcgcgtaccgaccacgaaaatagtgtcagagaaagccgcctgtttttggcgttcgacgttgttggtggtagaaccacattcaaaatcgaaagtgccgttttgcagcagtggaatacggttttgtgaggtaatcggaatcagttttacctgcaagtccggtttgttgagtttctttttcactgcttcaacaatggcgttggagtaatcctgcgagtaacccaccactttttgctgattgtcgtaataagagaaaggcactgaagattcacggtgaccgacgacaatcacaccgtttttggcgattttgtccagagtactgcccgctgccggggcggcgtcatctgcctgtgccagtcctgcggaaagcgccagggcgaggattgctgtggcaggtttacgtaattgcatatccaactcctttatcttctgcgttaagaacgcatggatacccgttgtgagtgtttgtgttgttatcgtctgcaactttattgtgcagtgttgtgcctgttagggaaggtgcgaataagcggggaaattcttctcggctgactcagtcatttcatttcttcatgtttgagccgattttttctcccgtaaatgccttgaatcagcctatttagaccgtttcttcgccatttaaggcgttatccccagtttttagtgagatctctcccactgacgtatcatttggtccgcccgaaacaggttggccagcgtgaataacatcgccagttggttatcgtttttcagcaaccccttgtatctggctttcacgaagccgaactgtcgcttgatgatgcgaaatgggtgctccaccctggcccggatgctggctttcatgtattcgatgttgatggccgttttgttcttgcgtggatgctgtttcaaggttcttaccttgccggggcgctcggcgatcagccagtccacatccacctcggccagctcctcgcgctgtggcgccccttggtagccggcatcggctgagacaaattgctcctctccatgcagcagattacccagctgattgaggtcatgctcgttggccgcggtggtgaccaggctgtgggtcaggccactcttggcatcgacaccaatgtgggccttcatgccaaagtgccactgattgcctttcttggtctgatgcatctccggatcgcgttgctgctctttgttcttggtcgagctgggtgcctcaatgatggtggcatcgaccaaggtgccttgagtcatcatgacgcctgcttcggccagccagcgattgatggtcttgaacaattggcgggccagttgatgctgctccagcaggtggcggaaattcatgatggtggtgcggtccggcaaggcgctatccagggataaccgggcaaacagacgcatggaggcgatttcgtacagagcatcttccatcgcgccatcgctcaggttgtaccaatgctgcatgcagtgaatgcgtagcatggtttccagcggataaggtcgccggccattaccagccttggggtaaaacggctcgatgacttccaccatgttttgccatggcagaatctgctccatgcgggacaagaaaatctcttttctggtctgacggcgcttactgctgaattcactgtcggcgaaggtaagttgatgactcatgatgaaccctgttctatggctccagatgacaaacatgatctcatatcagggacttgttcgcaccttccttaggtaacatttagtttggctaaatgtaaagatattgctgttttattgtttgtttttgcgagatgcgccgcaccattccgaagcaaaattcttaaaatgcactcttttagtgctaccgctggattactgtggtgcaactaggttgtactgatgctgtttcagggtttgccttgtataacaaagcaatagatgtgccaaagttggataggagaatattgttatccggataatgcactgatgccgcatccggtgagcgtgccgaaatatgggatgtattccggcacgataagaagggattatttacgtcgctgacgcagactcatcaacacagcagcaaaaccaaacaatgccgtcagcacccacagcggccagttgccggtacgtgcgtatggtgtgagtccggtggtcggcgtcacgttagtggttaacacctcgcgggtgaactgcgggatcatcgcctgaatctcaccctgcgggccaatcaccgccgtaatgccgttgttggtgctgcgcaacagtgggcgcgccagctccagcgcacgcattcgcgccatctggaagtgttgccatggaccaatagatttaccaaaccacgcatcgttggagatagtcagcagatagtcggtatccgggcggaagttatcgcgcacttgctcgccgagaatgatctcgtagcaaatagccgcagtaagctcaataccatttgccgacagcggcggctggatatatggcccacggctgaacgacgacatcggcagatcaaagaacggtgctaacggacgcagaatcgactccagcgggacaaactcgccaaacggcaccagatggtttttgttatagcgatcggctgattcgtagctgtacggcgcacctttacccagcgtgatgatggtgttgtaggtatcgtagcggttctgcttattgagacgcgcgtcgacaatcccggttaccagcgagctacctttatcacgcaactcaccgtccagtgctttgaggaacggttgctgattaatttccagatcggttatcgccgactccggccagataatcaacgatgatttgcccatcagcggtgccgttgcgttgtagtaaatcttcagcgtattaagaagctggccttcgtcccatttcagcgattgcggaatatcgccctgaaccatcgaaacctgaatggttttctccggttgtggggtaaaccactggatgtaacgcagcgggaagggaagggcaaacagcacgacggccaccaccagcggacgccagttgcgtttgaccaacgccagtgccagcaggccactaaccatcatcagcaggaagttaatggcttccacgcccattatcggtgccagcccttttaacgggccatcaatctggctatagccgaactgtaaccacgggaagccggtcagtacccaaccgcgcagaaactcggtcacttgccagagggcaggggcggcaatcgctacgcgcagccaggtggttttcggccacagacgcgacagcacgccagcaaacagtccggtatacagcgacaaatacgccgccagcagcaccaccaggaagatgttaaccgggccaggcattccgccaaaggtcgcgatgctgacatagacccagttaataccgctgccaaagaggccaaatccccagcaaaagccaatagcggcagactggagtggacggcggttaaaggtcaacgcctgaagccccatcagcgaaataatcgccgcaggccagacgtcgtaaggagagaaggccagcgttccgcaggcaccgaataataacgccagcagcaggcgaatgcgctggcgttcaattaatgaggcaaaagccatgtagttatctatccagtttcggttttattcatccagcttcggctggggtgagtcatccgggattttgacatgaacctgaataatacgccgactgtcggccatcgccactttgaactggtaaccgtcgatgtcgatagtttcgccacgcgccggaagatgcccaaatgcctgcatcaccagaccaccgatagtgtcgacttcttcatcgctaaagtgggtgccgaacgcttcgttgaagtcttcaatggaagccagtgcgcgtacggtccaggtatgacgactcagctgacggaagtcgatatcatcttcttcgtcatactcgtcttcaatctcaccaacaatcagttccaggatgtcttcaatggtcaccagaccggaaaccccaccgaattcgtcaataacgatcgccatgtggtaacgctgagagcgaaactctttcagcatccggtctacgcgcttactttcaggaacgacaaccgcctgacgtaacactttgtccatgctgaaggcttcagcatcgctgcgcataaacggcagcaagtctttcgccatcagaatcccttcaatgtgatctttgtcttcgctaatcaccgggaaacgtgagtgggcggactcgatgatgacatcaagacattcgtccagcgtctggttgcgtttcagggtaatcatctgggagcgggggatcatgatgtcgcgaacgcgttggtctgcgatgtccatcaccccttcgagcatatcgcgcgtatcttcgtcgataaggtcgttctgcccggaatcacggatcagcgccagcagttcgtcacggtttttcggttcaccgtggaaaagttggctgagtaacagggagaaaaatcccttcttgttgcttatcgtgtcactactgtgtgaattgtcgtcgctcatggcgtcgtatgggttctcatgttagttaatcaaaacgccgtcgttaatcaccaacggcggggacgtctgccagtcaaatgcctggcaaattattctttctcggcaatgtacggatcctcatagcccagagcaagcataatctctgtttcgagggcttccatttcttctgcttcgtcatcttcgatgtgatcgtaacctaacaaatgcagactgccgtgcaccaccatatgcgcccagtgcgcctccagtggtttgccttgctcctgagcttccttctcaaccacctgacggcagataaccagatcgcccagtagcgacatttccatgccaggcggcacttcaaacgggaaggagagcacgttggtcggcttatccttaccgcgataggtcagattcagactgtggctttcggcggtatcgaccacgcgaatcgtcacttccgattcttcctgaaactgcgggatcaccgcattcagccatgtctgaaactggctctcttccggtaacccggaattatcttcacatgccagttgtaaatcgaggatcacctgactcatttttgttcctgttcttcgcgcttgcgttctgctgccagcgccgcttttcgtttttgttcggcttcttcccaggcttcataggcgttaacgatacgcgccaccacagggtgacgaaccacgtcttcgctgtggaagaagttaaagctgatctcttcgacatcggccagcacttcgatggcgtgacgtaagcctgatttagtattacgcggcaggtcgatctgtgtgacgtcgccggtgataaccgcttttgagttaaaaccgatacgggtcaggaacatcttcatctgttcgatggtggtgttctggctctcatcgagaatgataaacgcgtcgttcagcgtacgaccacgcatataggccagcggtgcgacttcaataacgttgcgctcaatcagtttctcgactttctcaaagcccagcatttcaaacagcgcgtcgtacagcgggcgcagatacgggtctactttctggcttaaatcgccaggcaggaagcccagtttctcaccggcttctactgccggacgagtcagcagaatacggcgaatttcctgacgctccagggcatcaactgccgcagccactgccaggtaggttttacccgtacccgccgggccaacgccgaaggtaatgtcatggtcgagaatattggcgatgtactgcgcctggtttggcgtgcgcggcttaattacgccgcgtttggttttgatattgaccgctttgccgtactccggcacgctctccgcgctttgctccagtacccgcgcttctttaatcgcaaggtggatctgttccggttcgatatcctgaatctgaccgcgcatcggggcagtatcgacatacaggctacgcagaatgtctgccgcagcggtgacgcaaatcggacggccggtcagtttaaagtggttatcgcggcgattgatctcgatgccgagacggcgttcgagctgcttgatgttgtcatcaaacgggccgcacaggctcaacagacgcgcattgtctgctggctccagggtgatttcgcgagtgtctatgttcaaaccgttcctcttatctgtatgccgccggaagctgaacattcaccggcctataaggaaattattcacgccacaggaaaaaggcgcaagcattgcaataaagatggggataaagagagaaaaaacaaggcccaccggaacggcaggcctgagaattacggctgataataacccacgccaaggtcgttttctttgcgggtacgggcaatcactgattccggtgtttctgccacgcgcagacccatttcatcttcagtacgcaccactttaccgcgcagagagttcgggtagacgtcggtaatttctacatcgacgaatttaccgatcatatccggcgtgccttcgaagttgaccacgcggttattttccgtacgcccggaaagctccatgatgctcttacgcgatgtaccttctaccagaatacgctgggtggtgccgagcatccggcggctccacgccatcgcttgctgattaatgcgctcttgcagaatatacagacgctgcttcttctcttcttccggaacatcatcaaccatatcggcggctggtgtacccggacgtgcagagaagataaagctgtagctcatgtcgaaattgacgtcggcaatcagcttcatcgttttctcgaagtcttcggtggtttcgccagggaagccaacgatgaaatcagaactgatctgaatatctggacgcgccgcacgcagtttacggatgatcgctttgtactccagcgccgtatgggtacggcccatcaggttcagaatgcgatcggaaccgctctgtaccggcagatgcaggaagctcaccagctccggcgtgtcgcgatacacttcgatgatatcgtcggtgaattcgatcggatggctggtggtaaagcgaatacgatcgatcccgtcgatcgcagcaaccagacgcagcagatcggcaaacgatccggtggtgccgtcgtagttttcaccacgccaggcgttcacgttctgaccgagcaggttgacttcacgcacgccctgagccgcaagctgggcaatctcaaacagaatatcgtcggacggacggcttacctcttcaccacgggtgtaaggcaccacgcagtaggtgcaatatttattgcagccttccatgatggagacaaacgcggtcggcccttcggcgcgcggttccggtagacggtcaaacttctcgatttccgggaagctgatatctacaaccgggctgcggtcgccacgcacggagttgatcatctccggcagacggtgcagcgtttgcggcccaaaaataatatcgacatagtgggcgcgctggcgaatgtgctcgccttcttgcgatgccacgcagccaccgacgccgataatcaggtctggattcttctcttttaacagtttccagcgacccaactgatggaagactttttcctgagccttctcgcggattgagcaggtgttcagcagcagcacatccgcttcttccgccacgtcggtcagttgatagccgtgggtggcatccagcagatcggccatcttcgatgaatcgtactcgttcatctgacagccccaggttttaatatggagttttttggtcatcgacttgctcttgcgaaatagtagccaggaatgcagggcgcatagtgtaatgctttgctgccgttgtgaccagtatgagcgttatcagcccttaggggtaaaaatcctgtaaacttaaagcatattgctaacaggatgattgaccatgacaaatcaaccaacggaaattgccattgtcggcggaggaatggtcggcggcgcactggcgctggggctggcacagcacggatttgcggtaacggtgatcgagcacgcagaaccagcgccgtttgtcgctgatagccaaccggacgtgcggatctcggcgatcagcgcggcttcggtatcattgcttaaagggttaggggtctgggatgcagtacaggctatgcgttgccatccttaccgcagactggaaacgtgggagtgggaaacggcgcatgtggtgtttgacgccgctgaacttaagctaccgctgcttggctatatggtggaaaacactgtcctgcaacaggcgttgtggcaggcgctggaagcgcatccgaaagtaacgttacgtgtgccaggctcgctgattgcgctgcatcgccatgatgatcttcaggagctggagctgaaaggcggtgaagtgattcgcgcgaagctggtgattggtgccgacggcgcaaattcgcaggtgcggcagatggcgggaattggcgttcatgcatggcagtatgcgcagtcgtgcatgttgattagcgtccagtgcgagaacgatcccggcgacagcacctggcagcaatttactccggacggaccgcgtgcgtttctgccgttgtttgataactgggcatcgctggtgtggtatgactctccggcgcgtattcgccagttgcagaatatgaatatggcacagctccaggcggaaatcgcgaagcatttcccgtcgcgtctgggttacgttacaccgcttgccgctggtgcgtttccgctgacgcgtcgccatgcgttgcagtacgtgcagccagggcttgcgctggtgggcgatgccgcgcataccatccatccgctggcggggcagggagtgaatcttggttatcgtgatgtcgatgccctgattgatgttctggtcaacgcccgcagctacggcgaagcgtgggccagttatcctgtcctcaagcgttaccagatgcggcgcatggcggataacttcattatgcaaagcggtatggatctgttttatgccggattcagcaataatctgccaccactgcgttttatgcgtaatctcgggttaatggcggcggagcgtgctggcgtgttgaaacgtcaggcgctgaaatatgcgttagggttgtagccttacaacattgccggatgcgtgccaaccgtaggtcggataagacgcggcagcgtcgcatccgacattgaaggataagacgtgtcaacatcgcattcgacattgaatgaacgcagaaaagcaaaaagctcgccgaagcgagcttttttaatgtggctggggtacgaggattcgaacctcggaatgccggaatcagaatccggtgccttaccgcttggcgataccccaactgggtgcacttacaaggtaagcgtcttgaataaattggctggggtacgaggattcgaacctcggaatgccggaatcagaatccggtgccttaccgcttggcgataccccaacaaattggttttgaatttgccgaacatattcgatacattcagaatttggtggctacgacgggattcgaacctgtgaccccatcattatgagtgatgtgctctaaccaactgagctacgtagccagattgtttcttcgatggctggggtacctggattcgaaccagggaatgccggtatcaaaaaccggtgccttaccgcttggcgataccccatccgtacaacgctttctggtgaatggtgcgggaggcgagacttgaactcgcacaccttgcggcgccagaacctaaatctggtgcgtctaccaatttcgccactcccgcaaaaaaagatggtggctacgacgggattcgaacctgtgaccccatcattatgagtgatgtgctctaaccaactgagctacgtagccatcttttttttcgcgataccttatcggcgttgcggggcgcattatgcgtatagagccttgcagcgtcaacctctttttcaaggaaaattgctcgaaagtgactgtttggttaggttgcgaacagcgtggcgctatattcgtcaattattgtttactttgtgttttttcccaccctacagccattcttttgtcatacaggatgaaattcggaatttaacaatagtggtgggaaattaatctatgaaatactggcctacagtgatgagttgtcaaacagtgatgtggcaaacccggaacatttccttactgcatatcagaatcaacaagcacctcaataactgaaacagccccggatttcaccggggctgtttcgcatttcttacttatacgccgactggtgaacaccaaccgcgcgaccagacggatcgtccattttcttgaacgcttcatcccattcgatcgctttagcggaagaacaagcgacggaaggaccgcccggcacgcactcagcggcgctcggaagcgggaatagttcttcaaagatctcccgatacaagtacgcttctttagaggttggcgtgttgtacgggaagcggaagcgggcagtttccagttgctgatcagaaacctgctgcgcagccacttctttcagggtgtcgatccaactgtaaccgacgccatcggagaactgctctttctgccgccaggccacgcttgcaggcagatacgcttcaaaacattcacgcaggatgtgtttttccattttgccgttaccgcacattttatcctgtgggttaatacgcatcgccacatcaaggaattttttgtcgaggaacggaacgcgtgcttccacgccccaggctgacatcgctttgttggcacgcgcgcagtcatacatatgcagggccagcagtttacgcaccgtctcttcatgcagttctttggcattcggtgctttgtggaagtaaagataaccgccgaacacttcatcagaaccttcaccggacagcaccattttaatgcccatcgccttgatcttacgcgacattaaatacatcggtgttgaagcgcgaatagtggtcacatcataagtttcgatgtggtaaatcacgtcgcggatggcatccagaccttcctgtacagtgaagtgaatttcgtgatgcaccgtgcccagatggtttgccacttcctgggctgctttcagatccggtgaacccggcagacctacagcaaaggagtgtaactgcggccaccaggcttcagagcgttcctgatcttccacgcgacgggctgcgtatttcttggtgatagcggaaataattgaggaatccagaccaccagaaagcagcacaccgtaaggcacatcagacatcagatggcttttaactgaatcttccagtgcctgacgcagctcgtttttgtcggtcacgttatctttcaccgcatcgtagtcgaaccagtcgcgatgatagtaagaacggatttcgccgtcctggctccacaaatagctccccgccgggaactctttaatcgtgcggcaaactggcaccagcgctttcatttctgaggccacatacagctgaccgtgttcgtcataccccatatacagtgggatgatccccagatggtcgcgaccaatcaggtaggcatctttttcgctgtcgtacagtgcaaaggcaaacatgccctgcaagtcgtcgagaaattccggccctttttcctgatacagcgcgaggatcacttcacagtcagacccggtctggaactggtaacgatcgccatattcggcgcgcaatgcctggtggttgtagatttcaccgtttaccgccagtacgtgggttttttgttggttgtagagaggttgcgcccccgcgttaacgtcaacaattgacagacgttcgtgggcgagaatggcgttatcgctggcataaataccggaccagtccgggccacgatgacgcatcaggcgtgacagctcgagggctttcttacgcagctcaactgcgtctgttttgatatcgaatacgccaaaaattgaacacataaccttctccgttaacctggtatttgttgcttgttgtgtttgcttgtttaaaaaaatgccgcaaagcagcactgtgcgcaagcgatttggcggtgaaaaaataaaaaacgtaatggtgattgtcgattggtgaaaaaaggtctggtgtgaggatatatttattgatgaatcgataatttttagcgggttttattgaatgtttatattttacgggggccaaattgctgacaaagtgcgatttgttcatgccggatgcggcgtgaacgccttatccggcctacaaaagcatgaaaattcaatatattgcaggagctgcgtaggcctgataagcgtagcgcatcaggcagtttggcgtttgtcatcagagccaaccacgtccgcagacgtggttgctattcagataacgtcgatttcagcgactgacgggtaaatccagctggggcggaaaggcatactgtcgatatcgtcgagcgacgaaacaccagaaagcaccagaatcgtctccagacctgcctggaagccggccagaatatcggtacgcaggttatcgccgacaatcaccgtttcttccgaatgcgcctgcattttgtttaatgctgcgcggatgatccacgggctgggcttaccaacatagaacggtttgcgcccggagattttctcaatccctgcacacaacgcgccacaagcgggataaaaaccgcgcccgtgggtgtccggattggtggcgataaaacgtgcaccgttagcgacgaaataggctgctttatgcatcatgtcccagttgtaggaacgcgtttcgccaacaatcacgaaatcagggttcacatcggtaatagtgaaaccggctttgtacagttcatgaatcagtgcgccttcgcccaccacatacgctttcttgccttcctggcgacgcaggaaatcggcagtcgccatcgcagaggtataaaacacgctgtcaggtacatcgacacctgcggtggcaaagcggttcgccagatcttgcccagtctgcgaaggatagttggtcagcaacaccagcggcaggcctttatccataatcccgtgcaaaaattccgctgcacccggtacggcgacgttatcgtgcatcagcacgccgtcgatatcgcaaattacatttttaatggtcatggactacccagaatattgacaacaataagcgccactataaaagcacattaattttccagcaaatgctggagcaaaataccgttgagcatggcgcgttttaccagcgcaaaagcgccgattgccgagcggtgatccagctcagaacgtaccaccggcagattagtgcgaaacgccttcagcgcctgggtattaatgcagctttcaatagcagggagcagcactttatcggcttcggtgatttcaccggcaataacaattttttgcggattaaataagttgatagcaatggcgatggttttacccagatgacgaccgacatactcaattacttccgacgccagactatcgcctttgttcgcggctttgcagatagttttgatggtgcagtcgtccagcggcacgcggctctggtagccctgctttaacagattcaacacccgttgttcaatggcagcgttggcagcgatagtttccaggcagccaaagttgccgcagtggcagcgttcacccagcggttcgacctgaatatggccaatttcaccgacgttgccgttgcggccaataaaaatgcgcccgttagagataatcccggccccggttccgcgatggacacgcaccagaatggagtcttcgcaatcctgacttgcaccgaagtagtgctccgccagcgccagactacggatatcgtgaccaacgaaacaggtcactttaaaacgttcttccagagcttctaccagcccccagttttctacctgaatatgcggcatgtaatgaattttgccgctgtccgggtcaacaagccctggcaggatcaccgaaatcgcgatcagctcgcgcagtttgcgctggtagctatcaataaactgagcaatggcattcaacagggcatgttccagcgtttgctgggtacgttccggcagcgggtaatgttcttctgccagcactttgctgctgagatcaaacagagtgatggtggcgtcatgacgaccaagccgtacgccgattgcgtggaaattgcgggtttcggtgacgatggagatagcgcggcggcccccggtggaggcctgctgatcaacttctttgatcagcccgcgttcgataagctgacgcgtaattttggttacgctggcgggggcaagctggctttgctcggcaatctgaatccgcgagattggcccgtactggtcaatcaggcgataaaccgccgcgctgttaagctgttttacgagatcaacattacctatctgagcttgtccgcctggtgtcatactttctcttattgagttacgacctcgttaccgttaacgatggtcttggtgattttaaaatcaggtgtgaatgcagtcaggttggctactttacctgcggcgagtgtgccgagacgtttctcaacgccaatcgcacgcgccggatagagcgtcgccatacgtagcacttcatccagtgcgataccgcaatgttcgaccagattacgcacgccttcaatcatggttaaggatgaaccgcttaacgtaccgttctcatccacacaaagtccgttacggtagtatattgttttacccgcaaaaatgaactgttcaatgttggcacctgctggcgcggtggcgtcagtaaccagacacagtttgtcgcctttcagacgtttagcgttgcgaatgttggcgtaatcaacatgcaggccatcagcaataataccgcaataaatgtcagcttcgtcgaggatcgcgcccgccaggccaggttcacgaccggtaatatacggcatcgcgttgtacagatgggtggcaaaggtaatccccgcgcggaaaccggcttttgcttctttcaacgtcgcgttggagtgaccggcagaaaccacaatcccggcatttgccagtttgctgatgacttccgcaggaaccatttccggtgccagggtcactttggtaatgacgtcggcgttttcacacaggaaatcgaccagcgcggcatcaggcttacgcacaaaattcggattatgggtgcctttttttaccagattcagccacggaccttccagatgcagacctaacgcctgattcggatgttttgccaggtactcgcgcataacgcgcacgccctgtttcatcagctcatcgctggtggtgataagcgtcggcagatagttagtacagcctgatttctcattggctttctgcatgatttccagcgtttccacgctgaccgcttcagcggtgtcgttaaactgtacgccgccgcagccgtttaactgcacatcgataaaaccgggggagagaatggccccgttcagtgaacgttgttcgatctctggcggcagttccgctaccggacagacgcttttaatcaggccatcagcgataacaaccgcgtggtcatcaagaaattcgtggccggtaaagatccggccctgggttaatgcatacattctgacccccgattttaaaaaatattgccctgagcaaggagccagggcagggataacaattacagacctttgatattttctgcttctaattcattgaaatatcttaaagtcttaactttcagctccatggtggaaggttcatcgcacaccatgatcgctttcggatgcagttgcagacagctgatggtccacatatggttcacgcaaccttcaacggcggcctgcagcgccagtgctttctggctacccagcaccagaatcatcacttcttcggcatccagcagtgtaccaacaccgacagtcagggcatattttggcacctgattaacatcgttatcaaagaaacgagagtttgcgacgcgagtgtcatgagtcagggttttgatacgagtacgagaagccagagaagacgccggttcgttaaatgcaatatgaccgtcgttacctacaccgcccataaacagatgaatttttccgtaagaacggattttttcttcatactggcggcactcggcgtcgatatccggggcgttgccgttgagaaggttgatgttttctgctggaatatcaacgtgatcgaagaaattacggtgcataaagctgtagtagctttccggatgctctttcggcagaccgacatattcgtccatgttgaaggtgacaacgtgcttaaagctgacctggcctgctttatgcatttcgactaacgctttataggtggtcatcggcgtgccgccagtcggcaggcccagtacaaacggacgatcggcagtcggtttgaacgcattgatacgattgacgatatggcgagcagcccatttgccgacctgttcagcggtagtcagggggatcagtctcattattcacctcaataagtaaaatgtaagccgttggcggattaggcatctttaagcgtaacctggatttgcgcagacaggcgtcaatccgacctgattttttgaatgataaaataagttttctggtttagccagtaaaagggagtgataataacgatatttggtgacaaaactcacaaaagacacgcgtttaatttgcgatacgaattaaattttcacacactctgtagcagatgatctaacaatctgattacagaacatcggcagtacaatttgcagcaaaataaaaatacggcttgaaacgagccaaatagggttctcgtagggggaataagatgaatattttaggttttttccagcgactcggtagggcgttacagctccctatcgcggtgctgccggtggcggcactgttgctgcgattcggtcagccagatttacttaacgttgcgtttattgcccaggcgggcggtgcgatttttgataacctcgcattaatcttcgccatcggtgtggcatccagctggtcgaaagacagcgctggtgcggcggcgctggcgggtgcggtaggttactttgtgttaaccaaagcgatggtgaccatcaacccagaaattaacatgggtgtactggcgggtatcattaccggtctggttggtggcgcagcctataaccgttggtccgatattaaactgccggacttcctgagcttcttcggcggcaaacgctttgtgccgattgccaccggattcttctgcctggtgctggcggccatttttggttacgtctggccgccggtacagcacgctatccatgcaggcggcgagtggatcgtttctgcgggcgcgctgggttccggtatctttggtttcatcaaccgtctgctgatcccaaccggtctgcatcaggtactgaacaccatcgcctggttccagattggtgaattcaccaacgcggcgggtacggttttccacggtgacattaaccgcttctatgccggtgacggcaccgcggggatgttcatgtccggcttcttcccgatcatgatgttcggtctgccgggtgcggcgctggcgatgtacttcgcagcaccgaaagagcgtcgtccgatggttggcggtatgctgctttctgttgctgttactgcgttcctgaccggtgtgactgagccgctggaattcctgttcatgttccttgctccgctgctgtacctcctgcacgcactgctgaccggtatcagcctgtttgtggcaacgctgctgggtatccacgcgggcttctctttctctgcgggggctatcgactacgcgttgatgtataacctgccggccgccagccagaacgtctggatgctgctggtgatgggcgttatcttcttcgctatctacttcgtggtgttcagtttggttatccgcatgttcaacctgaaaacgccgggtcgtgaagataaagaagacgagatcgttactgaagaagccaacagcaacactgaagaaggtctgactcaactggcaaccaactatattgctgcggttggcggcactgacaacctgaaagcgattgacgcctgtatcacccgtctgcgccttacagtggctgactctgcccgcgttaacgatacgatgtgtaaacgtctgggtgcttctggggtagtgaaactgaacaaacagactattcaggtgattgttggcgcgaaagcagaatccatcggcgatgcgatgaagaaagtcgttgcccgtggtccggtagccgctgcgtcagctgaagcaactccggcaactgccgcgcctgtagcaaaaccgcaggctgtaccaaacgcggtatctatcgcggagctggtatcgccgattaccggtgatgtcgtggcactggatcaggttcctgacgaagcattcgccagcaaagcggtgggtgacggtgtggcggtgaaaccgacagataaaatcgtcgtatcaccagccgcagggacaatcgtgaaaatcttcaacaccaaccacgcgttctgcctggaaaccgaaaaaggcgcggagatcgtcgtccatatgggtatcgacaccgtagcgctggaaggtaaaggctttaaacgtctggtggaagagggtgcgcaggtaagcgcagggcaaccgattctggaaatggatctggattacctgaacgctaacgcccgctcgatgattagcccggtggtttgcagcaatatcgacgatttcagtggcttgatcattaaagctcagggccatattgtggcgggtcaaacaccgctgtatgaaatcaaaaagtaatctgctttatgcctgatgcgacgcttgagcgtcgcatccaacaatgacaagcggtggagatcttctctgccgctttttttttcatcaatcatccccataatccttgttagattatcaattttaaaaaactaacagttgtcagcctgtcccgcttataagatcatacgccgttatacgttgtttacgctttgaggaatccacgatgagtgaggcagaagcccgcccgactaactttatccgtcagatcatcgatgaagatctggccagtggtaagcacaccacagtacacacccgtttcccgccggagccgaatggctatctgcatattggccatgcgaaatctatctgcctgaacttcgggatcgcccaggactataaaggccagtgcaacctgcgtttcgacgacactaacccggtaaaagaagatatcgagtatgttgagtcgatcaaaaacgacgtagagtggttaggttttcactggtctggtaacgtccgttactcctccgattattttgatcagctccacgcctatgcgatcgaactgatcaataaaggcctggcgtacgttgatgaactgacgccggaacagatccgcgaataccgcggcaccctgacgcaaccgggtaaaaacagcccgtaccgcgaccgcagcgttgaagagaacctggcgctgttcgaaaaaatgcgtgccggtggttttgaagaaggtaaagcctgcctgcgtgcgaaaatcgacatggcttcaccgtttatcgtgatgcgcgatccggtgctgtaccgtattaaatttgctgaacaccaccagactggcaacaagtggtgcatctacccgatgtacgacttcacccactgcatcagcgatgccctggaaggtattacgcactctctgtgtacgcttgagttccaggacaaccgtcgtctgtacgactgggtactggacaacatcacgattcctgttcacccgcgccagtatgagttctcgcgcctgaatctggaatacaccgtgatgtccaagcgtaagttgaacctgctggtgaccgacaagcacgttgaaggctgggatgacccgcgtatgccgaccatttccggtctgcgtcgtcgtggttacactgcggcttctattcgtgagttctgcaaacgcatcggcgtgaccaagcaggacaacaccattgagatggcgtcgctggaatcctgcatccgtgaagatctcaacgaaaatgcgccgcgcgcaatggcggttatcgatccggtgaaactggttatcgaaaactatcagggcgaaggcgaaatggttaccatgccgaaccatccgaacaaaccggaaatgggcagccgtcaggtgccgtttagcggtgagatttggattgatcgcgccgatttccgcgaagaagctaacaagcagtacaaacgtctggtgctgggtaaagaagtgcgtctgcgtaatgcttatgtgattaaggcagaacgcgtcgagaaagatgccgaaggtaatatcaccaccatcttctgtacttatgacgccgataccttaagcaaagatccggcagatggtcgtaaagtcaaaggtgttattcactgggtgagcgcggcacatgcgctgccggttgaaatccgtttgtatgaccgtctgttcagcgtgcctaacccaggtgctgcggatgatttcctgtcggtgattaacccggaatcgctggtgatcaaacagggctttgctgaaccgtcgctgaaagatgcggttgcgggtaaagcattccagtttgagcgtgaaggttacttctgcctcgatagccgccattctacggcggaaaaaccggtatttaaccgcaccgttgggctgcgtgatacctgggcgaaagtaggcgagtaattttaagtttcgctatgccggatggggcgtttacgtcgcatccggcaaggaacagacaaacagtttcaaacgctaaattgcctgatgcgctacgcttatcaggcctacatgatctctgcaatatattgagtttgcgtgcttttgtaggccggataaggcgttcacgccgcatccggcaagaaacagcaaacaatccaaaacgccgcgttcagcggcgttttttctgcttttcttcgcgaattaattccgcttcgcaatttatccataaaataaatttaaaataacaaaacataattaaataaaatgtaaccgctttcatcttgctggaatttcacgcttttattcttctgcaagcctttcaaccgcaaacttaagccttgtaacaaaaatcatcaaaatatgtgcggttgctcatgttcttacattctggttacagaaagagattgataattcgcgtcgcgaaaaatagtctgttcctgtagtcagcgagacttttctcaacgctacttttttaatttttattttttcgctgttcacctttggtgcagcaatttatacgtcaaagaggattaacccatgcgtacgtttagtggcaaacgtagtacgctggcgctggctatcgccggtgttacagcaatgtcgggctttatggcaatgccggaggctcgcgccgaaggattcatcgacgattcaaccttaaccggcggtatctattactggcagcgtgaacgcgaccgtaaagatgttaccgacggcgacaaatacaaaaccaacctttctcactccacctggaatgccaacctcgattttcagtccggttatgctgctgatatgttcggccttgatattgctgcgtttacggcgattgaaatggcggaaaacggcgacagctcccacccgaacgaaatcgcgttttcaaaaagtaataaagcctatgacgaagactggtccggcgacaaaagcggtataagcctgtataaagctgcggccaaatttaaatacggtccggtttgggcgagggcaggttacattcagccaactggtcaaacgctgttagcgccgcactggagctttatgccaggtacttatcagggggcggaagccggggcgaattttgattacggcgatgctggtgcgttgagtttctcctacatgtggaccaacgaatacaaagcgccgtggcatctggaaatggatgagttttatcagaacgataaaaccaccaaagttgattatctgcactcctttggggcgaaatacgacttcaaaaataacttcgtactggaagcggcatttggtcaggcggaagggtatatcgatcaatattttgccaaagccagctacaaatttgatatcgccggtagcccgttaaccaccagctaccagttctacggtacccgagataaagttgacgatcgcagcgtcaacgacctttatgacggcaccgcctggctgcaagcgttgacctttggttaccgggcggctgacgtagtggatttgcgcctcgaaggcacctgggttaaggctgacggtcagcagggatacttcctgcaacgtatgactccaacctacgcttcctcaaacggtcgcctggatatctggtgggataaccgttctgacttcaacgccaacggcgaaaaagcggtcttcttcggtgcgatgtatgacctgaaaaactggaatcttccaggcttcgccatcggcgcttcctacgtttacgcatgggatgctaaacctgcgacctggcagagcaatccggatgcgtactacgacaaaaaccggactattgaagagtctgcctacagcctggatgcggtctataccattcaggacggtcgcgccaaaggcacgatgttcaaactgcatttcaccgaatacgacaaccactccgacatcccaagctggggcggtggttacggcaacatcttccaggatgagcgtgacgtgaaatttatggtaatcgcaccattcaccatcttctgatgcccgacgcggcaggttttgtgcctgccgcacgtttgaggaatttgctatgaaaaaactgattctcatcgccataatggcatcggggctggtagcttgtgcgcaatcaaccgcgccacaggaagacagtcgtctgaaagaggcatacagcgcctgtatcaacaccgcacaaggttcgccagaaaaaattgaagcctgccagagcgtgttaaacgtgctgaagaaagagaaacaacatcagcagtttgccgaccaggaaagtgtacgcgtactggattatcagcagtgtctgcgtgcaacgcaaaccggaaatgatcaggcggtgaaagccgattgtgataaagtctggcaggaaatacgcagtaataacaaataagtgagagctgtaactctcgcttttcttatttcccttgcataaaaaagccaacccgcaggttggcttttctcgttcaggctggcttatttgccttcgtgcgcatgttcatcttcgcggcaatcgccttcggcacagtgaccgtaaagatagagactgtggttagtcaggcgaatgccatgttttgcggcaatttcacgctgacgcgcttcgatggaatcatcactaaattcgataaccttgccgcagtcgaggcagatcaggtgatcgtggtgatgttgctgtgtcagttcaaatacggatttaccgccttcaaaattgtggcgggtgacgataccagcgtcgtcaaactggttcagtacgcgatataccgtagccagaccaatttcttcacccatatcgatcagacgtttgtataaatcttccgcactgacgtgatggttgtccggctcctgaagaacttccaggatttttaaacgaggaagcgttactttcaggccagctttctttagggcggtattgttatcagtcatgcggaatctgtcctgttactaagcggttcacttcattagaagaagtgacagaatttgctcttgagataatgcgtatcattatagaattgccacgcctaaatgaaaaccacaagtccctggcaaatattgttaataaaaacgtggcacagcttacatttacaacggcaaggccacttgaacaccgggacattgtacaggtacaacagcaaaagttacaaatttgtagcaattattttgattggcattatctattaatacggcgtagacatgagtctacgccgcatcacatcaggcattgagaatttcgtcgagatgcaactcttcagaaatctgtttaacccatttttctacacgttcagcggtcagttccggctgacggtcttcgtcgatagccagaccgacaaagtggtcgtcatctgccagaccttttgatgcttcgaaatgatagcccgcagttggccagtgaccaacgatggttgcaccgcgcggttcaatgatgtcgcggatggtgcccaatgcgtcgcagaaatattcggcgtaatcttcctggtcaccacaaccaaacagcgcaaccagtttgccgttgaaatcaatctcttcgagagtcgggaagaagtcatcccagtcacactgcgcttcgccgtaataccaggttgggatgcccagcagcagaatgtcataagcttccagatcttctttgctgctttttgcaatgtcatggacatcggcaacgtctttaccaagctgtttttgaatcatttttgcgatattttcggtattaccggtgtcgctgccgaaaaagatgccagtgatagccatgagtgaaataacctcttgaaacttattgaaatgggggtggaaaattgcccacggataaaggcaatcatagcagaacaggcagtcttgcggaatcagcaaacgagcaggactgcacactgtgctacatgaaagtggaaatttaaacgatgccctgactacgcagcgccgccagttgctgcattaacatctcttcgatcagttcgctacggctcatattgcgcgactccgccagctcgttcagcgcctcgacagcttccgcgttcagcttcagttcgacacgcttaaggccacgtactttgtcgcgttttagctggttgcgtttattaatacgcagctgttcatcgcgcgaaagcggattagttttcggtcgtcccggtcgacgctcgtgcgcgaacagatctaatgtcgtacggtccgtttgttctttggccatgatcttggtgacttcgggggaaacaatcagccaggcctctgcccggatggatagcgcgccataatacatcagcgcgatgagtcacgccaacgcccacgcgcggaaagcgacgcggacgctgggtttttaatcagttgcgttaatcattgagatagcgacggatagcgcgtaataccgcatccggtttttcagcatggacccagtgacccgcgcctgcaatcacatgcgcccgtgcctgtggaaattgagccagtaaatcatcacggtactgctcgctaacatacggagaattgccgccagggataaacagggcagggtgatcccatgccgggattttctcccaacctacaatatgcggatactgatcccacaataccggcacgttaaagcgccactccccgtcaacaaaagatttcagcagaaactgaatcaccccttcttcattaagatgctggcgcattattgctgctgcttgctggcgagtttgtgcgtccgattcactgaccgcgttgatagccgcaaaaatctcatcatgacggcgtacgtgatagtcgaccggcgcgatatcgatcgccaccagtttatcgatgcgatcggaggctagtgcagtaagtgccattaccgctttaccgcccatggagtgaccgataaatgttgctttgtcgatctgctgtgcatccagagtatcaacaagatcctgcgccatcgccgggtaattcattaccggatctctcggtgaaagaccgtggttacgcatatcaacctggatgatattgtgatcgtttaccagatcgcgagccagtacgccaaggttgtcgaggctgccaaacagaccgtggacaagaacgatgggagaattattgtgctggttttgtgcagtttgcgcgcggatattcaatttcatggcaaagttctttttttcgcgttgtcgggttagggtattatgttgaccattgtgccacagggctgcaacaaataaggtttattccgagtttttctgcaagccaggcttgacgctatccgctgccgggatttattcatatactcctggcgacttgtattcagctaagacactgcactggattaagatgaaaacgattgaagttgatgatgaactctacagctatattgccagccacactaagcatatcggcgagagcgcatccgacattttacggcgtatgttgaaattttccgccgcatcacagcctgctgctccggtgacgaaagaggttcgcgttgcgtcacctgctatcgtcgaagcgaagccggtcaaaacgattaaagacaaggttcgcgcaatgcgtgaacttctgctttcggatgaatacgcagagcaaaagcgagcggtcaatcgctttatgctgctgttgtctacactatattctcttgacgcccaggcgtttgccgaagcaacggaatcgttgcacggtcgtacacgcgtttactttgcggcagatgaacaaacgctgctgaaaaatggtaatcagaccaagccgaaacatgtgccaggcacgccgtattgggtgatcaccaacaccaacaccggccgtaaatgcagcatgatcgaacacatcatgcagtcgatgcaattcccggcggaattgattgagaaggtttgcggaactatctaaaacgttgcagacaaaggacaaagcaatggcaatccacaatcgtgcaggccaacctgcacaacagagtgatttgattaacgtcgcccaactgacggcgcaatattatgtactgaaaccagaagcagggaatgcggagcacgcggtgaaattcggtacttccggtcaccgtggcagtgcagcgcgccacagctttaacgagccgcacattctggcgatcgctcaggcaattgctgaagaacgtgcgaaaaacggcatcactggcccttgctatgtgggtaaagatactcacgccctgtccgaacctgcattcatttccgttctggaagtgctggcagcgaacggcgttgatgtcattgtgcaggaaaacaatggcttcaccccgacgcctgccgtttccaatgccatcctggttcacaataaaaaaggtggcccgctggcagacggtatcgtgattacaccgtcccataacccgccggaagatggtggaatcaaatacaatccgccaaatggtggcccggctgataccaacgtcactaaagtggtggaagacagggccaacgcactgctggccgatggcctgaaaggcgtgaagcgtatctccctcgacgaagcgatggcatccggtcatgtgaaagagcaggatctggtgcagccgttcgtggaaggtctggccgatatcgttgatatggccgcgattcagaaagcgggcctgacgctgggcgttgatccgctgggcggttccggtatcgaatactggaagcgtattggcgagtattacaacctcaacctgactatcgttaacgatcaggtcgatcaaaccttccgctttatgcaccttgataaagacggcgcgatccgtatggactgctcctccgagtgtgcgatggcgggcctgctggcactgcgtgataagttcgatctggcgtttgctaacgacccggattatgaccgtcacggtatcgtcactccggcaggtttgatgaatccgaaccactacctggcggtggcaatcaattacctgttccagcatcgtccgcagtggggcaaagatgttgccgtcggtaaaacgctggtttcatctgcgatgatcgaccgtgtggtcaacgacttgggccgtaaactggtagaagtcccggtaggtttcaaatggtttgtcgatggtctgttcgacggcagcttcggctttggcggcgaagagagtgcaggggcttccttcctgcgtttcgacggcacgccgtggtccaccgacaaagacggcatcatcatgtgtctgctggcggcggaaatcaccgctgtcaccggtaagaacccgcaggaacactacaacgaactggcaaaacgctttggtgcgccgagctacaaccgtttgcaggcagctgcgacttccgcacaaaaagcggcgctgtctaagctgtctccggaaatggtgagcgccagcaccctggcaggtgacccgatcaccgcgcgcctgactgctgctccgggcaacggtgcttctattggcggtctgaaagtgatgactgacaacggctggttcgccgcgcgtccgtcaggcacggaagacgcatataagatctactgcgaaagcttcctcggtgaagaacatcgcaagcagattgagaaagaagcggttgagattgttagcgaagttctgaaaaacgcgtaaacacatttaataaaaaaagggcggtcgcaagatcgcccttttttacgtatgacaaacacagaattgcctgatgcgctacgcttatcaggcctacgaggatggtgcaatatattgaatttaagcgattttgtaggccggataaggcgttcacgccgcatccggcaaaaacaacgaacactttgtcaacaaactgagtagctcaaggaaatcccaatgaagaccaacaggagtctggtcgtcatagtgtcactaattaccgccacattactgctgactgcatgcgcccaacctgaacaatcatcattagctggcgactggttactgacccctaaagataaaaccagaggattaacgggtagcattgcggtaaatattgcacctttccggtgtaagacaaattgccgtggtgataacttacctgataatacccgccgctggcagttgtcaggcgggaacgaaaaagaacttacttatcttcataatatgtcagcacaagaaaaggtcggtttaaatcccggttggcaatgctacacctcattttttatgcgggtttgccagggcaagcccggcactcgaccgatagtcaatgaggattatgtcagcgaaagcggattttttggctcgatgatgcatgtcgggattattgagttacgacgctgccagtcagaaaattgccagcaagaattgaaagcgataaatacacattaaaatagtgagtccgggaatgaaacccggacctgaacatgtcttattgcgtgaatgtttctttcatttgatactgcatttcccagagttcagtaagcgaaataacttttcttgttcttgcttcttcactttgtacccataagaaagggtagaacgtgaaggcttccgttgccgataattttattacgtcttctcgccattgctgccatcgtacattttcatagaaggtatctaaatcaccggataatgcccactgaagaaactcagaatatccaacttccagactttcccaattcagcgtatctggcgcaaaataataaacgcagccagtatcttccccaagatcgccaccattaagagcaaaaattacccctgcgacatcgtcagcgatgggtaaagcccgcacgcctgcgaattcagggcgttgtgtccaacttactggatctcgtggcaaccgggggtgaccagatcctgctatgcgtaactaaccattatcaatcagcagacctccggagccatagacaagcgcacccatcggtgattttgttgtcacctgtaattgataaagtgcggtttcggctaaatctttattaaccggtaagagttcggtatggtttgtggcgtcttttaaccagttctggattattggccaggctgaatcttcagtatttactaactgattcatttcacgcatcgctacttgctccttgtgtgctacggtgtcatttatgatgaggaattgtatggaacattttttaaatattaagttccttatatttgaataaaaaatgactttatccatacattgccacttttttcaaagcataaaccgatacccaataccggtttcagtaataaaatggcgaggccgggccggatcctgttccagtttttgtcgcagatgccccatataattacgcaaatagttgctgtgttcgatcgcgtttagaccctacatctgccggatgcggcataaataacgaactatttgccaacaaacagaaagggcgatcattcaatcgcccttttttactttgttttattaaccgtgtttatttttcagttcaaagcgtggtgataccagaccatacagtgtccaaccaaggaaggtcacgatggaaccgtacagcatggcttcttccccggatgagtacagcgcataaaagctatacatcgcgccaacaaaagcaacaaagtttgcaactttcgcttttgaggggggcacattagcgaccttctgaataatgactaatgccgccattgacagaatatacggaatgatattggtcaccacggccaggttaaccagcacgttgaactgactgtttagcgacgggctaatggtcatcagtgccaatccactctgaataatcacaatggtcaacattccctgcaccggtgcatccactttggttacacgggagaaaattttagggaagtagccttcatcagatgaagatttaaacacctgggcaatggtgaactgccagccaagtagcgaaccgcagcaggacatcaccatcagcgccataatgactttacccacttccggcgtgaacatctgcgcgaaggccagaccaaatggtgccgttgaatttgccagctccatatttggcacaatcccggcaatcacgttggtggagacgatataaatcaccgccgcacctaacgtaccgccgagtaccgcgattggcacattacgttccgggttttccactacatcagtattcgcacacgcagactccagaccaagaaaagcccacagcgtcatagcgatggaagaacctaccgcactgaagaacggtgcatgatgcggattccaggaatcaacgtacagcgtcgggctaaaccagaaccagccaataatgcacagaccgacgaccggaataatgaccccccacacggtaatgctactgatttgcccggtaatgcgcgcaccaccaaagttagccacggtacaaatccacagcaccccgatggtcgcaagaccaatctgcactggcgacaaactcgcgccgagcagttcggtgccgtaaccaaccgccgaaatagcaatcgcgacgttagcaatcagcagtgagacgccgtaggtatagttcgccataaagttaccggatttaccgaaagcatactcggcataaccgcccataccgcctgatttacggctgaacataccgcattttgcgaatgcccatgccagtgccattgagcctacggctgtcaccagccaggagataattgagattgtcccgacttcggcaagctttgtcggcagcatgatgataccggagcccatcatgttgaccatcgtcagtatggttaactgaacgacgcccattttgttcgatttagcctgactcataatttttcccctttcaacagggtgctttgcgcatcacgaggcttgatgacatagcaccaaacttgcttacgaccatcatgttcttcgatatagacaccctgcagctccggtgcaaaacctggcagcaggttgatcccttcttccagagcgctgaagtaacgcagaacagcaccaccccagatttcacccggaacaacacacagcacacccggaggataaggaagcgcaccttcggcagcgatacggccttctgcatccggcagacgaaccagttccacttcaccgcgtaaataggcgtagttggcttcttgcggattcatgctgacgcgtgggaagtgctccttacggaacatctctttttgcagttgtttcacgttgtggcgggcatacaaatcatgcatttcctgacacaactgacgcagggtataaccggcgtagcgctcttcatgctgtttgtagatggaaggtagcacttctgctaatggcgcgtcggactcaagcagtttttcgaagcgtaccagcagggcaacaagttgctgaagtttggccatatcttctgccggagtcagcaggaagaggatggagttaagatcgcatttttccggcactacgccattttcgcgcaggaagttagcaagaatcgtcgcgggtacaccgaacgcttcatattcgccgttacgtgcatcaatacctggggttgtcagcaacagtttgcatggatcgacaaagtattgattctctgcatagccttcaaaagaatgccagtgttcccctggtacaaactggaagaagcgcagatcaaccgcaatttgcgctgtttcatacgactgccagggtttaccatccaccagttcaggtacgaacggacgaatatgctgacagttatcgaggatcagtttgcgggcattaatgccatttaccacacaatccatccacatattacgaccgctgacaccttcatgcattttggcgttgatattcagtgcggcaaacagcggatagaacgggctggtggaggcgtgcatcataaaggcgttgttcatgcgtttgtgcggtacataacgctgttgccctttgatgtggctgtcttttttatgaatttgtgaagtctgagaaaaaccagcctgttgtttatgcacagattgcgtaaccagaatacccggatcgttctcattaagatccagcaacagcggcgaacagtccgccatcatcggaataaactgttcatagccgacccatgctgagtcaaacaggatgtagtcacacagatgaccaattttatccaccacttggcgggcgttataaatcgtaccgtcgtaggtgcctaactgaatcacagcgaggcggaaaggacgagcctcttttgcccgctgcggtgcgacttccgcgatcagctcacgcaggtaactttcttcaaaacagtgcgcatcaatgccaccgataaagccatacgggttacgtgccgtttccagataaaccggtgttgcaccagcctgtagcaacgctccgtggtggttagatttgtggttattgcgatcaaacagcaccagatcacccggtgttagcagggcgtttaaaaccactttgttagaagatgaagtgccatttaaaacgaagtaggttttatcggcattaaacacttttgccgcatgttgctgtgcaatgcatggcgcgccttcgtgaatcagcagatcgcccatcgctacgtcggcgttgcacaagtcggcacggaacagcgcctcaccaaagtattccacaaactgattccccgccggatggcgacggaaaaattcgccgccctgatgaccagggcaatcaaacgcgctgttaccttgattgacataatcgaccagtgcgcggaagaaaggtgggcgcagttgagtttcataatggctggcagcggtttctaactggcgaccataaaattctcgtcgcgattcgcaattctcaaagacacccgaaatacggggcaaatactctgcgggtacacgttcttgattttcagtagcaataaataccgggatgccataacccgtggcatcgatttcatcgagttttccgcatgtaacatcgttgagcgataaaactattgccgccacatcgatattacgactttcattaatgtagatacattctcgctgcgtggtaaaacagtccgggcaagaatcactaaccgcaatttttaattttgacatttttcatctctttattttaggtaatagcaggtcctcaatttctcgaatgagaaatcgatcgtgccggaaaaaagcaaagttaccccgctgataaataaatcaggtagattgcttttttcagaatgcagaaacccttaccagtcaggtggctgataatacaagggttaacagagaatgagcactgcggaatacaggcatatgcctgtaatacagagagtcaggaagacctgtacgctgaagtgcccttagtcggtagactaacgggcattgaagaagtgaaagtcgaagctattgcgatgagcaaacttcataatatgagttgtccgccttatatggggcatagtgcggctgttattttccatttaatttacctttcctgatgtgaatgaaggtgaagatattctatccaggaaatacggttgaactgtgaaggtgatcaataaaaaatgatcaatcttaatttatttaatgatgagctttttactcagtaatataaaatattgaattgttatttttgtgtgttgtttaagataaaaagccgtatttattattacggctttaattaataaaaggcaggctgtattaaaattaatattcaaagcataaaccgatagccaataccggtttcagtaatgaaatggcgtgggcgggcgggatcctgttccagtttttgtcgcagatgtcccatataaatacgcaaatagtgactgtgttcgaccgcgtttggcccccacacctggttaaggagctggcgctgggtgagtacttttccggcattgttgagcagcaccgccagcaggcggaactcaattggtgtgagatgcacctcttcctcaccccggtgaatcacgcgggcggctaaatcgacggtaacatcggaaaattttaccagcggatcgggcgcggtggtggcagagtggcggcgtaatgcgacgcgcagacgggcctgcaattcgccaatgccaaacggcttactcagataatcatccgctccggcatccagcgcggcgattttgtcgctctcttcgctgcgtgcggaaagcacaatcaccggcaccgcgctccactggcgcaggtcgcggataaactcaatcccatcaccatcgggcaggccgagatcgagaataatcaaatctggcttacgggttgccgcttccagcaagccgcgttgcagcgtttcggcctcaaagacgcgcatcccgtcgccctccagcgccgtgcgcagaaagcgacgaatagcctgttcatcttcaacaatcagaacgtttgtcacatatcctcatgaaattcttcaagttcaggggcagtttgctggggaagtgtaacacgaaaacaggcaccaccttccggtcggttgaacgcggtaatagtgcccccgtgtacatccactatcgcccgacaaattgccagtccaagccctacccccggtactgccgactctttattcccgcgagcaaacttatcaaatatcgtctgctcctggcctggcggaagaccggggccgttatcccagacatccagttgtagattttcgccctcaacgtgggcatcgataccaatttcggcctgcgcacccgcatatttcaccgcgttctccagcagattaatcagcacccgttcaaagagtggcccgtcaacgtggattaaggtcagcggttctggcagagaaagattgatgggcgacgataaacccggttccagcatttgcagcgcgctgccgactacttcttccagcgttaaccactctttcttcaaattaaagccgccggactgaattcgcgccatatccagtagattattcaccagtcgggtagtgttcagcacatgctgacggatctcgctggcctggcgggcgtggggtgatccttcgcttgccagatcgagcgttaagatttctgcctgaccaaacagcaccgtaagcggcgtgcgtaaatcatgcgaaagcgccgccagcagggcgttgcggatctgttcacgttcgcttgccatccgcgcctgttcttcgctggcggttagcgtcagccgctcaagggcattggcgactaacagcgtaaacgtctccagcaggcgctgctgttccgggatcatcaactggcgcagattccccggctccaccaccaccagcccgtaggttttctcgccgctttttagcggcaaaatctggtacggtacaccgggtaacgtgtcggtgcccgcgcccgcaggcaggcctttatcaaaactccactgcgcgatggcatcgtcccacggcgtcattccttgcggatgtgttaacggctgcaatttaccgttgtcatcgggcaacaacacctgactgcgggcatgaaacgtggaggcaataaattgttcgctggtggcagcgatatcctgcggactgcggcccaccgccagagctttcgacatttcatataagtgccgtgtgcgttgctcgcggtaacgggctacccgcgcctgataacgcacgccagcagtaaggttcccgatcaccagcccgacggttaacatcaccgcgaaggtcagcagatattgcacatcagagacggcgagcgtgccgcgtggggcgataaaaaagagatcgaaactcactacattaatgacggtggcaaccactgaaggccagcgtccataaaatagcgccaccaccaccacgccaagcagatacagcatcaccaggttggcggcatcaaacgccatcagccactgcatggcaattaaggtgataacggcgcataacgcggcggcaaccacgcatccctgaatttgtacacgccacttgtctttaaaagagcggttatccggcgcgttgttaatcgtgcgggcgggtggttcatcaagcgcgaccagcacctgatcgagatcgggggcgatgcgcgccagtcggtcagcaaacgtttcccgacgccaccagcggcgcgaggccgggcgaccgagaataatcttgccgagattatgttcacgggcataacgcactaccgctttctcttccgctggatcagaaagtgttgccgtctccgcgcccagttcctgcgccagacgtaaggcgctgagaattgcccgacgttttttttccggtaagcggtgcagggcaggggtttcaacatacaccgcgtgccagacgctacccagccgtgacgccagccgcgccgctgcgcggaccagtttttcgctgccggtgttatggccgatgcataaaaggatcgcgtcgcgcgtgtgccacactttctcttcgccaggatgcccccgccaggcgcgcatttgctcatcaacgcgatcggcagtacggcgcagtgccagttcgcgcagggcgatcagattacctttgcggaaaaaatgttcaatggcgcgctccgcctgcccggcaatatagactttgccttctttcagccgctggcgcagatcgtccgggggcaagtccaccagcaccacgtcgtcggcggcatcgaaaaaaggatcgggcacggtttcccgtacctgaattccggtgacgccgctgaccacatcattcagactttccagatgctgaacgttgacggtagtgaaaacatcaatgccagcttccagcagttcttcgatatcctgccagcgtttgggatgacgggaacctggcgcattactgtgcgccagttcgtccattaagatcagcgccgggcggcgggcgagggcggcatcgagatcaaactcgctgatatgccgcccacggtacgcctggcgttttaacggcagaacagccagcccttccagcatggcggcggtatcttttcgcccgtgggtttctaccacgccaaccacaatatccagcccttgcgcccgcagtcgctgggcttctgccagcatcgcccaggtcttcccgacgcctgcacaggcaccgaagaaaactttcagcttcccccgatgcggcgcggcagtttgttccagcagacgatcggggtcgggacgtaagggttcgttattcatcaagtttatccagcgccagattgagttcaacaatgttgacaaccggctggccgatatatttcaccagcggttgttggctgtattttgcgatcagttgcgtgagctgttcaacgctgagattacgcgctttcgccacgcgtgggatttgccaggccgccgcttgcggggtgatattattgtccagcccgcttgccgatgccgtcaccagttcaaccggaacgctcgcgctggcatccgggttagcggcccgtaatgcagcaacgcgtgcggctattagtttatccagctcagggttactgaccgccagattgctcccgccagaagcctgtggattatagggcatttctgccgttgccgacgggcgaccatgaaaatagccgttgccggtaaaattctgcccgattaatgccgaaccgcgcaccgtatcaccttcacgaatcaacgaaccattggcctgccagggaaaccaccattgccccagtacggtggtcagcagcgggtaaacgccgccagtaatcaataacagaaagataaatgttgataatgccggacgtaatccactcatggtaaacctcacaccagaccgcaaacggtcagcagtaaatcaatgactttgataccgataaacggcaccagcagcccacccagaccgtaaatccataagttacggcgcaacatggcagaagcggtaagcggtttataactcacgccttttaacgccaggggaatcaaaaagacgataatcaaggcgttgaaaatcaccgcactgaggattgcggagtcgggcgaatgcaggcacatgatgttcagcgcatttaactgcggatacgttgccgcgaatgccgccggaataatggcgaagtatttcgccacatcgttggcaatgctgaaggtggtcagcgagccacgggtcatcagcatctgtttgccaatgtgcaccacctcgatcaacttggtcgggttagagtcgagatcgaccatattgcccgcctctttcgccgcctgggtgccggagttcatcgccaccgcgacatctgcctgcgccagcgccggagcatcgttggtgccgtcgccggtcatcgctaccaaacgaccttccgcctgatactgacggatcaatgccagcttggcctccggtgtcgcttcggcgagaaaatcatcgacacccgcttccgcagcaatcgcggcggcagtcagacggttatcgccggtaatcatcaccgttttaatgcccattttgcgcagctgggcgaagcgctctttaataccgcctttgacgatatctttcagcgcaataacgcccagcacacgagaaccttccaccaccaccagcggcgtggctccctgacgcgcaacctgatcgactttttgatcaacatcggtagggaagtgaccaccgttagcctcaacatggcgacgaatggcatcgacagaacctttacggatcatgcggttgtcgatgttgatcccgctcatccggctttgcgcagtaaacggtacaaaggtggcatggagcgactgcacatcgcgctcgcgcaggttaaaacgctgcttggcgaggatcacaatactgcggccttccggcgtttcatcagccagcgaagccagttgtgcggcgtcagccagcgttttttcatccacgccctgcgcggggataaactccgacgcctgacggttaccgagtgtgatggtgccggttttatccagtagcagaacgtcaacgtcacctgccgcttcaactgcacgtccgctggtggcaatcacattcgcgcctagcatccggctcatcccggcgacgccgatcgctgacaacaggccgccaatagtggttgggatcagacagaccagcagcgccaccagtaccgttacgctgactgcattaccgccccacgcggaaaacggccacagcgtggcggttgccagtaaaaagacgatagtcagggcaatcagcagaatggtcagggcaatttcgttcggcgttttgcgtcgctgtgcgccttccaccatcgcgatcatccgatccagaaatgtctcgccggggttaacgctacactcaatcaccagccagtcagaaagaatacgcgtgccgccggtgacggaggcaaaatcgccgccggattcacggatcaccggtgccgattccccggtgatggcgctttcatcgaccgatgcacccccttcaataacttcaccatcgcaggggataatatcgccagcttctaccagtacgatatcgcctttacgaagttggtcggcaggaactttgtccgccgcagcgccatatttcggctcacgcagcttgcgggcaaaggcagtttttttcacccctttcagactgttggcctgcgctttactgcggccttctgccagcgcctcggcgaaattagcgaacagtacggtgatccacagccaaccgctaatggccgcgctaaacagcgcattgccgggcatcgcaccgcttgccatcgcgatgctaatacaggtggtcagcagactgccgatccagacgataaacatcaccggattgcgccattgcgcctgcgggtttaattttttcaccgcttctttcagcgcctgaacgacaagtgttggttcgaatagcgccagttgtttacgactcatattcagtgctcactcaatatcatcaggagagatattccgccaccggaccaagcgccagggcagggataaaggtcagtgcgccaaccagcaacacggtgccgattaacaggccaacaaacagcgggccgtgcgttggcagcgtgccggagctggcggcttggctctttttactcaccagcgaaccggcaattgccatcaccgggataatcaccccgaagcgaccgacaaacatgcagaacgccagtaaacagttccagaacggagagttggcgcttaatccggcaaaggcgctgccgttgttgttagcggcggatgacacggcgtacagcacttcgctaaaaccatgcgggccagggttgagcatggcgctacgtccggcgtcggtcatcatcgccaacgccgcgcccatcagcaccagcgtcggggtaaccagaattgccagtgcagtcagtttcatctcgcgtacgtcgatttttttacccagatattccggtgtacgaccaatcatcagcccggcaataaacaccgccagcaggacaaacagcatcatgccgtaaagaccagaaccgacaccgccgaacaccacttcaccaatttgcatcagccacatcggcaccatgccaccgagagcggtaaacgaatcatgcatcgcaatcaccgcgccacaggaagccgccgtcgtcacgaccgcaaacaggctactgaccagcacgccgaaacggctctctttaccttccatattgatgctgctgtccgtgcccagtgccagcagatgaggattaccctgaacttctgcccacatcaccacgcctacgcagatgacaaaaatcactgacatcgcccacagcaacatgcgcccctggcggcgatcgcccatcacttcaccaaaggcaaagcacagcgccgttgggatcaagaagatcgccagcatctgcacgaagttggtcagtgcggttgggttttcaaacggatgcgacgagttggcattaaagaagccaccgccgttagtaccgagcatcttgatcgcttcctgagaagctacaggccccatgggtaacagctgttgcgctccttcaacggtattcacagcctgataaggcagaaagttttgcagcgcaccttgttgaataaaaaacagtgcaatcaacaacgccacagggactagcacccataacgtgatgcgtagcagatcgacccaggcattcccgagcgtgctcatgctctggcgggtaaacgcacggatgagggcaaaaatcaccgcaatcccgctggcggcagaaagaaagttttgcaccgttaagcccgccatctggctgaaatagctcaacgtggtttcaccgctataagattgccagttggtattggtgacaaagctgacggcggtattcagcgccagatcccacgacagccctggcaactgctgtggattaagcggcagatagtgctgaccgagcaacataaaaaacagcaccgccagccccagcatgttcaggccgagaatggcacaaagatattgcttccagttcatctcacggtcagagacgccaagtgcgcgaaaaagtacgcgctcaacgcccgttgtaccgggaagaggaatgtcattaatcagccgcgccagcccgctgcctaaaggacgcgccagcaccattaacaccagtaaaaacgtggcgatcagtaagaacccttgcgcagccatcagaacgcctccgcattgatcagggcataaaccagataacccagtaataaaaacaccagcaatacgccggttatcacgcctgcactcacagtgcacctccagtggcctaaaagtgataccggaagggtagaattctggctgcaaagatttcgcaaaaatctgcgggcggggtgtaaaaaaagtataaaaatggcaaaagccatgatttaactaatgtttagtattaatttaacttttgtgtaacttaattacaggatgaatgtaaataaaccatcaataagcaaaaataagtggtcggatgagtagtaaaattacacaaaaggcggtactattttcatcagataaacaaattcatttttccggtgccattcaccgggtagatacaaaagggggagaaaagtatggaactctacagagaatatcctgcatggcttatctttttacgccgtacttatgcggttgcagcgggcgttctggcgctgcctttcatgcttttctggaaagaccgcgcccgcttttacagctacctgcatcgcgtctggtcgaaaaccagcgataaaccggtgtggatggatcaggccgaaaaggcaactggtgatttttattgattgctgagttttgaatacattgaaaaccgccagcggaaacgctggcggttttttgtatcaggaagatgttcagaggaatatttagacatcgttataccaatcgaaacatatattcatgaaatatatataaatattttcctaattgttcttatctgacagatatctcacttaaggctttcttataaatctgtagggtttcgcctgtcagcagacaaataacccgataaaacaaggatgagcagatgagcggaaaaccggcggcgcgtcagggcgacatgacgcagtatggcggtagcattgtccagggttcagccggggtacgcatcggtgcccccaccggcgtggcctgttcggtgtgccccggcggggtgacgtccggccatccggtcaatccgctgctcggtgcaaaggtccttcccggtgaaaccgacatcgccctgcccggcccgctgccgttcattctctcccgcacctacagcagttaccggacaaaaacgcccgcgccggtggggagcctcggccccggctggaaaatgcctgcggatatccgcttacagctgcgcgataacacactgatactcagtgataacggcggcagaagcctgtattttgagcacctgtttcccggtgaggacggttacagccgcagcgagtcactgtggctggtgcgcggcggcgtggcgaaactggatgaaggtcaccggctggccgcactctggcaggcgctgccggaagaactccgcttaagtccgcatcgttatctggcgacaaacagtccgcaggggccgtggtggctgctcggctggtgtgagcgggtgccggaagcggatgaggtgctgcctgcgccgctgccgccgtaccgggtactgaccgggctggtggaccgcttcgggcgcacacagacgttccaccgcgaagccgccggtgaattcagcggcgaaatcaccggcgtgacggatggtgccgggcgtcacttccggctggtactgaccacgcaggcgcagcgggcagaagaagcccggcagcaggccatttccggcgggacggaaccgtccgcttttcctgataccctgccgggttacaccgaatatggccgggacaacggcatccgtctgtctgccgtgtggctgacgcacgacccggaatacccggagaatttacctgccgcgccgctggtgcgctatggctggacgccccgcggcgaactggcggcggtgtatgaccgcagcaatacacaggtgcgcagctttacttacgatgataaataccggggccggatggtggcgcaccgtcacacgggccgaccggaaatctgttaccgttacgacagcgacgggcgggtgacagaacagctaaacccggcaggcttaagttacacgtatcagtatgagaaggaccgcatcaccatcaccgacagcctgaaccgccgtgaagtcctgcacacgcagggtgaaggcgggctgaagcgggtggtgaaaaaggaacacgcggacggcagcgtcacgcagagtcagtttgacgcggtgggcaggctcagggcacagacggatgccgcaggcaggacaacagaatacagtccggatgtggtgacgggcctcatcacgcgcatcaccacgccggatggcagggcatcggcgttttactataaccaccacagccagttaacgtcagccaccgggcctgacgggctggaaatacgccgggaatatgatgaatggggccgtctgattcaggaaactgcccctgacggcgatatcacccgctaccgttatgataatccacacagtgacttaccctgcgcaacggaagatgccaccggcagccggaaaaccatgacgtggagccgttacggtcagttgctgagcttcactgactgttccggttatgtaacccgctatgaccatgaccgttttggtcaggtgacggcggtgcaccgcgaggaagggctgagtcagtaccgcgcatacgacagccgtggacagttaattgccgtgaaagacacgcagggccatgaaacgcggtatgaatacaacgccgccggtgacctgaccaccgtcattgccccggacggcagcagaaacgggacacagtacgatgcgtggggaaaagccatctgtaccacgcagggcggtctgacgcgcagtatggaatacgatgctgccggacgggtcatccgcctgaccagtgaaaacggcagccacaccaccttccgttacgatgtactcgaccggctgatacaggaaaccggctttgacggccgcacacagcgttatcaccacgacctgaccggcaaacttatccgcagcgaggatgaggggctggtcacccactggcactatgacgaagcagaccgcctcacgcaccgcaccgtgaatggcgaaaccgcagagcggtggcagtatgacgaacgcggctggctgacagacatcagccatatcagcgaagggcaccgggtgacggtgcactatggttatgacagtaaaggccgcctcgccagtgaacacctgacggtgcatcatccgcagacgaatgaactgctctggcagcatgagaccagacatgcgtacaacgcacagggactggcgaaccgctgtataccggacagcctgcccgccgtggaatggctgacctacggcagcggctggctgtcaggcatgaaactcggcgacacaccgctggtggagtacacccgcgaccgcctgcaccgggaaacgctgcgcagcttcggccgttatgaactcaccaccgcttatacccctgccgggcagttacagagccagcacctgaacagcctgctgtctgaccgcgattacacctggaacgacaacggcgaactcatccgcatcagcagcccgcgccagacccggagttacagctacagcaccaccggcaggctgaccggcgttcacaccaccgcagcgaatctggatatccgcatcccgtataccacagacccggcaggtaaccgcctgcccgacccggagctgcacccggacagcgccctcagcatgtggccggataaccgtatcgcccgtgacgcgcactatctttaccggtatgaccgtcacggcaggctgacagagaaaaccgacctcatcccggaaggggttatccgcacggatgatgagcgcacccaccggtaccattacgacagtcagcaccggctggtgcactacacgcggacacaatatgcagagccgctggtcgaaagtcgctatctttacgacccgctgggccgcagggtggcaaaacgggtatggcggcgtgaacgggacctgacgggctggatgtcgctgtcacggaaaccgcaagtgacctggtacggctgggacggcgaccgcctgaccacgatacagaacgacagaacccgcatccagacgatttatcagccggggagcttcacgccactcatcagggttgaaaccgccaccggtgagctggcgaaaacgcagcgccgcagcctggcggatacccttcagcagtccggtggcgaagacggtggcagtgtggtgttcccgccggtgctggtgcagatgctcgaccggctggaaagtgaaatcctggctgaccgggtgagtgaggaaagccgccgctggctggcatcgtgcggcctgacggtggcgcagatgcaaagccagatggacccggtatacacgccggcgcgaaaaattcacctgtaccactgcgaccatcgcggcctgccgctggcccttatcagcacggaagggacaacagcgtggtacgcagaatacgatgaatggggtaacctgctgaatgaagagaacccgcatcagctgcagcagcttatccgcctgccggggcagcagtatgatgaggagtccggcctgtattacaaccgccaccgctattatgacccgctgcaggggcgatatatcactcaggatccgattgggctgaaagggggatggaatttttatcagtatccgttgaatccgatctcaaatatagatccattaggattagaaacactaaaatgcattaagccactgcattcaatgggcggaactggtgaaagaagcggtccagatatatgggggaatccgttctatcatcaatatctttgtgtcccagatggtaaaggggactatacttgtggtggccaagaccaacggggagaatcaaaaggagatggtctatgggggccaggtaaagcaagtaatgatacaaaagaagctgctggccgttgtgacctcgttgaaaccgataatagttgtgtggagaactgtttaaaagggaagtttaaagaggtaaggccgcgttattctgtattgcctgatatattcacacctataaatttagggctatttaaaaactgccaagactggtctaatgattctttagaaacatgtaagatgaagtgctccggaaataacattggacgttttattagatttgtattcaccggagtgatgtaatgaaatatattatttttttattcagagctatatggctggctttatcgcttttaatactattcttttccatgcatagactttcactattagactccactcgtgatgtgagcgagttaattagtctcatgtcttatggaatgatggtaatatgttttccaacaggcatagtattctttattgctctaatatttatagggactgtatcagacattattggcgtaaggattgatagtaagtatattatggcgataataatatggctttattttctgtcaggagggtatattcaatggtttgtattaagtaagcgcattataaacaaataaattaagttaattgctcttattattatatgtaacctgggcattgatatcccgtatgccacagacccggcaggtaaccgcctgcccgacccggagctgcacccggacagcaccctcagcatgtggccggataaccgtatcgcccgtgacgcgcactatctttaccggtatgaccgtcacggcaggctgacggagaaaaccgacctcatcccggaaggggttatccgcacggatgatgagcgcacccaccggtaccattacgacagtcagcaccggctggtgcactacacgcggacacaatatgcagagccgctggtcgaaagccgctatctttacgacccgctgggccgcagggtggcaaaacgggtgtggcgacgtgaacgggacctgacgggctggatgtcgctgtcacggaaaccgcaagtgacctggtacggctgggacggcgaccgcctgaccacgatacagaacgacagaacccgcatccagacgatttatcagccggggagcttcacgccactcatcagggttgaaaccgccaccggtgagctggcgaaaacgcagcgccgcagcctggcggatacccttcagcagtccggcggcgaagacggtggcagtgtggtgttcccgccggtgctggtgcagatgctcgaccggctggaaagtgaaatcctggctgaccgggtgagtgaggaaagccgccgctggctggcatcgtgcggcctgacggtggagcagatgcaaaaccagatggacccggtgtacacgccggcgcgaaaaatccacctgtaccactgcgaccatcgcggcctgccgctggcgcttgtcagcacggaaggggcaacagaatggtgcgcagaatacgatgaatggggcaacctgctgaatgaagagaacccgcatcagctgcagcagcttatccgcctgccggggcagcagtatgatgaggagtccggcctgtattacaaccgccaccgctattatgacccgctgcaggggaggtatatcactcaggatccgattgggctgaaggggggatggaatttttatcagtatccgctgaatccggttcagtatatagattcaatgggactggcatcaaaatatggacacttaaataatggcggatatggagcgagacccaacaaaccgcctacgcccgatccaagtaaattgccggacatagcgaaacaattaagactgccatatcctattgaccaggccagtagtgcgcctaatgttttcaaaacattcttcagagcattaagcccttacgactacacactgtattgcaggaagtgggtaaaaccaaatctgacttgtacgccacaggatgattcccagtatccagggatggatacaaagacagcaagtgattacctgccacagacaaattggccaacaactcaattaccaccaggatatacttgtgcagaaccctatttattcccagacattaataaacccgatgggccagcaacagcagggatagatgatttgggtgaaattttagctaagatgaaacagagaacatcgagaggaataagaaaatgaaaagagttttgttctttttgctgatgatatttgttagttttggtgttatagctgattgcgaaatacaagctaaagatcatgattgttttactattttcgctaagggtactattttttccgcgtttcctgtcttaaataataaagccatgtggagatggtatcagaatgaggacatcggtgagtattattggcaaacagaactgggtacatgtaaaaataataaattcacaccaagcggggcgagactcttaattcgcgtcgggtcactacgccttaatgaaaatcatgccatcaaaggaacgttgcaggagttgataaatacagcagaaaaaacggcgtttctcggcgatcggtttagaagttatataagagcgggtatctatcaaaaaaagagcagtgatccagttcagttgttggcagtccttgataattcaatcatggtaaaatattttaaagatgagaaaccaacttatgctcgaatgacagcacatctcccgaacaaaaatgagtcttacgaatgtttaataaagatacagcatgaactaattcgtagtgaagagaaataaaatctcttcctgagaaaacaaattaatcattgtgaaaaattatataactcatggaataggtgtttattttgcgttccatttgcagggaaagatcacgtaacgctacttttttgtactaaataattcgaattttaagttcaacaattgagatactacttattgtctaaagctgtttttcatagcttatacatgatcaaatactccttacataaataaggtgaacaaatggaacttaaaaaattgatggaacatatttctattacacccgattacagacaagcctggaaagtggtgcataaattgtcagatattctactgttgactatttgtgccgttatttctggtgcagaaggttgggaagatatagaggatttcggggaaacacatctcgattttttgaagcaatatggtgattttgaaaatggtattcctgttcacgataccattgccagagttgtatcccagggaaagatcacgtaacgctacttttttgtactaaataattcgcattttatgtttaaaaattgagatattccttattacctaaagctgtttttcatagcttatacatgatcaaatactccttacataaataaggtgaacaaatggaacttaaaaaattgatggaacatatttctattattcccgattacagataagcctggaaagtagagcataaattgtcaggcatcctactattgactatttttgccgttatttctggtgcagaaagttgggaagatatagaggatttcggggaaacacatctcgatttcttgaagcaatatggtgattttgaaaatggtattcctgttcacgatactattgccagagttgtatcctgtatcagtcctgcaaaatttcacgagtgctttattaactggatgcgtgattgccattcatcaaatgataaagacgtcattgcaattgatggaaaaacgctccggcactcttatgacaagagtcgccgcaggggagcgattcatgtcattagtgcgttctcaacaatgcacagtctggtcatcgggcagatcaagacggataagaaatccaatgagatcacagctatccctgaacttcttaacatgctggatattaaaggaaaaatcatcacaactgatgcgatgggttgccagaaagatattgcagagaagatacaaaaacagggaggtgattatttattcgctgtaaaaggaaaccaggggcggcttaataaagcctttgaggaaaaatttccgctgaaagaattaaataatccagagcatgacagttacgcaatgagtgaaaagagtcacggcagagaagaaatccgtcttcatattgtttgcgatgtccctgatgaacttattgatttcacgtttgaatggaaaggactgaagaaattatgcgtggcagtctcctttcggtcaataatagcagaacaaaagaaagagccagaaatgacggtcagatattatatcagttctgctgatttaaccgcagaaaagttcgccacagcaatccgaaaccactggcacgtggagaataagctgcactggcgtctggacgtggtaatgaatgaagacgactgcaaaataagaagaggaaacgccgcagaattattttcagggatacggcacatcgctattaatattttaacgaatgataaggtattcaaggcagggttaagacgtaagatgcgaaaagcagccatggatagaaactatctcgcgtcagtccttgcggggagcgggctttcgtaatctttccctgctttttgtactaaataattcgcattttatgtttaaaaattgagatattccttattacctgaagctgttttttattgcttatacatgatcaaatacttcttacataattaaggagaacaaaatggaacttaaaaaattgatggaacatatttctattatccccgattacagacaagcctggaaagtggaacataaattatcggatattctactgttgactatttgtgccgttatttctggtgcagaaggctgggaagatatagaggattttggggaaacacatcccgattttttgaagcaatatggtgattttgaaaatggtattcctgttcacgataccattgccagagttgtatcctgtatctgtcctgcgaaatttcatgagagctttattaactggatgcttgactaccattcttcagatgataaagacgtcatcgcaattgatggaaaaatacaccggcattcttatgacaagagtcgccgtaagggagcgattcatgtcattagtgcgttctcaacaatgcacagtctggtcatcggacagatcaagacggataagaaatccaatgagatcacagctatccctgaacttcttaacatgctggatattaaaggaaaaatcatcaaaaccgatgcgatgggttgccagaaagatattgcagagaagatacaaaaacagggaggtgattatttattcgctgtaaaaggaaaccaggggcggctaaataaagccttcgaggaaaaatttccgctgaaagaattaaataatcccaagcatgacagttacgcaattagtgaaaagagtcacggcagagaagaaacccgtcttcatattgtttgcgatgtccctgatgagcttattgatttcacgtttgaatagaaagggcagctatggttagaaactacctgacgtcagtccttgcggggagcaggctttcgtaaatttgtcctgctacaacaggattaacttcacaaatatcatttctcaacgtctacacttactcctgtaaaccgctcaggagcagtaatgaatctacaacgatttgatgacagcaccctaatccgtatctttgcccttcatgagttacatcgactgaaagaacatggcttaacgcgcggggcgcttctcgattatcacagccgctataaactcgtctttctggcgcattctcagccggagtaccgcaaacttggcccgttcgtggctgatattcaccagtggcaaaatctggatgactattacaaccagtaccgccaacgcgtagttgttttgctttctcaccccgccaacccgcgcgatcacaccaatgttttgatgcacgttcagggttattttcgcccgcatattgattccacagaacgccagcagctggctgcgcttatcgacagttatcgccgtggcgagcaaccacttcttgcgccgctgatgcgtatcaaacactatatggcgctttatcctgacgcctggctttcagggcagcgttatttcgaactttggccgcgtgtgattaacttgcgccattcaggagttttatgactacccatctggtctggtttcgccaggatttacgtctgcacgataatctcgcactggctgccgcctgccgcaattcgtctgcacgcgtgctggcgttgtatatcgctacaccacgccagtgggcgacgcataacatgtcgccgcgtcaggctgaacttatcaatgctcaactgaatgggctacaaatagcgcttgcggaaaaaggtattcctttattgttccgtgaagtggatgactttgtcgccagtgtcgaaatagttaaacaggtgtgcgcggaaaacagcgttacccacctgttttataactatcagtatgaagtgaatgagcgggcgcgggatgtggaagttgaaagagcgctgcgtaacgtggtgtgtgaaggatttgatgacagcgtgatcctgccgcctggcgcggtgatgaccggtaatcacgagatgtacaaagtctttacgccttttaagaatgcctggctgaaacggctgcgggaagggatgccggagtgcgtcgctgcgccaaaagttcgtagtagcggatcgatagagccctcgccatccattacgctgaattatcctcgtcagtctttcgatactgcgcattttccggtggaagaaaaagcggcgattgcgcaattacgccagttttgccagaacggtgccggagaatatgagcaacaacgagattttccggcagtggaaggcaccagccgtttgtcggccagcctggcaacgggcgggttatcgcctcgccagtgcttgcatcgcttgttggctgaacagccgcaggcgctggacggtggggccggtagtgtctggcttaatgagctgatctggcgcgagttttaccgtcacctgataacgtatcacccctcgttgtgtaaacatcgtccatttattgcctggacggatcgtgtacagtggcagagcaatcccgcacatttacaggcctggcaggaaggcaaaacgggatacccgattgttgatgccgctatgcgtcagcttaacagcactggctggatgcataacaggctacggatgattacagccagttttctggtgaaagatttattgatcgactggcgcgaaggcgagcgatatttcatgtcgcagctgattgatggtgatttggcagccaataacggtggctggcagtgggccgcttcaaccggaaccgatgcagcgccgtattttcgtattttcaacccgacaacccagggcgagaaatttgatcatgagggcgagtttatccgccagtggctaccggaactgcgcgatgtgccagggaaagtggtgcatgagccgtggaagtgggcgcagaaagcaggtgtgacgctggattatccgcaaccgatagtcgagcacaaagaagcgagagtacaaacgttggcagcgtatgaggcggcgcggaaggggaaataacagacgcgtcaggcaatcgagcccagatgccggatgcggcgtgaacgccttatccagcctacaaatttgtgcaaattcaataaattgcaggaaatacgtaggcctgataagacgcgtcaagcgtcgcatcaggcatcggtgctggcctattaagactccagcgccagcgcgcggtttctgaatttcagcgcctgatacagccaaatcatcagtaccagtcctacacacgccagtgcgccccaggtaatttgatcaaatacttcaatatatgcattgatggagtagttgatcgccccggaagcatcaaacgaagcctgcgatgtctgatcggcaatcacgcccgccagatagttcgcgatcgcgccagaaagcagcatgtagatgccggttaatacgccggtcacaccggggatttcaatgcgcgtaatttgcgacatggcaaccgggtcgataaacagttccgcaaagcccatcaccgccaggcctaataccatcagtggcagagaagagtgaccatacattgcggaccagcgggcgcttaaggtcagaatgcagaatccggcgctcatcaggccaaggccaagagcaaatttcccccagatgcgcacggtacgattacccgcgacactctcttttaccacccacgccaggaacacaccgcacagcataactgcgaaggcattaatcgactggaacatcgcggtcggaacggtataaccaaacatatcgcggttaacgaagcggtcgatataaaggctaatcgagctaccgccctgttgtgcgaaggcccagaacaacatactgaagaaggtgagcgtcacaatcagccccagctccttccgctgtttctggttttctgctttgcgataaatttttgccagtacacccaggccaataatagtcgcgacaattaaggcgtataccgaccactctttccagaacagtatggtaatcagtgcaggcgttgccaccagcagaaccagcagccatccccagttcggcaggagaaagtttgtcgcacgcagtacttttttgttaacgccgcgggtatgagtgaaatgacgattgccacataagaaaatgaccagacccgcgatcatgccaaccgccgccaggccaaagcccatcgcccagctgtactcttcctgggcgtaaccacaggcgataggtgcgataatagaccccacgttacccgccgcatacatcagcgagaaaccgccatcacgacgcggatcggttggctcatacagctcgccgagcagacagcttacgttagatttaaacaggccatagccgcagacgataatcgccagggacagatagaggaatgacggatggatctcactggcacccagcaccacatgaccgatcgccatcaacaacgcccccagcatcaccgccatgcgattgccgagaactttatccgccaaaaagccaccgaggattggcgtgacatacaccagcgaacagtaggcgctaaataactcgtaggcgtgagtatcgttgtattttagttgattggtgagatagagaatcagcagggcacgcatgccgtaaaagctaaaatattcccagatttgcagcgcaacgacatagtaaatagcgcgcggctgtgatgcgtgtttattcataataattccacaattgacggcaacgtcacgtaatagttgcgcggcgtgcttgtgtttccttaaagttaaaactttgatacagatctgattatttatgcaatatgctgtctgattgcataaatatacattagctgaagcgtgatgatataaacaatttgcgtcttttggcgtcgggtttgtttcttaatatgtcaaaagattggctatcgacgaactggcgaggtaacgctatgttaacggtgtagctatcagaatacggaaggcgcgaagatgaaaaacaccgaactggaacaactgattaacgaaaaactgaacagcgcggcgattagtgattacgcgccgaatggtttgcaggtggaaggcaaagagacggtgcaaaaaattgttaccggtgtcaccgccagccaggctttgctcgatgaggcagtgcgtctgggcgcggatgcggtcattgtgcatcatggctacttctggaaaggagagtctccggtcattcgcggaatgaagcgtaaccgtttaaaaacgttgctggcgaatgatatcaacctgtatggctggcatttgccgcttgacgcacatcctgagctgggcaataacgcacagctggcggcgttactggggatcacggtcatgggcgaaattgagccgttggtgccgtggggcgaactgaccatgcctgtgccgggactggagctggcttcctggattgaagcgcgtctgggacgtaagccgttatggtgtggcgataccggacctgaggtggtccagcgcgtcgcctggtgcacgggcggcgggcaaagttttatcgatagcgccgcgcgttttggcgtggatgcttttattactggcgaagtttctgaacagaccattcattcagcccgcgagcagggattgcatttttatgctgcaggtcaccatgccactgaacgtggtggtattcgcgcattgagcgagtggctgaatgaaaataccgatcttgatgtgacctttattgatattcctaatcctgcataacgaataatcagagggatcgaaagtgcaacgagcgcgttgttatctgataggtgaaacggcggtagtgctggaactggaaccgccggtgacgctggctagccagaaacggatctggcgactggcgcagcgtctggtggatatgccgaatgtggttgaagccattcccggcatgaacaatatcacggtgattttgcgtaatcctgagtcgctggcgctggatgccatagagcgtttgcaacgctggtgggaggagagcgaggcgctggagccggagtctcgctttattgaaattccggtggtttacggtggtgcaggcggaccggatttggcggtggtcgcggcgcattgcgggttgagcgaaaaacaggttgttgaattgcactcctccgtggaatacgtggtctggtttttaggttttcaaccgggcttcccgtatctcgggagtttgccggaacaactacacacgccacggcgcgctgaaccgcgcttactcgttccggcaggttctgtcgggatcggcgggccgcagactggtgtttatccgctggcaacgccgggtggctggcagttgattggtcatacctcactcagcctgtttgatccggcgcgtgacgaacccatcttattacgtccgggagacagcgtgcgctttgtaccgcagaaggagggagtatgctgaagattattcgtgcgggcatgtataccactgtgcaggatggcggtcgtcacggttttcgccagtcgggtatcagccactgcggcgcactggatatgcccgcgttacgcattgctaacctactggtgggtaatgacgccaatgcccccgcgctggagatcacgctcggtcagttaactgttgagttcgaaactgatgggtggtttgctctgacgggtgccggttgcgaagcgcggctggatgataatgccgtctggaccggctggcgattgccgatgaaagcaggccagcgtttaacgcttaaacgcccgcagcacgggatgcgcagttatctggcggtcgcgggtggtattgatgttccgccggtaatgggctcatgcagcaccgatctcaaagtggggattggcgggctggaaggccgtttactgaaggatggtgaccgactcccgattggcaaatcgaagcgtgattctatggaagcgcagggcgttaaacagctgctgtggggcaaccgcattcgcgccttgccggggccggaatatcatgagttcgatcgcgcctcgcaggatgcattctggcgttcgccctggcagcttagctcgcaaagtaaccgcatgggctatcgcttacaggggcaaattttaaaacgcaccaccgatcgcgaactgttatctcacggtttgttaccgggcgtggtgcaggtgccacataacgggcagccgattgtgttgatgaacgacgcacagaccaccggtggttacccgcgtattgcctgtatcattgaggctgatatgtaccatctggcgcaaattccgctcggtcagccgattcattttgtccagtgttcactggaagaggcactaaaagcacggcaagatcagcaacgttattttgaacaattagcgtggcggctgcacaatgaaaattgacctgaacgccgatctgggcgaaggctgcgccagcgacgcagagctattaacgctggtttcctctgccaatattgcctgtggatttcatgcaggcgatgcgcaaatcatgcaggcttgcgtgcgtgaagcaataaaaaatggtgtcgcgattggcgctcacccgagttttcccgacagggaaaattttggtcgcagcgccatgcagctgccgccagaaaccgtttacgcccagacgctgtatcaaattggcgcgctggcaacgattgcccgtgcgcaaggcggcgtaatgcgtcatgtcaaaccgcacggcatgttgtacaaccaggcggcgaaagaagcacaactggcagacgccatcgccagagcggtatacgcttgcgatccagcattgattctcgtcgggctggcgggaagcgagctgattcgtgcaggcaagcaatatggtctgacaacgcgcgaggaagtgtttgccgatcgcggttatcaggctgacggctcgctggtgccgcgaagccagtcaggcgcgttgattgaaaacgaagaacaggcgctggcgcaaacgctggagatggtgcaacacggcagagtcaaaagtatcaccggcgaatgggcaacggtcgcggcgcaaacggtctgcctgcatggcgacggcgagcacgcactggcgttcgcccgccgactacgctctgcatttgccgaaaaggggattgttgtcgcagcataaccccgattaataaagaatgaaaaaaggatatcaccatgcctgaaggcccggagatccgccgtgcagcggataacctggaggcggcgatcaaaggcaaaccactaactgatgtctggtttgccttcccgcagttaaaaccttatcaatcacaacttatcggtcaacacgttacccatgtggaaacgcgtggtaaggcgttgttaactcatttttccaacgacttaacgctctacagccataatcagctttacggcgtctggcgcgtggttgataccggcgaagagccgcagaccacgcgagtattgcgggtaaaactgcaaacggctgacaaaaccattctgctttatagcgcctcggatattgagatgttgaccccggaacaactgaccacgcatccgtttttacaacgcgttggtcccgatgtgctggatccgaatctgacgccggaggtggtgaaagaacgattattgtcgccgcgctttcgtaaccgtcagtttgctggattactgctcgatcaggcgtttctggctgggcttggcaattatttgcgggtggagatcctctggcaggttgggttgactggaaatcataaagcgaaagatctcaatgcggcgcaactggatgcactcgcacacgcgttactggagattcctcgattttcctacgctacgcgggggcaggtggatgagaataagcatcatggggcgctgtttcgctttaaggtttttcatcgagatggcgaaccgtgcgaacgttgtggcagcatcattgagaaaaccacgctgtcatctcgcccgttttactggtgccctggctgccagcactaggccgaccgcttcggcgcataggttgaaataaaccgcgcaatggcaggccctgtcagcaaaatactgaacaggcgtagggtttgcatcgccataatgagcgccatatcggcattgctccctgcggcgatgaccgccacggtatcaagcccgccggggctggtggcgaggtaggcagtcataaaatcaatgtgcataaaccgggtcagcccccacgccatacccgcacaaatagccagcagagcaaaaatcgacagcaggatttgcggtagcgggcgtagtgcccgcagtaagatttgtttatcgaaaccaagaccaatccgccagccaattgccatatacgccatcgccagcagccattccggtagttcgatggtgatgagctgaccagactggagcactgcgcccgccagcatcgggatgagcatcgtgccggaaggaagacgcagcaggcatcccactgtaccggcaacgaccgcgagcaaaatagtaagcaggagattaatgctcactggcgggaaccagacgatatgctggttaaccgcttcagcgttatcgcccagcatcatgcgggtgaccagaacagcggcccccgcgacgaacagcactcgcagatattgcataaacgccaccaggcgaatatctgcgccgtaatcttgcgccatagcgaccattgccgccgcgccgccaggagaggagccccaggcaccggtatttccaggcaatgagctatagcgcaccaataaccaacccacaatggcgctggaaagcagcgttaccagtaaaattgcaagcacgatcggccagttgacggccagggtggtgagaatcgaaccagtgaggttttgcgcaatcatgcagccaagaatggcctgggcggcgagaaaagcagagcggggaagttgcagagtaattccgcgcatactaaagatgatcccggcgatcatcggcccaagtaatagcgccgccgggagatgtaccgcgaggaaaccaatagaaaggagaagtgatagcacacataacattccccactgcaaaactggcatccttcgctccctcattattttctctttggtgtatcgatacagcataaagaaagctgggccaggaaaaaataacagcaatcaaggaaaaggggaaaatcagcaattttctgaaagagatgccctttccggcggcaaagggcatcatggtaaatcagttatagttaatcttaaaaagcaccactgtatcgaaggggccagcctcgatgggggtgcctggaatggacgaaagttcagccgtataggttttttcgtagaccaacatgtcactggtgaaatcggcgtattcagcatatttattgaaggtataaggcgaggcgttttcatccagtaaacgtagcttcagaccattaccaatcaacaatgctttatcttcttcaaccaacgtttcttcggtataaaaggaggaactgactttaaatccgtcggtgcattgatcgttttggctcttggtcgttttaatactgaacgttttcgacattgtgtggcgacgtatatccagcaaattaaatttaccaaaatcaatcacctgtgtttccggtgaaatggaaaaattgacgctgcaatccagcacgcgaatgttttccagaccagtaatatgatatttcaggttttgggcagtagggtcttcgttaacgctaccggcaccgtcaaattgcacgacgatatagtcgctaagcgtactttgataatcatgcggcggcatttctcgtattttgacgtataaccgcatgcgagcgagaaaggtacgcgacatatgaatattagcgggatcgcccgagcaaattttgttctgccatcccatcgcgatgatctgctcaggggtataaatatcaatgttcttactgtcgatacactggttagtgtcgatgcgactttttcccagactggcatcgtaatcgacaccgttgtatgtcacgccgagttgataataacgatcctgcacccccggataggggtttacccaggcgtagacatgctcgctttcaaagttgccgttggtattgttgtcacaatagacgggaattttaatatcgtcagattcccagatcttatcaccgggtttggcattgcctggtacagcaaacggttgaatcgcttctgatttttctactgcgccaccagatgtaccaaaatagcagttcagcgccattgcagacttcaacggcagaaataacaggcagatgacgagcaacaatcccttgccagcactcatttcgcctccactgcttgtaaacggcattgtccgctgcagttgagcgtcgtcatgcgtaatgcgccgtaatcatccatgtaaccgagataaaactggctgccgctataacttccggtgtttgtgttgaccgtactaaaaggtgcaaccatcacggttttgaagcctgggagaacgcctttttcatttctccccagataggcaatggtcagataatacgcggtaggatttttcagtgtcagttggttgccctgctggctgacctgtaactgcagttcgaccttttctcctgctttcttgcgtaatgcagccggtcgccagaacaatttaatacgactttgaatagcgacctgaagtatcgcatggtcgctgcttttatccggagcgggaggaatttcgcgcatattgtagaaaaatagcgtttcgcgatcgccaggtaattgtgtggttgaggcttgtttcacaacccgcacctgcgatgtcgctttcggttccagacgttgaatagggggcaaagcgaccagaagagcatcgcttttctcccctttttcattttctatccaggaataagcaagataaggcagtttgtcactttggttttcgatacgcaggctggtggctttgtcattggcgttaaacacaatgcgtgtgcgatcgggttgcaccgcagcattgcaacccaagctgatggttaacaacattaagggtaatcctttaataaatgtcattctcttttccttaattaatgacaaggtaaaatcaggcgtttggtcgtgtcttccagacgttctggcagatgaataatgcagctttgctcaccccagaccacggtaaacagttgattttcagcgacaccgcttaaccaggcatgtccttcctcgccaaccatacccacgctaatgccgctgtcatcctggcggatatccgcaccgaggggagggaactgaccgctggcgttgcgtatgatgacgttaacgtctttaccggaacgggaagccagtgatttgtaacctatcgcgccttcaatccatgtttccttgatgacgttttctgcaactgttacgccgtcgggtaagtcattcatgttcaccgccacggtggaaggctggtaactggaaatcaacggcaccaccgcaatgccaaaatggttggtgtagtcgagattgccctgaaccggaatatctgccacgccatcggtgctgaccatcaggcgtggttcattggtggagctgcggcgatgaaatgctgcaccatattgggttgcggtgaaagaaccgctccagctgctgctgacggaactgtaatcactggcggcataggtaccagaaatatcccactcacccgctgaactcaggtgctgatagttaccgctcacctgggctccattgtccggacgatcggattgcagtccggcagacatgccccagctattacgttcatccagcgtatcgttccacgacatgcggtgtatggtgctgtggctactgttttgcatgtcatagccaacccgaccaccgttaccgaaggggagcgaaatcgacagataaatctggttgtcgcgatctttatcttcgtagtgggtcgtattgaatgacgtcgaaatcgagatatctctccagtcaccaatatcaacattaaaacctgctgtgatgttggcggtcgtggaggcgtctgcattccaccaggtttgatgtagcaggttggcgtaaagattgaggtttagtggggtaatcggttggcccacggataagctgatcgtctgtttttcgtcctgcgcatcgctgtcgttgtatttgtgatccagatagttggcgtagctgtgaaaatgacgatctgagaagcgataagcggcgagcgaaatcgtgctgttggtggcatccacttgtttgctgtaattaaaacggtagcttaagccccgctcgtcctgctgagtatcaaaatggctactggcccaggtgacatcaaaggacagtgcgccaagccacagcatattttgcccgatacccattgcggcagaatggtagtcatcatcagaaatcagcaggccgccgtacagcgaggtgtttgagagcatcccccaggaaacttcattgctaaaaaaggtttcattttcagtttgatgtgacatggaaggccgtggctgacccgcggccaatttatagcgaacctgtccctggcgagtcaggaagggcgtcgatgctgccgaaacctggaaattgttcacccgaccatcttcttccgtcactttgacatccagcgtgccctgaacagactgattgaggtcatcaataataaacgggcctggcgggacttttttctggtaaatgacgcggcctgattgactgatcgtcaccgtggcattggtctgtgcaataccgctaatttgtggggcgtagccacgcagctcccacggtaacattcgatcgtcactcgccagtgccgcgccggtataagaaaaaccatcgaaaatattggaactgaaatcggtttcgccgagggttaacttagagcctaattgcggtaatggacgaaaaagataggtgcgcgatattccgcctgactggtcatggttatcttcgctatcggtcttattaagctggtaatcactgcgtaagcgccatgccccggcgttaattccggcggtaccgtaggcattcaggttagtgctgctgctgccgtcctgtgggcggtagctgctggcaaacaagttgtaatccatcaggacaccggcaacaccttctttccatgtagaggggggagcccagttttctgagtgccacgccagccaggcttgcggaatactaatattcagttgctgattggcttgatcgaaattgaagagcatttcaggtcgggaactgaaatcaatacaccgatctatctgtggcaaggactgacggatatctggttttaaaccaaatttatcgaccagtgaatcattgatgcatggaatggttttgtcaccctttttttgccagttaattttttgcccattactgattttgttgttattcaccgcaacgctaacaaaatattcaccgggagcaatgactcctttttcctttaataatgaaatatcaatgcggtcgcgcattgatttatcgagaacattcagattgaattcgaccgccattgcgcaaggcatcgccatgaccaggcaggatacaaaagagagtcgataaatattcacggtgtccatacctgataaatattttatgaaaggcggcgatgatgccgccaaaataatacttatttataatccagcacgtaggttgcgttagcggttacttcacctgccgtgacatcgactgcattatcaatttgttccatccaggcgaaaaagttcagcgtctgttctgatgagcttgcatccaggtcaagatctggcgcggctgaacctaatacgatgttaccgtcatttttgtccatcagtcgtacaccgaccccagttgcttcgcctgcactggtgttgctcaacaaaggcgtagcaccagttgtcttagccgtgctatcgaaggttacgccaactttggataccggcattccgctaccgttgtcagaagcaggcagatcacagttgatcaagcgaatgtcgacggccactttattgctatgatgctcccggtttatatgggttgtcgtgacttgtccaagatctatgtttttatcaatatcttctggatgaatttcacaaggtgcttcaataacctcccccttaaagtgaatttcgccagaaccttcatcagcagcataaacaggtgcagtgaacagcagagatacggccagtgcggccaatgttttttgtcctttaaacataacagagtcctttaaggatatagaataggggtatagctacgccagaatatcgtatttgattattgctagtttttagttttgcttaaaaatattgttagttttattaaatgcaaaactaaattattggtatcatgaatttgttgtatgatgaataaaatataggggggtatagatagacgtcattttcatagggttataaatgcgactaccatgaagtttttaattgaaagtattgggttgctgataatttgagctgttctattctttttaaatatctatataggtctgttaatggattttatttttacaattttttgtgtttaggcatataaaaatcaacccgccatatgaacggcgggttaaaatatttacaacttagcaatcaaccattaacgcttgatatcgcttttaaagtcgcgtttttcatatcctgtatacagctgacgcggacgggcaatcttcataccgtcactgtgcatttcgctccagtgggcgatccagccaacggtacgtgccattgcgaaaatgacggtgaacatggaagacggaatacccatcgctttcaggatgataccagagtagaaatcgacgttcgggtacagtttcttctcgataaagtacgggtcgttcagcgcgatgttttccagctccatagccacttccagcaggtcatccttcgtgcccagctctttcagcacttcatggcaggtttcacgcattacggtggcgcgcgggtcgtaatttttgtacacgcggtgaccgaagcccatcaggcggaaagaatcatttttgtctttcgcacgacgaacaaattccggaatgtgtttaacggagctgatttcttccagcattttcagcgccgcttcgttagcaccgccgtgcgcaggtccccacagtgaagcaatacctgctgcgatacaggcaaacgggttcgcacccgaagagccagcggtacgcacggtggaggtagaggcgttctgttcatggtcagcgtgcaggatcagaatacggtccatagcacgttccagaatcggattaacttcatacggttcgcacggcgtggagaacatcatattcaggaagttaccggcgtaggagagatcgttgcgcgggtaaacaaatggctgaccaatggaatacttgtaacacatcgcggccatggtcggcattttcgacagcaggcggaacgcggcaatttcacggtgacgaggattgttaacatccagcgagtcgtgatagaacgccgccagcgcgccggtaataccacacatgactgccattggatgcgagtcgcgacggaaagcatggaacagacgggtaatctgctcgtggatcatggtatgacgggtcaccgtagttttaaattcgtcatactgttcctgagtcggtttttcaccattcagcaggatgtaacaaacttccaggtagttagaatcggtcgccagctgatcgatcgggaaaccgcggtgcagcaaaataccttcatcaccatcaataaaagtaattttagattcgcaggatgcggttgaagtgaagcctgggtcaaaggtgaacacaccttttgaaccgagagtacggatatcaataacatcttgacccagcgtgcctttcagcacatccagttcaacagctgtatccccgttgagggtgagttttgcttttgtatcagccatttaaggtctccttagcgccttattgcgtaagactgccggaacttaaatttgccttcgcacatcaacctggctttacccgttttttatttggctcgccgctctgtgaaagaggggaaaacctgggtacagagctctgggcgcttgcaggtaaaggatccattgatgacgaataaatggcgaatcaagtacttagcaatccgaattattaaacttgtctaccactaataactgtcccgaatgaattggtcaatacttccacactgttacataagttaatcttaggtgaaataccgacttcataacttttacgcattatatgcttttcctggtaatgtttgtaacaactttgttgaatgattgtcaaattagatgattaaaaattaaataaatgttgttatcgtgacctggatcactgttcaggataaaacccgacaaactatatgtaggttaattgtaatgattttgtgaacagcctatactgccgccaggtctccggaacaccctgcaatcccgagccacccagcgttgtaacgtgtcgttttcgcatctggaagcagtgttttgcatgacgcgcagttatagaaaggacgctgtctgacccgcaagcagaccggaggaaggaaatcccgacgtctccaggtaacagaaagttaacctctgtgcccgtagtccccagggaataataagaacagcatgtgggcgttattcatgataagaaatgtgaaaaaacaaagacctgttaatctggacctacagaccatccggttccccatcacggcgatagcgtccattctccatcgcgtttccggtgtgatcacctttgttgcagtgggcatcctgctgtggcttctgggtaccagcctctcttcccctgaaggtttcgagcaagcttccgcgattatgggcagcttcttcgtcaaatttatcatgtggggcatccttaccgctctggcgtatcacgtcgtcgtaggtattcgccacatgatgatggattttggctatctggaagaaacattcgaagcgggtaaacgctccgccaaaatctcctttgttattactgtcgtgctttcacttctcgcaggagtcctcgtatggtaagcaacgcctccgcattaggacgcaatggcgtacatgatttcatcctcgttcgcgctaccgctatcgtcctgacgctctacatcatttatatggtcggttttttcgctaccagtggcgagctgacatatgaagtctggatcggtttcttcgcctctgcgttcaccaaagtgttcaccctgctggcgctgttttctatcttgatccatgcctggatcggcatgtggcaggtgttgaccgactacgttaaaccgctggctttgcgcctgatgctgcaactggtgattgtcgttgcactggtggtttacgtgatttatggattcgttgtggtgtggggtgtgtgatgaaattgccagtcagagaatttgatgcagttgtgattggtgccggtggcgcaggtatgcgcgcggcgctgcaaatttcccagagcggccagacctgtgcgctgctctctaaagtcttcccgacccgttcccataccgtttctgcgcaaggcggcattaccgttgcgctgggtaatacccatgaagataactgggaatggcatatgtacgacaccgtgaaagggtcggactatatcggtgaccaggacgcgattgaatatatgtgtaaaaccgggccggaagcgattctggaactcgaacacatgggcctgccgttctcgcgtctcgatgatggtcgtatctatcaacgtccgtttggcggtcagtcgaaaaacttcggcggcgagcaggcggcacgcactgcggcagcagctgaccgtaccggtcacgcactgttgcacacgctttatcagcagaacctgaaaaaccacaccaccattttctccgagtggtatgcgctggatctggtgaaaaaccaggatggcgcggtggtgggttgtaccgcactgtgcatcgaaaccggtgaagtggtttatttcaaagcccgcgctaccgtgctggcgactggcggagcagggcgtatttatcagtccaccaccaacgcccacattaacaccggcgacggtgtcggcatggctatccgtgccggcgtaccggtgcaggatatggaaatgtggcagttccacccgaccggcattgccggtgcgggcgtactggtcaccgaaggttgccgtggtgaaggcggttatctgctgaacaaacatggcgaacgttttatggagcgttatgcgccgaacgccaaagacctggcgggccgtgacgtggttgcgcgttccatcatgatcgaaatccgtgaaggtcgcggctgtgatggtccgtgggggccacacgcgaaactgaaactcgatcacctgggtaaagaagttctcgaatcccgtctgccgggtatcctggagctttcccgtaccttcgctcacgtcgatccggtgaaagagccgattccggttatcccaacctgtcactacatgatgggcggtattccgaccaaagttaccggtcaggcactgactgtgaatgagaaaggcgaagatgtggttgttccgggactgtttgccgttggtgaaatcgcttgtgtatcggtacacggcgctaaccgtctgggcggcaactcgctgctggacctggtggtctttggtcgcgcggcaggtctgcatctgcaagagtctatcgccgagcagggcgcactgcgcgatgccagcgagtctgatgttgaagcgtctctggatcgcctgaaccgctggaacaataatcgtaacggtgaagatccggtggcgatccgtaaagcgctgcaagaatgtatgcagcataacttctcggtcttccgtgaaggtgatgcgatggcgaaagggcttgagcagttgaaagtgatccgcgagcgtctgaaaaatgcccgtctggatgacacttccagcgagttcaacacccagcgcgttgagtgcctggaactggataacctgatggaaacggcgtatgcaacggctgtttctgccaacttccgtaccgaaagccgtggcgcgcatagccgcttcgacttcccggatcgtgatgatgaaaactggctgtgccactccctgtatctgccagagtcggaatccatgacgcgccgaagcgtcaacatggaaccgaaactgcgcccggcattcccgccgaagattcgtacttactaatgcggagacaggaaaatgagactcgagttttcaatttatcgctataacccggatgttgatgatgctccgcgtatgcaggattacaccctggaagcggatgaaggtcgcgacatgatgctgctggatgcgcttatccagctaaaagagaaagatcccagcctgtcgttccgccgctcctgccgtgaaggtgtgtgcggttccgacggtctgaacatgaacggcaagaatggtctggcctgtattaccccgatttcggcactcaaccagccgggcaagaagattgtgattcgcccgctgccaggtttaccggtgatccgcgatttggtggtagacatgggacaattctatgcgcaatatgagaaaattaagccttacctgttgaataatggacaaaatccgccagctcgcgagcatttacagatgccagagcagcgcgaaaaactcgacgggctgtatgaatgtattctctgcgcatgttgttcaacctcttgtccgtctttctggtggaatcccgataagtttatcggcccggcaggcttgttagcggcatatcgtttcctgattgatagccgtgataccgagactgacagccgcctcgacggtttgagtgatgcattcagcgtattccgctgtcacagcatcatgaactgcgtcagtgtatgtccgaaggggctgaacccgacgcgcgccatcggccatatcaagtcgatgttgttgcaacgtaatgcgtaaaccgtaggcctgataagacgcgcaagcgtcgcatcaggcaaccagtgccggatgcggcgtgaacgccttatccggcctacaagtcattacccgtaggcctgataagcgcagcgcatcaggcgtaacaaagaaatgcaggaaatctttaaaaactgcccctgacactaagacagtttttaaaggttccttcgcgagccactacgtagacaagagctcgcaagtgaaccccggcacgcacatcactgtgcgtggtagtatccacggcgaagtaagcataaaaaagatgcttaagggatcacgatgcagaacagcgctttgaaagcctggttggactcttcttacctctctggcgcaaaccagagctggatagaacagctctatgaagacttcttaaccgatcctgactcggttgacgctaactggcgttcgacgttccagcagttacctggtacgggagtcaaaccggatcaattccactctcaaacgcgtgaatatttccgccgcctggcgaaagacgcttcacgttactcttcaacgatctccgaccctgacaccaatgtgaagcaggttaaagtcctgcagctcattaacgcataccgcttccgtggtcaccagcatgcgaatctcgatccgctgggactgtggcagcaagataaagtggccgatctggatccgtctttccacgatctgaccgaagcagacttccaggagaccttcaacgtcggttcatttgccagcggcaaagaaaccatgaaactcggcgagctgctggaagccctcaagcaaacctactgcggcccgattggtgccgagtatatgcacattaccagcaccgaagaaaaacgctggatccaacagcgtatcgagtctggtcgcgcgactttcaatagcgaagagaaaaaacgcttcttaagcgaactgaccgccgctgaaggtcttgaacgttacctcggcgcaaaattccctggcgcaaaacgcttctcgctggaaggcggtgacgcgttaatcccgatgcttaaagagatgatccgccacgctggcaacagcggcacccgcgaagtggttctcgggatggcgcaccgtggtcgtctgaacgtgctggtgaacgtgctgggtaaaaaaccgcaagacttgttcgacgagttcgccggtaaacataaagaacacctcggcacgggtgacgtgaaataccacatgggcttctcgtctgacttccagaccgatggcggcctggtgcacctggcgctggcgtttaacccgtctcaccttgagattgtaagcccggtagttatcggttctgttcgtgcccgtctggacagacttgatgagccgagcagcaacaaagtgctgccaatcaccatccacggtgacgccgcagtgaccgggcagggcgtggttcaggaaaccctgaacatgtcgaaagcgcgtggttatgaagttggcggtacggtacgtatcgttatcaacaaccaggttggtttcaccacctctaatccgctggatgcccgttctacgccgtactgtactgatatcggtaagatggttcaggccccgattttccacgttaacgcggacgatccggaagccgttgcctttgtgacccgtctggcgctcgatttccgtaacacctttaaacgtgatgtcttcatcgacctggtgtgctaccgccgtcacggccacaacgaagccgacgagccgagcgcaacccagccgctgatgtatcagaaaatcaaaaaacatccgacaccgcgcaaaatctacgctgacaagctggagcaggaaaaagtggcgacgctggaagatgccaccgagatggttaacctgtaccgcgatgcgctggatgctggcgattgcgtagtggcagagtggcgtccgatgaacatgcactctttcacctggtcgccgtacctcaaccacgaatgggacgaagagtacccgaacaaagttgagatgaagcgcctgcaggagctggcgaaacgcatcagcacggtgccggaagcagttgaaatgcagtctcgcgttgccaagatttatggcgatcgccaggcgatggctgccggtgagaaactgttcgactggggcggtgcggaaaacctcgcttacgccacgctggttgatgaaggcattccggttcgcctgtcgggtgaagactccggtcgcggtaccttcttccaccgccacgcggtgatccacaaccagtctaacggttccacttacacgccgctgcaacatatccataacgggcagggcgcgttccgtgtctgggactccgtactgtctgaagaagcagtgctggcgtttgaatatggttatgccaccgcagaaccacgcactctgaccatctgggaagcgcagttcggtgacttcgccaacggtgcgcaggtggttatcgaccagttcatctcctctggcgaacagaaatggggccggatgtgtggtctggtgatgttgctgccgcacggttacgaagggcaggggccggagcactcctccgcgcgtctggaacgttatctgcaactttgtgctgagcaaaacatgcaggtttgcgtaccgtctaccccggcacaggtttaccacatgctgcgtcgtcaggcgctgcgcgggatgcgtcgtccgctggtcgtgatgtcgccgaaatccctgctgcgtcatccgctggcggtttccagcctcgaagaactggcgaacggcaccttcctgccagccatcggtgaaatcgacgagcttgatccgaagggcgtgaagcgcgtagtgatgtgttctggtaaggtttattacgacctgctggaacagcgtcgtaagaacaatcaacacgatgtcgccattgtgcgtatcgagcaactctacccgttcccgcataaagcgatgcaggaagtgttgcagcagtttgctcacgtcaaggattttgtctggtgccaggaagagccgctcaaccagggcgcatggtactgcagccagcatcatttccgtgaagtgattccgtttggggcttctctgcgttatgcaggccgcccggcctccgcctctccggcggtagggtatatgtccgttcaccagaaacagcaacaagatctggttaatgacgcgctgaacgtcgaataaataaaggatacacaatgagtagcgtagatattctggtccctgacctgcctgaatccgtagccgatgccaccgtcgcaacctggcataaaaaacccggcgacgcagtcgtacgtgatgaagtgctggtagaaatcgaaactgacaaagtggtactggaagtaccggcatcagcagacggcattctggatgcggttctggaagatgaaggtacaacggtaacgtctcgtcagatccttggtcgcctgcgtgaaggcaacagcgccggtaaagaaaccagcgccaaatctgaagagaaagcgtccactccggcgcaacgccagcaggcgtctctggaagagcaaaacaacgatgcgttaagcccggcgatccgtcgcctgctggctgaacacaatctcgacgccagcgccattaaaggcaccggtgtgggtggtcgtctgactcgtgaagatgtggaaaaacatctggcgaaagccccggcgaaagagtctgctccggcagcggctgctccggcggcgcaaccggctctggctgcacgtagtgaaaaacgtgtcccgatgactcgcctgcgtaagcgtgtggcagagcgtctgctggaagcgaaaaactccaccgccatgctgaccacgttcaacgaagtcaacatgaagccgattatggatctgcgtaagcagtacggtgaagcgtttgaaaaacgccacggcatccgtctgggctttatgtccttctacgtgaaagcggtggttgaagccctgaaacgttacccggaagtgaacgcttctatcgacggcgatgacgtggtttaccacaactatttcgacgtcagcatggcggtttctacgccgcgcggcctggtgacgccggttctgcgtgatgtcgataccctcggcatggcagacatcgagaagaaaatcaaagagctggcagtcaaaggccgtgacggcaagctgaccgttgaagatctgaccggtggtaacttcaccatcaccaacggtggtgtgttcggttccctgatgtctacgccgatcatcaacccgccgcagagcgcaattctgggtatgcacgctatcaaagatcgtccgatggcggtgaatggtcaggttgagatcctgccgatgatgtacctggcgctgtcctacgatcaccgtctgatcgatggtcgcgaatccgtgggcttcctggtaacgatcaaagagttgctggaagatccgacgcgtctgctgctggacgtgtagtagtttaagtttcacctgcactgtagaccggataaggcattatcgccttctccggcaattgaagcctgatgcgacgctgacgcgtcttatcaggcctacgggaccaccaatgtaggtcggataaggcgcaagcgccgcatccgacaagcgatgcctgatgtgacgtttaacgtgtcttatcaggcctacgggtgaccgacaatgcccggaagcgatacgaaatattcggtctacggtttaaaagataacgattactgaaggatggacagaacacatgaacttacatgaatatcaggcaaaacaactttttgcccgctatggcttaccagcaccggtgggttatgcctgtactactccgcgcgaagcagaagaagccgcttcaaaaatcggtgccggtccgtgggtagtgaaatgtcaggttcacgctggtggccgcggtaaagcgggcggtgtgaaagttgtaaacagcaaagaagacatccgtgcttttgcagaaaactggctgggcaagcgtctggtaacgtatcaaacagatgccaatggccaaccggttaaccagattctggttgaagcagcgaccgatatcgctaaagagctgtatctcggtgccgttgttgaccgtagttcccgtcgtgtggtctttatggcctccaccgaaggcggcgtggaaatcgaaaaagtggcggaagaaactccgcacctgatccataaagttgcgcttgatccgctgactggcccgatgccgtatcagggacgcgagctggcgttcaaactgggtctggaaggtaaactggttcagcagttcaccaaaatcttcatgggcctggcgaccattttcctggagcgcgacctggcgttgatcgaaatcaacccgctggtcatcaccaaacagggcgatctgatttgcctcgacggcaaactgggcgctgacggcaacgcactgttccgccagcctgatctgcgcgaaatgcgtgaccagtcgcaggaagatccgcgtgaagcacaggctgcacagtgggaactgaactacgttgcgctggacggtaacatcggttgtatggttaacggcgcaggtctggcgatgggtacgatggacatcgttaaactgcacggcggcgaaccggctaacttccttgacgttggcggcggcgcaaccaaagaacgtgtaaccgaagcgttcaaaatcatcctctctgacgacaaagtgaaagccgttctggttaacatcttcggcggtatcgttcgttgcgacctgatcgctgacggtatcatcggcgcggtagcagaagtgggtgttaacgtaccggtcgtggtacgtctggaaggtaacaacgccgaactcggcgcgaagaaactggctgacagcggcctgaatattattgcagcaaaaggtctgacggatgcagctcagcaggttgttgccgcagtggaggggaaataatgtccattttaatcgataaaaacaccaaggttatctgccagggctttaccggtagccaggggactttccactcagaacaggccattgcatacggcactaaaatggttggcggcgtaaccccaggtaaaggcggcaccacccacctcggcctgccggtgttcaacaccgtgcgtgaagccgttgctgccactggcgctaccgcttctgttatctacgtaccagcaccgttctgcaaagactccattctggaagccatcgacgcaggcatcaaactgattatcaccatcactgaaggcatcccgacgctggatatgctgaccgtgaaagtgaagctggatgaagcaggcgttcgtatgatcggcccgaactgcccaggcgttatcactccgggtgaatgcaaaatcggtatccagcctggtcacattcacaaaccgggtaaagtgggtatcgtttcccgttccggtacactgacctatgaagcggttaaacagaccacggattacggtttcggtcagtcgacctgtgtcggtatcggcggtgacccgatcccgggctctaactttatcgacattctcgaaatgttcgaaaaagatccgcagaccgaagcgatcgtgatgatcggtgagatcggcggtagcgctgaagaagaagcagctgcgtacatcaaagagcacgttaccaagccagttgtgggttacatcgctggtgtgactgcgccgaaaggcaaacgtatgggccacgcgggtgccatcattgccggtgggaaagggactgcggatgagaaattcgctgctctggaagccgcaggcgtgaaaaccgttcgcagcctggcggatatcggtgaagcactgaaaactgttctgaaataaatatctgtaataagaaatagccctcgccgcttccctctacaggaatggcgaagggctgtcggtttcgacatggttggccatcgtatgatggccttttttgtgcttatcgcgatgattttcgctgcgctatcagggtaaatttatagtcatcggtattaaaagcgttgcggctatattcaaacacccgaccatcaactaaatatccacgcgatactttttcaagaatcggctttgtctggctgatattaagcagacggctcatctcttcggttggcatcagaggaatgatttcctgttcgctacgatcgataaccattttcttcacttcttcgataaagtgatatttcgaattttccatgacctgccaggtgagatccgggaacaacgcaagcggcatccaggtttcttccagcgccattggcttttgcttgcgatagcgcacgcgcttcacatgccacacacgatcctgcggggtgatttgtagctgttgctgaagaaaatcgtcagccggaatcacttcgaatatcagaacttcactgtgtgtatcgacgtgacggtccgacagtttttcatcaaaactggttaactgaaaaatatcgtaattgacccgctcttctttgacgtaagtcccgctgccctgaatgctttcgaggatctgctgctcgactagctggcgcaaagcctgacgcaccgtaacccggctgacgccaaactctgtttgtagcgctgattcagtgggtaacgcatcgccaggtttaagctcgccacgcgcaatttgttcacgaatgcgatcggcaatctgccggtataagggcttgtgtcccatttttagtatctcattaatacgaatttaaccattatgcccgataaattcatcctgtaaataatacaaatacaatacaaataatttcaatcaagtgaaattgatcacataatggtattgttttatcgggcacactggcgcgactataaaaacgatcaagtgaggatcatgatgaatctgacgactctgacccaccgcgatgcgttgtgtctgaatgcgcgctttaccagccgtgaagaggccatccacgcgttgactcaacgtcttgctgctctggggaaaatttccagtactgagcaatttctggaagaagtgtatcgccgtgaaagccttggcccgaccgccttaggtgaagggttggctgtgccgcatggcaaaactgctgcggtaaaagaagcggcgtttgcggtcgccacactcagcgagccgcttcagtgggaaggcgttgatggcccggaagcagttgatttagtggtgctgctggcgattccccccaatgaagcgggtactacgcatatgcaactgctgacagcgctgaccacgcgccttgcggatgatgagattcgggcgcgtatacagtcggcgacgacgcctgatgagttgctctcggcgctggatgacaagggaggcacgcaaccttctgcctctttttccaacgcgccaactatcgtctgcgtaacggcctgtccggcgggtattgctcacacctatatggctgcggaatatctggaaaaagccggacgcaaactcggcgtaaatgtttacgttgaaaaacaaggcgctaacggcattgaagggcgtttaacggcggatcaactcaatagtgcaaccgcctgtatttttgcggctgaagtcgccatcaaggagagtgagcgttttaatggcattcccgcgctttcagtgcctgttgccgagccgattcgccatgcagaagcgttgatccaacaagcgcttaccctcaagcgtagcgatgagacgcgtaccgtacagcaagatacgcaaccggtgaaaagtgtcaaaacggagctgaaacaggcactgttgagcggaatctcttttgccgtaccgttgattgtcgcggggggcacggtgctggcggtcgcggtattactgtcgcaaatcttcgggctacaagatctgtttaatgaagaaaactcctggctgtggatgtaccgcaagctgggcggcgggctgctcggaattttgatggtaccggtgctcgcggcctataccgcctattctctggcagataaaccggcgttagcgccaggctttgcggctggacttgccgccaacatgatcggctccgggtttctcggcgcggtcgttggcggattgatagccggttacttgatgcgctgggtgaaaaatcacttgcgtcttagcagtaaattcaatggattcctgactttttatctctacccggtgctcggtacgttgggagcgggcagtctgatgctgtttgtggtgggggaacctgtcgcctggatcaataactcgcttaccgcctggctgaacggtctgtcaggaagtaacgcgctgttgctgggtgccattctcggttttatgtgttcctttgaccttggagggccagtgaataaagccgcttatgcattctgcctgggcgcaatggcgaacggcgtttacggcccgtatgccattttcgcctccgtcaaaatggtttcggcatttaccgtaaccgcttccacgatgctcgcaccgcgcctgtttaaagagtttgaaattgagaccgggaaatccacctggctgttagggctggcaggtattaccgaaggggcgatcccgatggcgattgaagatccgctgcgggttattggttcgtttgtgctgggctctatggtaacgggcgctattgtcggtgcgatgaatatcggcctttcgacacccggtgccggcattttctcgctctttttacttcatgataatggcgcgggcggtgttatggcggcaattggctggtttggcgcggcattggtgggggctgcaatctcgactgcaattctcctgatgtggcggcgtcacgcggttaagcatggcaactatctgactgatggcgtaatgccataaacaaaaaggaaacgacgatgaaagcagtatctcgcgttcacatcaccccgcatatgcactgggatcgagagtggtatttcaccaccgaagagtcacgtattctgctggtcaataatatggaagagatcctgtgccgactggaacaggacaacgaatacaaatattacgtactcgacgggcaaacggcgatcctcgaagattatttcgcggtgaaaccggaaaacaaagaccgtgtgaagaaacaggtagaagccggcaagttgattatcggcccctggtatacccagaccgataccacgattgtttctgcggaatccatcgtccgtaatctgatgtacggaatgcgtgactgcctcgcgtttggcgagccgatgaaaataggttatttaccagattcctttggcatgtccgggcaactgccgcatatctacaatggatttggcattacccgcaccatgttctggcgcggatgttcggagcgccacggtactgataaaaccgagtttttgtggcaaagcagtgacggtagcgaagtgacggcgcaggtgctgccgctgggctacgccatcggtaagtacttacctgccgacgaaaacggattacgtaaacgcctcgacagttattttgacgtgctggaaaaagcgtctgtaaccaaagagattttgctgccgaatgggcatgaccagatgccattgcagcaaaatatcttcgaagtgatggataagctacgtgagatctaccctcaacgtaagtttgtgatgagccgctttgaagaggtatttgagaagatcgaagcgcagcgagataatctggcaaccctgaaaggggaatttattgatggcaaatatatgcgcgtgcatcgcaccatcggttctacgcgtatggatatcaaaattgcccacgcgcgtattgaaaataagattgttaatctgctggaaccgctggcaacactggcctggacgttgggttttgaataccaccacggcttgctggagaaaatgtggaaagagatcttaaaaaatcatgcccacgacagtatcggctgctgctgtagtgacaaagttcatcgcgaaatcgtcgcccgcttcgaactggctgaagacatggcggataatctgattcgtttctacatgcgcaaaattgccgacaacatgccgcagagcgacgccgacaaactcgtcctgtttaacctgatgccctggccgcgtgaagaagttatcaacaccactgtgcggctgcgcgccagccagtttaatttgcgggacgatcgcggtcagcctgtaccgtattttattcgccatgcccgtgagatcgatccaggcctaatcgatcggcaaatagttcattacggtaattacgatccctttatggagtttgatatacagatcaaccagattgtcccttctatgggctatcgcacgctttatatcgaagcgaatcagcctggcaacgtaattgcggcaaaaagtgacgctgaagggatactggaaaatgctttctggcaaattgcgctcaatgaggatggttctctgcaactggtagataaagacagcggtgtgcgctatgaccgggtattgcaaattgaagaaagctctgatgatggtgatgaatatgactattcacccgcaaaagaagagtgggtaattaccgcagcgaacgcgaaaccgcaatgcgatattattcatgaagcctggcagagcagggctgttatccgctatgacatggcagtgccgctcaatttgtcagaacgcagcgcccggcaatccactggcagagtaggggtggtgttggttgtcactcttagtcataacagcaggcgtattgatgtggatatcaatcttgataaccaggctgacgatcatcgccttcgtgtcctggtccctacaccttttaacaccgacagtgttctggcagatacgcagtttggttcgctaacgcgccccgtgaacgacagtgcaatgaacaactggcagcaagaaggctggaaagaagcgccggttccggtatggaatatgctcaactatgttgccttacaggaagggcgtaacggcatggctgtctttagcgaagggttacgtgaatttgaagtcatcggtgaagagaagaaaacctttgccattacgttgctgcgtggcgtgggcttactgggcaaagaagatctgcttttaaggcctgggcggccttcgggaattaaaatgccagtcccggactcacaactacgtggtctgctttcttgtcgcctaagtttattgagttataccggtacgccaaccgccgctggtgtagctcagcaggcgcgagcatggctgactccagtacagtgttacaacaaaatcccatgggatgtgatgaagctcaacaaagccggattcaacgtgccggaaagttatagtttgttgaaaatgcccccagtgggatgcctgataagcgcacttaagaaagctgaagaccgacaagaagtgattttacggctgtttaatccggctgaatcagcaacctgtgatgcgactgttgctttcagtcgcgaggtgatttcttgctcagaaacgatgatggatgaacacattaccaccgaggaaaatcaaggttcaaatctatcggggccttttttacccggccagtcacggacgttcagttaccggcttgcctgaatagcaatcaaaccgaagccacatatgcgcggccagattgttgacaaagggcgctttgttcatgccggatacggcatgaacgctttattcggtctacaaaagcaggcaaattcaatatattgcagagatgatgtagacactggcaagcgtagcgcatcaggtaattttgcgtttatcttcactctcaagccacgtatatgtggctttatttttaacaaaataataaccctgggtgagttaattataatataattataagttaactaaatgttaatattggcggggtggatttatgcctttattagtaatcctgaaactctgcgtcgtattagccagtgaccaaaaaaagaattaaggtcaaccgtgctgtttttgcttcgtctctttttatctttaattgccaaccgaaactaatttcagccttataactcacacattttaaacataaatgtcactaaagttaccttattgaaacatgattaacataatttgtaggaattgatatttatcaatgtataagtcttggaaatgggcatcaaaaagagataaattgttctcgatcaaattggctgaaaggcggtaatttagctataaattgatcaccgtcgaaaaatgcaaatttgcttcaacaaaaacctgtttattgtaaggattttgcggcgtaatatatacgtgggatcaatttgagtttttattaacatgtttgcaacctttctttacgccgtttttgtgtgcattcacatggtatgatgaaagtgttcaaacaaatttctattggggcatgcgtgtgaccctttctaacggggttcactctcggagtcttcatgcgatgagcaaggagtcatgatgttagatatagtcgaactgtcgcgcttacagtttgccttgaccgcgatgtaccacttcctttttgtgccactgacgctcggtatggcgttcctgctggccattatggaaacggtctacgtcctctccggcaaacagatttataaagatatgaccaagttctggggcaagttgtttggtatcaacttcgctctgggtgtggctaccggtctgaccatggagttccagttcgggactaactggtcttactattcccactatgtaggggatatcttcggtgcgccgctggcaatcgaaggtctgatggccttcttcctcgaatccacctttgtaggtctgttcttcttcggttgggatcgtctgggtaaagttcagcatatgtgtgtcacctggctggtggcgctcggttcaaacctgtccgcactgtggattctggttgcgaacggctggatgcaaaacccaatcgcgtccgatttcaactttgaaactatgcgtatggagatggtgagcttctccgagctggtgcttaacccggttgctcaggtgaaattcgttcacactgtagcgtctggttatgtgactggcgcgatgttcatcctcggtatcagcgcatggtatatgctgaaaggtcgtgacttcgccttcgctaaacgctcctttgctatcgctgccagcttcggtatggctgctgttctgtctgttattgttctgggtgatgaatccggctacgaaatgggcgacgtgcagaaaaccaaactggctgctattgaagccgagtgggaaacgcaacctgcgcctgctgcctttactctgttcggcattcctgatcaggaagaggagacgaacaaatttgcgattcagatcccttacgcactgggcatcattgcaacgcgttccgtggataccccggttatcggcctgaaagagctgatggtgcagcatgaagaacgcattcgtaacgggatgaaggcgtactctctgctcgaacaactgcgttctggttctaccgaccaggcggttcgtgaccagttcaatagcatgaagaaagacctcggttacggtctgctgctgaaacgctatacgccaaacgtggctgatgcgactgaagcgcagattcaacaggcaaccaaagactccatcccgcgtgtagcgccgctgtactttgcgttccgtatcatggtggcgtgtggcttcctgcttctggcaatcatcgcgctctctttctggagtgtcatccgcaaccgcattggcgagaaaaaatggcttctgcgcgccgcgctgtacggtattccgctgccgtggattgctgtagaagcgggctggttcgtggctgaatatggccgccaaccgtgggctatcggtgaagtgctgccgacagctgtggcgaactcgtcactgaccgcaggcgatctcatcttctcaatggtgctgatttgcggcctgtataccctgttcctggtggcagaattgttcttaatgttcaagtttgcacgcctcggcccaagcagcctgaaaaccggtcgctatcactttgagcagtcttccacgactactcagccggcacgctaagacaggagtcgtcaaatgatcgattatgaagtattgcgttttatctggtggctgctggttggcgttctgctgattggttttgcagtcactgacggtttcgacatgggggtgggcatgctcacccgtttcctcggtcgtaacgacaccgagcgtcgaattatgattaactccattgcaccacactgggacggtaaccaggtttggctgatcaccgcgggcggcgcactctttgctgcctggccgatggtctatgccgctgcgttctccggcttctatgtggcgatgatcctcgtgctggcgtctttgttcttccgtccggtcggttttgactaccgctccaagattgaagaaacccgctggcgtaacatgtgggactggggcatcttcattggtagcttcgttccgccgctggtaattggtgtagcgttcggtaacctgttgcagggcgtaccgttcaacgttgatgaatatctgcgtctgtactacaccggtaacttcttccagttgcttaacccgttcggcctgctggcaggcgtggtgagcgtagggatgatcattactcagggcgcaacctatctgcaaatgcgtaccgtgggcgaactgcacctgcgtacccgtgcaacggctcaggtggctgcgctggtgacactggtctgtttcgcactggctggcgtatgggtgatgtacggtatcgatggttatgtcgtgaaatcgacaatggaccattacgcagcctctaacccactgaataaagaagtggttcgtgaagctggcgcatggctggttaacttcaacaacacgccaattctgtgggctattccggcactgggtgtggttctgccgctgctgaccatcctgactgcacgtatggataaagccgcgtgggcgtttgtgttctcctccctgacgctggcctgcatcatcctgacagccggtatcgcaatgttcccgtttgtgatgccgtccagcaccatgatgaacgcaagtctgacaatgtgggatgcaacttccagccagctgacgcttaacgtcatgacctgggttgcggtggttctggtaccgatcattctgctctacaccgcctggtgttactggaaaatgttcggtcgtatcaccaaagaagatattgaacgtaacacccactctctgtactaagtaaggagctaaaaatgtggtatttcgcatggattctgggaacgcttcttgcctgttcgtttggggtaatcaccgcgctggcgcttgaacacgtcgaatcaggcaaagccggtcaagaagacatctgatgagtaagattatcgcgactttgtatgcggtaatggacaagcgccccctgcgggcgctttccttcgtgatggcgcttctgttagcaggatgtatgttttgggacccatctcgttttgccgcgaagaccagtgaactggaaatctggcatggtttattgctgatgtgggccgtctgtgctggtgtgattcacggcgtgggctttcgtccgcagaaggttctttggcaagggattttttgcccattgcttgccgatattgttctcattgtcgggctgattttcttcttcttttaaatcagaattctctttaaaaaattatgggccgctccaggcccataaatttttacgctcccttaacttgccctcattcccaaacctcaatcgcgcgcgtatagtagcagcgtttaaaagctctaacttttgttgcattaccgggatgtaaagtgaatacaacgctgtttcgatggccggttcgcgtctactatgaagataccgatgccggtggtgtggtgtaccacgccagttacgtcgctttttatgaaagagcacgcacagagatgctgcgtcatcatcacttcagtcagcaggcgctgatggctgaacgcgttgcctttgtggtacgtaaaatgacggtggaatattacgcacctgcgcggctcgacgatatgctcgaaatacagactgaaataacatcaatgcgtggcacctctttggttttcacgcaacgtattgtcaacgccgagaatactttgctgaatgaagcagaggttctggttgtttgcgttgacccactcaaaatgaagcctcgtgcgcttcccaagtctattgtcgcggagtttaagcagtgactgacatgaatatccttgatttgttcctgaaggctagccttctggttaaacttatcatgttgattttgattggtttttcaatcgcatcttgggccattattatccagcggacccgtattcttaacgcagcggcgcgcgaagccgaagcgtttgaagataaattctggtctggaatcgaactctctcgcctctatcaagagagccaggggaaacgggataatctgactggttcggaacaaatcttttacagcgggttcaaagagtttgtgcgcctgcatcgtgccaatagccatgcgccggaagccgtagtggaaggggcgtcgcgtgctatgcgtatctccatgaaccgtgaacttgaaaatctggaaacgcacattccgttcctcggtacggttggctccatcagcccgtatattggtctgtttggtacggtctgggggatcatgcacgcctttatcgccctcggggcggtaaaacaagcaacactgcaaatggttgcgcccggtatcgcagaagcgttgattgcgactgcaattggtctgtttgccgctatcccggcagttatggcctacaaccgcctcaaccagcgcgtaaacaaactggaactgaattacgacaactttatggaagagtttaccgcgattctgcaccgccaggcgtttaccgttagcgagagcaacaaggggtaagccatggccagagcgcgtggacgaggtcgtcgcgatctcaagtccgaaatcaacattgtaccgttgctggacgtactgctggtgctgttgctgatctttatggcgacagcgcccatcatcacccagagcgtggaggtcgatctgccagacgctactgaatcacaggcggtgagcagtaacgataatccgccagtgattgttgaagtgtctggtattggtcagtacaccgtggtggttgagaaagatcgcctggagcgtttaccaccagagcaggtggtggcggaagtgtccagccgtttcaaggccaacccgaaaacggtctttctgatcggtggcgcaaaagatgtgccttacgatgaaataattaaagcactgaacttgttacatagtgcgggtgtgaaatcggttggtttaatgacgcagcctatctaaacatctgcgtttcccttgcttgaaagagagcgggtaacaggcgaacagtttttggaaaccgagagtgtcaaaggcaaccgaacaaaacgacaagctcaagcgggcgataattatttcagcagtgctgcatgtcatcttatttgcggcgctgatctggagttcgttcgatgagaatatagaagcttcagccggaggcggcggtggttcgtccatcgacgctgtcatggttgattcaggtgcggtagttgagcagtacaaacgcatgcaaagccaggaatcaagcgcgaagcgttctgatgaacagcgcaagatgaaggaacagcaggctgctgaagaactgcgtgagaaacaagcggctgaacaggaacgcctgaagcaacttgagaaagagcggttagcggctcaggagcagaaaaagcaggctgaagaagccgcaaaacaggccgagttaaagcagaagcaagctgaagaggcggcagcgaaagcggcggcagatgctaaagcgaaggccgaagcagatgctaaagctgcggaagaagcagcgaagaaagcggctgcagacgcaaagaaaaaagcagaagcagaagccgccaaagccgcagccgaagcgcagaaaaaagccgaggcagccgctgcggcactgaagaagaaagcggaagcggcagaagcagctgcagctgaagcaagaaagaaagcggcaactgaagctgctgaaaaagccaaagcagaagctgagaagaaagcggctgctgaaaaggctgcagctgataagaaagcggcagcagagaaagctgcagccgacaaaaaagcagcagaaaaagcggctgctgaaaaggcagcagctgataagaaagcagcggcagaaaaagccgccgcagacaaaaaagcggcagcggcaaaagctgcagctgaaaaagccgctgcagcaaaagcggccgcagaggcagatgatattttcggtgagctaagctctggtaagaatgcaccgaaaacggggggaggggcgaaagggaacaatgcttcgcctgccgggagtggtaatactaaaaacaatggcgcatcaggggccgatatcaataactatgccgggcagattaaatctgctatcgaaagtaagttctatgacgcatcgtcctatgcaggcaaaacctgtacgctgcgcataaaactggcacccgatggtatgttactggatatcaaacctgaaggtggcgatcccgcactttgtcaggctgcgttggcagcagctaaacttgcgaagatcccgaaaccaccaagccaggcagtatatgaagtgttcaaaaacgcgccattggacttcaaaccgtaatcgcgatgttgactgttcggacggtcaacatcaggcaccggttgccacggggttctggtagttttgtgtattttagtttgttaacattctgctaaattatcgtgggccatcggtccagataagggagatatgatgaagcaggcattacgagtagcatttggttttctcatactgtgggcatcagttctgcatgctgaagtccgcattgtgatcgacagcggtgtagattccggtcgtcctattggtgttgttcctttccagtgggcggggcctggtgcggcacctgaagatattggcggcatcgttgctgctgacttgcgtaacagcggtaaatttaatccgttagatcgcgctcgtctgccacagcagccgggtagtgcgcaggaagtacaaccagctgcatggtccgcactgggcattgacgctgtagttgtcggtcaggtcactccgaatccggatggttcttacaatgttgcttatcaacttgttgacactggcggcgcaccgggtactgtacttgctcagaactcgtacaaagtgaacaagcagtggctgcgttatgctggtcataccgccagtgatgaagtgtttgaaaaactgaccggcattaaaggtgcgttccgtactcgtattgcctacgttgttcagaccaacggcggtcagttcccgtatgaactgcgcgtatctgactatgacggttacaaccagtttgtcgttcaccgttcaccgcagccgctgatgtctccggcgtggtcaccagacggttctaaactggcttatgtgaccttcgaaagcggtcgttccgcgctggttattcagacgctggcaaatggcgctgtacgtcaggtggcttcattcccgcgtcacaacggtgcacctgcattctcgccagacggcagcaaactggcattcgccttgtcgaaaaccggtagtctgaacctgtacgtaatggatttggcttctggtcagatccgccaggtgactgatggtcgcagtaacaataccgaaccgacctggttcccggatagccagaacctggcatttacttctgaccaggccggtcgtccgcaggtttataaagtgaatatcaacggcggtgcgccacaacgtattacctgggaaggttcgcagaaccaggatgcggatgtcagcagcgacggtaaatttatggtaatggtcagctccaatggtgggcagcagcacattgccaaacaagatctggcaacgggaggcgtacaagttctgtcgtccacgttcctggatgaaacgccaagtctggcacctaacggcactatggtaatctacagctcttctcaggggatgggatccgtgctgaatttggtttctacagatgggcgtttcaaagcgcgtcttccggcaactgatggacaggtcaaattccctgcctggtcgccgtatctgtgataataattaattgaatagtaaaggaatcattgaaatgcaactgaacaaagtgctgaaagggctgatgattgctctgcctgttatggcaattgcggcatgttcttccaacaagaacgccagcaatgacggcagcgaaggcatgctgggtgccggcactggtatggatgcgaacggcggcaacggcaacatgtcttccgaagagcaggctcgtctgcaaatgcaacagctgcagcagaacaacatcgtttacttcgatctggacaagtacgatatccgttctgacttcgctcaaatgctggatgcacatgcaaacttcctgcgtagcaacccgtcttacaaagtcaccgtagaaggtcacgcggacgaacgtggtactccggaatacaacatctccctgggtgaacgtcgtgcgaacgccgttaagatgtacctgcagggtaaaggcgtttctgcagaccagatctccatcgtttcttacggtaaagaaaaacctgcagtactgggtcatgacgaagcggcatactccaaaaaccgtcgtgcggtactggtttactaagagaattgcatgagcagtaacttcagacatcaactattgagtctgtcgttactggttggtatagcggccccctgggccgcttttgctcaggcaccaatcagtagtgtcggctcaggctcggtcgaagaccgcgtcactcaacttgagcgtatttctaatgctcacagccagcttttaacccaactccagcaacaactttctgataatcaatccgatattgattccctgcgtggtcagattcaggaaaatcagtatcaactgaatcaggtcgtggagcggcaaaagcagatcctgttgcagatcgacagcctcagcagcggtggtgcagcggcgcaatcaaccagcggcgatcaaagcggtgcggcggcatcaacgacgccgacagctgatgctggtactgcgaatgctggcgcgccggtgaaaagcggtaatgcaaacacggattacaatgcagctattgcgctggtgcaggataaatcccgccaggatgacgcaatggtggcatttcagaatttcatcaaaaattaccctgattcaacttacctgccaaacgccaattattggctgggtcagttaaactacaacaagggtaaaaaagatgatgcggcgtactattttgcttcggtagtgaaaaactatccgaagtcaccaaaggctgcagatgcgatgtttaaagtcggcgtcatcatgcaggacaaaggtgacaccgcaaaagcgaaagccgtataccagcaggttatcagtaaataccctggtactgatggcgctaaacaggcacaaaaacgtctgaacgcgatgtaatgcataacacacgaccagaagtcgcattatttctggtcgtgtcgtgcgaatcataagcagttgagtgatctacatcgaaatttttgttgcgctcaagtctgaaatcagtaatatatgccgccgttgccacgggatatcaaacaaaccgaaagcaacgaaaaagtgggtcgttagctcagttggtagagcagttgacttttaatcaattggtcgcaggttcgaatcctgcacgacccaccaatcgctaaggtggaagcggtagtaaaacgtgaaggataacgttgcatgagcaacggcccgaagggcgagacgaagtcgagtcatcctgcacgacccaccactaacatagttagttgtagtatccagcgtagtatcgggtgattagctcagctgggagagcacctcccttacaaggagggggtcggcggttcgatcccgtcatcacccaccaccgggtcgttagctcagttggtagagcagttgacttttaatcaattggtcgcaggttcgaatcctgcacgacccaccagttttaacatcgaagacagatgttaagcgtgtaggataacgttgcgtcagcaacggcccgtagggcgagcgaagcgagtcatcctgcacgacccaccactaatgacggtgggttcggtggaagtagtttgtagtatccagcgcagtatcgggtgattagctcagctgggagagcacctcccttacaaggagggggtcggcggttcgatcccgtcatcacccaccactcgggtcgttagctcagttggtagagcagttgacttttaatcaattggtcgcaggttcgaatcctgcacgacccaccagttttaacatcaaactcagatgttaagcgtgaaggataacgttgcgccagcaacggcccgtagggcgagcgaagcgagtcatcctgcacgacccaccaatcttaaagattggccccgagtaaaaatctttcaggtaacacccgtatgggtcgttagctcagttggtagagcagttgacttttaatcaattggtcgcaggttcgaatcctgcacgacccaccaatttaaaggtggttactggtagagaacgtgaaggataacgttgcgttagcaacggcccgaagggcgagacgaagtcgagtcatcctgcacgacccaccatcctgaatgattaaggcagcataatcccgcaaggggtcgttagctcagttggtagagcagttgacttttaatcaattggtcgcaggttcgaatcctgcacgacccaccaatgtaaaaaagcgccctaaaggcgcttttttgctatctgcgatactcaaagattcgaacctgcagcaggtttgagttgagcgcagcgaaacaacggagccgctcgcggcgacggcccgaagggcgagcgaagcgagtcatcctgcacgacccaccaatgtaaaaaagcgccctaaaggcgcttttttgctattcaggcatcctcaatttcactttgtaaacctgatgacatcgtcagagcttactgtgcaagcaactctatgtcggtggaattaggcgtaaaatgacgcatcctgcacattaggcgtaattcgagtgacttttccccaccattcgactatcttgtttagcatataaaacaaattacaccgataacagcgaatattacgctaatgtcggttttaacgttaagcctgtaaaacgagatggtaagatgagcgtaatgtttgatccagacacggcgatttatcctttccccccgaagccgacgccgttaagcattgatgaaaaagcgtattaccgcgagaagataaaacgtctgctaaaagaacgtaatgcggtgatggttgcccactactataccgatcccgaaattcaacaactggcagaagaaaccggtggctgtatttctgattctctggaaatggcgcgcttcggtgcaaagcatcccgcttctactttgttagtcgctggggtgagatttatgggagaaaccgccaaaattctcagtccggaaaaaacaattctgatgccgacacttcaggctgaatgttcactggatctcggctgccctgttgaagaatttaacgcattttgcgatgcccatcccgatcgtactgtcgtcgtctacgccaacacttctgctgcggtaaaagcgcgcgcagattgggtggtaacttcaagcattgccgtcgaacttattgatcatcttgatagtttgggtgaaaaaatcatctgggcacccgacaaacatctggggcgttacgtgcaaaaacagacgggtggagacattctatgctggcagggtgcctgtattgtgcatgatgaatttaagactcaggcgttaacccgcttgcaagaagaatacccggatgctgccatactggtgcatccagaatcaccacaagctattgtcgatatggcggatgcggtcggttccaccagtcaactgatcgctgctgcgaaaacattgccacatcagaggcttattgtggcaaccgatcggggtattttctacaaaatgcagcaggcggtgccagataaagagttactggaagcaccaaccgcaggtgagggtgcaacctgccgcagctgcgcgcattgtccgtggatggccatgaatggccttcaggccatcgcagaggcattagaacaggaaggaagcaatcacgaggttcatgttgatgaaaggctgcgagagagggcgctggtgccgctcaatcgtatgctggattttgcggctacactacgtggataacgaataataaggcgtaacgttacgctttgggggaaagatggatttttttagtgtgcagaatatcctggtacatataccaataggggcaggcggttatgatctctcatggatcgaagcggtaggcacgatcgccgggttgctgtgtattggccttgccagtctggagaagatcagcaactacttctttggcctgatcaacgtcaccttgtttggcattattttctttcagattcagctgtatgccagcctgctattacaggtgtttttctttgccgcgaatatttacggttggtatgcgtggtcgcgacaaaccagtcagaacgaggcggagttgaaaattcgctggttgccattgccgaaggcactcagctggttggcggtttgcgttgtttcgattggtctgatgacggtatttatcaatccggtgtttgcatttttgacccgcgtggcagtcatgatcatgcaagcattaggattacaggttgtgatgcctgaactgcaaccggacgctttcccgttctgggattcatgcatgatggtgttatctatcgtggcaatgattctgatgacgcgtaagtatgtggaaaactggctgttgtgggtgattattaacgtgattagcgtcgttatttttgcacttcagggcgtttacgccatgtctctggagtacatcatcctgacctttattgcgctcaacggcagccggatgtggatcaacagcgcacgtgaaagaggctcacgcgcgctgtcccattaatggtgatgatgtgaatggccagacaccccttcattcaggtggcagtctggcccatgacaaggttgatattccatctgaatggtggcgtgctcaatctgatagtgatccatcaggtagtgttggatctgatccaacaaggcatcgtgatcgtgtggcgggatcacctgcacatgcaacgtcatcaccggcttctcgcctaccatccatacatgtacatggtgcacattgcggacttccgggatttcccggcacatacgacgcttcagttcagcgatatccagcgataccggtgcaccttcaagtaattcattcacgctatctttcaacagtcgccacgcgctacgcagaaccagaagcgacaccagtatcgagagaatggggtcagcaggtgtccagccagtccagataataatcaacgcggcaataatagccccaaccgaacccagcaggtccccgagcacatgcagtgccgctgctcgtacgttgaggtttttctcttcgctgccgtgatgaagtaaccagaaagaaagtatatttgccagcaacccagccacggcaattgccatcatcatgccgccctcgaccggacgcggcgtgcggaagcgttctatcgcctcccagacaatcaaaatggtaattaccacgagggctatggcattcacaaacgccgcgagcgtggtcagtcttagccaaccgaaagtgtggcgaatggtgggaggacgacgtgaaaattgcacggcgagtagggcgaaaagcagggcggcagtatcggtcaacatatgacccgcatcggccagcaatgccagagaaccagaaagaaaaccaccaacgacttctaccagcataaacccggcagtcacgccgaaagcatacaacaagcgacgagcattattatcttctggcaggtgtgaggacgtgtgtgagtgtgagtgcgccatgacgagtcatcccttaattattctcacttaactttatgacatcatactgcttttagaagtgaaaaattaaaagggagagactccgctctcccattattggctattttgcagggttactgcgtggtaccgtcggttttggtatcgacatcattattgatgccatcaccggtttgtacctttttattgatatccggacagcgaccatctttgcacatggtgttcttgtgctcttcatctttggtcattccgtcattgttcattgaagaaccatccgaatgcagcattgtgccgccagaaccggtatttaccccgttattgtcgacgttatttggcgcgacattttcacgggcgtcaggggctacctggcccgcatcagctgcggcgtttgcctggccgttattagtttgcgctccgctatcggcagccagtgcggcaccgctggcaaggcttagagtggcagtcagaaataatgtggccagttttgtcattttcataggatgctcctgttatggtcgttatgtcggataacctcttccaacagtgcatttgcaggtgaatataaggcattggtttaagatttcagccaggttatgaaacgcagcagagaatcttgaaataattaacaaacaaaggagttacagttagaaattgtaggagagatctcgtttttcgcgacaatctggcgtttttcttgctaattccaggattaatccgttcatagtgtaaaaccccgtttacacattctgacggaagatatagattggaagtattgcattcactaagataagtatggcaacactggaacagacatgaattatcagaacgacgatttacgcatcaaagaaatcaaagagttacttcctcctgtcgcattgctggaaaaattccccgctactgaaaatgccgcgaatacggttgcccatgcccgaaaagcgatccataagatcctgaaaggtaatgatgatcgcctgttggttgtgattggcccatgctcaattcatgatcctgtcgcggcaaaagagtatgccactcgcttgctggcgctgcgtgaagagctgaaagatgagctggaaatcgtaatgcgcgtctattttgaaaagccgcgtaccacggtgggctggaaagggctgattaacgatccgcatatggataatagcttccagatcaacgacggtctgcgtatagcccgtaaattgctgcttgatattaacgacagcggtctgccagcggcaggtgagtttctcgatatgatcaccccacaatatctcgctgacctgatgagctggggcgcaattggcgcacgtaccaccgaatcgcaggtgcaccgcgaactggcatcagggctttcttgtccggtcggcttcaaaaatggcaccgacggtacgattaaagtggctatcgatgccattaatgccgccggtgcgccgcactgcttcctgtccgtaacgaaatgggggcattcggcgattgtgaataccagcggtaacggcgattgccatatcattctgcgcggcggtaaagagcctaactacagcgcgaagcacgttgctgaagtgaaagaagggctgaacaaagcaggcctgccagcacaggtgatgatcgatttcagccatgctaactcgtccaaacaattcaaaaagcagatggatgtttgtgctgacgtttgccagcagattgccggtggcgaaaaggccattattggcgtgatggtggaaagccatctggtggaaggcaatcagagcctcgagagcggggagccgctggcctacggtaagagcatcaccgatgcctgcatcggctgggaagataccgatgctctgttacgtcaactggcgaatgcagtaaaagcgcgtcgcgggtaaggtttaattgtcggatgcgccgtcagagtggcgtatccgatgaatcaccacaggcctgataagtcgcgcagcgtcgcatcaggcaatgtgctccattgttagcaacaaaaaagccgactcacttgcagtcggctttctcattttaaacgaatgacgtttacttcgctttaccctggtttgcaaccgccgctgctttcgctgcgatctcgtcagcattacccagataatagcgtttcagcggtttgaaattctcgtcgaactcatacaccagcggcacgccagtcgggatattaagctcaagaatctcttcttcgctcatgttatcaagatatttcaccagcgcacgtaaagagttaccgtgtgcagcgatgatcacgcgctcaccgctcttcatacgcggcagaatagtttcattccagtaagggatcacgcggtcaatggtcagcgccaggctttccgtcagcggcagttctttctcgctcagtttcgcgtaacgcggatcgtgacccggataacgctcatcatctttagtcagttccggcggagtcactgcaaaaccacgacgccactgtttcacctgctcgtcgccatacttttcagcagtttccgctttgttcagaccctgcaacgcaccgtagtgacgttcgttcagtttccaggatttctcaacgggcagccatgcctgatccagttcgtccagcacattccacagggtatggatagcgcgtttcagcacagaagtgtaagcaaagtcaaagctgtaaccttcctctttcagcagcttacctgctgcttttgcttcgcttacgcctttctcagacagatccacgtcgtaccaaccggtgaaacggttttctttgttccactgactttcgccatgacgaaccagaaccagcttagttacagccatatacttactcctcaaatcatcttttaatgataataattctcattatattgccgcgacgaagcaacagcaatgcttacgcataaccatagcgaaaatagtggcgcagtgtaaggttgttgtgaatattgagttgcaaatatgtcggtgtttgctggtgatttgaacaatatgagataaagccctcatgacgagggcgtaacattactcagcaataaactgatattccgtcaggctggaatactcttcgccaggacgcaggaagcagtccggttgcggccattcagggtggttcgggctgtccggtagaaactcgctttccagagccagcccttgccagtcggcgtaaggttcggttccccgcgacggtgtgccgccgaggaagttgccggagtagaattgcagagccggagcggtggtgtagaccttcagctgcaatttttcatctgctgaccagacatgcgccgccactttcttgccatcgcctttggcctgtaacaagaatgcgtgatcgtaacctttcactttgcgctgatcgtcgtcggcaagaaactcactggcgatgattttggcgctgcggaaatcaaaagacgttccggcgacagatttcaggccgtcgtgcggaatgccgccttcatcaaccggcagatattcgtccgccagaatctgcaacttgtgattgcgcacgtcagactgctcgccgtcaagattgaaatagacgtgattagtcatattcaccgggcaaggtttatcaactgtggcgcgataagtaatggagatacggttatcgtcggtcagacgatattgcaccgtcgcgccgagattacccgggaagccctgatcaccatcatctgaactcagggcaaacagcacctgacgatcgttctggttcacaatctgccagcgacgtttgtcgaacccttccggcccgccgtgcagctggttaacgccctgacttggcgaaagcgtcacggtttcaccgtcaaaggtataacggctattggcgatacggttggcataacgaccaatagaggcccccagaaacgcggcctgatcctgatagcattccgggctggcacagccgagcagcgcctcgcggacgctgccatcggaaagcggaatacgggcggaaagtaaagtcgcaccccagtccatcagcgtgactaccatccctgcgttgttacgcaaagttaacagtcggtacggctgaccatcgggtgccagtgcgggagtttcgttcagcactgtcctgctccttgtgatggtttacaaacgtaaaaagtctctttaatacctgtttttgcttcatattgttcagcgacagcttgctgtacggcaggcaccagctcttccgggatcagcgcgacgatacagccgccaaatccgccgccggtcatgcgtacgccacctttgtcgccaatcacagctttgacgatttctaccagagtgtcaatttgcggcacggtgatttcgaaatcatcgcgcatagaggcatgagactccgccatcaactcgcccatacgtttcaggtcgccttgctccagcgcgctggcagcttcaacggtgcgggcgttttcagtcagtatatgacgcacgcgttttgccacgatcgggtccagttcatgcgcaacagcgttgaactcttcaatggtgacatcacgcagggctggctgctggaagaaacgcgcaccggtttcgcactgttcacgacgggtgttgtattcgctgccaaccagggtacgtttgaagttactgttgatgatgacgacagccacacctttgggcatggaaactgctttggtccccagtgagcggcaatcgatcagcaaggcatgatctttcttgccgagcgcggaaattagctgatccatgatcccgcagttacagcctacaaactggttttctgcttcctgaccgttaagcgcgatttgtgcgccgtccagcggcagatgataaagctgctgcaatacggttccgaccgcgacttccagtgaagcggaagaacttaacccggcaccctgcggcacattgccgctgatcaccatgtccacgccgccgaagctgttgttacgcagttgcagatgtttcaccacgccacgaacgtagttagcccattgatagttttcatgtgcgacaatgggcgcatcgagggaaaactcgtcgagctgattttcataatcggctgccatcacgcgaactttacggtcatcgcgtggtgcacaactgatcacggtttgataatcaatcgcgcagggcagaacgaaaccgtcgttgtagtcggtgtgttcaccaatcaaattcacgcggccaggcgcctgaatggtgtgagtggcagggtagccaaatgcgttggcaaacagagattgtgttttttctttcagactcatttcttacactccggattcgcgaaaatggatatcgctgactgcgcgcaaacgctctgctgcctgttctgcggtcaggtctcgctgggtctctgccagcatttcataaccaaccataaatttacgtacggtggcggagcgcagcagaggcggataaaagtgcgcgtgcagctgccagtgttgattctcttcgccattaaatggcgcgccgtgccagcccatagagtaggggaaggagcactggaagaggttgtcataacgactggtcagctttttcaacgccagcgccagatcgctgcgctgggcgtcggtcaaatcggtgatccgtaaaacgtgggctttgggcagcagtagcgtttcgaacggccaggcagcccagtaaggcacgacggctaaccagtgttcggtttcgacaacggtacggctaccgtctgccagctcgcgctgaacataatccaccagcattggtgatttctgttcggcaaaatattctttttgcaggcggtcttcgcgctcagcttcgttaggcaggaagctatttgcccaaatctgaccgtgcggatgcgggttagagcagcccatcgccgcgcctttgttttcaaaaacctgcacccatgggtacgttttccccagttctgcggtttgctcctgccaggttttgacgatttccgtcaatgctgcaacgctgagctctggcagcgttttactgtgatccggtgaaaagcagatcacccggctggtgccgcgcgcgctctggcaacgcatcagcggatcgtgactttctggcgcatctggcgtgtcagacatcaaagccgcaaagtcattagtgaaaacgtaagtcccggtgtaatcggggtttttatcgcctgtcacccgcacattacctgcgcagaggaagcaatctggatcgtgcgcaggtaacacctgtttggctggcgtttcctgcgccccctgccaggggcgcttagcgcggtgcggtgaaaccagaatccattgcccggtgagcgggttgtagcggcgatgtggatgatcaacgggattaaattgcgtcatggtcgttccttaatcgggatatccctgtggatggcgtgactgccagtgccaggtgtcctgcgccatttcatcgagtgtgcgcgttacgcgccagttcagttcacggtcggctttgctggcgtccgcccagtaggccggaaggtcgccctcgcgacgcggtgcaaaatgataattaaccggtttgccgcaggctttgctgaaggcattaaccacgtccagcacgctgttgcctacgccagcgccgaggttgtagatgtgtacgcctggcttgttcgccagtttttccatcgccacgacgtgaccgtccgccagatccattacgtggatgtaatcgcgtacgccagtaccatcttcggtcggataatcgttaccaaaaatcgccagcgagtcgcgacggcctacagcaacctgggcgatgtatggcatcaggttattcggaatgccttgcggatcttcgcccatatcgcccgacggatgcgcgccaaccgggttgaagtagcgcagcagggcaatgctccagtccggctgggctttttgcagatcggtgaggatctgttccaccatcagcttgcttttgccgtaagggctttgcggtgtgccggtcgggaagctttcaacgtatggaattttgggctgatcgccataaacggtggcggaggagctaaaaataaagtttttgacgttagcggcgcgcatggcgctaatcaggcgcagagtgccgttgacattgttgtcgtaatattccagcggtttttgtaccgattcgcccacggctttcagcccggcgaagtggatcacggtgtcgatagcgtgatcgtgcaggatctcggtcatcaacgcttcgttacgaatatcgccttcaacaaacgttggatgtttgccgcctaaacgctcgataacaggcagtacgctgcgcttactgttacagaggttatcaagaatgatgacatcatgaccgttttgcagtaattgcacacaggtatgacttccaatgtaaccgctaccaccggtaaccagaactctcataattcgctccattaggcttatggtatgaaataaccatagcataacaaagatgcgaaaagtgtgacatggaataaattagtggaatcgtttacacaagaatttagccgttttttatgcgcgattaagtgattataaaacagagggtttatgaatgattgcgctttttatctgaaaaaagacgcggtttcatgcctgcatgcgtcgaaccgttggccggagagggtgctaaggccgcctccggcaaggtcagcactaccgactcaatatatttttgtcagcacatagcgatagagtccaccgtccggcacgaactcaagacgatgggtaatacaggcaggcgcatcttcagcgtggtgcgaaacaaacaacaattgcgtttcaccttcgctaatcagcacatcaacaaaacggcggataagctggcgattcagcggatcaagcccctgtagtggttcatcgagaataagcaacgtcggatgtttcaccagtgcgcggacaatcagcgccagacgctgctgtccccaggaaagactatggaacggagcgtcagccgtgcgtttatcaatgccgagaatatccagccactgctgcaccagtttttgctggcgatccgaaacggcctgataaatgccaatcgaatcaaaatagccagaaagaatcacattacgcacggtagtgctgacccggtaatccagatgcaaactactgctgacgtaaccgatatgctttttgatatcccagatggtttcgccgctgccgcgacgtcgtccgaaaagcgtcaaatcgttgctgtaaccttgcggatgatcgccagtaaccaggcttaataacgtcgattttcctgcaccatttggcccgacaatttgccagtgttcgcctggattcacctgccagctaaggttattaagaatggggcgatcgttataagaaaccacgccattgttcagcacaatgcgcggttcgttggcgggtaaggcgtgacgtgctgaaggttcatccggctccggcagttgcacaccttcaagctgttcactatgcgccagttgcgcgacgagtgcttgttggagcagttcctctttagcgccagtttccgctaacgtgcaatccgccagcacgccagcaaactggacaaactccgggatctcatcgaagcgattgagcaccagtaccagagtaataccggactgatgtaacgaggcgagtcgctcagccagctgctgacgtgaggcaacatccaggccatcgaacggctcatcaagaatcaacaagtcaggctccgacatcagcgcctgacacagcagggtttttcgcgtctcgccagtggaaaggtatttaaagcgtcggtcgaggagggcggtaataccgaactgctgcgccagttgcatgcaacgcggtgcatcctttacttcatcctgaatgatctcagccgtagtgcgtccggtgtcatcttcgccagggccgagcatatcggtgttattccgctgccattcgtcgctgacgagtttttgcaattgctcgaaggagagacgagtgatgtgggaaaactggctttgccgttcacctttcaaaagcggaagttcccccgccagcgcgcgggccagggccgatttcccgcttccattcgaaccgacaaacgcccaactatcacccgcgtttaacgttagctgaggcaattgcagcgtttttgtgtcgctaagacgaaacgtgccttgcaaaatttgcaacgatgacattttatatcccactttgtgcagcgattactgacagggatacgtgtttcataacaaattgtcaacacgcttagcacagcgtggcgataatcacgctgtcggcattaaagtaggccgtgacattctgtccttgctgaagagaagtcgcttcatttaccggcactgtggcgcacagtgtttgcccgtcgggtagcgccattaatacttcgcactgctctgcgccgcgctcaatatgactaataatacccggtaattggttgtcagcgttttgcgcgaccgcctcgtcctgagtaatacctacccacggcgcttttagcaatatcaacacttctttgccttcatccagccccagacgcgcgccgctttgtgcggtaattgcgactttcaggcgtgtttttccgtcagccagtaagacatcaacatgctgttgaacgtcatcatgatcgcgggcggtgatggtaccgaaccactggttacgggcgctggtttgcagtgaaaaacgtgagatcgcggccagcaggctgttcagcggcagggcgtcatcgtcacttaacacatcaaaggctttttgctggatttgcgccagtaagtcatagagctgaatcagtcgctgaccatagcgggtcagtactgcgccgccgccacctttaccgcctgttgcgcgctcgaccagaatatgctcacttaactgattcatctcgttaatggcatcccaggcgcttttatagctaataccggcatctttcgctccctggctaatggaaccggaaagcgcaatgtgttttagtagcgaaatgcggcgcgggtcggcgaataatttttgttggagcttaagggtgagaaggatttcggcctgcataacaatgtcctggcaaaagtcttattgtgacggaaaacgaacgccacgcaaagctgaccgcacaaaaggggagtgcttttctgtgcttagcggttagaatagtctcatgactatatctggagttgaccatgttagagttattaaaaagtctggtattcgccgtaatcatggtacctgtcgtgatggccatcatcctgggtctgatttacggtcttggtgaagtattcaacatcttttctggtgttggtaaaaaagaccagcccggacaaaatcattgattccctgaatgcccgcttagtcgggcattttctttttctcaacttcctgcttttcctgccgatattttttcttatctacctcacaaaggttagcaataactgctgggaaaattccgagttagtcgttatattgtcgcctacataacgttacattaaggggttaccaatggctcgtaaatggttgaacttgtttgccggggcggcactctctttcgctgttgctggcaatgcactggcagatgaagggaaaatcacggtgttcgccgccgcatcactgactaacgcaatgcaggacattgctacgcagtttaaaaaagagaaaggcgtggatgtggtttcttctttcgcttcgtcatctactctcgcccgtcagattgaagcgggtgcgcctgcggatctgtttatttctgccgatcagaaatggatggattatgcggttgataaaaaagcgatcgatacagctacgcgtcagacactgctcggcaatagcctggtcgttgtagcaccgaaagccagcgtgcagaaagatttcaccatcgacagcaaaaccaactggacttcactgctgaatggcggtcgcctggcggttggcgatccggaacatgttcccgctggcatttatgcaaaagaagcactgcaaaaactgggcgcatgggatacgctctctccgaaactggccccagcggaagatgttcgtggggcgctggcgctggtcgaacgtaacgaagcgcctctgggcattgtctacggttctgacgcagttgccagcaaaggggtaaaagtggttgccaccttcccggaagattcacataaaaaagtggaatatccggttgctgttgtggaagggcataacaatgcgacagtgaaagcattttatgattatctgaagggaccgcaggcagcggaaatctttaaacgttacggatttacaatcaagtaatgatactgaccgatccagaatggcaggcagttttattaagcctgaaagtttcttccctggctgtgctgtttagcctgccgtttgggatcttttttgcctggttactggtgcgttgcacgtttccgggcaaagctctgctcgacagcgtactgcatctaccgctggtgttaccgcccgtggtcgtcggttacttattattagtttcgatgggacggcgcggatttatcggtgaacgtctgtatgactggtttggtattaccttcgcctttagctggcgcggcgcggttctcgctgccgccgtcatgtcgtttccgctgatggtgcgggcaattcgtctggcgctggaaggggttgatgtcaaactggaacaggccgcaagaacactgggggccgggcgctggcgcgttttctttactatcacgttaccgctgaccttaccgggaattattgttggtacggtactggcttttgctcgttctctcggtgagtttggtgcaaccatcacctttgtgtcgaacattcctggtgaaacgcgaaccattccttctgccatgtataccctgatccagacccccggcggggaaagtggagcggcgagactgtgcattatttctattgcgctggcgatgatctccctgttgatttcagaatggctggccagaatcagccgtgaacgggcggggcgctaatcatgctggaactgaatttttcccagacgttgggcaaccattgcctgactattaatgaaacgctgcccgccaatggcatcactgctatctttggcgtctccggtgccggaaaaacttcgctgattaacgccatcagtggactgacgcgcccgcaaaaagggcggattgtcctcaatgggcgggtactaaatgatgccgaaaaaggtatctgcctgacgccggaaaagcgtcgcgttggctatgtttttcaggatgcgcggctgttcccgcattacaaagtgcgtggcaatctgcgctacggcatgtcgaaaagtatggtcgatcagttcgataagctggtggcgcttttaggcattgaaccgttgcttgaccgtttaccaggcagcctgtccggaggcgaaaaacagcgcgtggcgattggtcgggctttgctgacagcaccggaattgctgttgctggatgaaccgctggcgtcactggatattccgcgtaaacgcgaactgttgccttatctgcaacggctgacacgggaaatcaacattccgatgttgtatgtcagccattcgctggatgagatcctccatctggcagacagagtgatggtactggaaaacggtcaggtgaaagcctttggcgcgctggaggaagtgtggggcagtagcgtgatgaatccgtggctgccgaaagagcaacaaagtagcattctgaaagtgacggtgcttgagcatcatccgcattacgcgatgaccgcgctggcgctgggcgatcagcatttgtgggtcaataagctggacgaaccgctgcaagctgcgctacgtatccgcattcaggcttccgatgtttctctggttttacaaccgccgcagcaaaccagcattcgtaacgtattgcgggcaaaagttgttaatagttatgacgacaacggccaggtggaagtggaactggaagtcggcggtaaaacgctgtgggcgcgtatcagcccgtgggccagggatgaactggcgatcaaacctggcctgtggctgtacgcgcaaattaaaagtgtgtcgataaccgcctgattaaatcaggtggctataaatgaactgggcaatgctgtcggtggtgttatcaccaatcacaatgttggcgcgcgcttttaccgcgtcatcggcgttgcccatcgccacgcctgtaccagcggcttccagcatactgatatcattaaagttatcgccgaatgccacgacgttttccatcgaccaaccttgcgcctcaacccatttcgtcaaacgtttacctttgctgttgccgccgcgtgcaatatcaacctgatcgtgccaggaccattcacactccagtcccagttcatgttcgacatgcttaccaaaatgctgcaattgcggcaggtcatcgtgcgtcagggcgaacttccatacggcgttaacttgttgcgccgtttcagccagagaagcgacttgtgtgaaagtcggacgctgttccggcggcagggtttgcgcccagttagatgtgcgaatgacatgcccggtcgggtgctcatagaccattgcatcatcgacatacatcagaccgtgaatgtggtgttcattcagcatctcaatgagttgcagggctttaataacgggcattgggtccgcttccagcacggtttttgcatgataatcatacaaataggtgccattacagcaaatagcaggtgtatccagcgccagcgcctgataaaaaggatgaatagcgacgtgatggcgacctgtgacgatgattaattgatagcctgcttcgcgagcgcgggccagggcttctatcgatgaaggaagcagggtctttttcggggtcaataaggtgccgtctaagtcgagagcaatcacgcgtgtggtcatggcgtattccagattaaggttaagaattttcgtctgcgcgaatggtacaccgataccactatcggacaaaattctgcgttttaattcagcattcaccgccaaaagcgactaattttagctgttacagtcagttgctaaatgcaaaggagcattcatgaagcaaacagtttatatcgccagccctgagagccagcaaattcacgtctggaatctgaatcatgaaggcgcactgacgctgacacaggttgtcgatgtgccggggcaggtgcagccgatggtggtcagcccggacaaacgttatctctatgttggtgttcgccctgagtttcgcgtcctggcgtatcgtatcgccccggacgatggcgcactgacctttgccgcagagtctgcgctgccgggtagtccgacgcatatttccaccgatcaccaggggcagtttgtctttgtaggttcttacaatgcgggtaacgtgagcgtaacgcgtctggaagatggcctgccagtgggcgtcgtcgatgtggtcgaggggctggacggttgccattccgccaatatctcaccggacaaccgtacgctgtgggttccggcattaaagcaggatcgcatttgcctgtttacggtcagcgatgatggtcatctcgtggcgcaggaccctgcggaagtgaccaccgttgaaggggccggcccgcgtcatatggtattccatccaaacgaacaatatgcgtattgcgtcaatgagttaaacagctcagtggatgtctgggaactgaaagatccgcacggtaatatcgaatgtgtccagacgctggatatgatgccggaaaacttctccgacacccgttgggcggctgatattcatatcaccccggatggtcgccatttatacgcctgcgaccgtaccgccagcctgattaccgttttcagcgtttcggaagatggcagcgtgttgagtaaagaaggcttccagccaacggaaacccagccgcgcggcttcaatgttgatcacagcggcaagtatctgattgccgccgggcaaaaatctcaccacatctcggtatacgaaattgttggcgagcaggggctactgcatgaaaaaggccgctatgcggtcgggcagggaccaatgtgggtggtggttaacgcacactaaccgctgatttacccggcgcagtctctcctgcgccggtgtattaacctatctcctgtaacgcgtgtctctggcgttcgacgatattggtccacaaattgtctttatcgtcagtccataaattaatcagcaaggcaaaaaagcgttctgctgctggagaaagtacggcatctttacggcgaattattcccaatgttcgacgtataacgggttccaccaatgggataccaataatcgaagaatagggcgcatgaggcattgccaggccaggaagcgccgaaatccccagtcccgcctccaccagtcctaatgacgtcgaaagatgacgcacttcgtaaaaccagtccagcttccagggcttgtcggccagctgttgttctatcaacagtcggttgccgctggaggagcgtacgccaatcattttgtaacccactaactcctgccattctacaagctgctttttggccaatggatggtcacgccgacaggccagcacgaacggctcgttgaccagtggggtaaaatcaatggatgaatttgtgacgttgttcatgtttatgccaaagtctgattcgttacacagcaccgattccatgcaattattcgtgccttgttccagaatccgcactttaatattgggatacagctcattaaatttaccgattgccagcggtaaaaaataaaatactgcggtcggaatacacgctaacgtcaccataccacgatgataagcattcatatcacgaatattaaaaagcgtttcatcgaatttctttattaattcccgcgcctccgggagcaacctttttcctgcttttgttaacgtaaccttgcgagttgtacgctcaaatagttgaacatgtaaatcttcctccatcttttttattcttcgcgttaatgcaggttgcgtaatattgagtaatttagcggcattgttaaacgaactggactctgccagtatgacaaatgccttcatacttgataattcatgcttcattattactccggaaaatggaagcgacgattttgggtggctggccgttaaaaattttaactgcatttagccaacttaaattaatgaaaaaatgttattaatcgttgagctaaagtcattagagatgctttgcccttaatgtaaccatatcgcaataagttatgtttttaaattgagggcattattatgaaaaaaataccctgcgtgatgatgcgaggtggaacctcgaggggcgcgttcctgttagcggaacatttacccgaagatcaaacgcagcgcgataaaatattgatggcaattatgggttccggtaacgatctggaaattgacggtattggcggcggtaatccactgaccagtaaagtcgccattattagccgttccagcgatccgcgtgctgatgtcgattatctgtttgcgcaggtaatcgttcatgagcaacgtgtcgataccacgcctaactgcggcaatatgctgtctggtgttggggcattcgccattgaaaatggtttgattgcagcgacttcgccagttactcgcgtacgtatccgcaacgtcaatacgggtacgttcatcgaagctgatgtgcaaacgccaaatggtgttgtcgagtacgagggtagcgccagaattgacggcgtaccgggtactgccgcaccggttgcgctcactttcctgaatgccgctggaaccaaaaccggaaaagttttcccgactgataatcagattgattattttgacgatgtcccggtgacctgtatcgatatggcgatgccagtcgtcattattccggctgaatatctgggaaaaacaggttatgaattaccggcggaactggatgccgacaaagcattattagcccgcattgaatctatccgtctacaagcgggtaaagcaatgggcttaggtgatgtcagtaatatggttatccctaaacctgtgcttatttctccagcgcagaaaggcggggcaattaatgtgcgttattttatgccgcattcttgccatcgcgcgctggcgataaccggtgctattgctatttccagtagttgtgcattggaaggcaccgtcacccgacaaatcgtcccttctgtaggatacggcaatatcaatattgaacaccccagtggtgcgctcgacgttcatttaagtaatgaaggtcaggatgccacgacgttacgcgcatctgttattcggacgaccagaaaaatattttccggtgaagtttatcttccctgaaaaaattcgttgtcaggataaggacaatcaataaaggacttctgtatgagtcatacagaaagaacaggattttaaatgaataagaaatcgttatggaagctaattctgatattagcgatcccatgtattattggttttatgccagctccggcaggattaagcgaactggcgtgggtgctttttggtatttacctggcggccattgtggggctggttatcaagcctttcccggaacctgtcgtactgttaattgccgttgctgcctcaatggtggtggtcggtaacttatccgacggtgcgtttaaaaccaccgccgtattaagcggttactcttcaggtaccacctggctggtgttctcggcgtttaccttaagcgccgcatttgtgaccaccggtttaggtaaacgtattgcctatctgctgattggtaaaatcggtaacaccacgctgggtctgggttacgttacggtattcctcgatctggtactggctccggcaacaccgtctaacaccgcgcgtgcgggcggcattgtgttaccgatcatcaacagcgtggcggtggctttggggtccgaaccggaaaaaagtccgcgtcgtgtcggacattacctgatgatgtccatttacatggtcaccaaaaccaccagctatatgttctttaccgcaatggcggggaacattctggcgctgaaaatgatcaacgacattctgcacctgcaaattagctggggtggatgggcgctggcagccggattgccgggcatcattatgctgctggtcaccccgctggtgatttacaccatgtatccaccagaaattaagaaggtggataacaaaaccatcgctaaagcgggccttgccgaactaggaccgatgaaaatccgcgaaaaaatgctgctcggtgtctttgtgctggcgctgctgggctggattttcagtaagtctctgggggttgatgaatccaccgtggcaatcgttgttatggcaaccatgctgctgctgggtatcgttacctgggaagacgtggttaaaaataaaggcggctggaataccttaatctggtacggcggtattatcggcttaagctccttattatcgaaagttaaattcttcgaatggttagctgaagtctttaaaaataacctggcatttgatggtcacggtaacgttgctttcttcgttattattttcctcagcattatcgtgcgttatttcttcgcttccggtagtgcctatatcgttgctatgttaccggtatttgccatgctggcgaacgtctccggcgcaccgttaatgttaaccgcgctggcactgttgttctccaactcctatggcggcatggttactcactatggcggcgcggcaggtccggtcatctttggcgtgggttataacgatattaaatcctggtggttggtcggtgcggtactgacgatattaaccttcctggtgcatatcaccctcggcgtgtggtggtggaatatgctgatcggctggaacatgctgtaaatattctcgtcatacttcaagttgcatgtgctgcgtctgcgttcgctcaccccagtcacttacttatgtaagctcctggggattcactcgcttgtcgccttcctgcaactcgaattatttagagtatatccatttattatctttctgcgcacttcacggtgcgcagatatctggagcatttgatgatcaagttatctgaaaaaggcgtgtttctcgccagtaataacgaaataattgccgaagaacatttcaccggcgaaattaaaaaagaagaagccaaaaaaggcactattgcctggtctattctctcttcgcataatacgtccggaaatatggataaacttaaaattaagtttgattcattagcctctcacgatattacctttgttggtattgtacagaccgctaaagcgtccggtatggaacgtttcccgctgccgtatgtgctgaccaactgccataactcactctgcgccgtcggcggcactattaacggtgatgaccatgtttttggtttatcggcggcccagcgttatggcggtatttttgtgcctccgcatattgcggtcatccatcaatatatgcgtgagatgatggcaggcggcggcaaaatgatcctcgggtcagacagccacacccgttacggtgcattagggacaatggcagtcggtgagggcggcggtgagttggtaaaacagctgcttaatgacacctgggatatcgactatccgggcgtggttgcggtgcatctgaccggaaaacctgcgccgtatgtggggccacaggatgtggcgctggctatcattggcgcggtgttcaaaaacggttacgtcaaaaacaaagtcatggagttcgttggaccgggcgttagcgcgctctctaccgatttccgtaacagcgttgacgtgatgaccactgaaacgacctgtttaagttctgtctggcaaaccgatgaagaagtccataactggctggcgctgcacggtcgcggccaggattactgccagcttaaccctcaaccgatggcgtactacgatggctgcatcagcgttgatttaagcgccatcaaaccaatgattgcgctgccgttccacccgagcaacgtgtatgaaatcgacacactgaaccagaacctgaccgacattctgcgtgagattgaaattgagtccgaacgcgtggcgcacggtaaagccaaactctcgctgctggataaagtggaaaatggtcgcctgaaagtgcagcaggggattatcgcgggctgttctggcggtaactacgaaaacgtcatcgcggcggcgaatgcactgcgcggtcaatcctgtggcaatgacaccttctcgctggcagtttacccgtcatcacagccggtgtttatggatctcgccaaaaaaggtgtggtagcagatttgattggcgcaggcgcaatcatcagaaccgcgttctgcggcccatgctttggcgcgggcgatacgccaatcaacaacggtttgagtattcgccacaccacgcgtaacttcccgaaccgcgaaggctctaagccagctaatgggcagatgtcagcggtggcgttgatggacgctcgttctatcgctgcgactgcggcaaacggtggctatttaacctctgccagcgaacttgattgctgggacaacgtgccggagtacgccttcgatgtaacgccgtataaaaaccgtgtttatcagggctttgtgaaaggggcaactcagcaaccgctgatttacgggccgaacattaaagactggccggaattgggtgcgctgactgacaatatcgtcctgaaagtgtgctcgaagatcctcgacgaagtgaccaccaccgacgaactgattccttccggtgaaacctcttcttatcgttcaaatccgattggtctggcggagtttaccctgtctcgccgcgatcccggttatgttagcagaagtaaagcgactgctgagctggaaaatcagcgtctggcggggaatgtcagcgagctgacagaggtgtttgcgcgcattaagcagattgctggtcaggagcatattgatccgctgcaaactgaaattggcagcatggtctatgcggtgaaaccaggcgatggttctgcgcgtgaacaggcggcgagctgccagcgtgtgattggcggtctggcgaatattgccgaggagtacgcgactaaacgctatcgttctaacgtcatcaactgggggatgttaccgctgcaaatggcggaagtaccaacctttgaagtgggggattacatttacatccctggcattaaagcggcgctggataatccgggtacgacgtttaaaggttatgtgatccatgaagatgcgccggtaacggaaattacgctctatatggaaagtctgactgctgaagagcgcgagattatcaaggcgggtagtttgattaacttcaataaaaaccgtcagatgtaaaaagcgccatgtgaatgtaggtcgcattcggcacttattgtcggatgcgatgcttgcgcatcttatccgacctacgaatcgcatcgaatctgtaggccagataaggcattttcgcagcatccggcacttattgtcggatgcgatgcttgcgcatcttatccgacctacaaatcgcatcgaaccgtaggccggataaggcgtttacgccgcatccggcaaatagttaattgctcttacttcttcgcctctgcaaccactttactacccacgccgcggttattgtattcccacatgcggttgtagttagtgtcattcagattgcgctgtatttcgtcgttatcatctacgctgccggtattacccgcaaacggacgattagagatcaccgcatcggcccacggtttagccgtgttaaaaccttcgttgatggcgctatcacggatcaccacctgaccgttggtattggcatcaacatccagcgagcggcccagttgcgccacaccatcaccgaaagcattgaaacggctgtttacggcgaggaaaccgtagtaaatgttggacagcgtagccggtgcaaacacatacgcttcttgctgagtacgtgagttcaccacgcggaattcggtgttatcgaacaccactgcgccgcgaccagaaacgatatccacatccccttcaatgtagctgttggtcaccagcgtacgcggctgacgattcgtttccagacggttctgcacaccgctgttggtgacaaagaaggtgttctgacgaccgagaatgttaacgttgttaatctgtacctggtcaccatcagtacgcagtgccaccgccggatggttacctgcatctacgctatcgcccagcgtgttttcgatggtcagattttgcagttgcaggccattgttttgtgaccagaagaccgcagagcagagaacaccgatactgtcgctgcgtttgctctggcagctatcgtacatataccacgctggtttacctggcatatatttgccgcgcgggttgacgtcgtgacgccagtcggcagggctcatgccaccatcaagggaaagcccaatcttcacatcaatcggtttttcacctgtaccgtacagagtaattccacccggagcggcagggacatataccgttccctgatactcaccaggcatcacggcaatatactggcgcttgttggtacgcttgataattgccgcatctaccgccgcctgaatcgtggtatgcgttacaccttgagtgcccgccgggccgacaacaaagtcaggttgcgcaggcagggtaatcggggaaggattccacgctgcagcacctggtgtcagggatgcaaaatagtgttgagcatcgaaattctgcgcttcttttgccgacagaatcgggcgagaagaggtaccaggcgcggtttgatcagaaggacgttgatcgggcggggttgagctacaggcggtcagcgtcacgccaaaagccaatgccagcgccagacgggaaactgaaaatgtgttcacaggttgctccgggctatgaaatagaaaaatgaatccgttgaagcctgcttttttatactaacttgagcgaaacgggaaggtaaaaagacaaaaagttgtttttaatacctttaagtgataccagatggcattgcgccatctggcagagtgattaactaaacatcgcagtaatcgaggcgcttgccagagagtggaaatgaacgttaaacccgaccatcgcgccgctggcaccttcatcgacatcaatacgttctatatccagcgcgtgaacggtaaaaatgtagcgatgagtttcgcctttcggcggtgctgcgccatcgtacccggttttaccaaagtcggtacgcgtctgcaaaacgccgtctggcattgctaccagaccagagccaaacccttgcggtaatacgcgggtatcagcgggtaagttaacaactacccagtgccaccagccggagccggttggcgcatccgggtcgtagcaggtgacaacaaaacttttcgttcccgcaggaacatcatcccacgccagatgcggtgaaatattatcgccatcgtaacccatgccgttaaagacatgacgatgcggcaatttatcgccatcgcgcagatcgttactgatgagtttcatgaaccctcctttcttgtttgcagaaagtgtagccagaaaccctcacgcggacttctcgttattggcaaaaaaatgtttcatcctgtaccgcgcggttaaccgctgcggtcagacgctgcaactgttgcgggagaataatatagggcggcatcaggtaaatcagtttgccaaaaggccggatccagacaccctgttcgacaaagaatttttgcagcgccgccatattcaccggatgagtggtttcgaccacgccaatggcccccagtacgcgcacatcggcaaccatttcggcatcacgggcgggggcaagttgctcgcgcagctgtacttcaatatccgccacctgttgctgccagtcgccagattcgagaatcgccaggctggcgtttgctgccgcgcaggccagcggattgcccataaaagttggcccatgcataaagcaaccggcttcaccgttactgatggtttctgcaacctcgcgcgtggtgagtgtggcggaaagggtcattgtgccgccggttaaggctttaccgaggcacaaaatgtccggcgcgatttctgcatgttcacaggcaaacagtttcccggtacgaccaaatccagtggcgatctcgtcggcaatcagcaagataccttcgcgatcgcatattttgcggattcgttttaaccattccggatggtacatgcgcatcccgcctgcgccctggacaatcggctcaatgatcaccgccgcgatttcatgacgatgcgccgccatcaggcgggcaaagcccaccatatcgcgctcatcccattcgccatccatgcggctttgcggggcgggagcaaacaggttttctggcaggtagcctttccacagactgtgcattgagttatccggatcgcacaccgacatcgcgccaaaggtatcgccatgataaccattgcggaaggtcagaaaacgctggcgcgcttcgcctttggcttgccagtactgcaacgccattttcatcgccacttccaccgctacggaaccggagtccgcgagaaaaacgcactccagcggttgcggcgtcatcgccaccagtttgcggcacagctcaatggctggcgcatgggtgataccgccaaacatcacatgcgacatggcatcaatttgcgacttcatcgccgcattaagctgcgggtgattgtagccgtggatcgccgcccaccaggacgacataccgtcaaccaggcgtctgccgtcagacaaaatcagctcgcaaccttcggcgctcaccaccggataaaccggcagaggggaggtcatggatgtgtatgggtgccagatatggcgttggtcaaaggcaagatcgtccgttgtcataatcgacttgtaaaccaaattgaaaagatttaggtttacaagtctacaccgaattaacaacaaaaaacacgttttggagaagccccatggctcaccgcccacgctggacattgtcgcaagtcacagaattatttgaaaaaccgttgctggatctgctgtttgaagcgcagcaggtgcatcgccagcatttcgatcctcgtcaggtgcaggtcagcacgttgctgtcgattaagaccggagcttgtccggaagattgcaaatactgcccgcaaagctcgcgctacaaaaccgggctggaagccgagcggttgatggaagttgaacaggtgctggagtcggcgcgcaaagcgaaagcggcaggatcgacgcgcttctgtatgggcgcggcgtggaagaatccccacgaacgcgatatgccgtacctggaacaaatggtgcagggggtaaaagcgatggggctggaggcgtgtatgacgctgggcacgttgagtgaatctcaggcgcagcgcctcgcgaacgccgggctggattactacaaccacaacctggacacctcgccggagttttacggcaatatcatcaccacacgcacttatcaggaacgcctcgatacgctggaaaaagtgcgcgatgccgggatcaaagtctgttctggcggcattgtgggcttaggcgaaacggtaaaagatcgcgccggattattgctgcaactggcaaacctgccgacgccgccggaaagcgtgccaatcaacatgctggtgaaggtgaaaggcacgccgcttgccgataacgatgatgtcgatgcctttgattttattcgcaccattgcggtcgcgcggatcatgatgccaacctcttacgtgcgcctttctgccggacgcgagcagatgaacgaacagactcaggcgatgtgctttatggcaggcgcaaactcgattttctacggttgcaaactgctgaccacgccgaatccggaagaagataaagacctgcaactgttccgcaaactggggctaaatccgcagcaaactgccgtgctggcaggggataacgaacaacagcaacgtcttgaacaggcgctgatgaccccggacaccgacgaatattacaacgcggcagcattatgagctggcaggagaaaatcaacgcggcgctcgatgcgcggcgtgctgccgatgccctgcgtcgccgttatccggtggcgcaaggagccggacgctggctggtggcggatgatcgccagtatctgaacttttccagtaacgattatttaggtttaagccatcatccgcaaattatccgtgcctggcagcagggggcggagcaatttggcatcggtagcggcggctccggtcacgtcagcggttatagcgtggtgcatcaggcactggaagaagagctggccgagtggcttggctattcgcgggcactgctgtttatctctggtttcgccgctaatcaggcagttattgccgcgatgatggcgaaagaggaccgtattgctgccgaccggcttagccatgcctcattgctggaagctgccagtttaagcccgtcgcagcttcgccgttttgctcataacgatgtcactcatttggcgcgattgcttgcttccccctgtccggggcagcaaatggtggtgacagaaggcgtgttcagcatggacggcgatagtgcgccactggcggaaatccagcaggtaacgcaacagcacaatggctggttgatggtcgatgatgcccacggcacgggcgttatcggggagcaggggcgcggcagctgctggctgcaaaaggtaaaaccagaattgctggtagtgacttttggcaaaggatttggcgtcagcggggcagcggtgctttgctccagtacggtggcggattatctgctgcaattcgcccgccaccttatctacagcaccagtatgccgcccgctcaggcgcaggcattacgtgcgtcgctggcggtcattcgcagtgatgagggtgatgcacggcgcgaaaaactggcggcactcattacgcgttttcgtgccggagtacaggatttgccgtttacgcttgctgattcatgcagcgccatccagccattgattgtcggtgataacagccgtgcgttacaactggcagaaaaactgcgtcagcaaggctgctgggtcacggcgattcgcccgccaaccgtacccgctggtactgcgcgactgcgcttaacgctaaccgctgcgcatgaaatgcaggatatcgaccgtctgctggaggtgctgcatggcaacggttaataaacaagccattgcagcggcatttggtcgggcagccgcacactatgagcaacatgcagatctacagcgccagagtgctgacgccttactggcaatgcttccacagcgtaaatacacccacgtactggacgcgggttgtggacctggctggatgagccgccactggcgggaacgtcacgcgcaggtgacggccttagatctctcgccgccaatgcttgttcaggcacgccagaaggatgccgcagaccattatctggcgggagatatcgaatccctgccgttagcgactgcgacgttcgatcttgcatggagcaatctcgcagtgcagtggtgcggtaatttatccacggcactccgcgagctgtatcgggtggtgcgccccaaaggcgtggtcgcgtttaccacgctggtgcagggatcgttacccgaactgcatcaggcgtggcaggcggtggacgagcgtccgcatgctaatcgctttttaccgccagatgaaatcgaacagtcgctgaacggcgtgcattatcaacatcatattcagcccatcacgctgtggtttgatgatgcgctcagtgccatgcgttcgctgaaaggcatcggtgccacgcatcttcatgaagggcgcgacccgcgaatattaacgcgttcgcagttgcagcgattgcaactggcctggccgcaacagcaggggcgatatcctctgacgtatcatctttttttgggagtgattgctcgtgagtaaacgttattttgtcaccggaacggataccgaagtggggaaaactgtcgccagttgtgcacttttacaagccgcaaaggcagcaggctaccggacggcaggttataaaccggtcgcctctggcagcgaaaagaccccggaaggtttacgcaatagcgacgcgctggcgttacagcgcaacagcagcctgcagctggattacgcaacagtaaatccttacaccttcgcagaacccacttcgccgcacatcatcagcgcgcaagagggcagaccgatagaatcattggtaatgagcgccggattacgcgcgcttgaacaacaggctgactgggtgttagtggaaggtgctggcggctggtttacgccgctttctgacactttcacttttgcagattgggtaacacaggaacaactgccggtgatactggtagttggtgtgaaactcggctgtattaatcacgcgatgttgactgcacaggtaatacaacacgccggactgactctggcgggttgggtggcgaacgatgttacgcctccgggaaaacgtcacgctgaatatatgaccacgctcacccgcatgattcccgcgccgctgctgggagagatcccctggcttgcagaaaatccagaaaatgcggcaaccggaaagtacataaaccttgccttgttgtagccattctgtatttggttaaattgcgagcgagatcgcgtcttcgattgactgcaatttaaccaattaaattctaaaataatcacgaaaaaaattttacttccgcctcatgcggcgaatgtgggaattgcccaggcggcgggggataggggctggagacagttatccactattcctgtggataaccatgtgtattagagttagaaaacacgaggcaagcgagagaatacgcggcttgcacgcgaattggcgttaaagacggctcaaagaaatatcttttattttttaactggttagataaatgcaatggcagtcactgaacaggcatctcttgccataaaactgtcatcactcatcttgacaaatgttaaaaaagccgttgctttggggataacccggtaaggccggagttttatctcgccacagagtaaattttgctcatgattgacagcggagtttacgctgtatcagaaatattatggtgatgaactgtttttttatccagtataatttgttggcataattaagtacgacgagtaaaattacatacctgcccgcccaactccttcaggtagcgactcatgagtaaaccgttcaaactgaattccgcttttaaaccttctggcgatcagccagaggcgattcgacgtctcgaagaggggctggaagatggcctggcgcaccagacgttacttggcgtgactggctcagggaaaaccttcaccattgccaatgtcattgctgaccttcagcgcccaaccatggtacttgcgcccaacaaaacgctggcggcccagctgtatggcgaaatgaaagagttcttcccggaaaacgcggtggaatatttcgtttcctactacgactactatcagccggaagcctatgtaccgagttccgacactttcattgagaaagatgcctcggttaacgaacatattgagcagatgcgtttgtccgccaccaaagcgatgctggagcggcgtgatgtggttgtggtggcgtctgtttccgcgatttatggtctgggcgatcctgatttatatctcaagatgatgctccatctcacggtcggtatgattatcgatcagcgcgcgattctgcgccgactggcggagctgcaatacgctcgtaatgatcaagcattccagcgtggtactttccgcgttcgtggcgaggtgatagatatcttcccggcagaatcggatgacattgcacttcgcgtggaactgtttgacgaggaagtggaacgattgtcgttatttgacccgctgaccgggcagattgtttccactattccacgttttaccatctacccgaaaacgcactacgtcacaccgcgcgagcgcatcgtacaggcgatggaggagatcaaagaagagctggccgccagacgcaaagtgctgttggaaaacaacaaactgctggaagagcagcggctgacccagcgtacccagtttgatctggagatgatgaacgagctgggctactgttcggggattgaaaactactcgcgcttcctctccggtcgtggaccgggtgagccaccgccgacgctgtttgattacctgcctgccgatgggctgctggtcgtcgatgaatctcacgtcaccattccacaaattggcggcatgtatcgcggtgaccgggcgcgtaaagagacactggtggagtacggcttccgcctgccatcagcgctggataaccgtccgcttaagtttgaagagttcgaagcattagcgccgcaaaccatctatgtttcggcgacgccgggtaattacgagctggaaaaatccggcggcgatgtggtggatcaggtggtgcgtccaaccggattgcttgacccgattatcgaagtgcggccggtggcgacacaggttgatgatcttctttcggagattcgtcagcgagcggcaattaacgaacgcgtactggtcaccacactgaccaagcggatggcggaagatcttaccgaatatctcgaagaacatggcgagcgcgtgcgttatcttcactcagatatcgacaccgtcgaacgtatggagattatccgcgacttgcgtctgggtgagttcgacgtgctggtagggatcaacttactgcgcgaaggtctggatatgccggaagtgtcgctggtggcgatcctcgacgctgacaaagaaggcttcctgcgttccgaacgttcgttgatccagaccattggtcgtgcggcacgtaacgttaacggtaaagcgattctctacggcgataagatcaccccatcaatggcgaaagcgattggcgaaaccgaacgtcgccgtgagaaacagcagaagtacaacgaggaacacggaattacgccgcaaggcttgaacaagaaagtggtcgatatcctggcgctggggcagaacattgccaaaaccaaagcgaagggcagaggaaaatcgcgcccgattgttgagccggataatgtgccgatggatatgtcgcctaaagcgttgcagcagaaaatccatgagctggaagggttgatgatgcaacacgcgcagaatctggagttcgaagaagcggcgcaaattcgtgaccagttgcatcagctgcgtgagctgtttatcgcggcatcgtaacaggatagcgaagaagactgatgacaaacggaaaacagcctgatgcgctacgcttatcaggcctacattttctccgcaatatattgaatttgcgcggtttgtaggccggataaggcgttcacgccgcatccggcataaacaacgcgcactttgtcttcaataggaagccggaattttccttcggatttccgttaacctaaagcctgtaacgccttttccagcgcgttatgtaacaactggcggtcatgacgatacggaatatcgctggcctccagtacctcctggatcacaatccgctctttcaccgccgagacatccacttttggcccgacgatgaccgcatcaatgacctttttaccaacatactgctccataattgccagcttgctttccagcttcaaattagccgcaggtaaactcaactcacgccccagattgccgatataaaccatcggcgctggcgtgcggcgtaatgcctgggcgatttccttcagcagcagaattggcatcaggctggtataaaaactgccaggcccaataatgatgagatccgcttcattgatagcgtgaaccgcctcacgcgttgcgggtacattaggcgttaacaataactcttgaatcggcgtagttaactggtcgatattgacctcgccgtaaacttcatgcccctgatcgtcaatcgccatcagatcaacaggatgctctgacattggaatcaaatgcgtatccactttcagcagattacgaattaaattgatggcttccagaggccgcacgctaaggtgatccagcgcctttaacatcaagtttccgagattatgaccggaaagttcgccattgccaccaaaacggtattcaaacatcgcggaggcgacgctcggttccgttatcagctggttgaggcagttgcgcatatcgccccaggcaatgccgccttctgaacggcgaatacgccccgtcgagccaccattatcggtggtggtgacgatacccgttaaacgagaacccaaagacgaaagtgatgagagaacgcgtcccagtccatgccctccgccgagagcaacgacacgatcaagatcagccagcgtacgattgcgcatatagtttcctggagtcagattatccgcgctacagtagcgcaaattgcggggaaacagcaattaacctgccaatattgaggatacaaactattttcttctacctctaaaggacgatgcacgctatgcctccctgatgatgtatatcaaagtaaaaccgccattttcccttattctgtagcgaaatagcacgatcatgacgctatatacatgattacatagcgaaagtgtggatggtaaaaatctcatttacacgctagtatcggcataaccactaaacactctagcctctgcacctgggtcaactgatacggtgctttggccgtgacaatgctcgtaaagattgccaccagggcgaaggaagaaatgacttcgcctcccgtatctggaaaggtgtacatggcttcacaactgactgatgcatttgcgcgtaagttttactacttgcgcctgtcgattaccgatgtgtgtaactttcgttgcacctactgcctgccggatggctacaaaccgagcggcgtcaccaataaaggctttcttaccgtcgatgaaattcgccgggttacgcgcgccttcgccagactgggcaccgaaaaagtgcgcctgacaggaggagagccgtctttacgccgcgactttaccgatatcatcgccgctgtgcgggaaaacgacgctatccgccagattgcggtcacaaccaatggttaccgtctggaacgcgatgtggcgagctggcgcgatgcgggacttactggcattaacgtcagtgtcgacagtctggacgcccgccagtttcacgctattaccgggcaggataaattcaaccaggtcatggcagggattgatgctgcatttgaggccggttttgagaaggtcaaagtcaataccgtgctgatgcgtgatgttaatcatcaccagctcgacacctttctgaactggatccagcatcgccctatccagctgcgtttcatcgaactgatggaaacgggcgagggcagcgagctcttccgtaagcatcacatctctggtcaggttctgcgtgacgagctactgcgtcgcggctggatccaccaattacgtcaacgcagcgacggtcccgcgcaagtcttttgccatccagattacgccggagagattggccttatcatgccgtatgaaaaagacttctgcgccacttgcaaccgcctgcgcgtttcctccattggtaaactccatctctgcctgtttggtgaaggcggcgttaacctgcgcgatctgctggaagacgatacccagcaacaggcgctggaagcgcgtatttcagcggcgctgcgggagaagaaacagacccatttcctgcatcaaaacaacaccggtattacgcaaaacttatcgtacattggcggctaaaacgtcaaaaggagagatcagatgagtcaggtaagcactgaatttatcccgacccgtattgctattcttacggtttctaatcgtcgcggtgaagaagacgatacctccggtcactatctgcgcgattcggcgcaagaagcgggccatcacgttgtcgataaagccattgtgaaagaaaaccgctacgctattcgcgctcaggtatctgcgtggatcgccagcgacgatgtacaagtggtattgattacgggtggtactggcctgacggaaggtgatcaggctcccgaagcattgctgccgttgttcgaccgtgaagttgaaggttttggtgaagtgttccggatgttgtcgtttgaagagattggcacttccacgttgcaatctcgtgcggtagcgggcgtcgccaacaaaacgctgattttcgccatgccgggttcgaccaaagcgtgccgtaccgcatgggaaaatatcatcgcgccgcagctggatgcccgtacgcgtccgtgtaatttccatccacatttgaagaaataagtatgtcgcaactgacccatatcaacgccgctggcgaagcgcacatggtggatgtctccgccaaagcggaaaccgtgcgtgaagcgcgggcggaagcctttgtcaccatgcgcagcgagacgctggcgatgattattgatggtcgccaccacaaaggcgacgtatttgccactgcgcgtattgccggtattcaggcggcaaaacgcacctgggatctgatcccgctctgtcatccgctgatgctcagcaaagttgaagtcaatttacaggccgagccggagcacaatcgggtgcgtatagaaaccttatgccgcctgaccgggaaaaccggtgtcgaaatggaagcattaaccgcggcctccgtggcggcgctgaccatttatgacatgtgcaaagcggtgcaaaaagatatggtgattggtccggtacgtttgctggcgaagagcggcggcaagtcgggtgactttaaggtggaagcggatgattaaagttctttttttcgcccaggtgcgcgagttggtgggaacagatgcaaccgaagtggctgcggatttcccaactgttgaagcgttacgccagcacatggctgcgcagagcgatcgctgggcgctggcgctggaagatggcaaattactggctgccgtcaaccagacgctggtgagttttgaccatccgctgactgacggcgacgaagtagctttcttcccgccggtaaccggaggttaagatggcagaaaccaaaattgttgttggtccgcagccgttcagcgtaggagaagagtacccgtggctggcggagcgtgacgaagacggtgcggtagtcacctttactggtaaggtgcgcaaccataacctgggcgacagcgtcaacgcattaaccctcgaacactatccggggatgactgaaaaagcactggcagaaattgttgatgaagcgcgtaaccgctggccgctggggcgcgtcactgtgattcaccgcatcggggaattatggccgggcgatgaaatcgtttttgtcggtgtcaccagtgcgcatcgcagcagtgcgtttgaagccgggcagtttattatggattatctcaaaacccgcgcaccgttctggaagcgcgaagccacgccggaaggcgaccgctgggttgaagctcgggagagcgatcagcaggcggcaaaacgctggtagttttttgttagccggataaggcaccgctgcgtccggcaatttcaccgctcagtacatacgtttacgctgcgtcgatgcacagcctcatcattttgcagtatccttaagatattccttatatcttcaggagatcgtcatggacagattcccacgttctgattcaatcgtacaaccccgggctggcttgcaaacttatatggctcaagtctatggctggatgaccgttggcttgttgctgaccgcatttgttgcctggtatgcggctaattccgcggccgtgatggagctgttgttcactaaccgtgtctttttaatcggtctgatcatcgcgcaattagcattggttattgtgttatcagcgatgattcaaaagctgagcgcaggtgtaacgacgatgctctttatgctttattcggcgctgacgggtcttacgctttccagtatattcattgtctataccgctgcttctatcgccagtactttcgtcgttactgccgggatgttcggcgcaatgagcctgtacggttacaccacgaagcgcgatttaagtggctttggcaatatgctgtttatggcgttaatcggcattgtgctggcatcgctggtcaacttctggttgaaaagcgaagcattgatgtgggcagttacctacatcggcgtgattgtctttgtcggattgacggcgtatgacacgcagaaactgaaaaatatgggtgagcagattgatacccgcgacacgtcgaacctgcgcaaatattccattcttggcgcgttaaccttgtatctggacttcatcaacctgttcctgatgttgttgcggatcttcggcaaccgccgttaattctttttcaccatcactatcccggccatgtgtcgggatttttttcttactaaaaacgacacttaacaagtaccaggtataaaatatgccttatggacgagcggaagcgttttctgtatccataaatgcaaaagtattttgtatgcgtggttttaaatttattgatggtgaatattaatattttttctaaggataactaaaagaatggaatcatactcgcaaaacagcaataaattagattttcagcacgaggccaggatattaaacggtatatggctcattaccgctttaggtttggtggcaaccgcaggactagcctggggagctaagtatatcgaaattacggcaaccaaatatgattcaccaccaatgtatgtcgccatagggttattattactttgtatgtatggcttaagtaaggatatcaacaagataaatgccgccatcgcgggcgtaatatatctgtttttactctctttggtggcgattgtcgttgcaagtttagttcctgtatatgccattatcatcgtgttcagcactgcgggcgcgatgtttttaatcagtatgctggccggtttattatttaatgttgatcctggttctcaccgttttatcattatgatgacgttgacagggttggccctggtaatcatcgtgaatgcggcattaatgagtgaacggcccatttggataataagttgcttaatgattgtgttatggtcaggcattatctcgcatggacgaaataagctccttgaattggcggggaaatgccatagtgaagagttgtggagtccggttcgttgcgcttttacaggtgcattaacactctattactattttatcggcttctttgggatacttgccgcgatagctataacgcttgtctggcaaaggcatacgcgtttttttcattagccgtaaatgcacatactaaagaacttaactaaacttcacatcgccgcttcatttttcgcccgtagcttcttcgcctggctttccagcaacaggtaacagatcagcgccagcagcagtgggataaagtaatacagcacacggtaagcgagtagggcggcgataattgtacctttggaggtatgctccccagccagtagtgcgataaacaccgcttccagcacaccgatccccgccggaatatgcacgatgacgccagcaatactactaaccagtaacacgcccagtacaaagaaatagttcacgctttgaccaagtaacagccagataatcgcccccattaccatccagttaacgctggaaatcagcatctgagcgagggcgaatttccatgaaggcagcaccagcttttgccctttgatggtcatatggcggtgcttcgcgaaagcgcaaaaccacaaataaaccgcgataatcatcagtaagccaatgccgagaatacgcagcgtagtttgatcgacataccagtgatccggcaactccaccacgcctgcggtaaagataatccctgccagtaaaatgtagcccagccagttggtggtaatactgagcgagaaaatccgcgtaatagtgctaccgggcaaccccagacgagagtacaaacgatagcgcataccaatgccgccgacccaggtactgagcgtcaggttgaaggcgtagcagataaacgacaccagcatcacctggcgcttcgccagtttgtgaccgcagtaaaagcgggcgagcaggtcatagcagccgtaaatcagatagctgacgaccaccagcccgaccgcactaagcagcgcaacgcgattgtagtcgcggatgaccttccagacctcttcccagtccacttttttggcgtagaccaccagcaacacaatcaccgcgataaaaaacagccaggtgaggatcttctttgctaagcgccagcgcgggtgtgatttactcatcagggttttacccccgtgttttcagtttctacccgatcctgcgtttccattgtcggttgtgcgggcggatcaacctgcgccagacgtggcgtgtgtgccggaagccagccaaccagcgccgggaagtggcgtaaaaagtggaacgccagcacgcttttggtcaggttccaccaggtgcgtttgggcagcatggtttcatccacctgctgacaatctgcggcaataatgccgttcagattatcgcgcagcgtctggttaaaatgacgatcgtggatgatgacatttgcttcgagattcagtgacaaactgagcggatcgagattactggaccctactgtcgcccagtgatcgtccatcaatgccactttgccgtggagcgggcggcggcggtactcaaaaacctgaacgccgcctttaaccagatagttatacagcaagcgcgcaccgactctgacaatcggcatatccggttcgccctgaatgatcagtttgatccgcaccccgcgccgtgccgctttacgcaaggcgtgtaaaaatcgatagccggggaagaagtaggcgttggcgataatcacttcccgccgcgcctgagtgagcattttcaaataatggcgttcaatatcatcgcgatgttcttcgttatcgcgccagaccagcaatacctgcgcttctcccggctggcggttctcttccgctttgtgatgacgtcgccaccagcgtcgtgccgcgctctgtccaggcaggttttccagctcaaactggagaatatcttcgacaatcggcccttcaaggcgtaccgcgtaatcctgtttagcctctggaccgtagctggacatatgctcggcggagtaattcagcccgccaataaaggctatacgcgcgtcgatcaccacaattttgcgatgcatccggcgaaacacattggtgcgcataccaaaaaggcgagggcggggatcgtagtagcggaacactacgccagctgccgtcagttcattgacaaactcatcgctgagatccggcgaaccgtagccatccagcaagacttccgctttaaccccgcgttgcgctgctgccagtagtgccgcatgcagttgtttgccgacgtcatcctcaaaccagataaacgtttcaagaatgatgcgttcttgtgcctcgccaatcgccttaaacaccgcgggataatattgctcgccgttttccagcaactggatcttattgccttcgcgccagctacatttcataaatgaatctccgcacttaaaggggcatgatcagaaaggtgtcgccatgtccgcagcggcaacgcggttggcgcgctggcgctggcatttttgacgtagatcctgtccagtcgtagtagaggaaattgcaccggaaacgtgcgcgccgggcgtccgtgggcgcgggtaaaaatctcatccagtccggcctgcacttttaacggatgattagctttttgccgccagtcattgaaatcacccgccaccaataccggttcgccgtccggtagctcattcacccattcggcgagcatcgcaagctgcgcctgacggtgcgcctcacgcaggcccagatgtacgcacatcacatgaatcgcttttccggtcatcggcggcacaatgcggcagtagagcacgccgcgcttttccgcaccatcgaccgaaacatcgcgattctcataatgttcaatgggataacgcgacagtacggcgttgccgtgatgcccttccgggtatacggcattgcgaccgtaggcaaaatcgctccacatagtgtcggcgagaaactcgtagtgcgaggtatcgggccagttttccacatgcagcggatgaacttcgtgcgcgcccatcacttcctgcaggcaaacaatatcggcgctgacggtacgcacggcgtcgcgaagttccggcaaaatgaagcgtcggttaaacgcggtaaagcctttgtgaatattgatggtgagcaccttgaacgaaaattgttgtgtttgatcgggcataattttcctgtctttgcctcttatctcattgaaatagtgtagtcggcgtcacaaaaaggtgcggtcttacggaattttccgtaaagttcggtactctgagtaagtagagataaattcttcaggagagaagccatgaagtggcaacaacgtgttcgtgtcgcaacgggtctaagttgctggcagattatgttgcatttactggtagtggcgctgctggtggtgggctggatgagtaagactctggttcacgtcggcgtgggattatgcgcactgtattgtgtcacggtagtgatgatgctggtgtttcagcgccaccccgagcaacgctggcgtgaggtggcagacgtgctggaagagctgaccacgacctggtattttggcgcagcgctgattgtgctgtggctgttgtcccgcgttctggaaaacaactttttgctggcaattgcagggctggcaatccttgccggcccggcggtagtgtctttgctggcgaaagataagaagttacatcaccttacgtctaaacatcgcgtacgccgctgaccctgtcgtggccgttatcaccagtagcggccacaaactattccacacaatatccagactcgcatccttcaaataaatctgcttggtaatgtccgtaaagtggcgaatagggttaatccacgtcaggttttgcagccataccggcatgttttccaccggagaaacgtaaccggaaaggagaatggcgggcatcataaagacaaacacgccgataaacgcctgctgttgtgttgaacagagtgatgaaatcaacagaccgaatcccaccagcgataaaccataaatcaccatcgtaaagtagaacagcgccagcgatccggcgaaggggatttgatacgcccagataccaatcgccagcacaatggtggcctggaaggtggcgacaattaacgccggtacggctttgccgatgaagatctgccaggtggtgagcggcgaaaccagtagctgatcgagcgtaccttgttcacgttcgcgggcgacggaaagtgaagtgacgatcattacgccgatagtggtgatcatggcgatcagtgacggcaccacaaaccatttgtagtcgagattcgggttataccagttgcgtaccaccagctcgctgttgttaggtttcggttttccttccagcagctcctgctgataatttttgacgatctgttgcaggtagttggcggcaatttgcgcactgttggagttacgcccgtcgaggatcaactgcaaaggcgcggtctggaaggtatccagtttgcgcgagaagtcagccgggaaacgcaccagtagtaacgccttttgtgtgtcgatggttgggcggatctcctgtgggcttttcagcagcagcacatgagtaaaggcgctggcgcgggcaaaacgttgggtcagctccaccgaatgctcgccgttatcttcatcgtagatggcgatggtggcgttagtcacttccagcgtggcggcgaacgggaacaggatcacctgaattagcacgggtaaaatcagaatcgcgcgggtttgcggttcgcgcagcaacgactgcaactctttgcggattaacgtccataagcgatgaaacatgctcttctccctaatccagccgacgtttggttttcagccacgtcaggccgataaacatcaccgccgaagcgatcaaaaacagcacgtttaccaccagcaccactggaatattcccggcgaggaacaggctttgcagggtgctgacgaaataacgagcgggaataatgtacgtcaccgcgcggatcaccgcgggcatactgtcgatctgaaaaataaagccggaaagcataatcgacggcagaaaagcggcgttcagggcgacctgagcggcattgaactggttgcgggtaatcgtggaaatcagcagccccatccccagggtactgagtaaaaacaggctggagataaaaaacagaatcagcagcgacccgcgatacggcacgccgagaataaacactgacaccagcatacacagcaacatcgccagcatcccgagaaagtaataagggatcagcttacacagcagcagttccgtgcgggtaatctccgtagagagcagagcctccatggtgccgcgttcccattctcgcgccaccaccagcgaggtgagaatcgcgccgatgaccgtcatgataatggtcaccgcaccggggataatgaagtgctggctaatcgccgccgggttaaaccagtagcgggtttgtacatcaataagcggttcaaaagtctgcccgttgtcctccgctcgctgcatttgccagatctgccagatcccttcgacatacccctgtacaaagttagcggtattcggctcactgccgtcggtgatcacctgaatcggtgcggtggcgttggcgcgctccatctgttccgcaaaatccaccggaataaccaccagaccgcgaattttccccgcctgcattttggcgatcagttcctgacggttatcgctgatggtggcgtcgatgtagggcgaaccggtcatggtgtgggtgaaatccagcgccgcttcgctacgctgttccagtaaaatcccgacccgcagcttgctggagtcgaggttaatgccgtaaccaaaaataaacagcagtagcagcgggatcactaccgcaatcagccagctactcggatcgcgaacgatctgccgcgtctctttaacgcacagcgcccgtacgcgacgccaggacaggatcgggttactcattgctatgctccttatcccagtcgtggatcaactgaataaaggcttgctccatggtgggatcgggttgctcatcgttagccgactgtgctttcaaatcgtccggcgtgccgctggcgattaatttcccgcggtacaccaggccgatgcggtcgcaatattccgcttcatccataaagtgggtggtgaccatcaccgtgacgcctttctctaccatgctgttgatgtgcagccaaaattcacggcgggtgagggggtcaacgccggaagtcggttcgtcgagaaacagaatgtccggttcatgcatcagcgaacaggccagcgccagccgctgtttaaaacctaatggcagttcatcggtggcgtgggaggcgatacttttcaggccgaacgcctcgctcatgcgggagattttttcgttctgcgcccgaccgcgtaagccatacacaccagagaaaaagcgtaaattctgttcgaccgtcaggttaccgtagagcgaaaatttttgcgccatatagccgagatgctggcgcgctttaccggaactctctttcagatccatccccagcaccagcgcctggccggaagtcggcaccagcaaaccgcacatcatcttaaaggtggtcgatttacccgcgccgtttggccccagcaaaccaaaaatctccccacgtttaacggcaaagttgacgtgatcggtggcggcaaaatccccaaatttcttggtcagttctttcgcttcgatcaccgtctcgccgggtgtgccttctaccgtatgtaatattgcgcccagcggcgattccgaggttccggcaccgcccagcaaatcaataaacgcatcttcaaaacgcggcgtagtttcgttgatgttgatttccggcatcccgtcggcatggcgaatatcgtctggtgtggcctcttttttgaggatcagacgtaccgatttcccctgaatcatgccgtcgctgacctgcggcagtttcaaggcgcgttgcaacagtttgcggttgccctcgtgtggactggtcatcagaaagctgcgtccggccatggtttgtgtcagggcttttggttctccctgatacagcaactcgccttcgttcatcagtaacacgtcacggcactgctcggcttcgtcgagatacgaggtactccagaggattaacatcccttcgcccgccagctcatgcaccatctgccacagttcgcgccgtgagatagggtcaacgccgacgccgggttcatcgagcagcaacactttcggttcgcccaccagggtacaggccagaccgagtttttgtttcatcccaccggagagcttgcccgccaggcgtccggtaaacggcccaagagacgtaaactccagcaggcgagcaaaagtttgcttacgtgcctcgccggtgacgctgcgcaaatccgcgtacagattgaggttctccatcaccgtgagatcttcatacagaccaaatttctgcggcatataaccgagcacggcgtgcagcgcgccgtcgtttttgatcggatcaaagccaatcaccgtggcactgccgctgtcgggtttcagtaatcccgccaacatccgcatcagcgtggttttacctgcaccgtccggccccaccaaccccgtcacataaccggcgtgaatggtacaatcgagcggcgcgacggcgggcttgtccatgcccggaaagcgtttttccaggccgttcagcgtgataacggcatcattcatgtcctgcctcgtcaccgaattgtaccgtcactggcattccctggcgtaacgcatcatcggcgtcggtcaccacaatacgcaggcgatagacgaggtcggtacgcagatccggcgtttcgacggttttcggggtaaattcagcagtcggcgaaacgaaaccaatctgcccgtgatacggcttgtccgggcgaccatcggtataaagcagcactttgcgccccggctgggcctggtcaagattacgttcatcaacataagcgcgcacccacaccggacgcgttagtgaaacggtaaacaccgtgccaccttcattgaggaccgtgcctggctccaccgcgcgcgttaacagcgtgccatcagacggggctatcaacgttgagtcctgtaaattcaactccgcctgcgccagttgcgcctgcgcctgttcgaggctggctttcgcctgagcgatgtcctgttcacggttaccggaacggtactgacgcaatttatcctgtgctgatttcagcgttgcctgcgcctggtcgcgcgaggagcgggcattttccaggtcatttgccgaaatagtgcggcttttccacaacccttgctggcggttatagaagttctgcgcatagtcataggcggcttgcgcctgtttcaccgctgcggcggcctgagcgatttcttcattgcgatacccggcaagcatcaggtcatactgcgcctgtgccaccgaaacacccgctttcgcctgcatcagggcaatctcatacggcttgtgatccagttcgcccagcacctggcccgctttgatagcatcaccttcgtccaccgccagcgattcaacgcgccccccaacacggaaactaagatttaccgtacgaatatccacgttgccatacagcgtcaggccgttatcctggcggctttgataccaccagtagcctccggcaaccacggcggcaagtaccactaccgccaatccgatcacgacaggttttttcatcactacaaactcctttgcgataatccttgcaaaatcaggtcgatatgacaggtcaccgtctggttgatcagttcggtcttttcttcatcgaacgcggtccagccggtacgtaacagaattgtttctttgccaagacggaacgccagaatctcaccaatcaacgcatgggtatgaaggatcatgcgggtgtcattggcgtcgcagccggtccaggcggcaatcaggcgtgtcaggtggctgtgtagcggactaatcacctgttcgtgcaccaggtggtaggctgccgtgggagagagctgctcacgggagataaacttgctgaggttgacggtgtcatcctgggtgagcagcttaatcatgttcctgcaggcgcgaaggatcagttcacggatggcagcccgatcaggctgtggttgcgcgaacaagcgttcggcttcctcggcatgcggacggaactgctcgccaataaaatcggcaatccactgggcgcaggcgaggtacaaatcttctttcgaaccgaagtagtaggtgatggcagcgatattctgcccggcctgggcggctatctcgcgagtggtggcgttcattccatattcaccaaactgcgccagtgcggcagcaatcagctgttttttcgcctgttcacccttgattgtcatggcaggattattcatcgcacagtccattcttaatcaaatgattgattaagattatgactccataggggagttgtccagtatggctaagaattttagcaacgccagtcacagggataatttatgcgctgcgtcacaaaaactgctacactccgctccctcatgacattgtggtttttgtcattttccttttcagtatctccctgaaaactacaccggtaacggtcggggcggttcggagtagttatgtctttcgattctttgggtttaagccctgatatcctgcgcgccgttgccgagcagggttaccgtgaacccacccctattcagcagcaggcgatccctgcggtgctggaaggccgcgacctgatggctagcgcccagaccggcaccggcaaaacagcgggctttacgctgccgctgttgcaacacctgatcactcgccagccgcacgccaaagggcgtcgtccggtacgtgcgctcattcttaccccgacccgtgaactggcggcgcagattggcgaaaacgtccgtgattacagcaaatacctgaacattcgttcgctggtggtgtttggtggtgtgagtattaacccgcagatgatgaaactgcgtggcggcgttgatgtgctggtggcaaccccgggacgtttgctggacctggaacatcagaatgcagtgaagctggatcaggttgaaatcctcgtcctcgatgaagctgaccgcatgctcgacatgggctttatccacgatatccgtcgcgtgttaacaaaactacctgcgaagcgccagaacctgttattctccgcgaccttctctgacgatattaaagccctggcggaaaaactgttgcacaacccgctggaaatcgaagtggcacgccgcaataccgcgtctgatcaggtgacccagcacgttcactttgtcgataagaaacgcaaacgcgaattgctgtcgcacatgattgggaaagggaactggcagcaggtgctggtgtttacccgtaccaaacacggcgctaaccatctggctgaacagctcaataaagatggcatccgtagtgcggcgatccacggcaataaatcgcaaggtgcgcgtactcgtgcgctggctgattttaaatcgggcgatattcgtgtactggtggcaactgacatcgctgcgcgcggcctggatattgaagagctgccgcacgtcgtcaactatgaactgccaaacgtacctgaagattatgtccaccgtatcgggcgtaccggtcgtgcggctgctaccggtgaagcgttgtcgctggtgtgtgttgatgaacacaaactgctgcgtgatatcgaaaaactgctgaaaaaagagatcccgcgcattgcgattccgggctatgagccggacccgtcaatcaaagccgaaccgatccagaacggtcgccagcaacgtggcggcggcggtcgtgggcaaggtggtggtcgcggtcaacagcaaccacgccgtggggaaggtggcgcaaaatctgcaagcgcgaaacctgcagaaaaaccgtctcgccgcctcggcgatgccaaaccggcaggcgaacaacaacgtcgccgccgtccgcgtaaacctgccgctgcgcagtaatcttttatgccgggctatgcccggcatcaggctgatgaacaaacgcaaaactgcctgatgcgctacgcttatcaggcctacgtgaactctgcaatatattgaatttgcatgcttttgtaggccggataaggcgtttacgccgcatccggcatttcacaacaagcacttgtcagcaatttgagaacacgggaaaaaatttatctgttttaccgcccataagccaccgagacgttacttctctatagccaattgttcgcgcaactccattaaaaggtagcccagtcgattcttgcccttaccatgaccaccgtctccccagtaagcatcgttttccgtatgctcaaccagttttgcgggcgcggttgccagcaagagcgcacgcagttctgcatgctgttcgaatttagcgcgaagtgcttttcgcatcacctgttctttgaccgactcccagtttttacgcagaggcttagaacgatcgcgccccatgcgtgcggcgaccataggggaagaaacccgacggatctcttcgcggtatttttcatcaaggaatttttgtgcctgaaaatagtgttctgaggtaggccaggttttcccgtcaaccttgatgggccaggcggcaaagttagaaaaatcaccgtagtcatcgctggtgctgtagaaatttatgatggtgtcttgcatgacgtgttggatcctttgtgctcgaacgggcattaaaccgcattatgttggtggttattgcgagccgctttccagaaacagaaaaaccattacccctgaaaaccgaaaaatgccacaatattggctgtttatacagtatttcaggttttctcatggcattaaccgccgcgcttaaagcgcaaattgccgcctggtataaggcgcttcaggaacagatccccgactttattccccgtgcgccgcagcggcagatgattgcggacgtcgccaaaacgctggccggagaagaagggcgacatctggcgattgaagcccccaccggcgttgggaaaacgctctcttatttgattcccggcatcgccattgcccgcgaagagcaaaaaacgctggtggtgagtaccgccaacgtggcattgcaggatcagatttacagcaaagatttaccgctgctgaaaaagatcattcccgatcttaaattcactgccgcttttgggcgtgggcgctacgtttgtccgcgtaatctgacggcgctcgccagtactgaacccacgcaacaggatctgctggcgtttcttgacgacgaactgacgccgaacaatcaggaagagcaaaaacgttgtgcgaagctgaagggcgatctcgatacttataaatgggatggtctgcgcgatcatactgatatcgctatagatgacgatctctggcgtcgtttaagtaccgacaaagccagctgcctcaaccgcaattgttactactatcgtgaatgcccgttttttgtcgctcgtcgggagattcaggaagcggaagtggtggtggcaaaccatgcgctggtgatggcggcgatggaaagcgaagcggtattgcctgacccgaaaaatttactgctggtgctggacgaaggccatcacctgccggatgtggcgcgggatgcgcttgagatgagcgccgaaatcaccgcgccgtggtatcggctacagctggacttgttcacgaaactggtcgctacctgcatggagcagtttcgcccgaagaccatcccaccgctggcgatccctgaacgtttgaatgcgcattgtgaagagttgtatgagcttatcgcctcgttaaacaacattctcaatctctacatgcctgccgggcaggaggcagagcaccgttttgcgatgggcgaactgccagatgaagtgctggagatctgccagcggctggcaaaactcaccgagatgctgcgtggcctggcggagttatttcttaacgatttaagtgagaaaaccggcagccatgacattgtacgtctgcatcggttgattttgcagatgaaccgcgcgttggggatgttcgaggcgcaaagcaaactctggcggctggcttcgctggcgcaatcttccggtgcaccggtgaccaaatgggcgacgcgggaagagcgcgaagggcagctacacctctggtttcactgcgtgggaatacgtgtcagcgatcagctggaaaggctgctgtggcgcagtattccgcacattattgtcacctccgcaaccttgcgttcgctgaacagtttttcgcgtttgcaggagatgagtggtctgaaagagaaagcgggcgaccgttttgtggcgctggattccccctttaaccactgcgaacagggcaaaattgttattccccggatgcgcgttgagccttccatcgacaacgaagagcagcatattgccgaaatggcggcctttttccgtaagcaggtggagagcaaaaaacatctcggtatgttggtactgtttgccagcggacgggcgatgcagcgctttctcgactatgtgacggatttacgtctgatgttgctggttcagggcgatcagccgcgttaccgtttagttgaactgcaccgcaaacgcgtcgccaacggtgagcgcagcgtgctggtgggcttacagtcatttgccgaagggcttgatttgaaaggtgatctgctcagccaggtgcatatccacaaaatcgcttttccgcccatcgacagcccggtggtgatcaccgaaggggaatggctgaaaagcctcaaccgctatccgtttgaggtgcaaagcctgccgagcgcctcgtttaacctgattcagcaggttgggcgactgattcgaagccacggttgctggggcgaagtggttatctacgacaaacgcttgctgaccaaaaattatggcaagcgactactggatgcattaccggtatttccgatagagcaaccggaagtccctgaaggtatagttaaaaagaaagaaaaaacgaaatccccacgccgtcggcggcgttaatgatgtgagtcaggtaaggagtcgtaaatggactatcgcaaaatcattaaagagatcgggcgcgggaaaaaccacgcgcgcgatttagaccgggatactgcgcgcggtctgtatgctcatatgctcaatggtgaagtccctgaccttgagttgggcggcgtattgattgcgctgcgtatcaaaggagaaggggaagcagagatgctcggcttttacgaagccatgcaaaatcacaccatcaagctgacgccgccagcaggcaagccgatgccgattgtcatccccagttacaacggcgcgcgtaaacaggccaacctgacgccgttgttggcgattctcctgcacaaactcggttttcctgtggtggttcacggggttagcgaagatccaacccgcgtgctgactgaaaccatttttgaattgatgggtattacgccaacgttgcacggcgggcaggcgcaggcgaagctcgacgaacatcaaccggtgtttatgccagtcggcgcgttttgcccgccgctggaaaaacaactggcgatgcgctggcggatgggcgtgcgtaacagtgcacataccctggcgaaactggcgacgccatttgccgaaggtgaggcgctgcgtctttccagcgtttcgcatccggaatacattggacgcgtcgcgaagttctttagcgatatcggcgggcgggcgctactaatgcatggtactgaaggtgaagtgtatgctaatccgcagcgctgcccgcagatcaatctcattgaccgtgaagggatgcgggtgctgtatgaaaaacaggacactgctggtagcgagttactgccacaagcaaaagatccggaaaccacggcgcagtggattgagcgttgccttgctggcagcgaaccgattcccgaatcgctgaaaatccagatggcttgctgcctggtggctacgggtgaagcggcaactatcagcgacggcctggcgcgcgttaatcaggcattttaattcttttctcagccggatgagccatgtcatccggcttttaccccaccgcaatatgaaattcctgcatctttattgaccttcccacgcccggcgtgcagcataaaaatacaacaaacacataacataaacaggagttaaccatggaaagtggtcatcgctttgatgctcagacgctgcacagttttattcaggctgtatttcgtcagatgggtagcgaggaacaagaagcgaaattagttgccgatcatttaatcgcggcaaacctggcagggcatgattcacatggtattggcatgatcccaagctatgtacgctcctggagtcaggggcacctgcaaattaaccatcatgccaaaaccgttaaagaggcgggggcggcggtcacgctcgatggcgatcgcgcatttggtcaggtcgcggcacatgaagcgatggcgctggggattgagaaagcgcatcagcacggtattgccgccgtggcgctacataactcgcatcatatcggccgtatcggttactgggcggagcagtgtgcagcggcggggtttgtctctatccactttgttagcgtggtcggtattccaatggtcgcgccgttccacggtcgcgacagccgctttggcaccaatccgttctgtgtggttttccctcgtaaagataatttcccgctgttgcttgattacgccaccagcgccattgcatttggcaaaacccgcgtcgcctggcataaaggcgtccccgtgccgccaggttgcctgattgacgttaacggcgtgccgacgaccaatccggcggtaatgcaggagtcgccgttgggttcgctgttgacctttgccgaacataaaggctacgcccttgcagcgatgtgtgaaattcttggcggggcgctttccggcggtaaaacgacgcatcaggaaacgttacaaaccagtcccgatgccattcttaactgcatgaccactatcatcatcaacccggaactcttcggcgcgccggattgtaacgcgcagaccgaagcctttgccgagtgggtgaaagcctcgccgcatgatgatgataagccgattttgctaccgggcgagtgggaagtgaacacgcgtcgcgaacggcagaagcaggggattccactggatgcgggaagctggcaggccatttgtgatgcagcgcggcagattggtatgccggaagagacgttgcaggctttctgtcagcagttagccagctaaaaaaaagcccgtccagtggcggacgggcaaacaagggtaacataggatcaatgagggttagagcatatgcgtctgtcggcaaacagacagggaaatacttgtgctggacgtagcgtaaacgcctgatccgtccaacggttcggattttgtaggcctgataagacgcggtagcgtcgcatcaggcatctgttgccggatgcggcgtaaacgccttatccgtcctacgaattacttataaattaccgcagtaccgcttaatttattgttgttggtggcggaagtgatgctgtatccactggcaccggctgccgcggctttctcagccagtttcgcttccagggcatcgagggtggatgcgccatcggcagaaaccacgccgattttattcatgttctgtgcctgggatgccgttaccggttccgccgcgaacacgccaaatgacagagttgaaagagccatagcagcaacaacagtattgatagttttcataattaatctctcgcaggtgatttttgtataagtgacgttgtttcgtcgatgtgatgagtatcacgtttttttacgagagataaaatcgaagagaattgaccgccttgttcaaataaattgattgatatctaacctactgataaaccatttatttgttgtacttatgaacttgttttataccgcgtggcagtcacagcagcgttaaaggcacggaatgacacgcaaaatacaaattatactcgctatgcatctcgccagttgtagttaacgtaactggctgtctttcgaacctctgcgattatatcctgtataagctggtttttgtaaatctttctcctgctgacaatgaatacataagcgcacgccaggaatggcttcccgacgggcctgcgggatgggggcaccgcactcttcacattcatccaggctttcgccgcgcggaatttcaccccgagcgcgggcaatcgcatcttcaattgtactgttgatctgttcgttgacggcgtcatcgttagcccaaccggatgccatatcgacctccccatatcaatacttgtacagttaagtgtagctaatccagggacgaactcgggcagttcaagcatcagatctccgaccattcccgcagcagattatgataaagattaagcagcgacaggatctcttcactttcgccgtagcggcttttcagcgactgaatattgttgtccagttcaaacagcatggcgcgctttttatcatcgcggatcatcgactggatccacataaatgatgccactcgtacgccgcgggttacgggtgtcacgcaatgcaggctgctggagggatacaacacgagatcgcctgccgggagttttacccgatgttgtccgaaggtgtcattaacgaccagttcgccgccgtcgtagctttgtggatcgcttaaaaacagcgtggcagaaaggtcagtacgcatccagccgttttgtggatggctgcgtactgcgccatccacatggaaaccataggtttcattgttctgatagcgattaaacagcggcgtggaaagggtacgcggcaaggccgcggcaaagaataaagcatgttggttaaccgcgttcagcacctcattttgcagggcggcgtataacgtgctgcgggtgtcgacctgttgattgttcttaacttgcgcaccttgtgcgccggtggtgacgcgtccatccacccattcggcttgttccagttgttcgcgaaaacgagcgacgtcctgtggcgataacacgccgggaatgtggtacatcatacaatttctccaaaaagtggggcctgcgccccacatctgaatcagaaatgcatattggctgtgagcaagaaggttcttggctcgcccgggtgataacggtagccgctcttgttgattgaggcgacgtaatcggtatcaaacaggttgtaaacgtttagctggaagtcgagattgcgattaactcgataccccagtttggcatcggcgacccagtaaccttcggtaaacgctggcgttcccaccgcgccgtctgaacctttatgcatactgccgatatagcgtgcgcccgcgccaacagagatatcgtcggttgcctgatattggctccataaggtgaaggcgtgctccggggtatacggcagcgatgaggaaccatcctgggcaacatctttgccgtttttgatggttgctttttgctgggtatagccgccaatcacctgccacgcgggagtgatattcccggccacggatatctcatagccttcgacgcgtttcttaccgtattgcgagtaagttccgtcatcattttgctcaacttcattttcgatatcagtgcggaacagcgcggcggtgagcaacagacgtttatccagaacctgccatttggtgccaatctcgctggtgttggctttttgcggtttaaaatcggtgcggttggcactgttaccgctgccagactgcgcaagggcgaagttgttgccgcccggaggctgctgggaaacggcatagttaatatagacattgccgttttccgtcaggtgatacagcgccccggctttccagttcatcagattgcccgacttggcggtgtcgacggtggtgaccggagaaccttttgccacaccagttgggcaggtgatggcaccgcgtccgctgccgccgcaggcggtggcactgtcatattcagtatgataattatccagacggatcccgccgttcagctcaaaatcacgggtgatttgcagcgtatcaaaggcgtaaattgcgaaggtatccgtctgaccattggcgtttgcgccgttgcgcgtcaggccgccgggatgaatgctgctgtcaggatgataaatatttaccgcgggtaacgtcaccggattaacgccgtagttagtctgcgtttcacgggtaaattccacgccggtactgacatcatgaccgatagaaccggtatagaacgtcgaggtcaggttggtctggttggtgagaattttattactcacatctttggtattcgccgtgcgtgaccaggtccagctattcacatcgctggtgggctgagtaatattcgacgccccgcccataatcgccgtcatcaggtaatcctgctttacgcgcgaccaacgggtagtattgcgaatggtggtgttatcgttgatgtcgtgctcaaaacgcatggtggcggtgtcggtggtcgaatcgtcgtaatcggaatccgtgccgtaaaagttatgagtatcaacttttccggaatgattcagggccgccgttcccgcagatggggcagaatagcccggcaaaccgatggtcggaatgccgccgtctggcgtgttgtgctgggtgacatgcagataattaagatacaaacgattcgctgtaccaaggccaaaagcgacagaaggggcgacgccgtaacgctcatttttgactttgtcgcgtccggcatcgtgcgttttttcgcccattacattcaggcgcaccgcggtggtatcaccaatgacctgattgacgtccagcgtgccgcggcggaaccaggcgctgccaatactggcggaggcgtcaatgccggaatcattgcgcggctgcttgctgatcatattgatcgagcctgtcggtgcgctgcgcccgtagtcggtgccggacggccctttaatcacttcgacctgctcggtattgaaggtgtcgcgcgagacgctgccgatatcgcgaatgccatcaatataaatactgttagaggtatcggcaccacgcatataaatggcgtcgccagtggtggagttaccgttctcacccgcaaaaaacgcacccacgccggggacgtttttgagcgcgtcggtaaggttggttgcgccctgatctttaatcacttgttcagaaattaccgtcatcgtgcgggtagtatccgctaccggacgcgagaatttcggatcggcagattgttgtggcgcataaagcgaaggcgttgatgcttcgacaaccagcgtgtcatccgcgttagtttgcccttcggcggcgagtgcctgagccacaggcgtgatgccaatacaaagaccggcaaagaacgtgagcgaatgaaattgtctggcagggaaattgcgattgttttccattttgcaggtgactttttcttatatgttgaaattttcactgccacgagaaagcctctctgcggatgcgatgccactgttaatcccgtgatagtgctcgtgaaagtgataataattttgataagcattatcacttggagcgattttctatcacccattgcgcgaaaaagaaatacatttatttacattgagttcatatttgatgttttttgattacaaaacagacgaaaactgcatccagaggcgaatgcagttacgttggtggggttatttgtagatggttgcagtaccgaacatctggtcatttccgcctgcggaattaatgacataacctttcgcgccttgttcgcgcgctttttctgccagtttatcctccagatcgcttaggtttgatgcgccagttgccgaaacggtaccggcgggccgtagctgaccgctgtccaggttactcatcggttgcgcggcataagccgtgagagagattccgctcaggacggtggcaatcagtagtgtgaggcactttttcataatgacatcctcataaatacaacgggtagtgcctgataagtgtaggtcgcctgcgcgatgcaaatgacgcaaaaaattgacagagatgtgcttattttttgaacgatatatttttacaaaataagacaaatcaatgacatgcataatgctgatttttatgatgaattgccataaaccatagccatgttaaggttttggggaatgataaacgcagccagatatttaccctgtcgcgttatgcgggtatcttacgccgctgcttaaaggagaatgctatgtccgcccagaaaccggggttgcatccgcgcaaccgtcatcacagccgctacgatctcgccacgctttgtcaggtcaatcctgaactcaggcaattcctcacgcttacacccgccggggagcaaagcgtagactttgccaatccgctggcggtgaaggcgctcaataaggcgttgctggcccatttttacgccgtagcgaactgggatatccccgacggttttctctgcccaccagtaccgggccgggcggattatattcatcaccttgccgatttactggcagaagcaagcggaacaattccagcgaatgccagcattctggatatcggcgttggtgcgaactgtatttatccgctgattggcgtacatgaatatggctggcgttttaccggtagtgaaaccagcagccaggcgttaagcagtgcgcaggcgattatcagttctaatccggggcttaaccgcgccattcgtctgcgtcggcaaaaagagagtggggcgatttttaacggcatcatccataaaaacgagcaatacgacgcgaccttgtgtaacccgccattccacgattccgccgctgcggcacgggcaggtagtgagcgtaaacgccgtaacctggggctgaacaaagacgatgcactgaactttggcggccagcaacaggagttgtggtgtgaaggcggtgaagtcacctttatcaaaaagatgattgaagagagcaaaggcttcgcgaagcaggtgatgtggtttacatcactggtatctcgtggtgaaaacttaccgccgttgtatcgtgccctgacggacgtgggcgcggtgaaggtggttaaaaaagagatggcccaggggcaaaagcagagtcgctttattgcctggacctttatgaacgacgagcagcgccgccgttttgtcaatcgccagcgttaaagcgttggttcccccggcggtaacggttcagccggggtcgcgcccggagcaggcagcacctgataagtctgcactggcgcgcgaacgcccgccaggtcgaaatgttttttcacctggctgtcgagggcaaagcgtaccgtccactgtttgagtggcagcgtggtgaacgaaacacgcagtgtaaacgcggtattgcttaagccgacaatcccggcaaaattcggttcaccaataatcagcccgcgaatttcttcgttttccattaattccgctaccgcatctttcagtgcctgattggctttatcagcatcttcatggcgatcaacatcataatttgccaccaccgaaccaatgccgcggacaaagttagcaaaggtggttatcgaagaccacggaatgatgtgatacgccccggtatcctgtcgtacgcccacggagcgaatcgacatccgttccactgtgccggtcaacggcccgatagtcaccaaatctccagtgttcatgccgttttcaaactgaataaataccccggtgataatatctttcaccagcgtttgcgaaccaaacgagatagccagacctaatgccccggcacctgccagcaatggcgcgatattgacgccgatttccgacaacacaatcatgatggtgatggtactgataatcaccgccagcgcgttacgaaacagcgtaagcagggtacgcgtgcgggcgctgggtagcgggcggccatgaatatccgaagccagccggttttcgatcaaactggcgagcaccgtccagccaaccgccgagaagaaaagaatgagtgcgatacggatcaggatatctacggttttctgccccgcgccgttttgcagccagttccagaaatcgaacaatccccatgcgctcaacagcaacattaccgccacgcagactgtcagaatacgcgccgttttcagcgccgccgacagccagccattcaaccgtttttgcagctccggatagttacgctgagtatgtggcgagagagtgatggttttcgccagccagcgggaaaacataccggaaacaaacgctgcgataccaataatcgccaggctgcgcaccgttgcacccatcataaatttcaggctgttgcccggatcgaacaacgaaaagaaaaacagcacgataaaataggcgcttgccagccagtgccacaccagcgcaaaggcgcggataaacaggctgaaaaaggccagcgaatgctccgcgaagttgagcaaatgctgggtaatctcttttttattacgaaagatcaggtacaacgcccagacggtcatgcacagcataatgatgacgttcgccagcgcacctatctgtacattcacctgattagagataatcggcacggccacaatcaggccataacctatcaaactgcttaaccagctcaggcgacgactccagtaacgggcgctctcgtcctgaatcgtgaacgggcgcagctccgccacgtttgggcaaaaaatcaggcgtagtacggctttgaaaaattcaatgagggcaaaggcgttgagaaacaaactttgttggaaagcgatggtgcgactgcctgcattcaggttgtcgcttaatacctggccgacaaataatgtcagggccagtaacagcaggtcgataataaacgccccgataatcatcgccggaagctgcaaccagttgctgcgctcacgatttttttgccgcgcccactgacccattttgcgatacagcggcagtgcgcacaggcgaatcagccagtaaaaaccaaacactaataccgctaacattgaaaaatgggtcagcgcattgctgaaggtttgtggattaaacggcttatgcggggagccggtgatattgcgataaagttgcccgaagcgggcggaaagggcttcaccataatggcggctgacttcggtgaccttttgcagcacggtttgctcttcgaccagcgtcggcggcactatttttggtaccggttcagcagggggcgtagcggcaacggtgcgcaactggtcgatcaactctttacgcgaggtgtcattatccagcacatccgccagtgcgccataggccgcttttttttgttcgatatccggttccggggccggttcagtcgttgagtccgttgtcgttgtggttgtaacgccgggtatggataccgcgtgggcaggtgcgcccagcaggcagaagaggatgaacaggatccaccgcatgactcctccagtgagaaaatagagcaaaaagataagtatagatgctggaggaggggcgattttaaatgagaggaatctggtgtgcctccctttcgggtgaaagggaggaagggatattaagcaggttgctgacaacgtgcgggcttttttgccggatgcggcgtgaacgccttatccgtcctacaagttcatgcaattttaataagttgccagatatcctgtaggcctgataagcgtagcgcatcaggcaatgtgtcttattaagagacgtgctgcaaaaattcctgcaagcgctggctcggcgggttcttgatcaacacctgcggattgccatcttccgcaatccggcctttgtcgataaagatcagccgcgaagctactttctcggcaaaaccgatttcgtgggtcacgatcaccatcgtcatcccttcttcagccagatcctgcataaccttcagcacttcatggcgcagttccgggtcaagagcggaagtcggttcatcaaacagcatcattttcggcttcaccgccagcgcgcgggcaatcgccacacgctgctgttgaccaccagaaagttcggaagggtagtgatgtgcacgttctgccagaccgactttcgccagcagctcacgtgccagtttttccgcctcttctttgttcgcgccacgcacgcgtagcgggccaaacatgacgttttccagcgctgtcagatgcgggaagaggtaaaactgctggaacaccatacctgcttcctggcgaatcaggcgctcgtcaactttcggatcgttaaccttcaggccatcgacaatcagatcgccggaggtgatttcttccagtttgttgatgcagcgcagcagggtcgatttaccggaaccggacggcccgataatcaccacgacttcgccctgggcaatgttcaaatcgatattgtgcagcacctgggttgggccaaagtgcttggagacgtttttaaattcaatcacaggattttcatccttctttccagacgacgcagaataaagctcagcaccagggtaataatcagatagaacaccgccacggcgctccagatctcaagggcgcggaagttaccggcaataatttcttgcccctgacgggtcagttccgccacgccgatcacaataaacagcgaggtgtctttaatgctgatgatccactggttacccagcggcggcagcatacgacgcagtgccagcggtaaaatgacgtagcgaatggtttcccaacgtgaaagaccgagcgccagtcctgcttcacgaaaacctttgtggatagacagcaccgcaccacgcgtgatttccgcaatatacgcgccggagttgatcatgatggtgaccaccgccgcagtaaatgggtcgatgcgtaagtcgttaaacgccatcggcagggcgaaataaataaacatcacctggacgacgataggtgtgccgcggatcacttcaataaagaccagcgcgacgtggttggctatccaacctccgaaggtgcgtgcaaaacctgccagcaatccgattaccagaccgcctgccagaccgaggaccgaaatccacagggtcattttggcaccttcaatcagaagcggaatggcaggccagatggcactccagtcaaactgcatatgttgttcctgttaccgtggtgtaaataatcaaattcagggtaattaatggccccggagcgggtttgcgcccctcaccctaatcctctccccataggggagagggaactgccagtgcgttttacaggtgtagcgttattatttcggttcagtaccgaaccattttttgtagatttcgttgtaagttccgttctcgcgcagggttttcaacgcgccgttgactttgtcacgcagctcgtcgctacctttcgggaacgcaataccgtattgctgcgcttccagagagtcacctaccgctttgaactgaccgttaccggcggttttgatgaagtacagaatgtttggcgtatcgtgcagaacggcgtctgcgcggttggtgcccagttccatataggcgttatcgatgttcgggaactgacgcagatctttagttttgatgtttgctttcgcgtaatcaacggagccagtaccgctcttcacagcaaccactttcccgtcgagatctttcacgcttttcacatcgttattgttagctttcaccatcactaacaggccgcttttgtagtagccgtcagagaaatcgatcgcttttttacgctcgtcggtgatggtaatgcccgccagcgccagatcgacgtttttggtttgcagtgccggaatgatcccactgaaatccatcggcttcagttcgtaatccagcttcagctctttagcgatggcagcccacagatcaacgtcaaagcccacatatttatcgccctgtttaaattcaaacggaacgaaggcggtatccgtcgcgacaactaattttttatccgcggcatgagaagaaaccgcaaaagccagggtcagtgcagccagtgaaacttttaatacagacttcatagcatttccttttttctatccacgggacgatcccctgcgtgacattcacatatatgaaaaaatcgtgccagttttgcaactccttgatttttcgagatgcggcaaaaacgtgatgcacgatttatagggcaataccctgaagatgcaccattctggggcaccaatctggtgcgctaaaattgtgcactcaacacagtgattatttagcgtaaaacctgatgaaaaaacaatctttatgtaacgattgtgtgatgatgtggatacaaaaaatttacttaatcagctggagatagcagatggatgcactaaataagtgcgttgaggtgggctgcaaaacaaaacggcctcctgtcaggaagccgcttttatcgggtactaaagttctgcaccatcagcgatggatttattcgatgttagactcgataaaccacaggaatttatccaggtcgcgagacgcggcggtcaggatatctgcggtgtcgtcatctttcgcttcgccaatcgctttgcgtacgtcattagcgacgattgcgtaacggtcagccagttctttcaggtgatcctgaacgttgtggatgtccagcgggtaacttttcagcggggttttgctgttgataacttgagtggtccccagagctacaccgcccagctgcactgcacgttctgccatggtatccagatgatcgatcagtgcggtgcggaagccatccagcatttcatgtacggcaatgaagttagcgccgcgcatgttccagtgcgcttgtttggtaatcaaagaaagatcaataaactggataacctggcgattcagcaactctactgttgcttttttctcgctgtcggagacatcgttgcgggtataaagcagattggtcgcttttgatttaactaatttagcggtactcataatttcatatcctcttgatgttatgtcccagtaattaacgagattaagtatagcaccggctatgtgttccgctattctggctgttcctatcacactaatagtggtaacaagcgtgaaaaacaaaactaataaagattcaatgagttagatatattgataagaacaattcttatttatctgctcgccaggaattttcggaataaatatgcttttgcataattcgatatataaagacggtgtagaggaaaagtagcgagaaattctgcatggttatgcataaccatgcagaaatgtaaatttaattaatgtctaattcttttattttgctctctttgcgtactgtcagcgtagaccccattgaagcggcgatgatagcgccgagcgccagtagctgtatgggtgtcagtgtttctccgaggaaaatcatcccggaaacggcagccagcgccggttccatgctcatcagcgtaccaaatgtccgtgttggcaaacgggtgagggcaatcatttccagcgaataaggcagagcggtcgagagaatagcgacagccagacccaatggaataaccgaccagtgccagagtgcttcaccagcctgaagcgctccaattggcacgaaaattaacgctgcaatcaacgaaccaattgccaccgtcgcagggccatgttccgctcctgcgcgttgcccacttaaaatgtaaatagcccaacaagccccggcccccagtgccagcgcacagccggttaaatcgacatgggaaacgtcttgccccagcggtagcaggaaccacagaccaagaaccgccagcacaacccagacgaaatctaccgggcgacgagaagagaacagcgccaccgccagtggtccggtgaactccagcgccaccgcaatacccagcggtactgtctgaatagaaagataaaaaagataattcatcccacccagcgaaacgccgtaaaacaacagcggtaaccgttgctctttggcaaagcgcagtcgccatggcttaaagaacgcgatgaggatcagcgttcctaatgccagacgcagcgcagtgacacccggtgcgcccaccagaggaaaaagtgacttagctaacgaggctccaccctgaatagacgccatggcaacgagcaatatgactattggtaaccagaccggcattttacgtaatgaaccaggcatcctttctcccacaaatatctagacttaagtaaagcgtggagtgtactggatatacccaatgctggttgagcatttgttgaaaaaattttcccccgttttgactaaaatgcgccaggattgatggaatcattagtctggtgattaggaataatctggatgaatgacagggaaaacatgcgtaatacttacgcagttctctgaaaaagtgatttaaatttagatggatagcggtgtatggaaacgttctgttacatgaaatggcccgttagacatcacaaatcgcgaagagtttcccattaatttttgatatatttaaaacttaggacttatttgaatcacatttgaggtggttatgaaaaaaattgcatgtctttcagcactggccgcagttctggctttcaccgcaggtacttccgtagctgcgacttctactgtaactggcggttacgcacagagcgacgctcagggccaaatgaacaaaatgggcggtttcaacctgaaataccgctatgaagaagacaacagcccgctgggtgtgatcggttctttcacttacaccgagaaaagccgtactgcaagctctggtgactacaacaaaaaccagtactacggcatcactgctggtccggcttaccgcattaacgactgggcaagcatctacggtgtagtgggtgtgggttatggtaaattccagaccactgaatacccgacctacaaacacgacaccagcgactacggtttctcctacggtgcgggtctgcagttcaacccgatggaaaacgttgctctggacttctcttacgagcagagccgtattcgtagcgttgacgtaggcacctggattgccggtgttggttaccgcttctaatcactttggtgatataaaaaatccgcctctcggggcggatttttgtttttaaggtttcgggtcgaaaatatcggttccgagatggttgtaatccaccttctgtaactggaagttggtgatgtatatcggcccggctttcttctcagatataaacgggtatttgatgttaatttccttcgctttaatccccgtccactgggagaaaaagcctaagaagtcattggctgagcggcgggctttaatcacacgatgcgctttatcgtcgctggaaatgaccataaaaggcacctggaaattttgctgatatttatcatcatgggcaaggtattgcacgtctttaccgcgctctttaaaggccagaccgtggtcagaaaagtaaaccagcgagaagctgctgccgctgttgcgtaactgatcgtacagcttgcgcagtaaatcgtccgtttgcgtcatggtatagagatagcacgacgtttctttcgattgcacaaaggtttcgtattttccttgtgtcctgtcgcaggcctgcggatgtgagcccatcagatgtagaacaatcagctgcggttgcgagtgctcttgcgccagcacttgagcggtcatatccagtaacgcttcgtctttggtgtttttatctgcttcaaaattaccttctttcaggaagtacacttcatctgctcgtttggcgatgctggcgatagcggtatcgtattcgccgatttgaccctggttggaaaaccaccaggtctggaagcccgcgcgatttgccagggtgacaaagttatcctgaaactgtggtttgccatcgacaacgcgattgagcgttaagccaagcgatttctgcgtggagccactggcggcaatgtagtcagcaaatatcaaaccgttaacgctgctggcaaacggggtattgtcccagtgaccgccaaaggcaccgagggcatcgcgacgcgcgctttcaccgatcaccaccacataggtctgatacttcggcttaacggcagtgaccgtccaggtatctttcattccggaaagttttgccatccgttcttgctcttcaatcacctcgttattattgacgatgacatccttagcaaaacgaaataccggatagccagtatctttcagtttaaatacgccaccccaggccaggttttgcacgggagcaacaaaaaatgtcgccacactgaataccagacacaggctgtcgaaggtattccagcgcgctttttcattctctttttttcgcctgattgctattacgccgagcgcaaaaataaataagccgaccaggtagctgtaccacggaaaaatcgtcaggatttcggtcgactcttccatattggtggagtgcaatgccagcaatgtattgaaattaggcgcgccgtaggcctgagcaaaagggaaataacaagccgccaccagcgaactgacaccgaccagaactttttgtacgcgaggcaatgttcgccatagcaaaagcaaaatagccgtaaacgcagcggtgtagagcaaactgaaggggtaacctaagccgaggttaattaatagcgactgtaaaaagtagaacgcagtccacgggctaaatacccggctacgggtaacaagcgattctttgagggttaaattcatatgccactatcgtaacaaacgccatgtgcttaccctggcgtcaagggtcaatacctgcaagagtgcgtgaagagtggaaaggggtccgcatccgcgagccgcaatatacgcagggctgcaagaagatagagcgagccgccgttcaggtcaactactgacgaacaaatcttttgcgaaggggattgcaaatccgacaaaaagtggggtttttcagaccaaaacgcgttatgcctgcatgaaagcaggagtgaagcggcgtaccgcgacgccgctatttatcggaaggtttatcttgctgcggtttgttgttgaccatatcgcacaacatagagagcagcattaaccgtactttaaagggagaatgactaaacacgcgcatacacctcttgaactcattcataagacctcctgacttgctaatcccgtcgatccttgagggatgattgcattacatacagatatagcacaggctatattatatagctattgctaaaacgttaattttttgtaccttcgcaactctggtttacaatgtgcgcacgaaatgagaacgctatgtatgcgtcaccataatgaggaagcacaatgagtcgtcgcgcaggtacgccaacagcaaaaaaagtgacgcagttagtgaacgtggaagagcacgttgaagggttccgccaggtcagagaggcgcatcggcgcgagcttattgatgattacgttgagctgatttctgacttgatcagggaagtgggggaagctcgtcaggtggacatggctgctcgtctgggagtttcgcaaccgacggtggctaaaatgcttaagcggctggcaaccatggggctgattgaaatgatcccctggcgtggcgtgtttttaacggcagaaggagagaagctggcgcaggaaagccgcgagcgacatcagatagtcgaaaatttcttgttggtgttgggcgtcagtccggaaatcgcccgtcgcgacgcggaaggcatggagcaccatgttagtgaagagacgctcgacgcttttcgtttgtttacccagaaacacggtgccaaatgagcctgccttttttacgcacgctgcaaggcgatcgtttttttcagttattaattcttgttggtatcggattaagctttttcgtgccctttgcaccgaaatcctggcctgctgctatcgactggcacaccatcatcaccttaagcggcctgatgctgctgaccaaaggtgtggagttaagcggttattttgatgtgctggggcgcaaaatggtgcgccgctttgctacggagcgtcggctggcgatgtttatggtgctggcggcggcgctgctttctacctttctgaccaacgatgtcgcgctgtttattgttgttccgctgactatcacgctaaaaagactgtgtgagatcccggttaatcggctgattatttttgaggcgctggcagtcaacgctggttcgctactgacgccaattggcaacccgcaaaatattcttatctggggacgttctggtctttcgtttgccggatttattgcccaaatggcaccgctggctggcgcaatgatgctgacgctcctgctcctgtgctggtgttgtttccctggaaaggcgatgcaataccatacgggggtgcaaacaccggagtggaaaccgcggctggtgtggagttgtctggggctgtatatcgtctttctgacggcgctggagttcaaacaagagctgtggggactggtgattgtggcggcaggctttgcgctgctggcacgtcgcgtggtgctcagtgtggactggacgctgctgctggtgtttatggcgatgtttatcgacgtccatttactgacccagcttccagcgttgcaaggcgtgttgggtaacgtgagtcatctatctgaacccgggttatggttaacggcaatcggtttatcgcaggtgatcagtaacgtgccgagtaccatattgttgctgaactatgtgccgccgtctttattactggtatgggcggtaaacgtaggtggctttgggttattacccggatcgctggcaaatttgattgcgctacgtatggcgaacgatcgccgcatctggtggcgtttccatctctattcaataccgatgctgttgtgggcggcgttggtgggatatgttttgttagttatactcccggccaactagggtctggcaaataaaaaaggcggattatgagtccgccttttgctttaagttttgaagattaattcagacgaaccggcatcccggagcggtttttaatcgcttcatcaagaacaacctggtcaacatctggctgaccggtcactgtctgcacgctcttcgtcagggtaattggcacaatttcctgaccttcaaactgggcttcggtggtagacagcgggttatggacttcaatataacggctgccgtctggctcggtggtcgcttttaccggctcatcaataaactgtacgcgggtaccgaccggtactttctcgaacaggaatttgatgtcttcgttacgcagacgcacacaaccatgacttacacgcaggccgataccgaagttggcgttggtgccatggatagcatacaggcgaccgatatagagtgcatacagccccatcgggttatccggacctgccggaacgacagccggaagcggttcgcccgcagcgcggtactctgcgtgcattttggcggtcggcgtccaggtcgggcctgcttttttacgctcaactttggtggtccagttgataggcgtatctttgcctaactgaccaatgccgatcggcagcacgataacggtgttggtccctttcggatagtaataaagacgcatctcagcactgttaatgacgatgccttcatgaacggtatccggcaggatcagctgctgcggaatgttcagtacagtaccgcctttcggcaggaaggtatccacacccgggttcgcttccatcatattggaaagccccatctggtactcggcggcaaaatactccagcggctgagtgttaccttcaggaatggtgatcacctgattctgaccaaccaggcgactcccgtcggttggcagaggataagttaccgcagaggcggtactgcaaaagccgacaacagcgaaggccgctgcgaataatgttttcaatttcatattcatgttaagcgagattttgtgcctggcaggccattgggttgagaatattagagtattggaagcgcattataagttcattccagctcacagtgaaatcagatgtgtacgaaatcacattttttgcctttggcttgagtgtagaccttaagcgaggagcaggatcttctttcagacttatggcataatgcgcggtttgtcatatctcttttcaggatacgcctgtgttagtttccagtaacgtcaccatgcagttcggcagtaagccgttgtttgaaaacatttccgtcaaatttggcggcggcaaccgttacggcctgattggcgcgaacggtagtggtaaatccacctttatgaagatcctcggcggcgaccttgagccgacgctgggtaacgtttccctcgatcccaacgagcgcattggtaaactgcgtcaggatcagtttgcctttgaagagttcactgtgctggatacggtgatcatggggcataaagagttgtgggaagtgaagcaggagcgcgaccgcatctatgctttgccggaaatgagtgaagaagacggctataaagtggccgatctggaagttaaatacggcgaaatggacggttactctgcggaagctcgcgccggtgaactgttgcttggcgtgggaattccagtggaacagcactacggcccgatgagtgaagttgctcctggctggaagctgcgtgtgcttctggcgcaggcgctgtttgctgatccggatattctcctgctcgacgaaccgaccaacaacctcgacatcgacaccattcgctggctggaacaggtgctgaacgagcgtgacagcaccatgatcatcatctcgcacgaccgtcacttccttaacatggtctgtacccacatggcggatctggattacggcgagctgcgcgtttatccgggtaactacgatgagtacatgacggcggcgacccaggcgcgtgaacgtctgctggccgataacgccaagaagaaagcgcagattgctgagttgcaatctttcgttagccgctttagcgccaacgcctcgaaatctcgccaggcaacttcgcgcgcgcgccagattgataaaatcaaactggaagaggtgaaagcctccagccgtcagaacccgttcatccgttttgaacaggataagaaactgttccgtaacgcgctggaagtggaaggtctgaccaaagggtttgataacggtccgctgtttaaaaatctcaacctgctgctggaagtgggtgaaaaactggcggtactgggtaccaacggcgtcggtaaatcaacgctgctgaaaacgctggtgggcgatctgcaaccggacagcggcaccgtaaaatggtctgagaacgcgcgcattggttactatgctcaggaccacgaatatgagtttgaaaatgatctgaccgtgttcgaatggatgagccagtggaagcaggaaggcgatgacgagcaggcggtacgcagtattctcggtcgtttgctgttcagccaggacgacatcaaaaagccagctaaagtgctttccggtggggaaaaagggcggatgctgtttggtaagttaatgatgcagaagccgaacattctgatcatggacgaaccgaccaaccacctggatatggaatccattgagtcgctgaacatggcactggaactgtatcagggcacgctgatctttgtttcacacgaccgtgagttcgtaagctccctggcgacccgcattctggaaatcaccccggaacgcgtgatcgactttagcggtaattacgaagattacctgcgtagtaaagggatcgagtaagtgattatccgtcaccccgatactgtcggggtgacggcggctgatgacaaatgcaaaatagcctgatgcgctacgcttatcaggcctacgcagtacctgcaatatattgaatctgcaggactttgtaggccggataaggcgttaacgccgcatcaggcattaacaaagcgcatttgtcagcaatctgagtaacgtcgaatcgattttcttaatcccacatcaattcacttccattaattctcaaacatccatgcccaacgctcgcttaccgtgaatgttgaggtcggcaagcgtaaagcgtccttcccagtttgtttcatagtcctcgcgcgggaagtcgcccggcgatgcgcctttttccagtgcggccttcaccttgtgcgcgtaggcaagatttttctcgcacatcggtgccgcaggaatgtacatcacgttgccccaaccttgttgattttcaacgggggcaacggaatggatgacgtcgcagtgccaccagacggagtctccggcttcgagttttggaatgctggttaacgcctcaatcaacagtggatgccattgctctgataccggcaatactcttccgggcgctacgccgcacagttcatcctccggcacatcatcaagcagcggacgtaacagtacgtacgccatagcttcaggaatgggcacgacgtgcagcagcccctgaccaggcagcatatcagagagcgctgtccagccctggaatgtccgaaacacggaacatttggtggtgttgtccaccgtgtactcttcaacttccgtacgatgtgccgcatgccagggatcatattgcgccagattgccattaaagacgttggcgaaaacgcgctgatacgctggaagcagccagcgttccagtgccccggagtcggtatgcgctccaagacctttggaggtcgttccgggcggacggcggcggatacggtcagggtagatgacgctcacatccgggttaaaccattgctttccatcactttcaaatgtccacagacgattgagaaacgactgcgcattcgccatttcttcactctggcgggcctgcatttgcgcctgcgaccagtagatggggtaaatctcgggacgtgaagcgctgagcgtcccgaagaaattatcgccggggcctttgtagacctcgtcaaagcggttgcggtccagatagtccagcatcgactgatcccagcctagcgcttgttcgcgggggaaatggccttttatcaccgcacaaccgcgacgtttaatctgttcgcgctgctctgcagtaacatgacctgctttgatatcggcataagacagcaccggccagacggcatcgccctgtgctttgagtgcgttgatttcagccactcgcgtggcaatgtcatcgcttagctgattaaagatctgctggacgtcgccaagctgcgcccgcagcgcgtgcttcatctgacggatagctgctttgtgatcggcaggcaatgtgtcgctggtaaaagtagaagccataaccacctctcattaactttcattcgaaaccattctgatttgcatgtgacaatataagttataaataagttaatgcaagtttaatgatttgatgtgatgtacaggatgtaaaaagaagggaaaaccggagcgcacggctccggtagagaggtcagctgttaaaaggggatgtgttatccagcaccgcctgaatcacattcagcgcgccttcatgattattatcatcggtagcgtaacgggcgatttgtttaatgttttccgcagcattgcccatcgcaaaggaataacgcgccattttcagcatctccgcatcgttaccgctgtcgccaatcgctaccacattttgcggtgacagatcccagcgtttcagtaaccgcgaaataccgtttgctttatgtagaccgggaataatcaggtcgataaagccaaaaccactggtaacgggtttcataatgccatcgagcgctacgtgcagtttgtcgatcactaacgggatttgttcatccggcaggttgagcgaaaacttgaacagtacgtcgtcaatctcctgataatcttttacaggtttcaggcgatggtagtgttttgccatcagtgcgacaaatgcttcgggggcattttcgctgacatatgcactttgcagaccgcaggcgacaaaattgagttgcttatcttttagcaactcgccaataacaatccgcgattcatgtcgggtcagttcgccgtggaacaactgcttgccatgttcgtaaaccagtgcgccgttttccgcgacaaaagagatctcatcctttagctcaggaaagaatgaaataagctggtaatactgattaccgctggcaacaacgaacttaatgccgcgctttttcagttcctgatattgcgccataaaacgtggttggttgtacgttttggcgtcgttaagaaaagtaccgtccatgtctgtgacgataacttttacgctcataggtgtgctcctggctcgaaaatgaaaccgtaacagtgtaataacaatgtgacgcagagcacaaattatatttcgaatgaaagtaaggatgaaattgatgatgtgaatgatttagcccggcgacgacgccgccgggccgaggagattacagcatatgttcagtacgggcgatgatatcgtcctgagcgtctggagagagcgcggtgaagaacgcggaatagcccgcgacacgcactaccagatcgcgatactgatcgggatgttttttcgcatccagcagcgtttcgcgggaaacgatgttgtactgaatatgccagcctttatgcacttcaaagaaggtacgcagcaggatcatcagtttctgcttgtcagattcgttctccagcgttgccggattcagtttctggttgagcaacacgccgccgagaatcgctgccgtaggcagtttacccactgagccaatgaccgcagtagggccaagatggtcagtaccggaggccgggcttgcgccttctgccagcggggtgtgggctttacgcccgtccggtgttgccatagtctgcgcgccaaacggtacgttagcggagattgatgacgtacccgcgtaatagttgccgccaaccggaccacgaccgtagcgcggattatggtactgtttcagttcgtcgatataggtctgataagcgcgagccagcagcgtatcgacagtatcatcgtcgttgccgtacttcggcgcaccgttaatcagccgctgacgcagctgctcgtgagtcaggccgtcgaagtcatctgccagtgcggcagcaagctgttgctgaccaatcgcaccttgttcaaacaccagtttcttcactgccgccaggctgttgccgaggttggcaatgccgacctgcaggccagaaacccagtcatatttcgcgccgccttgcttgatacttttcgctcgctcaatacagtcatccaccagcgccgagcagagaatatcgtgcacgttctcttccagcatggtgtcgacgacatattcgatttcgattgatttgcgggtgtagtaacggatttgcgtatcccacgcgtccatcacttcatcgaagttgttgaagttacctgccgacaacgctttttcttgtggcaggaacactttgccgctggtggcatcatgcccgccttccagcgccgccagcatcacgcgggcgaagttgataaagctcatgccggtacagcgatagccccatttgccaccgacggcggtttctatacaaccaatcgctgcgtagtcataagcgtcctgcggttcaataccgagtttaataaattccgggatcacgatttcgtcgttgttgaacgccggcatcccgaagccgcaacggatcacctgtacgcaggcgtcgaggaaatcgttgctcattcctgcatggtaacgcacgctgaggttaggctgagtggaacgcaggcgaccgcaggattcgaggatcgcgtaagagagtggattcaccgcgtccattggttgaccatcaaccagattttgcccgccaatagtgacgttctgatacagcggacttcccgcagaggcttttgagtgtgagccggagcggatcttgttcacttccagcagtttcagccagcagctatgcagcatctcgatggcgtgttcgcgatccagcgtctggttgagttcaacgtcgcggcgatagtacgggtagagatactggtccatacgaccaaacgatactgagtgaccgttagattcgatctgcaaaatcaactggatgaagtaacacagttgcagcgcctgccagaaagtctgcggcggctggtgggcgataagatcgcagttttctgccatcgccagcagttcatcgcgacggctttcgcgggtttcggtcgcggccatttcacgcgccagggcagcgaaacgttcaatgtgttcactgactgccaccagcacgatatcaatcgctttcaggaattgctcaccgtgtaaatcttccagcaccgtcaggttgatgcgcgagcgacgttccgctacttcctcgcgcagaccatcaagccctttttccagcagcagcgggaaattcaccgccaggtgcgcatcgccggaggtcatattgccttccgctttaatgattccggtcgccagcagacctttttgctcatcggtaaacatgccgtagcagcgatcctgtacggtctgaccgcgccaccacgggcacacttcatgcagaacgcgtttgttctcttcgctcaccgcaaagccagcaccgggacgatctgccagatcatcaatctctttttcgatccacgagacagtatattccgggaagatcggcgcggcgcgaacttcgcttgcctggttgccaatgatcaactcatcgtgtttgatccagatggtgcgattcgccaggtgatgcgccagtgccagcgcgcgacgtaccgggatcggcttatcgagatgttgttgatacatctcggtatagtgctgcgcgcgctcggtacagactggcggtttcacaatatgcaccagcgcatttttgtgcgctttaatgcggtcgctgagcgtgtccagtttcagtgtggtcatggttgttatcctcgtaaggtcgcggttaaccctttctggcaggcatactgctgggcaaagtcgagcagttctggcgcatcaagcggtttttccggggcgtcatagggcagattaagtaagtgatatttgttgatgcccagcgtgtggtagggcagaaaatgaatttcgccaacgtgcagctcgtcggcggcaaaatcggtaatggcttttacagaggtttcgtcggcattaaagccctgaatcagcggcacgcggataatgatttttttgcccgctgcggcgagttttttcaggttatccagcactctggcggcgttaccgtcggtccactgtttaaacggcgcgtcggcaacgtgttttaaatcggcaagaaacagatcgatatagggcagagaaggggcgatatatttccacggcacatgcagacaggtttctaccgcagtatgaatgcctgcctcgtggctggcttgcagtagcgccatcgccatttccggctgcataaagggctcaccacccgaaagcgttaaaccgccgccgctgcgatcgtaaaacggtttatcgcgcagaacggtcgtcatgatctcctcaacgcttttcacttcaccacacacggttaatgcctgtgtcggacagcagtcggttaacgccgtcagatgctccggggttaacttttcccgatgaataagcaaaccattcagcgcgcgctcaatcacttccggcgcggccttagcgcacagctcgcagccttccagacacagtcgtgcgtcatacagcagatcctgcgtgcgggcgcggctttccgggttctgacaccagcggcagcccagcgaacagcctttaagaaatacgaccgtgcggataccggggccatcatgggtcgagtagcgctgaatattgaaaatcatagttgcctctctatttcgttcaagcattaaaatactttcgaatgaaagttagattgatgtgcgtcaactgttcagagagttttcccgtgatagtctacattcagacaaaaagtacattttgaggatggttatggaactgtatctggatacttcagacgttgttgcggtgaaggcgctgtcacgtatttttccgctggcgggtgtgaccactaacccaagcattatcgccgcgggtaaaaaaccgctggatgttgtgcttccgcaacttcatgaagcgatgggcggtcaggggcgtctgtttgcccaggtaatggctaccactgccgaagggatggttaatgacgcgcttaagctgcgttctattattgcggatatcgtggtgaaagttccggtgaccgccgaggggctggcagctattaagatgttaaaagcggaagggattccgacgctgggaaccgcggtatatggcgcagcacaagggctgctgtcggcgctggcaggtgcggaatatgttgcgccttacgttaatcgtattgatgctcagggcggtagcggcattcagactgtgaccgacttacaccagttattgaaaatgcatgcgccgcaggcgaaagtgctggcagcgagtttcaaaaccccgcgtcaggcgctggactgcttactggcaggatgtgaatcaattactctgccactggatgtggcacaacagatgattagctatccggcggttgatgccgctgtggcgaagtttgagcaggactggcagggagcgtttggcagaacgtcgatttaaccggacgttctgcatcctcataaattgctgatgacgtggcggagtgccgcgtcttatcaggcctggaggtggcaattactgcccacacacctcacaccccggattacgcatcagtttcatttcgcgaaactgacaggtcatcgcatcgtacatgacgattttcccgctggccggtttgccataacctgccagcattttgatcgcttccattgcctgcaacgaaccaattacgccgatcaacggtgccattacgcctgcttccacgcaggttaatgcattttcaccaaacaaacggctaaggcagcgatagcacggttcaccgtcctgataagtaaagacggtgatttgaccttccatacgaattgccgcgccggaaaccagcggtaccttcgcggcaaaacagcctgcgttcagttgattacgtaccgcaacgttatccgtacagtcgagcaccagatcgtgttcagcaatcaatgctgcaagttctgcgtcatccagcagtgcattgactggcgtaatcgcgatatgtgggttgatccgcgtcagggcgtcacgggcggattccaccttcggttgcccgaccgtggcatcactgtgcagtgtctggcgttgcagattcgagagcgaaaccgtgtcgaagtcgagcagcgtcaggttaccgacaccggcgcttgccagatactgcgaggctgcacagccgaggccgcccaggcccactatcagcacgcgagaatctttcagcgcctcctggccgtcaaaatcaaagccgcgcagaatgatttgccggttgtagcgcagcatctcctgatcgctgagttccgccattacaggcctccgaacaacgcgttaaacggttctacttccacccattcgcccacttccacattgccgcgatcgcgttccagcacgataaagcagttgccgaggctaaaggagctaaatatatgtgaaccctgatgtccggtggtcgtcacttccagttcgccatcggcgttgcgttgcagcacgccgcgctggaaatcaagacgtcctggcgtttttttcaggcgggacgctgtgcgtacgcgctggcgcgcgggcaggccgctggcggtgttaccgcttagttttgccagcaaaggctgtaccagttgatagaaggtcagcgtcgctgaaaccgggttgcccggcaggccgcagaaccagctattgctgagtttaccgaacgcgaacggtttacctggtttaatcgccagcttccagaaggcgatctcccccagctcttcaagaatcgttttggtgtaatccgcctcacccactgaaacaccgccggaactgatcaccacatccgcctggctgtcggcttcaataaatgcggcgcgcagggcatggggatcgtcgcggataatccctaagttaattacctcgcatcccaactgttctaacatcaggtgtacggcgagacggttggtatcgtagatttggccgtcgcccagcggctgaccgggcaactggagttcatcaccggtagaaaaaagcgctacacgcactttacgaatcaccggaacttcggcaatccccagtgaagcaattactggcagctctgcggtagtcaggcgagttcccgccgggaaaacaaccgcacctgcagagatatcttcaccgcgacggcgaatattttgcccgctacgcacttcagcagtaaaacgcacgccattgtccatttgttcagtctgctcctgcatcaccaccgcttcgcagccttccggcaccggcgcaccggtcataatacgaatgcaggtacccgcaggccattcaccatggtatggctgaccggcaaaggatttaccggcaacgggcagcggttgcccggaggcaatatcggctaaacgcaccgcgtagccgtccattgcggagttatcaaaccccggaacatcaagcggcgaaacgacatcgctcgccagaatacgaccaaaacactgtaccagtggcagcgtttcctgggcggtcagtggggtgacgcgagaaagcatctcattaagcgcggtgtcgagcgacatcaatccggtggtaaattccatgaaaacactcctgcggaggcaaaatcgaatttgcctattatgtcagaaaaacgccacagactgtatgccacctcgggcgtagcgctgggtcctgcctttacatgccatatccatctttctatattcaaaaattgaatgagtaattcataaaaattctgatatttatagcaaaagtggcgaaccacccttaatggacgaatactatgggcaaagcagtcattgcaattcatggtggcgcaggtgcaattagccgcgcgcagatgagtctgcaacaggaattacgctacatcgaggcgttgtctgccattgttgaaaccgggcagaaaatgctggaagcgggcgaaagtgcgctggatgtggtgacggaagcggtgcgtctgctggaagagtgtccactgtttaacgccggaattggcgctgtctttacgcgtgatgaaacccatgaactggacgcctgtgtgatggatggtaacaccctgaaagccggtgcggtggcgggcgttagtcatctgcgtaatccggttcttgccgcccggctggtgatggagcaaagcccgcatgtgatgatgattggcgaaggggcagaaaattttgcgtttgctcgtggcatggagcgcgtctcgccggagattttctccacgtctttgcgttatgaacaactactggcagcgcgcaaggaaggggcaaccgtcctcgaccatagcggtgcgccactggatgaaaaacagaaaatgggcaccgtgggggccgtggcgttggatttagacggcaatttggcggcagccacgtccacaggcggaatgaccaataaattacccggacgagttggcgatagtcccttagtgggtgccggatgctacgccaataacgccagtgtggcggtttcttgtaccggcacgggcgaagtcttcatccgcgcgctggcggcatatgacatcgccgcgttaatggattacggcggattaagtctcgcggaagcctgcgagcgggtagtaatggaaaaactccctgcgcttggcggtagcggtggcttaatcgctatcgaccatgaagggaatgtcgcgctaccgtttaacaccgaaggaatgtatcgcgcctggggctacgcaggcgatacgccaaccaccggtatctaccgtgaaaaaggggacaccgttgccacacagtgatgaacttgatgccggtaatgtgctggcggttgaaaatctgaatattgcctttatgcaggaccagcagaaaatagctgcggtccgcaatctctcttttagtctgcaacgcggtgagacgctggcaattgttggcgaatccggctccggtaagtcagtgactgcgttggcattgatgcgcctgttggaacaggcgggcggtttagtacagtgcgataaaatgctgttgcagcggcgcagtcgcgaagtgattgaacttagcgagcagaacgctgcacaaatgcgccatgttcgcggtgcggatatggcgatgatatttcaggagccgatgacatcgctgaacccggtatttactgtgggtgaacagattgccgaatcaattcgtctgcatcagaacgccagtcgtgaagaagcgatggtcgaggcgaagcggatgctggatcaggtacgcattcctgaggcacaaaccattctttcacgttatccgcatcaactctctggcgggatgcgccagcgagtgatgattgcgatggcgctgtcatgccgcccggcggtgctgattgccgatgagccaaccaccgcgctggatgtcactattcaggcgcagatcctgcaattaatcaaagtattgcaaaaagagatgtcgatgggcgttatctttatcactcacgatatgggcgtggtggcagagattgccgatcgggtactggtgatgtatcagggcgaggcggtggaaacgggtaccgtcgaacagatttttcatgcaccgcaacatccttacacccgtgcgctgttagctgctgttccgcaacttggtgcgatgaaagggttagattatccccgacgtttcccgttgatatcgcttgaacatccagcgaaacaggccccccccatcgagcagaaaacggtggtggatggcgaacctgttttacgagtgcgtaatcttgtcacccgtttccctttgcgcagcggtttgttgaatcgcgtaacgcgggaagtgcatgccgttgagaaagtcagttttgatctctggcctggcgaaacgctatcgctggtgggcgagtctggcagcggtaaatccactaccgggcgggcgttgctgcgcctggtcgaatcgcagggcggcgaaattatctttaacggtcagcgaatcgataccttgtcacccggcaaacttcaggcattacgccgggatattcagtttatttttcaggacccttacgcttcgctggacccacgtcagaccatcggtgattcgattatcgaaccgctgcgtgtacacggtttattgccaggtaaagacgcggctgcacgcgttgcgtggttgctggagcgcgtgggcctgttacctgaacatgcctggcgttacccgcatgagttttccggcggtcagcgccagcgcatctgcattgctcgcgcgttggcattgaatccaaaagtgatcattgccgacgaagccgtttcggcgctggatgtttctattcgcgggcagattatcaacttgttgctcgatctccagcgtgatttcggcattgcgtatctgtttatctcccacgatatggcggtggtagagcggattagtcatcgtgtggcggtgatgtatctcgggcaaattgttgaaattggtccacggcgcgcggtcttcgaaaacccgcagcatccttatacgcgtaaattactggcggcagttccggtcgctgaaccgtcccgacaacgaccgcagcgtgtactgctgtcggacgatcttcccagcaatattcatctgcgtggcgaagaggtggcagccgtctcgttgcaatgcgtcgggccggggcattacgtcgcacaaccacaatcagaatacgcattcatgcgtagataacattcaggcggagaataaaatggcaagagctgtacaccgtagtgggttagtggcgctgggcattgcgacagcgttgatggcatcttgtgcattcgctgccaaagatgtggtggtggcggtaggatcgaatttcaccacgctcgatccgtatgacgcaaatgacacgttatctcaggccgtagcgaaatcgttttaccaggggctgttcggtctggataaagagatgaaactgaaaaacgtgctggcggagagttataccgtttccgatgacggcattacttacaccgtgaaattgcgggaaggcattaaattccaggatggcaccgatttcaacgccgcggcggtgaaagcgaatctggaccgggccagcgatccggcgaatcatcttaaacgctataacctgtataagaatattgctaaaacggaagcgatcgatccgacaacggtaaagattaccctcaaacagccgttctcagcgtttattaatattcttgcccatccggcgaccgcgatgatttcaccggcagcgctggaaaaatatggcaaggagattggtttttatccggtgggaaccggaccgtatgaactggatacctggaatcagaccgattttgtgaaggtgaaaaaattcgcgggttactggcagccaggattgcccaaactggacagcataacctggcgtccggtggcggataacaacacccgcgcggcaatgctgcaaaccggtgaagcgcagtttgctttccccattccttacgagcaggccacactgctggagaaaaacaaaaatatcgagttgatggccagtccgtcaattatgcagcgttatatcagtatgaacgtgacgcaaaagccgttcgataacccgaaggtccgtgaggcgctgaattacgccattaaccgtccggcgctggtgaaagttgcctttgcgggctatgcaacgccagctactggtgtggtaccgccaagtatcgcctacgcgcaaagttataaaccgtggccttacgatccagtgaaagcgcgcgaattactgaaagaggcgggatatcccaacggtttcagtaccacgctgtggtcgtcacataaccacagcaccgcgcagaaagtgctgcaatttacccagcagcagttagcgcaggtcgggattaaagcccaggtgactgcgatggatgccggacagcgggcggcagaagttgaaggtaaagggcaaaaagagagcggcgtgcggatgttctacactggctggtcggcttcaaccggcgaagcggactgggcactatcgccgctgtttgcctcgcagaactggccaccgacgctgtttaataccgcgttttacagcaataaacaggtggatgacttcctggctcaggcactgaaaactaatgatccggcggaaaagacccgcttatataaggcggcgcaggatatcatctggcaagaatcgccgtggatcccgctggtggtagaaaaactggtgtcggcacacagtaaaaacctgaccggtttttggatcatgccagacaccggcttcagctttgaagacgcggatttgcaataagcaacgcagggagtggaatgcttaattacgttatcaaacgcttactggggttgattccgacgctgtttatcgtctcggtgctggtgtttttatttgtccatatgctgcccggcgatccggcgcgattgattgccgggcccgaagctgatgcgcaggttatagaactggtgcgtcagcagctggggttggatcagccgctgtatcaccagttctggcactatatcagcaatgctgtgcagggggattttggcctgtcgatggtgtcgcgtcgtccggttgccgatgagattgccagccgctttatgccaacgctgtggctgaccataaccagtatggtctgggcggttatatttggtatggcggcgggaattatcgccgccgtctggcgtaaccgttggccggatcgattgagtatgaccattgcggtgtcggggatctcgtttccggcatttgctctggggatgcttttaattcaggtattctccgttgaactgggctggctgcctaccgtgggagcagacagttggcagcactacattttaccctccctgacgctcggcgcggcagtggccgccgtgatggcgcgctttacccgcgcgtcgtttgtcgatgttttaagcgaagattatatgcgtaccgcgagggcgaaaggggtgagcgaaacctgggttgtcctcaaacacgggctacgtaacgcgatgatcccggtagtgaccatgatgggcttacagtttggctttttgctcggtggttccatcgttgtggagaaagttttcaactggccgggacttggacgcttactcgttgactccgtagaaatgcgtgattacccggtgattcaggcggaaattctgcttttctcgctggaatttattcttatcaacttagtggtggatgtgctttacgccgccattaacccggctatcaggtacaagtaaggatgcgactatttaactggcgacgtcaggcggtgttaaacgccatgccactggtcaaacctgaccaggtacgtacaccgtggcatgaattctggcgacgatttcgccgtcagcatatggcgatgaccgccgcattattcgttattttattgattgtggtggccatttttgcacgctggatcgctccctatgacgccgaaaattattttgattatgacaatctgaataacggaccttctttgcagcactggtttggcgtcgattcactggggcgtgacattttcagccgtgtcctggttggtgcgcaaatctcgctggcggcgggcgtgtttgccgtgtttatcggtgcggcgatcgggacgttgctgggcttgctcgctggatattatgaaggctggtgggatcggctgatcatgcgcatttgcgatgtgctgtttgccttcccgggtattttactggcgatcgctgttgttgcggtgttgggaagcggcattgctaacgtgattattgcagtcgccattttttccatccccgcgtttgcccgcctggtgcgcggcaacacgctggtgttgaaacagcaaacctttattgagtcagcacgcagtattggtgccagcgatatgaccgttttgttgcgtcatatcctgcctgggaccgtctcttctatcgtggtgtttttcaccatgcgcattggtacctcgattatctctgccgccagcctctcatttctcggcctcggtgcgcagccgccgacaccagagtggggagcaatgctcaatgaggctcgagcggatatggttatcgcgccgcatgtcgctgtttttccggccctggctatttttctgaccgtactggcgttcaatttgttgggcgatggtttacgcgatgcgctggatccgaaaattaaaggatagttacgtttgaatattgcttgaaagggtaatcacctcacaggaaattattgccctaagcaagtgttgtaactttctgctgattttgtagaatcgggtaatttggttaaaaagccgcagcaagggacaatttttgcagcggcacagcgttcagatagttattttgttaaatgtattaacatgctgagtttatacgaaaagataaagataaggctgataattttatttttattggcagcactgtcatttattggtctttttttcatcattaactatcaactggtatcggagcgcgcggtaaaacgtgccgatagccgctttgaacttattcagaaaaacgttggctatttctttaaagatattgaacgttcggccctgacattaaaggactcactgtatttattaaaaaatacagaggagattcaacgcgccgtgattcttaaaatggaaatgatgccatttttagactcggtgggactggtacttgatgataataaatattatcttttttcgcggagggcgaatgataaaatcgttgtttatcatcaggaacaagtaaatggaccgcttgtcgacgagtcagggcgggttatttttgccgattttaacccatcgaaacgaccgtggtcggtggcttcagatgactctaacaacagctggaatccggcatacaattgctttgatcgtccgggtaaaaaatgtatctcttttacgctacacatcaacggcaaagatcacgatttgttagcggtggataaaattcatgtcgatttaaactggcgatatctgaacgagtatcttgatcaaatcagcgctaatgatgaagttctatttttgaaacaaggccatgagatcattgccaagaatcaactcgctcgtgaaaaactgattatttataatagcgaaggtaattataatattattgattctgtcgatactgaatatatcgaaaaaacatcagcggtgccaaacaacgcattattcgaaatctatttttattatcctggcggtaatttattgaacgcatcagataaacttttttatctgccgtttgcgttcattattatcgtattgctggtggtttatttaatgaccactcgtgtgttccgtcggcaattttctgaaatgacagagctggttaatacgctggcgtttttgcctgactcaacggatcaaatcgaggctctgaaaattcgtgaaggcgatgcgaaagagattatcagcatcaaaaattcgatcgcggaaatgaaagatgccgaaattgaacggtcaaataaattgctctcactgatctcttacgatcaggaaagtggttttattaaaaatatggcgattattgagtctaacaataatcagtatctggctgtggggatcatcaaactgtgtggtctggaagccgtggaagcggtgtttggtgttgatgagcgcaataaaatcgtcaggaaattgtgtcagcgaattgccgagaaatatgcgcaatgctgcgatatcgtgacattcaatgccgatctctatttacttctgtgtcgggaaaatgtacagacatttacccgtaaaatagcgatggtaaacgattttgacagcagctttggctaccgcaatctgcgcatccataagtctgccatttgtgaacctttgcagggggaaaacgcctggagttacgcagaaaaactgaaactggcgatttccagtatccgtgaccatatgttctcagagtttattttctgtgatgacgcgaaactcaacgaaatagaagagaatatctggattgcgcgtaatattcgccatgcaatggaaattggcgaactattcctcgtctatcaaccgatcgttgatattaacacccgcgccattctgggcgcggaggcgttgtgccgttgggtgtctgcggagcgggggatcatttcaccgctgaagttcattaccattgctgaagatatcgggtttatcaatgagctgggttatcagattattaaaacggcaatgggtgaattcagacattttagtcagcgtgcgtcgctgaaggatgatttcttactgcatattaatgtttcgccctggcagttaaacgaaccacactttcatgagcgttttaccaccatcatgaaagaaaatggcctgaaggcgaacagcctctgtgttgagatcactgaaaccgtgatcgagcgaattaatgaacatttttatctcaatattgaacaactgcgtaaacaaggggtacggatatcgattgatgactttggcaccggtttgtcaaacctgaaacgtttttatgaaattaatccagacagcataaaggtggactcgcaattcaccggcgatattttcggtactgcgggaaaaattgtgcgcattattttcgacctggcacgctataaccggatcccggtgattgcggaaggcgtagagagcgaagacgttgcgcgcgaattaatcaaattaggatgtgttcaggctcaggggtatctgtaccagaaacccatgccattctccgcctgggataaaagtggaaaattagtaaaagagtagtttacgtatgtccagaatcaataagttcgtacttacagtcagtctgctgatttttatcatgatttcagcagttgcctgcgggatctacactcaaatggtaaaggaacgggtgtatagcctgaaacagtccgttattgatactgcttttgcggtggcaaatattgctgaatatcggcgtagcgtggcaattgatcttatcaacacgctaaatcccacggaggaacagctgttggttggtttgcgcacagcttacgccgactcggtttccccctcttatttgtacgatgtcggtccttatctgatttccagtgacgaatgtattcaggtaaaggagttcgagaaaaattattgtgcagatattatgcaggttgtgaagtatcgacatgtcaaaaatacagggtttatctcttttgacggtaaaaccttcgtctattacctctatccggtaactcacaatcgtagtctgatatttttgcttggtctggagcgtttttctttactgtcaaaatcgctggcgatggacagcgagaacctgatgttctctctatttaagaacggtaaaccggtgaccggtgatgaatataatgctaaaaacgccatcttcaccgtttcggaagcgatggagcacttcgcctatttgccgaccggattgtatgtatttgcgtataaaaaagatgtttatttgcgggtttgtacattgattattttctttgccgcattggtggcagtgatatcgggtgccagttgcctctatctggtacgcagagtgattaatcgtggtattgtggagaaagaagccatcattaataaccattttgaacgcgtactggatggcgggcttttcttttcggctgccgatgtcaaaaaactctacagtatgtataactcggcgttcctggacgacctgaccaaagcaatgggcagaaaatcctttgacgaagatttaaaagcgctgccggaaaaaggcggttatttgtgcctgtttgacgtcgataaattcaaaaacattaacgacaccttcggtcatttgctgggcgatgaagtgttgatgaaagtggtgaaaatccttaaatcacagatcccggtagataaaggtaaagtctaccgcttcggcggtgacgaatttgcggtgatttatacgggtggaacgctggaagagttgctatcgattctaaaagaaatcgttcatttccaggtgggaagcattaatttaagtaccagtatcggtgtagcacattcaaatgaatgtcctaccgtcgaacgcttgaaaatgctggcggatgagcggctgtataagagtaagaaaaacggcagggcacagattagctggcagtaatcattattcgcaggccggacaaatgattttgcccggcctgaattaattaaacccggctaccccacaaatcgtactcatcggcgtgctcgactttcacacgcaggatatcacccggcttaacgttggtttcaccattgagataaaccgcgccgtcgatttccggtgcatctgccatgctgcgaccaatcgcgccttcttcgtccacttcgtcgataatcaccagaatttcacggcccactttctcttgcaggcgctcggcggaaatctgctgctgcagctgcatgaaacggttccagcgttcttctttaacttcttccggaacctggtcaggcagggcattggcgtctgcaccttcaaccgggctgtatttaaagcagccaacgcgatccagacgcgcttctttcaggaagtcgagtagcatctggaaatcttcttctgtctcgccagggaagccgacaataaaggttgagcgtagggtcagttccgggcagatttcgcgccactgtttgatgcgcgccagttggcgatctacagaacccggacgcttcatcagtttgagaatgcgcgggctggcgtgctgcaacggaatgtccagatacggcaggattttgccttctgccatcagtgggatgacgtcgtccacatgcggataagggtaaacgtagtgcagacgtgtccagatccccagtttcgataactgttcgcacaggctgaccatgctggtttttaccggctcgccgttgtggaagccagtacgatgtttaacatcaacgccataggcggaagtatcctgcgagatcaccagaatctctttaacgcccgcatctaccagacgtttcgcttcacttaacacttcgccaatcggacggctcaccaggtcgccgcgcatagacggaataatgcagaaggtgcagcggtgattacagccttcagaaattttcagataggcataatgacgcggcgtcagtttcacaccttgttctggcaccaggctcaggaatgggttgtgtttcggttttggcacgtagtgatgaacgtgctccagaacctgctcatagctatgaggcccggtgatttccagcactttcgggtggacttcgcggatctgatcttcttttgcccccagacaaccggtcacaataaccttgccgttttcattcaacgcttcaccaatggcttccagtgattcttgtaccgcgctgtcaataaagccgcaggtgttgacgatcaccatgtccgcatcgtcatagctcggtaccacgtcataaccttcagtgcggagttcggtgagaatacgctctgaatcaacaaggtttttcggacagccaagggaaacaaagccgattttcggctggggagttactttgctcatagcttaaaaaatattcagttacaggaaaggtcagggcagggattctacagagttctggataaaatttgtatcgcaatctcattcgctggcggaggcgaaggaaatgtaaattttgttaattcggcgtgaagaattgatcctggacagcattttgctcaaaaaatagccatactatttaattgcaacaaggctgggaagaggaggatcgaagtatgttcgttgacagacagcgaatcgatctgctgaaccggttgatcgacgcacgcgttgacctcgccgcatacgtgcaactgaggaaggcaaaaggatacatgtccgtcagcgaaagcaatcatctacgagataacttttttaaactgaatcgcgaactgcacgataaatcgctgcggttgaatcttcatctggatcaggaagagtggagtgctcttcatcatgctgaagaagcattagcgacagccgcagtatgtttgatgagtgggcaccatgattgcccgactgttattaccgtcaacgccgataagcttgaaaattgtctgatgagcttaacgctgagtatccagagcctgcagaagcacgccatgcttgagaaggcctgaaaactaagggggagaaagcgtctcccccttcatgtttaagtttttgtaaaaatgaatttgttatctcctccactgactacgctttaagccagagtcaatccggaggcgttatgcatcgacaatcctttttccttgtgccccttatttgtctttcttccgctctctgggcggctcctgcaacggtaaatgtcgaagtactgcaagacaaactcgaccatccctgggcactggcctttttacccgataatcacggtatgttaatcactctgcgcggcggcgagttgcgtcactggcaagcaggaaaaggattatctgcgccgctttccggagttccggacgtttgggcgcacgggcagggcggcctgctggacgtggttttagcgcctgattttgctcagtctcgccgcatctggttaagttattccgaagttggcgatgatggcaaagccggaactgctgtgggttatggccgcttaagtgatgatctctcaaaagtgaccgacttccgcaccgtctttcgccagatgccaaaactgtctaccggcaaccattttggcgggcggctggtattcgacggtaaaggttatctttttattgctctgggcgaaaacaatcagcgcccgacggcgcaggatctggataaattacagggcaaactggtgcgtctgaccgaccagggcgaaatcccggatgataatccttttataaaggaatccggtgcgcgcgccgagatctggtcttatggcattcgtaatccgcaaggaatggcgatgaatccgtggagtaatgcactgtggctgaatgaacatggcccgcgcggtggtgatgaaattaatatcccgcaaaaaggcaaaaactacggctggccgctggcaacctggggaatcaactattcaggctttaagataccggaagcgaaaggggagatcgtcgccgggaccgagcaacctgttttttactggaaagattcgcccgctgtgagcggcatggccttctataacagcgataaattcccccagtggcagcaaaaattatttattggcgcgctgaaagataaagatgtcattgtgatgagcgtcaacggcgacaaagtgacagaagatggccgtattttaacggacagagggcagcgaattcgtgatgttcgcactggacccgacggttatttatacgttctcaccgacgagtccagtggggaattacttaaagttagcccacgcaattagctaacgggaatcatcaccactttgcgcactgcggggcgttcagtgagttgctgataccagcgttgcagatttggacgcggtgtccaggtcaggccaacgttaaacaaattgtagatgaacggtgcgatagcgatatcgcccacaccaaactcgtcgccagagaaccattttacttttgccagttccgcatcgagcagggcaaacagggcgtcgcactctttgcaactggcatcaatggcggcctgatcgcgctcttccggtggtgttctgactaatcccatcaggatcccgcgatgagcattactgagcgtctggtttgcccagtccatccatttttccgcttccgcacgacgtgccggtgagtcgatccacaggcgtttttgcccgtactgtgccgccagatagcggacaatggcgtttgattcccaaagaatgagatcactttcgtcgtcacgcaacaacggcaccagcccgttagggttcatcgccagaaaatcagcatcgtgatttatcccaaactcacggcccgcgagaatttgctcataaggtagttccagttcttcgagcgtcagcaatactttttttacgttagttgaattattccgaccccacagcgtaatcatactcaccccttttccgacaggcagccacaggctgaacaggactccgatggtgaagtaaagttaacttttaagcaacagctggcaaaaaaatgacaccagaagcagcgaagcggcaggatattgcataaactttaaaaactttaccaacttacggtttctttaagtttgtgtgtgcgttattaatcaccaaacttatcatacggcgatataacgtattttttttgaatggatactcgggtggcatttatgacgcaatactcctctctccttcgtggtcttgcagcgggttctgcatttttattcctttttgccccaacggcattcgcggcggaacaaaccgttgaagcgccgagcgtggatgcgcgtgcatggattttaatggattacgccagcggtaaagtgctggcagaaggcaatgcggatgagaaactggatcccgcgagcctgactaaaatcatgaccagctatgtggttgggcaggcgcttaaggccgataagattaaactcaccgatatggtgacggtcggtaaagatgcctgggcgacgggaaatccggcactgcgtggttcatcggtaatgttcctcaaaccgggcgatcaggtttcggtggcagacttgaacaaaggtgtgattatccagtccggtaatgacgcctgtattgcgctggctgattacgttgccgggagccaggagtcatttattggtctgatgaatggttatgccaaaaaactgggtctgaccaacactaccttccagacggtgcacggcctggatgcgccggggcagttcagcaccgcgcgcgatatggcattgctgggtaaagcattgatccacgatgtgccggaagagtacgccattcataaagagaaagagttcaccttcaacaaaattcgtcagcctaaccgtaaccgtctgctgtggagcagcaatctgaatgttgatggcatgaagacaggaaccacggcaggcgcgggatataatctggttgcttcggctacccagggcgatatgcgtttaatctccgtagtgttgggggcgaaaaccgaccgtatccgttttaatgagtctgagaaattattgacctggggtttccgcttctttgaaaccgtgacgccaattaaacctgatgccacctttgtgactcagcgcgtctggtttggtgataagagcgaagtgaatctcggggcaggtgaagcgggctcagtgaccataccgcgtgggcagctgaaaaacctgaaagcgagttatacgttaacggaaccgcagcttaccgcaccgctgaaaaaaggtcaggttgtcgggaccattgatttccagcttaacggtaaatccattgagcagcgtccgctgatcgtgatggaaaatgtggaagagggcggattctttggtcgggtgtgggatttcgtgatgatgaaattccatcagtggttcggcagctggttctcttaatcttctgataaccggatggcgcgaaacgtcatccggttatacgtcattaatacatcaacttaatgcgctgcgtctgcgcgtacttcacatactcatcttccgggcaacaatcgctcaccacaatatcaaagcgtttcaggtcacccatgcgcgccggacgcaccttgccaaatttactgtggtcgacaaccagcacatgcttttgcgccatcgacatggcccagtgttttaccggcaactcttcaagattaaaacaggtagcgcctttactgacatgcacgcccgccgcagaataaaaagcgatatccgggcaaaaattattcagcgtttgctgaaaatcgatgggtttgaaaatggcgttgctggcgtgaaattcaccaccgcaaagaaacgcgcggcaatggggtttctctttcagcgccagaaaggtatttagcgaataacaaacggcggtaaaagggatttcattatcaatcgcttcaataatccacggcgtggtggtgccacagtcaaaaaagagggtctgatcgggttctaccagcgtcgcagccagttttgccgcccggcgtttttcttccaccaggcgggatttttgatcgcttaacaggtaatggctggcactgcgcggttccagaacaatatagccgccgagcaaaacgacgggcgcactgtggttgttcagatcgcgacgaatcgtcatctccgaaaccccaagcagggcggcggcgtctttaagatgtaacttatcgctgcgttttaattcttgcagcagctgcccgatacgctcttcgcgacgtgtttccataatccctctgaatagttattgaagcgagccgctcaatactacactttttagcagagatcagtcacgcacccagcctttgcggatcggtaatgcaaaacagacgcgataccacgattgcagacgttgatagagtttatgccccatcgcttgccagataatctgggcactaaggcagccaatcatacctgccagcaatccaccgagcatatccagcggccagtggacgccaagataaacgcgcgaccaggcaatgacgacggccagcaccattaaaagtgagccggaccacaggcgatgccagcataaaaatgccagtgcaaaggtgaaaatcaccgtaccgtgatcgcttgggaatgagtcatccgccgcatgatgcaggaagttatagccgatattttcgacaaagggtcggtcgtgcggaaaaagatgtcccatcgtccaggacacaaacaggctgaccgccagcgcgatagcgatttttatcaccagttgccgttgtgctgtaagcccccacaaccaaagtaccacggccagcaacggcaccacggtaatcaaatctttagcaataaaaatcgccaacgagatcatccacggagccgagtctggcgtcgcgttaataagagagaatagagagagattcaaattttccagcataacttcccgacgcaaagtgattaaaagggagccaatacaggcaagtcgttgagaataaagtgcaggttaaactgggtaaagcggcatcgtcttatttccctcaagcggcctgtttacggtgggtgattgtaacgggcataggttaaataaaacttaaagaaagcgtagctatactcgtaataatgtaagaatgtgcttaaccgtggtttcagctacaaaattcgctttctcgttagctgcgcttttattaaactctgcgcgattattattggcgaagaaattgcatgcaaaataaattagcttccggtgccaggcttggacgtcaggcgttacttttccctctctgtctggtgctttacgaattttcaacctatatcggcaacgatatgattcaacccggtatgttggccgtggtggaacaatatcaggcgggcattgattgggttcctacttcgatgaccgcgtatctggcgggcgggatgtttttacaatggctgctggggccgctgtcggatcgtattggtcgccgtccggtgatgctggcgggagtggtgtggtttatcgtcacctgtctggcaatattgctggcgcaaaacattgaacaattcaccctgttgcgcttcttgcagggcataagcctctgtttcattggcgctgtgggatacgccgcaattcaggaatccttcgaagaggcggtttgtatcaagatcaccgcgctgatggcgaacgtggcgctgattgctccgctacttggtccgctggtgggcgcggcgtggatccatgtgctgccctgggaggggatgtttgttttgtttgccgcattggcagcgatctcctttttcggtctgcaacgagccatgcctgaaaccgccacgcgtataggcgagaaactgtcactgaaagaactcggtcgtgactataagctggtgctgaagaacggccgctttgtggcgggggcgctggcgctgggattcgttagtctgccgttgctggcgtggatcgcccagtcgccgattatcatcattaccggcgagcagttgagcagctatgaatatggcttgctgcaagtgcctattttcggggcgttaattgcgggtaacttgctgttagcgcgtctgacctcgcgccgcaccgtacgttcgctgattattatgggcggctggccgattatgattggtctattggtcgctgctgcggcaacggttatctcatcgcacgcgtatttatggatgactgccgggttaagtatttatgctttcggtattggtctggcgaatgcgggactggtgcgattaaccctgtttgccagcgatatgagtaaaggtacggtttctgccgcgatgggaatgctgcaaatgctgatctttaccgttggtattgaaatcagcaaacatgcctggctgaacgggggcaacggactgtttaatctcttcaaccttgtcaacggaattttgtggctgtcgctgatggttatctttttaaaagataaacagatgggaaattctcacgaagggtaaaaaaatgcctgactgctttgtgcgatcaggcattctcgaattaatggtgatggtcgtcaatctggtgttcgataaccatcccttcacctacgctggcaagatggcgaacataaggatgcgggcggtaagccggagctggcgcaggagccacatagacggtttgcggcacagtcgcgacgctgaccgcttgtggaacgctgactgaatcaggaaccacaaccactttgtatccactcggcacatcgacggtgacactttgcgccatcgccacaccagtaaagcccattaaaagcgcgcccaacagtagacaatttttcataatcatttcgcctgaaataatgcagcgggttaatttccgcgaattatgcagccttcattcaggcattgtgttgccgggcgtgctgccggttttattggtcaaatggcgcttcgtgtttaagaactttatcgatcacatccagtacgccttcacggttattggagcctgcgcggtattttgccgctgcgacgaccgcgctaccggcattttccattgcaaaactaaagcctgcctgacgcagcatctcaatatcgttaccgccatcgccaaagaccaccacttcgctgtcgtctattccccataatttctgcagttggcgaaggccattggctttatgtacgccggggataatcagatcgatgctgccgttgccggtgtggaccgacaccataatatcgccgatggcctcatgtaatgctttttgtacttgtggaatcagttcatcggaaagattcaggccaaacttaaagaagatatcctctaagttgtcaaagttatcgacgtattccagacggtgataatacatttccgccaccgttttcatggcatcgtcatattttttgagtgtataggcactattttttccgcaggcaataatttccacttccgggcgcgtcagcaaatgttccacgacagtagcaaacgcatccttcgatagctcgccattaaaaacatctttgccttcgctcactacccagccgccgttttcagccacaaaggcaatttcattagcaatttcagggaagaaagagatcaactgataatattgattcccgctggcgactacaaagcgaattccttgtgctttcatttgctgatactgagccataaaccgctcacggttataggttttttgatcgcttaagaaagtaccatccatgtctaccgcaattaatttaatgctcatcaactattctccatcgccgtctgcgttttggtatcgggtttggcgacggctttcgcgacaatagccgcgagaataaccagcgccagtacaaccagcattgcactacgtaatccataatgttcgccgagatagcccagcagcggcggcccgacgaggaaagccagataaccggtcgttgctaccacactgacgcgggttggtgcatcggggccggtatcgctggcggcagaaatggtcagcgggaagcccagcgaggcacccagtccccagagtacaacagacaccccagcgacccaggcgctatcgacaaaaataatcagcccaatacccaacgcccccattagtgcactggcccgaaccacggcaacgcgactgtaacggtcgatgaaccaaccgccggtgaagcgtccaacggtcatccccagggtaaaaccggcataaatcagcgagccggaagtagggctaaaaccgtgaccgtcaaccattaataagggtaaccagtcgttggcagaaccttcggcaaaggccatcgccagcaccacaacacctatcagcagcaactggatatcgcgataaaaaggtacgcctttttcgccatgctgggtgccatcggcagcatttttgcccgtaccgtcagggattgcctgaatggcgatataaataggtgcgatacctaccagcgccgccaataaaatgtgcaccgttgccggaacgccaaaggccgtcagtgccatcccgacacctgcgcctgccagcgtgcccaggctataaaaaccgtgcatcatcggcaaaaccgtcttattcatttctcgctcaacggcagcaccttcaacgtttatcgccacttccgcagaaccaaaacttgccccaaagacgccgagaccaacggcaaagagcaggggcgatgtcagccagagtgccagacttaatatcatcatcccgatcaatgcgcaggacatcgtgaccaggatgacattacgtgtcccaaagcgtttcactaaccacgccgagcagagaataccgctcatcgaaccgatcgacagaccaaagagaacaccgcccatttcagcgatcgagacagagagaatatcgcggatagcaggcgtacgggttgcccaggacgccattaacaggcctggcaaaaagaagaacataaacagcgcccaggttcggcgtttcaatgcattacgtgaagaatttacggtcatagatcacgtcaaaataagaagagggaagacaacattagcaaggttgtgtacatttgtacacaattgcagagagaggaaatgacatgcgtcgcgctaacgatccgcaacggcgagaaaaaattatccaggccacgctggaggcggtgaaactttacggaatacatgctgttacgcaccgcaaaattgctacccttgccggggtaccgttgggatcgatgacctactatttttcaggaattgatgagttgttactggaggcgttcagcagttttactgagatcatgtcccggcaatatcaggcattttttagcgatgttagtgatgctccgggcgcatgccaggctatcaccgatatgatctacagctcacaggttgcaacgccggataacatggagctgatgtaccagctctacgcgctggctagccgaaaaccgctattaaaaacggtaatgcaaaactggatgcagcgcagtcagcaaacgctcgaacaatggtttgaacccggaaccgcccgcgcgcttgatgcgtttattgaggggatgacgctgcattttgtcaccgaccgtaagccgctatcgcgcgaggagattttgaggatggttgagagggttgcagggtagtagataagttttagataacaaaaaacccatcaaccttgaaccgaaatggcggggttgatgggctccacaaaatggggacatcaaagaaaagcagtggcactaattaagactgatgccctgcggaaaagttctgcggttgtgcaaaaaaatttcattttcagggcaacttcagttttatcctaatcctggccataccatgacgatgattgtccctgccagcgtcagcaggacgttggcgattgcataggtgcccgcatagcccagcgccgggatgttactgcgagctgtatcactgatgatctccattgccggcgcgcaggtacgtgcgcccatcattgcgccgaacaacagcgcgcggttcattcgcaatacataagcaccgaacaagaaacagataaccacgggcaccagactgacaatcaatccggcaatcaacatctgaccgccaatcgcgcccaggccgttattaataccgctaccggcgctcagaccaacgcctgccataaacaccatcaagccgaactctttcaccatgcttaatgcaccctgcggaatgtaaccgaaggtcgggtggttagcacgcataaagcccagcataattccggcgaataacaacccggcagcgttccccatgccgaaactgaatgtgctgaactggaaggtgatcatcccgatcatcagcccaataacaaagaaggcgcagaatgccagcaggtcagtgacctggctgtgaatcgagataaagccgatgcgatcggcgatggtttttacgcggcgggcatcgccgctgacttgtaaaacgtcacctttgttaagcacgacgttgtcatctatcggcatctcaatctggctacgaatgacgcggttaaggaagcaaccgtgatcggtcaacttcagttgtgcgagacgtttacctacagcgttatggtttttaacgaccacttcttcagtgacgatacgcatgtcgagaaggtcacgatcgaaaacttctttaccgttacggaagctgggatcgagtcgggcatgggcgtcgggatagcctaccaacgctatttcatcgcccatttgtagcacggcatcaccgtctggatttgccagaatcccgttacgtcgaatacgttcaatgtagcagccggtttgtcgataaatacccagttcacgcagatttttgccgtcggtccaggccaccagttccgggccgacgcgataggcgcggatcaccggtaaataaaccttacggttggcatcagtgtccaggccacgttcgcgggcgatttgctgggcgctggtctgtaagtcctgatgctgcaatttcggcaagtaacgcgcaccaacaatcaaactcaccagaccgattaaataggttaaggcatacccgaggctcagattatccagtgccagtgagagctgcctgctttccatgccggaatgacgcagtgtatcgccagcaccgaccagaaccggtgtcgacgtcatagagcctgctaacataccggccgtcaggccaatatcccagccaaacagcttacctaaccctaaggcgatcaccagcgcactgccaaccatcaccagtgctaacattaggtaatttttcccatcgcgaaaaaaaatggaaaaaaagttcggtccggcttcgaccccgacgcagaaaataaacagcataaagccaagattaagcgcatcggtgttaatgctgaaatgttgttggcctaataacagcgatacgactaaaacgccaatggaattacccagttggatcgaaccaagtcgtaactttccgagacatagcccaagcgcgaggaccacaaataataacagaatgtaattcccatttaacaattcggcgacgtttatattcacggaggctaacttcttgtttactagtaagctgttgaaagaaatggtaatttacgataatgttttttaccagaattcagggcgcagattcattcagcgcacctaaacgatagtaaagtaacaatatattttactagtgtaatcacattaggtatcaacggctatatgaattgcgttggcctatattagcatggaatgcgaagcggctttatcttactgaacgccacactggcgaaaaatgtgttcgatagacgcagtgtcaggaggaacgagtgaaacataaacaacgttgggcgggggcaatctgctgttttgtcctcttcattgtggtgtgcctttttctggcgacgcacatgaaaggcgcttttcgggctgccgggcatcctgaaatcggcttgctatttttcattcttcctggagcagtcgccagcttcttttcacagcgtagagaagtcctgaaacctctgtttggcgcaatgctggcggcaccctgttcgatgctcattatgcggctgtttttttcaccgacgcgctcattctggcaagagctggcatggttactaagcgcggtgttctggtgtgcgctgggggcactgtgtttcttatttatcagtagtttgtttaaaccacagcacagaaaaaatcagtaaagccctcaacgcgagggcttgtcagacgatcaggcgtccagattttctttcacccatgcagcaaaatcggtatagccgccgatatgttgctgatcgacaaaaatctgcggcacggtttctacgggtttacctgccttttgttgtagatcttctttagtgatcccttccgcacgaatatctacatactgatactgaaaatcatcgcgttcattgctcaatttctcagccagatcttttgcacgcacacagtaagggcaacccgaacgaccaaaaataacggtttgcattatttctctcctcatagatttatgcctgtaatgatcacgctaaaatgtattcgctgaaagtaggtttaacctgttgcattaattgctaaaagctataactgttaaacacaatacagtgaaaagttttagactgaaggctcactttgcagagggaagcgtatgcgcgcgatcggtaaattgcctaaaggcgtgttgatactggaatttatcggaatgatgctactggcggtggcgctgctgtcggtaagcgactccctgtcgctgcctgagccattttctcggccagaagtgcagattctgatgatttttctcggtgttttgctcatgcttcccgctgcggtggtggttattcttcaggtggcaaaacgtcttgccccacagctgatgaaccgtccaccgcaatattcacgttcagaaagagaaaaagataatgacgccaaccattgaacttatttgtggccatcgctccattcgccatttcactgatgaacccatttccgaagcgcagcgtgaggcgattattaacagcgcccgtgcgacgtccagttccagttttttgcagtgcagtagcattattcgcattaccgacaaagcgttacgtgaagaactggtgacgctgaccggcgggcaaaaacacgtagcgcaagcggcggagttctgggtgttctgtgccgactttaaccgccatttacagatctgtccggatgctcagctcggcctggcggaacaactgttgctcggtgtcgttgatacggcaatgatggcgcagaatgcattaatcgcagcggaatcgctgggattgggcggggtatatatcggcggcctgcgcaataatattgaagcggtgacgaaactgcttaaattaccgcagcatgttctgccgctgtttgggctgtgccttggctggcctgcggataatccggatcttaagccgcgtttaccggcctccattttggtgcatgaaaacagctatcaaccgctggataaaggcgcactggcgcagtatgacgagcaactggcggaatattacctcacccgtggcagcaataatcgccgggatacctggagcgatcatatccgccgaacaatcattaaagaaagccgcccatttattctggattatttgcacaaacagggttgggcgacgcgctaaaaccgccacgtcgatgtatgatacgcgggcttttgaccaggtctgacagagaggtgcagggtgaaaattgccatattgtcccgggatggaacgctctattcgtgtaagcggctgcgtgaagccgctatacagcgcggtcacctggttgaaattcttgatccgctttcttgctacatgaacataaatcctgcggcgtcttctattcactacaaaggccgcaagttaccccattttgacgcagtgatcccgcgtattggcaccgccattaccttttatgggacggcggcactgcgccagttcgagatgctggggagctatccgctcaatgagtcggtcgccattgcccgggcgcgtgacaaattgcgttccatgcaactgctggcgcgtcagggcatcgacctgcctgtcacgggcattgcgcattcgccggatgataccagcgatttaatcgacatggtcggtggtgcgccgctggtggtcaagttggttgaaggcacgcagggaattggcgtcgtgctggcggagacgcgtcaggcggcggaaagcgtgattgacgctttccgcggtctgaacgcgcatattctggtgcaggaatatatcaaagaggcgcaagggtgcgatatccgctgtctggttgttggcgatgaagtggtcgctgcgattgaacggcgggcgaaagagggcgattttcgttccaatttgcatcgtggcggcgcggcaagcgtcgccagtatcacaccacaggagcgtgaaatcgcgataaaagccgcgcgaacgatggcgctggacgttgctggtgtggatattctgcgtgctaatcgcgggccgttggtgatggaggtgaatgcgtcgccggggctggaaggaatagaaaaaaccaccggtatcgacatcgcgggtaaaatgatccgctggatcgaacgccacgctacgacagaatattgcctgaaaacgggtggttagtcgcaatcacattactgatcatggttttgcctgcgctttttgcgtaagctgtgccggtctttttatcgaaagaggttgtacaaaattatgacatcgctggtcgttcctggtctggatacgctgcgtcaatggctcgatgacctggggatgagtttttttgaatgtgataactgtcaggctctgcatctgccccatatgcagaatttcgacggtgtctttgatgccaaaatcgatctgatcgataacacgatcctgttttctgccatggcggaagtccgaccttcagccgtattgccgctggcggcggatttatctgccatcaatgccagttcgctgaccgtgaaagcatttcttgatatgcaggatgataatctgccaaagctggtggtttgccagtctttatccgttatgcagggcgtaacctatgagcagtttgcatggttcgtgcgtcagagcgaagagcagatttcgatggtcattcttgaagctaatgcccatcaactgctgttaccgactgatgatgaagggcaaaacaacgttaccgaaaactatttcctccactgataactcctttcgagcacgcagtcgctggtgcagtggctgcgcgctgcaaaattatctgctgtttttaaccttttcttaaagattatttcacttctcttgtgtcgatttggctttatcacatagagcaaatatgcataaaaatttgttaaataccgttttttaatccgagctatagtctcaaaccctggctaaagttattcttgcgatgcttttatatagcgagcagtgctggccgggagaaagttctcttttcttacaccgcgccgataaaaaatatgcacgtttattgcatatctttcagtgtgacaacttttgttcgtttgttaacgaactttcagaaggaaagagatatgaccgccttaaataaaaaatggctatcgggtctggttgcgggtgctctgatggccgtctctgtcggcacgctcgcggctgaacaaaaaacactccacatttataactggtctgattatatcgccccggacacggtggccaattttgaaaaagaaaccggtattaaagtcgtctacgatgttttcgactctaacgaagtactggaaggcaaattaatggccgggagtaccggctttgatctggtggttccatctgccagctttctggagcgccagttgactgcgggagttttccagccgctggacaaaagcaaattgccggagtggaagaatctcgacccggaactgctgaagctggtcgccaaacacgatcccgacaataaatttgctatgccctatatgtgggcgacgaccgggattggctataacgttgataaagttaaagcggtgctgggcgaaaacgcgcccgtcgatagctgggacttgatcctcaaacctgaaaatctggaaaaactgaaaagctgcggtgtctctttcctggatgcgccagaagaagtttttgctaccgtgttgaattatctcggcaaagatcccaacagcactaaagcggatgattacaccggaccggcaacagatctgctgttaaagctgcgcccgaacattcgttatttccattcatctcaatacattaacgacctggcaaacggcgatatttgcgtcgctatcggctgggcaggtgatgtctggcaggcgtcaaaccgcgcgaaggaagcgaagaatggcgtgaatgtctcgttctcgattccaaaagaaggggcgatggcgttctttgatgtattcgccatgcctgcggatgccaaaaacaaagacgaagcctatcagttcctgaattacctgctgcgcccggatgtagtagcgcatatttccgaccatgtgttctatgccaacgccaataaagcagccacgccgctggtgagtgcggaagtccgtgagaacccaggtatttatccgcctgcggatgttcgtgcgaagctgttcactctgaaagtgcaggatccgaaaatcgaccgtgtgcgcacccgcgcgtggaccaaagtgaagagcggaaaataatccgcagtcgtagatgccggaggggcgcaccacacccgccggcaattcgcaccattatggtgcgcttgcacacattcaatgccggagagcagccgtgaatgacgctatccctcgcccgcaggcgaaaacccgtaaggcgctgacgccgctattagaaatccgcaacctgaccaaatcctacgatggtcaacatgcggtggatgatgtcagcctgaccatctacaaaggtgaaatcttcgcgctgctgggcgcatccggctgtggcaagtccacgctgctgcgtatgctggcaggtttcgaacaaccttctgccggacagataatgcttgatggcgtcgatttgtcacaggttccgccttacctgcgccccatcaatatgatgtttcagtcttacgcgctgtttccgcatatgaccgtggaacagaacatcgcttttggcctgaaacaggacaaactaccgaaagcggaaattgccagccgggtcaatgagatgctcggcctggtgcatatgcaggagttcgccaaacgcaaaccgcatcagctttccggtggtcagcgacaacgtgtggccctggcccgaagccttgcgaagcgcccgaaactattactgctcgatgagccgatgggcgcgctggataaaaagctgcgtgacaggatgcagcttgaagtggtggatattctggagcgcgtcggtgtgacttgtgtgatggtcacccacgatcaggaagaggcgatgaccatggcggggcgcatcgccattatgaatcgtgggaaatttgtccagattggcgaaccggaagagatctacgagcatccgactacccgctatagcgccgaatttattggctcggtaaacgtctttgaaggcgtactcaaagagcgtcaggaagatggcctggtgcttgattcgccggggctggtgcatccactgaaagtcgacgcggatgcctcggtggtcgataacgtgccggtacatgtggcgctgcgcccggaaaaaatcatgctttgcgaagagccgcccgccaatggttgtaacttcgcggtgggggaggtgatacacattgcctatctcggcgatctttcggtgtatcacgttcgtctgaaaagtgggcagatgattagcgcccagctacaaaacgcccatcgtcatcgtaaagggttaccgacctggggcgacgaagtgcgtttgtgctgggaagtggacagctgtgtggtgctgacggtttaaggagcaaagatgagtacacttgaacctgctgcccagtcgaaaccgccgggcggatttaagctgtggttgtcgcagctgcaaatgaagcatgggcgcaaactggtcattgcgttgccatatatctggttgatcttgctgtttctgctgccatttctgattgtctttaaaataagcctggcggagatggcgcgcgctattccaccttataccgaactgatggagtgggctgacgggcaactgtccatcactcttaatctcggtaattttctgcaactgaccgacgatccgctctatttcgatgcttatctccagtcgctacaggtggctgcgatttcgacattttgctgtttactgatcggctatccgctggcgtgggcggtggcgcacagtaagccttcgacccgtaatattttattactactggtgatcctgccgtcgtggacctcgtttctgatccgcgtttatgcctggatgggaatattaaaaaacaacggtgtgctgaataattttctgctgtggctgggggttatcgatcaaccgctgaccattctgcataccaatctggccgtttatatcggcattgtttacgcttacgtgccgtttatggtactgccgatttataccgcgttgattcgtattgattattcgctggtggaagcagcgctggatctcggtgcacgaccgctgaaaacgttctttactgtgatcgtgccgctgactaaaggtgggattattgccggatcgatgctggtgtttatcccggctgtgggcgagtttgtgatcccggaactgctcggtggcccggacagcatcatgatcgggcgcgtgctatggcaagagtttttcaataaccgcgactggccggtggcctcggcggtagcgatcatcatgttgctgctgctaattgtgccgataatgtggttccacaaacaccagcaaaaaagcgtgggagaacacggatgaataatttaccggtagttcgttcgccctggcggattgtgattttgctgctgggctttacctttctctacgcgccaatgctgatgctggttatctattcgtttaacagctcgaagctggtgacggtgtgggccggctggtcaacgcgctggtatggtgagttattgcgcgatgacgcgatgatgagtgcggttggtttaagtctgacaattgcggcctgtgcggcgacggcggcggcgatcctcggaactattgcggcggtggtgctggtgcgctttggcaggtttcgcggatcaaatggctttgcctttatgatcaccgcgccgctggtaatgccagatgtcatcacgggcttgtcgctgttgttattattcgtcgcgcttgctcatgccattggctggcctgcggaccgcggtatgctcaccatctggctggcgcatgtcactttttgtacggcttatgtggcggtcgttatttcttcaagattgcgggaactggatcgctcgatagaagaagcagcgatggatctcggtgcgacgccgctgaaagtgtttttcgtcattacgctaccgatgatcatgcccgcgatcatttctggctggttactggcttttactttgtcgcttgatgatctggtgatcgccagctttgtttccgggccgggagccaccacgttaccgatgctggtcttttccagcgtgcggatgggggtgaatccggaaatcaacgccctggcaacattgatcctcggcgcggtcggaattgtcggatttatcgcctggtatctgatggctcgcgcagaaaaacagcggatacgcgacatccagcgtgcaagacgtggctgaagacactaaaatttgccaacctggctacataatgccgcgcatgtcgcggcattgttttcatggaagacgaaacgttgggattttttaagaaaacatcttcatctcatgctcgcctgaatgtgcctgcgctggtgcaggtggcggcgctcgccattattatgatccgtggcctcgacgtgctgatgattttcaatacgctgggcgtgcgcggtattggcgagttcattcatcgcagcgtacaaacctggagtttaacgctggtctttttaagcagtctggtgctggttttcattgagatctggtgtgcgttttcactggtgaaagggcgtcgctgggcgcgctggctatatctgctgacacaaatcaccgccgcaagttacttgtgggcggcttcgctggggtacggttatccggagctgttcagcattcccggtgaatcaaaacgtgaaatcttccatagcctgatgctgcagaagctgccggatatgctcatcctgatgctgctgttcgttccctcgaccagtcggcggttcttccagttgcaataatgtgtataatcgtcgcccctgatgatgtgaaggtcaatgtatgcagtgcgcactttacgacgcgggtcgctgtcgttcctgtcagtggataatgcagccgattccagagcaactctccgctaaaaccgccgatcttaaaaatctgctcgccgactttccggttgaggaatggtgcgcgccggtgtcaggcccggaacaagggtttcgtaataaagccaaaatggtggtgagtggtagcgttgaaaaaccactgctcggtatgctgcatcgcgatggcacaccagaagacctttgtgactgcccgctttatcctgcctcatttgcgcccgtttttgcggcgctaaaaccgtttatcgcccgagcggggttaacgccctacaacgtggcgcgtaagcgtggcgaactgaaatacattctgctgactgaaagccagagtgatggaggcatgatgctgcgctttgtactgcgttctgataccaagctggcgcaactgcgtaaggcgctgccgtggttacacgaacaactaccgcagctgaaagttattaccgtcaatattcagccggtacatatggcgattatggaaggggagacggagatctacctgaccgaacaacaggcactggcggagcgttttaatgacgtaccgctgtggatccgtccgcaaagtttcttccagactaatccggcggtcgccagccagttgtacgccaccgcgcgcgactgggtacgacagctgccggttaaacatatgtgggatctgttctgcggtgtggggggctttggtttacactgcgcgacgcctgacatgcagttaaccgggatcgaaattgcatcagaggccattgcctgtgcaaagcagtcagccgctgaactgggcttaacgcgtttgcaatttcaggcgctggactccactcagtttgccaccgctcagggggatgtgccggagctggtgctggttaacccgccgcgccgcggcattggtaaaccgctgtgtgattatctctcaacgatggcaccgcgttttatcatctactccagctgtaacgcccaaactatggcgaaagatatccgcgaactgcctgggtttcgtattgaacgggtgcagcttttcgatatgttcccgcataccgcgcactatgaagtgctgacgctgctggtgaagcaataaaaaagccgcatgtgcggcttcagattgctgacaaagtgcgcgttgtttatgccggatgcggcgtaaacgccttatccggcctacaaaagcgtgcaaattcaatacattgcatgggccatgtaggcctgataagcgtagcgcatcaggcaattttacctttgtcatcagtctcaagccgcggttgcggctttctgaatcttactgtgggaaccactggtcactgattttttgataagtaccgtcagctttaattgctgccagcgcgttattcagtttttccagcagggctttgttatccggacgtacagcgatgcccaggccggtgccaaaatattgcggatcggtcactttctcagtagcaacaccaagttgtggattggttttcagccattcgtttaccaccgctgtgtcaccaaataccccatcaatacgaccatttttcagatcgataaaggcattctgataactgtcataagagacagttttcacttccgggtgctgatcctgaatatatttctggtgcgtagtaccgttttccatcccaatacgtttgcctttcagatcggcaaacgttttgtaggtatcttttttggcaatcacgacggctgagttttcatagtagggcgtggtaaacgatacctgtttgctacgctccggggtgatatccataccggagattacggcgtcatattttctgaatttcagggacgggatcaggctgtcgaacgcgtgattagtaaaagtacattctgcctgcatttgtttgcacaaggcttttgccagatcgatatcaaagccgacaatctcattattagcacctatagattcaaagggtggataggtggctgaaacgccaaaattgattttctctgcggcagaagcaccgaaagtaaaggaagcaagtaaagcggcaagaactaactttttcatgatggaactcccgtctgtcaatcttatgatttttggccgtgtctgcggcatgggataacaatgccatcaagtgaatttatatgcaataaacatgattaaataatttaaatgaaataaaaaagacggacaacttagtgggttgtccgtcttcattataagaatttatgcactatgtaggccggataaggcgtccccgccgcatccggcacaggcaccgtgctgatgtctgatgcgacgctggcgcgtcttatcagacctacaaaaccccccggcgaatgtacgcagccacattaatttcgccgttcgaatgccagcgctttgcgctcgatcagacgcatcatcagcgtcagcaggccgttaacgaccaggtaaataatccctgccgcaccgaacaccattacatcgtaggtgcgtccgtacaacaactggctgtatcccatcacttccatcagcgtaatggtgtatgccagagaggtacttttgaataccagcaccacttcgttggaataagaagagagcgagcgtttaaaggcatacggcagcaggatcgccagcgtatcttttttgctcattcccagggcgctacaggactgccactgaccttccgggatcgcacgaattgcaccgtaaaacagctgcgtggtatacgccgcactattcagcgacaacgcaatcagcgcacataaccacggttctgacaacaaatgccacagtgccggatactcctgcaaagtcggaaactggcccggcccgtaataaatcaggaagatctgcaccagcagcggcgtaccggtaaacagcgtgatataaccccgcaccagccacaccagcaccggcgttttcagcgtcaggatgatggtaaaaatcaatgccagaatcagtgccacaatcagcgaggcaacggttagcgtcaggctggtgtgtagccctttcatcagttcgggtaaatactcaaacattagctgggcctccgctcaaaacgtgtcgcgcgcaggtcaatgcgtttgagaatgtactgactgagcagggtgatcaccaggtaaatcgccgccgccacaatgtaccaggtaaatggttcctgggtacgagtagcgatgctttttgtttgcagcattaaatcattcacactaatcaaactgaccagcgcggtatctttcagcagcaccagccactggttaccgaggccaggcagcgcatgacgccacatctgcggcatcaccagacggaaaaagatagccgatttcgacagccccagcgcctgaccagactcccactgacccaccggcaccgctttcaacgcgccccgaagcgtttgcgaggcataggcggcatacagcagtgacagagcgatgacaccacaaaggaacgggctaacgtcgaagttctcaatgtccatctgcactgggatctgcacgaacccaagattgatagtgaagccatccgaaagcgtcagcagcagctgcgaggagccaaaatagataaacagcaccaccagaatttctggcaggccacgcagaatggttaccagcgctgaacctgcccacgcgacaggacgccattttgccgactcccataccgcaaagaacatcgccagcgccagcccgacaatcaatgcacaaacggcaaggccgacggtcatcccggcggcgcttgctaaaggaaaaaattcattcatcaggaattacttctggaaccatttgttgtagatggtttcgtaagtgccatctttcttcactttttccagcgcagtgttgagtttctgctgcagctcagtgttgccctgacgtaccgcgatgccgaggccagtgccgaagtaatctttatcggtcactttgtcgcccaccgccgccagtttcgggttatctttcagccactcagtgaccactgcggtgtcaccgaagacgccgtcgatacgcccgttttgcagatccagttttgcgttctggtagctgtcatacggaacggtagtgatttccgggtgcttatccataatgaatttctggtgtgtcgtcccgttctgtacgccgacttttttgcctttcagctgatcaacactggtgtatttgccttgctgacccacaaacagggcagagttgtcatagtacggggtggtaaacagcacctgcttttcacgctccggagtgatatccatgcccgccatcacggcttctacgcgacggaatttcaggcttgggatcaggctgtcaaacgcctggttagagaaagtgcaggttgcatcaatctctttacacagcgcttgtgccaggtcgacgtcaaaaccaacgatctggttgtttgcatcaatcgattcaaacggaggataggaggcttcggtagcaaaacgaatggtttcggcagctgtggcggaaagactaaaacctgcaattaacgcggcaatcagaacttttttcattgttgttatcccgaatcttagtgagagagatagtttttaaatgcttcggtttgcggctcggtaaagcagctcgcgtcgccttgttctacgatatgaccattttccatatacaccactcggctggcggttttacgcgccacttcaacttcgtgggtgacgatcacctgggtaatattcgtttctgccagctcacgaatgatgctgacgatttgtgccgtaatttccgggtccagtgcggcggtcggttcatcgaacagcagtacctgcggttccatcatcaacgcacgggcaatagcaacacgctgctgctgaccaccagaaagatgcagcgggtaacgatcgctataaggtttgagacgcagacgttccagcagtttttctgcacgggccagcgcctgatctttactcaaccccagtacacggcagggcgcttcaatcaggttttgctgcacggtcagatgcggccacaggttgtattgctgaaacaccatgccaacgttacgacgcaaatcgcgaatcgctttgtcagagggtgttttggtgaaatcgaaatggttgcctgcaatgttgagcgtaccggagcgcggcatctcaagcagattgagtacacgcagcagcgagcttttacccgcgccgctggggccaagtaacaccagcgtttcgccctgtgggcaatccagcgtgatatcgaacagcgcctgatgcgcgccgtagaagcaattaatgccgtttaattgaatactcattgacactcgtatactggcagtctgatagctattgaggtcgaagatagtacctttgacagaataattatgcaatatttctgctttaaaagttaaaagcaaagcgcattattcaataaacatagcacaaaataacgggggcggtggtcggcgagcataaatgtcggcattcctcacgaaatgccggacaatttacggggtttattggttgatcaaggcgttagcgattctcgatggactgacggagcgtacccgccgtggcatgaacgctaccgcctaagtaacgcacatcgtcgatgacccaacactggccttcctgaatcattaacacttcatcctgccaaccctggtcaccctgtttgagatccacgcgcaatggaatgttacgggcatcacgattagggatagtcgatgcactggcaacgtgggcgctatctggcaaggtggttcgactggagaatggatcgttggtcagtagttcccgatggttattatcccgggaggcatcgctaagcagtgtcgccagtttgtcgctcagataagggcgcaaggcggtgatgtcgttgctgcggtgcaaaatgcggtagtcataaaattgctgggccacgttatccgggcctccttcaacgcaaggaccactgcgtgtgccgttatctttataagctggagtgactgtggtgcaggcactgaggagcagtgcgcaggggataagcattgtcaatttgctgtagcgcataatgatttccttataagcgatcgctctgaaagcgttctacgataataatgatatcctttcaataatagcgtatcagtctgataatgcttttgagatcgaaggcttagcaaacaaggagatcgatcatgcaattttctacaaccccaactctggaaggccagaccatcgttgaatattgcggtgtggtgaccggcgaagcgattttaggtgccaatattttccgtgatttctttgccggtatccgcgatatcgttggcggacgttccggtgcgtatgaaaaagaactgcgtaaagcacgggagatcgcctttgaggaattaggctcccaggcgcgggcgctgggggccgatgccgtcgtcggtattgatatcgactacgaaacggtcgggcaaaacggcagtatgctgatggttagcgtcagcggtacggcggtgaaaacgcgtcgatgagaagattcttctggctggtcgctgccgctctgttattggcagggtgtgcaggcgaaaaaggcattgtcgagaaagagggatatcagcttgatacccgacgccaggcgcaggcggcgtatccgcgcattaaagtgctggtgatccactacaccgcagatgattttgatagctcgctggcgacactgaccgataagcaggtcagctcgcattatctggtccctgcggtaccaccgcgatacaacggtaaaccgcgcatctggcaactggtgccggaacaagaactggcctggcatgcggggattagcgcctggcgcggggcaacgcgccttaacgacacctctattggcattgagctggaaaaccgtggctggcaaaaatcggccggagtgaaatattttgccccgtttgaaccggcacagattcaggcgcttattccactggcgaaagatattattgcccgttatcacatcaagccggaaaacgtagtggcacatgcggatatcgcaccgcagcgcaaagacgatccggggccattatttccctggcagcaactggcgcagcaggggattggtgcctggccggatgcgcagcgggttaacttttaccttgccgggcgcgcgccgcacacaccggtagataccgcgtcattgctggagcttttggcgcgctacggttatgacgttaaacctgatatgacaccgcgcgagcagcggcgcgtgattatggcattccagatgcatttccgcccgacgttatataacggcgaagcggatgcagaaactcaggcgattgccgaagcattgctggagaaatacgggcaggattagcgcggcagttttccgtggtcgcgtagccaggcggcagttttctcgataccttcatccagggtgatgaccggctgataacctaactcttcctgcgcacgcgtaatatccagcgtaaagtcaaaattcaacttggagacgccgtagtgggtcagcggcggctcttttgctgacttgcggcctaaacgctccatgctgcgggcgatcatatccagcatcgggtaggggacggaacgaatacgacagtcaatattcaactcgtcgatcagcttctgcacgatgctgcgcagtgtgcgatgctcgccgttggtgatgttgtacacacgcccggaaggtagcttatcgcaggcttcctggcttgccagccacattgcgtgcacggcattttcatagtaggtcatatcgaccagcgcactgccgccatgcggtaacagaatactgccgtagtggtgcatcatatgcgccagacggggaataaagactttatcgtgcggtccgaacagactttgtgggcgcagaatagtaaagcgcgtttgtggattcgcctgcgaaagcatattgatcacttcttcgctggctgctttgctgcgggcaaactcgttggcgaagcggtgagggcgaaaatcttctttaatatcgcgatggtggtgataatcgaagtacagggagggggaagagatatgaataaagttacgcacaccccaggcgacagcccattcacccaggcggcgagtggcgcgaacgttagccagatcgaaagcctgttgtgtcccccagggtgaggtaaagctggagcagtgccacagcgtatcaatgcccgcgagcatcactttagcttgtgatgaaaccagctcggtcagatccgccggaacaaactctgcgcccattttttccagcaatttgcccattgcctcgttgcgaccggtcgctcgcacgctgatgcctttctggcataaaaactctaccgcgtttcgacctaagccgctggtggcgccggtaaccagtaccttcatatcaatccactgttgttgagaaaataacgtgcgcattcttccgtgatttcccccatgatgcaatgggaaacatgaaagaataacgcaggttttgtcgattaatctgtgctttgttctgccagtctggcgatttgttttgccattccgcgaaaaataaacagatgcgcggggatcatcaataaccagtaaaacagccccggcataccgtgcggatgccagaaagcgcggacatcgatagtacgatagtcgcctttatcttccaggctaaaacacagtcgtcccagccccggcgctttcatgccaaataacaacgtaagttgtttttccggttcaacgacaatcactttccagctatccaccgcatcgccagtctgtaaatattcgcgctccgggcggcctttcgccagcttatgaccgatcgcgcggtccatcaacgcccgtgtctgccacaaaatattgccaaagaaataacgctctttaccgccgatttggttcactacctgccataaagcagcaaggctggcggacgttttaacggtaaaccccgcctgtttggcaaaataaccgtactccggtcgccagcgggcaaaggcctgagcgtcgtagccccagtcgctggagttgaccagtttttcctcctctttcaacgtgctacgtaccgcgtcatcgaaagcgatcagccgttgtgggatgagtgcacgtagcgcggtatcatccgccagcagatcgtgtttcagcccctgaatcaacgccctggcggtggtgggcggtacggaagtaatcacattgagaaaccacaccgaaatccagcgggtggggagggggatggggatcaaccagcggcgcttaccgctcaccgccataaaatgttcaaactgttgctgataactgagcacctctggtccggcggcttcgaagatgcggtgttcgctggccggatgatctaacaacgcaaccagatagtgcagcaagttttccagcgcaatgggcgtggtgcgtgaacgaacccagcgcggaggcgttaagactggcaggttgtagaccatatcgcgcatgacttcgaacgccgcggaacctgcgccaacgataattccggcccgcagttcggtcacgggtacattcgcttcacgcagaatgtccgccgtagcctgacgagcacgcagatgatccgactgctcatgtggcggggcctgcaacgaactaagaaagattaattgcttaactggtacttcacgtagcgcatcgcggacgttgagagccacctggcgctcctgagcgataaaatcgccgccttcgcccatgctgtgcaccagaaaatagaccgtatcgatatcctgcaacagggccggtaggttatccggccagctgagatcgactttatggcaactgacgtttgccagttgcagctttgcaagcctgtcgacatgacgtgccgccgccaggatctgatgcccttgctggctgagtgtgcgcaccagatgctgaccaatgtagccactggcaccgagaactaaaatgcgttgcggcacgtctctctccttaacgcgccaggaatgcacgccagtgggcggcgacttccgccagttgttcgcgcgagacgtcaagatgcgtcaccaggcggacaatcggcgaggcgttaatcagcacgtttctcgctttcatgtattcgcctaacgcggcagcattttcttccccgacgcgaacaaacagcatattggtgtcctgacgcatcacatccgcgcctgcttcacgcagctgctccgccatccaggcagcgttgtcgtggtcttcctgcaagcgcgcaacgttatttttcagggcatatatcccggcggcagccagaatgccggactggcgcatcccgccacctgtcattttccgccagcgaatggcacgtttaatgtaatcacgattaccgacgagtaatgaaccgactggcgtcccaagacctttcgacaggcaaatggtgaacgaatcacaatattgcgtgatctctttcagttcgcagccgtaagccaccacggcattaaagatgcgcgcaccgtcaacatgcagcgccagattgcgctcgcgggtaaattcccatgcttctttcaggtattcccgcggcaacactttgccgttgtgggtgttttccagactgagtaatttggtgcgggcgaaatggatatcgtcgggtttgattttcatcgccactttatccagcggtagcgtgccgtcggcagccgcgtctatgggttgcggttgaatactgcccagcaccgccgcgccaccggcttcaaacagatagttatgcgcggcctgaccgacaatatactcttcgccgcgttcgcagtgactgagcagagcgaccaggttggcctgagtgccggtaggcagaaaaatggcggcttctttaccggaaagctctgctgcgtagtcctgcagagcattaacggtagggtcgtctccgtaaacgtcgtccccaaccggggcggccatcatcgcttcgagcatggcgcggcttggtcgggtaacggtatcactgcgtaaatcaatcatggcatgtccttattatgacgggaaatgccaccctttttaccttagccagtttgttttcgccagttcgatcacttcatcaccgcgtccgctgatgattgcgcgcagcatatacaggctgaaacctttggcctgttcgagtttgatctgcggtggaatggctaactcttctttggcgaccaccacatccaccaacaccggaccgtcgatggagaaggcgcgttgcagggcttcatcaacttcagacgctttttctacacggatacccgtaatgccgcacgcttcggcaatgcgggcaaagtttgtgtcgtgtagttcggtgccgtcagtcaaatagccaccagctttcatctccatcgccacaaagcccagcacgctgttgttaaagacgacaattttcactggcagtttcatctgcactactgagaggaaatcgcccatcaacatgctaaaaccgccatcgccgcacatggcgaccacctgacgttctggctctgtcgcctgcgcacccagcgcctgcggcatggcgttagccatcgaaccgtggttaaacgaacctaacaggcgacgcttgccgttcatttttagataacgtgccgcccacaccgttggcgtaccaacgtcacaggtgaaaatagcgtcatcggcggcaaaatgactaatttgctgcgccagatattgcgggtgaatggctttctcgctcggtttagctaaatcgtccagccctttgcgggcgtcgcggtaatcttccagcgctttatccagaaacttgcgatcggctttttcttccaccaatggaagcaatgcacgcagagtcgacttgatatcgccgaccagtgccatatccaccttgctgtgagcgccgatgctggctgggttgatatcaatctgaatgattttggcatcggtcgggtagaaggcgcggtagggaaattgcgtgccgagtagcactaacgtgtcggcgttcatcatggtatggaaacctgacgagaagccgattaacccggtcattccaacatcatacggattatcgtattcgacatgttctttaccgcgcagggcatgaacaataggcgctttaattttcccggcaaactcaactaactctttatgcgcccccgcgcagccgctgccacacatcagggcgatattgctggaataacgcagcagttgcgccagtttgcgtaactcttcttcttccggcgtcacgactggttgtggcgcatgataccagtgcatggttgccccttctggcgcaggttttaacgccacgtcgcctggtaacacgacaaccgaaacgccacggttaagcaccgctttgcgcatggcaatcgccagtacttgtgggatctgctccgggctggaaaccagctcgcaatagtgactacattcgcggaatagctcttgtgggtgggtttcctggaaatagccgctgccaatttcgctggagggaatatgagcggcaatcgccagtaccggaacgtgattgcggtggcaatcgaacaggccgttgattaagtgcaggttgccggggccgcacgatccggcgcagaccgccagttctccgctaagttgtgcttcagcgccagcggcaaaggccgccacttcttcgtggcgggtggacatccactcgatggtgcccatgcgattaagactgtcactaagaccgttcagagagtcgcctgtgactccccagatgcgtttcacccctgccgattcgagtgttttggcgatataagctgcaaccgtttgtttcatggttctccatctcctgaatgtgataacggtaacaagtttagttcatctgacggagggggaagggatgggagagaaaggaggcactaacggttaaatagcccgatgaaaggaatatcatcgggcataaggcgattatgcgagaaccaaatccccctgcggatggcaggagcaggccagtacgtaaccttcagcgatttcggcgtcggtcagcgtcattgtgctgctcaccgtatattcaccggaaaccacttttgtcttacagcagccgcaaacacccgcacggcaggcagcgacaaccggaacgttattgctttccagcgcctccagtagcgtggtgccaaccggggcgtaaaattctcgtgccggttgcagtttggtgaatttcagaccgctggtcgccgcttctgctactggggtgaagaatttctctttaaagaaacgcgtcacgccgagcgctttcacttcctgctctacccaatccatatacggagccgggccgcaggtcatcacggtacgtgaagctaagtcaggtacacctgccagcagttcgcgagtgagacgaccagcgataaagccttcggtaacgttattttctgccaccagcgttaccggatagttacgccactcatcggcgaaaataacatcctgcggcgtacgcacgttgtagatcacccgcacatcggcctgtggacggttcttcgcaagccagcgacgcatcgacataatcggcgtgacgccgcagcctgccgccagcaacaggaatttatcttctgctttatcgtcgcaggtaaattcccccatcgcgtccgaaagccagagataatcaccgcgttttacatcgcgcgtcagccactgggagccgacaccgtcatcaatccgccgcacggtcagggtgatatattcactcacgcctggcgtggaggaaatggtgtaagcacgcagcgtttccgctgagtttcgcacgctgaccagtgcatattgcccggcgcgatatgggtagtaatcgtggcaaatcagggaaatcgtccacacatccggcgtttcttgcgtaatgtgatgaacctgcatccgccacgggcattgattcgttggcatcgtcatcgacaaactccttacgcgctcaacagttgcttcatgtcttcttcaacagtggtgatagaacgcaggccgaatttctcgttcagcaccgccagcaggtctggtgtcaggaaaccaggtgcagtcgggccggtgacgatatttttcacgcccagagaaagcagcgtcagcagaatgacgatcgctttctgttcaaaccaggagagcaccagcgacagcggcagatcgttgacaccgcagcccagtttctctgccagagtgacagccagaataatcgctgagtaagcatcgttacattgacctgcatctaccagacgcggcagaccttcgatatcgccaaactcaagtttgttaaagcgatatttaccacaggcgagggtcaggatcaggcagtcatccggcacgctggtggcgaaatcggtgaagtagtggcgctcgccgcgtgcgccgtcacagccaccaagcaggaagatatgacgcagtttttcacggctcaccagatcaatcagcgtatcagcagcgccaagcagcgtctggcgaccaaaacccacggtgataaggtgcggaatttcgctgtacgggaagcctgccatctgttgcgcctgggtgataaccgcagagaaatcatcaccgtccagatgacgcacgccaggccagccaacaatgctgcgggtccagatacgatcgtcataagcgcctacggttgggtcgatgatgcagttcgaggtcatcacgatggggccagggaaacgagcgaactccacttgctgattctgccagccgctgccgtagttaccgaccagatgcttgaatttacgcagctccgggtagccatgcgcaggcagcatttcgccgtgggtgtagacattaacgcccgtgccttcggtctgttccagcaggttgtagagatctttgagatcgtgaccggaaatcagaatgcatttacccgccgtcgctttgacgttgacctgggttggcgtcgggtgaccgtatttaccggtttcgcctgcatccagaatgctcatcactttgaagttcatctggccgatttccattgaacactcaagaagcgcgttcatatcggcaggccaggtccccagccacgccatgattttatggtactgggcataaatatcgttgtcgtattgaccgagaacatgcgcgtgttccatataggccgccgcacctttcaggccatacaggcacagcagacgcaggccgagaatgttttcgccaatcgccgctttatctttgttaggggtaaattctgctgcctgacgttgcagctcgccgagatcgtcgctcaccagttgcaggtcagccatcgggttatcgacgcgcgcgttggcatctacagccaggcattgcgctttcagcgcctcgcgcagggcaatcgcttcacgagcgtagccgacaatacgcggagaatcgaagttaacgttggtcagggttgagaaaaaggcacgtggcgcgaagctgtcaacatcgtggttgatgatgccgtattcacgcgcttttaccgcccaggcagaaagcccttgcagcgccgcgatgagtaaatcctgaaggtcagaagtttccgccgttttaccacacatcccctgcgcgtatgagcagccgtttcctgccggagtacggatagtttgttcacattgcacacaaaacatgatcacaccttttaaagttatatttaatatacatgtttaaggttaagacgcttaacgcggggataaaagggatttttcatgcaactttaagggagattgatttagcgcaattttggcggcagggatctaccgccagagaggtattacgcagagaaaaaggcgatgaggatcggcactaacaggctaagaataaaaccgtgaacaattgccgccgggaccatatccagcccgccagtacgttgaagaacgggcagggtgaaatccattgatgtggcaccgcataagcccagtgcagtagagcggctgcggcgaatcagcccagggatcaacataatagcaatcagttcacgggccagatcattaaaaaacgccgcgctcccgattaccggaccaaaagattcggtcaataaaataccggaaagagaataccagccgaaaccggaggccattgccagcgcggtattgatggggagatcaagaataaaggcgttaattaaaccaccaattaatgaactgacaaccaccaccacggcgacaatcattccccggcgattaaggacaatctgctttaaggtcatgccattattgcgcaactgaataccaacgaggaaaagtagcaaaattaacgtgtattcactggcttcggtcgcgtgttgtaagaaagccagtccacttagaccaatggcaaaaccaatcactactacgccgcacagttttagcgactccagcgccatcgcaatacgcgacgggagtttttcttgctgatggtggttgcgccacggcaggcctcgctccagccacatcagggcggcaatattacacagtaaaataacggtaatactgacggcagaataatgcagaatcgccaacaggttactggcgaggttatcgagaaacgccagactgatacccataaaaaagagaataaggtaaaccatccagcttaatagctgattaataacttttaacgcagcttgttggcgaagcggaatgaggtaacccacaatcaggggaaccagaatgattaacagcccagaaaacatgaaaacccagtccttgcaaagatgaagtcgaaatgcgcgatgacacactactgaaagcggaaggacgagtaaagttgcaattaaaaggaaatgttatgcataaggagcagtagagtattcgttttcatttaaagatattcttgcgctttaattacaaactgcaccgatgttggtggcgtcaaaatcgccgaggcgttccctgaaggccggggcagcccacatggatgtgggctgagggcgcgttttacagggatgttacctcgcgcccgacccggtagccgtaagggataagtcgagggcaccgcgcagcggcgattttgttcgccagagcccgggggtgcagggggcggcggcgattggccgccccctgcgcgctccttgcgccagtggcaatatgttgcttagctcatgaaaggagcgcaacaagatgatgaatcaacatataacaacatcttaaaaaaaggcctgacattacgccaggccttctgcgttaattaatcacgcttttccagcagggtccggtaaatcagaccaccgataatgccgccgacaattggcaccacccagaagaaccacagttgttctaatgcccagccgccctggaagatagcaaccgcggtgctgcgcgccgggttaacagaagtgttagtcaccggaatactaattaagtgaatcagggttaaggccagaccaatagcgatcggcgcaaaacctgccggcgcgaatttgtcggttgcgccgtggatcaccaacaggaaacctgcactcaataccagttcaactaccagcgcggaaagcatggaataaccgcctggtgaatgctcgccataaccgttagaagcaaaaccgctggctgccgcgtcaaaacccgttttaccactggcaattaaatacagcagcgccgctgcaacaataccgccgacaacctgggcaattacgtagccaacgacttcttttgccggaaaacgtccgccagcccataaaccaatagtgaccgccgggttaaaatgaccaccagaaatatgaccaacagcaaaggccatcgtcagaacggtcagaccgaacgccaacgccacgccggcaaaaccaatgcctaattccgggaagcctgcggccagtacagcactaccacagccaccaaaaacaagccagaaagtaccaaaacattcagctgctaattttctgaacatatccaccacaattaaaaattgaccctgtgaaaaatatggtcgttttatagggtcgtcgtaaaaaagtgacgacggaaataatgcgcggctattttaaaaacgaaggcgagtcattcaccagataaataaatccagtaaatttgatttagggcaacagcgggttgccccatatagtcatttgtctgattgacagtgtagtgcacgcaaaagatttaatcctttaggcgtaataaaaaataatttatcatgctaattatttgattttgttgtttttgcagacttatcagcaagagggagtataacgcgattattcgctcatttttcagacatttgccatgcttaaatgtgatgtcatcacgtattagcaaggcctttcccgttatactgccagcgtaaaggataagtcacatatttctggaggggatatgattcttgagcgcgttgaaattgtgggttttcgcggtatcaaccgtttgtcgttgatgctggaacaaaacaacgtcctgattggggagaacgcgtggggtaaatccagcttgctggacgccttaactctgctgctatcgccagaatcagatctctaccattttgagcgcgacgatttctggttcccgccgggagatatcaacgggcgagaacatcatctgcatattattttgaccttccgcgaatcgctgccaggccgacatcgggttcgccgttatcggccgctggaagcgtgctggacgccatgcaccgatggctatcaccgtattttttatcgtctggaaggggagagtgcggaagacggcagcgtgatgacactgcgcagttttctcgataaagacggacatccgattgatgtcgaggatattaacgatcaggcacgccatctggtgcgtttaatgccggtgctgcgcttgcgtgatgcccgttttatgcgccgtattcgtaacggcacggtgccaaatgtccctaatgtggaagtcaccgcgcgccagctcgatttcctcgcccgtgagttatcctcacatccgcaaaatctctctgatgggcagattcgtcagggactttccgcaatggtacagctgcttgagcattatttctctgagcagggggccggacaggcgcgatatcgtttaatgcggcggcgagccagcaatgagcaacgaagctggcgctatctggatatcatcaaccggatgattgaccgacctggtgggcgctcgtatcgggttattttgctcggcctatttgctactttgttgcaggcaaaaggcacattgcgactggataaagacgcccgtccattgttgctgatcgaagatccagaaacccgtttacaccccattatgctttcagttgcctggcatctgttgaatcttctgccattgcagcgcattgccaccaccaactcgggtgagttgctttcgttaacgccggtagagcatgtttgccgactggtacgtgagtcctcgcgcgttgccgcctggcgtctggggccgagtggcttgagtaccgaagatagccgacgcatatcctttcacattcgttttaaccgtccgtcatcgctgtttgcacgctgctggttgctggtggaaggggaaacggaaacctgggttatcaatgaactggcgcgtcagtgcggacatcattttgatgccgaagggatcaaggtcattgagtttgcccagtccgggctaaagccactggttaaatttgcccgccgaatggggattgaatggcatgtactggtcgatggcgatgaagcagggaagaaatatgccgctacggtacgcagcctgttgaataacgatcgggaagccgaacgagaacatttaacggcgttaccggcgctggatatggaacattttatgtatcgccagggattttccgatgtgttccaccgcatggcgcaaatcccggaaaatgtaccgatgaatctacgcaaaattatctcgaaagcgatccatcgctcttccaaacccgatcttgccattgaagtggcaatggaggcaggacgtcgtggtgtggactccgtaccgacgctgctgaaaaaaatgttctcacgcgtgctgtggctggcgcgcggtcgcgcggattaaccgcgaaacatcgtggccatttgtggctgaatagcgtcgagcatctcatagcgccgacggtattcagcccgttttttactggcgatttcggcaatctcttttcgtgctatctgtgctggaaggcggtaatggcgttcagcatcacatacgccgccaaccgattcccagaaagcgttgtaatcagcgtggatcttgccttctttatcgcgataacgcaggctgcggtaaatatgcgtttcattgctgacggcaataatctgctctacctgcaaacgttgggcaaacagacaggccgcttccatcacgaggcgtttgggaaatagcccgtggcaggctttcgtcgcattctggatttcctgatgtggaatttcccattttgcgccttgcagtccgccaataaacatcgttcttttcccctgatattcacacagggtaaacgtgatctctgccagaggaataccttcgctgttgcggaacaggattgtgctgtcaccttctttatccattgagatcatcatggtcagctcaagcgtgaactgctcgccgtttttgccttccagcttcgccagttgcagcccgggggtattcaaatataagctgaattcttccgccgacatacattcgcggagtaacgcataatggtaacgtaacgcctccagcaattgcttacggctaagattcgccgcaaggtaagggcgatgcagacgcacaggcagtcgcggctggcgcgttaacaatacattgagattaggccagtgggaaagttcgttcatccactcaacgcttaaacgcggcataatcaacgagcgcagcaaaaatttctggcgaaaactacggcgatgccagaatttacccggccgacactgtccacgtgccagactaagaaaaagtgacaggctgctgagagattcagatggcgtaaaggtccgttcagttagctgcgacatattcatgaaatcaatggttatacatggcgtcgatttcaccattgcgtatcttaaccaaacatcaatagtgtgattactaacgtaaattttagggttttgttgatatttcgttgaagttaatgacccggattggcatatggagtattcagaaaatttatgaaaaagcggaaaaccgtgaagaagcgttacgttattgcgctggtgatagtcatcgccggactgattacgttatggagaattcttaacgcacccgtgccgacttatcagacgctgattgtgcgccccggtgatttacagcaaagcgtgctggcgaccggaaagctggacgcgctgcgtaaggttgatgtgggcgcgcaggtcagcggtcagttgaaaactctgtcggtggcgattggcgataaagtaaaaaaagaccagcttttaggggttattgatcctgaacaggctgaaaaccagattaaggaggtcgaagcaacgctgatggagctacgtgcgcagcggcagcaggcggaagcggagctgaaactggcgcgggtgacgtattcccgtcagcaacgtctggcacaaacgaaggctgtttcacagcaggatctcgacaccgccgcgacggagatggctgtgaaacaggcgcaaattggcaccattgacgcgcaaatcaagcgcaatcaggcttctctcgatacggctaaaaccaatctcgattacactcgcatcgttgccccgatggccggggaagtcacgcaaatcaccactctgcaaggccagacggtgattgccgcacaacaagcaccgaacattctgacgctggcagatatgagcgccatgctggtaaaagcgcaggtttctgaagcggatgtaatccacctgaagccggggcaaaaagcctggtttacggtgcttggcgatccactgacgcgctacgaggggcaaatcaaggatgtactaccgacgccggaaaaggttaacgacgctattttctattacgcccgttttgaagtccccaaccccaatggtttgctgcggctggatatgactgcgcaagtgcatattcagctcaccgatgtgaaaaatgtgctgacgatccctctgtcggcgttaggcgatccggttggcgataatcgttataaagtcaaattgttgcgtaatggtgaaacacgcgagcgtgaagtgacgattggcgcacgtaacgataccgatgttgagattgtcaaagggcttgaagcgggcgatgaagtggtgattggtgaggccaaaccaggagctgcacaatgacgcctttgctcgaattaaaggatattcgtcgcagctatcctgccggtgatgagcaggttgaggtgctgaagggcatcagcctcgatatttatgcgggtgagatggtcgcgattgttggcgcttcgggttccggtaaatcgaccctgatgaatattctcggctgtctggataaggccaccagcggcacctatcgcgtcgccggtcaggatgttgccacgctggacgccgatgcgctggcgcaactgcgccgcgagcatttcggctttattttccagcgttaccatttgctttcgcatttaaccgccgagcagaacgttgaagtacccgccgtctatgctggtcttgagcggaaacagcgactgcttcgtgcccaggagttgctgcaacggctggggctggaagaccgtacagagtattatccggcacagctttcgggtggtcagcaacagcgcgtcagcatcgcgcgggcattgatgaacggtggtcaggtaattcttgccgatgaaccaaccggcgcactggacagccattctggcgaagaggtgatggcgatcctgcatcagctgcgcgatcgtgggcatacggtgattatcgtcacccacgatccgcaggtcgctgctcaggccgagcgggtgatcgaaattcgcgacggcgaaattgtgcgcaatcctcccgccattgaaaaagtgaatgttactggcgggacggaacctgttgtcaacacggtgtctggctggcggcagtttgtcagcggttttaacgaggcgctgacgatggcatggcgggcgctggcagcgaataaaatgcgtactttactgaccatgctggggattattatcggtattgcgtcggtggtttccattgtcgtggtgggtgacgccgccaaacaaatggtgctggcggatattcgttctattggtacgaatactattgatgtctatcccgggaaagattttggcgatgacgatccgcaatatcagcaggcgctgaagtacgacgacttaatcgccatccaaaaacaaccgtgggtcgcctcagccacacctgccgtctcgcaaaacctgcgcctgcgttataacaatgttgatgttgctgccagtgccaatggcgtgagcggcgattattttaatgtctatggcatgaccttcagtgaaggaaacacctttaatcaggagcagctgaacggtcgtgcgcaggtcgtggttctcgacagtaatactcgccgccagcttttcccccataaagcagatgtggttggcgaggtgattctggtcggcaatatgcccgccagagtcattggtgtggcggaagaaaaacagtcgatgtttggtagcagtaaagtgctgcgtgtctggctaccttacagcacgatgtccgggcgagttatgggccagtcgtggcttaactccattactgtcagggtgaaagaaggatttgacagcgccgaggcggaacagcaactcacgcgtttactttcactgcgccacggaaagaaggatttctttacctggaacatggacggcgtcttgaaaactgttgaaaagaccacacgtactttacaactgtttctgacgctggtggcggtgatttcgctggtggtgggcggtattggtgtaatgaatattatgctggtgtcagtgaccgagcggacgcgggaaattggcattcgcatggctgtaggtgcgcgagcaagcgatgttttgcaacagttcctgatcgaagccgtactggtttgcctggtcggtggcgcgttgggaataacactgtcactgttaattgctttcaccttgcagcttttcttacccggctgggagattggtttttcaccgttggcgctgctgctggcgtttctctgctcgacggtcaccgggattttatttggctggttacccgcacgaaatgcggcacgactggatccagtagatgctctggcacgagagtaatttttgagataaaaatgccagccgatcgggctggcattttgcctttaggatgtacacaatgagacagaagagctatgcgactgccgcttctacttcgacgggcacaataacactggcgtgattgccttttggcccctggtggacatcaaactgaacggattgtccagcttttagcgttctgtaaccatccatctgaatggtggaataatgagcgaaaatatcttcgccgccgccttcagggcagatgaaaccaaaccctttggcattgttgaaccacttaacagtacccttttccatgcttcgacatccttcgcaaatcttatacaagtaagatggaataaaccggggtcagagagggggctgttcaaaacctcgccaactctagaaatacaatttagagaattagggcgagccgtcaagcatttgacaggggacaaggggcaggtatgaatcaaaaatttgaagcagttaacgctattgacaggaatgtgacagatgtcgctgatgccaacgatagatgatagttatctatcatgtggagtagattggtcaggcaaataagctcttgtcagcggcagggcgttctgccgataaccgtaaccgaagatgataactgacaatgggtaaaacgaacgactggctggactttgatcaactggcggaagaaaaagttcgcgacgcgctaaaaccgccatctatgtataaagtgatattagtcaatgatgattacactccgatggagtttgttattgacgtgttacaaaaattcttttcttatgatgtagaacgtgcaacgcaattgatgctcgctgttcactaccaggggaaggccatttgcggagtctttaccgccgaggttgcagaaaccaaagtggcgatggtgaacaagtacgcgagggagaatgagcatccattgctgtgtacgctagaaaaagcctgaatgcaggcataaaaattgggggaggtgcctatgctcaatcaagaactggaactcagtttaaatatggctttcgccagagcgcgcgagcaccgtcatgagtttatgaccgtcgagcacttgttactggcgctgctcagtaacccatctgcccgggaggcgctggaagcgtgttctgtggatttggttgcgctccgtcaggaactggaagcctttattgaacaaaccacacccgttctgcctgccagtgaagaggagcgcgacacacagccgacgctgagttttcagcgtgtactgcaacgtgcggtcttccatgtccagtcctccggtcgcaatgaggttaccggtgcaaacgttctggtcgctatctttagcgaacaggagtcgcaggcggcatatctgttgcgtaaacatgaagtcagccgtctcgatgtggtgaactttatctctcatggcacgcgtaaagacgagccgacacagtcttctgatcctggcagccagccaaacagcgaagaacaagctggtggggaggaacgtatggagaatttcacgacgaacctgaatcagcttgcgcgcgtgggcggaatcgacccactgattggtcgtgagaaggagctggagcgtgctattcaggttctctgccgtcgccgtaaaaacaacccgctgctggtgggggaatctggtgtcggtaaaaccgcgattgcggaaggtcttgcctggcgaattgttcagggcgatgtgccggaagtgatggctgactgtacgatttactctctcgatatcggttctctgttagcgggcacaaaatatcgcggcgactttgaaaaacgttttaaagcgttgctcaagcagctggagcaggacactaacagcatcctgtttattgatgagatccacaccattatcggtgcgggtgcagcgtctggtggtcaggtcgatgcggctaacctaatcaaaccgttgctctccagcggtaaaattcgtgtaattggttcgacaacctatcaggagttcagcaacattttcgagaaagaccgtgctctggcgcgtcgcttccagaaaattgatattactgaaccgtcgatcgaagaaactgttcaaatcatcaatggcctgaaaccgaagtatgaagcgcaccacgacgtgcgttataccgcaaaagcggtgcgtgcggcggtagagctggcggtgaaatacattaacgatcgtcatctgccggataaagccattgatgttatcgacgaagcgggcgctcgcgcacgcctgatgccggtaagcaaacgcaagaaaaccgttaatgtggcggatattgagtccgtggtggcccgtattgcacgcattccagagaagagtgtttctcagagtgatcgtgataccctgaaaaacctcggcgatcgcttgaaaatgctggtcttcggtcaggataaagccattgaggcgctgactgaagccattaagatggcgcgtgcaggtttaggtcacgaacataaaccggttggttcgttcctgtttgccggccctaccggggtcgggaaaacagaggtgacggtacagctttcgaaagctttgggcattgagcttctgcgctttgatatgtccgagtatatggaacgccataccgtcagccgtcttattggtgcgcctccgggatacgttggttttgatcagggcggtttgctgactgatgcggtcatcaagcatccacatgcggtgctgctgctggacgaaatcgagaaagcgcacccggacgtgttcaatattctgttgcaggtgatggataacggtacgctgaccgataacaacggacgcaaagcagacttccgtaacgtggtgctggtgatgaccaccaacgccggggtacgggaaactgagcgcaaatccattggtcttatccaccaggataacagcaccgatgcgatggaagagatcaagaagatctttacaccggaattccgtaaccgtctcgacaacattatctggtttgatcatctgtcaaccgacgtgatccatcaggtggtggataaattcatcgtcgagttgcaggttcagctggatcagaaaggtgtttctctggaagtgagccaggaagcgcgtaactggctggccgagaaaggttacgaccgggcaatgggcgctcgtccgatggcgcgtgtcatccaggacaacctgaaaaaaccgctcgccaacgaactgctgtttggttcgctggtggacggcggtcaggtcaccgtcgcgctggataaagagaaaaatgagctgacttacggattccagagtgcacaaaagcacaaggcggaagcagcgcattaatctgattgttaggtaggttggtcaagtccgtaatctcgaaagaggttacggactttttgtttatggggtggaggaggttcagaccctttttttaatgatgatggtaagttgttgataattagtgctgcgggaaggtaaggataaaaaagggtgctgcaggagaatgggatggttttgctttattaacaacgggctaaacgtgtagtatttgagttcactgccgtacaggcagcttagaaattcacaggtaacatactccacccgcccaccatgttcactgccgtacagacagataaaatgcgaaaaaaaagctcgcactttcgtacgagctcttctttaaatatggcggtgagggggggattcgaacccccgatacgttgccgtatacacactttccaggcgtgctccttcagccactcggacacctcaccaaattgttttgctaccaaacctcatgggtggcaacggggcgctactatagggagttggagtaaaacggtcaagaagaattttaatgataattattgtttgctcatactgtaaacaagttgtgcagtatatctacatcgagacaagttacggacttatacttccaaagtacttcatacatatcacaaaataaaaaggccggttaaaccgaccttttactcgttctttctcttcgcccatcaggcggtaaaacaatcagcgactacggaagacaatgcggcctttgctcaggtcgtacggggtcagttcaacagtcactttgtcgcccgtcaggatgcggatgtagtttttgcgcattttaccggagatgtgtgcagtaaccacgtgaccgttttctaactctacgcggaacatggtattaggcaacgtttcaagaacggtaccttgcatttcaatattgtcttctttggccatctaatcctctggggtatcactaccgtaatttgaaccggcaagataatgccgaagttctgtaaataagtaaagatttgcgcgctaaatcgcaacaaacaggttcggcacattactccgaaaacacacggctaagccgcaccaaaagcgcaacgtataagggagcggtgagataaacgatgggcgttacctgacgcgaaaaattccttatcggcagcggggtaatgagcgtaaccaactctgcgaccgcaattataacactctggggagaaatgtgccgaaaacattcattcttgtggtgaaaacaagcatcgtggtacccagaaattattcggcaatcgtccgaggcgcatttgattgagataattaaggtaatcccggcggggaatttcgcaggcaccaagcgatgctgtgtgatcgttaaggacctggcagtcgataagcttaccgccatgaccgataaattcctcacagaataccagaagcgccgttttagacgcattttccatccggctgaacatggactcgccacaaaatagcgttccctgggccacgccgtacataccgccgacaagctcatcttcacgccagacttcaatggagtgggcatggccgagttcgtgaaggcgatggtaggcttcgaccacgccacgcgtgatccaggttccttcttcgcgatcgctggcacagccttcaatgacctgaccaaaagcgtaattcatcgtgacacgatagggcgagcgtttatgaaatcgcttcatactacggctgatatgcagtgattctggccatagcaccgcgcggggatcgggcgaccaccagaggatggggtcgcctggagaaaaccacggaaaaataccacgctggtaagccattaacaggcgcgcagggctaagatcgcccccaagtgccagcaggccgttaggctcacgtaatgcgccttccggggaagggaaggctattgaatggcgagaaagctgaaccaggcgcatgaccgcaaaactccacgcaagtcggatcgttcaataatagcttacaaaccctgcttgaactggtaataacgcccctgtctggcaagcagttctgcgtgagtaccttgctcaataatttgcccgttgtccatcactattatttgttggaaacgagagagtccgcgaagtcgatgggtgaccattaacaccgttttctcacgcatcatttctgcaagcaattcaaggatctggctttcggttgtggcatctaagccttcggtaggttcatccagcaacaccagtggcgcatcatgtaacagcgcacgggcgatagccagacggcgcagttcaccaccggagagctggcgtccgccttcacctaaccaactgttgagacctgcatcctcgagcagcttttccaggccaacgcgacgcaagatctccgacagagcctcatcactactgccaggcgaggcgagtaaaagattatcacgcagcgtggcgctaaacagatgcactcgctgaggaacaacgctgatggtctgtcgtagagccgcttcattcaggctggctatggggctatcgttaagcaaaatctcgccctgttgcgggtcccatgcgcgggtcagctgttgtaacagtgttgatttgccgcatccggttcgcccgagaatcgctatatgttccccggcgtttacctgaagagaaatccctttaagtgcctgttgagattgctccggataagtgaactgaacatcccgtaacgtcagcgaaacgcgatcggcaacacgagtttgggtatcaggaaaggtgacctccggtttttgatccgttaagtcagagatacgtacggcagaggcaatgacttgccccagatgctgaaatgcacccgttactggtgccagtgcttcaaacgcggctaacgcgcagaagacaaacagggcaattaacgcgccgggttgagcattgccgccaacgccgccagacgccatccacagcatcaggatcaccgctaacgcgccaatgagcagcattatcgcttgcgacaatgcggtcagttcagattgacggcgttgcgcttccagccattgaatttctgtattctctagttgcgtgcgataacgatcgctggcaccaaaaatggtcagctcagcttgcccttgcagccaggccgtcagttgttggcgatactgtccgcgaagatgagtcagattttgcccggtgctttttcccgcacgataaaacagcggtggcatcaggaaaagcgtcagtaacataatgccgcccagcgtaaaggcgagggtgaaatcaaggaaacttaacccgattgtcaccaccataatcaccacaaaagcgcccaccagcggcgagataacgcgcaggtaaagatgatcgagcgtatcaacatccgccaccacgcgattgagcaattcgccctgacgatagcgcgccagtccggcaggggagaggggcagcaatttgctgaaggtgtaaatgcgcagatgctgcaacacgcggaaagtcgcgtcgtgacttaccagacgttcaaaatagcgcccggcagtacgggtgattgctgcgccacgcacgcccgcagcgggtagcatatagttgaagctgtacagtccggcaacccccgcaaccgctgaggccgagaggaaccagccggaaagtgtcaacagaccgatactggcgagcagcgtcacaattgccagcacaataccaagacttaacatccatttatgacgtttatacagtgccagatagggtagcaaagcgcgcatttaaatctcctcctgacgatgggccagtaatgtggcgaatgggccaccagccacacttaattccgcgtaacgtccttgctcaataatccggccatcctgcataacccaaatgacatcccagtcagcaagatcttctaactggtgggtgaccattaacgttgtctggcgcagagaggcggcattcagcgcctccattacgcgctgttcactgtgagcatcaaggctggcagcgggttcatccaacagtaatagcgaacagggatttagtaacgcacgggccaccgccacgcgctgcgcctgccccacggaaaggcgggcagcctggtcgccaacaggcgtatcaacgccttgtgggaggagcggtagaaactcgctgacccaggcgttatccagcgctgcttgtaattcttgttcgctggcatcaggtcgcgccagtagtacgttatcccgcaatgttgctgccggtaattgtgggttttgcccaacccaggagagatgtttacgccatgattctggtgataaatcgcgtaattctatcccgttgattcgtagcgatccctgatatgagagaaaaccagaaagcgcgttcagcagtgagcttttacctgaaccgctgcgaccaaccaacaccgcacgttggcctgctggcaaagtaaagttcagcggtccggccagcgttttaccttccggcgacgtgataaacagctcctcggcctcaatggtcaccggatcggtcgatgctaattccgcctcaccacgttgcggatgggcgagcggggtttccataaacgttttcagactgtcagctgcgccaacagcctgggctttagcatgataaaacgtaccgagatcgcgtaatggctggaaaaactctggcgcaaggatcagggccagaaaacccgcagccagcgtcacaccggtatcgtagtgaccaaaatccagctcgccgagataggaaaaaccaaagtagaccgccaccagagcaattgacagcgaggtaaaaaattcgagaatgccggaggataaaaacgccagccgtagcacttccattgtccgttggcggaaatcttccgaagcagaacgaatactttcaatttcagcttcaccacgaccaaaaatacgcaatgtttccatgccgcgcaggcgatcgaggaaatgcccacttaagcgagcaagagcgagaaagttacgtcggttagcatcggcagcccccattccaaccagcgccataaacaacggaattaacggtgcagtgcccagcagaatgagcgccgcagcccagttagaggggaagattgccaccacaatcagcaacggcaccgacactgccagcgccatttgcggcagatagcgtgcatagtaatcatgcatatcgtcaatttgctcgagtaccagcgtcgcccagctccccgcaggtttaccctgaatccacgctggccctgcttgttgcagacggtcgagaacctgacggcggatggcaaagcggatatgctgcccggcgtgataacccacccgttcgcgtaaccagaccacccatgcgcgcagtacaaaggtcagaaccagtaacgtaaagggaagcagcagggcttcacggggaatattctccataatcatatgttgcagaattcgcgccatgaaccaggcctgggcaatgatcaatatgccgctcacaaagcccagcagacgagaaatattcagccaacgttgggagatgacgctttgctgttttaaccagcgggttaactctttttgacgagatttattcattgcacgcttagcaggtgagttatcagaattatttgcagagcaatgttacaacggggaaaaaataaaggcgacccatagtcgcatggtgtcgccttctttacttttgttactgatttgtaaaattattttgcgtcagctaaaccatcgaggtagcgttccgcatcaagtgctgccatgcagcctgtaccggccgaagtaatggcctggcgataaatgtgatccatcacgtcgcctgcggcaaagacgccaggaatgctggtctgggtggcattaccatgaatacccgactgtactttgatgtagccgttttccagttccagctgcccttcgaaaatcgcagtattcgggctgtgaccgatagcaacaaacagaccggcaacgtcgagtgactcgatgttatcgctgttttgcgtatcgcgcagacgaacgccagtgacacccatttgatcgccggtcacttcttccagcgtacggttggtgtgcagaatgatgttgccgttctccactttatccatcaggcgcttaatgaggattttttccgcgcggaaaccgtcacggcggtgaatcagatgcacttccgaagcgatgttagacagatacagcgcctcttcaaccgcggtattgccgccgccgatgaccgcaactttctggttgcgatagaagaaaccgtcgcaggttgcacaagcagaaaccccacggcctttaaaggcttcttcagagggcaggccgagatagcgtgcagaagctccggtggcaataatcagcgcgtcgcaagtgtattcgccgttatcgccattcagacggaacggacggttttgcagatccaccttgttgatatgatcaaaaatgatctcagtttcaaacttggtggcatgttcgtgcatgcgctccattaataacggaccggtcagatcgtttggatcgccaggccagttttccacttccgtggtggtggtcagttggccgcctttttccatgccggtaatcagcacaggttgcaggttggcgcgcgccgcgtagacagcagcggtgtatcccgccgggcctgaacccaggataagcagtttactgtgtttggtcgtgcccatgagatccccatagttgttggcagacaatgggcaggattgtagggaatttacagacgtaaaaaaagagtatgacgattttgttaacaatttgtgcaatcggcagcatcgataagcaggtcaaattctcccgtcattatcacctctgctacttaaatttcccgctttataagccgattaaatgatgaataaacgcccctgttaatgaatatctggcatgttgtactaaaaatcgatgttttgctttgacaatcccctggtgttttgcgaaaacattcgaggaagaaaaaaaacagtattcttatatgcgcataaccatgcatgtaaataccatgtttaccgtgctagtgaaatctacgtatggcgtggacagacgccattcgtgatgtcgatagctgccacaaggcaacggtcttctcaccgtagacccaggcattgcgcgccgtgaatcttcatgatttcggtctatcgtgacgggtagcgactctgaacagtgatgtttcagggtcagacaggagtagggaaggaatacagagagacaataataatggtagatagcaagaagcgccctggcaaagatctcgaccgtatcgatcgtaacattcttaatgagttgcaaaaggatgggcgtatttctaacgtcgagctttctaaacgtgtgggactttccccaacgccgtgccttgagcgtgtgcgtcggctggaaagacaagggtttattcagggctatacggcgctgcttaacccccattatctggatgcatcacttctggtattcgttgagattactctgaatcgtggcgcaccggatgtgtttgaacaattcaataccgctgtacaaaaacttgaagaaattcaggagtgtcatttagtatccggtgatttcgactacctgttgaaaacacgcgtgccggatatgtcagcctaccgtaagttgctgggggaaaccctgctgcgtctgcctggcgtcaatgacacacggacatacgttgttatggaagaagtcaagcagagtaatcgtctggttattaagacgcgctaacacggaacaggtgcaaaatcggcgtattttgattacactcctgttaatccatacagcaacagtactggggtaacctggtactgttgtccgttttagcatcgggcaggaaaagcctgtaacctggagagcctttcttgagccaggaatacattgaagacaaagaagtcacattgacaaagttaagtagcggccgccgccttctggaggcgttgctgatccttattgtcctgtttgccgtctggttgatggctgccttactaagctttaacccttcggaccccagctggtcgcaaacggcctggcatgaacctatccataatttaggtgggatgcccggtgcgtggttggcagatacgctgttctttatttttggcgtgatggcttacaccattcccgtcattattgtcggcggttgttggtttgcctggcgtcatcagtccagcgacgaatacattgattattttgccgtttcgctacgcatcattggcgttttggcgctcatccttacctcctgtggtctggcggcaatcaacgctgacgatatctggtattttgcctccggtggcgtcattggcagcttactaagcactacgctacaaccactgctacacagtagcgggggaactattgcgctgctctgcgtttgggcagcgggcctgacgttgttcaccggttggtcatgggtgaccattgctgaaaaactcggcggctggattttaaacattctcaccttcgccagtaatcgtacccgtcgcgatgatacctgggtcgatgaagatgagtatgaagacgacgaagagtatgaagatgaaaatcacggcaaacagcatgaatcacgccgtgcccgtattcttcgcggcgcgctagcgcgtcgtaaacggttggcggaaaaattcattaatccgatggggcggcaaacagacgctgcgttgttctccggtaagcggatggatgatgacgaagagattacctacactgcacgcggtgtggctgccgacccggacgacgtcctattttcgggcaatcgtgcaacgcagccagaatatgacgaatacgatccattattaaacggtgcgccaattaccgaacctgtcgctgtagcagctgctgctaccacggcgacacaaagctgggctgcgccggttgaacctgtgactcagacgccgcctgttgcctctgttgatgttccacctgcgcaacctacagtagcctggcagcctgtaccgggtccacaaacgggagagccggttattgctcctgcaccggaaggttacccacagcagtcacaatatgcgcagcctgcagtgcaatataatgagccgctgcaacaaccagtacagccgcagcagccgtattatgcacctgcagctgaacaacctgcgcaacagccgtattatgcccctgcgccagaacaaccggtggcaggtaacgcctggcaagccgaagagcagcaatccacttttgctccacagtctacataccagactgagcaaacttatcagcagccagccgctcaggagccgttgtaccaacagccgcaacccgttgaacagcagcctgttgtggagcctgaacccgttgtagaagagacaaaacccgcgcgtccgccgctttactactttgaagaagttgaagagaagcgagcccgtgaacgtgaacaacttgcggcctggtatcaaccgattccagaaccggttaaagaaccagaaccgatcaaatcttcgctgaaagcaccttctgttgcagcagtacctccagtagaagccgctgccgctgtttccccgctggcatctggcgtgaaaaaagcgacactggcgacgggggctgccgcaaccgttgccgcgccagtcttcagtctggcaaatagcggtggaccgcgtcctcaggtcaaagaggggattggtccgcagttgccacgaccgaaacgtatccgcgtgccaactcgtcgtgaactggcgtcttacggtattaagctgccctcacagcgtgcggcggaagaaaaagcccgtgaagcccagcgcaatcagtacgattctggcgatcagtacaacgatgatgaaatcgatgcgatgcagcaggatgaactggcacgtcagttcgcccagacacagcagcaacgctatggcgaacagtatcaacatgatgtgcccgtaaacgcagaagatgcagatgctgcggcagaggctgaactggctcgtcagtttgcgcaaactcaacaacaacgttattccggcgaacaaccggctggggcgaatccgttctcgctggatgattttgaattttcgccaatgaaagcgttgctggatgatggtccacacgaaccgttgtttacgccaattgttgaacctgtacagcagccgcaacaaccggttgcaccgcagcagcaatatcagcagccgcaacaaccagttccgccgcagccgcagtatcagcagccacaacagccggttgcgccgcagccacaatatcagcagccgcaacaaccggttgcgccacagcagcaatatcagcagccgcaacaaccggttgcgccgcagcagcagtatcagcagccacaacagccagttgcgccacaaccgcaggataccctgcttcatccgctgttgatgcgtaatggcgacagccgtccgttgcataaaccgacgacgccgctgccttctctggatttgctgacaccgccgccgagcgaagtggagccggtagatacctttgcgcttgaacaaatggctcgcctggtggaagcgcgtctggctgatttccgtattaaagccgatgtcgtcaattactctccggggccggttatcactcgctttgaattgaacctggcaccgggcgtaaaagcggcgcgcatttctaacttgtcacgggaccttgcccgttcactttcgacggtggcggtgcgtgtcgttgaagttattcctggcaaaccctatgtaggtctggagttaccgaataaaaaacgacaaaccgtttatctgcgcgaagttttggataacgccaaattccgcgataatccgtcgccattaaccgtggtgctgggtaaagatatcgccggtgagccggtggttgccgatctggcgaaaatgccgcacttgttggttgcggggactaccggttccggtaaatctgtcggtgtgaacgcgatgatcctgagcatgctttataaagcacagccagaagatgtgcgtttcatcatgatcgacccgaaaatgctggagctttcggtttatgaaggcattccgcatctgttaacggaagtcgttactgatatgaaagatgccgccaacgcgctgcgctggtgtgttaacgagatggagcgtcggtataaactgatgtctgcgctgggtgtgcgtaatctggcgggttataacgaaaaaattgctgaagccgatcgcatgatgcgtccgattccagacccgtactggaagccgggtgacagtatggatgcccagcatccggtgctgaaaaaagaaccatacattgtggtgttggttgacgaatttgccgacctgatgatgacggtaggtaaaaaagtggaagagctgatagcacgtctggcgcaaaaagcccgtgccgcgggtatccacctcgtactggcaactcagcgtccatcggttgatgttattactggtctgattaaagcgaatattccgacccgtatcgcctttaccgtatccagtaagattgactcacgtaccattcttgatcaggctggcgcggaatcactgctgggtatgggggatatgctctactctgggccgaactccacgttgccggtacgtgtccatggtgcttttgttcgcgatcaggaagttcatgccgtggtgcaggactggaaagcgcgtggtcgcccacagtatgttgatggcatcacctccgacagcgaaagcgaaggtggtgcgggtggtttcgatggcgctgaagaactggatccgttgttcgatcaggcggtgcagtttgtcactgaaaaacgcaaagcgtcaatttctggcgtacagcgtcagttccgcattggttataaccgtgcagcgcgtattatcgaacagatggaagcgcaggggattgtcagcgaacaggggcacaacggtaatcgtgaagtgctggccccaccgccgtttgactaactaatgcatcgtatgccggataaggcgcggtagcgtcgcatccggcactctatcaactgaaaattcagtattttcttctttcctcaagctgattattagcctggaatagagagtagagggaactcccgatcgggagtgacgtaatttgaggaataatgatgaaaaaaattgccatcacctgtgcattactctcaagcttagtagcaagcagcgtttgggctgatgccgcaagcgatctgaaaagccgcctggataaagtcagcagcttccacgccagcttcacacaaaaagtgactgacggtagcggcgcggcggtgcaggaaggtcagggcgatctgtgggtgaaacgtccaaacttattcaactggcatatgacacaacctgatgaaagcattctggtttctgacggtaaaacactgtggttctataacccgttcgttgagcaagctacggcaacctggctgaaagatgccaccggtaatacgccgtttatgctgattgcccgcaaccagtccagcgactggcagcagtacaatatcaaacagaatggcgatgactttgtcctgacgccgaaagccagcaatggcaatctgaagcagttcaccattaacgtgggacgtgatggcacaatccatcagtttagcgcggtggagcaggacgatcagcgcagcagttatcaactgaaatcccagcaaaatggggctgtggatgcagcgaaatttaccttcaccccgccgcaaggcgtcacggtagatgatcaacgtaagtagaggcacctgagtgagcaatctgtcgctcgatttttcggataatacttttcaacctctggccgcgcgtatgcggccagaaaatttagcacagtatatcggccagcaacatttgctggctgcggggaagccgttgccgcgcgctatcgaagccgggcatttacattctatgatcctctgggggccgccgggtaccggcaaaacaactctcgctgaagtgattgcccgctatgcgaacgctgatgtggaacgtatttctgccgtcacctctggcgtgaaagagattcgcgaggcgatcgagcgcgcccggcaaaaccgcaatgcaggtcgccgcactattctttttgttgacgaagttcaccgtttcaacaaaagccagcaggatgcatttctgccacatattgaagacggcaccatcacttttattggcgcaaccactgaaaacccgtcgtttgagcttaattcggcactgctttcccgtgcccgtgtctatctgttgaaatccctgagtacagaggatattgagcaagtactaactcaggcgatggaagacaaaacccgtggctatggtggtcaggatattgttctgccagatgaaacacgacgcgccattgctgaactggtgaatggcgacgcgcgccgggcgttaaatacgctggaaatgatggcggatatggccgaagtcgatgatagcggtaagcgggtcctgaagcctgaattactgaccgaaatcgccggtgaacgtagcgcccgctttgataacaaaggcgatcgcttttacgatctgatttccgcactgcataagtcggtacgtggtagcgcacccgatgcggcgctgtactggtatgcgcgaattattaccgctggtggcgatccgttatatgtcgcgcgtcgctgtctggcgattgcgtctgaagacgtcggtaatgccgatccacgggcgatgcaggtggcaattgcggcctgggattgctttactcgcgttggcccggcggaaggtgaacgcgccattgctcaggcgattgtttacctggcctgcgcgccaaaaagcaacgctgtctacactgcgtttaaagccgcgctggccgatgctcgcgaacgcccggattatgacgtgccggttcatttgcgtaatgcgccgacgaaattaatgaaggaaatgggctacgggcaggaatatcgttacgctcatgatgaagcaaacgcttatgctgccggtgaggtttacttcccgccggaaatagcacaaacacgctattatttcccgacaaacaggggccttgaaggcaagattggcgaaaagctcgcctggctggctgaacaggatcaaaatagccccataaaacgctaccgttaatgttatcgttgcggtaatgttgttactgtatccctgtggtcgcaggctgtggccacatctcccatttaattcgataagcacaggataagcatgctcgatcccaatctgctgcgtaatgagccagacgcagtcgctgaaaaactggcacgccggggctttaagctggatgtagataagctgggcgctcttgaagagcgtcgtaaagtattgcaggtcaaaacggaaaacctgcaagcggagcgtaactcccgatcgaaatccattggccaggcgaaagcgcgcggggaagatatcgagcctttacgtctggaagtgaacaaactgggcgaagagctggatgcagcaaaagccgagctggatgctttacaggctgaaattcgcgatatcgcgctgaccatccctaacctgcctgcagatgaagtgccggtaggtaaagacgaaaatgacaacgttgaagtcagccgctggggtaccccgcgtgagtttgactttgaagttcgtgaccacgtgacgctgggtgaaatgcactctggcctcgactttgcagctgcagttaagctgactggttcccgctttgtggtaatgaaagggcagattgctcgcatgcaccgcgcactgtcgcagtttatgctggatctgcataccgaacagcatggctacagtgagaactatgttccgtacctggttaaccaggacacgctgtacggtacgggtcaactgccgaaatttgctggcgatctgttccatactcgtccgctggaagaagaagcagacaccagtaactatgcgctgatcccaacggcagaagttccgctgactaacctggtgcgcggtgaaatcatcgatgaagatgatctgccaattaagatgaccgcccacaccccatgcttccgttctgaagccggttcatatggtcgtgacacccgtggtctgatccgtatgcaccagttcgacaaagttgaaatggtgcagatcgtgcgcccagaagactcaatggcggcgctggaagagatgactggtcatgcagaaaaagtcctgcagttgctgggcctgccgtaccgtaaaatcatcctttgcactggcgacatgggctttggcgcttgcaaaacttacgacctggaagtatggatcccggcacagaacacctaccgtgagatctcttcctgctccaacgtttgggatttccaggcacgtcgtatgcaggcacgttgccgcagcaagtcggacaagaaaacccgtctggttcataccctgaacggttctggtctggctgttggtcgtacgctggttgcagtaatggaaaactatcagcaggctgatggtcgtattgaagtaccagaagttctgcgtccgtatatgaacggactggaatatattggctaatacccaatttttctgaatctaaaaagcgcctgcgggcgctttttttgtctccctttgataccgaacaataattactcctcacttacacgtaatactactttcgagtgaaaatctacctatctctttgattttcaaattattcgatgtatacaagcctatatagcgaactgctatagaaataattacacaatacggtttgttactggaatcaatcgtgagcaagcttgagtgagccattatgaaaacgaaaatccctgatgcggtattggctgctgaggtgagtcgccgtggtttggtaaaaacgacagcgatcggcggcctggcaatggccagcagcgcattaacattaccttttagtcggattgcgcacgctgtcgatagcgccattccaacaaaatcagacgaaaaggttatctggagcgcctgtacagttaactgtggtagtcgctgcccgctacgtatgcacgtcgtggacggtgaaatcaaatatgtcgaaacggacaataccggcgatgacaattacgacggcctgcaccaggttcgcgcctgcctgcgtgggcgttccatgcgtcgccgtgtctacaatccggaccgcctgaaatatccgatgaaacgagtcggggcgcgcggtgaaggcaaattcgagcgcattagctgggaagaagcctacgacatcatcgcgaccaatatgcagcgcctgatcaaagagtacggcaacgagtctatctatctgaactatggcaccggtacgctgggcggcaccatgacccgctcctggccgccgggaaataccctggtcgcgcggctgatgaactgctgcggcggctatctgaaccattacggcgactactcctccgcgcaaattgcggaaggtttgaactatacctacggcggctgggcagatggcaacagcccgtcggatatcgaaaacagtaagctggtagtgctgtttggtaataaccctggcgaaacgcgaatgagtggcggtggggtgacttactatcttgaacaggcacgccagaaatctaatgcccgcatgatcatcatcgatccgcgctataccgacaccggtgccgggcgcgaagatgagtggatccctattcgtccgggaacagatgccgcactggttaacggtctggcgtacgtcatgatcactgaaaacctggtggatcaggcattcctcgataaatattgcgttggctacgatgagaaaaccctgccagccagtgcgccgaaaaatggccactataaagcttatattctgggtgaagggccagatggcgtggctaaaacgccggaatgggcctcgcaaatcactggtgttccggcagacaaaatcatcaaattggctcgtgaaatcggtagtaccaaaccggcgtttatcagccagggatggggcccgcagcgtcacgctaacggtgaaatcgcaacccgtgctatctcgatgctggcgattctgaccggtaacgttggtattaacggaggcaacagcggcgcgcgtgaaggttcatacagcttaccgtttgtccgtatgccgaccttggaaaacccgatccagaccagcatttcgatgtttatgtggaccgatgccattgaacgtggcccggaaatgacggcgctgcgtgatggtgtacgcgggaaagataagctggatgtgccgatcaaaatgatctggaactatgccggtaactgcctgattaaccagcattctgaaatcaaccgtacccatgaaatccttcaggatgataagaagtgcgagctgattgtggttatcgactgccacatgacctcatcggcgaaatatgctgacatcctgctgcctgactgcaccgcttccgaacagatggactttgcgctggatgcatcctgcgggaatatgtcttacgtgattttcaacgatcaggtgattaaaccgcgctttgaatgtaagaccatctatgaaatgaccagcgaactggcaaaacgtcttggcgttgagcaacagtttactgaaggccgtacccaggaagagtggatgcggcatctgtatgcccagtcgcgggaagcgattcctgaactgccaacgtttgaagagttccgcaagcaggggatctttaaaaagcgcgacccacaagggcatcacgttgcttataaagccttccgtgaagatccgcaggcaaacccactgactacgccatcgggcaaaattgagatttattcgcaggcgctggctgacattgccgctacctgggaattgcctgaaggcgatgtgatcgatccactgccgatctacacgccgggctttgaaagttatcaggatccgctgaacaaacagtatccgctgcagcttacaggtttccactataaatctcgcgttcactcaacttacggcaacgttgatgtgctgaaagcggcttgccgtcaggaaatgtggatcaacccgcttgatgcccaaaaacgcggtatccacaacggcgataaagtcaggatctttaacgatcgtggtgaggttcatattgaggcgaaagtgacgccacgaatgatgccgggtgtggtcgcactgggtgaaggtgcctggtatgacccggatgcaaaacgtgtcgataagggtggttgtattaacgtactgaccactcaacgtccgtctcctctcgctaaggggaatccgtcacatacaaaccttgttcaggttgaaaaggtgtaaggagtaaccgatgacaacccagtatggattttttattgattccagccgttgcaccggttgcaaaacctgcgagctggcctgtaaagactacaaagatttgacgccagaagtcagcttccgccgcatttatgaatatgctggcggcgactggcaggaagataacggtgtctggcaccagaacgtgtttgcctactatctgtcgatttcatgtaaccactgcgaagatccggcttgtactaaagtctgcccgagcggtgcgatgcataaacgtgaagatggttttgttgtggtcgatgaagatgtgtgcattggctgccgctactgccatatggcttgcccgtatggcgcaccgcaatataacgaaacgaaaggccatatgaccaaatgcgatggttgttatgaccgtgttgcggagggtaaaaagccgatctgtgttgaatcttgtccgctgcgggcgctggatttcggccctatcgacgagctgcgtaaaaaacatggcgatctggcggccgttgcgccgttgccgcgagctcactttaccaaaccgaatattgtgatcaaacccaatgccaatagccgcccgaccggggataccactggctatctggcaaacccgaaggaggtgtgagatgggaagtggatggcatgaatggccgctgatgatcttcacggtcttcgggcaatgtgtagcaggtggttttatcgttctggctttggcgctgctcaaaggcgacctgcgagcagaagcccagcagcgtgttatcgcctgcatgtttggtttatgggtgctgatgggcattggctttatcgcctctatgctccatcttggttcaccaatgcgcgcttttaactcgctcaaccgggtaggggcttcagcactcagtaacgaaatcgccagcggttcgatcttttttgccgtaggcggcatcggctggttgctggcaatgctgaaaaagctgtcaccggcattgcgtacgctgtggctgatagtgacgatggttcttggcgtcatctttgtctggatgatggtgcgtgtgtataacagcattgataccgttccgacctggtacagcatctggacgccgatgggcttcttcctgacgatgtttatgggcggcccgttactgggttacctgttgttgagtctggctggcgtcgatggctgggcgatgcgtctgctgccagcaatttctgtactggcactggtagtgagtggcgtggtgtcagtgatgcagggcgcagagctggcgactattcatagttctgtgcagcaggccgcagcgctggtgccggactatggtgcgctgatgtcctggcggatcgtgcttttggccgttgccctgtgcttgtggattgcaccacagctaaaaggttatcagcctgcggttccgctactttctgtatcattcattctgcttctggcaggggaattaatcggtcgcggcgtattctatggtttgcatatgaccgtggggatggccgtcgcaagctaatcataacaaccggggtttcggccccggttctcttttatttctgcttcgttaacgtgtcataactggtcatcaaattacgataatcaggaatgtggttagagaacaacgtcgccagtccttcaatatcattacgccagtcgcgatgcagctcgcacgccacgccgaaccatgtcatcaattgcgcaccagcttgcgacaagcgatcccatgccgaatgccgggtaatttcattaaaggtccctgacgcgtcagtcacgacaaagacgtcaaacccttcttcaatggctgaaagcgccgggaatgccacgcaaacttcggttaccacaccggcaataattaactgttttttacctgtcgctttgacagcttttacaaaatcttcgttatcccaggcgttaatatttcccgggcgagcaatgtaaggtgtatcggggaattgtgctttcagttctggaactaatgggccgttaggaccggtttcaaaactggtggtaagaatagttggtaagttgaaatacttagccaggtcacccagcgccagcacgttatttttaaacttatcgggttcgatatcccgtacaagggaaagtaaaccagcctggtgatcaacaagcaaaacggcagcatcatttttatcaagacgaacatacggtttggtcatcctcttctcctttcgagagtcagtggtacgtctgaaatcgatcagacgcgatgcattgctctgaaagcatagacgggaaatatgagtttgctgtgaccatgaaatttttcgactgaacgaagcgtatgaaatttgtgttagttcaataaaaacaatcagatgagactaatcatctcttcagcattagcgttatgaatgagtaatataaatcgataataccgccgctgggatatcgcgtattttcacccattgacaatgtttttggcggtggcatgatgcgcatgaaatttgaacttcctcacggttttaattcatgtccacgtatacccagcctgtcatgcttttgctgtctggcctgcttttgttgactctggcgattgcggtgttaaatacactcgtgccgctttggctcgcccaggaacacatgtccacatggcaggtaggcgttgtcagctcatcctattttaccggcaaccttgtcggtacattgctgacagggtatgtcattaagcgcattggctttaaccgcagctattatctggcctccttcatttttgccgctggctgtgccggccttggcctgatgattggattctggagctggttggcttggcgttttgtcgcgggcgtcggctgtgccatgatttgggtggttgttgagagcgcgctgatgtgcagtgggacgtcacgtaaccgtgggcgtttgcttgctgcgtatatgatggtttattacgtgggaacgtttttaggccagttactggtcagcaaagtttcaaccgagctgatgtccgtattgccgtgggttacaggtttgacgttggcagggatcttaccgctgttgtttacgcgtgtgctgaatcagcaggctgaaaaccatgattcgacgtcaattacgtcaatgctaaaactccgtcaggcgcggcttggcgtgaatggctgcattatctcaggaatcgttctgggatctctatatggcctgatgccgctgtacctcaatcacaaaggggtgagcaatgccagcattggtttctggatggcggtactggtcagtgcgggtatccttggacaatggccgattggacgtctggcggataagtttggtcgactgctggtgttgcgtgttcaggtctttgtcgtcattctcggcagtatcgcgatgcttagccaggcggcgatggccccagcgttattcatcctcggtgccgctggctttacgctatatccggtggcgatggcatgggcttgcgagaaagttgaacatcatcaactggtggcgatgaaccaggccttactgttgagctatactgtgggaagtctgcttggcccgtcatttaccgctatgctaatgcagaatttctccgataatttattgtttatcatgatcgccagcgtatcgtttatctatttgctgatgctgctgcgcaacgccggtcatacgccgaaacccgttgctcacgtgtaaatgaattcaagcagagtgtgaacttactgtttcacactctgcttttttgtttcttctatctgacttgctttattccaaattttattcgtttaaaaataaaatgtgcagcaggttataattttgcatttcgctatttccgcacttcttatttgccgcgcataatccctcgttttaccgatgcccctttaattttggcgaaggatttgtctatggctgggaatgttcaggaaaaacagttgcgatggtacaacattgcgctgatgtcttttatcactgtctggggttttggcaacgttgttaataactatgccaaccaggggctggtggttgttttttcatgggtgtttatctttgcactctatttcacaccttatgcgctaattgttggtcagttaggctcgaccttcaaagatgggaagggcggggtcagtacctggattaaacacacgatgggacccggactggcttatctcgccgcgtggacctactgggtggtgcatattccctatctggcacaaaaaccccaggcaattctgattgcgctcggttgggcgatgaaaggcgacggttcgctaatcaaagaatattcagtcgtagcgttacaggggttaacgctggtgctgtttatcttctttatgtgggttgcttcacgcggtatgaaatcgctgaaaatcgtcggttctgtggcagggattgctatgtttgttatgtcactcctgtatgtggcgatggcggtaaccgcgcctgcaattactgaagtgcatattgcgaccacaaacattacctgggaaacgttcattcctcatatcgactttacctacattaccactatttcaatgctggttttcgcggttggcggagcagagaagatttctccttacgttaatcaaacgcgcaacccaggaaaagaatttccaaaagggatgttatgcctggcggtgatggttgcggtttgtgccattctgggctcgctggcgatggggatgatgtttgattcgcgtaatatcccggatgacttaatgaccaacggtcagtattacgcctttcagaagctgggcgagtattacaacatgggtaatactttaatggtgatttacgccattgcgaataccctgggacaagtagcggcgctggtattctcgattgatgccccgcttaaagtgctattaggtgatgctgacagcaaatatattccagccagtttatgtcgtaccaacgcttctggtacgcccgttaatggctattttctgaccctggtactggtggcgattctgattatgctgccgactctcggcattggtgatatgaacaatctctataaatggctgttgaaccttaattcggtagtgatgccgctgcgttatttatgggtatttgttgcatttattgcagtcgttcgcttggcgcagaaatataaaccagaatatgtctttattcgtaataagcctctggcaatgaccgtcgggatttggtgttttgcctttaccgcctttgcctgtttgacggggatcttcccgaaaatggaagccttcactgcagagtggaccttccagttggcgctgaatgttgcaacgccgtttgtgctggtaggattaggactgatattcccgctgctggcgcgtaaagcgaatagtaaataattattgtggtcggtgacgctgactctggcagatctgacccgtttttacataatcgagaaatgcgcgcaagccgcaggacatatactggcggtttggataatagatctggaagcctggacgctctgtgctccagtcttccagtacacattctaaacgaccagtatcaaggtactccttgatctgttcatagagcagatacccgataccagcacccatcaaaacggcctccagttcagcatcaacatcatccagaatgatatttcctgcgacagcaatttccagctcctttgcaaattgccagtggaaaggtttgccgctgggataacgaaaaacaacacattgatgattaagcagatcatgaggatggcggggtttgccatatcttgcaaagtactctggcgttgctgctacacataatttcactggcgggccgatcgccacgctgatcatatctttttcgacgatgcaactaagtcgaacgccagcgtcaaagccctgttggacgatatcgacaagagagtcgtcagttgtgagctcgactttaatatcaggatattcacgtgtgaaaccaaccagtaaagacattaaaaatatacgtgcagctacccgggcggcattgattttgagcgttcctgtcggtgtcagacgaaaatcattcatctcatctaacatgatctgaatttcgtcgaaagctgggcgcaatcgttcatagagattagaacccgcttccgttaacgatacgcttcgggttgtccgattgaataagcgaattttaagacgttgttccagtgttttaatactatggctaatggcggacgaggataagcctaactcatcgcccgctgcacgaaagctttgattacgggccacggcaaagaaagtggcaaagtcagacatattcatccgcattagtgaaaatccttcattaactcatcctgaatcatcacgtttacaggattatgccgcctgcgtaaagtgcgctccagaacttaacgtggaggtaaaattatgcagtctgaacgtatttatttggtatgggcccatcctcgtcatgattcattgaccgcacatattgctgatgcgatccatcagcgggcaatggagcggaaaatacaggtgacggaactcgatttatatcggcgtaatttcaacccagtgatgacgccggaagatgaaccagactggaagaatatggataaacgttattctccagaggttcatcagctttattcagagctgcttgaacatgacacgttagtggtggtttttcctctctggtggtacagcttcccggcaatgctaaaaggatatattgacagagtatggaataatgggctggcttatggagatgggcacaaattaccattcaataaagttcgttgggtggcgctggttggaggagacaaagaatcatttgtccagatgggctgggaaaaaaatataagcgattatttaaaaaatatgtgcagttatcttggtattgaagatgccgatgtcactttcttgtgtaatacagtggtattcgatggggaagaacttcacgcgagctattatcagtcgttattatctcaggtacgggatatggtagatgcactataagatgtgttaaaaacgctgtagcagaatgaagcgcggaataaaaaagcggcaactcaataaagttgccgctttacggggaaattagaacattaccttatgaccgtactgctcaagaatgcctttcacgcgttccatggtctctttcttcggtggtttaacaccgtcgagtttgtactcttcacccattgccacccatttgtgtttgcccagctcgtggtaggggagaagctcgattttctcaacgttgcccatatcacgggtaaattcaccgaggcgatgcgctgaatcgtcatcgtcagaccagcctgggacaacaacgtagcggatccacaccttcacatttttgttcgccagatatttagcgaactccagcgtgcggtggttggaaactccaaccagattttggtggatctcgtcgttcatctgtttgagatcgagcattaccaggtcggttacttccagcagttcatcaatcaccggatcgtaacgacgaacaaaaccgttggtgtccagacaggtatgaatgccttcttttttgcaggcgcggaaccagtcacgaacaaactcagcttgcaggattgcttcaccgccggatgcggtaacgccgccgccggaagcgttcataaagtggcgataggtcaccacttccttcatcaaatcttcaacggtaacttctttaccgccatgcgtgtcccaggtgtcgcggttatgacaatacaggcagcgcatcaggcagccctggaaaaaggtgataaagcgaatacctgggccgtctacggttccacaggattcaaaggagtgaatgcgaccaataactgacattgcggtgtttctccagatgtggcccatctgaggccgtgttggtgcgcagctcgaaggctacgtcgagtctgttttggcagtcaccttaaagtatagatagctgacaaaaaaggctctcgcgctaaaaaaggccccactttcgtggagcctttattgtacgctttttactgtacgatttcagtcaaatctaattacatagattgagtgaaggtacgagtaataacgtcctgctgctgttctttagtcagcgagttgaaacgtactgcgtagccagatacacggatggtcagctgcggatatttttccgggttttccatcgcgtcgagcagcatttcacggttcatcacgttaacgttcaggtgctgaccaccttcgatggatgcttcgtggtggaagtaaccatccatcagaccagccaggttggtcttacgaacttcgtcgtctttacccagtgcgttcggaacgatagagaaggtgtaggagataccatctttagcgtaagcaaacggcagtttagcaacggaagtcagagaggctactgcacctttctggtcacgaccgtgcatcgggttagcacccggtccgaacggcgcgccagcacgacgaccgtctggggtgttacccgttttcttaccatacacaacgttagaagtgatggtcagaacagactgagtcgggatagcgtcacggtaggtgtgcagtttctgaattttcttcatgaaacgttctaccaggtcaacagccaggtcatctacacgcggatcattgttaccaaactgcgggtattcgccttcgatttcgaagtcgatagccagaccgtcttcgtcacgaatcggtttaactttcgcatatttgattgcagacagggagtcagcagcaacggacagaccagcgataccacacgccatggtgcggataacgtcacggtcgtgcagcgccatcagagaggcttcgtagctgtacttgtcgtgcatgtagtggatgatgttcagtgcagtgatgtactgtttagccagccagtccatgaagtgatccatgcgctccatcacttcatcatagttcaggacatcgcctttgatcggttcagacttcggaccaacctgcattttcagtttttcgtcaacgccgccgttgattgcgtacagcatggttttcgccaggtttgcacgcgcaccgaagaactgcatttgtttaccaacgatcatcgggcttacgcagcaagcaatagcgtagtcatcgttgttgaagtccggacgcatcaggtcatcgttctcatactgcagagaagaggtgtcgatggacactttagcggcgaatttcttgaagttcagcggcagtttttcagaccacagaatggtcatgttcggttccggagacggacccatggtgtacagggtgttcaggaaacggaagctgtttttggtaaccagggtacgaccgtcgaggcccataccaccgatagattcggttgcccagatcgggtcgccagagaacagttcatcgtattccggagtacgcaggaagcgaaccatacgcagtttcatgaccaggtggtcaaccatttcctgcgcttcttgttcggtgatcttgccagctttcaggtcacgttcgatgtacacatccaggaaggtggaggtacgaccgaaggacattgcagcaccgttctgagacttaacagcagccaggtagccgaagtaagtccactggatagcttcctgagcgttggtagccggaccagagatgtcgtagccgtatttcgcagccatttctttcatctgacccagagcgcggtgctgttcagcgatttcttcgcgcagacggatagtctgttccaggtttacgccgttttccagatcagcctgcagagaagtgaactgtgccagtttgtctttcatcaggtagtcgataccgtacagcgcaacgcgacggtagtcaccgatgatacggccacggccatatgcatctggcagaccggtcagaacaccagatttacggcaacgcaggatgtccggagtgtaaacgtcgaacacgccctggttgtgagttttacggtattcagtgaagatttttttgatcatcggatccagttcgcggttgtacgctttgcaggaaccttcgatcattttgataccaccgaacgggataagagcacgtttcagcggagcttcagtctgcagaccaacgattttctcaagctgcttgttgatgtagccagcgtcgtgagaggtgatggtggaagcaacagcggtgtcaaagtcaactggcgcgtgagtgcggttttccagtttaacgccttccattactttgtcccacagggtggtggtcgcttcagtagcgccagccaggaaggactcgtcaccctcgtacggagtgtagtttttctgaatgaagtcacggacgtttacttcattctgccagtcacctttggtaaaaccttcccaggctgtggctaacttttcattaagctcggacatgtaacacctaccttcttaagtggattttttatttactgcgtacttcgacaaccattaatggtggtcgttttcacgcaggtaaatgacccagtatgtcaacccaaccaacaaaccaccaccgataatgttgccgatcgtaaccggaatcaggttatcagtgatgaaattcatcacggtcaggtgagaaaaattttccggtgcagaaccgactgcggtccaaaattccggggatgcgaagtcgcggattacaatacccatcgggatcataaacatgtttgcgatactgtgctcaaaaccgctggcaacaaacatcgcgaccggcagcaccataatgaacgctttgtccatcaggctgcggccagaataactcatccatactgccagacataccatcaggtttgccaggataccaagacagacggcctcaataaaagtatggtgcactttgtggtcggcggtttgtaggacgtttagtccccattgaccatttgcggtcatatactcgccggaaagccacattaaaagtacaaacagcagtgcgccgaccaggttgccaaaatagacatttagccagtttttcgccaactgaccccaggtgatgcgcccactcgccttagcaacaacaatcaacacggtggaagtaaagagatcggctccgcagacaacacaaagaatcagccccagagagaagcaaatgccgccaaccagttttgccatgccgaagggcattgtgcctgtgccagtggttgctgtgatatagaagacgaatgcgattgagatgaaaacaccggcggtaatcgccagatagaaagtcttaagcggatgtttcgttgctttatagacacccgcctcttcggccactttggccattgcagcaggaagtaaaagatcaaaagggttgtcagctttcacactaactctctctttattaagtcggcgacgagatactaacaaagcattatagatgagaaattgatatagatcatatctcgcctggcttataggcccgtaactcgcatggtttttatgcaaatacggagtaaatatttgattatccaaataaaaataaattttaaaaattaacaaatgagttgaattttttccgcatcctccgctaaaacagttaattaaaagggagcatcaggcgaataaagtaacaatatcgatcgtatttattaaatacaaattaccgatatttaaccttataattacaattattttattaatgcaaatatatgtaaagcggggcattaaaaaaacgccccgtaatataactcagactaatcattaagcctacattgcgtaggctatttgattttattttgcccagaatgctgctttggcgcgctgcagcttttcgtaggccttcaacaacgactgatgtgcagcaaacgcgtgcagatcgctatctaccggttgcaggccgtaaaacgccgcttcgccgctcattgccgcactggcggcttctacggcatctgcgccgtacatgcgaacaaacgcattcagatattgcagcggctggcgatcttcttcctgtgccagtaataacaacgtttgcaggcagcgataatagttggcgcgttccggactaaatactgatgagttaaactccatcgtccattcggtccagaccagagcctgttccagatcgccaccagccagcgccagcatggcttttaattcaccgatacgcagggtgtaccaaccgttatccgacccggtcgccagacccaacagctcacgcacgcgggtaaagtcatcaaaaccttcttcatccagttgctcgatgaggttcaggtaatcttctttttcccactcgctgcctggtagcgaaagaatcgtttcacgtaaatggctgcccatactgttattcgcgagccacagatcttcagccggataaatatcggacatgccaggcacgataatacggcaagcataaacgcccagatgctcgtaatcggcaatataaacttctttatcttctttgttgaagatagccatcagtgtggcgaactcttcttccgtggtgccggagaaattccagtccacaaacggataatcggcatcctgcttgaacaggtcccaggagattaaaccgctggaatcgataaagtgcgtttcgaggttggtatgttcagcgacttcttcatcatcgaaggttggcggagtaaacacatccaaatctttcaggccacgaccttgcagcagctcggtcacggtacgttccagtgctacgccaaaatcaggatgcgcaccgaaagaggcaaagcaggtaccgttagcaggattgaacagtaccacgcaaatcaccggatactggccgccaagcgaaccgtcataagcgaagattgggaaaccctccgcttccagcgtttcgatggcttcaactactgctgggtaacgcgccagcacgtctgccgggatctctggcaggctgatgctttcagcaataatgcggtttttcacgtagcgttcgaaaacttcagacaatccctgaacgcgtgcttcgttgcgggtattacctgcggacataccgttggagacgtacaggttaccaatgatattcatcggaatataaacggtctgattgtcggactgacgcgtaaacggcaggccgcaaataccacgatcttcgttaccggattgtaggtcaatcagcatgctgccggtcagttcattctccggatcataaaacgcgcgcagacggtcatcgagcagcccttctggcacatcgtcattttcggtcagtgggaaccatttttcgttgggataatgcacgaacggaccgttggcgatggtttcgcccagccagaagtccgcaaaaaagtagttggttgagagacgctcgaaatattcaccgagtgcagaagccagcgccgctttcttggttgcgcctttaccgttggtaaaacacagtgcgcactctttgtcgcgaatatgtacagaccagacgttaggcacgggattcagccaggaggcctcttcaatctgaaagccgaggtctgaaagtttttgctggaagcgagcgatggaatcttccagagcggcatctttgccggggataaatgtttgcgtcatgaaaatcactttagtcgtacggaaagcgcgcaataatacgggttttatctcaaaggcgctatcaccgccgccatgccgatgaactgttgactatgcttttagcggataaaccacgttaagagcataaaaatgaaggcgttcgatctccaccgtatggcatttgataaagtgccttttgatttccttggcgaagttgcactacgtagtctttatacctttgtactggtctttttgttcctcaaaatgaccggaagacgcggtgtgcggcagatgtcgctgtttgaagttttaatcattctgacgctgggatcagcggcgggagatgtggcgttttatgatgatgtgccgatggtcccggtacttatcgtctttattactctggcgttgttataccgcctggtaatgtggttgatggcgcacagtgaaaaactggaagatcttctggaaggcaagccagttgtcattattgaagatggcgagctggcctggtcgaaactcaataactccaacatgacggaatttgagttctttatggagctacgattgcgtggcgtggagcagctggggcaggtacgtctggcgattctcgaaaccaacgggcaaatcagtgtctatttctttgaagatgacaaggtgaaaccgggtttacttattttacccagtgattgtacgcagcgttacaaagtggtgccggagtcggcggactatgcctgtattcgttgtagtgaaatcattcatatgaaagcgggggaaaaacaattatgtccgcgctgtgcaaatccagaatggacgaaggcaagtcgggcaaaacgggtgacctgacagtaaaaacatcggctttttgctaataatccgagagattcttttgtgtgatgcaagccacatttttgccctcaacggttttactcattgcgatgtgtgtcactgaatgataaaaccgatagccacaggaataatgtattacctgtggtcgcaatcgattgaccgcgggttaatagcaacgcaacgtggtgaggggaaatggctcaaatcttcaattttagttctggtccggcaatgctaccggcagaggtgcttaaacaggctcaacaggaactgcgcgactggaacggtcttggtacgtcggtgatggaagtgagtcaccgtggcaaagagttcattcaggttgcagaggaagccgagaaggattttcgcgatcttcttaatgtcccctccaactacaaggtattattctgccatggcggtggtcgcggtcagtttgctgcggtaccgctgaatattctcggtgataaaaccaccgcagattatgttgatgccggttactgggcggcaagtgccattaaagaagcgaaaaaatactgcacgcctaatgtctttgacgccaaagtgactgttgatggtctgcgcgcggttaagccaatgcgtgaatggcaactctctgataatgctgcttatatgcattattgcccgaatgaaaccatcgatggtatcgccatcgacgaaacgccagacttcggcgcagatgtggtggtcgccgctgacttctcttcaaccattctttcccgtccgattgacgtcagccgttatggtgtaatttacgctggcgcgcagaaaaatatcggcccggctggcctgacaatcgtcatcgttcgtgaagatttgctgggcaaagcgaatatcgcgtgtccgtcgattctggattattccatcctcaacgataacggctccatgtttaacacgccgccgacatttgcctggtatctatctggtctggtctttaaatggctgaaagcgaacggcggtgtagctgaaatggataaaatcaatcagcaaaaagcagaactgctatatggggtgattgataacagcgatttctaccgcaatgacgtggcgaaagctaaccgttcgcggatgaacgtgccgttccagttggcggacagtgcgcttgacaaattgttccttgaagagtcttttgctgctggccttcatgcactgaaaggtcaccgtgtggtcggcggaatgcgcgcttctatttataacgccatgccgctggaaggcgttaaagcgctgacagacttcatggttgagttcgaacgccgtcacggttaatgccgaaattttgcttaatccccacagccagcctgtggggtttttatttctgttgtagagagttgagttcatggaatccctgacgttacaacccatcgctcgtgtcgatggcactattaatctgcccggttccaagagcgtttctaaccgcgctttattgctggcggcattagcacacggcaaaacagtattaaccaatctgctggatagcgatgacgtgcgccatatgctgaatgcattaacagcgttaggggtaagctatacgctttcagccgatcgtacgcgttgcgaaattatcggtaacggcggtccattacacgcagaaggtgccctggagttgttcctcggtaacgccggaacggcaatgcgtccgctggcggcagctctttgtctgggtagcaatgatattgtgctgaccggtgagccgcgtatgaaagaacgcccgattggtcatctggtggatgcgctgcgcctgggcggggcgaagatcacttacctggaacaagaaaattatccgccgttgcgtttacagggcggctttactggcggcaacgttgacgttgatggctccgtttccagccaattcctcaccgcactgttaatgactgcgcctcttgcgccggaagatacggtgattcgtattaaaggcgatctggtttctaaaccttatatcgacatcacactcaatctgatgaagacgtttggtgttgaaattgaaaatcagcactatcaacaatttgtcgtaaaaggcgggcagtcttatcagtctccgggtacttatttggtcgaaggcgatgcatcttcggcttcttactttctggcagcagcagcaatcaaaggcggcactgtaaaagtgaccggtattggacgtaacagtatgcagggtgatattcgctttgctgatgtgctggaaaaaatgggcgcgaccatttgctggggcgatgattatatttcctgcacgcgtggtgaactgaacgctattgatatggatatgaaccatattcctgatgcggcgatgaccattgccacggcggcgttatttgcaaaaggcaccaccacgctgcgcaatatctataactggcgtgttaaagagaccgatcgcctgtttgcgatggcaacagaactgcgtaaagtcggcgcggaagtggaagaggggcacgattacattcgtatcactcctccggaaaaactgaactttgccgagatcgcgacatacaatgatcaccggatggcgatgtgtttctcgctggtggcgttgtcagatacaccagtgacgattcttgatcccaaatgcacggccaaaacatttccggattatttcgagcagctggcgcggattagccaggcagcctgaatgaacaacgggcaataaatagccaaatctttctttatcaaaacgtcggcacattgtcggcgttttttttcggaccttgtgagtcattttgattaatggtagcgtcgcttgtcaatgtaagttgttgatacataatatttatatatgattaatcaacggatgattcacatgaagaatactaaattactgctggcgattgcgacctctgcagcattactgacagggtgtcaaaatacccacggtattgataccaatatggctatcagctccggtttaaatgcctataaagcagcaacattaagcgatgccgatgcaaaagcgattgccaatcagggctgtgccgaaatggacagcggcaatcaagtcgcaagtaaatccagcaagtacggtaaacgtctggcaaaaatcgccaaagcattgggtaacaatattaatggcacgccggtcaactataaggtttatatgaccagcgacgtcaacgcatgggcgatggcgaacggctgtgttcgtgtctacagtggcctgatggacatgatgaatgacaacgaaattgaaggcgttctgggccatgaactgggccacgtcgcgttgggtcactcgctggctgaaatgaaagcttcttatgcgatcgttgccgcacgcgatgccatttcagctaccagcggtgtggcttcccagctttcccgctcacaattaggtgatatcgcagaaggcgctatcaatgctaaatactcccgtgataaagagtccgaagcagatgatttctcctttgatctgttgaagaaacgtggcatcagcacccaggggctggttggcagctttgaaacactggctagcctggatggcggtcgcacccagtccatgtttgactctcacccaccatcaacagagcgtgcgcaacacatccgtgatcgtatcgcctctggtaagtaaatcattgtcatctttcgggctggtcttctgccagcccgctataattgcgcaataaatccccatctgaatacagacaaaactggtttttgcacacaacgttaacgatttgtggcgtcggcgcgtataatgcgcgcggttatgttaacggtacgcctgttttaaggagataaagatgacggcaattgccccggttattaccattgatggcccaagcggtgcagggaaaggcaccttgtgtaaggctatggcggaagcgttgcaatggcatctgctggactcgggtgcaatttatcgcgtactggcattggcggcattacatcaccatgttgatgttgcgtcggaagatgcgctggtaccgctggcatcccatctggatgtacgttttgtgtcgaccaatggcaatctggaagtgatcctcgaaggggaagatgtcagcggcgaaattcgtactcaggaagtggcgaatgcagcttcacaagtcgcggcattcccacgcgttcgtgaagcattattgcgtcgccaacgcgcgtttcgcgaattaccaggtctgattgccgatggccgcgacatgggaacggtggtattccctgatgcaccagtgaaaattttccttgacgcctcctcggaagaacgtgcgcatcgccgcatgctacagttgcaggagaagggctttagtgttaactttgagcgccttttggccgagatcaaagaacgcgacgaccgcgatcgtaaccgagcggtagcgccactggttccggcagccgatgctttagtgttggattccaccaccttaagcattgagcaagtgattgaaaaagcgctacaatacgcgcgccagaaattggctctcgcataagcgaccgaatttgcagtacccccgttgcaatggaatgacagcgggtatgttaaacaaccccatccggcatggagccaggtggacgttaaatataaacctgaagattaaacatgactgaatcttttgctcaactctttgaagagtccttaaaagaaatcgaaacccgcccgggttctatcgttcgtggcgttgttgttgctatcgacaaagacgtagtactggttgacgctggtctgaaatctgagtccgccatcccggctgagcagttcaaaaacgcccagggcgagctggaaatccaggtaggtgacgaagttgacgttgctctggacgcagtagaagacggcttcggtgaaactctgctgtcccgtgagaaagctaaacgtcacgaagcctggatcacgctggaaaaagcttacgaagatgctgaaactgttaccggtgttatcaacggcaaagttaagggcggcttcactgttgagctgaacggtattcgtgcgttcctgccaggttctctggtagacgttcgtccggtgcgtgacactctgcacctggaaggcaaagagcttgaatttaaagtaatcaagctggatcagaagcgcaacaacgttgttgtttctcgtcgtgccgttatcgaatccgaaaacagcgcagagcgcgatcagctgctggaaaacctgcaggaaggcatggaagttaaaggtatcgttaagaacctcactgactacggtgcattcgttgatctgggcggcgttgacggcctgctgcacatcactgacatggcctggaaacgcgttaagcatccgagcgaaatcgtcaacgtgggcgacgaaatcactgttaaagtgctgaagttcgaccgcgaacgtacccgtgtatccctgggcctgaaacagctgggcgaagatccgtgggtagctatcgctaaacgttatccggaaggtaccaaactgactggtcgcgtgaccaacctgaccgactacggctgcttcgttgaaatcgaagaaggcgttgaaggcctggtacacgtttccgaaatggactggaccaacaaaaacatccacccgtccaaagttgttaacgttggcgatgtagtggaagttatggttctggatatcgacgaagaacgtcgtcgtatctccctgggtctgaaacagtgcaaagctaacccgtggcagcagttcgcggaaacccacaacaagggcgaccgtgttgaaggtaaaatcaagtctatcactgacttcggtatcttcatcggcttggacggcggcatcgacggcctggttcacctgtctgacatctcctggaacgttgcaggcgaagaagcagttcgtgaatacaaaaaaggcgacgaaatcgctgcagttgttctgcaggttgacgcagaacgtgaacgtatctccctgggcgttaaacagctcgcagaagatccgttcaacaactgggttgctctgaacaagaaaggcgctatcgtaaccggtaaagtaactgcagttgacgctaaaggcgcaaccgtagaactggctgacggcgttgaaggttacctgcgtgcttctgaagcatcccgtgaccgcgttgaagacgctaccctggttctgagcgttggcgacgaagttgaagctaaattcaccggcgttgatcgtaaaaaccgcgcaatcagcctgtctgttcgtgcgaaagacgaagctgacgagaaagatgcaatcgcaactgttaacaaacaggaagatgcaaacttctccaacaacgcaatggctgaagctttcaaagcagctaaaggcgagtaattctctgactcttcgggatttttattccgaagtttgttgagtttacttgacagattgcaggtttcgtcctgtaatcaagcactaagggcggctacggccgcccttaatcaatgcagcaacagcagccgcttaatttgcctttaaggaaccggaggaatcatgaccaagtcagaattgatagaaagacttgccacccagcaatcgcacattcccgccaagacggttgaagatgcagtaaaagagatgctggagcatatggcctcgactcttgcgcagggcgagcgtattgaaatccgcggtttcggcagtttctctttgcactaccgcgcaccacgtaccggacgtaatccgaagactggcgataaagtagaactggaaggaaaatacgttcctcactttaaacctggtaaagaactgcgcgatcgcgccaatatttacggttaagttttttactcaaacttgaacgagagaaaagcacctgtcgggtgcttttttcatttctctaatctggaactggaagctgcctcgcagagttttgaacagttttcaccctttcgttaaattcttctgaatatgcctcggggaacgcaaaattcccaccagacaaccgctcaacaaagttgcacactttccataaacagggaggggtgcatgaaaataacgacagtcggtgtatgcataattagcggaatttttccgttgctgattttgccccaattgcctgggacattaacccttgcgtttctgactctcttcgcctgcgtactggcatttatccctgttaaaaccgtccgttatatcgcgctgacgttgctgtttttcgtttggggcatattatcagcaaagcaaattttgtgggcaggagaaaccttaactggcgcgacgcaggatgcaattgttgagatcactgcaactgacggcatgaccactcattacggtcaaattactcatctacaaggtcgacgtatattccctgcgtcaggtctcgtgatgtatggcgaatatcttccgcaagcggtttgtgctggacaacaatggtcaatgaaactcaaagttcgtgcagttcatggccaacttaatgatggcggctttgatagccagcgttatgccattgcccagcatcagccgctcaccggccgttttctgcaggcaagtgtcattgaaccgaattgtagcctgcgtgcacagtatctggcgtcactacaaacaacgctgcaaccctatccgtggaatgcggttattcttggtttaggtatgggggaacggttatccgtccccaaagaaatcaaaaatatcatgcgcgatactggaacggcgcatttaatggcgatatcgggattgcacatcgcttttgcggcgttgctggctgccggactcattcgcagtggacaaatttttctgcctgggcgctggatccactggcaaataccattaattggcggaatctgctgtgctgctttttatgcctggttgacgggaatgcaacctcctgcattgcgtaccatggtggcgcttgctacgtggggaatgcttaagttaagtgggcgacagtggagtggctgggatgtatggatatgttgtctggcggcaattttgctgatggatcctgttgccattctctcgcaaagtttatggctctctgccgctgcggtcgcggcattgatattttggtatcagtggtttccctgtcctgagtggcaactgccgccggtattgcgtgcagttgtttccctcatccatctgcaactgggaatcacacttctgcttatgcccgtgcaaatcgtcatatttcatggcattagtctgacctcgtttattgcaaatctattagcaattcccttggtgacatttatcacggttccgttgatcctcgccgcgatggttgtgcatttaagcgggccgttaatcctggagcaagggttatggtttcttgccgaccggtctttggctttacttttctgggggttaaagagtttgccggaagggtggatcaacattgctgaatgttggcaatggctatcattttccccatggttcttactggtggtatggcgattaaacgcctggcgaacgttgccagcaatgtgtgtggctggaggcttgctgatgtgctggccgctgtggcaaaaacctcgacctgacgagtggcagctgtacatgcttgatgtcgggcaagggctggcaatggtgatagccagaaacggcaaagcgattctctatgacacaggactggcctggcctgaaggggatagtgggcaacaactgattatcccctggctccactggcataatcttgaaccggaaggcgttattctgagccatgaacatctggatcaccggggagggctggattcaatattgcatatatggccgatgttatggatcagaagtccgttaaactgggaacatcatcagccctgtgtgcgtggcgaagcgtggcaatggcaaggattgcgtttcagcgcgcactggcctttacaaggtagcaacgataaaggaaataaccattcctgtgtggttaaggttgatgacgggacgaatagcattcttctaaccggtgatattgaagccccagctgaacaaaagatgctaagccgttactggcagcaagtgcaggcaacattgcttcaggtacctcaccatggcagtaatacctcatcatcgttgccattaattcagcgagtgaatggaaaagtggcactcgcatcggcatcgcgctataacgcatggcgactgccctctaacaaagttaagcatcgctatcaactgcaaggatatcaatggattgatactccacatcaaggtcaaacaacggtcaatttttcagcgcaaggctggcggattagcagcctcagggagcaaattttacctcgttggtatcatcagtggtttggcgtgccagtggataacgggtagaatatgcggctatttcaacaaatgctggttttttgaatgcataacgacaaagatctctctacgtggcagacattccgccgactgtggccaaccattgcgcctttcaaagcgggtctgatcgtggcgggcgtagcgttaatcctcaacgcagccagcgataccttcatgttatcgctccttaagccacttcttgatgatggctttggtaaaacagatcgctccgtgctggtgtggatgccgctggtggtgatcgggctgatgattttacgtggtatcaccagctatgtctccagctactgtatctcctgggtatcaggaaaggtggtaatgaccatgcgtcgccgcctgtttggtcacatgatgggaatgccagtttcattctttgacaaacagtcaacgggtacgctgttgtcacgtattacctacgattccgaacaggttgcttcttcttcttccggcgcactgattactgttgtgcgtgaaggtgcgtcgatcatcggcctgttcatcatgatgttctattacagttggcaactgtcgatcattttgattgtgctggcaccgattgtttcgattgcgattcgcgttgtatcgaagcgttttcgcaacatcagtaaaaacatgcagaacaccatggggcaggtgaccaccagcgcagaacaaatgctgaagggccacaaagaagtattgattttcggtggtcaggaagtggaaacgaaacgctttgataaagtcagcaaccgaatgcgtcttcaggggatgaaaatggtttcagcctcttccatctctgatccgatcattcagctgatcgcctctttggcgctggcgtttgttctgtatgcggcgagcttcccaagtgtcatggatagcctgactgccggtacgattaccgttgttttctcttcaatgattgcactgatgcgtccgctgaaatcgctgaccaacgttaacgcccagttccagcgcggtatggcggcttgtcagacgctgtttaccattctggacagtgagcaggagaaagatgaaggtaagcgcgtgatcgagcgtgcgactggcgacgtggaattccgcaatgtcacctttacttatccgggacgtgacgtacctgcattgcgtaacatcaacctgaaaattccggcagggaagacggttgctctggttggacgctctggttcgggtaaatcaaccatcgccagcctgatcacgcgtttttacgatattgatgaaggcgaaatcctgatggatggtcacgatctgcgcgagtataccctggcgtcgttacgtaaccaggttgctctggtgtcgcagaatgtccatctgtttaacgatacggttgctaacaacattgcttacgcacggactgaacagtacagccgtgagcaaattgaagaagcggcgcgtatggcctacgccatggacttcatcaataagatggataacggtctcgatacagtgattggtgaaaacggcgtgctgctctctggcggtcagcgtcagcgtattgctatcgctcgagccttgttgcgtgatagcccgattctgattctggacgaagctacctcggctctggataccgaatccgaacgtgcgattcaggcggcactggatgagttgcagaaaaaccgtacctctctggtgattgcccaccgcttgtctaccattgaaaaggcagacgaaatcgtggtcgtcgaggatggtgtcattgtggaacgcggtacgcataacgatttgcttgagcaccgcggcgtttacgcgcaacttcacaaaatgcagtttggccaatgatcgaaaaaatctggtctggtgaatcccctttgtggcggctattgctgccactctcctggttgtatggcctggtgagtggcgcgatccgtctttgctataaactaaaactgaagcgcgcctggcgtgcccccgtaccggttgtcgtggttggtaatctcaccgcaggcggcaacggaaaaaccccggtcgttgtctggctggtggaacagttgcaacagcgcggtattcgcgtgggggtcgtatcgcggggatatggtggtaaggctgaatcttatccgctgttattgtcggcagataccacaacagcacaggcgggtgatgaacctgtgttgatttatcaacgcactgatgcgcctgttgcggtttctcccgttcgttctgatgcggtaaaagccattctggcgcaacaccctgatgtgcagatcatcgtaaccgacgacggtttacagcattaccgtctggcgcgtgatgtggaaattgtcgttattgatggtgtgcgtcgctttggcaatggctggtggttgccggcggggccaatgcgtgagcgagcggggcgcttaaagtcggttgatgcggtaatcgtcaacggcggtgtccctcgcagcggtgaaatccccatgcatctgctgccgggtcaggcggtgaatttacgtaccggtacgcgttgtgacgttgctcagcttgaacatgtagtggcgatggcggggattgggcatccgccgcgcttttttgccacgctgaagatgtgtggcgtacaaccggaaaaatgtgtaccgctggccgatcatcagtctttgaaccatgcggatgtcagtgcgttggtaagcgccgggcaaacgctggtaatgactgaaaaagatgcggtgaaatgccgggcctttgcagaagaaaattggtggtatttgcctgtagacgcacagctttcaggtgatgaaccagcgaaactgcttacgcaactaaccttgctggcttctggcaactagttacgccgcggcagcgttcgattgatggagtcatgaatgtcgctgccgcacctctcccttgctgatgcgcgtaatcttcaccttgccgcacaaggcctgttaaacaaaccccgccgtcgagcgtcgttggaggatattccggcaacgatctcccgcatgtccttgctgcaaatcgataccatcaatattgttgcccgtagtccatatctggtgcttttcagtcgtctgggaaattatcctgcccagtggctggatgagtctctggcgcgtggcgaattaatggaatactgggcgcatgaagcctgctttatgccgcgtagcgactttcgtcttattcgccaccgcatgctggcacctgaaaaaatgggctggaaatacaaagacgcctggatgcaggaacatgaggcggaaattgcacagttaattcagcatattcatgataaggggccggtacgttcagccgattttgagcatcctcgtaaaggtgcaagcggctggtgggaatggaagccgcataaacggcatctggaaggtttatttactgccggaaaggtgatggtgattgaacggcgcaacttccagcgcgtttatgatttaacccaccgtgtcatgcctgactgggatgatgagcgcgatctcgtttcgcaaacagaagcagaaatcatcatgctggataacagtgcgcgtagcctgggaatattccgcgaacagtggctggcagattactatcggctgaaacgtccggcactggcggcgtggcgcgaagcgagggctgaacagcagcaaatcattgctgtgcatgttgaaaaattgggcaatctttggctgcatgatgatttgctgccgctactcgagcgagcgctggccggaaagctcactgcaacgcacagcgcggtactttcgccttttgatcctgttgtctgggatcgcaaacgcgcagagcagctttttgattttagctaccggctggagtgctataccccagcgccgaaacgccagtatggctattttgttctgccgttattacatcgtgggcaattagttgggcgaatggatgccaaaatgcatcgccagacaggcatccttgaagttatctctctgtggttacaggaaggtattaaaccaacgacaacgctgcaaaaagggctacgtcaggcgattactgatttcgctaactggcagcaggcaacgcgggtgacattaggatgctgcccgcaaggcctctttactgattgccgcaccggctgggaaatagaccccgtcgcataaatgattatgataagatttatgcattcataacccgatccatctggaggaactatggatcatcgtctgcttgaaatcattgcctgcccggtttgcaacggaaaactttggtataaccaggaaaaacaagagcttatttgcaaactggacaacctcgctttcccgctgcgtgatggcattccagtgttgctggaaacggaagcccgcgtgctgactgctgatgagagtaaatcatgagttttgtggtcattattcccgcgcgctacgcgtccacgcgtctgcccggtaaaccattggttgatattaacggcaaacccatgattgttcatgttcttgaacgcgcgcgtgaatcaggtgccgagcgcatcatcgtggcaaccgatcatgaggatgttgcccgcgccgttgaagccgctggcggtgaagtatgtatgacgcgcgccgatcatcagtcaggaacagaacgtctggcggaagttgtcgaaaaatgcgcattcagcgacgacacggtgatcgttaatgtgcagggtgatgaaccgatgatccctgcgacaatcattcgtcaggttgctgataacctcgctcagcgtcaggtgggtatggcgactctggcggtgccaatccacaatgcggaagaagcgtttaacccgaatgcggtgaaagtggttctcgacgctgaagggtatgcactgtacttctctcgcgccaccattccttgggatcgtgatcgttttgcagaaggccttgaaaccgttggcgataacttcctgcgtcatcttggtatttatggctaccgtgcaggctttatccgtcgttacgtcaactggcagccaagtccgttagaacacatcgaaatgttagagcagcttcgtgttctgtggtacggcgaaaaaatccatgttgctgttgctcaggaagttcctggcacaggtgtggatacccctgaagatcttgagcgcgttcgcgctgaaatgcgctaatttcacttcacgacacttcagccaattttgggaggagtgtcgtaccgttacgattttcctcaatttttcttttcaacaattgatctcattcaggtgacatcttttatattggcgctcattatgaaagcagtagcttttatgagggtaatctgaatggaacagctgcgtgccgaattaagccatttactgggcgaaaaactcagtcgtattgagtgcgtcaatgaaaaagcggatacggcgttgtgggctttgtatgacagccagggaaacccaatgccgttaatggcaagaagctttagtacgcccggaaaagcccgacaactggcatggaaaaccaccatgctggcaagaagtgggactgtccgtatgccgactatttatggtgtgatgacgcatgaagaacaccccggccccgatgtcctgctactggagcggatgcgtggtgtttcggtggaggcaccagcccgaacaccagaacgctgggaacaactcaaagaccaaatcgttgaagccttactggcctggcaccgtcaggacagtcgcggttgcgtcggcgcggtcgacaatactcaggaaaatttctggccctcatggtaccggcaacatgttgaagtgctatggaccacgctcaatcagttcaataacaccggtctgacgatgcaggataagcggatcctgtttcgcactcgcgaatgtctcccggcattatttgaaggctttaacgacaattgtgtgctgattcacggtaacttctgtttacgcagcatgttgaaagattcgcgcagcgatcagttactggcgatggtcgggccgggactaatgctttgggcaccgcgagaatacgaactgttccgactaatggataattctctggcggaagatttgctctggagttacctgcaacgcgcgccagtggcggagtcgttcatctggcggcgttggttgtatgtgttatgggatgaagttgcgcaactggttaataccggacgatttagtcggcgcaacttcgatctggcatcaaaatcactcttgccgtggctcgcctgacgaaccttttagccactgccagatacggccaagcgtttcatagccaacacgatcgctatgcatcaaccagaccggagaagggattgcccgttcccacgggttaagcggcgagtcgatggccaactgattcgccggggctggtagcggatttaacccttcctgctgaaaaaagatcatcgcccgcggcagatgtgatgcggaggtcaccagcaggaaaggggcgtcaccaatcgcctgtttcactgctgcagcttcttcttcggtatcttttggcaaatccagggtgataatttgctcgcgcggcacgcccagcgattgcgcaactctggcacctacttccgctgtactcaccgtattggtttttgctacgcctcccgtgaagatcagttttgatcccggattttcgcgccataagcgaataccttcattcaggcgtggcagactgttattgattaaattagagctcggtgcccactgcgggttccaggtataaccacctccgagcaccacgatatagtccactttttgcgaattattccatgtcggataggtgctttcgatgggacgcagcaggcggtcggctaccggttgcaaactcaataacaagagcgccagccacccaatgctaataaaaatcttcccggttttttgaaaacggctaaaccacagcagcgccaggccagcgccaataatcaacaacatcagcggaagtggcagcaacatattgccaatcacttttttcagtgtaaaaagcatcctttctggttccttttttaaccatatagcaagggatcgccagcgatattacaccagacgggttcattctcgccgtggctgtgacaaaatagcgtctttatcagaaaacgtcttagccaaccggtggagaaagcaatgcaggatcgcaattttgatgatattgcggaaaagttttcccgtaacatttacggcaccaccaaagggcagcttcgacaggctattctgtggcaggatctcgatcgcgtgctggcggaaatgggcccgcaaaaactgcgtgtgctggatgctggcggtggagaagggcagaccgcaatcaaaatggccgagcgtgggcatcaggtcattttatgcgatctttctgcgcagatgatcgaccgcgcaaaacaggcggcagaagcaaaaggtgtgagcgacaacatgcaatttatacattgcgccgctcaggatgttgcttcgcatttggaaacgcccgttgatctgatattgttccatgcggtgctcgagtgggtggctgatccccgcagcgtattgcagaccctctggtcagtgttgcgtccaggcggcgtgttgtcgttaatgttctacaatgcgcatggtttgttgatgcataacatggtcgccgggaattttgattacgtgcaggcgggaatgccgaaaaagaaaaaacggacgctttcgccagattatccacgcgacccggcgcaggtttatctgtggctggaagaagctggttggcaaattatgggtaagacaggcgttcgcgtgtttcatgattatctgcgcgagaaacaccagcagcgcgactgctatgaagcattacttgaattagaaacgcgttattgccgtcaggaaccgtatattaccctggggcgttatattcatgtcaccgcgcgcaaaccgcagagcaaggataaagtatgagtgaattttcccagacagtccccgaactggttgcctgggccagaaaaaatgacttctccatctcgctgccggtagaccgactctcttttctgctggcggttgccacgctgaacggcgagcgtctggatggtgagatgagtgaaggcgagctggtggatgcattccgccatgtgagtgatgcgtttgagcaaaccagcgaaaccatcggcgtgcgcgccaataacgcgatcaacgacatggtgcgtcaacgtctgctgaaccgctttaccagcgagcaggcggaagggaacgcaatttaccgtctgacgccgctcggcatcggcattactgactactacatccgtcagcgcgagttttctacgctgcgtctttctatgcagttgtcgattgtggcgggtgagctcaaacgcgcagcagatgccgccgaagagggcggtgatgaatttcactggcaccgtaatgtctatgcgccactgaaatattcggtagcagaaattttcgacagtatcgacctgacgcaacgtctgatggacgaacagcagcagcaggtgaaggacgatatcgcccagttgctgaacaaagactggcgggcggcgatttccagctgtgaattgttgctttcggaaacttccggaacgctgcgtgaattgcaggatacgctggaagcggcaggcgacaaattgcaggctaatctgttgcgcattcaggatgcgacgatgacccatgacgatctgcatttcgtcgatcgtctggtgttcgatctgcagagcaaactcgatcgtattatcagttggggccagcaatccatcgacttgtggattggctacgaccgccacgtacacaaatttattcgtaccgcgatcgatatggataaaaaccgcgtctttgctcagcggttacgtcagtcggtacaaacctattttgatgagccgtgggcgctaacttatgccaatgccgatcgtctgctggatatgcgtgacgaagagatggcactgcgcgatgaagaagtgactggggaacttcctgaggatctggaatacgaagagtttaacgagatccgcgaacagctggcggcgatcatcgaagaacaacttgccgtgtacaaaaccagacaagtgccgctggatcttggtctggtggtacgcgaatatctgtcacagtatccgcgtgcacgtcactttgacgttgcgcgtattgttattgatcaggcggtacgtcttggcgtagcgcaagcagatttcaccggactgccagcgaaatggcagccgattaatgattacggagccaaggtacaggcgcatgtcatcgacaaatattgaacaagtgatgccggttaagctggcgcaggcgctggcgaatccgttatttccggcgctggacagcgccttacgttcaggacgccatattggcctcgacgaactggataatcatgcattcctgatggattttcaggaatatctggaagagttttacgcgcgttataacgttgagcttattcgcgcaccagaagggttcttctatttacgcccacgttccaccacgctgatccctcgttccgtcttgtcggaactggatatgatggtcgggaaaatcctctgttatctctatctcagcccggaacggctggcgaatgaggggattttcacccagcaggaactgtacgacgaactgctcaccctggccgatgaagcaaaactgctgaaactggtgaacaaccgttcaaccggttcagacgttgaccgtcagaagttgcaggagaaagtacgttcttcgctcaaccgtctgcgtcgtttaggcatggtgtggtttatgggccacgacagcagcaagtttcgcattaccgaatcggtgttccgcttcggagccgatgtgcgtgctggcgacgatccccgtgaagcacagcgtcgcctgattcgtgatggcgaagcaatgccgattgaaaatcatctgcaactcaacgatgaaaccgaagagaatcagccagatagcggagaggaagaataatgattgaacgcggtaaatttcgctcactgacgctgattaactggaacggcttttttgcccgaacttttgaccttgacgagctggtcacgacgctttctggcggtaacggggcgggtaaatccaccaccatggcggcgttcgttacggcgctgatccccgacctgaccctgctgcatttccgtaacactacggaagccggggccaccagcggttcgcgcgataaaggtctgcacggtaagctgaaagcgggtgtctgttattcgatgctcgacaccattaactcgcgccaccagcgcgtggtggtcggtgtgcgtctgcaacaggttgccggacgcgatcgtaaagtggatatcaagccgtttgccattcagggactgccgatgtcggtgcagccgacacagctggtgaccgaaaccctgaacgaacgccaggcgcgcgtgctgccgcttaacgagctgaaagacaagctcgaggcgatggaaggcgtgcagtttaaacagttcaactccattactgattaccactcgctgatgttcgatctgggcatcatcgcgcgtcgtctgcgctccgcatctgaccgtagcaaattctatcgtctgatcgaagcttcgctgtatggcgggatctccagtgccattacccgttctctgcgcgactacctgttgccagaaaacagcggcgtgcgtaaagcgttccaggacatggaagcggcgctgcgtgaaaaccgtatgacgctggaagcgattcgtgtcacccagtcggaccgcgacctgtttaagcatctgatcagcgaagccaccaactacgtggcggcggactacatgcgtcacgccaacgagcgccgtgtccatctcgacaaagccctggagtttcgtcgcgagctacatacttcgcgtcagcaactggcggctgagcagtacaaacacgtcgatatggcgcgtgagctggcagagcacaacggtgccgaaggcgatctggaagcggattatcaggcggccagtgatcacctgaacctggtgcaaaccgcactgcgtcagcaggagaagatcgaacgctacgaagcggatctcgatgagctgcagatccgtctggaagagcaaaatgaagtggtggcagaagccatcgaacgccagcaagagaatgaggctcgtgcggaagctgccgaactggaagtggacgagctgaaaagccagcttgctgactaccagcaggcgctggacgtccagcaaacgcgcgcgatccagtataaccaggcgattgctgcgcttaatcgtgccaaagaactgtgccatctgccggacttaaccgccgactgcgccgccgaatggctggaaaccttccaggcgaaagagctggaagcgactgaaaaaatgctctctcttgagcagaaaatgagcatggcgcaaaccgcgcacagccagtttgagcaggcttatcagctggtggtggcaatcaacggcccactggcgcgtaacgaggcgtgggatgtcgctcgcgaactattgcgcgaaggggtcgatcagcgtcacctggcagagcaggttcagccgctgcggatgcgattaagcgaactggaacagcgtctacgcgagcagcaagaagctgagcgtctgctggcagatttctgcaaacgtcagggcaagaattttgatatcgacgaactggaagccctgcatcaggaactggaagcacgcattgcctctctttccgatagcgtgtctaacgcccgtgaagagcgcatggcactgcgccaggagcaggaacagctgcagtctcgcattcagagtttgatgcagcgtgcgccggtttggctggcagcgcaaaacagtctcaaccagttgagcgaacagtgcggcgaagagtttacctccagccaggacgtcaccgaatatctgcaacagttgctggagcgtgagcgagaggcgattgttgaacgcgatgaagtgggcgcgcgcaaaaacgccgtcgatgaagagatcgaacgtttaagccagcctggcggctctgaagatcagcgtctgaacgcgctggcggagcgttttggtggtgtgctgctgtcagaaatttatgacgacgttagcctggaagatgcgccgtacttctcagcgctgtatggcccgtcacgccacgccatcgtggtgccagatctgtcacaggtaactgaacacctggaaggcttgaccgattgcccggaagatctctatctgatcgaaggagatccgcagtcattcgatgacagcgtgttcagcgttgatgagctggaaaaagcggtagtggtgaaaatcgccgatcgtcagtggcgttattcacgtttcccggaagtgccgctgtttggtcgtgctgcgcgtgaaagccgtattgaaagcctccatgccgagcgtgaagtgctttccgaacgcttcgccacgctctcctttgatgtacagaaaactcagcgtctgcatcaggcgttcagccgctttatcggcagtcatctggcggttgcgtttgagtctgacccggaagcagaaatccgtcaactgaacagccgtcgcgtcgaactggagcgggcgttaagtaatcatgaaaatgataaccagcagcagcgtattcagtttgagcaggcgaaagagggcgttacggcgctgaaccgcattctgccgcgtctcaacctgttggctgatgacagcctggcggatcgcgtcgatgaaatccgcgaacgtctggatgaagcccaggaagccgcgcgttttgttcagcagtttggcaatcaactggcgaaactggaaccgattgtttcggtattgcagagcgacccggaacagttcgaacagttaaaagaagattacgcgtactctcagcagatgcagcgcgatgcccgtcagcaggcgtttgccctgacggaagtggtgcagcgtcgtgcgcactttagctattctgactcggcagaaatgcttagcggtaacagcgatctcaacgaaaaactgcgtgaacgtctggaacaggcggaagcggagcgtacccgcgctcgcgaagcgttgcgcggtcacgcagcgcagttgagtcagtacaaccaggtgctggcttcgctgaaaagttcttacgacaccaaaaaagagctactcaacgatctgcaacgtgaattgcaggatatcggcgtgcgtgctgatagcggggcagaagagcgggcgcgtattcgccgtgacgagctgcatgcgcaactgagcaataaccgttcacgccgcaatcaactggaaaaagcgcttaccttctgcgaagcggagatggacaacctgacccgcaaactgcgcaagctggagcgggattactttgagatgcgcgagcaggtagtgaccgccaaagcgggctggtgtgcggtgatgcgcatggtgaaagataacggcgttgagcgccgcttacaccgtcgtgagctggcttatctctccgctgatgatttgcgttccatgtcggataaggcgttaggtgcgctgcgtctggcggtggcggataacgaacatctgcgcgacgtgctgcgcatgtcggaagatccgaaacgtccggagcgtaaaattcagttcttcgtggcggtttatcagcatctgcgtgaacgtattcgtcaggatattattcgtaccgatgatccggtggaagctatcgaacagatggagattgaacttagccgtctgaccgaagaattaacctcccgtgaacagaaactggcgatcagttcccgcagcgtggcgaacatcattcgcaaaaccattcagcgcgagcagaaccgtatccgtatgctcaaccaggggttgcagaacgtatcgtttggtcaggtgaacagcgtgcgtctcaacgtgaacgtgcgtgaaacgcacgccatgctactggatgtgctctctgaacagcacgagcagcatcaggatctgtttaacagcaaccgtttgaccttctcggaagcgctggcgaaactgtatcaacgtcttaacccgcagattgatatggggcagcgcacgccgcagaccatcggtgaagaactgctggattaccgcaactatctggaaatggaagttgaggttaaccgtggttccgatggctggctgcgcgcagagtctggtgcattgtcgaccggtgaggcgattggtaccggtatgtcgattctggtgatggtggtacaaagctgggaagatgaatctcgccgcctgcgcggtaaagatatctctccttgccgcctgctgttcctcgatgaagcagcgcgactggatgctcgttctatcgccacgctgtttgaattgtgtgagcgtttgcaaatgcaactcatcatcgcagcgccggaaaatatcagcccggagaaaggcaccacctataaactggtgcgtaaagtcttccagaataccgaacacgttcatgtcgtcggcctgcgaggatttgcgccgcaactccctgaaacgcttccaggaactgacgaagcgccttctcaggcgagttaaaattaaggcggcagcaatgccgccttttctttttccgaaaactccgtttctgcactaaaaaagtggcacattacggcgcgcttttctttaaacttctttacattaggttatgtaaaaacgtatcggcgtttatatactgaagataagcctgatgagtaacaggcttgctcgtcatactttcgtgagtattggcgttgtacaggcaagtcgtaaaataacagcctggctattcagagtatgataaaaacagggggcaagggatgttgcttaatatgatgtgtggtcgtcagctgtcggcaatcagtttgtgcctggccgtaacattcgctccactgttcaatgcgcaggccgatgagcctgaagtaatccctggcgacagcccggtggctgtcagtgaacagggcgaggcactgccgcaggcgcaagccacggcaataatggcggggatccagccattgcctgaaggtgcggcagaaaaagcccgcacgcaaatcgaatctcaattacccgcaggttacaagccggtttatcttaaccagcttcaactgttgtatgccgcacgcgatatgcaacccatgtgggaaaaccgtgatgctgttaaagccttccagcaacagctggcagaggtggcgattgccggtttccagccgcagtttaataaatgggtagagttactgaccgatcctggtgttaacgggatggcacgcgacgtggtgctctctgatgcgatgatgggctatctccatttcattgcaaatattccggtcaaaggcactcgctggctatatagcagtaaaccttatgcacttgcaacgccgccgctctcggtgattaaccaatggcagctggcgctggataaaggtcaattgcctacgtttgttgcaggactggcaccgcagcatccgcaatatgcggcgatgcatgaatcgttactggccttactctgtgacaccaaaccgtggccccaactgaccggcaaagcaacgttgcgcccagggcagtggagtaacgacgtaccggcgttgcgcgaaatattgcaacgcacaggcatgttggacggggggccgaaaattactctacctggcgatgacacgccaactgacgcggtagtcagcccatccgctgttactgttgaaacagcagaaactaagccgatggataagcaaacgacgtctcgtagtaaacctgcgcctgccgttcgcgccgcctacgataatgaactggtggaagccgttaaacgttttcaggcatggcaaggattgggggcagatggtgctattggcccggcaacacgtgactggttaaacgtaacgcccgcccagcgtgctggtgtgttggctctcaacatccagcgattgcgcttgctgccaacagagctttctaccgggatcatggttaacattccggcctattcgctggtctactatcagaacggcaatcaggtgctggattcgcgagtcattgtcggtcgccccgatcgcaaaacgccgatgatgagcagtgcccttaacaacgtagtggtaaacccgccgtggaacgtacctccaactctggcacgcaaagatattctgccaaaagtgcgcaacgatccgggatatctcgaaagccatggctatacggtgatgcgcggctggaacagcagagaagcgattgacccatggcaggttgactggtctacaatcacggcctcgaatttaccgttccgcttccagcaggctccaggcccacggaactcgctggggcgctataaattcaatatgccgagttcagaggccatttatttgcatgacacgccgaaccacaatctgttcaagcgtgatacacgcgcattgagctcaggctgtgtacgagtgaataaagcttccgatctggcgaatatgctgttgcaggatgcaggctggaatgacaaacgtatttctgatgcgctgaagcagggtgatacacgttacgtcaatattcggcagtcgattccggtgaatctctactacctgacggcctttgttggtgcagatggtcgtacccagtatcgtacagatatttacaattatgatctgcctgcgcgatccagctcgcaaatcgtatcgaaagcggaacaattaatcaggtaaatgaagtagttcggggaaatcagttgtcgtaataattagcatgattgggggcgattctctgcagcccccgtcactgctggggttgagtcatcttgacgtctgctttacgggcggttaaggtgcctcttgtgcgccagaagtgcatataaacgataacattgacctgtagacttgattatcatggacaaattcgacgctaatcgccgcaaattgctggcgcttggtggcgttgcactcggtgccgccatcctgccgacccctgcgtttgcaacactctctaccccacgcccgcgcattttgacactcaataatcttcataccggagagtcaatcaaagcggagtttttcgatggcagaggctatattcaggaagaattggcaaaacttaaccattttttccgcgattaccgcgcgaacaaaataaagtccatcgacccaggattattcgaccagttgtatcgcctgcaagggttgttaggcacgcgcaaaccggtgcaactcatttccggttatcgttctattgataccaacaatgaactacgcgcccgcagccgtggagtagcgaagaaaagctatcacactaaaggccaggcgatggatttccatattgaaggtatcgcgttaagcaatattcgcaaagccgcgttatctatgcgcgcaggtggtgtaggatattatccacgtagtaactttgtgcatattgataccgggccagcacggcactggtagtaattgcttaacgaaacaggggcagtatgaactatcgtattattccggtcaccgcattctcccagaactgttcattaatctggtgtgaacaaacccgtctggccgcactggtcgatcctggcggcgatgcggaaaaaatcaaacaggaagttgatgacagcggcctgacactgatgcagatcctgctgacgcatggtcatctggaccacgttggcgcagcggcggaactggcgcaacattacggcgtgccggttttcggcccggaaaaagaagatgagttctggctgcaaggcttgcctgcgcaaagtcgtatgtttggtctggaagagtgccagccgctgacgccagatcgttggctgaacgaaggcgataccatcagcatagggaatgtgactttacaggtgttacattgccctgggcatacgccgggtcatgtcgtgttttttgatgatcgggcaaagctgctgatttctggcgatgttattttcaaaggcggagtagggcgcagtgacttcccgcgtggcgatcataatcaactgatttcttcaatcaaagataaattgctgccactgggggatgacgtgatatttattccgggtcacggaccattatccacacttggttatgaacgcctgcataatcccttcctgcaagacgaaatgcccgtctggtaaggcacataaaaaagcccgcttttaatgctggcctggatttctggcaaagtgcgctttgtttatgccggatgcggcacgagcgccttatccggcctacaaaatcgtgcaaattcaaaatattgcaggggacgcgtaggcctgataagcgtagcgcatcaggcaatgttgcgtttgtcatcagtctcagcccgcttttcagcgggcttcattgtttttaatgcttacagcactgccacaatcgcttcgcacagcggagccatgttatctggtgtcatcccggccacatttacgcgaccagaagcaaccgcatatacgccaaactcttcgcgcagacgcagcacttgttcttttgtcaggccactgaaggagaacatgccgttctgtttgatgataaagctgaagtcgcggtttgcgcctttttcctgcagcgtattgacgaacaactgacgcatacgctgaatacgctggcgcatatcagtcagctcttgttcccaaatcgcacgtaacgcatcgttgctcaggatggtggcaacaacagaagcgccgtgtgctggtgggttagagtagttagcgcgaatcgccgctttcatttggctgaatgcgcgatcaacggtttcactgtcggcagcaaccagagtacaagcgccaacacgctcgttgtacaggccaaagtttttagagtaggaactggcaacaatcagctctttatgcatagccgcgaaagcgcgcagtccttcagcatcttcttccagaccacgggcaaaaccctggtaagcgaagtcaaacagcggtaaccagcctttctcaacggagagttgtgccagtgtttgccattgttccagcgtagggtcgataccggttgggttatggcagcagccatggaacagcactacgtcgccagcctgagcttcattcaggctgttaatcagtgcatcgaagtcaagagtgtgattttccgcatcataataagcgtattcacgaacttccagacctgcagagttaaagacgctcttatggttcggccagcttgggttgctcacccacacacgcttaacgctggtattttttgccaggaaatcggcagccacgcgtagtgcgccagtgccccccggagtctgtgccgtgcgagcacgtttgtcattgatcagggcgctacctttaccaaacagcagttcctgagtgcagcgaccaaattcagggatgccgtcaatgccgaggtaatttttggtggtttcattttcgagcagatactgttcagcctttttcacgctggtcagtaccggggttttgcccgtctcatctttatagacaccaatcccgaggttaattttgccgggacgttcatcggcacgaaacagatcggccaggcccagaatcgggtcggcaggagcggcggtaatgttctcaaacatgacgaggttccattatggttacagaagggaagtccgctatcagggtaacgggagatttacaaaattccaactattactgatgaaaacgcaggctgtttttgcaagacgtgagattgctctggaaggtataaaaaaaacaggaccaaagtcctgttttttcggcatttaacaaagaggtgtgctattagaactggtaaacgatacccacagcaacggtgtcgtctgaacctacgcccagtttgttgtcagaatcgatctggttgatgatgtagtcaacataggtggacatgtttttgttgaagtagtaggttgcgcccacttcaaagtagttcaccagatcaacatcaccgataccttctacgtctttcgctttagatttggtgtaagcgatggacggacgcagaccgaaatcgaactggtattgcgcaactaacagaacgtcttgcgttttgttggcgaagccgctggtgtttgtaaatttattagtgatcggcgtagcgttacgggtttcaccgtagttcgctgccaggtagatgttgttcgcgtcgtacttcagaccagtagcccactgttcagcttttttaccgttgccaagaggttgagcttcttgcaggttggtacggtcagctgcaccataagcaccaacgataccaaagccttcgtattcgtagctgatagaaccgccaacaccgtcgccgttagaacggcgtgcagtgtcacgctcgtttttacccaggtactgaacagcgaagttcaggccatcaaccagaccaaagaagttggagttacgataggtagcaacgccgccaacacgaccaacgaagaagtcatcgctgtatgcagtatcaccaccaaattctggcagcatatcggtgtaacccagtgcatcataaaccacaccgtagttacggccgtaatcgaaagaaccaacgtcagcgtatttaagacccgcgaatgccagacgcgttttgttaccagtttgagcgtcagcgccttcagagttgttaccctggaagttatattcccactgaccataaccggtcagatcggaattgatttgagtttcccctttaaaaccaagacgggcataggtcatgtcgccattgccaccgtaactgttttcaccgttacccttggaaaaataatgcagaccaacagctttaccgtacagatctactttgttgccatctttgttatagatttctgcagcgtttgcagtacctgctactaacagagcagggacgatcactgccagaatattgcgcttcatcattatttattaccctcatggttttttttatgacacctgccactgccgtcaataagttctgtcaataaaaatttacggaactattgatgagagtttggtgtctttatgtgtctgcaggcatctttccattcaaactaacgtttcgctaccgtgaaagtgctacaaagataaagatttggtttcaaaaagaaaaaatatgtaaccaaaagtaaaatttaaggaactttgtgaacaccgtcatatttccatagagacgtgatgatatttacagcaattttaatctatttatatgatttccttatatttaaattaactaaacggaaattttgtttctgatggaaactttatcgacctggcacaaaatcttctttcagacatccagaatgccaaaaaatagtatgaaaattgtgctattagctaagaaaaaactaatccgcaataagaatgcggattagtttttgcgcgtaaatgttgcaatgtaatattccgtaacaggatgatcgttatggcggggttgcaaatagattgcttgacttaacaaacagataacttgacagaaaagataaaaaaagagccagcgggcgctggctcttgaagacgctaaattagaagctggcgttacgcggagtacgtgggaacggaatcacatcacgtacgttttgcacgccagttacgtaagcaatcagacgttcaaaaccaagaccgaaacctgaatgcggaacagtaccgtagcgacgcagatcgcgataccaccagtaatcttctttattcaggcccatttccagcatacgctcgtccagcacgtccagacgttcttcacgctgggagccaccaatgatctcaccgatgcccggagccagaacgtccatagccgcaacggttttaccgtcttcgttaaggcgcatatagaacgctttaatatctttcggatagtttttaaccactaccggtgctttaaagtgttcttccgccagataacgctcatgctcagaagagagatcgactccccagtaaaccgggttttcaaacttcctgccgcagttttcgagaatggtcactgcgtcggtataatccacctgcgcaaaatcggcttcaatgaagcgttccagacgtgaaacggcatctttatctacgcgttcagcgaagaatttcatgtcgtcagcgcgttcttcgagaaccgctttgaagacatatttcagcatggcttcagccagacccgcaatatcgttcaggttagcaaacgccacttccggctccagcatccagaattccgccaggtgacggctggtgttggagttttcagcacggaaagtcgggccgaaggtataaattttggacaatgcgcaagcgtaggtttcgccgttcaactggccagatacggtcaggaaagactctttaccaaagaagtctttgtcgaaatccactttgccctgatcgttacgcggcaggttttccagatccagcgtagaaacgcggaacatttcgcctgcaccttcggtatcagatgcggtaatcagtggcgttgaaacccagaagaatccctgctcgttaaagaagcgatgcagcgcctgcgccagcgtatggcgaacgcgcgcgacggcaccaatcaggtttgtgcgcggacgcaggtgagcgacttcacgcagatactcaatgctgtggcgttttgccgccatcgggtaagtgtctggatcttcaacccaaccagcaacttcaaccttgctggcctgaatttcaaattgttgcccctggcccggcgacgccacgactttacccgtcacaatgaccgagcagccggtggtcagacgcaggacgtcttcattgtaattgggcagagaattattgatgacagcctgtacaggatcaaagcaggaaccgtcataaacggcgaggaaggagatgccagcttttgaatctcggcgggtacgtacccatccgcgcacggtgacttcgctgtcaacggctacacggccctggagtacgtcggctacaggcacaacgctcataatattctctctgttaatagtcggaaaaaataaacacttgtccacccgtaaatggggggatacctatgttacctggcatctgcaatcagacaagcagaattcgcaaatgcagcgaaagatttcggaattaaaggtaaaaaaagggagccgattagctccctgatgatattaactggcttttttaatatgcggaaggtcgaacgctttgcgcagcgcccgaacaaacgctttatcatggcagatagttttgccagggctgtcagaaagtttcgccaccggtttaccgttacactctaccaacttaatgacaatattcaggggttttacctgggggatatcgcaggtcaggcgagtcccaataccaaaacttaattgcacgcgggaagagaagtggcggtatagctcaaccgctttgcgtaaatccagattgtcagagaaaaccagcgttttactctgtggatcaattcccagcttttcataatgtgcaatggctttttcaccccattcaaccgggtcgccagagtcatgacgcaggccctgataccgactagcgaactcgacaccgaaatcacgcaggaaagcatccatagtgatgcagtcggttaatgcaatgccaagttggtcgggatactcttccagccaggcagcaagtgcagctcgctggctgttggctagatccgggctgatttgctgatgtgcctggaaccattcgtgtgcctgtgttcccatcggcgtgagggaaagccgacgcgccagatcgtagttgctggtgcccacaaaccaggattcctgttgcagacgcttaacgatggtttcttgtacttcgcgagaaaaacggcgacgggtgccaaaatccatcagatggaagcgcgacatatcaagaccggcggttaacgccgagaagtcgactaatttgctttccagcgtgtcgagggcttgcgcaacgtcggcctgcggtgagcgatagcgatgtaccatttcactgataaccgccagcaaaggaacttcccagaggatgacttcacgccacgggccgcttaaacgaatatccagcttgccattatcgttggacacggtgacttgttccgggttaaagcggaactcgcgtaaccagttaagatagtcggccttaaagaaaggcagggcagaaagccactgatattcatcatcctgcaggcgcaggtgctgcatcgcctgaacctgttcacgaatagcatcggcataaatacccagcagatcgtcacctcggcaacgaaactccgccgcgacatgcacatcgtaatagtgatgaaacacggcttgctgcatatgcaacttataagcatctgtatccagcaacgagtgcagaacaggagaagcgaattgtgtcataggtgcgcagtagcgtcctcgtacaggagcgtttagtacaataaacatcttcaggaactgctggagtataccttgtttcgcaatttattgaaccccgatcacaccatatgccacctttctggtcgatggcattacgcggtgtatgttataaaaatgtagcaataaaggcgtttgtacctgaaaagatgaagattctgcatagcgcgatttacgcaacaggaatagactgaacaccagactctataaaagatgctaaaggttatttatgactcaacagccacaagccaaataccgtcacgattatcgtgcgccggattaccagattactgatattgacttgacctttgacctcgacgcgcaaaagacggtcgttaccgcggtcagccaggctgtccgtcatggtgcatcagatgctccccttcgtctcaacggcgaagacctcaaactggtttctgttcatattaatgatgagccgtggaccgcctggaaagaagaagagggcgcactggttatcagtaatttgccggagcgttttacgcttaagatcattaatgaaataagcccggcggcgaataccgcgctggaagggctttatcagtcaggcgatgcgctttgcacccagtgtgaagccgaaggtttccgccatattacgtattatctcgaccgcccggacgtgctggcgcgttttaccaccaaaattattgccgataaaatcaaatatcccttcctgctttccaatggtaaccgcgttgcgcaaggcgaactggaaaacggacgccattgggtacagtggcaggacccgttcccgaaaccgtgctacctgtttgcgctggtggcaggcgactttgatgtactgcgcgatacctttaccacgcgttctggtcgcgaagtagcactggagctgtacgtcgatcgcggcaaccttgatcgcgcgccgtgggcgatgacctcgctgaaaaactccatgaaatgggatgaagaacgctttggcctggagtatgacctcgacatctatatgatcgtcgcggtggatttcttcaatatgggcgcaatggagaataaggggctgaatatctttaactccaaatatgtgctggcccgcaccgacaccgccaccgacaaagattacctcgatattgaacgcgttatcggccatgaatatttccataactggaccggtaaccgagtgacctgtcgcgactggttccagctcagcctgaaagaaggtttaaccgtcttccgcgatcaggagttcagctctgaccttggttcccgcgcagttaaccgcatcaataatgtacgcaccatgcgcggattgcagtttgcagaagacgccagcccgatggcgcacccgatccgcccggatatggtcattgagatgaacaacttctacaccctgaccgtttacgagaagggcgcggaagtgattcgcatgatccacaccctgcttggcgaagaaaacttccagaaagggatgcagctttatttcgagcgtcatgatggtagtgcagcgacctgtgacgactttgtgcaggcgatggaagatgcgtcgaatgtcgatctctcccatttccgccgttggtacagccagtccggtacaccgattgtgaccgtcaaagacgactacaatccggaaaccgagcagtacaccctgaccatcagccagcgcacgccagccacgccggatcaggcagaaaaacagccgctgcatattccgtttgccatcgaactgtatgataacgaaggcaaagtgatcccgttgcagaaaggcggtcatccggtgaattccgtgctgaacgtcactcaggcggaacagacctttgtctttgataatgtctacttccagccggtgcctgcgctgctgtgcgaattctctgcgccagtgaaactggaatataagtggagcgatcagcaactgaccttcctgatgcgtcatgcgcgtaatgatttctcccgctgggatgcggcgcaaagtttgctggcaacctacatcaagctgaacgtcgcgcgtcatcagcaaggtcagccgctgtctctgccggtgcatgtggctgatgctttccgcgcggtactgcttgatgagaagattgatccagcgctggcggcagaaatcctgacgctgccttctgtcaatgaaatggctgaattgttcgatatcatcgacccgattgctattgccgaagtacgcgaagcactcactcgtactctggcgactgaactggcggatgagctactggctatttacaacgcgaattaccagagcgagtaccgtgttgagcatgaagatattgcaaaacgcactctgcgtaatgcctgcctgcgtttcctcgcttttggtgaaacgcatctggctgatgtgctggtgagcaagcagttccacgaagcaaacaatatgactgatgcgctggcggcgctttctgcggcggttgccgcacagctgccttgccgtgacgcgctgatgcaggagtacgacgacaagtggcatcagaacggtctggtgatggataaatggtttatcctgcaagccaccagcccggcggcgaatgtgctggagacggtgcgcggcctgttgcagcatcgctcatttaccatgagcaacccgaaccgtattcgttcgttgattggcgcgtttgcgggcagcaatccggcagcgttccatgccgaagatggcagcggttacctgttcctggtggaaatgcttaccgacctcaacagccgtaacccgcaggtggcttcacgtctgattgaaccgctgattcgcctgaaacgttacgatgccaaacgtcaggagaaaatgcgcgcggcgctggaacagttgaaagggctggaaaatctctctggcgatctgtacgagaagataactaaagcactggcttgataaataaccgaatggcggcaatagcgccgccattcggggaatttacccctgttttctcaggcgagtttcagattcaccacgttgcatcacccgttgcaacacctccgcttccagctccgctaatcgcaccgaccctaatcgacgcggacgggggatatccactgtcaaatccagaccaatttttccctcttcaattaacagcacccggtcagccatcgctaccgcttcgctcacatcatgcgtcaccaacagtacggtaaagccgtgctcctgccaaagtgacacaatcaaatcctgcatctcgagtcgcgttaaggcgtccagcgccccgagcggttcatcaagcaacaataatcccggtcgatgaatcaacgctcttgccagcgccactcgctgtttctgcccgccagaaagtgcggcaggccattcccctgcgcgattctccagtcctaccgcagccaacgctcgacgtgcggcatcgcgccactggcctttaaggcctaacccaacgttatcaatcaccgatttccacggtagcagacgcgcatcctgaaacatcattcgcgtgtcttcctgaatttcagccagcggtgtggtgcccgctaacacatcgcctgcggttggcgtttccagacctgccagcaggcgcagcagggtacttttgccaccaccgctgcggcccaccaccgccacaaactgacctgccggaatatgtaaatccagttggttcaggacgatattttccgcgtaatgtttgcttactgcattgagcaacaatggcgtgccctggttcagacgagcagtattcataccgtggcctccttcaaatgataagccgggttccagcgcaaccagaggcgctctaacagctgcgcgctgacgtcagccagtttgccgagcagggcgtaaagaataatagcgactaccaccacgtccgtttgcaaaaactcccgcgcattcatcgccagataaccaatgcctgaattggcagaaatggtttcggcaacaatcagcgtcagccacatcaggcccaacgcaaaacgcacgccgaccataattgagggcagggcaccaggcaggatcacatggataaacagcggtatgccggataatccatagctacgcgccatctccaccaacccgcgatcgatattacggatgccatgccaggtgttgatataaatggggaatagcgtaccgagcgccaccagaaagatttttgcggattcatcaatgccaaaccacaaaatcaccagcgggatcagcgccagatgcggcacgttgcgcaacatctgaattgaggtatccagcagccgttctccccagcgagatagcccgctaatcagtcccaaaatcaaccccagcgatccgccaattgaaaagccaatcagcgcccgccaggagctgatcgccagatgctgccacagttcgccgctggcggagagcgtccagaacgccgtcaccactccttccggtgaaggcaaaatacgcgtcgacagccagccaaccgaggaggccagttgccacaccgccacgatgcccaccggtaaaaaccagggggcaacgcgcaataaccacttcttcactggcgttgccattatttcttccttagctttgcgcgactttacgggggataaaatcattcgccaccgcttcgccttgcggattcagcggctgcggctggggaatttccgggatggcgacatccagaagcgggaacagcaactcgccaacccgatacgcttcttccagatgcggatagcccgaaagcacaaaactgtcgatgccaagcgcggcatattcgttgattcgcgcagcgaccgtaggaccatcgcccaccagcgccgtcccggcaccgccgcgcactaagccaacgcccgcccataaattggggctgatctccagattgtcgcgcttgccgttatgtaacgccgccattcgctgttgccctacggaatccgtccgggcgaatgcggcctgtgctttggcgatagtttcatcatcaagatgcgagattaaccgctcggcggcctgccacgcttcgtcgttagtttcacgaacaatcacatgcagacgaataccgaaacgaattttgcgtccatgcgcggcagctttcgcccgcacttgttcgattttctctttaaccagttccggcggttcgccccaggtgaggtagagatcaacctgttctgccgccagctcctgggcgacatctgacgatccgccaaagtaaagtggcggatacggctgttgaatcgccgggaagagcagttttgctccgcgcacatgaatatgtttaccgttgaaatcgacggtttctctctgcaataaacgccgccagacctgggtaaattccgccgaggcttcgtagcgctcgctatgatcaaggaacactccgtcgcctgccagctcttgtggatcgctgcctgtgaccaggttaaacaacgcacgtccatttgagagacggtcaagcgtggcggcctggcgggcggcaacggtaggtgaggttacgctgggacgcagggcgacaagaaacttcagccgctgcgtcaccgggatcatcgatgcggcaaccagccacgcatcttcgcaggagcgccccgttggaattagcacaccggtatagccaagacgatccgccgcttgcgcaatttgttgcagataaccgtgatcaaccgggcgtgaaccttcttccgttcccagataatgcccgtcaccgtgggtcggtaaaaaccagaacatattcagactcataattgttttccttccagttgagtgggctgccagatgcgctggcgaatatcgacttttttcggcaccagacgattttcataaaacagatctgccgtttgctgctgtaaggcggcaacctcggcgttaaccggtttgatggtggtaggagggcgatgatctaagtaagaggcaatcaccggtgccggtaagcccatcgtttttgccagtaaagcgatgctttgctcgcgctggctgcgggttaacgcatcggcctcactaaaggttgccagtacgccctgaataaaagcgccgtttttttctgcatagggacgagctgccagataaaacgatccagtttgattgagatcggtgccgtctttcagcacccgcacgccgccctgtaataatgcagcagagtagtagggatcccagatagcccaggcgtcaacgttaccttgctggaacgcggcgcgggcatcagcgggcgtcaggtaagtgggttggatatcggtaaacttaagtccggcctgacgcagtgcacgcagtaaaaggttgtgtgaactggaacctttctgaaaggcaactttgtgacctttaagatcggctacggttttgatcgggctgttttctgccaccagaatcacttcggctttgggcttcggtggctcgacgcccacgtacaccaaatcagccccggcagcctgggcaaagattggcggaatatccccggtactgccgagatcaatactgccaacgtttaacgcttccaacatttgcggacccgcggggaactccacccaggagatttttgattccggatagcgtttttccagtaactggtggctttttgccagcaccataccaatactgcctttctgatagcctatacgtaacgcttcaggcgaggattctgcagcaaccgcaaaagtagagacgctaagcaatcccgccagcgccagtttaatgatgttacgcatgggcattacctcgcagagacagaaggtcaggaacctgaacatcgcggcggtgcaatgcctgccagaaagtttctagcgcggtatcaagacgggtttgcagatttggcgtgaactggggtctgtgatggtaatcaattacttgtgagtcatcggcaaacacgccgtgcaggatctcctgagctttcagtgcgcttaaaactggtttaagggcataatcgaccgccagcagatgggccacggtaccgcccgtcgccagcggtagcaccactttgccttgcaaagcgcgttctggcagcaggtcgagcagggttttcaacgcaccggaataggcggctttatacacaggcgtggcgacaatcagcccatcggcctgttgcagctgttcggtgaaggtcttgagtgccggactatcgaaacgagcataaagtagatcttccggggcgaagttttgcagattccagtgataaacctctacatccaggccatttagtttttcccgcgcatattccagcaaggagctggagcgagaaggaaagcgaggactacccgccagggtgatgacacgcatactctctccttataaccaattgttctttttttgttaacattgataacaattcggtcagtctgtcggagagacaagaaaattccaaatataaattttgtgtatctttttctgaaaataaactaaagaaagggctttatatatcacgcatatttatttattggatagtcattagatgttgaatcaatgaattactcgttcagttaatatttaaatattcatgaaatctataaattaaagatttgtcacttattggatttagtatgcttgatttaaatggcggacaattattgttattattaagtctaatgtcatttaaaggcattatcatatttacgaagagatcaggatgataacgatgaaaaaaagtgtattgacggcgtttataactgtggtatgtgcaacgtccagcgttatggctgctgatgataatgctatcacggatggctcagtaacatttaatggtaaagttattgctccagcttgtaccctggtagctgcgacgaaagattccgtggtgactttgccagatgttagtgccacgaagttgcaaaccaatggtcaggtttctggcgtgcaaattgatgtgccaattgaattaaaagattgtgatactaccgtaacaaaaaatgcaacgttcacctttaatggcactgcggatactactcagattacagcgtttgctaaccaggcctcatctgatgctgctacaaacgtggccctgcaaatgtatatgaatgatggtacaacggccatcacgccagacacagaaaccgggaacattttgttgcaggatggagatcagacgttgacttttaaagttgattatatcgctacggggaaagcgacttcaggtaatgtgaatgcggtaacaaatttccatattaactattattaatagaactcattaattgttttattaattagtacccctccagtgttctggaggggatattcatattttttaagagtgactatttatgaaaacttgcataacaaagggaattgtgaccgtaagtttaacggcaatattactcagctgctcatccgcatgggcggcaggtaaaggcgggattggacttgcagcaacacgtcttgtttattcagaaggtgaagagcaaatttcactgggtgtacgtaacaccagtccggatgttccttatcttattcagtcatgggtgatgaccccagataataaaaaatcagcagactttattattacaccaccgctatttgtgctgaatccggcaaatgagaatctgttacgcattatgtacattggagcgccgttggcgaaagacagagaaacccttttcttcactagcgtacgggcagtcccttcaacaacgaagcggaaagagggaaataccctgaagattgccacacaaagcgtcatcaaacttttctggcgaccaaaaggtttagcgtatcccttaggcgaggctccggcgaaactgcgttgcacttcgtcagctgacatggttacggtcagtaacccaacaccttatttcattaccctgacagacctgaaaataggtggaaaagtagttaaaaatcaaatgatttccccctttgataaataccaattttctctgccaaagggggccaaaaatagcagcgtaacgtatcgaaccatcaatgactacggggcggaaacgccgcaactcaactgtaaatcgtaagccgtcttcagttaagagagcgagatgtatagaactcatcgacaacacagcctgttaagctctggtggagtgccatcgtttattggtgggctggtggtgtttgtgtcggcagcgttcaatgcacaagctgaaacctggttcgatcctgcttttttcaaagatgatccctcaatggtggccgatttgtctcgtttcgaaaaaggacaaaaaataacgccaggggtttatcgtgtcgatattgttctgaatcagacaattgtagatacgcgcaacgtcaattttgttgagataacgccagagaaggggattgccgcctgtttgacgactgaaagcctggatgcaatgggtgttaatactgatgcgtttccggcttttaaacaactggacaaacaagcgtgtgtgccattggcggagattattccggatgccagcgtaacgtttaatgtgaataaactccgtctggaaatttcagtaccgcaaatcgccatcaaaagtaatgcccgtggttatgtcccccctgaacgttgggatgaagggatcaacgcgctattactgggatattcgtttagcggggctaacagtattcatagcagcgcagacagtgattctggcgacagctattttctgaatttaaacagtggcgttaatttaggcccatggagattgcgcaacaattcaacatggagtcgtagtagtggccaaaccgcagaatggaagaatctcagcagctatttgcaacgggcggttattcctctgaaaggcgaactgaccgtaggtgatgattatactgcaggcgattttttcgatagtgtcagctttcgtggtgtgcagctggcgtcagatgacaacatgctgccagacagcctgaaagggtttgcgcctgtggtgcgtggtatcgccaaaagcaatgcccagataacgattaagcaaaatggttacaccatttaccaaacttatgtatcgcctggtgcttttgaaattagtgatctctattccacgtcgtcgagcggtgatttgttagttgaaatcaaagaagcggacggcagcgtcaatagctacagcgtaccgttctccagtgtgccattactccagcgtcaggggcgaatcaaatacgcggtgacactggcgaaatacagaaccaatagtaatgaacagcaggagagcaaatttgcccaggccacgttgcagtggggcggaccgtggggaacgacctggtatggtggtggacaatatgctgaatattaccgtgccgccatgtttggtctgggatttaacctcggcgatttcggagcaatttcgttcgatgcgacccaggcgaagagtacgctagcagatcaaagcgaacataaaggtcagtcatatcgttttctgtatgccaaaacgctcaaccacttgggcactaactttcaattgatgggctatcgctattcgacgtcgggtttctacaccctttccgacaccatgtataaacatatggatggctacgaatttaatgacggtgatgatgaagatacgccgatgtggtcgcgttattacaatttgttttacaccaaacgtggcaaactgcaggtcaatatctcccagcaattaggcgagtacggttcgttttatttaagtggtagccagcaaacttactggcatacggatcaacaggatcggctattacagtttggctacaacacgcaaattaaagatctttcgctggggatttcctggaactacagtaagtcccgtggtcaacctgatgctgatcaggtgtttgctctaaatttttccctgccgctcaatctgttgctccccagaagtaatgatagctataccaggaaaaaaaattacgcctggatgacctctaacaccagtatcgataacgaagggcacactacacaaaacctgggtttaacggagacattactcgatgacggtaacctgagctacagcgtgcaacagggatataacagcgaggggaaaacggctaatggtagcgccagcatggattacaaaggggcgtttgcggatgcccgagtgggctacaactacagcgataacggcagtcaacaacaactgaactacgctctttcaggcagtttagttgcccattcacagggcattaccctggggcaatcgctgggggaaactaacgttctgattgcagcaccaggcgcagagaatactcgtgtggcgaacagcaccgggctgaaaactgactggcgcggatataccgttgttccttatgccacttcttatcgggaaaatcgaatcgcacttgatgcggcgtcgttaaaacgtaacgtggatcttgaaaatgcagtagtcaacgtggttcccaccaaaggggcgttggttctggcggagttcaatgcccatgcgggtgcaagggtattaatgaaaacatcaaagcagggtataccgctgcgttttggcgcgatagcgacgctggacggcgtacaggctaatagcggcataattgatgatgatggctcgctctatatggcgggtttaccggcgaagggaacaataagcgtgcgctggggcgaagctcccgatcaaatttgtcatatcaattacgagcttaccgaacaacaaattaactctgcgattacgcgaatggatgccatatgcagataatctttggagaaaaatgcgtgtcattactacgactattttttgccgccgtcttaatgttatggtgcgctcaaaccgctgcttatagcgggcagtgtcatactactcaggggaatccgtatattggcgtcaattttggcgttaaaaccctggaggaagaagcaaatacggcaggggtagttaaagacaaattttatcagtggaacgaatcgaatgattattatgtttcctgtgattgcgataaagacaatgtcagaagtggccgatgggcattcgccgcggattcaccgttagtctatttaggcgacaactggtacaaaattaatgactatcttgccgccaaagttttattgcaggttaaaggcagttctcctactgcggttcctttcgaaaacgtgggcacagggggggatacccgatggcatatttgcgaccctggcggtcaacgtttaggtgggcagggggcaagcggtaatagcggtagcttttccctgaaaatattgcagccgttcgttggctcggtcgtcattcctcctatggcgctggcgcgattatatgaatgctacaacatacccgcaggtgattcctgcacgactacaggtacaccggttttagtgtattacctgtctggtacgatcaattcacttggctcatgttccgtcaatgccggagagacaattgaagttgatttaggtgatgtcttcgctgccaatttccgtgttgtagggcataaacctcttggggccagaacggcagaacttgcaattccagtcaggtgtaacacgggaaacgcgggattagttaatgtcaacctgagtctgacggcaaccacagaccccagctatccccaggcgattaagacgtcacgtcctggcgtgggcgtggtggtgaccgatagccagaacaacattatttcccctgctggtggaacattaccgctctctattcctgatgatgcagacagtatcgcgcgaatgaatgtctatccagtcagcacgacaggtgtaccaccagaaaccgggcgatttgaagccacggcaacggtgagaataaattttgattaacgcgtgaacgtatgaagaaaaaaacgatatttcagtgcgttatcttgttctttagcattcttaacatccatgtcgggatggctgggcctgaacaagttagtatgcatatttatgggaatgtggtcgatcagggctgtgatgtcgccaccaaaagtgcattacaaaatattcatattggtgattttaatatcagtgattttcaggccgcgaataccgtaagcactgctgctgatttgaatatcgatatcaccggttgtgccgctggtattactggcgcggacgtcctttttagcggcgaggctgacacccttgcgccgacactgctcaaactaactgacacaggcggaagcggtggtatggcaacggggattgccgtgcaaattcttgatgcgcaaagtcagcaagaaatcccgctcaatcaggtccagcctcttacgcccttaaaagccggggataacacactcaaatatcaacttcgttataagtccacaaaggcgggagcaacgggcggtaatgcgacggcggttctctattttgatctggtttaccagtgaaggagtgatgttgaaacggataatctggattctgttcttattgggattaacgtggggctgtgagctatttgcccatgatggcacggtcaacattagcggatcgtttcgccgtaatacatgcgtgctggcacaggatagcaagcaaatcaatgtgcagttaggcgatgtctcgctgacacgtttttctcatgggaattatggcccggagaaatctttcatcattaatttgcaggattgcggaacagatgtcagcacggttgacgtcaccttttcaggaacccccgacggagtgcagagcgaaatgttgtccattgaaagtggtacggatgcagccagcgggctggcaattgcgattctggatgatgcgaagatattgattccgcttaaccaggcgagtaaagactacagcctacatagcggtaaggtgccattaactttttatgcgcaattgcgacctgtcaatagcgatgtgcagtcgggtaaagtgaatgccagcgcgacatttgtacttcattatgactaatacgtggaacagattggcgctcttgattttcgccgttttatcgctgctggtggcgggtgaattgcaggcaggagtggtggtcggcggaacgcgatttatctttccggcagacagagaatcgatatctattttactgactaataccagtcaggaatcctggcttattaacagtaaaatcaaccgcccaacgcgttgggccgggggggaagcgtcgacagtgccagcaccattactggccgctccgccacttattctcctgaagcccggtacgacaggcacgttgcgcttgctgagaacggaaagcgacatcttgcctgtggatcgcgaaacgctatttgagttaagcattgccagcgtgccatccggcaaagttgaaaatcagagcgtaaaagtggcgatgcgctcggtatttaaactgttctggcgacccgaaggtttgccgggcgacccgctggaagcttatcaacaattacgctggacacggaattcgcagggtgtacaactcactaacccaacgccttattacattaacctgattcaggtgagtgtaaatggtaaagcgttaagtaatgtgggagttgtgccgcctaaaagccagcgtcagacaagctggtgtcaggcaatcgcaccgtgtcatgtcgcctggcgggcgataaatgattacggcgggttgagtgcaaagaaggagcaaaatctgccctgaaacaggttcggaaaacgtttgcgttttttttgccgcaggtcaattcccttttggtccgaactcgcacataatacgcccccggtttgcacaccgggaatccaggagagttcatgtactaccccttcgttcgtaaagcccttttccagctcgatccagagcgcgctcatgagtttacttttcagcaattacgccgtattacaggaacgccgtttgaagcactggtgcggcagaaagtgcctgcgaaacctgttaactgcatgggcctgacgtttaaaaatccgcttggtctggcagccggtcttgataaagacggggagtgcattgacgcgttaggcgcgatgggatttggatcgatcgagatcggtaccgtcacgccacgtccacagccaggtaatgacaagccgcgtctctttcgtctggtagatgccgaaggtttgatcaaccgtatgggctttaataatcttggcgttgataacctcgtagagaacgtaaaaaaggcccattatgacggcgtcctgggtattaacatcggcaaaaataaagatacgccagtggagcagggcaaagatgactatctgatttgtatggaaaaaatctatgcctatgcgggatatatcgccatcaatatttcatcgccgaataccccaggattacgcacgctgcaatatggtgaagcgctggatgatctcttaaccgcgattaaaaataagcaaaatgatttgcaagcgatgcaccataaatatgtgccgatcgcagtgaagatcgcgccggatctttctgaagaagaattgatccaggttgccgatagtttagttcgccataatattgatggcgttattgcaaccaataccacactcgatcgttctcttgttcagggaatgaaaaattgcgatcaaaccggtggcttaagtggtcgtccgcttcagttaaaaagcaccgaaattattcgccgcttgtcactggaattaaacggtcgcttaccgatcatcggtgttggcggcatcgactcggttatcgctgcgcgtgaaaagattgctgcgggtgcctcactggtgcaaatttattctggttttatttttaaaggtccgccgctgattaaagaaatcgttacccatatctaattatttcttcgaattcctctttataagataatcagggctttattttcagccctggttgttttatattcatcgctgttgcttatttagacattttgtacttttattgttgaggttattaagcgaagcgacaatggattgtgttgctgcggttttatagggtaggggagaggcagatgcgaattaaaccagacgataactggcgttggtattacgatgaagagcacgatcgaatgatgctcgatttagccaatggtatgctatttcgctcacgttttgcgcgcaagatgttgactccagatgccttttctcccgcaggcttttgcgttgacgacgccgcgctctatttctcttttgaagaaaagtgccgcgattttaatttatctaaagaacaaaaagccgaactggtgctgaatgcactggtagcaattcgctatctcaaaccgcaaatgccgaaaagctggcattttgtttcccatggtgaaatgtgggtgcccatgccgggcgatgcggcctgcgtttggttgagcgatactcacgagcaggtcaatttgctggtcgttgaatctggcgaaaatgccgcactatgcctgctggcacaaccctgcgttgttattgcgggtcgcgcgatgcagttgggcgacgccattaaaatcatgaacgacaggctgaaaccgcaggttaatgttgacagcttcagcctcgaacaggcagtctaacgcgccaacttaagtgcagtcttcggtacacagctacagcaaagaatggtgccatcatcgcccattgctgattttttcagcggcgtgacttcgccttctaaaagctgaacacggcaacttccacaaatgcccgcgcggcaagaataagggatacgaattccctgattttctaattgctccagcaacacctgttggttatttccacgaaatgcctgtccctgccagtcaatatctacatttgcgtccggttgttgcgtgatgttggcggtatcatcagcggcagctgcgccgtaaatttttgccggagccgttgccagaatttccacctcatcgccaacgcgaatcacgccgctattacgggcaattaaattctgaccaaaatcgacatcgccgttatcctgggcagtgcggaaagattgcaatgtttttaatggttcgcctgccggatgtttttgccctttttctgggctgacggtggtgaaaatacagcggctacaaggtttaaccacatcaaacaccacatcaccaatgcgaatcactttccagcgatcttcttcccaggctgacgcgccggaaaccaccagattggggcggaattgctccatttttacactggccggacaacgttgttggagatcacgtaacgaggcttcgttagcaagaaggtaaggatagccatcagcaaatgacagaggtacagtgttgtggcgtttcacgcgccgggtcatttgtggccccacccagcgtaattgcacttcgcgggagaaaaatccacttagccatttgttgatcgcgtctggcgcaattcgcgcggtaaaatgtgtgccccaaacttcggttggtgcgtcttgtgtggcgaaatcagcaaaacgaacatatgcgctactgccatctggtgcggtgagatgcaagccatcatgcacaggtgaaggagtaaaccgtaccatctggggaaactggcgagcggtaataaacgtaccgtcaggttccgtgatcataaagatgcgatcgaaggccagaccactgacatctgccagagcatgtgtaagaccaatgccgcgcatcgatttaacaggatgaataaaaagccggattaatgtcgccacggtgcggtcctcaaatgaaaataagccctcaactttatgacatgacgcgcttattagctataatgcgcaacaattttcttagcgcctgtcccattaggctattttatttgtcagtttggccctgggttatgctcgaaatcctcacgtacttgtgtacgctccggtttctccgcgctgtccatgtccagactgactgcaacaattacgcctactgcggtaggctcttagagtaaaagtgacgatatgaattctctgtttgccagtacggcccgtgggctggaagagctgttaaaaactgaactggaaaacctgggggccgttgaatgccaggtggttcagggtggggtccatttcaagggcgacacacggcttgtttaccagagcctgatgtggagccgcctggcctcgcgtattatgttgccgctgggcgagtgtaaggtttacagcgatttagacctctatctcggtgttcaggcgatcaactggacagagatgtttaatcctggcgcgaccttcgctgtccacttcagtggtttgaatgacaccatccgcaacagtcagtacggcgcgatgaaagtgaaagacgcgatcgtcgatgctttcacgcggaaaaatctgccgcgtccaaatgttgatcgcgatgcgccggatatccgcgttaacgtctggctgcataaagaaaccgccagtatcgctcttgatctgagtggtgatggtttacatctgcgtggctatcgcgatcgtgctggtattgcgccgatcaaagaaaccctggcagccgctattgtgatgcgatccggctggcagccaggaacaccgctgctcgatccgatgtgtggttccggtacgttgctgattgaagcagcgatgctggcgaccgatcgcgcaccaggcttgcaccgtgggcgttggggctttagcggctgggcgcagcatgatgaagctatctggcaggaagtgaaagcggaagcgcaaactcgcgcccgtaaaggcctggctgagtatagctctcatttttacggttcggacagcgacgcacgggtgattcaacgtgcacgcactaacgcccgtcttgcggggattggtgaactgatcacctttgaggtgaaagatgtcgcgcaactgaccaatccgctgccgaaagggccgtacggcacagtgttgagcaacccgccatacggggaacgtctggacagcgaaccggcgctgattgcgctgcatagcctgctgggtcggatcatgaaaaaccagtttggtggctggaatctctctttgtttagtgcctcgccggatctgctaagctgcttgcagctgcgtgcagacaaacagtacaaggcgaaaaacggcccgctggactgcgtacagaaaaattaccacgttgccgaaagcactccagacagcaaaccggcgatggtagcggaagactacaccaaccgcctgcgtaagaacctcaaaaaattcgagaagtgggctcgccaggaagggattgaatgttaccgcctgtatgacgccgatctgccagaatataacgttgccgttgaccgttatgccgactgggtggtggtgcaggagtatgcgccgccaaaaactattgatgctcacaaagcgcgtcagcgtctgttcgatattatcgctgcaaccatttcggtactggggattgcgccaaacaaactggtgctgaaaacccgtgaacgccagaagggcaaaaaccaataccagaaactgggcgagaagggcgagtttcttgaagttaccgaatataacgctcacttgtgggtgaacctgacggattatctcgatactggtctgttcctcgatcaccgcatcgcccgtcgtatgctcggtcagatgagcaaaggcaaagatttcctcaacctgttctcttataccggcagcgccaccgtgcatgcgggattaggcggtgcacgcagcaccaccaccgtggatatgtcgcgtacttatctggaatgggcagaacgcaacctgcgtctgaatggcctgaccgggcgtgcgcatcgcctgattcaggccgattgcctggcgtggctgcgtgaggcaaatgaacagttcgatctgatctttatcgatccgccaaccttctctaactcaaaacgaatggaagatgcgtttgatgttcagcgcgatcatctggcgctgatgaaagatttgaaacgtctgctgcgtgcaggtgggacgatcatgttctcgaacaacaaacgtggcttccgtatggatctcgacggcctggcaaaactgggactgaaagcacaagaaattacgcaaaaaacgctctcccaggatttcgcccgtaaccgccagatccacaactgctggctgattaccgcagcctgaaaggaatagtaatgtcattaatcagtatgcatggcgcatggctgtcgttcagcgacgcgccgcttctcgataacgcagaactgcatatcgaagataacgaacgtgtttgtctggtgggccgcaacggcgcaggcaaatcgacgttaatgaaaatcctcaaccgtgaacaagggctggatgacggtcgcattatttacgagcaagatttgattgtagcgcgtctgcaacaggatccgccgcgtaacgttgagggtagcgtttatgatttcgttgccgaaggcattgaagaacaagcggaatatctgaaacgctatcacgatatttcgcgcctggtgatgaacgacccgagcgagaaaaatctcaacgaactggcgaaggttcaggaacagctggatcaccacaacctgtggcagctggaaaaccgcatcaacgaagtgctggcgcaactggggttagatcctaacgttgcgctgtcgtcgctttccggcggctggttgcgtaaagcggcattaggacgcgcgctggtgagtaatccgcgcgtgctgttgcttgatgaaccgacaaaccacctggatattgaaaccatcgactggctggaagggtttttgaaaactttcaacgggacgattattttcatctcccacgaccgttcgtttatccgcaatatggcgacgcgcattgttgatctcgatcgcggcaagctggtgacctatccagggaattacgaccagtacctgctggaaaaagaagaagccctgcgcgtggaagaattacaaaatgccgagttcgatcgcaaactggcgcaggaagaggtgtggatccgccaggggatcaaagcacgccgtacccgtaatgaaggccgcgtacgcgccctgaaagcgatgcgtcgcgaacgtggtgaacgtcgcgaagtgatgggtaccgcaaagatgcaggtggaagaggccagccgctccggtaaaatcgttttcgaaatggaagacgtttgctaccaggttaacggtaagcaactggtgaaagatttttctgcccaggttctacgtggcgacaaaattgccctgattggtccgaatgggtgcggcaaaaccacgctgctaaaactgatgctcggtcagcttcaagcggacagcgggcgtattcacgttggcaccaaactggaagtggcttatttcgatcagcaccgcgcggaactggatcccgataaaacggtgatggataaccttgccgaaggtaagcaagaggtgatggttaacggcaagccacgccacgtattgggctatttgcaggactttctgttccatccgaaacgggcgatgacgccggtacgtgcgctttctggcggtgagcggaaccgcttgctgctggcgcgtttgttcctcaaaccaagcaacttattgattcttgacgaaccgaccaacgatcttgatgtcgaaacgctggaactgctggaagaactgatcgacagctatcagggcacggtattgctggttagccacgatcgtcagtttgtcgataacaccgttacagaatgttggatcttcgaaggcggcggtaaaattggtcgttatgtcggcggttatcatgatgcccgtggtcagcaagagcagtatgtggcgctcaaacagcctgcggtgaaaaaaaccgaagaagccgccgcggcaaaagcagaaactgtaaaacgcagcagtagcaaactaagctataaattgcagcgcgaactggagcagctaccgcaattgctcgaagatctggaggcgaagctggaagccctacagacgcaagtggcggatgcttccttcttcagtcagccgcatgagcagacgcaaaaagtgcttgctgatatggctgctgcagagcaggagctggagcaagcctttgaacgctgggagtatcttgaagcgttaaaaaatggtggctgatcgcaaaatagtcgatttaaacagagacagctgacaacggtaaaattgcctgatgaactgggtttatcaggcatgaaaaccaacactttgttagtcatctgtaaaatagcgcatcattaaggagtaccaatgtgcgaacatcatcatgccgcgaagcacatcctgtgctcgcagtgtgacatgctggtggcgttaccgcgccttgagcatggtcagaaagcggcatgtccccggtgtggcacaacgttaaccgtggcgtgggatgcccctcggcagcgtcccaccgcctatgcgttggctgcactgttcatgctgttgctgtccaacttgtttccttttgtgaatatgaacgttgcaggagttaccagtgaaattacattactggaaattcccggcgtgcttttttctgaggactacgccagcctcggcacctttttcctgttgtttgtgcaactggttcccgcgttttgtctgataaccattctgttactggtgaatcgcgcggaattaccggtccgtttaaaagagcaactggcacgggtgctttttcaactcaaaacctggggaatggcggagattttcctcgcgggtgtgctggtcagtttcgttaaactgatggcttacggcagcattggggtaggcagcagctttctcccctggtgtttattttgtgtcctgcaactgcgcgcttttcagtgcgttgatcgtcgctggttatgggacgacatcgccccgatgccagaactgcgccagccgctaaaaccaggcgtcacggggatacgtcaggggctgcgttcgtgctcctgttgtacggcaatccttcctgctgatgaacccgtgtgcccgcgttgtagtaccaaagggtacgttcggcgtagaaacagcctgcagtggacactcgcgctgcttgtaacgtccatcatgctgtatcttccggctaatattttgcccatcatggtgacggatttattaggctcgaagatgccgtcgacgattctcgctggggtcattctgttatggagcgaaggctcttatcccgtcgctgcggtgatctttctggccagtattatggtgccaacgttaaagatgatcgccatcgcgtggctgtgttgggatgccaaagggcatggcaagcgcgacagtgaaagaatgcatttgatttatgaagttgttgagtttgtaggccgctggtcgatgattgacgttttcgttatcgcggtgctctcggcgctggtgcgtatgggaggtttaatgagtatttatccggcaatgggtgcattaatgtttgctttagtcgtcataatgacaatgttttctgctatgacgtttgacccgcgtttgtcgtgggatcgtcaacctgaatcagagcatgaggagtcctgacagtatggaatctaataatggggaagccaaaatccagaaagtgaagaactggtctcccgtgtggatatttcctatcgtcacggcgctcattggggcctgggttcttttttatcattacagccatcagggaccggaagtgaccctgatcaccgcgaatgcggaaggaattgaaggtggcaaaaccaccattaaaagccgtagcgttgacgtcggcgtggttgaaagcgccacactggctgatgatttgacgcacgttgaaatcaaagcgcggctgaattccggtatggaaaaattgctgcataaagacaccgtcttttgggtggtgaaaccgcagattggtcgcgaagggattagcggcctgggaacgctgctgtctggagtttatatcgaactgcagccaggcgcgaaaggcagcaaaatggataaatacgatttgctggactcgccaccgttggccccgcctgatgcgaaaggtatccgtgtgattctcgatagcaaaaaagccgggcagctctcgccaggagatccggtgctgttccgtggctatcgggtaggttcggttgaaaccagcaccttcgatacacaaaaacgcaatatcagctatcaactgttcatcaatgcaccttatgaccgactggtgaccaacaatgttcgcttctggaaagatagtggcattgcggttgatctgacgtcagcagggatgcgtgtggagatgggctcattgacaacgctgctgagtggcggtgtcagctttgatgtgccggaaggtctggatttagggcagccagtggcaccgaaaacagctttcgttttgtatgatgatcagaagagcattcaggattcgttgtacaccgatcacattgattatctgatgttctttaaagattcggtacgcggtctgcaaccgggagctccggtagagttccggggtattcgcctgggtaccgtaagcaaagtgccattctttgcgccgaatatgcgtcagacatttaacgatgattaccgtattccggtactgattcgtatcgagccagagcggctgaaaatgcagcttggcgaaaatgcggatgttgttgagcaccttggcgaattgttgaaacgtggtttacgcggatcgctgaaaaccggaaacctggtcactggtgcactgtatgttgatctcgatttctatccaaatacgcctgcaataaccggtattcgtgaatttaatggttatcagattatcccgaccgttagcggcggcctggcgcaaatccagcaacgactgatggaagcgttggataagatcaacaaactgccattgaatccgatgattgaacaggcaaccagtacgctttctgaaagtcagcgcacaatgaaaaacctgcaaacgacgctggatagcatgaacaagatcctcgctagccagtcgatgcagcagttgccgacggatatgcagtcaacgttgcgtgaattgaatcgcagcatgcagggcttccagcctggctccgcagcctacaacaagatggtggcggatatgcagcgccttgatcaggtgttgcgagaactgcaaccggtgctgaaaacgctcaatgagaagagtaacgcgctggtatttgaagcgaaggacaaaaaagatccagagccgaagagggcgaaacaatgaaaaagtggctagtgacgattgcagcactgtggctggccggatgcagctccggcgaaattaataaaaactattaccagttacctgtggtgcagagcggtacacaaagtaccgccagccagggcaatcgtctgttatgggtagagcaggtcactgttcctgactatctggcggggaatggtgtggtttatcaaaccagtgatgtgaagtatgtgattgccaacaacaacttgtgggccagcccgttggatcaacagttgcgcaacaccctggttgccaacctgagtacgcaactgcccggctgggtggttgcctcccagcctctgggaagcgcccaggacacgctcaatgttaccgtaacggagtttaacggtcgctatgatggcaaggtcattgtcagtggtgagtggctgttgaaccaccagggacaactgatcaaacgtccgttccgtctggaaggagtgcaaactcaggatggttacgatgagatggttaaagtgctggccggtgtctggagtcaggaagccgcttctattgcacaagagataaagcgtctaccttaattataaagatttgtaaatataaccgtctccggtatgttgcctgaggcggtttttttgtctctaacgtgcggaaaaatttgttcctcttcacattttttgtacaaccgacatgcccgtgtagctcacaaatatgacagtggcgtgaattttgcgcattgacggcagttatgattcgcggtattgcttaactgtgattgcacatttagtaatcactgttttcttttccaccagaaaccagtatgagggaaacgaggcatgaagagacaaaaacgagatcgcctggaacgggcacatcaacgtggttatcaggccggcatcgccggacgctcaaaagaaatgtgtccctatcagacgctgaatcaaaggtcacaatggctgggaggctggcgagaagccatggcggacagggtagtaatggcctgattctgtctctttaaaaagaaacctccgcattgcggaggtttcgccttttgatactctgtctgattataatcagaaggcagacgtatcctggaacagaccgactttcaggtcgctggcggtatagatcagacgaccatcaaccagcacttcgccatccgccaggcccataatcagacgacggttaacaatgcgtttaaagtgaatacggtaggtcacttttttcgctgtcggcagtacctgaccagtgaatttcacttcgccaacgcccagcgcgcggcctttaccttcgccgcccagccagccgaggtagaaccctaccagctgccacattgcgtccaggcccaggcatcccggcataaccggatcgccaataaagtggcatccgaagaaccacagatccggattgatatccagttctgcttcaacataccctttgtcgaagttaccacccgtttcggtcattttgaccacacggtccatcatcagcatgttcggtgctggcaattgcgggcctttagcgccaaacagttcaccgcgaccagaggcaagaaggtcttcttttgtataggattcgcgtttatctaccatgttctctgtaagccttattttattgaagcacgcaggatagctaacacgtgtacgctgaacaagtccgatcagttcggaataaaccagttcagccaacgtaatggccatggaaaacggtgacgtccttcctgttgcgatgcttgcgcgatacgttcctggatggtttgcatcagcgtcgtttggccttcgccatcccacaccagatttaataataacggcagtgcgtcagtcacatcgtctactgcccagatggtgaatttgccttcttctaccgctttcaccagttcactgtgaagacttaaatggcgaacgttagctgtggggataatgacaccttgtttcccggttaactcacgttgctggcaaatagcaaagaagccttcgattttctcatttaaaccaccgaccggctgggcgcgaccgaactgatcgactgaacctgtgatagcgatactctgattcaccggcacatcggcgagggcgcttatcagggcgcagagttcagccatcgaggcactatctccatcaacttcactgtatgactgctcaaatgtcagcgatgctgagaaggggatctgttgctcaagctgtagttccgacatcaggaacgcttgcatgatcatcatccctttcgcatggatattgccgccaagctccgctttgcgttcgatgtcggtgaattcaccatcgccaatatgcacaacgcagctaatgcgagaaggttcgccaaaagcgcgtggatgacccggaaattcaatgaccgaaagggcgttaatttgcccgatgcgttcgccttcggtttcaatcaggatttgctcctgaaggatctcatcctgcatacgttcagcgaggaaaccttcgcgccattcacgctgctgcagcattaagtttagctgctcgccggagaaggtgtcgccatcacacagggaggcgacctctttacactggcggaggatccactgcgggctaagcggaagtgtttcttgttcaccggtgtagcgtgctgcttcgcggataagtatcggccaggcatccgctcccggtgcaggtaagtgattatgtctggcggtaaatgtcacccagcgacaccactgggttactgactccgcatcgacaatctgcagagtatcttcaaattcgctataaatagcctgctctgaaagctctggctccatctcctggaaatcagccaatgattcgcgttcgcctaccagaatgactttcagcttcaatggcatcgaaggcacagagacggggagagggcgcgactcatcaaacgcaacccagtcaaaacgctcgcggttaacgatatttttcagccgcatccacagcagaggttgcgccagcagtgtacgcaaagagataatgagaataccgccatttgcctgatgcaccagaccaggctgcagggtaatgtcgccattaaactggcgcaggcagccaaagagttgctccgcttctacccagtcggcagcgacaacttgcgttaaagtcgcaaaattatcatctgcactcactgcgtgacgtaagcggatggagtggccggaaacctcatagtgaccgcccaccagttggcctgcatcgctttgtagcgtacgcgcggcattggcaataagattcagatactcagactcttccggggccttcgccagcataaaagaggaggatgctcgcgtatgcagcaactgctccagcgcaaattgcagccgcggttgagtatcactgaataaaggatcgttttcgtcaatcaaatgtggctgagcaaatatttcctgatagctatcggtatcaggaaccaggtcacgccatgcaagtttcgtaatggtcaaagttgatgttttttagtctgttgtcaaagccgcgattataccgtaaccggcactacagcacacgtagaaagcaccgacaatactcctggcatgggcgttaaagctcacaggatggagattcttttcttcactggcctaaaaagctgatattctgtaaagagttacacggtaacattgagatcgctatgaaatatcaacaacttgaaaatcttgaaagcggttggaaatggaagtatctggttaagaagcatcgcgaaggggagttaatcacccgttacatagaagccagtgccgcccaggaagccgtcgatgtgttgctctcgctggaaaatgaacccgtgctggtaaatggctggattgacaagcatatgaatccggaactggtcaatcgcatgaagcaaaccattcgggcaagacgaaagcgccattttaatgcggaacaccagcatacgcgcaaaaaatcgatcgatctggaatttattgtctggcaacgtctggctggtcttgcgcagcgtcgcggtaaaacgctttctgaaacgattgttcagctgattgaagatgcggaaaacaaagagaaatacgcgaataaaatgtcttctctgaagcaggatctgcaggcattgctgggtaaggaataactgacgaaagtcagttcaatttactaaaggcaaaaaaaaccccgcagcagcggggtttttctaccagacgagaacttaagcctgcggctgagttacaacgtctttgatacctttaacttcgatctctacgcgacgatccggagccaggcagtcgatcagtgcagcacgctgtttcacgttgtcacaggtgttgccagtaaccgggttggattcgcccataccacgtgcggagatcttgtctgccgggatacctttggagatcaggtaatcaacaacagactgagcacggcgctcggacagaccctggttgtaagcgtcagaaccgatgcggtcggtgtaacccagaacaactacggaaccgtctttcggatccaggttgctcagctggctgtacagctgatccagagcagcctgaccttccggtttcagggttgctttgttgaagttgaacagaacgtcagacttcagagtgaagtgcttggtctgtacttccggtgccggagctggagccggagcaactactggagctgcttcgccctgaccgaaacggtaggaaacacccaggctcagcatgccgttgtccggacgagtgccgatggtgtgtgcgtcaccgatgttgttggtccactggtattccagacgggtagcgatttcaggagtgatcgcgtactcaacaccgccagcgaagaccggagaaacgccggtgtcgtggtttttaccataaacgttggatttagtgtctgcacgccataccatgccacccagacgagtgtagatgtccaggtcgtcagtgattgggtaacccagtttagcggtcagttgaacgccctgagctttgtatgcaccgttttcaacgctgcctttgtacggcatacgacctaaccagtcgtaacccatttcaaagccaacatacgggttaacctggtaaccaccaaaagcaccagcgcccagttggttttcatgggtcgggccattgttgttgatgaaaccagtgtcatggtactgggaccagcccagtttagcaccagtgtaccaggtgttatctttcggagcggcctgcgctacggtagcgaaaccagccagtgccactgcaatcgcgatagctgtctttttcattttttgcgcctcgttatcatccaaaatacgccatgaatatctccaacgagataacacggttaaatccttcaccgggggatctgctcaatattaactctaccgatatcttcggcttatgccgagcacccctggcgatgtaaagtctacaacgtagttgaaaacttacaagtgtgaactccgtcaggcatatgaaaaaaaagtcttgtataaggtatgtttaatcttttttgtcagcgacaatttacagaagagaatcgcggaaaccgcttcagacaagcctccgcaaggaaaattagtcacgactgaaagcattggctgggcgacaaaaaaagttccaggattaatcctaaatttacttaatgatacaaattagagtgaatttttagcccggaaagttgtctcgtggcgtgagaggatgcgcttaccggacgcataataaaccccatagcgttaccttcatttgccgcatcaacaagttcagcatgctcttcttcagtcaaatcatctgccaaccaaccgatcaccacactgtaattgcccgtgcgtaaagcgcgaaccattgactccacagtgtggcaaggggagagctggctaatctgcattactttcgttaagggtagcccagatgcctgaacccattcccgactcagtttttgttgcggtgttaaccagagttgccagcgcgattgctgaccgagttgctgtaacaatggcaacagtagaagttgcgtcatcatgggctgatcttcgcgatagacaacttcactgataagcccggctgtagtgttttccgtagagacacgcgcaattttacttgctgcggatgagaacgacgaagaacgatgtgcatagcctgaagtgtacataatcaatccagcccctgtgagttactgtatggatgtacagtacatccagtgacaacaaagatcaaccctattttcggaaagagcctcgcaaattttgtcgttggtgacgggaaaacataaattaatcttgccccttaagaataagttgcctattttcgtagttaacggatccgttaatgtgaatcattcttttatgttatgattttaaaaggaattttatgaaaagcctctcctataagcggatctataaatcacaagaatacctggcaacgttgggcacaattgaataccgatcattgtttggcagttacagcctgaccgttgacgacacggtgtttgcgatggtttctgatggtgagttgtatcttcgggcttgtgagcaaagtgcacagtactgtgtaaaacatccgcctgtctggctgacatataaaaagtgtggccgatccgttaccctcaattactatcgggttgatgaaagtctatggcgaaatcaactgaagctggtgcgtctgtcgaaatattctctcgatgcagcgctgaaagagaaaagcacgcgcaatacccgggaaagactgaaagatttgcccaatatgtcttttcatctggaagcgattctcggggaggtggggattaaggatgtacgggcgttacgtatacttggggcaaaaatgtgttggttgcgactgcggcagcaaaacagtctggtgacagaaaagattctgtttatgcttgaaggtgccattatcggcattcatgaagctgcgctcccggtggcacgccgccaggagcttgcagaatgggctgactctcttacgccgaaacaggagtttcctgcggaacttgagtaatctggcgttgcagacgaccaatctcaggcagtaatgcaatcaataatccaacttgttgtacgaccagaggttctttgctgtctgcccgtggttcaagttgctgcatccgctgtttcaggctagctaatgcctcattgacgcgttcttcatcagcaggttgatgatgtaacgcgtcatcaacatagcaaactgcgtcatcaagaaacgccagaatttcaggattagttaactgctcccggtgagcaccgagggctgagatatagctggtaaacgtatggttaaggcacagcaaccgaaacgcggcttcgcgaatttgcggggtaacgttcggctcgctggacatatttgataccaccgacgccagctcagcatcacggttgtgtgcatcgcggcgggcaatacgatacgccagacggttatcacgcccctgatggtattgctccagtatggcatcgagataccgacagttggcctctgtggcgcgttcgagcatgcgcggcagattgcgaaactgccagtcaggccagatgtagctcactgccgcccacgcaatggcacaaccaatcagcgtatcgattacgcgaggtaacgctacttcaaaaccttcacccagtaagttaaaacacagtagcaccaaaagtgtgatgaacatcgttgcatgagcgtattgcacgttacggaaggcaaaaaagagcacgccggtaataaccagcagcaccagctgcccttccagtgatggcacaaaccacagcacaggaatgccaatggcgatacctaccagcgtaccaataatccttaacttcaggcggtggcgcgtggcgttatagtttggctggcagacaaacaaacttgtcagcaagatccaatacccgtgatgcattccggttatctgaatgatggcgtagccgaagcacaacaccagcgacattcttaccgcatgacggaagagggcggattccggcgtgaagtgacggctaagacgcagccagatatcactcaacccgtgcgggctgtcatcagcgagctcattttcgtcattattatggggtagtgcctgggcctgttctgattcaattgttgccagttgggcatcaatggcgcgtaaattgttcagcaaaaatcccagtgttttgagtaaatcggcgggtgcgccgttatcgcgcatccgctccagcgcagcatcaatatgcgtaaaagcgcgctcaaaatgcggatcatgttgataaggctgacgcaacaaaatacagcgtgacagttgctggcacgcctggccctgcatcgacatcagccgctgaaaacggaacagcacgtcgctgtggcgaaaatgttcacgcaatgtttgatactgaatatgagaagagctggcacgctcgtgaatatcctgtgcgacaaagtaataatgcagcgtgcgacgcgttccccgttgaccacgatcgccacgtaagcgggtcagcagcgagagtttcgtctgattcaatgtcgccatcagcagaccgttggcgagagccaaatcgtacagcggtgcctggctttgatcttcaatatcaggatcaaacatgcgcgacttgagctcaagataacgcgccagttgttcatagcaacgcgccaggttgtcctgcagcgggcggaccgggaacagcagatgaccaataagtgtcaggacgttgtaccagacggcaccggccagcagatacatcggctgctgataccagtgctcatacagtgatgttcccaacatagtgtaaatggcgatcagcaatgcaccgaaggcaattgttgcatagcgttgacccagaccgccgagcaaaatgaagccgctggtagagagcgttaagccaatcgcaaatagccagggccagggaaacagcaattctactgaggccgaggcgataaaaaagcagaacagcgtaatgatgaggttacgcaaacgtcccgccagtcggtcatcgagatcggtcagcgccgctgccaccatccccagcgttagcggaatcgtcagttttacatcacccagccaccacggaaacgctgtggttccacaaagcgcaataaaaatacgcgcgtaatacagccaggcgctgttccaggtatagcgtttgagcaaaggacttagcataaaggccatattagtggattattcaaaacgacgacgtgcattggcttcacgcgcagcttgcgctgtttctaccgataccacgcgacgaccaaccggccatagtgcaatagcggcaattttaaagttcgcaatgccgacaggaatgccaatgattgaaatacattgtgcgatgcccgttgcaatgtgcatcaggcataaccaccagccaaagaaaatcagccagaaaatattcaataccgtaccgccagtattcagcagcacatttttgccagccgggttcagttcatcgacatgaatagcttcattgccataaggcaccagagacagtttagtgatctcccagcaggatcgtgtcagcggtaaggtaaaaatcagcacaatactgaccagagtcgccaacagccagcccagagtggtggcaaatccgccaagcacaaagttcagaatgttcaaaacggtacgcataaaacctcgctttactgtggttttcagtaatgggcggcaattgtaacgtttttttgggctggagcacgttttctctgacggttacactgataagaaataatttcgtgtggatctacagagtcatggaactgaaagcgacaacgcttggaaaacgtctggcacagcacccttacgatcgggcggtgatcctcaatgccgggattaaagtctccggcgatcgccacgaataccttattcctttcaatcaattactggcgattcactgtaagcgcggtctggtatggggcgagctggaatttgtactgccggacgaaaaagtggtgcgtctgcacggcaccgaatggggcgagacgcagcgtttttaccatcatcttgatgctcactggcggcggtggagtggcgagatgagcgaaattgcgtctggtgttttacgccagcaactggatttgattgccacgcgcactggggaaaataaatggctgacgcgtgagcaaacctctggcgtgcagcaacaaatccgccaggctttgtcggcgttgccgttgccggttaaccgactggaagaattcgataactgccgtgaggcgtggcgtaaatgtcaggcctggttgaaagatattgaaagcgctcggttgcagcataaccaggcgtataccgaagccatgcttaccgagtatgcggattttttccgccaggtcgagtcttcaccgctgaatccggcgcaggcccgggcagtcgttaatggcgagcattctctgttagtgctggcaggtgcaggaagcggaaaaacgtcggtgctggtggcccgtgcaggctggttgctggcgcgtggtgaagcgtcccctgagcaaattttattgctggcgtttggtcgcaaagccgctgaagagatggacgagcggattcgcgaacggctacataccgaagacattaccgcacgcacgtttcatgcgctggcgctgcatattattcagcagggcagcaaaaaagttccgatagtcagcaaactggaaaatgataccgctgcccgtcatgaactctttattgctgagtggcgcaagcaatgcagcgaaaagaaagcgcaggcgaagggctggcggcaatggctgacggaagaaatgcagtggtcagtgccagaaggtaacttctgggatgatgaaaaattacagcgtcgccttgcctctcgcctcgatcgctgggtaagtctgatgcggatgcacggtggtgcacaggcagaaatgattgccagtgcacccgaagagattcgcgatctgttcagtaaacgtatcaagttgatggccccgttattaaaagcctggaaaggtgcgctgaaggcagaaaacgctgtcgatttttcgggccttattcatcaggcgattgtgattctggagaaaggtcgctttatcagcccgtggaagcatattctggttgatgaatttcaggatatctcgccgcagcgggcagcgttgttagcggcattacgcaagcaaaacagtcagacgacgttgttcgctgttggtgatgactggcaggcgatttaccgattcagcggtgcgcaaatgtcgctcaccaccgctttccatgaaaactttggtgaaggcgaacgctgtgatttagacacgacttaccgttttaacagtcgtatcggtgaggtggcaaaccggtttattcagcagaacccaggccagctgaaaaagccgctaaacagcttaaccaatggagacaaaaaagccgtcacgttattggatgagagtcaacttgacgctttgctggataagctctctggttatgccaaaccggaagagcgcattctgatcctggcgcgttaccatcacatgaggcctgccagcctggaaaaagcggcaacacgctggccgaagttgcaaatcgactttatgaccattcatgccagcaaagggcaacaggcggattacgtcatcatcgttggcttgcaggagggaagtgatggttttccggctgcggcgcgggagtcgattatggaagaggcgctactgccaccggttgaggatttcccggacgctgaagaacggcggttaatgtacgtggcgctgacccgggcacgccatcgggtatgggcactgtttaacaaagagaatccctctccctttgtggaaatactgaaaaatctggatgtgccggtggcgagaaaaccgtaagaaacaggtggcgtttgccacctgtgcaatattacttcagacggtccgcgagataacgctgataatcggggatcagaatatcgaccgcgtcgttgaaatgcggcgactggattatgaagtctgccgttgccacgttggtggcgaccggaatgttccataccgtcgccagacgcagcaaggctttcacgtcaggatcgtgcggcacggcatttagtggatcccagaagaaaatcaatacatcaattttcccttctgagatcaatgcgccaacctgctggtcaccccccattgggccactcaacatcgcgttgacgttcatgccggtcgcgcgggaaattaagttaccggtagtgcctgttgcatacagtacgtgttgttccagtaacggttgatgccgttccacccagctcatcagcatttgtttgcagtgatcgtgtgccaccagcgcaatatgtttccgcgcaggtaaagtgcgagtcgtcagttccataatgtacatccgtagttaactttcctacagattactgtaagcacttatcgctgcaagataaagaccgaaaaagcctgcgcacaggcacaaaaatctcaggaagatggttgtttttccgcccactgcaggaaagtatttcgcgtttgtgggtcagccagtttaaaccaatacttcagccgttgttctgtgagcacctgagactgcggtggaatagcatccagctcggaaacacccgaaagcagcgtactgtcatctgccatcatcgtggcaaattgcggtagtgaagcgcgtttcgcggatttgttatagcgttcaacctcgacctcataatcaatcgtttttgccgttgaggtaatggcgagaatatccagctttaccggaatcggcgtcgcatcgccatccaacaattcaaggcgcggcgcggcatcaaaatggttagcttcccgctcattctccaggcgaggcaggcgaaaattgacctggttgatgagctgggtattaaaactgaccaccagcggtggggagatatacagccgttcttcactattggaaagatgaatcgtcttctcaacgcgaaacactaactgatgcggtccattatccagttcaatgctgtccgcaccgcgcagcagagagctggaaaccttcttgccgtcgagtaccagaagatcgacatcggttgaaagccgcagcgtggtggcaaaaacggataccggcaaacataatgcaatcaaggtggtcacgatgccggttttcataggtagctcctgtcaaaagaccgcccgaataataatgtgtcaaaatttttctttaatcatacttactaacatatagacatatttcccgcttttgctctcattcattcgtattagctgcatggttggcatgtcggctttgtcgtacactttgttaaacagtctggaggaaataatgaaagaaaccgatattgcaggcattttaacgtccactcacaccattgcgctggtgggggcaagcgacaaacccgatcgtcccagctatcgcgtgatgaaatatctactcgaccaggggtatcacgtcattccggtttcgccaaaagttgccggcaaaacgctgctgggccagaaggggtatggcacgctggcagacgttccggaaaaagtcgatatggtcgatgttttccgtaattcagaagcggcgtggggcgtggcacaggaagctattgccattggcgcgaaaactctctggatgcaactgggggtgattaatgagcaagcggcagtactggcacgggatgccgggttaaatgtggtgatggatcgctgcccggctattgagatccctcgcctgggcctggccaaataaaaaatccccggaaggcaaaaaccttccggggatttgttcagggattagttacgcagacgcggggcctggagttgtttgcggatggtctgcgccagctcatccatggatggctgttcaggatgttcatcctgcaattcgctacttagctgggcttcagccaggtaggtatgaaccggtaggccgttatcgtcctccatcactacgtgataccacggagcggcgcgaagctcgtcattcaccgccagctcatcaggcgacggttcagagagcgaataaaccgggtcgatatccacgaccactccgagataacctaacagggaatggcggacctgctggccgataccgaatttgctggcaatcatagtcacctcccgggaaatctttacctttgatataagggtaaaattccacatttcaagttacatgacgcgacaggcaaaccctttcagatatagcccttccggataggtagcgatcaccggatgatcggctgcctgacggaactgctctataaattgtacatcacgaccggcatcaattgcggcatccgcgatgattttctgaaataaatcgctggtcatcagaccggaacaggagaaagtcaggagaataccgccttcattcagcagctgaatcgccagcatgttgatgtctttataaccacgacacgcgcccatcaactggcttttattctcaacaaacttcggcgggtccatcacgataacgtcaaatttttcaccgcgatcgcgataagtacgcagcaatttaaagacatcatcacggacaaactcagccttgctcagatccagtttgttcagctcaacgttctgccgtgcaatatccagcgcttcctgggaggtatcaacgctgacaacctggctgcaaccgcccatcagtgccgatacggcgaaaccaccggtataggagaaacagttcagcacacgtttattttcaacgtagcggcgggtagccaggcggctatcacgctggtccaggtagtagcccgttttgtgtccgtgctgaatatccaccagcagtttcattccgtgttcttcaatcggcagcagggcaggtggcaactcgccggtgacggggccctgggtcagctccattccttcttttttacgtaccgcgacgtcgctgcgatcgtaaatcgaacattccgggtacagcgtttgcagggcactaattaatgccgcgcgctgatattctgccccagcactcagcagttgcagcaccagaaaattaccgaaacgatcgatagtaatacccggcaggccatcagattctccggcgattaaacgatagctgtcgaggccatctttttgcgccagccagtcacgccatttttgtgcttgttgcaaacggcgggaaaaaaaagcaatgtcgatagactcagacgggtcaaacgtccagacgcgcgcccggatttgcgaagctggcgaataagcgccgcgtgctaaccattttccctgatgatcaacaatatcgatggtttcaccgaggctggctttaccttccatgcgggcaacggccccggaaaagacccacggatggcgacgaagtaatgatttttcgcgccctttggctaacactaaacgtacactcataatttacttttctgtcgatgcaaagaaatgggcgtcattgtccggagttttccatggatttgcaacgcgtccattaaggataaggagagcagcaatgtcgaaagtctgcataattgcctgggtttacgggcgagttcagggcgtaggatttcgctacaccacacagtacgaagcgaaaagactgggtttaaccgggtacgccaaaaatcttgacgatggcagcgtggaagtggttgcttgcggtgaagaagggcaggtggaaaaattaatgcagtggttaaagagtggcggcccgcgttctgcgcgtgtagaacgggtgctcagcgagccgcatcatccctcgggggaattaaccgattttcgtatccgttaaatacattttaccggttttggcaggccagcaattttggtggcttgcttagccggacctttcggaaacagtcggtataaatagcggctgttacctttttcttcgccaaatttattcgccatcgcttttaccagcatacgaatcgccggagaagtattgaattccagatagaaatcacgcacaaaacgcaccacttcccagtgttccggtgacagcgaaatcccttcgttctctgcaatcaccacagccagcggctcactccactggctgctttctttgagatagccttcggtatccgtttctatctctttaccttcgaagatcagcataattattactaccttaatcagactggcggcagtgtaacaaaaaacaaagccccgcataaagcgaggctatgaaagtgttagcgggtgagattaatcgcggctagcgaagcccagaatgctcagcaggctgacgaagatgttgtacagcgaaacatacaggctaaccgtggcacgaatatagttcgtctcaccgccatgaatgatgttgctggtttcaaacaagatagcgccagaggagatcagaatgaagaccgcgctgatcgccagatgcagagcaggcagctgcaggaagatattcgcaaccataccaatcagcaccaccacaatacccgccatcagcataccgccgaggaacgacatatctttgcgggtggtcagcacatatgcagagcagcagaagaacactaacgccgttccgcccagtgccatagcgattacgtcacccattccggcagacagataggtgttcagaataggtccgaggatataacccagaaaaccggtaaaggcgaatgcggagataatcccggtcggcttattcgccgttttataggtcaggaacatcaaaccatacatacccaccagcgtcagaatcagacccggagatggcagcatcagcaccgtactggcagttgcggtaatcgccgaaaaggccagcgtcaggctcagcagaaaataggtattacgcagcaccttatgggtgctaagcagtgatgtacggtcatgtgaagaactaacaatacgatccattgagtcactctctatgacagatgtaattaattaagcagcataatgataatgcgtaagggcacccagaagttttacccatctttacgcatttgatctggaacaggtttaacagcggattatcaggtcattaagcaaatataacgccctgagaatttcgacaggcaaaagaaaaaggggttagcatttagctaaccccttatcttatttggcggaagcgcagagattcgaactctggaaccctttcgggtcgccggttttcaagaccggtgccttcaaccgctcggccacacttccggaatgacgcgcactataaacatcccgatgcggcgtgtaaacccctaatttgtttgtttgcctgaaaaacagccaaaagtgcattgatagcgtgaaataacagcagattgatcatttcatcaccatgaattccttctcttttactcgtttagcaaccggctaaacatccccaccgcccggccaaaagaaaaataggtccatttttatcgctaaaagataaatccacacagtttgtattgttttgtgcaaaagtttcactacgctttattaacaatactttctggcgacgtgcgccagtgcagaaggatgagctttcgttttcagcatctcacgtgaagcgatggtttgccttgctacagggacgtcgcttgccgaccataagcgcccggtgtcctgccggtgtcgcaaggaggagagacgtgcgatatgaataacgaggaaacattttaccaggccatgcggcgtcagggcgttacccggcgcagctttctcaaatattgtagtctggctgccacgtcgctgggattaggcgcgggaatggcaccaaagattgcctgggcgctggagaacaaaccgcgcattccggtggtatggatccacggtctggaatgcacctgctgtaccgaatcttttatccgctccgctcacccactggcgaaggacgtcatcctttccctgatttccctcgattacgacgatactttgatggctgccgccggaacccaggcggaagaagtctttgaagacatcatcacgcaatacaatggcaaatatatcctcgcagtagaaggtaatccgccgctgggcgagcaggggatgttctgtatcagcagcggtcgaccgtttattgagaaactcaaacgtgccgctgccggagccagcgcgattatcgcctggggaacctgcgcgtcctggggctgcgtgcaggccgcgcgacccaatccgacgcaggcaacgcctatcgacaaagtcatcaccgacaaacccattatcaaagtacctggctgcccgccgatcccggatgtgatgagcgccatcattacttacatggtgacctttgatcgcttgccagatgtcgacagaatgggccgtccgctgatgttctatggtcagcgaatccacgataaatgctatcgccgcgcccacttcgacgccggagagttcgtccagagttgggatgatgacgctgcccgcaaaggttactgcctgtacaaaatgggctgcaaagggcctaccacctataacgcctgttcctccacacgctggaatgatggcgtttctttcccaatccagtctggtcacggctgcctgggctgtgcggaaaatggtttctgggatcgcggttcgttctacagccgcgtggtcgatattccgcaaatgggtactcattccaccgccgataccgtcggtttaaccgcgcttggcgtggtggcagcggctgttggtgtgcacgcagtcgccagcgccgttgaccagcgcagacgtcataaccagcaacctacagaaaccgaacatcagccaggcaatgaggataaacaggcatgagcactcagtacgaaactcagggatacaccatcaataatgccggacgccgcctggtggtcgacccgattacgcgcatcgaaggccacatgcgctgcgaagtgaatattaacgatcagaatgtgatcaccaatgccgtctcctgcggcaccatgtttcgcgggctggagatcatcctacaagggcgcgacccgcgcgatgcgtgggcgttcgttgaacgtatctgcggcgtctgtactggcgtacacgccctggcttcggtttacgccatcgaagatgctatcggtattaaagtgccggacaacgccaatatcatccgcaacattatgctggcaacgctctggtgccacgatcatctggtgcacttctatcagcttgccgggatggactggatcgatgtgttagatgcgctgaaagccgacccgcggaaaacctccgaactggcgcaaagtctctcctcttggccgaaatcatcccctggctatttcttcgacgtacaaaaccgcctgaaaaaatttgttgaaggcgggcagttggggatcttccgcaatggctactgggggcacccgcagtacaaactgccgccagaagctaacctgatgggctttgcccactatctcgaagctctcgatttccagcgtgaaattgtcaaaatccacgcggtctttggcggtaaaaacccgcatccaaactggattgtcggcgggatgccttgcgccatcaacattgacgaaagcggcgcggtcggggcagtcaatatggaacgcctgaacctggtgcagtcaattatcacccgcacggcggacttcattaacaacgtgatgatccccgacgccttagccatcggtcagttcaacaaaccgtggagcgaaatcggcactggtctttctgataaatgcgttctcagctacggcgcattcccggatattgccaacgactttggcgagaaaagtctgctgatgcctggcggcgcggtgattaacggcgacttcaacaatgtgctgccagtggatttggttgatccgcagcaggtgcaggagtttgtcgaccacgcctggtatcgatatcccaacgatcaggtcgggcgtcatccgttcgatggcatcaccgacccgtggtacaaccccggcgatgtcaaaggcagcgataccaacattcagcagctgaatgaacaggaacgctactcgtggatcaaagcgccacgctggcgcggtaacgcgatggaagtggggccgctggcgcgcacgttaatcgcttatcacaaaggcgatgctgcgaccgttgagtcggtcgatcgcatgatgtcggcgttgaacctgccgctttccggtatccagtcaacgttaggccgcattttgtgccgcgcgcacgaagcgcagtgggccgcaggtaagttgcagtatttcttcgacaagctgatgaccaacctgaaaaacggcaatctcgccactgcttccacggaaaaatgggaacctgcaacctggccgacagagtgccgtggtgtcggttttaccgaagcgccgcgcggggcgttaggccactgggccgccattcgcgatggcaagattgatctctaccagtgcgtggtgccgaccacctggaacgccagcccgcgcgatcccaaagggcagattggcgcttatgaagcggcgctgatgaacaccaaaatggcgatccccgagcaaccgctggagatcctgcgtactctgcacagctttgacccgtgcctcgcctgttcaacacacgtgctgggcgacgacggtagcgagctgatctccgtgcaggtgcgttaacagcgaaggagaatcatcatgcaacagaaaagcgacaacgttgtcagccactatgtctttgaagcgccagtgcgcatctggcactggttgacggtgttatgcatggcggtgttgatggtcaccggatactttatcggcaagccgctaccttccgtcagcggcgaggcgacgtatctgttctatatgggctacatcaggttaattcacttcagcgccgggatggtttttaccgtggttttgctgatgcggatctactgggcttttgttggcaatcgatactcccgcgagctgtttatcgtgccggtatggcgtaaaagctggtggcagggcgtgtggtatgaaatccgctggtatctgtttctggcaaaacgtccgagtgccgatataggccataatcccatcgcccaggcggcgatgttcggctatttcctgatgtcggtctttatgatcatcactggttttgcgctgtacagcgaacacagccagtacgctatttttgcgccgttccgttatgtggtggaatttttctactggacgggtggcaactcaatggacattcacagctggcatcggctggggatgtggctgattggcgcgtttgtgatcggtcatgtctacatggcgctgcgtgaagacatcatgtccgacgacacggtgatctccaccatggtcaacggctaccgtagccacaaatttggcaaaataagtaacaaggagcgttcatgagcgagcaacgcgtggtggtcatggggctgggcaacctgctgtgggccgatgaaggcttcggcgtgcgggtggcggaacggctgtatgcccattaccactggcccgagtatgtggagattgtcgatggcggtactcagggactgaacttgctggggtatgtcgaaagcgccagccatctgttgattctcgatgccattgactacgggctggaacctggaacgctgcgaacctatgccggagaacgcattccggcttatctcagcgcgaagaaaatgagcctgcatcagaacagtttctccgaagtgttggcgctggcggatatccgcggacatctgccagcacatattgccctcgtcggtctgcaacccgcaatgctcgacgactacggcggtagcctgagcgaactggcacgggagcaactgcccgctgcggaacaggcggcgctggcgcagcttgctgcgtggggaattgtgccgcaaccggctaatgaatcgcgctgtctcaattatgactgtctgtcgatggaaaattacgaaggcgttcgcttgcgccagtaccggatgacacaggaggagcagggatgagcaacgacacgccatttgatgcgttgtggcaacgaatgctggcgcgcggctggacgccagtcagtgaatcccgtcttgacgactggcttacgcaagcgccagacggcgtggtgttattaagcagtgacccgaaacgcacgccagaggtcagcgataatccggtaatgattggcgaattactgcgcgagtttcccgactatacatggcaggtggcgattgctgaccttgagcagagcgaagccatcggcgatcgctttggcgtctttcgctttcctgccactttagtgtttaccggcggaaactatcgcggcgtgctgaatggtattcacccgtgggcggaactgataaacctgatgcgcgggcttgtcgaaccgcagcaggagcgtgcctcatgagcgaaacttttttccatctgctggggccaggaacgcaaccgaacgatgacagtttcagcatgaatccactgccgatcacctgtcaggtgaatgatgaaccgagtatggcggccctggagcaatgtgctcacagcccgcaggtgattgcgctgttaaacgagttacaacatcaactaagcgaacgccaaccgccgttgggcgaggtgctggcagtcgatctgttaaatctcaacgccgacgatcgtcactttatcaatacgcttctcggggaaggggaagtgtcagtgcgcattcagcaggctgacgacagtgaaagtgaaatacaggaggcgatcttctgcggattatggcgggtgcgcagacgtcgcggcgaaaagttgctggaggacaaactggaggctggctgcgcgccgctggcgttgtggcaggcggcaacgcaaaatctcttgccgacagattcgctgttaccgccgcccattgatggcctgatgaatggcctaccgttggcgcatgagttactggcacatgtacgtaaccccgacgcgcagccgcacagcattaatctgacgcaattacccatcagcgaggctgatcggctttttctctcacgtctctgtgggccgggaaatattcagattcgtaccattggctatggcgagagctatatcaacgccacggggttacgccatgtctggcatttacgctgtacggacaccttaaaaggcccgttactggaaagttatgaaatctgcccaataccggaagtggtgctggcagcgccagaagatttggtcgactctgcgcagcggcttagcgaggtatgtcagtggctggcggaagctgcaccgacgtaaaaagacggtaagtatcgctttcagtcttatgaatatcgcaatcggcgaatacctctggtcgtagagtttcaggataaagagggagatctaccattatcgggttatttttctctcttcgcctacaggagtgcgcatgtgggatgtcattgatttatcgcgctggcagtttgctctgaccgcgctgtatcactttttatttgtaccccttaccctggggctgatttttttgctggctattatggaaaccatttacgtggtcaccggcaaaacaatctaccgcgatatgacgcgcttctggggtaagctcttcggtatcaattttgctcttggcgtggctaccggcctgaccatggagtttcagtttggtactaactggtcattctattccaactatgtgggcgatatttttggcgcaccgctggcgatggaagcattaatggccttcttcctcgaatccacctttgtcgggctgttcttcttcggctggcaacggctgaataaataccagcacctgctggtgacgtggctggtggcgttcggttcaaatctctctgcgttgtggatattgaatgccaacggttggatgcaatacccgaccggtgcgcattttgatatcgacaccctgcgtatggagatgaccagcttcagcgagctggtctttaatccggtcagccaggtgaaatttgtgcacaccgtaatggcgggctacgtgaccggggccatgtttattatggcgatcagcgcctggtatttactgcgcggacgggagcgcaatgtcgcattacgctcgtttgccatcggttccgtcttcggtactctggcgattatcggtaccctgcaactcggagacagttctgcgtatgaagtcgcgcaagtacaaccggtaaaactggcggcgatggaaggggagtggcaaacggaacctgcacctgcaccgttccatgtggttgcctggccggaacaggatcaagagcgtaacgcctttgccctcaaaattcccgcgctgctagggatcctcgccactcactcattagataaacccgtgccgggtctgaagaatttgatggctgaaacctacccacgcttgcaacgcggacgtatggcctggctgttaatgcaggaaatatcgcaaggcaatcgtgagccgcatgtgttgcaggcattccggggactggaaggtgacctgggctacggcatgttgctctcccgctatgcgccggatatgaatcatgtcacagccgcacagtaccaggcggcgatgcgtggcgcgatacctcaggttgcgccggtattctggagtttccgcatcatggtgggctgtggttccctgctgctactggtgatgctgattgcgcttgtccagacgctgcgtggcaaaatcgaccagcatcgctgggtgctgaaaatggcgctctggagtttgccgttgccgtggattgcgattgaagccgggtggtttatgaccgagtttggtcgtcagccgtgggcgatacaggacatcttaccgacatactccgcgcactccgctttaaccacaggacaactggctttctcactgatcatgatcgtagggctttacaccctgttcttaatcgccgaagtctacctgatgcagaaatatgcccgtctggggccgagcgcgatgcagagtgaacaaccgacgcagcaacaggggtaaaggagaaaatcatgtttgattatgaaacattgcgcttcatctggtggctgctgattggcgtgatcctggtggtctttatgatctccgacggatttgacatggggatcggctgtctgctgccgctggtggcgcgtaatgatgatgaacgccggatagtgataaacagcgttggtgcacactgggaaggcaaccaggtctggttgatcctcgctggtggggcattatttgccgcctggcccagagtgtatgcagcggcgttttccggcttttatgtggcgatgatcctggtgctgtgctcactgttcttccgcccgctggcctttgattatcgcggaaaaatcgccgatgcacgctggcgtaaaatgtgggacgccggtctggtcatcggcagtctggtgccgccggtagtcttcggtatcgccttcggcaacttgttgctcggcgtgccgtttgccttcacaccgcaattacgcgtggagtatctcggcagcttctggcaactgctgacgccattccctttattgtgcggattgctcagccttgggatggtgattttgcaaggtggcgtctggttacaactgaaaactgttggtgtgattcatctgcgttcacagctggcgaccaaacgcgctgcactgttggtgatgctgtgctttttgctggcgggttactggctgtgggtcggtattgatggctttgtactgctcgcccaggatgctaacggtccttccaatccgttaatgaaactggtggcagtgctacctggtgcctggatgaataattttgtcgagtcgcccgttttgtggatcttcccgctgctgggattcttctgcccattgctgacggtgatggcgatttatcgtggtcgcccgggttggggatttttgatggcatcattgatgcaatttggcgtgattttcacggcaggcatcacgctgttcccctttgtcatgccgtcaagcgtgagtccgatctccagcctgacgttgtgggacagtacttccagtcagctgacgctgagcattatgttggtaatcgtgctgatatttttgcccattgtgttgctctacactctctggagctactacaaaatgtgggggcgcatgacaacagaaactctccgccgtaacgaaaacgagttgtactaaggagcagaaacaatgtggtatttactttggttcgtcggcattttgttgatgtgttcgctctccacccttgtgttggtatggctggacccgcgtctgaaaagttaacgaacgtaggcctgatgcggcgcattagcatcgcatcaggcaatcaataatgtcagatatgaaaagcggaaacatatcgatgaaagcgatcttaatcccatttttatctcttctgattccgttaaccccgcaatctgcattcgctcagagtgagccggagctgaagctggaaagtgtggtgattgtcagtcgtcatggtgtgcgtgctccaaccaaggccacgcaactgatgcaggatgtcaccccagacgcatggccaacctggccggtaaaactgggttggctgacaccgcgcggtggtgagctaatcgcctatctcggacattaccaacgccagcgtctggtagccgacggattgctggcgaaaaagggctgcccgcagtctggtcaggtcgcgattattgctgatgtcgacgagcgtacccgtaaaacaggcgaagccttcgccgccgggctggcacctgactgtgcaataaccgtacatacccaggcagatacgtccagtcccgatccgttatttaatcctctaaaaactggcgtttgccaactggataacgcgaacgtgactgacgcgatcctcagcagggcaggagggtcaattgctgactttaccgggcatcggcaaacggcgtttcgcgaactggaacgggtgcttaattttccgcaatcaaacttgtgccttaaacgtgagaaacaggacgaaagctgttcattaacgcaggcattaccatcggaactcaaggtgagcgccgacaatgtctcattaaccggtgcggtaagcctcgcatcaatgctgacggagatatttctcctgcaacaagcacagggaatgccggagccggggtggggaaggatcaccgattcacaccagtggaacaccttgctaagtttgcataacgcgcaattttatttgctacaacgcacgccagaggttgcccgcagccgcgccaccccgttattagatttgatcaagacagcgttgacgccccatccaccgcaaaaacaggcgtatggtgtgacattacccacttcagtgctgtttatcgccggacacgatactaatctggcaaatctcggcggcgcactggagctcaactggacgcttcccggtcagccggataacacgccgccaggtggtgaactggtgtttgaacgctggcgtcggctaagcgataacagccagtggattcaggtttcgctggtcttccagactttacagcagatgcgtgataaaacgccgctgtcattaaatacgccgcccggagaggtgaaactgaccctggcaggatgtgaagagcgaaatgcgcagggcatgtgttcgttggcaggttttacgcaaatcgtgaatgaagcacgcataccggcgtgcagtttgtaatgcataaaaaagagcattcagttacctgaatgctctgaggctgatgacaaacgaagaactgtctaatgcgtagaccggaaaaggcgttcacgccgcatccggccactttcagttttactctttctcggagtaactataaccgtaatagttatagccgtaactgtaagcggtgctggcgcgtttaatcacaccattgaggatagcgcctttaatattgacgcctgcctgttccagacgctgcattgacaaactcacctctttggcggtgttcaagccaaaacgcgcaaccagcaggctggtgccaacagaacgccccacgaccgcggcatcactcaccgccagcatcggcggcgtatcgacaatcaccagatcgtaatggtcgttcgcccattccagtaattgacgcatccgatcgcgcatcagcagttcagacgggttaggtggcacctgaccgcgagtaatcacatcaaagcctcctttgccaaaatgctggatcactttgttgagctcatctttacctgccagatattccgacaagccatgttcattactcacggtaaacaggttatgcgaataaccacggcgtaagtcggcatcaataaataacactttttgatcggactgggcgatcaccgctgccagagttgaactgacaaacgttttaccactgtctggcgtcgcaccggtgatcattagaatgttattctccgtctccatcatagcgaaatgcagactggttcgtagcgcacgtacggcttccacagcagaatccgccgggttatccaccgccaggaaggggatatttttagtacgatggcgctgctgattagaaaataaatttttcttacgcagacgggtgcgtttatccagccactcggacattgggatagtggcataaacgctgatgccgtgctcttccagttgttccggggcttctacaccacgacgcaacatcgcacgcgccagcacggcacccacagaaataaacaggccaagaataaaaccaagcaccacgttcaacgcttttttcggtttcactggctgcggctgagtgactgccgggtcgataatccgcacgttaccaatggcactggatttcgaaatactcaactcctgctggcggttaagtaattgcagatataccgcacggcccgcttctacgtcacgacttaaacgcaacacttcctgttgggtggaaggcattgccgatacccgcttattcaggcgtttgcgttcttgctccagcgtctggcgtttttccagcagcgcacgataagttgggtgatctttcttatacagctgggagatctctgcctcgcggaaggtcagctcattgagttgattatcaacgttcacaatctgctcaagaacggctttggcttccaggttaaggtcaaccgaatcgcgctgctggcgataaacgttgagtttttcttccgcttggtccagctcgctgcgcacttcaggtaactggcgctgtaagaattcaaggctttgtgaatcctgcgccgcctggcgagcgatattctgttgcaaatagttgttagcgatgctgttcagaatacgagtaatcaactggggatcatcaccagtcatggtaagttccagcatcccgctttctttactgcgttcgctaacggtaaaggtttcctgcaatgcgttaatcgcttccagttcggtacgctggctcaggacaaactgtgttcctggtttggccttaatgtccgcgatagtcagcgcaacgccatctttttccagacgctggccgaccataccattgacggtgaactcttcaccttccagtgtatagtggccgttttccccaaccgtgagtgtcagttgctgatcctgaccattcagttgtggaatatgcatccagctgatcgccagctcacctggtttttctttggttaatctcgcccagccgcgacccacaatcggaaaatacttctgctcaactatgtcgcgcagattcagttcagcaatggttttaccgagaatcatgcgcgattgcagcagttggatctccggtgcagactcgggcgatgagttagggatcatatcgctcaggccgctgagaatggcgttgccctgtttttgctcaacctggaccagagtatctgcctgataaattggtgtgcttaacagcgagtaagcgacagcgatcagcgtgaataacgcggtcacgctgataataaacttacggtgatcccataactcgccgaccagacgaagcagatcgatctcattttcctgagtgctgcctggtggcgtattcatatttttagttgtcatcgtattttataaactcaaattaccggctgaggcgcttcgcccattcctgactggcgcgctccaacataccgtagacatgttcaaatgcgtcctgacttttacgatagggatccgggatctctttctgttccagccattgcccaaacagcattgtcttcccgcggacctcgggagcaattgcggtaacctgagcaatatgttccgactccattgccagaatcagatcgtaatttcgtgccatctcagcagtgagcttacgtccggcatgtccttcaagagatacgccatgattagcggcaacatctgccgctgtcgcatctgcagggtgttttaccagaccatgaacacctgccgatttgacttttacgcccggcagacgtttacgcagcaagcgctcgccaatgggcgaacggcaaatgttgccggtacaaaccaccaggattgagttaaattttagttgggccatgtttgaatccaccgtgaagtctctgtcaggtcatgcaccccggaaatcgtcggtaccagcagagaaatcacacggttccaacgagccagcggcgcggtagtgacataaacaatgtcgtaaggttcaagctggaattccgttccgagtatcattgccgatgcgtccttcgcattcagctgataaatattggcgattttgccattctgcttgttttgcgttgcacgaataacaaaaatccccgtcgcatcagcgacatcctgattcataccctcagcgttacccagcgcttccgccagggtcataccgctgcggtccattttcagcgtgctctgtttacccacttcacccatcacgaagactttcagatcatcgttgcgcggaataaataaaatatcgcccgggtgcagcagtttgttctggcgcaagtcgccacgctgcatcagcgcatagaggttcactttggtctttacgccattctgggtgagcaccacgttgcgccagtctgcatctgcggtcagaccgcccgcggcgttaatcgcatccatgatggtcagaggaatattggtaatcggctgctgacccgatttgctgacttcgccggtgacgtacgctttttgcgatcggaacgccgcgacgctgacatcgacttgcgggctttcaatgactgaatcgagacgcgctgtaatctcgttgcgtacctgggtaagtgttttcccggccactttcaggcgaccaatataggggtagaaaatcgcaccatcggcgttaacccagttgccggtatcactggcgctacggtattgccctgcgggggtggttagttccgggtgatcccagaccgtaaccatcaacacatcaccaatcccgatacgatattcatagtttgcgatttgctgctccagctccgggttagcctgcgacataatcggtttggcgcgcaactgatcaatcaatcctggcgtgacgggatagatattgaccattttgtccaggtcatactgattgtcaggtagttcaatgacatccttgttactggtcgataaattctgaccaggaacaagggtacatgctgtcaaagacagaacagccaatgtcagtaccgaaaacttaaaaatgttctttttcattggtttatatttatcagtcaatgtaatgttatgaattacgtcaggttattgtccaaccggtacttctcgctctgccgtcattggatagagctggtatttgcgtgacagcatttgtccaccatcacgcgtcaatggtgtccacgaaaccaccgcgcggttgcggttaggtccaatggtcatcaagtcgaatggaatcgagatataaaaacctttactaaagccgccttcgccgtagtcatctttagatacgttactgattgccgcccatacccctaccgccacgccgctgtcaaagcgtttggcgacgtcgatcgttgcgcctttatcttttgccagatattgcccaacgctaagtttcatcagtacgccattgagcgtcggcgggttccagtaagccgtcacgaaacctgttggcgtggaataatcggtgaaacgcatcatgttgtcccagtcacgttgcttcacgtagttaacgtccacacccagcgcccagcaggcatctagcgggcgataaagcagctcggaaccgacaccggcgtacatcgtttccagataaccgccatacacctggccatagaaaccattgcctaagtcagcaaaatagttcgcctgcaagttgttgagataaacgtcattgcgaacgtagtcacggatatgcgtgcgcacgcggggcagggtagagtccgcgggcaacagcgaagacttaaacttgtcgtagttgttgtaaatattggtgaaaataccgccatcaagcagcaggtggtcggtaaaccagtagcgggcactggacatcagccccagctggaacatatagaaatcttccgggccgcccagcgactgtgaaagtgttgggttgaaagagtagctaaagcgatcttcacgaatacggtagccccgaccaaaggcagaaagatcttcagcttcaacacgttgttgttgcagtggctctgattgaccaggcgctgtacctgccagctgtttgcgcaggctggctacgtcggtttcggtagtcaccatcgccatatgctcgcgcttttgcgtcacgctaatcttctcaacgccttgcggcaggttattcaccagaatccggttggcacgatcgaccgcttcacgagagtcacggtatttgtattgctgaccagacatatacagtgtcttatcgcgtagctgaatttctggcgcgtcaaagcccgcgttatacttcagggcggtaagttggtttgctaccgtggtgtactgcaatccttcagattcaggcgcaggttgatatgccggttttggcgtatcgcgcagggcagggcgcagatcgttgaaattggtccgtaacgtgaagccaaacatcaacgtgttaccgcgttcataactcaggttgagatctgcccagctggcagcgcgataaactgcgccgacgttgaaatggcttgcctgaggcagtttgccagcgaaatcattctggtaattgtttccatcgtattcgagtttcagacgcaggggattccacggcgtttgatactcaatgccgccaaagatggaagccgggccacgaaagatatcgctaaagctgatatcgcccgcatcgtgagactctgcgcgatgacaatatttatcgctcacccggcaaaacgggttggtaatattgcccgcattaccggcgtagccccatgccatcccgagggtgaaatcaaatggccccgcttgcttgctggccaccagatactcaccgtcaaacagacccgtaccagcaatatcacgtttaccaaacgccacttgcggtagccagtaaccttcttcccacaggcgaagtttaaaatcgaatgatttgtctttgtatgactgatcgccgctgaaatcttcccactggctatatttgcgtgtgcgcacatccgtataacgaatggtgccttccagccatgggaacagcgccacggaggtggagtagaaccggtattgatcgttatcccggtagttgacgctgaattcaccttccggtgcgatgcgcgcatttggcatctgcaacaatcctgtgccgccaaagtctgattgcgacgaacccagcggatccgggtaggttaatacttcagcatgacaggcactggagacggcaatggccaggcagcttaaaagataagaattcttcttcatcagtcaggaacacgttgcgttaaaacagacacaatctggtcatttaaatcagcatatttttcgggcagtacatgcgcagaaaagcccaaccaaagctggctgccaggcggtggttccacatgtcttttattccacagggcaacaggggcgacgacagtctcaccctcaggcgtaatcaccataacgttattcttgtccgcgcctgcaaggcgggggtgatcttgcagataatcggtaacgctacggcctgcctgccagggcaattgcccggccccagaaaccgcacccagcagagtaatagtcaccggacgctgtacggtatagagcgtatagtccccgaccaacgggggattgctgttctcatccactcgtacaaaatcagggtccagtttgaccggtaagcgaccagtgatattgagattgagtaactgctggcgcacggatttaatcgttgccgccacatcgtcgtcagcttctgcttcccaggaagcaagctgtgccatgacatgttggtagtctttaagcgctttagctttcgccgcagagtcggtcagcaaggcaccaggccaccagaggcgatcgcgcagttgcggttgtgtcaccaactggacaacattttccacggggccaacggaaagtgtctgttgttcgccaggcagataaatagtcaccgttccttgcgcaaaggcatggggtgtcattacgtaaagtacgctggcaatgaaatacgactgtaatttattcatggtgcgggtttaagaaacgtcatttctacgggaataacccctgcgcctaacatttgccgactttgacgaacctggccagtagccgaatcgacccagaatgtgttttgccactgtttttctggccgcgtggaagtcacctcttcctgccagacattacacagcacattgcgacccgcaatattcagcgtctctaatccagcaaaggaaaaagtagaactcagggtcgcagagcgaaaatggttgtcttcactccagagaatatcgcgcgtccagcggctgccatcttttattgccagcgcgttacgcagagggtcctgcccggaatttgtcacttccagcagattattattaagtttgacggtttttaaaagacgtccattgtgggtaaccagcatggcgttatcctgggataaccatttgctttgttcttgttctatatatcccagtaccacaaagattcgttgcccttcattaaggcgtaaatacatagtggaataaggcaacgcctggatctgctgatccgctacggtgatatcctgattatcgaaaaggctggcgcgaaatgtatcgaccatactttgctggctgtgcgtacatcccgcaagaaatagtgcgaaaatcgataaaataagagggcgcacctttaatccttgaaaggttaattaaaaaaatgcaaatctctaaagcccggtacgaatatcgcaaccgggtatcatttaactttaatttcgacgcgttaaagcagtattagcgtgtagtggacgtggtggttgaggtgttatgagaaccgccatcgccactgtcatttgctgcaacaactgccaacgtcgccacaccaacagccgttgccacaccgacaactgtcgccgtgccgacagcgccagcagccacgccaccagtggtagtagcagtcgtggttgcgccggtagtggtcgttgtggtgccagtagtacccgtcgttgcctcggtcccgtttgttgcttcaggggcagcaaacgcagctggcgtcgtcaacatgaaggccataaggattgcagaaagcttgtgtttcataacttttcctttattcatcgcatggacaatacgggtgatgctgccaacttactgatttagtgtatgatggtgtttttgaggttctccagtggcttctgtttctatcagctgtccctcctgttcagctactgacggggtggtgcgtaacggcaaaagcactgccggacatcagcgctatctctgctctcactgccgtaaaacatggcaactgcagttcacttacaccgcttctcaacccggtacgcaccagaaaatcattgatatggccatgaatggcgttggatgccgggcaacagcccgcattatgggcgttggcctcaacacgattttccgccatttaaaaaactcaggccgcagtcggtaacctcgcgcatacagccgggcagtgacgtcatcgtctgcgcggaaatggacgaacagtggggatacgtcggggctaaatcgcgccagcgctggctgttttacgcgtatgacaggctccggaagacggttgttgcgcacgtattcggtgaacgcactatggcgacgctggggcgtcttatgagcctgctgtcaccctttgacgtggtgatatggatgacggatggctggccgctgtatgaatcccgcctgaagggaaagctgcacgtaatcagcaagcgatatacgcagcgaattgagcggtataacctgaatctgaggcagcacctggcacggctgggacggaagtcgctgtcgttctcaaaatcggtggagctgcatgacaaagtcatcgggcattatctgaacataaaacactatcaataagttggagtcattaccgacaatacgtacgcttgagatcaggattgtctactttgagtataacatccttgtgaaatctccctttcctcataccgcttgcactatatactgcgggtaggaaaggcgcgcagagggaaatataagattgttaactatccccctctggaaatacgacttgtgagcataagataaatcttagcaaaatacaaattaaagataaggaaattgttacgaaagctattaattattgttggtaatatagtttcaagtggtactataactggctgttaaatggcatttataactattaggtgcagagatattcgcttaaatggattagtttctttgtggaaaagtaactgatgttataatgtatgatgttgactatttcactattccaataaaaccagtcagctttaaacaagcagcgtcatattaagagagataaacatttgccgctgttggtcctcgcaggccatttacgcggcaaaattccacacgtaatcctggtataagcacttctgcgtcgcggggagtgaatgcggaaatatggacctgaacttctttacgaccgtcggaggggataatgaatcctttgccgcttttgcgatcaaaggttttgacaattcctgtcattttacgggacaaacaaattccttactgaaaatactgcgctgcactatacggggttaataaaataaagccagcgatatttaagaccgccggacggctaaaataaaatttgcttaatctcaattatcatgcgttaatagctgcgtcggtttgaaagacagacagcatacaaagtagtttactaaagcagttctcattatcaggcattatccccttcttttgagtctctctcctgaacactaagtagtttctgtattaaagccctgtttgccgaaaggcccaaaatgaaggaagtaaaatatgtctaataaaatgactggtttagtaaaatggtttaacgcagataaaggttttggctttatcactcctgatgatggcagcaaagacgttttcgtccatttcaccgccatccagagcaatgaattccgcacgctgaacgaaaatcagaaagttgaattttctattgagcaggggcaacgtggccccgcggcagcgaacgttgttacgctctaaggttgccattattactcaacatctccatttccgctgtccatgttgtcatggttcacagtaccgcacatcggcattcgatgtgacggagcgaaaccctttgggcgctaagtgtattttttgtaaatcgacgatgatcacctttgataacgtcgcgctgcaaatacgcactgaccatgcgccgctggatttcacaaaataatatcaggctccctcgtggagccttttttatatctgccttatttttcttcaacgctgtatgtatagtaagcgataacctgttgattattgaatctttcggggagatggcttataacatttcttacctgaccagggtaccgggaaccaacaccttactggcgtgttgctgtcttttaagaccagaagaggttaacagtgaatattgaagagttaaaaaaacaagccgaaacggaaatcgccgactttatcgcgcaaaaaatcgccgagctgaacaagaatacagggaaagaagtctctgaaattcgcttcaccgcacgagaaaaaatgaccgggcttgaaagttatgatgtcaaaatcaaaataatgtgattttgtgaacatcaccccgtgcgaggtgatgttccgcttgttgctaatttagtgaccaatcattggcgcttgtggaattaagcgtcggtacaattcctccggcaccgggctttgccatactcccgcatacattgcgtaaccaatcaccgcaaacataatccccagaaccagtagcgtcattaaccagccagacaacgcaaaggcttttttatttgccgcaggtttttgcagtgaaaaggtcaatgttgaggctaccggacatgactctacgcaagtcatacagccggtacattccactgttcgtacctgaattaatttatcgaccgggatccgtgatgggcaattttttgcgcatttgccacagtcgatacaactttcggcattgcgacgaatcttaaacggcgacaatagcgaaaccacgcccatcagcgcgccatatgggcaaagataacgacaccaggcatggcgaataaacaggctggcaatcagcaaaacggtcacgctgattaatgtcgcggtccccatatgacgaaagaaatcgagcattttaacgtccatcaccacgctgtagggcgacaacataaaatagtgaatcgcctgagcgggcatcaataacgcgatatagataaaaaaactcaacagcaaatacttcacgccgcgcagaggaatatccagccagcggggaaggacacattgccgaccaaacagtttgttaccgagatcgccgattaattcagaaagcgtaccaaccgggcataaccatgagcaaaaggcctttttgagtaatagactgatgacgataaaagcgaccaataacagcatcgcggcggcgtggacggacggtaactgacctgttacaaggctatatttcagattcatcagcccggcaatcggtagccagccttcgatacctcccggtctggcgacaaatgtcgtgctacttgccgtttcgtaatagcgcacccaataccagaacgtgatggcaatataaatattcattgccaacagtaataattgcgtcgctttacgccaggtcgtggcattacgccagtcattccacggtaatttgccgcccgtcgtgcctggccgccgctgccagcgggttcttttattctctgccatgattttgccagtccgttaagttgtataccaaatgccactattctagttgttcttaactggctgatattgattcaaatcgcgttcaggtctttcttatgcaaccatgcttccagagcggcaacactgcgtgtaatttcttcgtgtggaaggggggcagataatggctgctgctccagttgtgcgcatagctggctggcgatatgcattcccagactcgagcaactgctttttagctgatgcgcggcacgctttattttctcgctatcctgactggcgcgggcaatgtcgatttcatcgagaagcggcagggcatgttgtgtaaataataccagccattcgtggatcttctccgtccccattaactgagcatcttcattgagttgcgatacatccagcgattgatcattattgacttgcagttggagatagtgcgccagtaactgaccgagcacttcacgcggcaccggtttagggataatcccgcggaataatgaactggtacgctggcgcagcgtttcgtcaatgacatgggcgctaaagccaatcaaaaccagcgacggatattgctgtgccagttgtcgggcaagcgtaatgccgtcgatatccggcagatcaaaatccaccagtgcggcagcaaacggttcgctattttgcagtgtctctaaagcctgcgcggcattgccaacagcaacaatctgcgcaccactggttttcagcatctcaatggtaattcgctgggttagcgggttatcttcaattaacagcaaacgtaaaccgtcaagacgcaccgcctgattgactgtttttggcacgggtgccgtggcaacacgtaacggcaagcgtaaacaaaaacagcttccaacctccggcgtgctggtggcgctcagttcgccgcccatcgcctgggccagacggctactgatagtcagtcccagcccggtgccgccgcgtttgccgcttacctgcacaaatggctggaagatttctgccagtttcgcgggatcaataccgcagccgctgtcttccacttcgaccagccattgctcgccatcagtgcgactacgcaggataatgtacccttcgtcagtaaaacgcagggcgttgctcaacaggttggttataacctgacgaatacgtcgtggatcgcccattaacgcgcacggcatatcatcggcaattgccgttgccaggcgaatcgggcgacctttcacccgtccgctcattaattgcagggtactttccagcagcgggcgcggttcaaagggctcatcgctgaccgaaacattcttgccacctgcttcgatagcggaataatcgagaatatcgttgaggatggtcagcaacgattcaccagagtcagtaattgcccgcaaatcatcacgctgggcgttaagtgcggggttatctgccagcagttgagcagtgccgagaataccgtacagcggtgtgcggatctcatggctcatcgccgccagaaacgccgattttgcctggctggctttttctgcttccgcccgtgcctgtcggtgttctatcaccagttcctgcaattcagctgtacgcgctttgacctgcgccgccagctgttcgcggtggcgattcagtgcatgaacattgctgcgaaacgcatccatcagccgcccgatggtatccagctcccgtacgccagcggtttccgggaaaggggagtcaatatcaccgtccagcagccgttgcagcgcctgcgtttgttcggcaagtggacgcgtgactgagcgataaaccacgcgccagaggatcagaatcagtgcgcaaagtgaaaccatccccagcaataacaggctgtattgcccgcgtgcactcgctttttccagatgcgccagtccgtgctgattacgcagctcaatggtgtcgaccagctgactgacttcgctactaaactgcgcgaactgggcgatgttattttgtgcgagagtttgtaggtgattgctgatttcactgtcctgctgatacagcgccagcaaatcgctatattggctaacggtagttaacgttgttgcgacctgcgcacgaacacccggatcttcaatgcgtatttgccgacgttgcagaattttcaccgcattattgagctgcttttccagcgttggtgcatttttctggatctgctccagccccagattcatcaccatttgctgcacccgcagagcgctaaggcgcagttcattcatctggttaacatactcaagatcgatatcaatcagccgatcgagtgcactttcagcagcctgacgctgatcttgttcgatcaaatcgtaaatcccggcctgggtcgctccagcggaagttgtcgcattattcgcctgaccttgcgccaggcgtgcgatctcatcggcggcagcgactatctgctgactgagttgctgttgttgctggcgcagttgcaaacgctgccccaccagttccccttgctgacgtaacgaacgggagatctcctgctcctgttgttcaatagcggtggtatcaaaaccttgttcccgtaacgcttgcagcaacgcattaatcttcaggctttgtgcggtgagcattcgcccctgcgcctgccacatcttttcgttatcggcactggtcaggttctgcgcggcgaaaagttcccaggcgctggcttcgctcaactggcgcgccatattcatggtaggaatcaatgcctgagtgttgtctttttccacctggctgataaagcgcaggttgtaccatcccaccagggtactggtcagggttaacagcgccatcagggcaaagcccatccagagtcttcgggtcagggttaaattcacggtcggtgcactttaggtgaaaaaggttgagtcgcaaagcggaatgcatctagcataaagccttattattgatgaggctatcatgcgcgtactgctatttttacttctttcccttttcatgttgccggcattttcggctgataacctgttgcgctggcatgatgcgcagcatttcacggtgcaagcctctacgccgcttaaagccaaacgcgcatggaaactgtgcgcgctttatcccagcctgaaagattcatattggttatcgttgaactatggtatgcaggaggctgctcgccgctacggtgtggatttaaaagtgctggaggcaggcggctacagccagttggctacccagcaagcacaaatcgaccagtgtaaacagtggggcgcagaggccattttgctcggtagtagcacgacctcatttcccgacctgcaaaagcaggtagcaagtctgccggtgatcgaactggtaaatgctattgatgctccccaggtgaaaagccgcgttggtgtgccctggtttcagatgggctatcaaccggggcgatatctggtgcaatgggcgcacggtaaaccactgaatgtgctgttgatgcccggacccgataacgccgggggcagtaaggagatggtcgagggttttcgcgcagccattgccggaagcccggtgcgtattgttgatattgcgcttggtgataacgatattgaaatccagcgtaacctgttgcaggagatgctggaacgccatccagaaatcgacgtcgttgccggaacggccattgcggcagaggcggcaatgggggaagggcgtaacctgaaaacgccgcttaccgtggtgtcgttttatctttcacatcaggtgtatcgcgggctgaagcggggaagagtgattatggctgccagcgatcaaatggtctggcagggggaactggcggttgagcaggccatcaggcaattacaggggcaatcggtttctgataatgtcagcccaccgattttagttctgacgccgaaaaatgccgaccgtgaacatattcgccgctcgctgtcaccagggggatttcgtccggtctatttttatcagcacacatcagcggctaagaaataaccttcaccatgttgcgtcaccagtaaatccgcgctgagtttatgacgtaaacgacgaattaacacatcgacggtgcgcaggtcagggttttccacccgacgcgcagaaagcatacgtagcagacgttcacggctgagaatttcgcccggattcgtcacaaatgccaccaacatttcatactctgcgcgggtcagtttaatcggctcgccatcccgctccagcgtatggcgcgacacattcaggcaataaccggcaaagcgatagcagttgtcctgagtgtgcggttgagcttgtcgcgcgaggtcgattcgccagagcagatttttcacccgtactaccagttcgcgcagttccagcggtttggtgacgtaatcgtctgcgcccatttccagcccaacaatacggtcaatccgatcgctgcgtccggtaaccagaataatccccaccgttgagcgttctcgcagggcgcgggttaacatcaggccattttcatcgggtaagttgatatccagcagaattaaatctaccgactgattctgcataatttcccgtagcccagcaccgctcgccgtaacggaaacggtatacccctcctgagtgaagtaggattgtaatcgcgcctgggtaaccggctcatcttcaacaataacaatgtgatgtggcatcagagggttttactcattctgttcatatctgttcatattctgccgtaagccgttcatcctgaccagtgccgctgttcatatttgctcattaagatcgcttcactaaaccataattctacaggggttattatgcggaaactctggaacgcgctacgccgacccagtgctcgttggtcggtactggcgctggtcgcaattgggattgtgattggcattgcgctgattgtattgccacacgttgggatcaaagtcaccagcacaaccgaattttgtgtcagttgccacagtatgcaaccggtgtatgaagaatataaacagtcggtgcatttccagaacgcctccggcgtgcgagctgaatgccatgactgtcatatcccgccggatattccaggcatggtgaagcgcaaactggaagcgagcaatgatatctaccagacctttattgctcactccattgatacacctgaaaaattcgaagccaaacgcgcggaacttgccgagcgtgaatgggcgcgaatgaaagaaaacaactcggcaacctgccgctcctgccataactacgatgcgatggatcatgcgaagcagcatcctgaagcagcacgtcagatgaaggtggcagcgaaagataatcaatcctgcatcgactgtcataaaggtattgcccaccagttaccggatatgagtagcggcttccgtaagcagttcgatgagctgcgcgccagtgctaatgacagtggtgacacgctgtactctattgatattaagccaatttatgcggcgaaaggcgataaagaagcctctggttctctgctgcctgcttcggaagtgaaagtccttaaacgtgacggcgactggctgcaaattgaaattaccggctggacggaaagcgccggacgtcagcgtgtactcacccaattcccaggtaaacgcatctttgttgcctcgattcgtggtgatgtgcagcagcaggtaaaaacgctggagaaaaccaccgttgccgacaccaataccgagtggagcaagttgcaggccactgcgtggatgaagaaaggcgacatggtgaacgatatcaaaccgatctgggcttatgcggattcgttgtacaacggcacctgtaaccagtgccacggcgcaccggaaatcgcccactttgacgctaacggttggatcggcacgctcaacggcatgattggctttaccagtctcgataaacgtgaagaacgcaccttgttgaaatatctgcaaatgaatgcgtctgacaccgcaggtaaggctcacggcgataagaaggaagaaaaataatgaacaataacgatctctttcaggcatcacgtcggcgttttctggcacaactcggcggcttaaccgtcgccgggatgctggggccgtcattgttaacgccgcgacgtgcgactgcggcgcaagcggcgactgacgctgtcatctcgaaagagggcattcttaccgggtcgcactggggggctatccgcgcgacggtgaaggatggtcgctttgtggcggcaaaaccgttcgaactggataaatatccgtcgaaaatgattgccggattgccggatcacgtacacaacgcggcgcgtattcgttatccgatggtacgcgtggactggctgcgtaagcgccatctcagcgatacctcccagcgcggtgataaccgttttgtgcgcgtgagctgggatgaagccctcgacatgttctatgaagaactggaacgcgtgcagaaaactcacgggccgagtgccttgctgaccgccagtggttggcaatcgacggggatgttccataacgcttcggggatgctggcgaaagctattgccttgcatggtaatagcgttggtacgggcggagattactctaccggtgctgcgcaggtgatcctgccgcgcgtagtcggttcgatggaagtgtatgaacagcaaacctcctggccgctggtattgcagaacagcaaaaccattgtgctgtggggctccgatttgctgaaaaaccagcaagcgaactggtggtgcccggatcacgatgtttatgaatattacgcgcagctaaaagcgaaagtcgccgccggtgaaattgaggtcatcagcatcgatccggttgtcacatccacccatgagtatctggggcgcgagcatgtgaagcacattgcggttaacccgcaaactgacgtgccgctgcaactggcgctggcacatacgctgtacagtgaaaacctgtacgacaaaaacttccttgctaactactgtgtgggttttgagcagttcctgccgtatctgctgggtgagaaagacggtcagccgaaagatgccgcatgggctgaaaaactgaccggcattgatgccgaaaccattcgtgggctggcgcggcagatggcggcgaacagaacgcaaattattgctggctggtgcgtgcagcgtatgcagcacggtgaacagtgggcgtggatgattgtggttctggcggcgatgctggggcaaattggcctgccaggtggtggttttggttttggctggcactacaacggcgcaggcacgccggggcgtaaaggcgttattctgagtggtttctccggctctacgtcgattccgcctgttcacgacaacagtgactacaaaggctacagcagcactattccgattgcccgttttatcgatgcgatcctcgaaccggggaaagtgatcaactggaacggtaaatcggtaaaactgccgccgctgaaaatgtgtatttttgccggaactaacccattccatcgccatcagcagatcaaccgcattattgaaggcttgcgcaagctggaaacggttatcgccatagataaccagtggacctcaacctgccgctttgccgatatcgtactgcctgcgaccacgcagtttgagcgtaacgatctcgaccagtacggcaatcactccaaccgtggcattatcgccatgaaacaggtggtgccgccgcagttcgaggcgcgcaacgacttcgatattttccgcgagctgtgccgtcgctttaatcgcgaagaagcctttaccgaagggctggacgaaatgggctggctgaaacgcatctggcaggaaggtgtacagcaaggcaaaggacgcggcgttcatctgccagcgtttgatgacttctggaataacaaagagtacgtcgagtttgaccatccgcagatgtttgttcgccaccaggcattccgcgaagatccggatctcgaaccgctgggcacgccgagtggcctgattgagatctactcgaaaactatcgccgatatgaactacgacgattgtcaggggcatccgatgtggtttgagaaaatcgaacgctcccacggtgggcctggctcgcaaaagtatccgttgcatctgcaatctgtgcatccggatttccgacttcactcgcagttatgtgagtcggaaacgctgcgtcagcaatatacggtagcgggtaaagagccagtattcattaacccgcaggatgccagcgcgcgcggtattcgtaacggtgatgtggtacgcgtctttaacgctcgcggtcaggtgttggcaggggcagtggtttctgaccgctatgcacccggcgtggcacgaattcacgaaggggcatggtacgatccagataaaggcggcgagcctggtgcgctgtgcaaatacggtaaccccaacgtgttgaccatcgacatcggtacatcgcagctggcgcaggcgaccagtgcgcacactacgctggtggaaattgagaagtacaacggaacagtggagcaggtgacggcgtttaacggccccgtggagatggtggcgcagtgcgaatatgttcccgcgtcgcaggtgaaatcatgaccacgctgacagcacaacagattgcctgtgtttacgcctggctagcgcagttgttctcccgtgagctggacgatgaacaactgacgcaaatcgccagtgcgcagatggctgaatggttttcgttgctgaaaagcgaaccgccgctcactgcggcggtgaacgagctggaaaaccgtattgccacgctgacagtacgtgacgatgcccgtctggaactggccgcggacttttgcggcctgtttctgatgaccgacaaacaagcggcgctgccgtatgcatcggcctacaaacaggacgagcaagagattaaacgcttgttagttgaggcagggatggaaaccagcggcaatttcaacgaaccggcagatcatctggcgatctatctcgaattgctcagccatctgcatttttcgctgggagaggggaccgttcctgcgcgaagaatcgacagtttgcggcaaaaaacactgacggcgctgtggcaatggttaccagagtttgttgcgcgttgtcgtcagtatgacagctttggtttttacgcggcactaagccagttattgctggtgttagtggagtgcgaccaccaaaacagataacgtcgtttgtgcgcctgaaaagacgcgtttagcgtcgcatcaggcattatggcgcagttgccggatgcggcgtgaacgtcttatccggcccacaggaactgtaatctttgtagaccggttaagatgcgtcatcgcatccggcaaacacacatcacggatgagctacaaaccgggaaagccgctggcgcagcaggcggttttcctgcttcaggtgcgcaatatcatccattaacgtcagcgccaccgcgatccccggccagtccagagccagttcatgacgcaggcgtaccgcgcgttgcaccacaatggcggcatggtcgtcaaatacccaggttgtttcctggatctcacgcggttcaaccacccccaaaccgacaatttcattcaactcctcttcagagatgccggtatgcaggcaaaattcggtaatagtaaaagtcaccgtaacattagccattatgctttcccccaatctttacgtggatcaaaagacgactgggcgtctgccagttgctgccacagcgcggcagtgttttcatccggtttcggcggcatcacgattttcagtaccgcatacagatcgccggtctgttttttgctcaccagacctttgcctttaacgcgcaatcgttgcccggcctggctgcctggcgggatagtcagcaaaatgctttctttcagtgttggaacggtgactttagcacccagcgccgcttcccacgggctaaccggcaccacaatttccagatcctggccgacaatatcaaacagcggatgtggcgcaatatgaatcaccagccacaaatcgccatttggaccgccgttttcgcccggcgtcccctggcctttcagacggatgcgttgaccattgccgacgcccgccgggatcttcacattcagcgttttcggaatttcctgttcgatcatgccaaaggcgttataaaccggcaggttatagctgatggtacgcttatgctcagtaagcgtttcttcgaggaataccgccacttcgatttcaatatcgtggccgcgtgtggcggggcgttgacggctctggcgggcatgctgaccgaaaattgacgagaagatatcgtcaaaatcttcggcgttaaaactctgaccgtcgccatggtggaactgacggttaaattgcggatcgttgcgatgttgccacatctgatcatactcagcgcgacgttgttcatcacttaacacttcccaggcttcagcgacctctttgaagcgggcttcggcatccggttctttgctgacatcaggatggtatttgcgggcaagtcgacgataggcggtcttgattgtcttgagatcgtccgtcggtttcacgcccatgatggcgtaataatcctttaattccatagcgttatctcgcgtaaatcaacacaaattgaaggaacccctgtaaggtaactcctataagtgtagggtaatcctcaaaatttcatatgccaacacagaatatgttattgaaatcatcgcggagaggaggtcgccatcaagatgggttgctgaacatattttaaacaggtgaaaaagggtgagcgatttttgatagttgaaccaggcactttaagtttaactagggcgtcattatttattaaattttatagacgctatatatgggtagtaatatacatggaattagttgcactgcaaataattatttgaaacaggcctggaacgatataaaaaatgagtacgaaaaaaatcaaacatattcaatcacgctttttgaaaacacactggtgtgttttatgcggttatacaatgaactcagacgtaaagtaaatgaagaggatactccatgtctggaatgtgaatcactagaaaaagaatttgaggaaatgcagaatgataatgatctatcattatttatgagaatattgcgtactaatgatacacaaatttattcaggggtttcaggaggtattacatatactatacaatatgttcgagatattgatattgttagagtgtccttgccgggcagagcttcagagtctatcacagattttaaaggttattattggtataactttatggagtatattgaaaacattaatgcgtgtgatgatgttttttctgagtattgttttgatgatgaaaatataagtgtccagccagagcggataaatacgccgggaatatctgatttggattctgacattgatttgtctggtatatcttttattcagcgtgaaactaaccaggcattaggattaaaatatgctcctgtagatggcgatggatattgtctgttaagagctatactggttttaaaacaacatgattattcatgggcgctggtcagttataagatgcaaaaggaagtttacaacgaattcattaaaatggttgataaaaaaacgatcgaggctcttgttgatacggcattctataatctcagggaagatgtaaagacgttatttggcgttgatctacaatctgacaaccaaattcaggggcagagtagtcttatgtcatggagctttctgttttttaaaaaacaattcattgatagttgcttgaataacgaaaaatgtatcctgcatttacccgagtttatatttaatgataacaagaacttgcttgctttagataccgacacgtcggataggattaaagcggtgaagaattttcttgttgttctttcagatagcatttgctcattatttattgttaatagtaatgtggcatcaatctccttggggaatgaatccttttcaacagatgaagatcttgagtatggttatttaatgaacactggcaatcattatgacgtttacctccctcctgaactttttgctcaggcttacaagttaaacaataaggaaatgaatgcgcaactcgactatttaaatcgttatgcaatttaatggcaaaggcatatgctaaaaaccattgttattagtctcacacttttttattggtaaatattgtctctgtattggtaacgccgcagatattctgtttagccacaggtgcaattatcagcggcgtacgcgaggcaggggctaatcaggcatagtttgcgtcaaaccttgcctgtttttgaagatgtatatagaaaaacaggcgttcaacaagccattttgcgaacctgttcccggaaaaaagtcatatttctgtcacactctttagtgattgataacaaaagaggtgccaggaatgaacaaaacgctaatcgccgcagctgtggcagggatagttttactcgcttcaaacgctcaggcacaaaccgtaccggaaggctatcagctacagcaagtgctcatgatgagccgccataacttacgtgcgccgctggcgaacaatggcagtgtgctggagcagtcgacgccgaataaatggccagaatgggacgtccccggtgggcaactcaccaccaaaggtggcgtgctcgaagtgtatatgggccattacatgcgtgaatggctggcagagcaggggatggtgaaatcgggggaatgcccgccgccgtacaccgtttatgcctatgccaatagtctgcaacgtaccgttgcgaccgcacagttctttattaccggcgcattcccggggtgtgatattcctgtgcatcaccaggaaaaaatgggcactatggacccaacctttaacccggtgatcaccgatgattccgccgcattcagtgaacaggcggtggcggcaatggagaaagagctcagcaaactccagcttaccgacagctaccagctactggaaaaaatcgttaactataaagattcccctgcctgtaaagagaaacaacagtgttcgctggtggatggcaaaaatacctttagcgccaagtatcaacaagaaccaggtgtttccgggccgctgaaagtcggcaactcgctggtagatgcgtttactttgcaatattacgaaggttttccgatggatcaggtggcctggggagaaatcaaatctgaccagcagtggaaggtgttgtcgaagcttaaaaacggctaccaggacagcctgtttacctcaccggaagtggcgcgcaatgttgcgaaaccgctggtcagttatatcgacaaagctctggtcaccgatcgcaccagcgcaccgaaaattacagtgttggttgggcacgactccaacattgcctctctgttaacggcgctggatttcaaaccgtatcagttgcatgaccagaacgaacgcacgccgattggcggcaaaatcgttttccagcgttggcatgacagcaaagccaatcgcgatttgatgaaaattgaatatgtgtatcagagtgcggaacagttacgtaatgccgatgcgttaaccctgcaggcacctgcgcagcgtgtgacgctggaattaagcggttgcccgatagacgctgatggtttctgcccgatggataagtttgatagcgtgttgaatgaagcggtgaaataacagaaaactcccccgcgagaagcgggggagtcgctggttaaacgtttttacgttcgatggtctgttcgccccaaaaaagcgaatctttatcggtcttagcaaaggctttgactaacacttcatcactaccttcttcccaaatcttttccgccattttttcgtcgtacccggcgacttcgaaaatggcctcggctatttccggcgacgtattgcgcagagatgcccattcaccgacgtgatgagctttcgcttcttgagttggcatgcgtatcctcctgttgaagattagccgttaagtttaactgccagacctgcgacatattccccttgataacgagcaatagacagttcttcctggctgggctggcgtgaaccgtcaccgcctgcgatggtggttgcgccgtacggcgtaccgccgcgaacctgtgaaacgtcaaataattcctgcgctgcgtagccaatagggacaattaccatgccgtgatgcgcaagggtcgtccaggtggatgtgatggtttgttcctgaccgccgccagtaccggtggaactaaagacgctcgccagttttccgtatagtgcgccggaagcccacaggccgcccgtctggtcgaggaaggtacgcatttgaccggacatgttgccaaagcgggtaggtgtaccaaaaataatggcgtcgtaatcggccagttcttgcggggttgcaaccggtgcagtttgcgttttaccgcctgctttttcaaataattgcggcggcatggtttccggtacacgcttaacgacaacttcagcgccatccactttgcttgcaccctcagcgactgcgcgtgccatcgtttcaatatgtccgtacatggaataataaagcaccagaactttagccatttctaaccactcctcgtgttatctctattccgtagcgattcgctaccacttatttaaagataagacgtccttttcagagtgcaaatttcacaaccacttatttgatttataacaactttcacaagcacgtaattttgtcgcaaaatgacacatttttatctcatcgcgtttttttaatcataagagcggcttatggataattattggagatgatatctattctcgctaagaagctgttgcaggatattaccaaacgcgggtctgcccgcgtcagttcactaagcttagtcccacgtagcgaaaatatggcagccgccatacgccgcgttaattctatgcaatatgatgtctatacccagacggaggtcagtaatggcaaaccatcgaggcggttccggcaattttgcagaagaccgcgaaagagcatcagaagcaggtaaaaaaggtggacagcacagcgggggtaatttcaagaatgacccgcagcgcgcatctgaagcaggtaaaaaaggtggtaagagcagtcacggcaaaagcgacaactagccgggctaatcaatgacgaatgcatttttgtctgtagctcgtcaaaaagccatcaccgccggttacccggtggttgatactgatgacaaatgtaagcttgcctgatgcgcgatgcttatcaggcctaccagaagattgcaatatattgaatttgcactgttttgtaggccggataaggcgtttacgccgcatccggcatgaacaatgcgtacgttgtcaacaatctgcaccgccggtaaccccggcggttttctgtttatggctcctgatgaacaacttctggcggtggaacgtcaaccaactttctgcttaacaacgcattgagtaaaatcgcgccaaaggttgctgtaccaatccctcccaacgtaaaaccgcccagcgtgagagcaaaatcacccgcgcccagcactaaggttactgcgaccataatcaaattaccgttctggcttaaatcgacacggttttgtacccatatccttgcgcctgcgacggcaatcagcccgaacacaacaattgatgcaccaccaataaccgcggccggaatggtatgaatcagcgcaccaaatttcggtgaaaagcccaacagcatggcgatgacggcagcagcaacaaacaccagcgtcgagtagactttggtcacggccatcacaccgatattttcagcataggtggtcacgccgctaccgccgacagagccggaaagcatcgttgccagaccatcgcctacgaatgcccgccccatatacgggtccatattgcgtccggtcatcccggcgactgccttgagatgacctaagttttccgccaccagaatcaccgccacgggcgcaatcagcatcattgcctgaccattaaaagcaggagtggaaaaatgtggcagaccgaaccaggcagcatggctgacgagagtaaaatcgacggcttttcccagccctaaaacgttggtcatcacgccatacagcagacaggcgacaattaatcctacgagaatcaataaccgctggatcatgccacgggtaaacaccgccaccagcccaatacacagcaccgtcattaccgccatccagctatcaaaggccgaagccgatacacttttcactgcgataggcgctaagttcaggccaatcgccatcaccaccgcacccgtcaccaccggcggcatcagtcgttcaatccagcgcgtaccgattttcatcaccaccaggccaatgacggtataaaccagcccacaggcgataatcccgcccagcgcaatgctgatattcgggttaatgccctgaccgttaaagcccgtcgcggcgatcaccacgccgacaaaagccgcgctggagccgagataactggggacgcgcccgccggtaataaagaaaaacagtaacgtgccgatccccgacattaaaatggaaagattgggatccagccccatcagaatcggcattaacaccgtcgcgccaaacatcgccaccgcgtgttgaacgcccattactgccgtctgagcaaacggcaatcgttcatccggcgcgaccacgccgctctctgtagaggtcgattttaactgccagtgaggaaaaccgaacattgccatcagctgtctccttaaggaggttaacaagcagggcgcatcagcgcgtgataactgcgatcgaaccacaccagcccgtagggtgtggtgtgacgatgaatcgcttcgatggcgcaaaacagaatgtcgtgggtgccgacgctcaccacctggctgatacggcagtcaaacgaaaccagagcctcttccagttgcgggcatccggtcacccccgtctgccagcgggcggcggcaaagcggtgttccatgggcgttttgccgccaaaaaggtttgaaagcggctcctgcccggcgctaagtgtatttacacacagcgttcgattttcattgaatgccggccagacggacgccccacgattcaggcacaccagtaatgtgggcggcgtatcggtcacactgcagacggcgctggcggtgaacccggcgcgcccggctggaccgtccgtggtgataatattgaccgccgcgcccatgcaggacatcgcatcgcgaaaagtttgttgatcgacaatgttcatagtttgctccttacaacagcccgcaggcttcttcaaaggacagacgtggcaggcgcgcataaagcttgctgctatcgccatagccgatattaatcagcagattgctcttcagcgtgctgcccgtaaaaaaggcgtcgtccacgtgttgacggtcaaagcccgacatcgggccggtatccagtcccagcgcccggcaggcgacgatcagataggccgcctgcatggaactgttgcgaaacgctgtttcttcggcaagttgtgggctggaggtaaaccaactgcgggcatcaccgtggggaaacagtagtggtaaccgttcataaaattcactgtcccaggcgacgatagcggtgacgggcgcggtcagggttttttgcagattgccgctggaaagtgccgggcgcagacgttcttttccttctgccgtgcgggtaaacacgatccgtgccggagaacagttagctgatgtcggcccccatttcatcagggcataaatctcccgtaacgtctcatcgctgacgggtgtctcccgccagccgttgtgagtgcgggcatcggtgaacagggtgctaagcgcacctgggctaacggcttcgttcatagcaattccttacagggcggcttcacggtgatgtaacaggctggcaagcccgttgagtaacagagcattaaacgtttcgggatcggtcacgttgcaggcgtgtccgccatagggcatcaccattttctggctatcgggcagggcggcatgaagttcactggaacatgctgttggcaccagcagatcatcactggcgcagatgatttgcaccgggcagcggatgcgatccgcatggtgactaaagtcagcgcgtttgagggcgttaagtcgacgcagtaaattatttttgccctgaaaatgcgccagtgccagcgcgtcttctgcctccaggcgaggtgcgcgggccgccatccagtcggcgggatagaggaacaacggctgcgcttccacccatgcctgcgcgccgccgctatacagtaatcgttcgcgaacctgaaaacagcggcgcgtatgggcgtttattcgtagccagccgttaacgctgatcagcacagttaccgacgcgggataatccagcgccagctgcattcccaccagcgcaccgagcgcatggccgaccactgcgtaatgctcaatccctgcggctaccagcgcctgatgcagttccgctgccatctgggcgatactgtaatcttctgccagcgtgtcgggattattgccggtgccgcgctggtcgtaacagactacctgatactcctgctccagcaccgccagttgcggtaaccagtaactgccgctacccccaagacccgaaatcaacaccactacgggcgcatcagcataagggggaggtgagagtgaaagtttcatcgcggcctcacttggcgatatgcgcaattgtggcgatttccaccagcgcgtcaggttttaccagtccgcactgaatgcagaatcgcgccggtttatcacccggaaaaaactcggcgtagatttcgttaatcgcggcgtaatttttccagtcggtaataaagatgctgttgaaggtcacatccgccatcgtgccacccgccgtctcgatcaccttgcggatagtttccagaacgtggcgggtttgcgcctttgggtcatcggcaaacagcacgttattatgttgatcaaaagccagcgtaccggagacatacaccacgccatcagccagcgtgccgggaacgaagggggccagcggtgcgctgctgccagcgggaataattacggattttggcatcgttaaactccttaagcgatatgagcaaaggacgtgggagaaagcgcgtcgcagaatgtttcgacgtcgctgacccagccaaaaaaggtttcgatattgaacaacgcggctttctgcgcaaatttcggccccgcctggtgagttgcgtcttcaagcaccacgccgaaatactccagaaaaaagccgtcgcgtagcgtcgattcgacgcagacgttggtagcgatgccggtgaaaaccagatggcgtattccgcggctgcgcaaaatgctgtccagcggcgtattgaagaaaccgctgtagcgcggcttcggcagcacaatatcgccaggctgcggcaccagttcatccaccagttgataatcccaggagcctttcgccagcaatttcccctgcagctgcggctgcttacgcatggttttcagggcgttcgatttatgaaaattcggtgagccgggtccgccagcctcgacatactgttcatcccagccattttgaaaccagatgatcagcatccctgccgctcgcgctgcggtcacggcggtttgaatgttggcaatgaccgggcgagtggttgagacatcaaacccggcgagatctaagtagccgcctggcgtggcataagcgttttgcatatccaccacgatcagcgcactttgctgcggatcgaaggtaatggcttccggtcgagcggttaaggtcgtcatcatgccacctcctgagtcagcgcaggtagatgggcgcggcattgcatcagtggttgaatgcgctcgccgaaggtttcgattcccgacagaaaatcgtcgaaggttaacagcacgccttcggcaccaggcacgcttgcgacttcatctaacatgcgcgcgacactggcgtaagaaccgactaacgtccccatattgatgtttaccgccgaagtgggatcggccatctgacgaacgttggtgtcagtaccggagcgggtatctttctgactttgttcggttagccagcttaacgcctcttcatccgcgcccgctttgtagtgttcccatttggcgcgagcggcatcgtcggtttcatcggcaatcaccataaacaacacataagagccaacgtcgcgtccggtttgctctgcggcctgtttcatccgcgcagcggtcggggcgaaagccgtgggtgtatttacgcctttgccgaaacagaagttgaaatcggcataccgggcggagaacgccatgccagcgtcgctttgcccggcgcagatcactttcatggggacactcggttgcggactcacgcgacaatcattcatggtgaaaaaatcgcctttaaaatcgcttttccccgtgccccacaggtcgcgcagcacctgaacatattcggtgagatagtcgtaacgacgggagaaatagtcatcgccaggccagatacccatctgctcatactcgggcttttgccagccagtcacgaggttgacgccaaaacgcccgccagagatggagtcgatggttgcggccatacgggcgacgattgccggaggtaacgttaaggtggcagcagtggcgtaaatctgaatgcgcgaggtcacggccgccagccccgccatcaaggtgaacgactcaaggttgtgatcccagaactcagttttgccgccaaagccacgcagtttgatcatcgacagggcgaaatcgaaatggtagtgctccgctttttgcacaatggctttattcagttcaaaggtcggcatgtactgcggcgcgtgggtcgaaatgagccagccgttgttgccaataggtacgaatacgccaattttcatcatcaacctctcttcgtctcgtaaagtgaaagtcagacggggcgctgcatcctgcatatccttttcagccgcgtattggcttgtttgcaaagcggatgccagtttttaaaaagttaatgttattaatctgttaacattacgttatctaaaatatctggtaaaaagtggactaaacggtcaaaacagttgcacataaaacatgcatctgtgcgcgatgagagtgcagaaggtcgaggccgggcgggggttttgctatcctgttgccaatctacaagaggggagagcgcatgacgcaaggcgcagtgaaaacaacgggtaaacgttcgcgcgcagtaagcgcgaagaaaaaagcgattcttagcgcagcactggacactttttcacaattcggttttcacggcacaaggctggagcagatcgcagagttggcgggtgtttcaaaaaccaatctgctgtattactttccgtcaaaagaggcgctgtatattgccgtgctgcggcagattctcgatatctggctggcaccgttaaaagcgtttcgtgaagatttcgccccgctggcggcgatcaaagagtacatccgtctgaagctggaagtctcacgcgattatccgcaggcttcgcgcctgttctgtatggagatgctggcaggcgcgccgctgttaatggatgaactgacgggcgatttgaaggcattaattgatgagaaatcggcgctgattgccggttgggtcaaaagcggcaaactcgcgccgattgatccgcagcatttgatttttatgatttgggcttccactcaacattacgccgatttcgcccctcaggtggaggcggtgacaggcgcgacgttgcgcgatgaggtatttttcaatcaaacggttgaaaacgtgcagcggattattattgaggggattcgaccacgttaaagatgccggaggaggttgtaacatcctccggctacctgtttaacctatagtcattaagctggcgttaccgccagcggcagcggtattcacactcagcgaacgctcgatatacagccgttccagaaggatattgctttcgccacgggcaaaaccctgcaccgaaacaattgtgccatcccgcgcggcaactgcttcacacaatgcgcgaagctgatccgaatcaccgtggaagatcaccgcatcaaacggttgagcggttatattttccgctttcgccagttgaatacgttcgctgactgccgatggcaatgccttcactaactgacgatgcagcgcgtcatccggccacagtacctggctgcccaccgccagcacggcggcgagctgagtcagcgcatcctgctcatcatcggcaatacacaacacgcgctcacgcggcagcagcgtccaggtgttgcgttcacccgtcggccccggcagcaatcgttgtgttcctgcctgcgccagctcgccatattgcgtacataacgcctgcaattctggacgatttgctgcccattcccgcagtgcatttagcggctgagtcaatgcggctttcaactgcgcatcgaccggatactttgcatcctgacgcgcgagcgtcactgccagcgcactttccgggcgattcgccagcagacggtagagatagagcggaccgcctgctttcggcccggtaccggacaacccttcgccgccgaacggctgcacaccaaccactgcgcccaccatattacggttaacatacaggttaccaacatgggccgagccagtgacctgggcgatggtttcatcaatgcgcgtatggacgccaagcgtcagaccataaccggaagcgttaatctgctcgatcagctctggtagctggttacggttgtaacgcaccacatgcagcaccggaccaaagacctctttttgcaattcggcaaagtcatccagttcgatcagcgtcggggcgacaaaggtgccgctttgccattcacgggcatcttcgctgttttcccgcaccgcctggaacaccggacggcctttgctacgcatggtctgaatatggcgctcaatattggctttcgcttcgctatcaatcactggaccgatatcggtggtcaggcgacccggattacccatccggcattcggccattgcgccgcgcagcattttcaacgtgtggtcggcaatctcatcttgcaggcacagcacgcgcagcgccgaacaacgctgacccgcactgtcgaacgccgaggccagtacatccacgacgacctgttcggtcagtgctgaagaatcgacaatcatcgcgttcatgccgccggtttcagcgatgagcggaatagggcgaccctgagcgtccaggcggctggcgatattgcgctgcagtaacgtagcgacttcggttgaaccggtaaacatcaccccgcgcacgcgatcatcacccgtcagttgcgcgcccacggtttcaccccgacctggcagcaattgcaccacgcctggcggtacacccgcttccagcaaaatggcgatcccttgcgcggcaatcagcggcgtttgttctgccggttttgccagcacgctgttacctgccgccagtgcggcggcgatctgcccggtgaaaatagccagcgggaagttccacggactgatacacaccacaggccctaatggacggtgggtttcgttagcgaaatcatcccgcacctgtccggcgtagtagtggagaaaatcgaccgcttcgcgcacttcggcaatggcgttactgaaggtttttccggcctcacgcaccagaataccaatcagttgctgcatctggctttccatcagcacggcagcgcggtgcaaaatcgctgcgcgttcagccggaggcgtggcaaaccagattggcgcgttattaaccgcactttccagcgcctgttctacttcacgcggcgtggcttcacgcacatagcccacaatatctttcggttccgcagggttaataacgggcgacatctcacctgccgctaccggttgttccagcattggcaaggcctgccatttttgcagtgcactattgagcagggcagaggagagcgaggccaggcggtgttcgttagcgagatccagccctgccgagttgtcgcgcccgtgaccgtaaagatcgcgcggcaggggaattttcggatgcggtaatccagtttgcccttcctgttgcgccagtttttctacagcagtgaccggatcggcgaccagttcatccagtggcaaagaggtgtcggcaatacggttaacaaacgaggtgttagcaccgttttccagcaggcgacgcaccagatacgccaacagcgtttcatgtgtgccaaccggagcataaatacgacacggacggttaagtttgccgtcggcaactttcccggtgacctgctcatacagtggctcgcccataccatgcaggcactggaactcgtactgacccgggtagtagttctgccccgccagttgataaatcgccgccagcgtatgggcgttgtgcgtcgcgaactgcgggtagattagattcggcaccgccagcagctttttcgcacaggcgagataagaaacgtcggtatacaccttgcgggtataaaccggataaccttcaaggccgtccatctgcgcacgcttaatttcactatcccagtacgcgcctttcaccaggcgaatcatcagacggcgacggctgcgggtggcgagatcaatcaggtaatcgatcaccaacgggcagcgtttttgataagcctgaataacaaaaccgatgccgttccagcctgccagttccggctcgaaacagagtttttccagcagatcgagggagatctccaggcgatcggactcttcggcgtcaatgttgataccaatatcgtactgacgcgccagcagggtgagtgatttcagacgcgggtaaagctcttccattacccggtcatactgggcgcggctataacgcggatgcagcgccgacagtttgattgaaatgcccggcccttcatagatgccacgaccgttagacgctttaccgatggcgtgaatcgcctgctgataggaaaccatatacgcctgtgcatctgcggcggtcagcgcggcttcgcccagcatatcgtaagagtaacggaaacctttctcttccagcttgcgggcattggctaacgcttccgcgatggtttcgccagtgacgaactgctcacccatcaggcgcatcgccatatccacacctttgcggatcagcggttcaccgcttttaccgataatgcggttcagcgagcgggagaggctggcttcgttatgggtggaaaccagtttgccagtaaacagcagcccccaggtggcggcattaacaaacagtgacgggctacgaccaatgtgtgactgccagttaccgttgctgattttgtcgcgaattaacgcgtcgcgggtggctttgtcgggaatacgcaacaacgcttccgccagacacatcagcgccacgccttcctgcgatgacagcgaaaactcctgcaataacccctggaccatacctgcgcgaccactggcatttttttgattacgcagtttatcggccagctgatacgccagtttgtgcgcctgttcagcaactggctgcggcaggcgggcttgttccagcagcatagaaaccgcttcggtttccgggcggcgataggccgcggtgatcgcggcgcgggaaaccgactggggcaatatttgctcggcaaagtcgaggaatggctggtgtggttcctctgccggagtcggtgcttcatcgctctcattggccgcgccagaaagcagcgcaggtagctccggcagagtatcgctgttttccagttgttcgagataagaaaaaatcgcctgcttaattaaccagtgtggtgtgcgatcgatacgtgtcgcggcagacttaatacgctcacgcgtcgcgtcgtccagcttaacccccatggtggtggttcccatgccattactcctgttgttcagaaaggtgcaacttaacgttatcgtgaaatatccatgatgttgcaactttgtgcaaccatgttaaatgtgacatgcgtagcaagcttaaaaatgaatgaaatgttaataaaagaaatcgatatgacagggattaaaaaaataactcagactttttctctgcggcagttaacatttttgaaaggtgcaaccgcaaaaaatgtgagagagtgcaacctgatgaaaaatagtgtcgctgagcactaaaatttaatgtaaatggtgtgttaaatcgattgtgaataaccagcgcttccggcaggatacggtcgccctggtaaaacataaactctgttaccccgttccggtggcagatataacggcaagtttcgacattgccgataataattttttggagactttagatggctattagcacaccgatgttggtgacattttgtgtctatatctttggcatgatattgattgggtttatcgcctggcgatcaacgaaaaactttgacgactatattctgggcggtcgtagtcttgggccattcgtgacggcattatcggcgggtgcgtcggatatgagcggctggctgttaatggggttgccgggcgctgtttttctttccgggatttccgaaagctggatcgccattggcctgacattaggcgcgtggattaactggaagctggtggccgggcggttgcgtgtgcataccgaatacaacaataacgccttaacactgccggattatttcaccgggcgctttgaagataaaagccgcattttgcgcattatctctgcgctggttattttgctgttcttcaccatttattgcgcttcgggcattgtggcaggcgcgcgtctgtttgaaagtacctttggcatgagctacgaaacggctctgtgggcgggcgctgcggcgacgatcctttacacctttattggcggtttcctcgcggtgagctggactgacactgtacaggccagcctgatgatttttgccctgatcctgacgccggttatcgtcattatcagtgtcggtggctttggtgactcgctggaagtgatcaaacaaaagagcatcgaaaacgttgatatgctcaaaggtctgaactttgttgccattatctcactgatgggttgggggctgggttacttcgggcagccgcacattctggcgcgttttatggcggcggattctcaccacagcattgtccatgcgcgtcgtattagtatgacctggatgatcctctgcctggcaggggcggtggctgtcggcttctttgggattgcttactttaacgatcatccggcgttggctggtgcggtaaatcagaacgccgagcgtgtgtttatcgaactggcgcaaattctgtttaacccgtggattgccgggattctgctgtcggcaattctggcggcggtaatgtcaaccttaagttgccagctgctggtgtgctccagtgcgattaccgaagatttgtacaaagcgtttctgcgtaaacatgccagccagaaagagctggtgtgggtagggcgtgtgatggtgctggtggtggcgctggtggcgattgcgctggcggcaaacccggaaaaccgcgtgctgggcttagtgagctacgcgtgggcaggctttggcgcggcgtttggtccagtggtgctgttctcggtgatgtggtcacgcatgacgcgtaacggtgcgctggcggggatgatcatcggtgcgctgacggttatcgtctggaaacagttcggctggctgggactgtacgaaattattccgggctttatcttcggcagtattgggattgtagtgtttagtttgctgggtaaagcgccgtcagcggcgatgcaaaaacgctttgccgaggccgatgcgcactatcattcggctccgccgtcacggttgcaggaaagctaagggacttagcctgcggcggttttgtttggcttcagcagcgggttgcgctcccttaatgtgcctcgccatataaattgaatggtgcagggagcgcgcagggggcggccaatcgccgccgccccctgctgtcccggccttcggggaacgcttcagcgattttgacgccaccaacacccgagctgttattatgttccgggcaaaaagttagatttgataatcgcggatggacgaaattgcttgatacacccgcttatcagttttacatggaagctctgatgcattgagtctggacagttttgtcggctggatacggcgtttacgcggcatccggcaagaacacatggttctttgcaaacaatcccatctttctaccctggaataatcgtttatatcccttggcattacctctctttgtttacattccaacatcattttataaacattccgcttgtgtttttctttgccgtaatgataatcgctatcactgcgatttacttttctttgcatagattgactcagaaaaacgtttaagggtgggtggcatgtttgttccgtttctcattatgttgcgcgaaggacttgaagccgcgctgattgtcagtttgattgccagctatcttaagcgtacccagcgaggccgatggattgtgtgatgtggattggcgtgttgcttgccgctgcgttgtgcctgggcttgggtatcttcattaacgaaaccaccggcgaatttccgcaaaaagaacaggaactgtttgaaggtatcgtggcggtgatcgccgtggtgatccttacctggatggttttctggatgcgcaaagtgtcgcgcaacgtcaaagtgcaactggaacaggcagtcgatagcgcattgcagcgtggaaatcatcatggctgggcgctggtgatgatggtcttttttgccgttgcaagggaagggctggagtcggtctttttcctgctggcggcatttcaacaagatgtcgggatctggccgccgctgggtgcaatgctcggtcttgctactgccgtggtgctaggcttcctgctctactggggcggtattcgcctcaatcttggtgcattttttaaatggaccagcctgtttattctcttcgtcgccgcagggctggcagctggtgccattcgcgcatttcatgaagccggattgtggaaccactttcaggaaatcgccttcgatatgagtgcggtgctctcaactcactcgctgtttggcacgctgatggaagggatttttggctatcaggaagcgccgagcgtcagcgaagtcgccgtctggtttatttatctcatcccggcgctggtggcatttgctctgccaccacgcgcaggggcgacagcgtctcgctccgcgtaacaaatacgacgcaaactcttgcttagttacaacatactttaaagggatagtctcgtcatgaccattaacttccgccgtaacgcattgcagttgagcgtggctgcgctgttttcttctgcttttatggctaacgccgctgatgtgccgcaggtcaaagtgaccgtgacggataagcagtgcgaaccgatgaccattacggttaacgccgggaaaacacagttcattattcagaaccacagccagaaggcgctggagtgggagatcctcaaaggcgtgatggtggtggaagagcgggaaaatatcgcccctggctttagccagaaaatgacggcgaatttacagcctggcgaatacgatatgacctgcggtctgctgactaacccgaaagggaagttgatcgtcaaaggtgaggcaacggcggatgcggcgcaaagtgatgcgctgttaagtcttggtggtgcaattactgcatataaagcgtatgtcatggcggaaaccacgcagctggtgaccgacaccaaagcctttaccgacgcgattaaagcaggcgatatcgaaaaagcgaaagcactgtatgcaccgacgcgccagcactatgagcgtattgaaccgattgctgaactgttctccgatctggatggcagcattgacgcccgtgaagatgattacgagcaaaaagccgccgacccaaaattcactggtttccaccgtctggaaaaagcattgtttggcgacaacaccaccaaagggatggatcagtacgctgagcagctttataccgatgtggtcgatttgcaaaaacgcatcagtgaactggctttcccaccttcaaaagtggtcggcggcgcagccggactgattgaggaagtggcagccagcaaaattagcggtgaagaagatcgctacagccacaccgatctgtgggatttccaggctaacgttgaaggctcgcagaaaattgtcgatttgctgcgtccacaactgcaaaaagccaacccggaactgctggcaaaagtcgatgccaactttaaaaaggtcgataccattctggcgaaataccgtactaaagacggttttgaaacctacgacaaattgaccgatgccgaccggaatgcactgaaaggaccgattactgcgctggcggaagatctggcgcaacttcgcggtgtgctgggactggattaagcgttatgcagtataaagatgaaaacggcgtgaatgaaccgtcacgccgacgtttactgaaagtgataggtgcactggcgctggcgggaagttgtccggtcgctcatgcacaaaaaacgcaaagtgcgccgggtacgctttcaccggatgctcgcaatgagaaacagccgttttatggtgagcatcaggcagggatcctgacgccacaacaggccgcaatgatgctggtggcgtttgatgtgcttgccagcgataaagccgatcttgagcggttgtttcgcttgttgactcagcgttttgcttttctgactcagggcggagcagcaccagaaacgccaaatccgcgcctgccaccactcgattccggcattcttggcggctacattgcgcccgataatctcaccatcacgttatcggtgggtcactcattgtttgatgagcgctttggccttgcgccacagatgccaaaaaagctgcagaagatgacgcgtttccccaacgactcgctggatgcggcgttatgtcatggtgatgtgttgctacagatttgcgccaacacccaggacacggttatccatgcgctgcgcgatatcatcaaacacacgccggatttgctcagtgtgcgctggaagcgggaagggtttatttccgatcacgcggcgcgtagtaaaggcaaagagacgccgattaatttgctgggtttcaaagacggcactgccaatcccgatagccagaatgataagttgatgcaaaaagtggtgtgggtaacggcagatcagcaggagcctgcgtggacaatcggtggcagctatcaggcagtacgcttgattcagtttcgagtggaattttgggacagaacgccgctgaaagaacagcagacgatttttggccgtgataagcaaaccggtgcgccgctgggaatgcagcatgagcatgatgtgcctgattacgccagcgacccggaagggaaggtgatcgcgctggacagccatatccggctggcgaatccccgcacggcggagagtgagtccagcctgatgctgcgtcgtggctacagttattcactgggcgtcaccaactccgggcaactggatatggggttgctgtttgtctgctaccaacacgatctggaaaaaggcttcctgacagtacaaaaaaggctcaatggcgaagcgctggaggaatacgttaaacctatcggcggcggttatttttttgcgctgccgggggtgaaggacgcgaacgattatttcggaagcgcgttattgcgggtttaatgtttttaggcggataaggcatttgtgcgcagatgcctgatgcgacgcttgcgcgtcttatcatgcctacaatcagtgcgggtttggtaggctggataaggcgttcacgccgcatccggcgatcgtgcactgatgcctgatgcaaatcctgctgaaagcacacagcttttttcatcactgtcatcactctgtcatctttccagtagaaactaatgtcactgaaatggtgttttatagttaaatataagtaaatatattgttgcaataaatgcgagatctgttgtacttattaagtagcagcggaagttcccggcagtgatagtcagtcactatggagatcgcggatggtaacgtcctgtactggacatgttttagataatcaacgcgccaccactcgcggagttttctcctccggtagtcatctcgtcactttgcattttcaacctcatcctttcttttcatgtgttaccgacgccgtaaacggtgcgcgtagccgtttttcggcattttatccaaaagcaaactatggcttacaaggaagccaaccctctgatgttcgtgcgcataatcgcgctgccaacggcgcgtgtgatgaatacaaacaactcaaggtgctctccatgggaagacaaaaagcagtgatcaaagctcgtcgcgaggcaaaacgtgtgctgagacgggattcgcgcagccataagcagcgtgaagaagaatcggtcacctcgcttgtgcagatgggcggcgtagaagccattggtatggcccgcgacagtcgcgatacttcgcccatcctcgcgcgaaatgaagcgcaattgcactatctgaaggctattgagagtaagcagctgatattcgccacgggcgaagccgggtgcggaaaaacctggatcagcgcagcaaaagcggcagaggccctgatacataaggatgtcgacaggattatcgtcacccgtccagttctgcaagccgatgaagatcttggcttcttacctggagatatcgcagaaaagtttgctccctattttcgcccggtctacgacgtgctggtccggcgcttaggggcttcctttatgcagtactgcctgcgaccggaaatagggaaggtggaaattgcgccgttcgcctatatgcgtggacgtacctttgaaaatgcagtcgtcattcttgacgaggcgcagaatgtgactgccgcgcaaatgaaaatgtttttaacccgcctcggggagaacgtgacggttatcgtcaacggtgatatcacgcaatgcgatttgcctcgcggcgtgtgctccggattaagtgacgcgctggaacgtttcgaagaagatgaaatggttgggatcgtccggttcggtaaagaggactgcgtacgttcggcactttgccaacgtacgctgcatgcctacagttaagtgtgttatcggtgcagagcccgggcgaaccgggctttgttttgggtgtttatgcccggactagcgctttttctgaaacaaccatttttatttgcccctggctggtgaagtgtacgctcatcctgtggcttttttgtagttgctgatagagctcatcaggtattgctaagctctctgcatattcttgcggcgtatattggtaggctgcatgatgctgctgtttttgaaaacgcagcttattgtacagcgcccagacaattaacacgacggcattcgccactgccagcaaaaaatagaactgaagtcggcttctggcctcgctttgccagtaataacccgtcagcagatccatggcgaataagaatatgaacaacgcaaataatgtccacaagatggttgtggcaacataatcaaccagtaaacgtactggtgattgtcgggtcgtaataattaaattgttcatattaacctctcagaatcccgcgatcgggacttacccaacgggcgcgttgctttttaggcatcaacatgactcgtgtaaatgataccaatgtcgttgccaggctcagcatccagaaaataaccgggaaccaaataatccagaaaagcgatgaagtcagattatgctcatagcgattctcgatcatcaggctgacaataaattgcagtaaacataacgtacacaataatattccggcagtatgtgtcgcagcgatatgtgtcaattcaatatttaacggtacaccggcaagttggactgcgtaaataatgaaaccgaccaggcaggtgaaggcccatattgtcgtcaggcagtattcaaaaaacagcggccacattcgaaagttttctttgcgccacaaccttgtcatatttttgaggaatacttctgcaccgccctgagcccagcgcaggcgctgtttccacagcccttttaacgtttcaggcattaatatccagcacagtgcccgtggctcgtaaaaaatcgtccactgattcaactgcagcttccagctaatatcaatatcttcggtgatcatatcgtcactccagtaacccacttctgccagggcgctgcgacgaaatgcggcaataacaccggaaacggtaaatacgtttccatagatacgctgggttcgcttgatcaaaccaataattgaggaatactcgccaacctgaattttacccaccagggtagaacgtgttcgaatacgaggattaccggttacggcacccacacgcgggttgtacaacatcggttccacaatatatgccgccgcatcgcggtctaataacgcatcgccatcaatgcacaccagatattcacttttcgccgcggcagctccggttttaagcgcaatggctttcccctggttttgcgccagatgaatgacccgcaaatggggaatttgtgcagccatgcgatccaggatggcacgggttttatctgttgaaccgtcatttacggcaataacttcaatgttctcataacgctgtgctaaagcggcgtgtatggtttcctcaacgtttttctcctcattaaaacagggaatgataatggagatagacggattatctttcaactggggagctggtgcgttttctccccacggccagtggcgttcacgatagacccagaaatagacgccgccaacaatccacataatggacataaaaaacggccagaagaaaacgaacctcatcatcagttcaccagagtgaaagtacgctacgcataggggtatgcataacaccagacataatataaaaaacgatacgatgcgattaatcatttttcggataccaggctgttgaaaactcaggacgaataaggtctatttcaggttggttatgcagaaaattgtcgggataataaccatagtttttcactccattcagttgtaataggctcatccagtgagcgagttgttgcgaagaaatagcctgatgctgaccatttttctgccagttttgtgcctgtaattctaaaatagatttgtctttagcctgagggatgtttttaatttgattggtcaattgtattaaccattggtcagccgatttttctgcgacaccttccagataaggcatagccataatagcggtccagtcatagctttttaggaaatcagcataattctgtgcaaaccaggcttcactttcaggttgtattaccggaagtgcaaaaatatttcgtgcagttttaatatgtggaccgcgaatggcttttacgcgcgcactaagttctaaagtgaagtcagttaacgcacgacttttaaagcgggcccactgtttaaattgctccgggttttgtcgaatttcgctcagactcccgctaaagcctgcttgctgataagccgtgatagccggtgcactggcatcttcataatctgaaagcaaagcatcatcgtggaacaatatgccatcaaaagcagcatgtccggcaagatcttcatataacatgccaacttgtgctctgactctgtcatcgaaaggagagagacggtgatattgttcaggatgaatttgtgcttttttctcccctgttggtaagtattttactcgcgttaatgtgggatctaaatcccagcttaataccggcatccacgcatagatgtttacacctgagcgggtacgtaattgccaggcaacccgactaaaaatatctgctttcattggtagcaaacgatttggaaaccagacctctttgaccagcccatcaccatcgggatcagcaaatgcctgcaaatacacggttgatatttgcatatctttcacccgctgaattagcacatcaatattgcgatccatttgctggaggttttcgtcataaacgtaatcaagatcgatatgcattatccgttgtggtgatttttcctgtacggtaataatttgctgggcaaactcttttaatgagggattattggcgattaatacccgcggaatggaatccaattgcgacgcatttgccaaacctgattcaagggtgaagaacatgtcataaccgagtttttttaattcctctatcgctatgccattcgcttcgccataaggccaaacaaaaacgtgtggatttacctcaacctttgtacgcaggtattccgtcatttttacagcatccagacgaattctttcccggtattctgctgcggtttcataccgtgcgtggtcagtaaaatatgcacgatttacatatacaggcaataagctgccggtggcattagcctgaataccgtagtgagaattccatgtatgagaagcgagctcaacgagccgggaacgcgcaacttctcgcacttgttgccacgtggcaaaatattctcgatcgaccaactcatcgccaaattttacttgtttatccgctggcgtatcgacccaactgccgacgggggcccatacagcaggccactggaaggcctgaagaattgggaagacgcgggtataaaaactctggtagccgtcatcaaaagtcagcactacagctttttccggtagcggttttcctcctcgatgtgcttcacgaatttgagcaatactgaccggttgataaccgttctcgcgcagccaggcaaattgttcacgcagtgctgatgtccgcactgacataaaacgctggtcggcagcttcgtcttcaacgttatgccatgaaatcgctacaaaaccattatgcggccacggttgctcggcgagtaaagattcgcgatcctgtggcggtataaatgatgttcttgactggctaatgcacgcggtgagcataattatactcaccagcatcaggagatatttatttccattacgtaacatatttatccttaaaatctgaatgtcatatcgaattcaacgtataagttgtgttctctgtcaccgtcataaggtcgtttttcccagcgtagcgttgcgccagcatcaatcacgtcattccaactaatgcgttgcccgtagccgagttgggtgacgacatccgtgccataatgtttttgccaggaggcaccaacacctgcgctgaatatttgctcccagctattttcatagcttcgccataacaaatggcttgcctcaaatgccggaacaatatcgaacgtttttatagggttgtagtatggggtatcgtgttctgtattttgttcgtaatacagactgggtaggaaatcgacaatcaaatatggtgaagaccagatgcgttcctgaccctcaagtgagacttcatgacgctggttactgtcggaaaaatcagtgaaagcccaggagacaccgtacttacgccgctcattttgataccagcgaacataagcctgagcactgttgcctgtaacaccatttttcattgcccgtaatggaacgcggtgagagaggcgttccagttgcgaaccaatacgccagttatcattaaaatcataccagccagacaggcgcgcgccgggtttatgctcatgattgaaaacgcgttcagcgtactctgcctcgagccagatattacgtgaccgccactcaacacccgcaagccagtcgcgaacaatcccttttccttcgctaaattgtccatcggcataaccgaatccagcaaaaccgcgccagttatccttcagcggtggtgaataaacgatggtggttaagtcgacatcatgtttaccactatccgggccttcggcatcaattcctgttgagccagcgatacgaagctctgcaagattatgtacatcaaccgcacgttttaatcgtacaacgccgggatcttgcggttcacgttcgacaacatcgtgcgttaagacagctgcctgctgccattcttgtaacgttaatgctgtccaggcttgttcaacctccagattaatattacgtggctcgatcacttctgctttttttaattcattttctgctgcacgaggccaaccgcgggcttgtaacacactcgcgtaatcaatgcgcagtccctgatttcctggtgcgttataagcaagctctctggctgtcatttcagcctgaggaagatcattactatattttgctacggttgagagaaacgaatgcccctgtaaccaggtatcattcgggatgctcgtaggcgtgcccattaaccgaaggaaaggcggcgaagtattaatggtatgttgggtgacagttagcgcgcccggataattttcactctccaggtggctgtaaaagagatccgcaagttcttcatcggataaatccggggcaatggtctccttgtgataaaagagctcggtcattattgactgtgcttttttcggctgatgatctttgagataagccgatgcaacccaatattgcccccagggcggaataatttgccccgtcttttttaatcgctgatagtgagaaataacgtctttataacgatcgcgagttaataacgcgccaagatgatcaacctgaatacgctggtactgggcagtgcggtctgggttatcgtgccacagaatttctaatgcagcgtattgggcgagggcgcgatcggcaatggcataacgttcactttcactgcgcgtaggcataaacgacagtctgaccagttcggcatgaatatcagcgcgaatatctggcgttaaattggcatcgtcaatcgcggcagcaagttgattattacgtaatgcctgcacgtattctgtgggatattgttgcgtagatgcattttcaggtaatgactctgtcatcgcccgtaattcatcctgatgacgccccgccagtttatagatataggcttctgcgagtaaattggctttgtccggtgctccagagttaagctgcttaagtttaaccagcgcagtatcatagtgaccagcatctgccagggttaaaatttgtccccgttgataatccttattttgcggctccagagagagcgccttttgccacagtgtaagcgagttttgccattgttgcaggttacgataagcgacggcgacagctgcataaccacgcgctggtaattgctgatgacggtagcggttgtaaacggtaataacctgtttatcttgcccggcccataaggcaatctgtaaccagtcagcaatttggttattgctgagtgctgattttagtgcaaaccatgacaaagctggctgagtattacccttgcgagcttcaataatcaatgcatcataggcgttattaacagcactcttcgccgcgggactcgctgctaaaaatgcggcagtaagaagtttcaaagcccatttggttttcgggcacctttttctgctacttgaatacatcctgtattactccatgtattgccaaaatctctctctgtatctaattacaggtaactgaaaagaaagatatttttgcacctcataatccgttattaaacgcggaagagagacgtgaattgttgatgatgagaagaagaaatgatgagcagagtgtccatataaaatccttttctcgcccgaaaatccattccaatgatgaggatcttcaggaatacggcataaatcccaatgcctttttcaaaataaattaggattaaaataattaaatcagtaaattccgatgcatgatttcggatttttcgaaagtcctgatgaaaggctgcgctacggcactcacggatttaattgttattcctaatgtatctatgaattaatgttttataaggattttctataaccatttataagtattttcaagcctggcttgttgcaaacaatgtataaagcacttaggcaataataattacattcagcaactatcatcatcggtattgtttgtgggcggaatttcatattgacaacagtacagttcttatatctattaataatagaaagggatctacaacctacagattggtgtagctttatggaaaaagactatttgagaattagtagtactgtattagtgagcttattgtttgggcttgctttggttttggtgaatagttggtttaatcagccaggcgttgaggaagttgttccacgatcaacctatctgatggtaatgattgctttattttttatcgatactgttgcatttatttttatgcagttgtatttcatttatgaccgtaggcaattttcaaactgtgtacttagtttggcttttctgagttgtttgatttactttgttataaccgtcattatcattcagcaaattattgaggagcgtttgacaagcagtgttgtccaaaatgacattgcaatctattatttgtttcgtcagatgagtttgtgcatattaatatttctggcattggtgaataaagttagtgaaaacacaaaacagcgcaatttattttccaaaaaaatgactttgtgcataagtttgttttttgtttttggggggccgatagttgctcacatactttctagtcattatgagagctacaatttacacattgccgagttaaccaatgaaaatggtcaggtggtttggaaagcctcatatgttaccataatgattttcatgtggttaaccttgctttcggttaatctatactttaatggtttacgctatgatatctggaatggagtgacggtgattgctttttgtgccgtactgtacaatatctctctgttatttatgagcaggtatagcgtgtccacttggtatattagtcgcactattgaagtagtcagtaagttaaccgttatggtaatatttatgtgccatatattcagtgcgctacgagtaacaaagaacattgcacatcgcgatcccttaaccaatatatttaacagaaattatttttttaatgaactgacagttcaatcagcatcagcccaaaaaacgccttattgcgtcatgattatggatatcgaccacttcaaaaaagtcaacgacacctgggggcatccggttggcgatcaggtgataaaaacagtggtgaatatcattgggaaaagcatacgaccagatgaccttttagcgcgcgtcggcggcgaagagtttggcgtcttgctgacggacatcgatactgaacgtgcgaaagctttagcggaaaggattcgggaaaatgttgagcgtttaactggcgataatcctgaatacgctataccacaaaaagtgacgattagtattggcgctgttgtgactcaggaaaatgcgttaaacccaaatgagatctatcgactggctgataacgcactttacgaggcgaaagagaccgggcgtaataaggtggttgtgagggatgtggtgaatttttgtgagtcaccataaagcggcattttgatcctacccacgtaatatggacacaggcctaagcgaggttcttgttttcaaattgttccggactgaggccgccacaccaactgtgccgccgccaccgattgtaatcacattcgatataattaaacaccgttgcccgcattatttcccggctgataaagtgttctccatggatacattccactttcagcgaatgaaagaagctttccacgcaggcattatcgtagcagcaaccttttgcgctcatacttccacgcagattatgccgcttcagttgcgcctgataatctgctgaacagtactggcctccacggtccgtgtgaacgataacgttccggggcctcttacgccgccacagcgccatctgcagggcatcgcaggccagttgcgccgtcatgcgtggcgacattgaccagccaataacggcacgtgaccacaggtcaatgaccactgccagatacagccagccttcatctgtacgtaagtacgtgatgtctcctgcccacttctggttcgggccactggcgtaaaaatcctgctccaacagattttctgacacaggcaggccgtgtgcgcggtagctgaccgggctgaacttccgggaggcctttgccctcagtccctgacggcgcaggcttgccgccacggtttttacgttaaaggggtaaccctgagcacgcagttcatccgtcaggcgtggggcaccgtaacgctgttttgaccgggtaaaagccgcgaggacaacgctgtcgcagtgttggcggaactgctgacgcgtgcttatccttgtccgccgctgacaccacgtataccagccgctgcgggccacccggagcacgcggcacattgctttgatgctgaactcagcctgatgtttttcaataaagacatacttcatttcaggcgcttcgcgaagtatgtcgcggccttttggaggatagccagctcttcatcccgttctgccagctggcgtttgagacgtgcaatctcggtagacatctccagttcacgttcagaagacgtctgctgattttgctgtttactgcgccagttgtagagttgtgattcatacaggctgagttcacgggctgcggcagtaacaccgatgcgttcagcaagcttcagggcttcactgcgaaattcaggcgaatgctgtttacggggttttttactggttgatactgtttttgtcatgtgagtcacctctgactgagagtttactcacttagccgcgtgtccactattgctgggtaagatcagtgcctggcacacgcgtttgatggaagacggcgttcaggcaatgcgcgattatcttgccggactggatatcgcttcgccagagcatcaggttctgatgaacgtaacagcaaaaagcgaggtcgctccgtcaattatcaaagaaaatctctcattacacttaactcatacggtgaaatggactgaatctctcgatacatttctgaatatgccaaccccggtagctttccttgaaataagtaataagccctatttggggaatatgttaaatgattttgctggcgtggatcagcaacgagttatgcattgtcgtaaagcatttagtgatgcaaaggtattcaaatgattcctgattatttaacttttattcgctttcaggataaacgaaatctgatatacatttatgctattggacttattctgataggcttttattggaagaatgcagggtttacttttccatcagaggatattggtgtagttagtgggattctggctctggtgctgtataattttatttttgatctcaaggcgtactgggcttataaatgcgtcacgaagaatatcgatttttcgtggtttaagaaaaagcagaaccacaaaatagaattatttcttacacaacctctggtggcaggatttctgtcgttaatcatgttgagtgcaatgagttgggggctataccagcttctaccctcgttatatgcgctgttcctgatttcgttacttgggccgttggtcatctttctgctgtttcggatgatccgcaccagttatgtcaagcaggtcgctatttcagtagcgaaaaaagtaaaatataaaagtctgactcgctatgtgctgctttcggtgtgcatctcaacggttgttaacctgcttactatcagcccgttgcgtaacagtgattcttttgtgacagaggggcagtggttaacgtttaaatcgataattgcattgctcattctttgtggcgtagtgttggcgattaatctgttttttctgcgcttctccaagcggtacgcttttctgggcaggctttttttgcaggaaatcgatctgtttttctccagtgaaaatgcgttgtcgaccttttttgccaagccgctttggcttcggttattcatattgctggttattgaagtgatgtggattacgctggtgtcggtattggcaacgcttgtagaatggcggatttggtttgaagcctattttttactctgctatgtaccgtgcttaatttactattttttctattgtcgattcctctggcataacgattttatgatggcatgtgacatgtatttccgttgggggcattttaataagtgaggaagtgataggaagtgaccagataatacatatatgttctgtactctcttgcgcattttgattgttgactgagtaaccagacagttgatgtgcacgatttcccctcgccctaacagacgtgggcgggggcacccggtgtgtgcaatatacgaaaaaaaagcccgtactttcgtacgagctcttctttaaatatggcggtgagggggggattgactcgcttcgctcgccctgcgggcagcccgctcactgcgttcacggtctgtccaactggctgtcgccagttgtcgacccccggtcggggcttctcatccccccggtgtgtgcaatacacgaaaaaaaagcccgtactttcgtacgagctcttctttaaatatggcggtgagggggggattgactcgcttcgctcgccctgcgggcagcccgctcactgcgttcacggtctgtccaactggctgtcgccagttgtcgaaccccggtcggggcttctcatccccccggtgtgtgcaatatacgaaaaaaaagcccgtactttcgtacgagctcttctttaaatatggcggtgagggggggattgactcgcttcgctcgccctgcgggcagcccgctcactgcgttcacggtctgtccaactggctgtcgccagttgtcgaaccccggtcggggcttctcatccccccggtgtgtgcaatatacgaaaaaaaagcccgtactttcgtacgagctcttctttaaatatggcggtgagggggggattgactcgcttcgctcgccctgcgggcagcccgctcactgcgttcacggtctgtccaactggctgtcgccagttgtcgaaccccggtcggggcttctcatccccccggtgtgtgcaatatacgaaaaaaaagcccgtactttcgtacgagctcttctttaaatatggcggtgagggggggattcgaacccccgatacgttgccgtatacacactttccaggcgtgctccttcagccactcggacacctcaccaaattgtcgttcctgtcttgctggaacgggcgctaatttagggaaatcatgacctgaggtcaacaaactttttgaaaaaatcgcgcgtttattcaaacttcaatcaatgtgtggttttaataagcgaaatctgctttttttgccaccgaccacggatttgttatgctggtggcctttgtagatcataacgataagtgcgaataaatttcgcacaacgcttttcgggagtcagtatggatatcatcttttatcacccaacgttcgatacccaatggtggattgaggcactgcgcaaagctattcctcaggcaagagtcagagcatggaaaagcggagataatgactctgctgattatgctttagtctggcatcctcctgttgaaatgctggcagggcgcgatcttaaagcggtgttcgcactcggggccggtgttgattctattttgagcaagctacaggcacaccctgaaatgctgaacccttctgttccactttttcgcctggaagataccggtatgggcgagcaaatgcaggaatatgctgtcagtcaggtgctgcattggtttcgacgttttgacgattatcgcatccagcaaaatagttcgcattggcaaccgctgcctgaatatcatcgggaagattttaccatcggcattttgggcgcaggcgtactgggcagtaaagttgctcagagtctgcaaacctggcgctttccgctgcgttgctggagtcgaacccgtaaatcgtggcctggcgtgcaaagctttgccggacgggaagaactgtctgcatttctgagccaatgtcgggtattgattaatttgttaccgaatacccctgaaaccgtcggcattattaatcaacaattactcgaaaaattaccggatggcgcgtatctcctcaacctggcgcgtggtgttcatgttgtggaagatgacctgctcgcggcgctggatagcggcaaagttaaaggcgcaatgttggatgtttttaatcgtgaacccttaccgcctgaaagtccgctctggcaacatccacgcgtgacgataacaccacatgtcgccgcgattacccgtcccgctgaagctgtggagtacatttctcgcaccattgcccagctcgaaaaaggggagagggtctgcgggcaagtcgaccgcgcacgcggctactaataaagcatcaggattcctgctatccttggcgggaattgaatacaggagagagttatgtatcccgtcgaccttcatatgcataccgttgccagcacacatgcatatagcacattaagtgattacattgcccaggccaaacaaaagggcattaaactttttgcgatcaccgatcatggcccggatatggaagatgcgccgcatcactggcacttcattaacatgcgtatctggccgcgagtggttgatggggtagggatcctgcgcggcatcgaagctaacattaaaaatgttgatggtgaaattgactgcagcggtaaaatgtttgactcgctggatctaattattgccggttttcatgagccggtttttgcgccacatgacaaagcgaccaatacacaagcgatgatcgccactatcgccagcggcaatgtgcatataataagccatcccggaaatcccaaatatgaaatagatgtgaaagccgttgctgaagcagccgcgaaacatcaggtggcgctggaaatcaataattcctcatttttacactcacgtaagggcagtgaagacaactgtcgtgaggtagccgcagcggtacgtgatgctggaggttgggtggcattaggctcggattctcacaccgcgtttaccatgggggaatttgaagagtgtcttaaaatcctcgacgcggtagattttccgccagagcgcattttgaatgtttctccgcgccgcttactgaacttccttgaatctcgcggtatggcaccgattgcggaatttgcagacctttaattactagtaatggaaatatattaatgaacgagttttctatcctctgtcgtgtgctgggttcgctctattaccgccaaccacaagatcctttactggtgccgctgtttaccctgattcgtgaggggaaactggctgcgaactggccactggagcaggatgagttgctgacacgtttgcagaaaagctgtgatatgacgcaagtctctgccgattacaatgcgttgtttatcggcgatgaatgtgctgtgccgccatatcgtagcgcatgggttgagggcgcgacggaagcggaagtgcgcgcttttctttctgagcgagggatgccattagcggatacgccagccgatcacatcggcacattgctgctcgcagcttcctggctggaagatcagtcaacggaagatgagagcgaagcactggaaacactgttcagtgagtatctgttaccctggtgtggtgcgttccttggcaaagtggaggcccatgcaaccacgcctttctggcgcaccatggcaccgctaacccgcgatgccattagtgcaatgtgggacgagctggaagaagattctgaagaataagtgtgatctacgtcactcataactgcaacggataatttgttgttgcataaaatgtgtgctcgatctcattcatggccgcgttttctgctatcatgcgcggcatgaacatacttctctctattgcaatcacaacaggcattctctccggtatctggggatgggtggctgtttccctgggcttactaagctgggcgggcttcctgggctgtacggcctactttgcctgcccgcaaggtgggctgaaagggctggcgatctccgctgcaaccctgcttagtggcgtggtgtgggcgatggtcattatttacggtagtgcactggcaccacatctggaaattctcggttatgtcataaccggtattgtcgcgtttctgatgtgtattcaggccaaacagctgctgctttcatttgttccggggacgtttataggcgcatgcgcgacgtttgccgggcagggtgactggaaactggtgttaccttcgctggcgcttgggctgatatttggttacgcaatgaaaaacagtggcctgtggctggcggcgcgtagtgcaaagacggcgcaccgtgagcaggaaatcaaaaataaagcgtgaggggcactcacgctttcgcttaaacagtaaaatgccggatgataattccggcttttttatctgtcaggattccggtggaaccgacatatggcggtatttcaccagaatgtcattctgccgttctgctttattttgcaaatcccacagaccacggtcgataccatcattaatcaggaaaatgacccctgtttcgatagccgacatcaggcacagcataacaggttcgttcgaggtgtaacccacttccccttcaagcaagcgctggtagtcaataaagcggaaaaccccggcctgaacttcataggaaagtatcgtcttactggtgttcaccgaagaaaggatctcgccggtactcacattgacgacgcgcaggttcacggcaatctgatcgagctggtattgcgtgtcggcaccgatgccaaaatatcttgccccaaccccgccagatttgacgttgctttcataaccgataatcgaaccttcaaccatgatatttgccgccgttaaagattgcagcgggattcggttattaatggcaaccgtgccgttttcttgtgccgcacgaataatcttgcgctcgttaagcaggttttgtaagccctggcgctccagcggtataaaccagcgagaatctttcagtgccgtgaccagcattgccgtggcgctttgcggaacagcagtggagaagttacttgccgggtagggtttaaattgcccggtttcgtcctgaatgttgtataccgaaacaaagattttacccgtcggcgctggcagatgggtcaaatctttgtagctctgagcacgaggcattaatgtcggtctggcggcttctttaggcggggcggttaagcatccgctcagtaacatgacggcaaccaaaagaaataagcgctgcatgattattttccttatgaagctggggcttaaaaatcggttgagttattttgtaaacccgaaacctggatggtcgaggtttgtccggttttacgatctgtcacgttcaactgcaattgaccatcgcggttggcaatatcgacaatataatcgttggtcaccatgcggcccggtttaccggtattaatattcgacagtagcccacctaaaatttgtgactggatggcctgagtaaagttatctaacgctgagggtgtttcaataccaaagtcatcgttatagctcggatctttataagagttttgggcctgagcgctatttaataaaaaagcgccattatttgggttaccaccaaagtttggattacggaactggaaagtcatggttccagcccaacttaatggcgaaataagcatgagtagaactactgcatgtttgacacgcattgcagcctccgaacaattttttatttagaattcatcatgcgccaaatcgcccgtacttaataacgcctgatttatctggcgacgatttagtgcttcttcagtttgaatcagtgcaaagacgacagttttctcgaagtctcttttcaacggaaataaaaaagtctggaaaataacgtcctgattgaccgttatagtgatccagcttccccatcgtgcactgggcctttcattaatcgttaagttacccgtatagtcactttcccatttatcactaaaggctcggtaaaaatcatggccaatagatgaaacagtatggtcagttagcaatcccgggacttctacctcaacggcgtgaagattccctgcggcgaacagaaattctgccgccacaatccagcgtaaataacgtttcatggctttatcgcctgaggttatcgtttgcccaggaaaccgcttgtgtccggttttttacggctatcttcttgaaaagattataaagatgcgttttaaccgtattttcgctgatgaacaacgaacgagcgatctcgttattagacgcgccgatacgcagcttattcaggatctctttttcccgatgagtaaggagggctgattccgtgctgttataacgatagttacctgaatgcgtaatcaggtagctggcaagcttttgcgtaaagtagcattcgccgcgcaggacgccttgcaacccattgacaacacgttcttgatcctccatggaataaaaaacgccgttgatatgaggccagttttcaatgtcgcggtacgggtaatcttcaggcgtatttagcaacaatattttgatattgttgtttttcctgctcaaagtatcctgccaataatggataagctttttatccgcttccatcatatccagaagaataatagagcctgaagagatatcgtccagagaacgttgaatattatgtaattttcctgtaattgccagcgattgtttaaggtgctgcaagagagctgtcgcctgcaaagaagatttagtgatcaacaataatgtatgaccatgaatactatggacttcattaaacatgatgaaaccccgctttttttattgatcgcacacctgacagctgcctctaaaatagaagcaccagaagtactgacagatgttgcactgctgtgtgtagtaataaatcagccctaaatgggtaaaatataaaactaatggattacatctgatttcaatctagccattacaaatcttaaatcaagtgttaaacatgtaactaaatgtaactcgttatattaaaatgttaaccttaaggttttattaagtttagaaatgatagaaaagttgtacatttggtttttattgcacaattttaaaaaatcatacaaatggtgataacttactaataatgcatataaaaaatatttcggtgtagtcctttcgtcatgtaaaacgttcttgttttttctccacacctccgtggacaattttttactgcaaaaagacgaggtttgtcacggcttgtgcgcaagacatatcgcagcaatcagcgacgggcaagaagaatgactgtctggtgctttttgatagcggaaaacggagatttaaaagaaaacaaaatatttttttgcgtagataacagcgtatttacgtgggttttaatactttggtatgaactaaaaaagaaaaatacaacgcgcgggtgagttattaaaaatatttccgcagacatactttccatcgtaacgcagcgttaacaaaatacaggttgcgttaacaaccaagttgaaatgatttaatttcttaaatgtacgaccaggtccagggtgacaacatgaaaaacaaattgttatttatgatgttaacaatactgggtgcgcctgggattgcagccgcagcaggttatgatttagctaattcagaatataacttcgcggtaaatgaattgagtaagtcttcatttaatcaggcagccataattggtcaagctgggactaataatagtgctcagttacggcagggaggctcaaaacttttggcggttgttgcgcaagaaggtagtagcaaccgggcaaagattgaccagacaggagattataaccttgcatatattgatcaggcgggcagtgccaacgatgccagtatttcgcaaggtgcttatggtaatactgcgatgattatccagaaaggttctggtaataaagcaaatattacacagtatggtactcaaaaaacggcaattgtagtgcagagacagtcgcaaatggctattcgcgtgacacaacgttaatttccattcgacttttaaatcaatccgatgggggttttacatgaaacttttaaaagtagcagcaattgcagcaatcgtattctccggtagcgctctggcaggtgttgttcctcagtacggcggcggcggtaaccacggtggtggcggtaataatagcggcccaaattctgagctgaacatttaccagtacggtggcggtaactctgcacttgctctgcaaactgatgcccgtaactctgacttgactattacccagcatggcggcggtaatggtgcagatgttggtcagggctcagatgacagctcaatcgatctgacccaacgtggcttcggtaacagcgctactcttgatcagtggaacggcaaaaattctgaaatgacggttaaacagttcggtggtggcaacggtgctgcagttgaccagactgcatctaactcctccgtcaacgtgactcaggttggctttggtaacaacgcgaccgctcatcagtactaatacatcatttgtattacagaaacagggcgcaagccctgttttttttcgggagaagaatatgaatacgttattactccttgcggcactttccagtcagataacctttaatacgacccagcaaggggatgtgtataccattattcctgaagtcactcttactcaatcttgtctgtgcagagtacaaatattgtccctgcgcgaaggcagttcagggcaaagtcagacgaagcaagaaaagaccctttcattgcctgctaatcaacccattgctttgacgaagttgagtttaaatatttccccggacgatcgggtgaaaatagttgttactgtttctgatggacagtcacttcatttatcacaacaatggccgccctcttcagaaaagtcttaatttgttgaaatatcgagcataagatgaatctggagagaatggtctgctgcgaatcagccaacctgaaagtatggataacacaaccctcaaggatgactaatcattgaggaaatagaataaatgttcagaccttttttaaactctcttatgctcggcagtttgttttttccttttattgccattgctggaagcaccgtgcaagggggcgtgatccatttttatggccaaattgtggaaccggcatgtgacgtcagcacccagtcatcacccgtagaaatgaactgcccacagaatggttctattccgggcaaaacctactccagcaaagcgttaatgagcggcaatgtcaaaaacgcgcaaatagcctcagtaaaagtgcagtatcttgataaacagaaaaagctggctgtaatgaacatcgaatataactaagtttctgaacaactcacgttgctgagcagaaaaatgcgatttaaccaaaaagcctgctgtacacttaagaaacaagaaggtgtaaggaggcgttatgaaaacgcgtattcatgttgtgcagggtgatattaccaaactggccgttgatgtgattgtgaatgcggctaatccgtcattaatgggaggcggcggcgtcgatggggccattcatcgcgcagcgggtccggccctgctggatgcttgtttaaaagtcaggcaacagcagggcgattgccctacggggcatgccgttattacgcttgcaggcgatcttcccgctaaagccgtagtgcacaccgtcgggccagtctggcgtggtggtgaacaaaacgaagaccagcttttgcaggatgcctatctcaatagcctacgactggtggcggcaaacagctatacgtcagtggcttttcctgcaatcagtactggggtttatggttaccctcgtgcggcagcggctgaaatcgcagtaaaaaccgtttcagaatttattacccgtcacgctttacccgaacaggtatactttgtctgttatgatgaagaaaacgcccacctctacgaaagactccttacccaacaaggagatgaatgatttgccccggctggcgagcgcggtgctgccactgtgttcgcaacatcccggtcagtgtggcctttttcctctggagaaaagtctggatgcgtttgccgcccggtatcgtctggccgaaatggcagagcatacgctcgatgttcagtattacatctggcaggacgatatgtcgggtcggttactgttttccgccctgttagccgcagcaaagcgtggcgttcgcgtccgtttgttgctggacgacaacaatacgcccggacttgacgacattttacgcttgcttgacagtcatccacgcattgaagtccggctttttaatcctttctcgtttcgcttgctgcgtccgcttggttatatcaccgacttttcccgtcttaatcgccgtatgcacaataaaagtttcactgtcgatggcgtggtgaccctggtgggaggacgaaatattggtgatgcctattttggagcaggggaggagccacttttttcggatttagatgtcatggcaataggacccgtggtagaggacgttgccgatgatttcgcccgctactggtattgcaaatcggtttcacccttacagcaggtgctggatgtcccggagggtgaaatggcggatcgcatcgagttacccgcctcctggcataacgatgccatgacgcatcgttatttacgcaaaatggaatccagtccatttataaatcatctggttgatggaacattgccgcttatctgggcgaagacacgtttattaagtgatgatccggcgaaaggggagggcaaggcaaaacggcattcactgttaccgcagcgcctgttcgatatcatgggctcacccagtgaacgcatcgatattatctcttcctattttgtaccgacacgcgcaggtgtggcgcaactcttacggatggtgagaaaaggggtaaagattgcgatcctaaccaattctcttgccgctaacgatgttgctgtcgtccatgccggatacgcgcgctggcgcaaaaaattgctccgctatggcgtggaattatatgaactcaagccgacgcgtgaacaaagtagtacgttacacgatcgcggcataaccggtaattccggagccagcctgcatgctaaaacctttagcatcgatggtaaaacggtgtttatcggctctttcaatttcgatccgcgttcaacattgctcaatactgaaatgggcttcgtgatagagagcgaaacgctggcacagttaattgataaacgctttattcagagccagtatgatgcggcctggcagctccgtctggacaggtggggacggatcaactgggttgatcgtcatgcaaagaaagagattattctcaaaaaagaacccgccaccagtttctggaagcgggttatggtcagactggcgtcgatattgcccgtggaatggttattgtaaatgtggcttaacgggctggtgctttatcgttctcacgcttaacaaccggtttaccagagaacaaaaacttcagtaacgggatgcgcaaatgaatttcatacagaattatcgcaatccctactacaaatatcaggccacagagaaaaccaagccagttggaggtgatgtgcggtgtaatgtatgcgccgaaaaacagcgttaacgggtggtgaaccagatagataaacagcgatgcgttaacaaaataagtcacccgcgctgactggaagttaagcaaacggtggccaaaggagaagaccacattcaccatccacagaccgaggaccatggtgatcaccgactcggtttcgtacatccaggcatcgccactgccatagcgctggttgagtaaataagcgacaaacgccaatgctgctgcaagggtacagccacgagacggcgtggtaaacaaggctttaagatgagggaaaatgaaagccagtgcgccgaggataaagaacggcaaataaaacagcgtttgcatgacaataaaattgaacatgccattactcagaatgggcggatacacaataaaaatcgttcttcttattaccgcataaccgatgccgaggcataaaaaaatcaccgatagttttaccatcgagaattttttattcgttttatcagaattttctaaattatttctgatgcgcttaaatatccatacgcacagcgtcgtcatgaccactaacaccagtaaaaaccacaggtgtgatattaattcccaggccaacgtattatatttgtcatacaatgacagcccaggccaactttccgcttttcctttgacatattgcagcataataaattgcggtaatgtcagtagggggatggctgttaacatcgggatacctacacgttcgacacgtactttccaccattttttcaagggatagcgtaaaaaaagcatgtaggaaaagtagccggatataacgaaaaatacctgcatgcggaacgagtggatgaagtcattaaaaagggtcagccacaatgatgattcggcgctattcacatgccatgtatggctcgaatagattaaagaaatatgaaaaggtatccctaacaacatcagccaggcgcggatggagtcgaggaaatattcacgttgcgcgggtactgggttcatatatggttaactaatctcggatttttcgtcttatccctgtcgggttatgcctttaggcttgttgccatagtgacaccgacctgaccgcgccaggcgcaggcttcaaggtttttatgcatagcatcatcgctaccactaaccagaatggaagcgtctgtaagacggttgataaataaatttgctggcaaaccctacacgaagtcgatgcttctgtctttaggagaagcacggaaagtgaaaacggttgcaatcaggtgcttaatccatgagccagcgtgctgaacgataccgggattctgttgtcggaatggctggttatccattaaaatagatcggatcgatataagcacacaaagggggaagtgcttactaattatgaaacataaactacaaatgatgaaaatgcgttggttgagtgctgcagtaatgttaaccctgtatacatcttcaagctgggctttcagtattgatgatgtcgcaaagcaagctcaatctttagccgggaaaggctacgagacgcccaaaagcaacttgccctccgttttccgcgatatgaaatacgcggactatcagcagatccagtttaatcatgacaaagcgtactggaacaatctgaagaccccattcaaactcgagttctaccatcagggtatgtacttcgataccccggtcaaaataaatgaagtgactgccaccgcagtcaaacgaatcaaatacagcccggattatttcactttcggcgatgttcagcatgacaaagatacggtaaaagaccttggctttgccggttttaaagtgctttacccgatcaacagcaaagataaaaacgatgaaatcgtcagcatgctcggggccagctatttccgcgtgattggtgcaggtcaggtttatggcctttctgcccgcggcctggcaattgataccgccttgccatcgggtgaagaatttccgcgcttcaaagagttctggatcgagcgtccaaaaccgactgataaacgtttaaccatctatgcattgcttgactcgccgcgtgcgacaggtgcttacaaattcgtggttatgccagggcgtgacacggttgtggatgtgcagtcgaaaatctatctgcgcgataaagtcggcaaactgggggttgcaccgttaaccagtatgttcctgtttgggccgaaccaaccgtcgcctgcaaataactatcgtccggagttgcacgactctaacggtctctctatccatgccggtaatggcgaatggatctggcgtccgttgaataacccgaaacatttagcggtcagcagcttctccatggaaaacccgcaaggctttggtctgttgcagcgcggtcgtgatttctcccgctttgaagatctcgatgatcgttacgatctccgtccaagcgcatgggtgactccgaaaggggagtggggtaaaggcagcgttgagctggtggaaattccaaccaacgatgaaaccaacgataacatcgtcgcttactggacgccggatcagctgccggagccgggtaaagagatgaactttaaatacaccatcaccttcagccgtgatgaagacaaactgcatgcgccagataacgcatgggtgcaacaaacgcgtcgttcaacgggggatgtgaagcagtcgaacctgattcgccagcctgacggtactatcgcctttgtggtcgattttaccggcgcagagatgaaaaaactgccagaggataccccggtcacagcgcaaaccagcattggtgataatggtgagatagttgaaagcacggtgcgctataacccggttaccaaaggctggcgtctggtgatgcgtgtgaaagtgaaagatgccaagaaaaccactgaaatgcgtgctgcgctggtgaatgccgatcagacgttgagtgaaacctggagctaccagttacctgccaatgaataagacaactgagtacattgacgcaatgcccatcgccgcaagcgagaaagcggcattgccgaagactgatatccgcgccgttcatcaggcgctggatgccgaacaccgcacctgggcgcgggaggatgattccccgcaaggctcggtaaaggcgcgtctggaacaagcctggccagattcacttgctgatggacagttaattaaagacgacgaagggcgcgatcagctgaaggcgatgccagaagcaaaacgctcctcgatgtttcccgacccgtggcgtaccaacccggtaggccgtttctgggatcgcctgcgtggacgcgatgtcacgccgcgctatctggctcgtttgaccaaagaagagcaggagagcgagcaaaagtggcgtaccgtcggtaccatccgccgttacattctgttgatcctgacgctcgcgcaaactgtcgtcgcgacctggtatatgaagaccattcttccttatcagggttgggcgctgattaatcctatggatatggttggtcaggatttgtgggtttcctttatgcagcttctgccttatatgctgcaaaccggtatcctgatcctctttgcggtactgttctgttgggtgtccgccggattctggacggcgttaatgggcttcctgcaactgcttattggtcgcgataaatacagtatatctgcgtcaacagttggcgatgaaccattaaacccggagcatcgcacggcgttgatcatgcctatctgtaacgaagacgtgaaccgtgtttttgctggcctgcgtgcaacgtgggaatcagtaaaagccaccgggaatgccaaacactttgatgtctacattcttagtgacagttataacccggatatctgcgtcgcagagcaaaaagcctggatggagcttatcgctgaagtcggtggcgaaggtcagattttctatcgccgccgccgtcgccgcgtgaagcgtaaaagcggtaatatcgatgacttctgccgtcgctggggcagccagtacagctacatggtggtgctggatgctgactcggtaatgaccggtgattgtttgtgcgggctggtgcgcctgatggaagccaacccgaacgccgggatcattcagtcgtcgccgaaagcgtccggtatggatacgctgtatgcgcgctgtcagcagttcgcgacccgcgtgtatgggccactgtttacagccggtttgcacttctggcaacttggcgagtcgcactactggggacataacgcgattatccgcgtgaaaccgtttatcgagcactgcgcactggctccgctgccgggcgaaggttcctttgccggttcaatcctgtcacatgacttcgtggaagcggcgttgatgcgccgtgcaggttggggggtctggattgcttacgatctcccgggttcttatgaagaattgccgcctaacttgcttgatgagctaaaacgtgaccgccgatggtgccacggtaacctgatgaacttccgtctgttcctggtgaagggtatgcacccggttcaccgtgcggtgttcctgacgggcgtgatgtcttatctctccgctccgctgtggtttatgttcctcgcgctctctactgcattgcaggtagtgcatgcgttgaccgaaccgcaatacttcctgcaaccacggcagttgttcccagtgtggccgcagtggcgtcctgagctggcgattgcactttttgcttcgaccatggtgctgttgttcctgccgaagttattgagcattttgcttatctggtgcaaaggaacgaaagaatacggcggcttctggcgcgttacattatcgttgctgctggaagtgcttttttccgtgctgctggctccggtacgcatgctgttccatacggtcttcgttgtcagcgcgttccttggctgggaagtggtgtggaattcaccgcagcgtgatgatgactccacttcctggggtgaagcgttcaaacgccacggctcacagctgctgttagggttagtgtgggctgttgggatggcgtggctggatctgcgtttcctgttctggctggcaccgattgtcttctcgttgatcctgtcaccgtttgtttcggtgatttccagccgtgccaccgttggtctgcgcaccaaacgctggaaactgttcctgatcccggaagagtattcgccgccgcaggtgctggttgataccgatcggttccttgagatgaatcgtcaacgctcccttgatgatggctttatgcacgcagtgtttaacccgtcatttaacgctctggcaaccgcaatggcgaccgcgcgtcaccgcgccagtaaggtgctggaaatcgcccgtgaccgccacgttgaacaggcgctgaacgagacgccagagaagctgaatcgcgatcgtcgcctggtgctgctaagcgatccggtgacgatggcccgtctgcatttccgtgtctggaattccccggagagatattcttcatgggtgagttattacgaagggataaagctcaatccactggcattgcgtaaaccggatgcggcttcgcaataaaaacgtagttgcctgatgcgctacgcttatcaggcctacatcgttcctgcaatttattgattttgcaagactttgtgggtcggataaggcgttcacgccgcatccggcaaaaacaacgagccaataaaaataccggcgttatgccggtatttttttacgaaagaggtatcaaatgcgtttaattgtggtgagcatcatggtgaccttgctgagtggctgtggcagcattattagtcgcactataccggggcaggggcatggcaaccaatattatcccggtgtgcaatgggatgtgcgtgactccgcctggcgttatgtcacgatccttgatctgccattctctctggtttttgatactttactgctgccgatcgacattcatcatggcccgtatgagtgattaacgttcatcccactcatcagctgctgcgcgtccttcctcggtatccagcggtggctcaagctgaaattccccctcgtcccattcatgtaatgtattctcttcctgccactcctggcgtatctctatctcatcatagtcgccatcaaaaacactttgcgcggcttcaccgctaagcataggtaaacattcaccttcttccccttcgtcggcaaaaaactcaacttgccacatgatgtcgccgtcctgcaaaacgtatttttgggcattgaactgttgcacattcgcatcttcggcgtcgatgccggggttgtctgcaagaaattcttcgcgtgcagcgtcaatggcttcttcaagcgttgcgtacatggtcatcacgattctccctttgagttgatgaggtttcagggaaaaggatagctgattctccgcttttgcaagtatgaaaggcgaaaaatcagttcgatacctggggtattcgacgacgacgtagactgttccatgaatagactgcgttgaataacactacgccagcggtgacgagaaataccgctctgaaaccgtagttcgctgaaatcgctgctcccatcaatggtccggtaacgttgccaatatcacgaaacgattggttatagctgaagatacgcccggcgatctggttgctcgagttgtaaaccaacagtgtctgtacggcggggagtagtgcaccatcggcggcaccgagcaaaaaacgtaaaatcccaagttgcaatggcgtctgaacgtaagacattgggatcaacagcagtacagaaaagatcagcgctgtaatcaggatcttttcgggtccgattcgatcgccaagtttgccgagtcgtggtgcacttagcagagccgccacgcctggcaccgaggcgatcatgccactgataaaggcgacgttactgacgttacccgccagttcgcggacatacagcgtcagaatgggggcaattgagcccgtcgccacctggatgattaacgtagtgacaaacaggctgagtaccagtttcgggtttttaagtgatgtcaccacttcccgcatgtgcagcatctcttttttgctgaccggctggaatttttctctgatgcaaaacagggtgacgaaaaagcagagtatgagcacactggcggtaataaagaataccggacgtaagccgtagctatcggcgagcaggccgccagccattgggccgagcaacgcaccactaacgccgcctgtggagagcgtacccagcgcccagccgcttttattacgcggtacttgtgtggcgataagagcattagcgttggggacaaatccgccaagtaacccaagaagcgcccgcaggatcaaaaactgccagatattttgtgccagccccatcaacaccatcacgatgcccatgccgagggcagagcgtaatagcatgagttttcggcctttacggtcggcgagtccaccccaaaacggtgaggcgatggccgaaaataaaaatgtaatgctgaagacaataccggaccacatattcagggcggagtgaccggtaacgccaagctgctcaacgtagaggggtaagaagggcattaccagactgaaggcggcaccggtaagaaaacagcctagccaggcgacgatcaggtttcgtttccagtttataggggtgtcattttcacagggtgacatagcaatccgctgttggtgcgccaggcgcggtgaacataagaagaaaagataagcacactaattatgcgcccgacttccagggggcgcaatccagagagcttttatcgctaaatcagggggatttgctgtggtaatgccggatgccattctgaagcatccggcatgggagatttaatagcgtgaaggaacgccttccgggcgtgttttaaagcgacggtgtaaccacatatactgctctggtgccatcatgatgcatttttcgaccactttgttcatccacgcggcggtagtttcggcatcatccagtggcggagaacactctggcggcagcataatcaattgataccctttgccatctggcttacggcgtggaacgaagggcaccagacatgcgccggacatccgtgccagcatccaggttccggtcgtggtcgcagcctgctcaacggcaaacaacgggacgaaaacgcttgagcgcgggccgtaatcatgatccggtgcgtaccagaccacttcgccttttttcagggctttaatcatgccttttaaatctttgcggtcgagcatcgatttatttgagcgcaaacggccccaggtttgtagccagtcaatcagtggattatcgttcgggcgataaacgccaatacccggttcctgcataccaaactgccgcgcacccagctccagtgtcagaaaatggatgccaactaacaggatgccgcgtttttgcgcctgcacgtcacgaatgtgttccatgccgatcacttccgtccagcgggcgattcggcggtccggccagaaccacgccatgccggtttccatcaggcccatgccaacggattcgaaattcttcaccaccattttacggcgttcttgttcgctcatttccgggaagcacagttccaggttgcgatgcacaatttttgcgcgtcgtttcataaaacgtaacgccagttttcctaatccacaaccgaggcggtagataaccgggtagggcaattgcacgactaaccaaagtacgccaatacccaaccaggttaaccaataacgcggatgaagcagtgcggtggagaacttgggtagattcgtcatatcaatcctgtttttcaacctattcgggcaattgtatgtattgtcgcattttttcgcccgcaaccaaaatttgtggctgaagactgggcgaaattgccgcgcttgtaaataacaaataatttttaatgcgcaaatgtagcgtaaaatgtgtggatgttaattatcgataattgctatatcatgccgcggatttttactttcccatctcgcaggaaccgtacaccatgccagtgttacacaaccgcatttccaacgacgcgctaaaagccaaaatgttggctgagagcgaaccgcgaaccaccatttcgttttacaagtatttccacatcgccgatcctaaggcgacccgtgacgctttatatcagctgtttaccgcgctgaatgtttttgggcgagtgtatctggcgcatgagggcattaacgcgcaaatcagcgtacctgcgagcaatgttgaaacatttcgcgcgcagctctatgccttcgacccggctttagagggtttacgcctgaatatcgcgttggatgatgacgggaaatccttctgggtactgcgcatgaaggtacgcgatcgcattgttgccgacggtattgacgatcctcactttgatgccagcaatgttggtgagtatctgcaagcggcggaagtgaacgccatgcttgacgatcccgatgcactatttatcgacatgcgtaaccactatgagtatgaagtggggcactttgaaaacgcgctcgaaattccggcagataccttccgtgagcagctgccaaaagcagtcgagatgatgcaggcacataaagataaaaaaatcgtcatgtactgcaccggcggcattcgttgtgaaaaggccagtgcctggatgaaacataacggattcaacaaagtctggcatatcgagggcggaattattgaatacgcccgtaaggcgcgcgagcagggcttgccggtgcgttttattggcaaaaattttgtttttgacgagcggatgggcgaacgtatatcggatgagattatcgcgcattgccaccagtgcggcgcgccgtgcgacagccataccaactgtaaaaatgatggctgccacctgctgtttattcagtgtccagtatgcgcggaaaaatacaaaggttgttgtagtgagatttgctgcgaagaaagcgcgttaccgccagaagaacagcgacgccgtcgggcaggacgtgaaaatggcaataagatctttaataagtctcgtggacgtctgaatacaacactgtgcattcctgatccaacagaataaatatcattgccggatgcgtgccatccggcaacatttcacgcttacttctgctgtacgccttccactgaaataatcagatccacttcctgagaagctggacctaaatctgtcttgatattgaagtccttgagcttaattttgccttcggcctcgaagcctgcacgtttaccaccccatgggtcgtcgccctgaccaattaatttcgcttccagcgtgacgggtttggttacgccattcagcgtcagatcgccggtaatatccagttcgtcaccgtctttcttcacgctggtggaggtgaatgttgcctgtggatattttgcggtattgaggaaatctgcactgcgaagatgtttatcgcgttcggcgtgattagtatcgacgctggtggtgttaattgtcacattcactttatcggcagccggatttttttcgtcaaaggtaaaagtaccgtcgaaatctttaaaggtgccgtataaccagctatagccaaggtgctggatgcggaaattaacaaaggcgtgctgaccttctttgtcaattttgtaatcggcggcaaccgctgaaccggcagagaacatcagggacgcgaaggttaaaccaagcaggctttttttcattttttatactccatagtcagatgacgactttcccagcatgcgcttcagagtgtcgtctttatcgatgaaatgatgcttcagggccataaatccgtgcataacggacagtactacgacgctccacgcgagccaaaaatgcagggcaccggcaaagtctgcctgtgcgccagcgtcggcaagggtcgcggggacgtcaaaccagccaaaaacgctgatcggtttaccatcggcagttgagatcagatagccgctgatgccgatggcgaaaagcaataggtacaatgcgagatgtccagctcttgcggcaagacgagtcatgggcgaataactcggcagcggacccggcggtggagatatgacacgccacagaacgcgaataaccagccccatcattaacaaaataccgatgcttttatgcagttcgggtgctttgtgataccagccatcgtaataactgagcgtgaccatccacagacctaaagcaaacatgccgtagacaataattgcgcttagccaatggaaggccgcagatataacaccatagcgttcaggggtatttgtgaatgacataagtgcatccaaaacgaatttgcgagagaaagaaaatggcgtgtcggagaatgaattgcaacacaaaaataacaaattgaatgatatttatttttatttcaataattttgaattaataatgaaagaatcttcataagtttagtgggttcagcatcagagatgtctggtgagtgctgtagaagcaggaataatctcattcaatttttcacgctaaatgaaagggagattaaatatttgtcagtttatgtcagtgcggaaaactaaaaataaaacacatagatcagatccataattgccaacaatccccagagaaaaagataaagcatcagatgctcgcgaatattattgatgagatagtgcaacagccgacgcattaaatactcctgtaaaaacggcctcattctggaggccgtaatgatgattattggaagcgggaaagcctgaatggcgtcaaatcaaaatcgctttttttgtcttgcgcaaaatcggcagctatttcccctaaaactgacgcaaatttaaaaccgtgcccactcaggccggtaatgagcagtgtattatcgtggccgggtagggtatcgataataaaatcttcgtcaggcgaattatcataggtgcaggcagcgccgtacaggcagcaaccgatacccggcaatacattgcgcaagaacgggaaggcttctgacccatcactggccacttccgcaaacggaacacgttcatccgctgaatggataacctggcctccgttatgtttgccaatcttcaacgcgtcgttttctgccggaaaaccataatattgatcgccattgggcagttcaccggtaaacgccgggaatttattcttcacgctatagcggccatcggcctgataccaggcaaatactttgcgtacgggctggacaggcagctccgggagcaggtcttttacccatgttcccgcgcagacaatcgcttttttcgcctgatactcaccgtcagccgtttcaatagttacgccatcatcgtcatgacgaattgcggtgaccgggcagttgaacagttgcgcacagcccgcttccttcgccagttggatccaggttttaatcgccagttcgctgcgcaaaaaaccggaatcagtttcaaataagccgatgtagttgtccgggacgcgtatttccggccagcgggccataatcccttgcgcatcgagcttttcaacgttgagttgccattgttcggcgctgtgggcgacgttggcgagaaatgtggaatcagccgggccaaggttaatgacgccagagcgtacaaaaatgggatcttcttcgttgtggcgggagagttcatcccacagcgtttgcgcgcggaggaccagcgggacatacttttcgccttcaccataagcatggcgaattaatcgcgtatcgccgtggtggctgccgtgttgatgcggtggcatatgggcgtcggtcattagcacgtttaaaccggcgcgggttgcataatacccggcggcagcgcctacggaaccgctgccaataatgatgagatcgtatttcatttttttctctctgctctcatggtttaagcagagtaattaactgaatgcagatatacaacccagaaatggtaaaggcaccggtgaggtgccttttgggtggatggtcatgtcatgttaatgacgccgatactcgtttacctggaaatcaccggattcaattttggcgattcctgcttctaatatcgaaataaattgtctggcaacatcagtggttaaccagagcgtctgaccaacttcagtcccttcctgctcggacttatttggggtctggtagtgcaaacgcaacatcagcgcatcatagctatcaacggtgctgatgtcccaccctacgagcggatgagtctgaatgacttcattatttttttccatcatggccccctaattcgtgttactagacaacgttattcgaggttcaatgcgtttttatctgaagcaacttcagtataccaataagtaagggtattcaccgaatttttaaagggggaaacagataaatttctgcttttaagatttatatgaacaataaaacagcatgtcattcatatttttttagcatattgtgcaattattttgaggaagtgtagaaattttgtactcaaaattcgtaagtaaaataaaaaagccggggcgacccggcaaaaaaaatcactgcatattattcgctgacaaaccagtcatcggcgctttcccacgtttcctggagaatttcactaatgcgctgtttatcttcttttgtcgcgccaataaccgataaattattcgctgcggcataacgtaccgatacgtggccttcattatcaggaaacgcatactgaatacggcgggaaagttcgccagccagggcgtcaatagccccagctggcaatggagaagttttcgctatggtgacttcaattcgcataatagccccctgttgaatatactggttatttatacaggtaaaataacctaatgacaacaggaagctacgatttttattgtttaacggaccagcgtaccgtttccccggcgaggaatggcaccagcgtgtcatcagtcagtgcgatgctttcagcaacctgttgctcttcacgtaccagttcgatgaatgtgtcgttgaccggcaacccatagaactgcgggccgtttacagaacagaatgcttcaaagtgctgcaaagcattcatttcttcaaagacggtagcgtaactgcccagcgcggttggggcgttgaagcagcccgcgcagccgcaactgctctctttgcgatgacgtgcatgtggcgcagaatccgtaccgaggaatactcgattaaaaccgctggcgaccagttcacgcaatgcctgttggtgaatattacgtttgaggatgggtagacaatacaggtgcggacgcacgcctccaaccagcatatggttgcggttaaacatcagatgctgcggagtgatggtggcagccagccgttcatttccgtcacggacatagtcggcagcatctttggtggtgatgtgctcaaaaacgactttcagcgcagtcaggcgctggcgcagaggttccatcacgctttctataaagcgcgcttcacgatcaaaaatgtcgatatctgcatgtgtcacttcaccatgcaccagtagcggcataccgattttttccatgcgctcaagtaccggcatgattgcgtcaattgacgtcacgccgtggctggagttagtggttgcgtttgccgggtaaagttttgcagcggtgaacacgccttcgttaaatccgcgctccagctcattaggatccagcgaatctgttaaataacaggtcatcaatggggtgaaatcgtgcccggcaggtacggcgtcaagaatacgctggcgatacgccacggcagcctcaacggtggtcacgggcggagccagattgggcattacgatagcccgtccataaatttcgctggtatatggcacgacagtttttaacatgtcgccatcgcggaggtgaaggtgccagtcgtctgggcggcggatctttaatacctgggatggtgcagtcattaatctctatgctccggctgaagggatgtttttgccggacacaaaggataagcggaaacgttttcctttgcacgaaaaataaagggcgcgaatgcgccctcgtgattaatcagtaaatggaatgacaatttcgcctggcttcacttcaatgcctttcgccagttttttcgccattgcttcgccctggctgccatcttcgcgcaggacgtaagcaggttgctggttaaagtaattgcgtaatgcctggttcaaatagggaagcaacgtttgcatcaccgtttgcattttttccggttgtaccgtcgcatcgaccacttccatctctttcaggaagatcgcacctttttctttatcaaacacgggcagcgctttcagcttcagtttcatggtcgctttctgactaccgaacagggagttcatgtccagattggcgtctccggttagggtaaccttattcggctcttcgcgaccaatttggctggtcaggtttgtcagaacaatatgggcgtcagccacgccgggtaaaccgatatcttttgagaaattattatgtttcgcaagcgactggttaatttcttgttcggtgatggtgtattgggtgagttgattacagccaacgagcaggccactgacgatcaatgcagcggcaaataaaaacttgttcatggtagtcctcgacatgaaatctgcgtcaatatcctgacacaacgcagcatgtgtcaccagcgataaactcgccagcagaaaaaactgaaaacggcggcaacccgcgaatacaggctgccgcggcgggtcaggattaaatcgccattgatgataacaaattgatttgtgtctgtttcgccatattatcgcggtaatcagcaacgcggcttggccagttaattccggctaccagcgtcagattacgcagtagcgggaatagctgaatatcatcttccgaaagttcgccattcacggcgttcggtttgacgatcagtttgtccagcgcacgtaaatcatcgctgatattcttaatcagaccgtcagagtgggccagcaggtcggcaaaattacccgcgctggcctctttcttgtcgacgaaatatttgcgcgcggcgggagtagaaaactcatcaaatgccgatttggcaaaacgcggcaacagcagtttgttggcgtagccattgaccttgcgcagccactcttcaatggcaggggaacgtttgccggtcagtaacggtttgccgtcgagtttatcgacatagtgaacgatgtccatgctttctggcatatagcggctgtcatctttttgcagaatgggaacctgtttttgaccgaccatccgggtgggtgtttctgcgtcgtcgttgagcagaacatgtaattcgacggggatatttttcaggccgaaaatcatgcgggctttgaggcagtaagggcagtgatcgtaaatgtatagcttcacgtgactcctccatttggctgtcagttcactttcagtatgaaggagtcaggggggagtatcaaatcaggcgtcgcgttcaagcaaacgacgcgcggcgcgtttctggctaaactgccaacccagcgcaaggaaagtgaagatgccaataatgcccagcatcatccacggaagctctggctggtgcgccgatttgcccaggtcaaacagccagccgccaccgatataaccaatagcgccgccaatcgccagacccagacggctaaaccccatatagctgccgcgagctcttgcgtccgccagcgaagcacttaaggtttcacgcgcaggctcggcaatgatcgacccgatataaaacagacaaatcagggtgaaaagttgttgcaggccgctgaccatgcccaccggcatcatgcttaatgacattatcaacagcccagccatcaaccggtgttccagacgaaaatgcttttcactccagcgggcgatagggtagagcaacgttaacgacagacacgcttcaatggcatacatccatttaacggcagagggcgcgccagccacgtcgttgaccataattggcagcatcagcatcacttgtacagccagcatgtagtaacccgccagcgtcagaacataggtgacaaaacgcttgtcacgcatcacgcgggtcatgccttcgcgaacgggcgtgcgtacggtggagagtttccatgctggtaacaaccacgcattgaacgccgcacatagcacaaatagaactgcccctgtggcgcagaccaggcgaaagtcgtattgcaacagccagctccccaacaatgcgccaatgaccgcaccggcactgtcctgcatcatcaacagcgagaaaaaacgaccacgctgctgtggacggattaatttcaccaccagcgccgaacgcggcggatcaaacaacgtgccaccgagtcccgagagcaggcatgaaaaccacaatagccacggttcgtgggcgatacccattgtggcgaatccggcggcgcgcatcagcataccggtaacaatcatcggtttggcaccaaagcggtcggcaattgcaccgccgaaaatacccagaccttgctgaataaattggcgtagaccgagagcaataccgaccatgacggcggcccagcccatttgatcaacgaagcggatagagatcagcgggaagacaacaaagaaccccagcacgaccagcatattatcgatgagcaggaaatatttacccaggttcctcgcctgcgacacgcgggacatttcccctcccgggaaataaaagatgagcactttctattctgcattgccgctaagacttttcccatcacttcggggacaatatttttttatcaaaacgtcgctttgatagagagtttttatcaaatatgtgaataatgcagaaaatggcattttggacttttcacagggtctggttgcgcaggtatagtaatacttacagcgtattaaagacgttacgggaaggagtaggtatagaatgtttggctatcgcagtaacgtgccaaaagtgcgcttaaccacagaccgactggtcgtgcgtctggtgcatgatcgtgatgcctggcgtcttgcggattattacgcagagaatcgccatttcctcaagccctgggagccagtgcgcgacgaaagccactgttatccatcaggctggcaggccaggctggggatgattaacgaatttcataaacaaggttcagctttctactttggcttattcgacccggacgaaaaagagattattggcgttgccaatttttccaatgttgttcgtggctcttttcatgcctgctatctcggttattcgattgggcaaaaatggcagggcaaaggactcatgtttgaagccctgaccgcagccattcgttatatgcagcgcacccaacatattcatcgcattatggctaattatatgccgcacaataaacgcagcggtgatttactggcgcgactgggttttgaaaaagaaggctatgcgaaagactatctgttgattgatggacaatggcgcgatcacgtactgacggcattaactaccccagactggacgcccggccgctaaggagaatctcatgaaatatcaacttactgcccttgaagctcgcgtgattggttgcttgctggaaaagcaggtgaccacgccggagcaatacccgctctcagtcaatggtgtagtcacggcctgtaatcagaaaacgaaccgtgaaccggtcatgaatctgagtgaatccgaagtgcaggaacagctggataatctggtcaaacgtcattatctacgcacagtgagcggttttggtaatcgggtcaccaaatatgagcaacgtttttgtaattcagaatttggcgatctgaaactgagcgcagcggaagtggcgttaatcaccacgttgttattgcgtggtgcccagacgccaggtgaactgcgcagccgcgccgcgcgaatgtatgaattcagcgatatggcggaagtggagtcgacgctggaacaactggcaaatcgcgaagatggtccttttgtggtgcgtctggcccgcgaaccgggtaaacgcgaaaaccgctacatgcatcttttcagtggtgaggttgaagatcagccggcggtgacggatatgtcgaacgcggttgacggtgatttacaggcccgcgtcgaagccctggaaatcgaagtggcagaactgaaacagcgtcttgattcgttgctggcccatctgggagattaaagtgaaaaaattacgtatcggcgtagtgggattaggtggcattgcgcaaaaagcgtggttaccggtgctggcggcagcgtctgactggacgttacaaggagcctggtcgcctacgcgcgcgaaagccctgccaatttgtgaaagctggcgcattccttatgccgattcgttatccagccttgccgccagttgcgatgcggtttttgtgcattccagcaccgccagccactttgacgtggtcagtacgttactcaatgcgggggtacatgtctgtgtcgataaaccgctggcagaaaatctgcgcgatgctgaacggctggtggaactggcggcgcggaaaaaactgacgttgatggtcggttttaaccgtcgtttcgcaccactctacggtgagttaaaaacgcaactcgccaccgcagcctcgctaagaatggataaacatcgtagcaatagcgtcgggccacacgatctttatttcacgttgctggatgattatctgcatgtggtggataccgcgctgtggttgtcgggcggcaaagcctctctggatggcggtacgctactgactaacgacgctggcgaaatgctgtttgccgagcaccatttttcggctggtcctttgcagatcaccacctgtatgcatcgccgtgccggaagtcagcgtgaaaccgtgcaggccgtgactgacggtgcgctcatcgacattacggatatgcgcgaatggcgtgaggagcgcgggcagggcgtagtgcataaaccgattcctggttggcagagtacgcttgagcaacgtgggtttgtcggctgtgcgcggcacttcattgaatgtgtgcaaaaccagacagttccgcaaaccgccggcgaacaggccgtgctggcgcaacgtatcgttgacaagatctggcgcgatgcgatgagtgaataaaccctgtaacatctggcggtagcaattcaccataatccaggtagactattcgcctctttcagcgcctgccttgcaggcgttttgcccgtgggtctggattagaacaccgatgaatttattaaaatcgctggccgccgtcagctcgatgaccatgttttcgcgtgtgcttggcttcgcacgagacgcaattgtcgccagaatctttggcgcagggatggcaaccgacgcctttttcgtcgcttttaaacttcctaacttgttacgccgtatctttgccgaaggggcattttcccaggcatttgtaccgattctggcggaatataaaagtaagcagggtgaagacgccacgcgggtctttgtctcttatgtttctggcctgctgacacttgcgctggcggttgtgacggtcgctggcatgctcgccgcaccgtgggtgatcatggtgaccgcgccaggcttcgctgacacagctgacaaatttgccctgaccagccagctactaaagattacctttccctatatcttgctgatctccctggcgtcgctggtgggagcgattctgaatacgtggaaccgcttctcgattccggcgtttgctccaacactgcttaacatcagcatgattggtttcgcgctgtttgccgcaccgtactttaacccaccggtgctggcgctggcgtgggctgttacggtcggcggcgtcctgcagctggtgtatcagctaccgcacctgaagaagatcggcatgctggtcctgccgcgcattaacttccacgatgccggagcaatgcgcgtggtgaaacagatgggaccggcgatccttggcgtctctgtgagccagatctccttaatcatcaacaccatttttgcctcgtttcttgcttccggttcggtgtcttggatgtattacgccgaccgcttaatggagtttccgtccggtgtgctgggcgtggcgcttggcaccattttgctgccgtcgctgtcgaaaagttttgccagtggcaatcatgatgaatacaaccgtttgatggactgggggttgcgtctttgtttcctgttggcgctgccgagtgcggttgcgttgggcattctttccggtccgttgaccgtttcgctgttccagtacggtaaatttaccgcgtttgatgcgctgatgacccagcgggcgttaattgcctactcggtgggtttgattggcctgattgtagtgaaagtgttggctcctggcttttattcccgccaggacattaaaacgccagtgaaaattgccatcgttacgctgattttaacgcaattgatgaacctggcgtttattggtccgttgaaacatgccgggctgtcactttctattggtctggcggcgtgtctgaatgcttcgctgctttactggcagttgcgtaagcagaaaatctttaccccgcaacccggctggatggcgtttctgttgcgtctggtggtggcggtactggtgatgtctggcgtgcttttaggtatgttacatatcatgccggagtggtcattgggtaccatgccctggcgtttactgcgtttaatggcggtcgtgctggcggggattgccgcgtacttcgctgcactggcggtactgggcttcaaagttaaagaatttgcccgccggacggtgtaacaatgcattccggcctgcagtgcaggccggagataatcttcagatcgaaatctttttaccgccgcgatgggttgttgaggtctgaccgttcgccccatatagcgtcggttcctgatgcggtttcaacatttccagcgcctgttgattgcgctcaatctgtccttccagtaaccagccgttatgttgattcatttggcgtagttgctgcgttttcacagtaatttcctgccagcgttgactaatatcaacgctatttgctgtattgggttctttcctgcgtaactgttcgaggtaatccagcgtcgccagcagtgagcttttttgttctgtaatccattgcaactggctgccgttgatctgccccatagagagatgttgctgctcttgatccattaccgttttgagatcgttaagcacagcggacatctggtcgaggatctctgcaagacgtgtcatacgatcagttactctgcaagtcttgctgcgcttcgttgatcagcgcatcggcaattttgccggtgtccatttttagttcaccgttacgaatcgccagttttaacgcttcgacacgttcaagattgatatcactgctgccgggttgcatcagttttgcttgcgcgtcgcttaacgtcacactggtgctggtggaggcggttgtttttgccgcccggctgttcgttaccggcgcgtcagtggtttcgcgcggttgaacggtgcttacaggcttcagaggcgaagtgcgatcaatactcatggtttattcctcattgagggcgcttttatcatgtgttgcttatttatcggcaagggacgggtaatctttaacagcttacaggtttataagaatattcccatctgcatcaacaacgccgctgactacctgtcccgataccatgcgcacccgcgcattctgtgcgacggctgcattgttcagcgcctgaccttctgcgttggcgctaaacccatcaccgctggcgatcacattgacgcgttgtcccgcttttacccgccatgcctggcgaaactgggttaactggataggttgatcgggtgatagatcgcgcaggctaatggcatcaacaagttgattgatatccagcaccgtacgcggtggcagggtatccagccgtccgcgtttcagtttgacattgccagcttccagctttcctccccgcgcaatgggcatcgcggcaaccacataatttcctgtggcctgtacattaacctgtaaatatcgtttgtcgttaccgcagcgtgccaacacattcacattgccccacaggcgggaattattgctcatcgaaagcaatggctgctcgcatggcggtagtagattgggcgctgtacgaatagaaacacgaacctcatcacttacccccgcgagttgggcgctaaaaaagttgtgcaattgcgatgtgagattgctcgccgtacttaacggactgaacagtatcgcgatgatcgccacgctacgttttattatcagcattttcgcccccagccatttctacaacgtgaattgtacctgtccgcaatgaccatcaacggcataaatagcgacccattttgcgtttattccgccgataacgcgcgcgtaaaggcatttaagctgatggcagaattttgatacctgcggaggagatatgctcgataagctcgacgccgccttacgttttcaacaagaggcgctcaatctgcgcgcccagcgtcaggaagtgctggcagcaaacatcgccaatgccgatacccctggttatcaggcgcgcgatatcgattttgccagtgaacttaaaaaagtcatgcaacgtggacgggatgcaaccagtgtggttgcactgacgatgacctcaacgcaacacattccggcgcaggcgctgacgcctcctaccgcagaactgcaataccgtattccggaccagccttcgcttgacggtaataccgtcgatatggatcgcgaacgcacccagtttgccgataacagcctgcaataccagatgagccttagcgcgttgagcgggcaaatcaaaggcatgatgaacgttttacagagcggaaattaacggatggcactgctgaatatttttgatatcgccgggtcggcgttaactgcccagtcccagcgcctgaacgtggcggccagtaatctggcgaatgctgatagcgtgaccggtcccgatggacagccatatcgggcaaaacaggtggtattccaggttaacgctgcaccaggtgctgcgacaggcggcgtaaaggttgccgatgttatagaaagtcaggccccggacaaactggtttatgaaccgggtaatccgctggcagatgcaaagggctacgtaaaaatgccgaacgttgatgttgtcggagagatggttaacaccatgtcggcgtcacgcagctatcaggccaatgttgaagtgctcaacacggtgaaaagcatgatgctgaaaacccttacgctcggtcaataaaggagaaagctatgtccattgcggtaaccaccaccgatccgacaaataccggcgtcagtaccaccagcagtagttcgctcacgggcagcaacgccgcagatttacaaagcagttttctgactttgctggtggcgcagctgaaaaaccaggacccgaccaatccaatggaaaacaacgagctgacgtcgcaattggcacaaatcagcacggtcagcgggattgaaaaactcaataccacgctcggatctatttccggacagattgataacagccagtcgttacaggccagtaacctgatcggtcacggcgtgatgatccccggcaccactgttcttgcgggaaccggcagtgaagaaggggctgtgaccacgaccacgccgtttggtgttgagctgcaacaggcggcagacaaagttacggccaccatcaccgataaaaatggcgcggttgtgcgcaccattgatattggtgaactgaccgccggagttcacagtttcacctgggacggtacgttgactgatggcagcactgcgccgaacggttcttacaatgtagcgattagcgccagtaacggtggtacacaactggttgcccagccgctgcagtttgctctggtgcagggtgtgatccgcggcaacagcggtaatacgctggatctcggcacttacggcaccaccaccctcgacgaagtacggcagataatttaagccttcacatttcaggagtcagtcatggccttttctcaagcggttagcggattaaacgctgccgccaccaacctcgatgttattggcaacaatatcgccaactccgccacctacggctttaaatcaggcacggcctcttttgccgatatgtttgccggttcgaaagtgggactgggggtaaaagttgccggtatcactcaggactttaccgatggcacgaccaccaacaccgggcgaggtctggacgttgctatcagccagaacggttttttccgtctggtagacagcaacggttcggtgttctacagccgtaacggacaatttaagctggatgaaaaccgtaacctggtgaatatgcaaggtttacagctgacgggttacccggcaaccggtacgccgccgactattcagcaaggggcgaatccgaccaatatttcgatcccgaataccctgatggcagcgaaaactaccaccacggcatcgatgcagatcaacctgaattccagtgatccgcttcctactgttacgccattcagcgccagcaatgcggatagctataacaaaaaaggttcggtgactgttttcgacagtcagggtaatgctcatgacatgagcgtctactttgtgaagaccggggataataactggcaggtctacacccaggatagcagtgatccaaacagcattgcgaagacagcgacaacactggaatttaatgctaatggcacattagtggatggtgcgatggcgaataatatcgcaaccggcgcaattaacggtgcagaacccgccacgtttagtctgagcttcctcaactccatgcagcaaaataccggcgctaacaatattgtggcaaccacccagaacggctacaaaccgggcgatctggtgagttatcaaatcaatgatgacggtacggttgtcggcaactattccaacgaacaaacccaactgctggggcagattgtactggcgaactttgccaacaacgaaggtctggcatccgaaggcgacaacgtctggtctgcgacgcaatcttctggcgtggcgctgttggggacagccgggacgggaaactttggcaccctgaccaacggtgcgctggaagcgtccaacgtcgatctcagtaaagaactggtcaatatgatcgttgcccagcgtaactatcagtctaacgcccagaccatcaaaacccaggaccagatcctcaacacgctggttaacttacgctaatcgctgacgggatagctcaatggatcacgcaatttataccgcgatgggagcagccagccagacactgaatcaacaggcggtaaccgccagtaatctggccaatgcctcaacgcccggttttcgcgcgcagttgaatgctttacgcgcggtgccagtggaagggctttctctgcccacgcgcacgttggtcacggcgtcaacgccgggcgcagatatgacgcccggcaaaatggattacacctcgcgcccgctggacgtcgcgttgcagcaggatggctggctggccgtgcagaccgctgacggcagcgaagggtatacgcgtaatggcagcattcaggttgatcccaccgggcaactgacaattcaggggcatccggtgataggcgaggctgggccaattgctgtgccggaaggggcggaaatcactattgctgccgatggcacaatctcggcgctcaatccgggcgatccggcaaatacggttgcgccagtagggcgtcttaaactggtgaaagccacgggcagcgaagtgcagcgcggtgacgacggcatttttcgtttaagcgcagaaacccaggccacgcgtgggccggtactgcaggcagatccaaccttgcgtgtgatgtcgggggttctggaaggcagtaacgtcaatgccgttgcggcaatgagcgacatgattgccagcgcgcggcgttttgaaatgcagatgaaggtgatcagcagcgtcgatgataacgcaggccgtgccaaccaactgctgtcgatgagttaattgaaaggatacatgacaagtataagttgcccgatgcgcaagtttatcgggtctatgggggcaatcgcaatttatcgattttgcgagcacttgtaggccggataaggcgtttacgccgcatccggcaagaagacatatgcactttgtcactaatccactacaggacattttatgatcagttcattatggatcgccaaaacgggccttgacgcccagcaaaccaatatggacgtcattgccaacaacctggcaaacgtcagtactaacggttttaagcgtcagcgcgcggtgtttgaagatctgctttatcaaaccattcgccagccgggggcacagtcttccgaacaaaccaccttaccctccggattacaaatcggcacgggggtacgcccggtcgccactgaacgcttacacagccagggaaacctgtcgcagaccaacaacagcaaagatgtcgcgattaaagggcagggctttttccaggtgatgttgccagatggttcatcagcctatacccgtgacggctctttccaggtggatcagaacgggcagctggtgacggctggtggttttcaggtgcagccagcgatcaccattccggcgaatgcgttaagtatcaccatcggtcgtgatggcgtggtcagcgtaacccaacaaggccaggcagctccggttcaggttgggcagctcaatctcaccacctttatgaatgacaccgggctggagagcattggcgaaaacctctacaccgaaacgcaatcctctggtgcaccgaacgaaagcacgccgggcctgaacggcgcgggactgctgtatcaagggtatgttgaaacgtctaacgtcaacgtggcggaagaactggtcaatatgattcaggtgcaacgcgcttacgaaatcaacagtaaagcggtgtccaccaccgatcagatgctgcaaaaactgacgcaactctaaggcttaaccggtggcaggttcaccggtttactgatttttgaagatgatagccatgcaaaaaaacgctgcgcatacttatgccatttccagcttgttggtgctttcactaaccggctgcgcctggataccctccacgccgctggtgcagggggcgaccagtgcacaaccggttcccggtccgacgcccgtcgccaacggttctattttccagtctgctcagccgattaactatggctatcaaccgctgtttgaagatcgtcgaccacgcaatattggcgatacgctgaccatcgtgttgcaggagaacgtcagcgccagcaaaagctcctctgcgaatgccagccgtgacggtaaaactaattttggctttgatactgtgccgcgctatttgcaggggctgtttggtaacgctcgtgccgatgtcgaagcctccggtggtaacacgttcaacggaaagggcggggccaatgccagcaatacctttagcggcacgttgacggtgacggttgaccaggtactggtcaacggcaacctgcatgtggtgggtgaaaaacagattgccattaatcagggtaccgaatttattcgcttctctggcgtggttaatccacgcactatcagcggcagcaataccgtaccgtctactcaggtggcggatgcgcgcattgaatacgtaggcaatggctacattaacgaagcgcaaaatatgggctggttgcagcgtttcttccttaacctgtcgccaatgtaagtgaggctgtggtgattaaatttctctctgcattaattcttctactggtcacgacggcggctcaggctgagcgtattcgcgatctcaccagtgttcagggggtaaggcaaaactcactgattggctatggtctggtggtggggctggatggcaccggtgaccagacaacccagacgccgtttaccacacaaacgcttaataacatgctctcacagctgggaattaccgttccgacgggcaccaatatgcagctaaaaaacgtcgctgcggtaatggtgacagcgtcacttcctccgtttggacgtcaggggcaaaccatcgatgtggtggtttcttccatgggaaatgccaaaagcttgcgtggaggtacgttgttgatgacaccgcttaagggcgttgacagtcaggtgtatgcgctggcgcagggcaatattctggttggcggcgcaggagcctccgctggcggtagcagtgttcaggttaaccaactgaacggtggacggatcaccaatggtgcggttattgaacgtgaattgcccagccagtttggcgtcgggaatacccttaatttgcaacttaacgacgaagatttcagcatggcgcagcaaatcgctgacaccatcaaccgcgtgcgtggatatggcagcgccaccgcgttagatgcgcggactattcaggtgcgcgtaccgagtggcaacagttcccaggtccgcttccttgccgatattcagaatatgcaggttaatgtcaccccgcaggacgctaaagtagtgattaactcgcgcaccggttcggtggtgatgaatcgcgaagtgaccctcgacagctgcgcggtagcgcaggggaatctctcagtaacagttaatcgtcaggccaatgtcagccagccagatacaccgtttggtggtggacagactgtggttactccacaaacgcagatcgatttacgccagagcggcggttcgctgcaaagcgtacgttccagcgccagcctcaataacgtggtgcgcgcgctcaatgcgctgggcgctacgccgatggatctgatgtccatactgcaatcaatgcaaagtgcgggatgtctgcgggcaaaactggaaatcatctgatgatcagcgacagcaaactactggcaagtgcggcctgggatgcgcaatcactcaacgaactaaaggcgaaagcgggcgaagatccggcggcaaatatccgtccggtggcccgtcaggtggaagggatgttcgtgcagatgatgttgaaaagcatgcgcgacgctttaccaaaagatggcctgttcagcagcgagcacactcgcctgtataccagtatgtatgaccagcagattgcccaacagatgacggcgggcaaaggtctggggcttgcagagatgatggttaaacagatgacgccagaacaaccattgccagaggagtccacgccagcagcaccgatgaaattcccgctcgaaactgtggtgcgttatcaaaatcaggcgctttcgcagctggtgcaaaaggccgtgccacgtaactacgatgattcgctgccgggtgacagtaaagcattcctcgcgcaactctcgctgcccgcccaactggcaagccagcaaagcggtgtgccacatcatttgatcctcgctcaggcggcactggaatctggttgggggcaacggcaaatccgccgcgaaaacggcgagccgagctataacctgtttggtgtcaaagcctctggcaactggaaagggccagttactgaaatcaccacgactgaatatgaaaacggcgaagcgaagaaagtaaaagcgaagtttcgcgtctacagctcgtatctggaagccttgtcggattacgttgggctgttaacgcgtaacccgcgctacgccgccgtgacgaccgccgcgagtgcggaacagggggcgcaggccctacaggacgcgggctatgccaccgatcctcactatgcccgcaaactcaccaacatgattcagcagatgaaatcgataagcgacaaggtgagcaaaacctacagtatgaacattgataatctgttctgaataactcaagtccggcgggtcgctgccgataatactctgtaattgaaggcttataaggaacctccatgtccagcttgattaataacgccatgagcggactgaacgcggcccaggcggcgttaaatacggcaagtaataatatctccagctataacgttgccggatatacccgccaaaccactattatggcgcaggccaatagcacgttgggcgctggcggctgggttggcaatggtgtctacgtttctggtgtgcagcgtgagtatgatgcgtttattaccaaccagttacgtgcggcgcagacgcaaagtagcggtctgactgcccgctatgagcagatgtcgaaaatcgacaatatgctctccaccagtacctcttcgctggcaacacagatgcaggatttcttcaccagcctgcaaacgctggtgagtaacgcggaagacccggcagcgcgccaggcgctgattgggaaatcagaaggattggtgaatcagtttaaaaccaccgatcaatatctgcgcgaccaggacaaacaggtcaatatcgcgataggtgccagcgttgatcagatcaacaactacgctaaacaaattgccagcctgaacgatcaaatctcgcgcctgacaggcgtgggggcaggggcgtcacctaacaatctgctggatcaacgcgatcaactggtgagcgaattaaaccagattgttggtgtagaagtcagcgttcaggatggcggcacttataacatcacgatggccaatggttactcactggttcagggaagtacggcgcggcaactggcggcagttccttccagcgctgacccttctcgtacgactgtcgcttatgttgatgggacggcaggcaatattgagatcccggagaaattactgaataccgggtcgctgggcggcattctgacattccgttctcaggatctggaccagacgcgtaatacgcttggacaactggcgctggcatttgccgaggctttcaacacccaacacaaagccggatttgatgctaacggcgatgccggtgaagatttctttgctatcggtaagcccgcggttctgcaaaacacgaaaaacaaaggtgacgttgcgatcggtgccacggtaactgatgcctccgcggtactggcgacagattacaaaatctcgttcgataataatcagtggcaggtcacccgccttgccagcaataccacttttacggtgacgccggatgccaacggtaaagtggcatttgatggtctggagttgacgtttacaggaacgcctgccgttaacgacagcttcacgctgaaaccagtaagtgacgccatcgtcaacatggatgtattaatcaccgacgaagcgaaaatagcgatggcgagcgaagaagatgcgggtgatagcgataaccgcaacggtcaggccctgctggatctgcaaagcaacagtaaaacggtgggcggtgcgaaatcctttaacgacgcttatgcctcgttagtgagtgatatcggtaataaaaccgcgacgttgaaaaccagtagcgccacgcaaggtaatgtggtgacgcagctttccaatcagcagcagtcgatttccggtgtcaatctcgatgaggagtacggaaatctgcaacgttttcagcagtattacctggcgaatgcgcaggttctgcagacggcaaacgcgatttttgatgcgctgattaacattcgctaaggggagataagatgcgtttcagtacacagatgatgtaccagcaaaacatgcgtggtatcaccaattctcaggcagaatggatgaagtacggcgaacagatgtcgacgggtaagcgagtcgttaacccttctgacgatcccattgctgcatcacaagccgtagttctctcccaggcacaggcgcaaaacagccagtacacgctggcgcgtactttcgccactcaaaaagtgtcactggaagagagtgtacttagccaggtcaccactgctatccagaatgctcaggaaaaaattgtctacgccagcaatggcaccttgagtgacgatgaccgggcctcgctggctacggatattcaggggcttcgtgaccagttgctgaatctggcaaacaccactgacggtaacgggcgctacatttttgccggttataaaacagagactgcgccgtttagcgaagagaaagggaaatacgtcggtggagcagaaagtattaaacaacaggtcgatgcttcgcgttcgatggtgatagggcacacgggtgacaaaattttcgacagtattaccagcaacgcggtagcggaaccagacggtagcgcttctgaaaccaatctttttgccatgctggatagtgccatcgcagccctgaaaacgccggtcgcggatagcgaagcggataaagaaaccgccgctgcggcgttagataaaaccaaccgcggactgaaaaactcgctgaacaatgtgctgactgttcgcgcggaattaggcacgcagctgaacgaactggagtcgctggattcattaggtagcgatcgcgctttagggcaaacgcagcagatgagcgatctggttgatgtggactggaatgcaactatttcatcttacatcatgcagcaaacggcattgcaggcatcgtataaagcatttaccgatatgcagggattgtcgctcttccagctcagcaaataatttcgctttaaaacatatcatgaaactgggtatgttttgtctgcctgctctgggatcgctggggcgggcatttttttgcctattttgcattgttggttagcaaggatgccattcgatgaattttaatatgttgattcaaagatgaaataaaaaagccctggcagttaccagggcttgattactttgagctaattattactcaacaggttgcggacgcgcaggagcggcagaggcatgatgtgttgccgtatgaccacctgcggcacctttaccttcgaaggcaaaagtagggcgctgccagtcactgtgacgcggtgcctccggaacatattccggtgctggagcgcgcgtcattggcgcggtagcgtggttatgctcaacggtgacctcaggttcgaccgcagctaccgtttcaacttctgctgcgacttcagcgactactggcgcggcaggttgagcaacaacttcaggttcagcaactacaacctcagcagtttcgacaacttcttcaatatctgccgtctcttcctgcggttcaaccaccggttctgcttgttctgcaacttcctgggctacggcaacatcagactcggtaatcacctgcggctgttcagttaccgcggcagcgatcacttcaggatgcgtcgtttcaaccacttccggttgcggttcggcaacctgaacgggggcttctacgacaccggccacttcttcaacaactggcgcgctaacaaccggttcgatagcggcggcgacagggacctcagtcaccatcggctgcacatgtacttcttcctgttcgcgctgctcttcaacctgtacatcttgcggacgtacaattggatagcggatccagactttgccagaggccagttccggagacgcgcacgctacggtcaacggcattggcgactgggttggataacgctcgtcacgatagcgacgacgacgctgaccacttacgcgcaggtgacgaggcgagcggcgagaacgacgcggcatgccaccgttgtcacggttatcagcattgttctcttcttgctgttctggtgcagtttgcgctacgactggcagcgggactttcaccagttctgtgcgtggagctggcgcttcctgaacaattggttcggcagcgacagtttcttcaaccaccggtgcgactaccgcttcttcggctacgctttgctcgtaacgcactttctgattgagctgacgctgtttacgacgcggctgaaccggacgtacacgttcttcctgttcggtttcctgaacagattgctcttcaacattcagcgccttcgcttcttgttgcgcctgacgtttatcatcattacggcggcggctacgttcacgacgcggcgcttgctgctcgtcggcggtacgcgctttttccgttacctcagcctgctgacggctctcacgcgtctcggcagtctgctgctgtgcctggcgacgattacgacggttttcttcgcgattatcgctgccttcagtacgttcactacgggtgtcgcggcgctcattacggtcacggcggttgttctgacgaggcttgcgacgatcctgttgacgttccggtttcgcttctgctttcggtgctggttgctcggtcggtttggtttcttcaccaccgctgaacagcgctttcagtgcgccgaagaagcggctcaacagcccaggttgtgcaggagctgctggtgttgccggtgcagctttcggtgctggagctacaacaggcgcggcaggttcagctggcgttggcgcaggcggcacatccggcatggcaaaggttgccagcgcaggttgttccggacgcttacgttcagcgaactcttcttcagacggcagcgccatcgcttcttcatgcagcttcggcagcatgtagcttaaggttggggtttcttcccctttacgcacgcgcagcacgtggtagtgcggggtttccatctgatcgtttggcacaattacacagcgcacaccgtcctgacgagtttcaatggcatttaccgcagaacgtttttcattcagcaggtaagaagcgattggcacaggaacaatggcgtgaacttcctgggtgttctctttcagcgcttcttcttcgatcagacgcagaatagagagcgacagcgattcgttgtcacgcacggtgccagtaccagaacaacgcggacaaacgtgatgactggattcacccagtgatgggctcaggcgctgacgggacatttccagcaggccaaagcgagaaatatggctgatttgaatacgcgcacggtcctgacgcaccgcttcacgcagacggttttctaccgcacgctggtggcgtactggcgtcatgtcgatgaagtcgataacaatcaggccgccgaggtcacgcaggcgcagctgacgagcaatctcatcggcagcttcgaggttagtgttaaacgcggtttcttcgatatcgccgccgcgggtcgcgcgtgcggagttgatgtcgatggccgttaacgcttcggtgctgtcgataacaatggaaccaccagacggcagacgaacttcacgctggaaggcggactcgatctgtgactcgatctggtagtggctgaacagcgggatctcgccggtgtacagtttgattttgctgctgaaatccgggcgacctaatgcagcgatatgctgacgtgccagttcgagcactttcgggttatcgataaggatttcgccgatgtcctgacgtaagtaatcgcggaatgcgcgaacgattacgttgctctcctgatgaatcaggaacggggccgggcggctttcagcggcttttttgatggcttcccagtgtttcagacggaagcttaaatcccattgcagcgcctcagcagatttgccgacgccagcggtgcgcacgataagccccatgccttccggcagttcaaggcttgccagtgcttcttttaattcggtacggtcgtcgccttcgatacggcgagaaatgccacccgcgcgcgggttgttcggcatcagaaccagatagctacccgccagactgataaaggtggttaatgccgcgcctttgttgccgcgctcttctttatcgatctgaacaatgacttcctgaccttcacgcaacacatctttaatgttgggacgaccatgagcactgtagttagcagggaaatattcgcgggcaatttcttttagtgggaggaaaccgtgacgttcagcgccgtaatcaacaaaagcagcttccagactcggttcaatgcgggtgattttacctttgtagatgtttgcctttttctgctcgtgccctggactttcgatatccaggtcatacagacgctgcccatctacaagggcaacgcgcaactcttcctgctgagttgcgttgattaacattcttttcatcgtaacttactcattattcttacattgacgactaagctgcgggcaaagtaacgcctttccgggtgtgaaccgatggcctcgtgtctagtcgcgtcgccaacctcacggttatcgtcagctcaaagaggcgcagagtgtcggttgcccgtttttcatgcggaaaaacagcgcaattatcaaagaaacagactgggtattactctccagaaatatttccatctaccggtaaggactgcaacccgcagcccgctaactgcctgaaagatcaatacgtcttacgccattgctgcgtggatgatcggtcgggcaaaatgggttattccgtaaaatttcttgttttaacaaggatggacacggaaacggcctcattattccactgcaagccttgttatagcaagatgacttttaccatttatcacccgcttactcacagttttttcacttcttgctggtgattggtttaataaccatcaataaagtgatcacgcagtgaagtaataaggtgcaaaagtaaatataagcatagaaaaatgagtggcgcgaatcctgttggctaattagaatcgccaaccatgaaaacagagactccatccgtaaaaattgttgctatcaccgctgacgaagcggggcaacgtatcgataactttttgcgtacccaattgaaaggcgtaccaaaaagtatgatttaccgtattttgcgtaaaggcgaagtgcgggtgaacaaaaaacgtattaagcctgaatataaactcgaagcgggtgatgaggtgcgtattccaccggttcgcgttgctgagcgggaagaagaggcggtttcgccacatctgcaaaaggtggcggcgctggcggacgtcatcttatatgaagatgatcacatcctggtgctgaataaaccttccggtacggcggtacatggcggcagtggtttaagcttcggcgttattgaaggtttgcgggcgttgcgcccggaagcgcggttccttgaactggttcatcgtcttgaccgggacacctcaggtgttttgctggtagcgaaaaaacgctcggcgttgcgttctctgcatgagcaattacgtgaaaaagggatgcaaaaagattacctggcgctggtgcgcggtcagtggcagtcgcatgtgaagagcgttcaagcaccgttactgaaaaatattctgcaaagcggcgaacgtatcgtgcgtgtgagtcaggaaggcaaaccgtcggaaacacgctttaaagtggaagaacgctatgcatttgccaccctggtgcgttgtagcccggtaacagggcgtactcaccagatccgtgtgcatacacaatatgcgggtcatccgattgcctttgacgatcgctacggtgaccgtgaatttgacaggcagctcactgaagcaggcacgggattaaatcgcctgttcctgcacgctgcagcgttgaagtttactcatccggggaccggtgaggtgatgcgtatcgaagctccgatggatgaaggtttgaagcgttgtttgcaaaagctgcgtaacgcgcgctaatacaagcatataaacctgataatgggcggttggcctgataaggcgtttacgccgcatcaggccgccagcaccgattgccggatgcgacgtaaccacatccggcgcaaaaaactatcccatcagcgggtttttcccttcccgacgtaacatctgacacagcgcgattagcggtaaaccaaccagcgtgttaggatcacgcccctctaaacgctcaaacagcgtaatgccaaatccttcactcttaaagctacccgcgcagtgcaggggatgctctttacgcacgtaattatcaatctccgcctcgctcaggtgacggaaatggacgtcaaaaggctccacttctgtttgcagatgcccattcgccgaattaaacaacgccagtccagtatagaaggtgacgatattgccgctggctttgcgtaattgcagacgggcattttcttccgttaacggtttaccggtgatttcgccatcaagaacacatacctggtctgaaccaataattaaatgatccggataacgtgacgccagagattgcgctttttcttgtgccagtcgaagcaccaactgtcgcggtgattcgtcgctgcgtggggtttcgtcgacctctggtgctgcacattcaaaagagatttgcagtttttccagaagagcgcgacgccatggcgaggtggaggctaaaataagtttaggcatatttttttccatcagatatagcgtattgatgatagccattttaaactatgcgcttcgttttgcaggttgatgtttgttatcagcactgaacgaaaataaagcagtaacccgcaatgtgtgcgaattattggcaaaaggcaaccacaggctgcctttttctttgactctatgacgttacaaagttaatatgcgcgccctatgcaaaaggtaaaattacccctgactctcgatccggttcgtacggctcaaaaacgccttgattaccagggtatctatacccctgatcaggttgagcgcgtcgccgaatccgtagtcagtgtggacagtgatgtggaatgctccatgtcgttcgctatcgataaccaacgtctcgcagtgttaaacggcgatgcgaaggtgacggtaacgctcgagtgtcagcgttgcgggaagccgtttactcatcaggtctacacaacgtattgttttagtcctgtgcgttcagacgaacaggctgaagcactgccggaagcgtatgaaccgattgaggttaacgaattcggtgaaatcgatctgcttgcaatggttgaagatgaaatcatcctcgccttgccggtagttccggtgcatgattctgaacactgtgaagtgtccgaagcggacatggtctttggtgaactgcctgaagaagcgcaaaagccaaacccatttgccgtattagccagcttaaagcgtaagtaattggtgctccccgttggatcggggataaaccgtaattgaggagtaaggtccatggccgtacaacagaataaaccaacccgttccaaacgtggcatgcgtcgttcccatgacgcgctgaccgcagtcaccagcctgtctgtagacaaaacttctggtgaaaaacacctgcgtcaccacatcactgccgacggttactaccgcggccgcaaggtcatcgctaagtaatcacgcatctgcgtgatgaagcttagtgaggattttccccaggcaactggggaaagaccaaaccgggcggcgacgataccttgacacgtctaaccctggcgttagatgtcatgggaggggattttggcccttccgtgacagtgcctgcagcattgcaggcactgaattctaattcgcaactcactcttcttttagtcggcaattccgacgccatcacgccattacttgctaaagctgactttgaacaacgttcgcgtctgcagattattcctgcgcagtcagttatcgccagtgatgcccggccttcgcaagctatccgcgccagtcgtgggagttcaatgcgcgtggccctggagctggtgaaagaaggtcgagcgcaagcctgtgtcagtgccggtaataccggggcgctgatggggctggcaaaattattactcaagcccctggaggggattgagcgtccggcgctggtgacggtattaccacatcagcaaaagggcaaaacggtggtccttgacttaggggccaacgtcgattgtgacagcacaatgctggtgcaatttgccattatgggctcagttctggctgaagaggtggtggaaattcccaatcctcgcgtggcgttgctcaatattggtgaagaagaagtaaagggtctcgacagtattcgggatgcctcagcggtgcttaaaacaatcccttctatcaattatatcggctatcttgaagccaatgagttgttaactggcaagacagatgtgctggtttgtgacggctttacaggaaatgtcacattaaagacgatggaaggtgttgtcaggatgttcctttctctgctgaaatctcagggtgaagggaaaaaacggtcgtggtggctactgttattaaagcgttggctacaaaagagcctgacgaggcgattcagtcacctcaaccccgaccagtataacggcgcctgtctgttaggattgcgcggcacggtgataaaaagtcatggtgcagccaatcagcgagcttttgcggtcgcgattgaacaggcagtgcaggcggtgcagcgacaagttcctcagcgaattgccgctcgcctggaatctgtatacccagctggttttgagctgctggacggtggcaaaagcggaactctgcggtagcaggacgctgccagcgaactcgcagtttgcaagtgacggtatataaccgaaaagtgactgagcgtacatgtatacgaagattattggtactggcagctatctgcccgaacaagtgcggacaaacgccgatttggaaaaaatggtggacacctctgacgagtggattgtcactcgtaccggtatccgcgaacgccacattgccgcgccaaacgaaaccgtttcaaccatgggctttgaagcggcgacacgcgcaattgagatggcgggcattgagaaagaccagattggcctgatcgttgtggcaacgacttctgctacgcacgctttcccgagcgcagcttgtcagattcaaagcatgttgggcattaaaggttgcccggcatttgacgttgcagcagcctgcgcaggtttcacctatgcattaagcgtagccgatcaatacgtgaaatctggggcggtgaagtatgctctggtcgtcggttccgatgtactggcgcgcacctgcgatccaaccgatcgtgggactattattatttttggcgatggcgcgggcgctgcggtgctggctgcctctgaagagccgggaatcatttccacccatctgcatgccgacggtagttatggtgaattgctgacgctgccaaacgccgaccgcgtgaatccagagaattcaattcatctgacgatggcgggcaacgaagtcttcaaggttgcggtaacggaactggcgcacatcgttgatgagacgctggcggcgaataatcttgaccgttctcaactggactggctggttccgcatcaggctaacctgcgtattatcagtgcaacggcgaaaaaactcggtatgtctatggataatgtcgtggtgacgctggatcgccacggtaatacctctgcggcctctgtcccgtgcgcgctggatgaagctgtacgcgacgggcgcattaagccggggcagttggttctgcttgaagcctttggcggtggattcacctggggctccgcgctggttcgtttctaggataaggattaaaacatgacgcaatttgcatttgtgttccctggacagggttctcaaaccgttggaatgctggctgatatggcggcgagctatccaattgtcgaagaaacgtttgctgaagcttctgcggcgctgggctacgacctgtgggcgctgacccagcaggggccagctgaagaactgaataaaacctggcaaactcagcctgcgctgttgactgcatctgttgcgctgtatcgcgtatggcagcagcagggcggtaaagcaccggcaatgatggccggtcacagcctgggggaatactccgcgctggtttgcgctggtgtgattgatttcgctgatgcggtgcgtctggttgagatgcgcggcaagttcatgcaagaagccgtaccggaaggcacgggcgctatggcggcaatcatcggtctggatgatgcgtctattgcgaaagcgtgtgaagaagctgcagaaggtcaggtcgtttctccggtaaactttaactctccgggacaggtggttattgccggtcataaagaagcggttgagcgtgctggcgctgcctgtaaagcggcgggcgcaaaacgcgcgctgccgttaccagtgagcgtaccgtctcactgtgcgctgatgaaaccagcagccgacaaactggcagtagaattagcgaaaatcacctttaacgcaccaacagttcctgttgtgaataacgttgatgtgaaatgcgaaaccaatggtgatgccatccgtgacgcactggtacgtcagttgtataacccggttcagtggacgaagtctgttgagtacatggcagcgcaaggcgtagaacatctctatgaagtcggcccgggcaaagtgcttactggcctgacgaaacgcattgtcgacaccctgaccgcctcggcgctgaacgaaccttcagcgatggcagcggcgctcgagctttaaaagaggaaaatcatgaattttgaaggaaaaatcgcactggtaaccggtgcaagccgcggaattggccgcgcaattgctgaaacgctcgcagcccgtggcgcgaaagttattggcactgcgaccagtgaaaatggcgctcaggcgatcagtgattatttaggtgccaacggcaaaggtctgatgttgaatgtgaccgacccggcatctatcgaatctgttctggaaaaaattcgcgcagaatttggtgaagtggatatcctggtcaataatgccggtatcactcgtgataacctgttaatgcgaatgaaagatgaagagtggaacgatattatcgaaaccaacctttcatctgttttccgtctgtcaaaagcggtaatgcgcgctatgatgaaaaagcgtcatggtcgtattatcactatcggttctgtggttggtaccatgggaaatggcggtcaggccaactacgctgcggcgaaagcgggcttgatcggcttcagtaaatcactggcgcgcgaagttgcgtcacgcggtattactgtaaacgttgttgctccgggctttattgaaacggacatgacacgtgcgctgagcgatgaccagcgtgcgggtatcctggcgcaggttcctgcgggtcgcctcggcggcgcacaggaaatcgccaacgcggttgcattcctggcatccgacgaagcagcttacatcacgggtgaaactttgcatgtgaacggcgggatgtacatggtctgaccgcgatttgcacaaaatgctcatgttgcgcgcagtctgcgtggttatgagtaataattagtgcaaaatgatttgcgttattggggggtaaggcctcaaaataacgtaaaatcgtggtaagacctgccgggatttagttgcaaatttttcaacattttatacactacgaaaaccatcgcgaaagcgagttttgataggaaatttaagagtatgagcactatcgaagaacgcgttaagaaaattatcggcgaacagctgggcgttaagcaggaagaagttaccaacaatgcttctttcgttgaagacctgggcgcggattctcttgacaccgttgagctggtaatggctctggaagaagagtttgatactgagattccggacgaagaagctgagaaaatcaccaccgttcaggctgccattgattacatcaacggccaccaggcgtaagtgaacatctccaggcggtcgttcgaccgcctgagttttatctttttgtcccactagaatcattttttccctccctggaggacaaacgtgtctaagcgtcgtgtagttgtgaccggactgggcatgttgtctcctgtcggcaataccgtagagtctacctggaaagctctgcttgccggtcagagtggcatcagcctaatcgaccatttcgatactagcgcctatgcaacgaaatttgctggcttagtaaaggattttaactgtgaggacattatctcgcgcaaagaacagcgcaagatggatgccttcattcaatatggaattgtcgctggcgttcaggccatgcaggattctggccttgaaataacggaagagaacgcaacccgcattggtgccgcaattggctccgggattggcggcctcggactgatcgaagaaaaccacacatctctgatgaacggtggtccacgtaagatcagcccattcttcgttccgtcaacgattgtgaacatggtggcaggtcatctgactatcatgtatggcctgcgtggcccgagcatctctatcgcgactgcctgtacttccggcgtgcacaacattggccatgctgcgcgtattatcgcgtatggcgatgctgacgtgatggttgcaggtggcgcagagaaagccagtacgccgctgggcgttggtggttttggcgcggcacgtgcattatctacccgcaatgataacccgcaagcggcgagccgcccgtgggataaagagcgtgatggtttcgtactgggcgatggtgccggtatgctggtacttgaagagtacgaacacgcgaaaaaacgcggtgcgaaaatttacgctgaactcgtcggctttggtatgagcagcgatgcttatcatatgacgtcaccgccagaaaatggcgcaggcgcagctctggcgatggcaaatgctctgcgtgatgcaggcattgaagcgagtcagattggctacgttaacgcgcacggtacttctacgccggctggcgataaagctgaagcgcaggcggtgaaaaccatcttcggtgaagctgcaagccgtgtgttggtaagctccacgaaatctatgaccggtcacctgttaggtgcggcgggtgcagtagaatctatctactccatcctggcgctgcgcgatcaggctgttccgccaaccatcaacctggataacccggatgaaggttgcgatctggatttcgtaccgcacgaagcgcgtcaggttagcggaatggaatacactctgtgtaactccttcggcttcggtggcactaatggttctttgatctttaaaaagatctaagttgtcattttccacccttataaaaggtccgcttgcgggccttttttcttagcttttattccgacttgttccgtagtgaacatgctgccacactaacaattctctgataaggagccggtatgttcttaattaacggtcataagcaggaatcgctggcagtaagcgatcgggcaacgcagtttggtgatggttgttttaccaccgccagagttatcgacggtaaagtcagtttgttatcggcgcatatccagcgactacaggatgcttgtcagcggttgatgatttcctgtgacttctggcctcagcttgaacaagagatgaaaacgctggcagcagaacagcaaaatggtgtgctgaaagtcgtgatcagtcgcggtagtggcgggcgagggtacagcacattgaacagcggaccggcaacgcggattctctccgttacggcttatcctgcacattacgaccgtttgcgtaacgaggggattacgttggcgctaagcccggtgcggctggggcgcaatcctcatcttgcaggtattaaacatctcaatcgtcttgagcaagtattgattcgctctcatcttgagcagacaaacgctgatgaggcgctggtccttgacagcgaagggtgggttacggaatgctgtgcggctaatttgttctggcggaagggcaacgtagtttatacgccgcgactggatcaggcaggtgttaacggcattatgcgacaattctgtatccgtttgctggcacaatcctcttatcagcttgtcgaagtgcaagcctctctggaagagtcgttgcaggcagatgagatggttatttgtaatgcgttaatgccagtgatgcccgtatgtgcctgtggcgatgtctccttttcgtcagcaacgttatatgaatatttagccccactttgtgagcgcccgaattagtcatgaaaaaagtgttattgataatcttgttattgctggtggtactgggtatcgccgctggtgtgggcgtctggaaggttcgccatcttgccgacagcaaattgcttatcaaagaagagacgatatttaccctgaagccagggaccggacgtctggcgctcggtgaacagctttatgccgataagatcatcaatcgtccacgggtttttcaatggctgctgcgtatcgaaccggatctttctcactttaaagccgggacttaccgctttacaccgcagatgaccgtgcgcgagatgctgaaattgctggaaagcggtaaagaagcacagttccctctgcgactggtagaagggatgcgtctgagcgattacctcaagcaattgcgtgaggccccgtatatcaagcatacgctgagcgatgataagtacgccaccgtagcgcaggcacttgaactggaaaacccggagtggattgaaggttggttctggccagacacctggatgtataccgccaataccaccgatgtcgcgttactcaagcgagcgcacaagaaaatggtgaaagcggtcgatagcgcctgggaagggcgtgcggacggtctgccttataaagataaaaaccagttggtgacgatggcatcaattatcgaaaaagaaaccgccgttgccagtgaacgcgataaggttgcctcagtatttatcaaccgtttacgcattggtatgcgcctgcagaccgacccgaccgtgatttacgggatgggagagcgttataatggcaaactttctcgtgcagacctggaaacgccgacagcgtataacacctataccattaccggtctgccgccaggtgcgatagcgacgccgggggcggattcgctgaaggctgctgcgcatccggcaaaaacgccgtatctctattttgtggccgatggtaaaggtggtcacacgtttaataccaatcttgccagtcataacaagtctgtgcaggattatctgaaagtgcttaaggaaaaaaatgcgcagtaagtatatcgtcattgaggggctggaaggcgcaggcaaaactaccgcgcgtaatgtggtggttgagacgctcgagcaactgggtatccgcgacatggttttcactcgggaacctggcggtacgcaacttgccgaaaagttaagaagcctggtgctggatatcaaatcggtaggcgatgaagtcattaccgataaagccgaagttctgatgttttatgccgcgcgcgttcaactggtagaaacggtcatcaaaccagctctggctaacggcacctgggtgattggcgatcgccacgatctctccactcaggcgtatcagggcggcggacgtggtattgaccaacatatgctggcaacactgcgtgatgctgttctcggggattttcgccccgacttaacgctctatctcgatgttaccccggaagttggcttaaaacgcgcgcgtgcgcgcggcgagctggatcgtattgagcaagaatctttcgatttctttaatcgcacccgcgcccgctatctggaactggcagcacaagataaaagcattcataccattgatgccacccagccgctggaggccgtgatggatgcaatccgcactaccgtgacccactgggtgaaggagttggacgcatgagatggtatccatggttacgacctgatttcgaaaaactggtagccagctatcaggccggaagaggtcaccatgcgctactcattcaggcgttaccgggcatgggcgatgatgctttaatctacgccctgagccgttatttactctgccaacaaccgcagggccacaaaagttgcggtcactgtcgtggatgtcagttgatgcaggctggcacgcatcccgattactacaccctggctcccgaaaaaggaaaaaatacgctgggcgttgatgcggtacgtgaggtcaccgaaaagctgaatgagcacgcacgcttaggtggtgcgaaagtcgtttgggtaaccgatgctgccttactaaccgacgccgcggctaacgcattgctgaaaacgcttgaagagccaccagcagaaacttggtttttcctggctacccgcgagcctgaacgtttactggcaacattacgtagtcgttgtcggttacattaccttgcgccgccgccggaacagtacgccgtgacctggctttcacgcgaagtgacaatgtcacaggatgcattacttgccgcattgcgcttaagcgccggttcgcctggcgcggcactggcgttgtttcagggagataactggcaggctcgtgaaacattgtgtcaggcgttggcatatagcgtgccatcgggcgactggtattcgctgctagcggcccttaatcatgaacaagctccggcgcgtttacactggctggcaacgttgctgatggatgcgctaaaacgccatcatggtgctgcgcaggtgaccaatgttgatgtgccgggcctggtcgccgaactggcaaaccatctttctccctcgcgcctgcaggctatactgggggatgtttgccacattcgtgaacagttaatgtctgttacaggcatcaaccgcgagcttctcatcaccgatcttttactgcgtattgagcattacctgcaaccgggcgttgtgctaccggttcctcatctttaagagagacatcatgtttttagtcgactcacactgccatctcgatggtctggattatgaatctttgcataaggacgtggatgacgttctggcgaaagccgccgcacgcgatgtgaaattttgtctggcagtcgccacaacattaccgggttatttacatatgcgggatctggtaggcgaacgtgacaacgtcgtattttcttgtggcgtgcatccactcaaccagaatgatccctacgatgtagaagatttacgccgtctggcggcagaagagggtgttgtagcgctgggtgaaaccgggctggattattattacacgccggaaactaaagtacgtcagcaagagtccttcatccatcatatccagattggtcgtgaactgaacaagccggttatcgtccatacccgtgacgcccgtgccgatacgctggcaattctgcgcgaagaaaaagtgacggattgcggtggcgtactacactgttttacagaggacagagaaacggcgggtaaattactggatctcggattttacatctccttttccggcattgtgaccttccgtaatgcggagcaactgcgcgatgctgcgcgttatgtccccctggatcggttactggtggaaactgactcaccttaccttgcgccggtaccgcatcgaggaaaagagaatcaacctgcgatggttcgtgacgttgcagaatacatggctgtgttgaaaggtgttgccgttgaagaactggcgcaggtaaccaccgataacttcgcccgtctgtttcacatcgacgcttcccgccttcaatccatccgttgaatgagtttttttaaagctcgtaattaatggctaaaacgagtaaagttcaccgccgaaaattgggcggtgaataaccacgtttgaaatattgtgacatatgttttgtcaaaatgtgcaacttctccaatgatctgaagttgaaacgtgatagccgtcaaacaaattggcactgaattattttactctgtgtaataaataaagggcgcttagatgccctgtacacggcgaggctctccccccttgccacgcgtgagaacgtaaaaaaagcacccatactcaggagcactctcaattatgtttaagaatgcatttgctaacctgcaaaaggtcggtaaatcgctgatgctgccggtatccgtactgcctatcgcaggtattctgctgggcgtcggttccgcgaatttcagctggctgcccgccgttgtatcgcatgttatggcagaagcaggcggttccgtctttgcaaacatgccactgatttttgcgatcggtgtcgccctcggctttaccaataacgatggcgtatccgcgctggccgcagttgttgcctatggcatcatggttaaaaccatggccgtggttgcgccactggtactgcatttacctgctgaagaaatcgcctctaaacacctggcggatactggcgtactcggagggattatctccggtgcgatcgcagcgtacatgtttaaccgtttctaccgtattaagctgcctgagtatcttggcttctttgccggtaaacgctttgtgccgatcatttctggcctggctgccatctttactggcgttgtgctgtccttcatttggccgccgattggttctgcaatccagaccttctctcagtgggctgcttaccagaacccggtagttgcgtttggcatttacggtttcatcgaacgttgcctggtaccgtttggtctgcaccacatctggaacgtacctttccagatgcagattggtgaatacaccaacgcagcaggtcaggttttccacggcgacattccgcgttatatggcgggtgacccgactgcgggtaaactgtctggtggcttcctgttcaaaatgtacggtctgccagctgccgcaattgctatctggcactctgctaaaccagaaaaccgcgcgaaagtgggcggtattatgatctccgcggcgctgacctcgttcctgaccggtatcaccgagccgatcgagttctccttcatgttcgttgcgccgatcctgtacatcatccacgcgattctggcaggcctggcattcccaatctgtattcttctggggatgcgtgacggtacgtcgttctcgcacggtctgatcgacttcatcgttctgtctggtaacagcagcaaactgtggctgttcccgatcgtcggtatcggttatgcgattgtttactacaccatcttccgcgtgctgattaaagcactggatctgaaaacgccgggtcgtgaagacgcgactgaagatgcaaaagcgacaggtaccagcgaaatggcaccggctctggttgctgcatttggtggtaaagaaaacattactaacctcgacgcatgtattacccgtctgcgcgtcagcgttgctgatgtgtctaaagtggatcaggccggcctgaagaaactgggcgcagcgggcgtagtggttgctggttctggtgttcaggcgattttcggtactaaatccgataacctgaaaaccgagatggatgagtacatccgtaaccactaatccgtaagacgttggggagactaaggcagccagatggctgccttttttacaggtgttattcagaattgatacgtgccggtaatgctgaaattacgcggtgtgccgtagacgatagaaccttccacgttggtatcgtaggttttgtcgaacaggttattgacgttcccctgtaacgagaagtttttcgtcacctggtagcgggtgaagagatccaccagcgcgtagctaccttgctcggcgcggaaggtgccatacggcgtcacggtgtcggtatacacgcgattttgccagttaacaccaccgccgaccgtcaactctggcatgacaggcaaccgatagctggtgaacattttaaccgtggtgcgtggcagattaggattaacggcgtttccttcgttatcctctgcaatatagcgcgttgcgccaaatgtcagctgccagttgtcggtaattgcgccgttgagttcaaattccacccctttactgactgtcccatccaccgctttataggcggtttcgccgttgctgccggggataggtgtaccggtggactgagcgacattatcctgctcaatacggaagatggctaacgtggtggtcagacggctattcatccagtccgatttcagacccagctcgtagttgttaccggtgattggagccagatatttgcctgaactgtcacgatcattttgcggctggaaaatagaggtatagctggcgtaggtcgaccagttgtcattgatgtcaaacaccagaccagcgtaaggcgtggtgtggtttttctccatgctgtaagtcagcgtatcaacccgccagttggtataacgtgcgccgaggatcagatgcagcggatcggcaagggtgacacgagtggcagcatataacgatttcatatgtgtggtatcgtcctgcgccaggctctgtggtgaccagtcggtttgtgggaaattgccattaaagttgtagaaactgccaatttcatccgggaagatgttggcccatgaactgaagtaacgattgttttgtttgctgtaactgccaccaaacattagattgtgctgacgaccaaacaattcataactaccgtcagcgaacaaatccagcgcatcaactttacgtttgccactgttccaaccggtgccgccgacataatcaaagccaggtccataattactgtatggcccaaccagcataccatccgctttgtttacataggcatcgacatacatcattttgctgtcaaattcgacttcagagtgggtggcattcagtgtcgcttgccaggtatcagcaaactgctgcttcagggtcataaagaccttgttgatctctttatcgttgtacgcccagtcaggtgcggtactgcgtgcgcgatcgtaactgttgctgctgccatcagtattccagcgcggtaaaccgccccaggtagggctattaacatcaatgcgctgatattcgtaaccggctgaaagcgtcgtaagatcgcctaaatcagcatcgacaatgcccgagaagaaggtcttttcactgttgtagcggtccagccatgagtcgttattctggtagccgccgacaattcgcgcgcggattttaccgtcttcggtgagtgggctttgtaaatccgccacataccgttctttgttccagctaccgtattccgccgagacatcgcctttaaattcacgactggtcgcgtgttttcgaaccatattaattgccgcagatggattacccgtcccggtcatgagtcctgtcgcgccacgcactacttctacgcgttcaaagagtgccatatcagaaagtgcgtcgcccagattccagcgcgattcaaaataggtggggataccatcaaccatatagttatcgatctggaatccgcgggaataataaagagcacgatcggaatccgcctgacttttgctgatccccagcgtgttttccatcacttcgcccagcgtttgtaactgctgatcttccatccgctgctggctaacaatagtgaccgactgaggaatatcacgttgagtcatctgcattttggtacccgcagaggtagacgttacgctgtaatcattttcgccatcatctggagctgtggctgaaccctcaacaatcaccgtttcttcagtggctggtgcagcaaaagcggcagaaggtaatagtgccagtgctatgcaaccggcaagtagtgacggtttggtgatggcttgatattgattatccctgttaaattgtgttgaaagcatttgaaatctcttggtttatgttgtcgtcaggctcatgccggaggagggtgatgagcgattatatttagtgtgcgaataattttgtttgtaaatgcaaatgagaaatatacgcattcatatttgtcatgtaaaccaaacagagaatgtcttttcagcgcattcgcaggcagaaatgggaataatggcgatatatacggcagcaaaacgattttttgcttaagaaatcgtgagttaaggttgaaagagcaggtttaactcgaccatactctatactcgcagtgtggcgcggcgtagcatggcgcaacgcatggctatttgaaaaaggaaaatgtcgtggcagaagaaactatattcagcaaaattattcgtcgtgagatcccctccgatatcgtctaccaggatgatctggtaacggcgtttcgcgatatttcgccgcaagcgccaacgcatattctgatcattccgaatatcctcattccgactgtgaacgacgtctcagctgagcatgagcaggcgctgggacgcatgatcaccgtagcggcaaaaattgctgagcaagaaggtattgccgaagatggctatcgtctgatcatgaataccaaccgccatggcggacaagaggtttaccacatccatatgcacttgttgggtggccgtccgctgggaccaatgctggcgcataaaggtctgtaacgatgagaaaaggatgctttgggctggtgtctctggtgttgttactgctggtgggctgtcgttcacatccggaaattccggtgaatgatgagcaatcgctggtgatggagtcatctttattggctgcgggcatcagtgcagaaaagcccttcctttcgacgtctgatattcaaccttcagcatcctcaacgctttataacgaaaggcaagaacccgttaccgttcattatcgtttttactggtatgacgccagagggctggagatgcatcctctggaaaggccacgcagcgttaccattcccgcacattcggcggtaacgctgtacggcagcgccaattttctgggggcgcacaaagtcagactttatctatatttgtaaggggtgaatcttgatgacaaaaatgagtcgctacgccttgattaccgcgctggcgatgtttctcgccgggtgtgtggggcaacgtgaacctgcaccggtagaagaagtgaaaccagcgccggaacaaccagccgagccacaacagcctgtccccacagtgccctcggtgccgacgatcccgcagcagccaggcccaattgagcacgaagatcaaactgcaccgcctgcgccgcatattcgccattatgactggaatggcgcaatgcagccgatggtcagtaagatgcttggggctgacggggtgactgcgggtagcgtcctgctggttgatagcgttaacaaccgtactaacggttcgctgaatgccgcagaagcgaccgaaacgctgcgaaatgcgctggctaataacgggaaatttaccctggtttccgcccagcaactgtcgatggcgaagcaacagttaggtttgtcgccgcaggacagtttaggcacccgtagtaaagccataggcattgcccgcaatgtcggcgctcattacgtgctgtactccagcgcctctggcaacgttaacgctccgaccctacaaatgcagctgatgctggtgcagacgggcgaaattatctggtcaggtaaaggtgccgtttcgcagcaataatcccatcacgcgcgacgaattgctgtcgcgctttttcccgcagtatcatcccgtcacgacgtttaatagtgggcttagtggcgggagttttctcattgaacatcagggccagcgttttgttgtgcgtcagccgcacgatcctgatgcgccgcagtccgcgttcttgcgccagtatcgggctttatcacaactacccgcatgcattgcaccgaagccgcatttatatctccgtgactggatggtagtcgactatctgcccggcgcggtaaaaacgtatttgccggataccaacgaactggcaggcttgctgtattatctacatcaacaaccacgttttggctggcgaataacgctgttgccgttactggaactgtactggcagcaaagcgatccggcgcggcggacagtgggttggctgcgaatgttaaaacgtctgcgcaaagcgcgggaaccacggcctttacgcttaagtccattgcatatggatgtccacgccggaaatttagtgcatagcgcgtcagggttaaaactcatcgactgggagtatgccggagatggtgatatcgcgctggaactggcggcggtgtgggtggaaaatactgaacagcaccggcaattggtcaatgactatgccactcgcgcgaagatttatccggcgcaattatggcgtcaggtcaggcgatggtttccctggctgctgatgctcaaagcagggtggtttgagtaccgctggcgacaaaccggcgatcaacaatttatcaggctggccgatgacacctggcggcagctattaataaaacaataaggagagcagtgtgggtccagtaatgttggatgtcgaaggttacgaactggacgcggaagagcgtgaaatactggcgcatccgctggtgggagggctgattctctttacgcgtaactatcatgatcctgcccagttacgtgaactggtgcgccagatccgcgcagcttcgcgcaatcgtctggtggtggcggttgatcaggaaggtggacgcgtgcagcgttttcgtgaaggttttacccgcttgccagcggcgcaatcattcgctgcgctgtcaggaatggaagagggtggcaaactggcgcaggaggcaggttggttgatggccagcgaaatgatcgctatggatattgatatcagctttgcgcctgtgctggatgtcgggcatatcagcgcggcgattggcgagcgttcttatcatgccgatccacaaaaagccctggcaattgccagccggtttattgatggtatgcatgaagccggaatgaaaacgaccgggaaacacttcccaggacacggtgcagtaacggcagactcacacaaagaaacaccgtgcgatccacgtccacaagcggagattcgcgctaaagatatgtcggtcttcagttccttaatccgcgaaaataaactcgacgccattatgcctgcgcatgtgatctacagtgatgttgatccgcgtccggcgagcggttctccctactggctgaaaaccgttttgcgtcaggaactgggttttgacggcgtgattttctctgacgatttatcgatggaaggtgccgcgattatgggcagttatgccgaacgcgggcaggcttcactggatgcgggttgcgatatgatcctggtctgcaataatcgtaaaggggccgtcagcgtgttagataatctgtcaccgatcaaggcagaacgtgttacacgtttgtatcataaaggttcattttcgcgacaggaactgatggactcggctcgctggaaagcgatcagcacccgtctgaatcagttacatgaacgctggcaggaagagaaagcaggtcactaaccctggcttatgtgaggaagcgatgattatctatttacacggttttgactctaacagtccgggtaaccacgagaaagtcttacaattgcagtttattgacccggatgtacgcttgataagctacagtacgcggcatccgaaacatgatatgcagcatctgcttaaagaagtggacaaaatgttgcaactgaacgttgacgagcgtccgctaatttgcggcgttggcttgggcggatactgggcggaacggattggttttctttgcgacatccgccaggtgatcttcaaccctaatttgttcccttatgagaacatggaaggcaagattgatcgcccggaagagtatgccgatattgccactaagtgtgtgaccaacttccgtgagaagaatcgcgatcgttgcctggtgattttgtcgcgtaatgatgaagcgcttaacagccagcggacatctgaagagttgcatcattattacgagattgtctgggacgaagagcagacgcacaaattcaagaatatctccccgcatttacagcgcattaaagcgttcaaaaccctcgggtaaatgccctcgtcgcatcaggtaaccttgccggtacctgatgcgctccgaattctgtgggtcggataaggcgtccacgccgcatccgacagtcgagcatcaatgcctgatgcgcttcttatcaggcctaccgaacgccctgcatacacccctcactctatatcactctcacaaattcgctcaaataataaacaataaactctgttttttgatctcacccggtaaagtcgcctatcttttcagcaacaaaacttgattaacatcaattttggtatgaccaatgcaccattcatgttattctcaatagcgaagaacattttcattgctgtaacctgttgttaattaagagctatgttaataaccattaattaacaattggttaataaatttaagggggtcacgttgactacgccattgaaaaagattgtgattgtcggcggcggtgctggtgggctggaaatggcaacacagctggggcataagctgggacgcaagaaaaaagccaaaattacgctggtcgatcgtaaccacagccacctgtggaaaccgctgctgcacgaagtggcgactggctcgcttgatgaaggcgtcgatgcgttgagctatctggcccatgcgcgcaatcatggtttccagttccagctgggttccgtcattgatattgatcgtgaagcgaaaacaatcactattgcagaactgcgcgacgagaaaggtgaactgctggttccggaacgtaaaatcgcctatgacaccctggtaatggcgctgggtagcacctctaacgatttcaatacgccaggtgtcaaagagaactgcattttcctcgataacccgcaccaggcgcgtcgcttccaccaggagatgctgaatttgttcctgaaatactccgccaacctgggcgcgaatggcaaagtgaacattgcgattgtcggcggcggcgcgacgggtgtagaactctccgctgaattgcacaacgcggtcaagcaactgcacagctacggttacaaaggcctgaccaacgaagccctgaacgtaacgctggtagaagcgggagaacgtattttgcctgcgttaccgccacgtatctctgctgcggcccacaacgagctaacgaaacttggcgttcgcgtgctgacgcaaaccatggtcaccagtgctgatgaaggcggcctgcacactaaagatggcgaatatattgaggctgatctgatggtatgggcagccgggatcaaagcgccagacttcctgaaagatatcggtggtcttgaaactaaccgtatcaaccagctggtggtggaaccgacgctgcaaaccacccgcgatccagacatttacgctattggcgactgcgcgtcatgcccgcgtccggaagggggctttgttccgccgcgtgctcaggctgcacaccagatggcgacttgcgcaatgaacaacattctggcgcagatgaacggtaagccgctgaaaaattatcagtataaagatcatggttcgctggtatcgctgtcgaacttctccaccgtcggtagcctgatgggtaacctgacgcgcggctcaatgatgattgaaggacgaattgcgcgctttgtatatatctcgctataccgaatgcatcagattgcgctgcatggttactttaaaaccggattaatgatgctggtggggagtattaaccgcgttatccgtccgcgtttgaagttgcattaatcgacgtacactggcggatgtggcataaacgcctcatccgcccttgaggaacagcgcgatcggcagccgcgttgtatcaggcatcctttcagactcctccgaatccttaagtatttccagccattcccgcgcttttcatcttctgtctgatagctgcttttctccttcgcttgcatgattggcataactgcaaagaaggaggtgttcccgtgaataaatcaatgttggcgggtatcgggattggtgtcgcagctgcgctgggcgtagcggcagtggccagtctgaacgtgtttgaacggggcccgcaatacgctcaggttgtttctgcaaccccaatcaaggaaacggttaaaacaccgcgtcaggagtgtcgcaacgtcacagtgacccatcgtcgaccggtgcaggatgaaaatcgcattaccgggtcggtgctcggcgctgttgctggcggcgtgatagggcatcagtttggtggtggtcgcggtaaagatgtcgccactgttgtgggggcgctgggtggtggatatgccggtaaccagatccagggctctctccaggaaagcgatacttacacgactacgcaacagcgttgtaaaacggtgtatgacaagtcagaaaaaatgctcggttatgatgtgacctataagattggcgatcagcagggcaaaatccgcatggaccgcgatccgggtacgcagatcccgctagatagcaacgggcaactgattttgaataacaaagtataacaaggctgtactctgcaatttggcccctcattcgctcaggctgaggggctttttttgcgacttatttcaccagttcgggccataaacgcaaagtcgttccggcaatctgcatcagtttttccagcgatgcaccttcgcgtgcgctgatcgacatcccctgaataatacaattaaggaattctgccagatgtgtcacgtcacagtggggcgggatttccccgcgcgcttgtcgttgacataaaaactgctgcaaagtgcgctcttgcatcgcatggcgtgatttcaacgtattggcgatatctcctgaatctggggagagggtggtgcagttgttgatcatgaagcagcctgccggggtgtctttgctggtaaagcagttggcgatggcagcaaaatagtcagccagcgcagactccacgcttttctcttcacaaaacagctgtgcttcatgcttagcggcaaaacgatcgatatagcggtcgagaacggcacgaaataacccctctttgttggtaaattccgcgtatagcgtgggcgctttggctccggtcgcttcgacgaggtccgcaagagaagtcgcttcataaccgtgttgccagaacaatttcatggccttatcaagcgcggcatccctgtcgaacacttttgggcggccacggcttttttttacacattgtgttgagtcagttgccatgatgccgttgtacctggtgactgtgaatgaaaggttattataaaaataatcacctccgttcaccagtccagatcccataaaaataattgctttctatttaactgaaatttaaagatttttaaattaattaatgattgttataaaaaatatcttgtatgtgatccagatcacatctatcatttagttatcgatcgttaagtaattgcttgcgacgtcattcatctgcataaggccactattatgaaaaacgtaaaaaccctcatcgctgcggcgattttaagctccatgtcatttgccagctttgcggctgtcgaagttcagtcaacgccagaaggccaacaaaaagtcggtacaatcagtgctaacgcggggacaaatctgggatcgctggaagagcagctggcgcaaaaagcggatgagatgggcgcaaaatctttccgtattacttctgtaaccggtccgaataccctccatggaacagcagtaatttataaataagcattaaccctcattaatgcctgctactgctgattttttccccgcgacatgccgtgtcgcggggatttttttatccgggctttacagcgtttgtgggctcacttgatgacggcggacatccaccggcatcccggaacggacatccatcacatgttgcatcacttcagcgtcagtttgtgctgcatctttaaatgattgcattgcgctattcagcgtaattggcagcagctgcggatcgtcatcaatcttctctgacagcggctgatgtacttcaaccagacgcgcaccgtttggttcggcagagacttttatcggagtgttgatgatattcactttggtgcctggggtgacctggctaaagagtgttttgatatcgtcatcccgcagacgaatacagccagaacttacccgcatgccaatgccgaaatcggcgttcgtaccatgaagcaaataaacgccgccataggccgccagacgaatcgcatgatggcccattgggttatccagtccagccggcactaccgcaggcaactcaattccctgtgctttataacgggcgcggatgtttgccgttggcgtccaggttgggtttgcacgtttgtctgaaacggtggtcaccattgtcggtgtcagcgtgtcaccacctaactgaccaatacctattggatacacggttaccgaatttttacccggcgggtagtaatagagacgcagctccgcaatgttgatcacaatgccttcgcgcggcgcatctggaagtagggtttgcaacgggatcgttaacacgctgcccgcgcgcggtacgtaaggatcaacgccggggttagcctgtaacagagcgagaaagccgacgttgtattttttggcgatggcttccagagaaccaccgtcattttccaccacatgaaatttgttttcgccaaccagacgactgcccgctggcggcagcggccaggtgttggcttttgccggtagcgccagcgccacggcagcggcgaacgtaaaaaacgttagccagcgagaaaaacgcgttttgatcatcaccaaaaatccataataaatataaggttattgtaataaacagataagcctgaattatggatggtgacagtgtcggatagtgcagggaagtgcaaagaatttgtaaatgttgcagatgggggcgcagaaacgcccccgatttaccattaagcgatcgcgttctcttccagttcacgcataaactggcgtacccattcgatacgcgttttccgctcactcaaatcctgaataaatttcaggcgcgtcggaccatcaaggcggtaatgctgcggctgtttttgcagcaaaccaatcaaccaggccggattaacgtgattcttctcggcaaattcgatcaccccgcctttctcattaccttccagcttcctgatccccagtttctgcgcttgctggcgcagacgggcaatatccagcagggtacgcgccggatctggcagcaggccgaagcgatcgataagctcgactttgatctcttccagttcgttttccgttttggcgctggcaatacgtttgtagaacgacagacgcgtgttcacgtcagggatgaaatcatctggcaatagcgacggcatccgcagctcgacttctgtttgctggctggtgagatcttccagcgacggctcgcgtccggctttcagtgcatcgacggcgttttccagcaactccatatacagcgagaaaccgatggtttccattgagccgctttgttcttcgccaagcagttcacccgcgccgcgaatctccagatcgtgcgttgccagcgcaaaacctgccccgagatcttccagcgaggcaattgcttcaagacgtttttgtgcatcggtagtcatcgcttttggatgcggtgtcagcaaccatgcatatgcctgatgatgcgaacgtccgacgcgaccgcgtaactggtgcagctgcgccagaccgaagtgatccgcgcgttcaatgataatagtgttggctgtcgggatgtcgatcccggtttcgataatggttgtacaaaccagcacgttgaaacgttgatgatggaaatcattcatcacccgttccagttcgcgctcgcgcatctgcccgtgaccgatggcgatccgcgcttctggcaccagttctgccagccgttcggcggctttctgaatgttttccacatcattgtagagataataaacctgtcctccgcgcaaaatttcacgcaggatcgcctcccggaccaccatgctgtcatactcacggacaaaggttttaactgccagacgacgggcgggcggcgtggcgataatcgacaggtcacgcattccgctcattgccatattcagcgtacgtgggatcggcgttgcagtaagcgtcagaatatccacgttcgcgcgcatcgctttaatgcgctctttatgacgcaccccgaagcggtgttcttcatcgacaatcagcaggcctaaatctttaaacttgacgtcactttgcagcagtttgtgcgtaccgatcagaatatcgattttcccttccgccacttccgcaaggatttgcgtctgctctttggcgctgcggaaacgggagatcatttcgatacgtaccggccagttggcgaaacggtcgcggaagttgtcgtaatgctgctgcgcgagaagggtggtaggcaccagcaccgccacctgcttgtggttatctactgccaggaaagctgcgcgcatcgccacttctgttttaccaaagccaacatcgccgcacaccagacgatccattgccagcggctgacacatgtcgctaagtaccgcattaatggcctgcgcctgatccggcgtggtttcaaacgggaagctgtcgcagaacaactgatactgctcacgatcgtgtttaaacgcgaagccctctttggcggcgcgttgcgcgtagatatccagcaattccgccgccacatcacgcactttttccgccgctttctgccgcgcgcgtgaccacgcatcgccgccaagtttatgcagcggggcgttttcttccgcgccacctgcgtaacggctaatcagatgcagtgacgacaccggaacatacagtttggcgtcgttggcataggtgagcatcagatactcgccagtaatgccacccgcttccagcgtggtcattccggcataacgaccgacgccgtgctccagatggaccaccggctgaccaatatgcagttccgcaaggttacggatcagtgtatcggggttgatggtgcggcgagaatcctgacgacgacgggcaacgcgttcaccgagcagatcgctttcgcaaatcagcgccagattacgcaccgtatcgacaaaaccatgttcggcagcgccaatcatcagataacgcccacggtcgctggcttcatcaagacgcataatgcgttgcggagcaattttaattcgtgcgagcagttcacccagcgcttcacggcgaccttcactttctaccgagaacaccaccggaccgtcgaaagtctcgaggaacttacgcagcgcatccagcggcgctttttgttgtgcctgaacggccaggtctggcagtttctggaaacctaaattggcattcgcggcttttgtcggtaaatgttcagtttttagctgcacccggggccagtttttcagctctgagaagagctcgtccacccgcagccagagcgattgtggtggcaacagcgggcgcatcggatcgacgccgcgattctcaaaacgcgccagcgtgtcagcctggaaacgttcggcactggtttccagatcgccagtattcacgagcaaggtattggcagggaaataactgaacagcggcggcagtggttcgctgaagaacaatggctgccagtactcgatcccggcaggtaatgtgcctttactcacttgctggtaaatatgttctggatcgcgcttcacttcgaaggtatcgcgccactggctgcggaacagttcaattgccgctttatcggtcggaaattcgtgcgcgggcagcagattgatcgcttctacttcctccagcgtgcgctggctgtcgacgtcaaacacccgcaggctgtcgatttcatcatcaaagaaatcaagacgataaggcagctcactccccatcgggaagagatccagcaacgcgccgcgcgtggcgtattcgccgtgctccatcacctggtcaacatggcgataaccggcgctgtccagttgggttcgtaatgcatctcgtgacaggcgctgaccttttttcatcaccagcgcatgaccgtggagaaaactgtgtgggcaaacgcgctgcataagcgtattcaccggaacaatcagtacgccacgctgcatcgtcggtagctggtaaagggtggaaaggcgcgaggagataatgtcctgatgaggcgaaaaactgtcgtagggaagagtttcccagtccgccagattcatcaccatttgatcggtaaactggctgatttcatcatgcaaacgcagagcattttgcatatctggtgcaatgagtaccaccggaccggcgtgacgttcggcaatttccgctaccagcgttgcacaggctgcgccggttaactcgcccagcagacgctgctcacccgctttgacgggcagcgtataacgatattgttcaggcataacggttgtcagattctcgttaggatatgcctcaacatatgggggcatatctctgataagcaatgctgttcattatccgtaatcgacatggtttagcaaattgaatcgccccggctggggcgatggcttagcgggagtaactgacggcagcgggcagtgaaggcggggagaacaacagatcgctgaatgcacgctgtgaaagttttcttaccagcaagcccgcaacagtacagatgaacaaactgacaaagggataaaccagcaggagtgtcagttcgacttgcggcgaccagcgtgctgcgttcatttgcgcaagcagagttaagctgaatatttcaaccagaatgcgatgggtggtgtagatagcaatggtgttggagccaatcacattcagcaggctggtggagcgcataccgaatcgttgctcgtattgataaaacagcttcatgatcaccacaatcgataccagcgacaacagcagcgagatagtaaacaaccaggcaccgaccgccagaacggtaagcaaagaagccatcagcagatggcggcgcaacggcacctctttaacacaggtcattattgttgcgccaaaccatgcgccaaggctgtaataaggcaaattgcggatcacactgttcattccccaccacggcgtgggaacgaaattaaccgccacactcagcagtacaaacaaggcgaatagtggcagcgccagacggctaaaaattttacataccacgaaatagacaattaacgcatacagataccacaagctggtgctggcggtgatcatcccgtgcaggaactcaccggtggaatcggcataagcggcattggaggcattgcttaaatcgcgctcaggtgccagccactggttcagcgcacttaacgccagccactgcaccacgccccaaagcgccagcacccagaagatgttccagatccgtttatcgagacaatttccccacggtacgctgtcgatatagcggcgaatcaaatagccggatataaagaaaaaaaccggcatacgaaagggggcaaggtaaagattgaaatagatccagcatttgctcaggacttccgataacggatgctgaaaagtggtcagatgcggataaaaggtaatgaccgagtgataaatcaccaccagacaaatacataaccctttgatctggttaatccatagctctttttgtttcatcaggacaacacgctcttttttaatttacatgcggttgatcctgcgggttatgacccgaggtgtaatgggtatctgtctgtattggatgatttttcagattaagatcaggcggcaagattgatgataaaacatggcaatttagccgattgatttacgggggcttttcagattagccctgacgatcacttacagttcagacgtttacccatcttgctttcgcttatatactcgtgtctttgctacagcaaccagacggatttcatgtaccaacctgtcgctctatttattggcctgcgttacatgcgtgggcgtgcagcggatcgcttcggtcgtttcgtctcctggctttctaccatcggcattaccctcggggtgatggcgctggtcacagtattgtcagtgatgaacggctttgagcgcgagctgcaaaacaacatccttggcctgatgccacaggcaattctctcttctgagcatggctctcttaacccgcagcaactcccagaaacggcagtcaaactggacggcgttaatcgcgtcgcacctattactaccggtgatgtggtactgcaaagcgcgcgcagcgtggcggtcggggtgatgctcggtatcgacccggcgcaaaaagatccacttacaccgtatctggtcaatgtgaaacaaactgacctcgagccggggaaatataatgtcatcctcggcgaacaacttgcctcacagctaggcgttaatcgcggtgatcaaatccgcgtgatggtaccatctgccagccagttcacgccgatggggcgtattccaagccagcgcctgttcaatgtgattggcactttcgccgccaacagtgaagtcgatggctatgaaatgctggtgaatattgaggatgcctcgcgtctgatgcgttatccggcaggcaatattaccggctggcgtttgtggctggatgagccgctgaaagtcgactcattaagtcagcaaaaactgcctgaaggcagcaaatggcaggactggcgtgatcgtaaaggcgagttgttccaggccgtacgcatggaaaaaaatatgatgggtttactgctgagcctgattgtcgccgttgcggcgtttaacattattacctcactagggctgatggtaatggagaagcagggcgaagtagcgatcctgcaaacgcaaggcttaactccgcgacaaatcatgatggtctttatggtgcaaggggccagcgccgggattatcggtgcgatcctcggagcggcgcttggcgccctgcttgccagccagttaaataatctgatgccgataatcggcgtcctgcttgatggcgcggcgctgccggtggctatcgaacctttacaggtcattgttattgcgctggtggcgatggctatcgcgctgctgtctacgctttacccttcatggcgcgctgccgccactcaacccgctgaggctttacgttatgaataagatcctgttgcaatgcgacaacctgtgcaaacgctatcaggaaggcagtgtgcaaaccgatgtgctgcacaatgtcagtttcagcgtcggcgaaggtgaaatgatggcgatcgtcggtagctctggttccggtaaaagtaccttgctgcacctgctgggcgggctggatacgccaacctccggcgatgtgatttttaatggtcagccaatgagcaaactgtcgtcggcagcgaaagctgaactgcgcaaccagaagctgggctttatttatcagtttcaccacctgctgccggattttaccgccctggaaaacgtggctatgccgctgctgattggcaagaaaaagcccgctgaaatcaacagccgtgcacttgagatgttaaaagcggtggggctggatcatcgtgcgaatcaccgcccatctgaactttctggcggcgaacgccagcgtgtggcgattgcccgtgcgctggtgaataacccgcgcctggtactggcggatgaacctaccggtaacctcgatgcgcgtaacgccgacagcatcttccagttgcttggggaattgaatcgcttgcagggcaccgccttcctggtggttactcacgacctgcaactggcgaaacgtatgagccgccagttagaaatgcgtgatggtcgtctgacggcggaactgagcctgatgggggcggagtaatggcgatgcctttatcgttattaattggcctgcgttttagtcgcggacggcggcgcggcggcatggtgtcgctgatctccgttatttctaccattggcattgccctcggcgtggcggtattgatcgtcggcttaagcgcgatgaacggctttgaacgcgaactgaacaaccgtattctggcggtggtgccgcatggtgaaatcgaggcggtggatcagccgtggactaactggcaggaagcactggatcacgtgcaaaaagtgccgggtattgccgctgccgcgccgtatatcaatttcaccgggctggtggaaagtggcgcgaatcttcgcgcaatccaggtgaagggcgttaacccgcaacaggaacagcgtctgagcgcattaccctcgtttgtccagggcgatgcgtggcgcaattttaaagcgggcgaacagcaaattatcatcggcaaaggcgtggcggatgcgctgaaagtgaagcagggggattgggtgtcgattatgatccccaactcgaatcccgagcataaactgatgcagccaaaacgtgtgcgtttgcacgttgccggtattttgcagttgagtggtcaactcgatcacagttttgccatgatcccgctggcggatgcccaacaatatcttgatatgggttccagcgtgtcaggtattgcccttaaaatgacggatgttttcaacgccaataagctggtacgcgatgcgggtgaagtgaccaacagctatgtttatattaaaagctggattggtacttacggctatatgtatcgcgatatccaaatgatccgcgccattatgtatctggcgatggtactggtgattggcgtggcctgtttcaacatcgtctccaccttagtgatggcggtgaaagacaagagtggcgatatcgcagtattaagaacgctgggggcgaaagatggtttaattcgcgccatctttgtctggtatggattgctggcagggctgttcggcagcctgtgtggtgtgattatcggcgtagtggtttcactgcaacttaccccgattattgagtggattgaaaagttgatcggtcatcagttcctctccagcgatatctattttattgatttcctgccatcggaattgcactggctggacgtcttctacgtactggtcacagcattgttgctgagtcttttggcaagttggtatccggcgcggcgcgccagtaatattgaccctgcgcgagtccttagcggccagtaaaggcagtacattaaaacaaggagcggcaatgtattacgggtttgatattggtggaacaaaaattgcgcttggcgtgtttgatagcggtcggcagttgcagtgggaaaagcgggtgccgacaccgcgtgacagctatgacgcatttttagatgcagtgtgtgagctggtagctgaagctgaccaacgttttggctgtaaaggttctgtcggcatcggtattccgggaatgccggaaacagaagatggtacgctgtatgccgccaatgtccccgctgccagcggtaaaccgctgcgtgccgacctgagcgcacgtcttgatcgcgatgtacgccttgataacgatgccaactgttttgccctttcagaagcctgggatgatgaatttactcaatatccactggtgatggggttgattctcggcaccggtgttggcggcgggctgattttcaacggcaaaccgattaccggtaaaagctacattaccggcgagtttggccatatgcgtctgccggttgatgcgttaaccatgatggggttggatttcccgttacgccgctgcggctgtggtcagcatggctgcattgaaaattatctgtctggtcgcggttttgcgtggctgtatcaacactattatcatcaaccgttgcaggctcccgaaattattgcgctttatgatcaaggcgatgagcaggcaagggcgcacgttgagcgttatctggatttattagcggtttgtctgggaaatatcctgaccatcgttgaccctgacctggtcgtcattggtggtggcttatcgaatttcccggcaatcacaacgcaactggcggacaggctgcctcgtcatctcttacctgtagctcgtgttccgcgcattgaacgcgcgcgccacggtgatgcgggaggaatgcgtggtgcggccttcctacatctaaccgattaaacaacagaggttgctatgctgtcgcgtcggggtcatcggttaagtcgttttcgtaaaaataaacgccgcctgcgcgagcgtttgcgtcagcgtatttttttcagagataaagtggtgccggaagcaatggaaaaaccaagagtactcgtactgacaggggcaggaatttctgcggaatcaggtattcgtacctttcgcgccgcagatggcctgtgggaagaacatcgggttgaagatgtggcaacgccggaaggtttcgatcgcgatcctgaactggtgcaagcgttttataacgcccgtcgtcgacagctgcagcagccagaaattcagcctaacgccgcgcatcttgcgctggctaaactgcaagacgccctcggcgatcgctttttgctggtgacgcagaatatcgacaacctgcatgaacgcgcaggtaataccaatgtgattcatatgcatggggaactgctgaaagtgcgttgttcacaaagtggtcaggttctcgactggacaggagacgttaccccagaagataaatgccattgttgccagtttccggcacccttgcgcccgcacgtagtgtggtttggcgaaatgccactcggcatggatgaaatttatatggcgttgtcgatggccgatattttcattgccattggcacatccgggcatgtttatccggcggctgggtttgttcacgaagcgaaactgcatggcgcgcacaccgtggaactgaatcttgaaccgagtcaggttggtaatgaatttgccgagaaatattacggcccggcaagccaggtggtgcctgagtttgttgaaaagttgctgaagggattaaaagcgggaagcattgcctgatgcactacgcttatcaggcctgcaaggggacgcaattaattgaatttgcgggttttgtgggccggataaggcgttcgcgccccatccggaataatacacgcgcacttttccggcctcttttatcgtttactcgtcaataacaatgcggcaataaacgtacagacaccaattagccctgcccagagtggcgatattctggtaatcgcaaagctattatcgatatacaaacataaagcctgataacccatattggcaatagtcatcgccactgcaaattttaacgcataaataaaacgagtcgtgtagtaaaagatcctggaaaataagataaacgtcgcagcccaggcgataaaacctaatgtgttggtgctgccggggggagcattttcatgctgttgtcctggatgcggataatacgttagtggcggcgtcgattgttttaatatctgtgcttgtagaacagccaatgcattattgattccctgataccagagatctgcatttaaataagccagcgtgtgattttctatcagaaggccgagatgtttatcgtccagaccactttcaacctggccgttggtgatcataattaaccgtggttcgcgggtagtaaatagtaacagaacacttccttttacatcactcaatgaagatgacgcatgcgccagcatcgctttaccattttgtctgagactggcttcattattaatgtcgggtaaaaccacaataaacggtgcaattcccgtttgttggcgaaaaagctcggctttatgcgcgatctcttcagcatctggtacagtaccggtaacgtccgtaaaaagtgtcttcattattggaattaatggcttgctggctgctgtcagaggcaggagtatcagtaaactgagcagtataatgaattttttcatgggcgggacttccgtttcctgcgtgattttttagaggagggcatacttattaataaaccgacggcgataaaaataacgcccataatgccgataaacccccatttaaaaaaattaacccacgggttatttatctcagccttttcaggatgcccgggagaataataaacattaactttatcgccttcgctgtcttcataaaaatcgctgccgatactcgaattgaaaattagcgtgtaatctggcgtcggtcgaaaggcaacgacgggataccacgaaccatctttacccgtgcgatgagaatgactggagtgccagacggtatcaacaatgacgccttcggtatgaatcgcgtctttgctataggtgaactggttataaaagacaacaacagaaatgaggatcagtaccagaccgataccgaggaatatacgaaagaaaactttactgtcctgactcattagccacatccttgctaactaaaaaacgggcggtaataccaccgcccgcttgctgaattaacgtcctgctttcagcttctgataatactcttcataaatgctgctggctgcgccaacgtcattctgccattcgccatttttaatggtttcagcatccgggtagagtgttttatcgttcgccacttctggacttaacagcttacgcgccgcaaggtttggcgttggataaccgatagtttcagcaacctgttttgccacatccgggcgcagcaggaagttgatcaatttcagcgcgccttctttgtttttggcatttgccgggatcgccaggctgtccatccagaaaatgccgccttctttcggccacaccacgtcaattggcgtacccgcctggcgtgcaacgaaagcagaaccgttccagatcatgccgaggttaacttcgccttccatgtacgggttcgccgggttatcggagttaaaggctgccacgtttggcatcagttttttcagctcgttatatgcagcttcaatctctttcggatcggtggtgttaccggagtagcccagcttacgcagcgccatctggaacacttcacgggcatcgtcggtcaacagcaggctgcctttgtactctggcttccacagatcggcccagctggtgacagatttcggatccaccgcatcaccgttaacaccaatcgccgtcgcaccccagatatacggaatggagtagtcgttattcgggtcaaaaggcttgttgagcatgtctggatcgagattgctgaagtttgttaacttcgacttgtcgatcttctggatcatcccttctttacgcattttatcaacgtaataggttgaaggaaccaccagatcataggcaccgtctttgtatgttttcagcttggcgtacatggtttcgttcgactcgtaagtcgaatagataaccttaataccggtttctttggtgaactgttcaagcagtcctggcggcacgtactcggtccagttgtagaaatacagcgtgttgttgtcatcggcgtgagcggcgctcatgcccagtgccagagcacccgccgcgagcaggtggcgtgaccattttttcatttaacgtcccctgtgttacctttcgttttatcacgagcaataagctggctggcaataaccatcaccagcgacagcaccagtaatatggttgccagcgcgttaacttccggcgatacgccgactttgaccatcgaataaatttttaacggcagaatttcataacttggtccggtgacgaacgaagaaactaccacatcgtccatcgacagggtaaagcttaacacccagcccgccgccaccgctggcattgccagtggcagaatgatttttcgcagaatggtaaattcgctggcaccgagatctttcgccgcttccagcattcgcacgtcaaaacctttcaggcgcgaatacaccgtcaccaccacaaatggcaggcagaaggtgatatgcgagaacagcagcgaccagaagccaagctgaatacccagcagcataaacagcaccagcagcgaaatcgccatcacgatatctggtgacatcatcaccacaaacagcattccgctaacgaacggcttaccacgaaagcgataacggtacagcgcaactgccgtcagtgaaccgataagcgtagcaaacgtcgccgaaaacaccgccattgttagtgaatgctgcgctgcctgtaacaggctgtcgttgttcatcagcaggctataccatttggtggtaaagccctgccagttgatgccaaagcgcgagctgttaaaggagttcacaatcaaaataatgattgggatatacaggtacgcgtagatagcggtcataaaaccgccgcgaagcagtcgaccgatcattcgagttccaccttcttattcagcaaacgagaagcgcgccagtaaaccagcaacatcaggcccattacgatagtcagcgtaatgctggtagctgcaccaaacggccagtcacgaatattaaggaactggaccttgatgacgttaccgatcagcaggtttttcgcaccgcccatcaggtcggatacatagaacaggcccatcgctggcagcatcaccagcagacatccggcaataattcccggcatcgtcagtggaataatgatacggataaaagtctgtaacttgctggcaccgagatcgcgcgccgcctcaagcaacggcttatccagtttttcgatactggagtacagcggcatcaccataaacggcagcagaatgtaaaccagaccgataatcaccgcactgggcgtgaacatgatacggattggtgtgtcgataacgcccagccagagcaaaaactcgttgagatagcctttggtgctgaggaaaattttcagcccgtagatacgaattaatgagttggtccagaacggaacaatcagcagaaacagcagcagcggacgcaccttgtgtggcaacttcgccagaaaccaggcaaacgggtagcccagcaccaggcaggcgagggtggcgatcagcgccatattcagcgagtgcaatagcacttcaaaatagagcggatcgagcagacgcgtgtagttatccagcgtaaagaccattttgacaaaactggcgtcgtcgcgggtcaaaaagctggtgccaatgatcatcaggttgggcagaaagacaaacaacacaagccaaccgacaatagtgacaatcactacattctggaacttacttgtgttcttcatcagccagtacgacctcccagctttctacccaattaatggccattttttggtcgagagagtggtcaaagtcaggatcgtcttcattgaagaattcgctgaccatcaccatcttgccattttccagttcaacaaccgactccagcgtcatgcctttgtagttacgctcgcgaacgtaaccaatcagcccttcagcgtggttgtcgtcgttaatctcttcaacacgtaagtcttccgggcgcagcagaacatgcagtttttgccccggttcaacggcgaagttaacgtagatattacattcgcggccttcaacgttggcgcgtacgcgctgctcgtctagacgttcgatgacagtggcgttaaacatattgatttcgccaatgaagccggcaacaaacaggtttttcggctcttcgtagatttcacgcggcgtgccgtcttgctcaatgcgaccatcgcgcatcaccacaatcctgtctgacatggtgagtgcttcttcctggtcgtgagtcacaaagacgaatgtaatgccaagcttacgctgtaacgctttcagctcgttctgcatttgcttacgcagtttgtaatccagcgctgagagcgactcatccagcaacaacagacgaggcttgttaaccaccgcgcgagcaatggcgacgcgttgctgttgaccaccagagagctgatgcggtttgcgttgagcgaaggtttccaactgcaccatccgcagggcttccatcacgcggggcgtaatttcagcagcgggggttttttgcatgcgcaacccaaaggccacattttcgaacacggtcatgtgggggaaaagtgcgtagctttggaaaacagtgttcacatagcggttttccgccggaacgtgggtgatgtcctcgttatccagcatgatgcgtccggaatcaacagtttccagacctgcaatcaggcgaagaacggttgttttaccgcagccagaagggccaagcagcgtgaggaactcgccattgttgatagtcagatccagctggggaatgacctctttaccatcaaagcatttgcgaattcccgccaattgcaccagcggtgaaagcgaactcggttgtttattcaattttttactctgtcccatgtaaacgcaacggatggcttaccgatgcggggtttgtggttaaccaccttggtgactcttaatgagggcggtaattctacggcaaaccgcttgaatcgccaatctttgttgtgaattactggcttagctttatattcattaaggtaatgctgataaatattcccgcttgcaggggtaaaagtgacctgacgcaatatttgtcttttcttgcttcttaataatgttgtcacaaaaagtgagggtgactacatggataaactacttgagcgatttttgaactacgtgtctctggatacccaatcaaaagcaggggtgagacaggttcccagcacggaaggccaatggaagttattgcatctgctgaaagagcagctcgaagagatggggcttatcaatgtgaccttaagtgagaagggcactttgatggcgacgttaccggctaacgtccctggcgatatcccggcgattggctttatttctcatgtggatacctcaccggattgcagcggcaaaaatgtgaatccgcaaattgttgaaaactatcgcggtggcgatattgcgctgggtatcggcgatgaagttttatcaccggttatgttcccggtgctgcatcagctactgggtcagacgctgattaccaccgatggtaaaaccttgttaggtgccgatgacaaagcaggtattgcagaaatcatgaccgcgctggcggtattgcaacagaaaaaaattccgcatggtgatattcgcgtcgcctttaccccggatgaagaagtgggcaaaggggcgaaacattttgatgttgacgccttcgatgcccgctgggcttacactgttgatggtggtggcgtaggcgaactggagtttgaaaacttcaacgccgcgtcggtcaatatcaaaattgtcggtaacaatgttcatccgggcacggcgaaaggagtgatggtaaatgcgctgtcgctggcggcacgtattcatgcggaagttccggcggatgaaagcccggaaatgacagaaggctatgaaggtttctatcatctggcgagcatgaaaggcaccgttgaacgggccgatatgcactacatcatccgtgatttcgaccgtaaacagtttgaagcgcgtaaacgtaaaatgatggagatcgccaaaaaagtgggcaaagggttacatcctgattgctacattgaactggtgattgaagacagttactacaatatgcgcgagaaagtggttgagcatccgcatattctcgatatcgcccagcaggcgatgcgcgattgcgatattgaaccggaactgaaaccgatccgcggtggtaccgacggcgcgcagttgtcgtttatgggattaccgtgcccgaacctgttcactggcggttacaactatcatggtaagcatgagtttgtgactctggaaggtatggaaaaagcggtgcaggtgatcgtccgtattgccgagttaacggcgcaacggaagtaagcgaaaagggatgcggcatgtgatgccgcatccggcttaaatccaaacttacccttcgaagaaccaatacccgctattgaccagcgccgcgagcatcgcgaggaatgacggatcttccagcgcatcgccaaaattctccgcagtcagcgcaatgttgctggcgagtgcatccagtgccggacggtgcggggaatcgatcttctcaccattggcatacacgtcgtcgccaatgcgcaatacgcgcagaccacccaggcgcaccagcacttcaccttgtttcagcgcatcgtagatttcatccggctgataaggcggctctggcggcgcgatatccagttcatgacgtgactgggatataaactcgccaaaccattgcttaaagtgttccggctggttgatcaattcgagcatcatctcacgcagtttatccatctcttgcggcagaacatccgcaggatgagcgcgaggtggaacatccggatcgctgtagtagttgccgcccagttcacgttgcagcacataatcggcaaatccactaatcagttcccgcgtatttggcgcgcgaaagcccacggaatagttcatcgcattttccagcgcgtagccttcatgcgggaatcctggcggaatataaagaatatcaccaggctccagctcttcatcgatgatggcttcgaacggatcgacctgtaacagatccggatgtgggcagtgctgtttcatttgcagcttttcgcccactcgccagcgacgacgtccggtaccctgaatgataaacacgtcgtactgatcgagatgcgggccgacgccgccgccgggtacagaaaaagaaatcatcagatcatcaatacgccagtccggtagttcacggaacggtcgcatcagcgcggcggtcggctcatgccagtggttcactgcctgtaccagtaatgaccagttggtttcaccgagatgatcgtagctttcgaacgggccgtggctgacctgccatttgccatcctggtgactgaccagtcgactgtcaacttcgctttccatcgccagacccgccaactcgtctggagagatcgggtcaataaaattattaaagccgcgttttaacaccaccgggcgtttctgccagtgacgttcaagaaaatcgggccagttaagagtgagttggtattccatgttaagcatccacaggctggtatctgcaaccgattataacggatgcttaacgtaatgcgtgaagtatgggcatatttattcatctttcggcgcagaatgctggcgaccaaaaatcacctccatccgcgcaccgcccagcatgctctctccggcgacgattttaccctcatattgctcggtgatttcgcgggctaccgccagccctacaccttgcccagggcgtaaagtatcaacccgttgaccacggtcgaaaatgacctctcgcttgcttaatggaataccggggccatcatcctcgaccacaatatagagatgctcgtcggtttgccttgcagaaatttcgacaaactcgaggcaatatttacaggcattatccagcacgttgcccatcacctcgacaaaatcgttctgctcaccgacaaagctgatctctggcgaaatatcgagagagatattgacccctttgcgttgatacactttgttcagcgctgaggtgagattgtccagcagtggggcgaccggatgcagctcgcggctgagcaatgtcccgccgcgcatactggcacgatgcaggtagtagccaatttgctgtgaaatgcggctgatttgctccagcattaccggctcagcatcactgacgctcatcttttcactacgcagagaacgcagcgtactttgcagcaccgccagtggcgttttcagactatgggtcaggtcggtgagcgtcgtacggtatttgtcgtaacgttcgcgttcactttttaacaatcggttcaggtttcgtaccagactggtcagttctcgcgttgtggctggattgagcaattcgcggttatgttcttccagttcgcggacttcttttgccagggcttcgatggggcgtaaactccaccaggcggcgacccacagcagcgggatcactaacagcagattggctgagagcacatagataaaccagctccagaccatataggaactttttagctccaccggaatggtatccaccaccacaatggttaattttggcatccgcgatgttgccgggtagacgtttactgccaccgagtgggtcatctccgcgtcgtcatcatcttcccgcacttcctgcaactgttgctgtatcgaatgatctccactcagcaagaggctggtatcgttaacatccgcttcaatttcatgaaaaccattcgatttcagccagtcaggctggatcatcttcatcagccagggcacgtcacgttgcgcccataaaagctgcccgttctcatcataaattagcgtcatggtggggctttgcttgtcgatattttcgggtaactcgacatgcaacttattgttttcccacttcgcaagggtatagaacagattgctctcgccacgtaacagccgaaacgtagttttatcgaaactgacgctataaccgatcagcgcgaccattccgtaggcaagcgaaagcaccagtactaccgctgccgttgccaacagaaaacgtacccgcagcgagagcgggaaaaaaagacgcagtaattttttcatcagcgcaattcgaacagatagccctggccgcgaacggtggtaatcacttcttggggatattgtgcctgaatttttttgcgcagacgtcccatcagtacatcaatggtatggctttcccgcagctccgcatccggatagagttggagcattaacgaatctttgctgaccactttgccattattgcgtatcaacgtttccataatagtgtattcgaacgcggtcagtttgatcacttcgtcattaatagataattcacggcgagagagatcaacctgaaacggggggagcgaaatgacctgtgaagccagaccgctattacgccgcattaatgcctgcattcgcgccatcacctcttcaatatgaaacggtttagtcacataatcatcagcaccggcacttaatacttcgactttgtcctgccagctttcacgggcggttaataccagaatcggcagtgaaacatcgttgctacgccagcggcgaatcagtgacagaccgtcctcgtctggcaatccgagatcgacaatcgcaatatccggtatatgttcattgagataataatcggcttctttggcatcttctgcgtcatcgacctgatgaccagcatcctgaatctgaactttaaggtggtgacgtaacaacgcattgtcttcaacaaccagtacgcgcatttttatttctccctgtcttaattattaaaatagtgtaacgcgattatgtggttatgggggtaaacattaaataaaccagcggggaggggaggtaaagtgaaaaaataaaaagcggataatcttaataagcaggccggacagcatcgccatccggcactgatacgaggtttatttcagctcatcaaccatcgtgatagctcgaccaatatagttagccggcgtcatcgctttcaggcgggctttctcttcttctggcaacgccagaccatcgataaactgcttcatgccttcggcgtcaacgcgcttaccgcgagtcagctctttcagcttctcgtacggtttttcgatgccatagcgacgcataactgtctggattggttcagccagcacttcccagttgtgatccagttcatccagcagatggtcacggttcacttccagtttgctcacgcctttcagggtggattgatatgcaatcaaggcataaccgatacccacgccgaggttacgcagcacggtagagtcggtcaggtcacgctgccagcgggaaaccggcagtttgcttgccagatgctgcaataccgcgttggaaaggcccagattcccttcggagttttcgaagtcgatcgggttaactttatgcggcatggtggaagaaccaatctcaccagcaatggttttctgtttgaagtggttaagggcgatataaccccagacgtcacggtcaaagtcgatcagaatagtgttgaagcgcgcaacgcaatcaaacagttcggcaatgtagtcgtgcggttcgatctgggtggtgtacgggttccactgaatacccagcgaggtgacgaactcttcgctgaactgatgccagtcaacttccgggtaagcggcgatgtgggcgttatagttaccgaccgcgccgttgattttgccgaggatctccacctggttaagctggcggtactggcgctccatacggtaggcgacgtttgccatctctttaccgatggttgacggcgtggctggctgaccgtgggtacgagacagcagcgggatatcgcgatactgaacggcgagatctttaatgccatcaatcagttgacgccagtatggcaggatcacttcatcacgcgcggttttcagcattaatgcgtgggagaggttattgatatcttccgaagtacaggcaaagtggatgaattcagaaaccgcgtgcagttccgggatctccgccactttttctttcaggaaatactcaaccgctttaacgtcgtggttagtggtacgctcgatagttttgatgcgcgccgcatcttcttcgctgaaactggcgacgattgcatcaaggtaaccgattgcgtcggcagcaaaagcaggaacttccttgatcgctgcgtgcgcggccagtttttgcagccaacgtacttcaacttgtacacggaatttcagcaaaccatattcgctgaaaatcccgcgcagcgcgctgactttatcgccgtagcgtccatcgacaggggaaacggcggtcagtgaggataattccatagatcacaactccggggttaaatgagcaagaatttgttttgcctgagtggtcaggcgattacgagaaaacatcagttgcagacgtccgccgccgacctggtgccagagcacggcggcgcgaatgcctgccagcagggttgcgcgaactttcgcctgcacttgtgggctttgcagtacagcaggggaaccggtgacctgaatgcgcgggccaagcgggctaatcacatcaacatagatagcagccatcgcgctcatcagcgtttcggactgtaaatcgaagtgttcgagctggcgttgcaggccgttgatccggttgcccagagtgtcgagcgcgcctttcgctgaggagagtttgcgctcaagcaccatcaagctgagtgtgtagcgggttaattcggcgtttaagccctggcgactgctggcattgagcacgccgagcagggtttccagcccgacgcgcaggttggcttcgctaccgccaaaaaccgccagcgtcgagctggggttcatatcaataatactgttgagtgagacgtgtagcgcatcggcatcacaatgcccctggtgagcgagttgttgcaccaggcgtgccgactgacaaataccggccagggcgagggtgatgtcatagtaattctttgccacgttcactgcttccttgttttaagtaaagataataatcagaccggcagcggcagacgctgctcaataataccgccaccgaggcacacttcaccgttatagaagacggcagactggcccggcgtcacggcggcaaccggttcatcgaaaatcacttcaatgcgatcatcgtccagcgccttgacggtgcaagggatatcggtctggcgatagcgggtttttaccgtgcaacgcatagtgccggtgaatggttcgcgatcgacccagtgcaactgctgggcaatcaacccgacagacatcagccgcgggtgttcatggccctgagcgacaaccagaatgttgttttcgacgtctttgtccaccacataccacggttcttcggtaccttctttggtgccaccgatacccagacctttacgctgaccgagagtgtgatacatcagcccctggtgctcaccaatttcatcgccatcgacggtaatgattttgcccggttgcgccgggagataacggcccaggaactcgcggaatttacgttcgccaatgaagcaaatgccggtagagtcttttttcttcgcggtgaccagaccaagatcttcagcaatcttacgcacctgcggtttttccagttcgccgaccgggaacaggctttgcgcaatctgctcatggctgagcgtataaaggaagtagctctggtctttattgctgtccagaccacgcagcaggcggctcttgccatcgacatcggcccgacgtacgtaatgaccggtagcgatataatcggcacctaaatcttcggcggcaaattcgaggaaggctttaaatttgatctctttgttgcacagaatatccggattcggcgtgcgaccggctttatattcggcaaggaacagttcgaagacgttgtcccagtactcggcagcaaagttaacggtgtgcagttcaatgccgagcttgtcgcagacagcctgggcatcagccagatccgctgccgctgtgcaatattcctcaccgtcgtcttcttcccagttcttcataaacaggccttcgacctgatatccctgttgttgcaacagccaggcagaaacggaggaatcgacaccgccggacatgccgacgattactttttttgcggtttcagacattggatcactcacgacattgaacttcaaggcggcgtattctatcacgcagccttttagatgacaccctttgtaaaaggccagttaaaatcgccaatcatctccagcggataacgttgcccgctttgataacaacgaatactttccgccaccagcggcgaacgaagatttgacgcctgtaaaatttcttcggcgctgacccaacggcagcagtcgatatcgctgtcatgaggctgggtcgggcatatttgctcaagctcaatggcaaagaggaaacgcaaaaacggcgttttatctggcgcaatccactgatgcatacgaataaagtgttgcggctgcgcgctgatgccggtttcttcccacagttcacgggcggcggcttccactaaggtttcatcggcttccagatgcccggcaggttggttccataacgctttaccattaatcgtctcttcaacgactaaaaatttgccttctgcgtgcaccacgcaagcaacggtaacgtgcggtttaaacattttgcatccttaatctgtcacttctcgccattcaccattggcaagattatccaaagagtaatcacccatcgcatagcgaatcagtcgcagcgtggggaagccaacatgggcggtcatgcggcgcacctggcgattacgtccttcatataaggtgatcttcagccagctggtgggaatacttttgcgttcacgaattggtggattccgcggccataaccacgcgggttcgtcaaccagctccgcgccggcgggcagggtagggccatcatttaaggttacgccattgcgcaaggcttcaagtgcgtcttgtgtgggaataccttccacctgcacataatagatttttccggtgcgtttacccggctgggttaaacgcgcctgcaacgcgccgttattggtcagcaccagcaacccttcgctatcgcggtcaaggcgacctgctgcataaacaccctgaaccgggatgaattcttttaatgttttgcgtccggcttcatcggtgaactgcggaagaacatcgtagggtttattgaacaggatcacacgcgtgggctggttttcaggtttacgcctggtagaacgttgcgagctgaatcgcttaacctggtgatttctaaaagaagttttttgcatggtattttcagagattatgaattgccgcattatagcctaataacgcgcatctttcatgacggcaaacaatagggtagtattgacaagccaattacaaatcattaacaaaaaattgctctaaagcatccgtatcgcaggacgcaaacgcatatgcaacgtggtggcagacgagcaaaccagtagcgctcgaaggagaggtgaatggaaagtaaagtagttgttccggcacaaggcaagaagatcaccctgcaaaacggcaaactcaacgttcctgaaaatccgattatcccttacattgaaggtgatggaatcggtgtagatgtaaccccagccatgctgaaagtggtcgacgctgcagtcgagaaagcctataaaggcgagcgtaaaatctcctggatggaaatttacaccggtgaaaaatccacacaggtttatggtcaggacgtctggctgcctgctgaaactcttgatctgattcgtgaatatcgcgttgccattaaaggtccgctgaccactccggttggtggcggtattcgctctctgaacgttgccctgcgccaggaactggatctctacatctgcctgcgtccggtacgttactatcagggcactccaagcccggttaaacaccctgaactgaccgatatggttatcttccgtgaaaactcggaagacatttatgcgggtatcgaatggaaagcagactctgccgacgccgagaaagtgattaaattcctgcgtgaagagatgggggtgaagaaaattcgcttcccggaacattgtggtatcggtattaagccgtgttcggaagaaggcaccaaacgtctggttcgtgcagcgatcgaatacgcaattgctaacgatcgtgactctgtgactctggtgcacaaaggcaacatcatgaagttcaccgaaggagcgtttaaagactggggctaccagctggcgcgtgaagagtttggcggtgaactgatcgacggtggcccgtggctgaaagttaaaaacccgaacactggcaaagagatcgtcattaaagacgtgattgctgatgcattcctgcaacagatcctgctgcgtccggctgaatatgatgttatcgcctgtatgaacctgaacggtgactacatttctgacgccctggcagcgcaggttggcggtatcggtatcgcccctggtgcaaacatcggtgacgaatgcgccctgtttgaagccacccacggtactgcgccgaaatatgccggtcaggacaaagtaaatcctggctctattattctctccgctgagatgatgctgcgccacatgggttggaccgaagcggctgacttaattgttaaaggtatggaaggcgcaatcaacgcgaaaaccgtaacctatgacttcgagcgtctgatggatggcgctaaactgctgaaatgttcagagtttggtgacgcgatcatcgaaaacatgtaatgccgtagtttgttaaatttattaacgggagcgtaacgctcccgttgttttttgttaggctgctaacggttatcaaaattttatcaaaaaaagttatcaaaacccctcggtagttttggggtaggctggccggtcaggtggtagttctactactagtctcccacatagatattccttagctttttattattgctggcggacgctcgttaatatttaaggtcttcattgattaagacatccccaaagttagttatgtattcactgttattaggacaattatgaattaccactccttacacccgctcaaatattgttaaattgccggttttgtatcaactactcacccgggactcgccaggggacagccaacaggcattgggtgcaatcaccttagcgttcaggtacatgcggaatgtaaaaaaggccgcgagcgcggccccttcacatacatctttagtactgagactgtttaacctagggaattattatcgtattatattgcattacaactcccaacagtgacatatgaacttcctgctttactccacgactttaatatttcaaggccatgtgaagaacatatttcttgcactgcgagttcatcgagtaatccatagtaagaaacactttttgaatttttgtaaatgtatccgtaaagatgttttcttcctgtttcgtattttttgaagtatgagcttttatattgatttacaataagagtctcacctcctgattttagtaatctcttgatgctaagaactattttgtcgattgtatcccgacaaggaacggcagagagaacattagagcaaaggatgaaatcgtaacccccaattattttgtcgacatcctcgaaagcaactgtatttgcatttttataatatcgtgggacatagtcaataattttagttttaattcctctaataatttgctctctttcaagttgccttttcgagtctagaaaagtaacttcatcaaatttactgattaattcatcagaatatctaagttttccgcagccaaaatcaagggcgtggccatttttctcaatgcttctaatatactcgcaaagatatctagagggcatcgtatgaggttttgctgcattctctgagcgaatattaactccgtgcatattatagttcaaagcaagtaccattcaattaatgttatttttagtgaaaaattcttttattttatcgtccgggatttttccgacttgactttcagttctgggcttaactgtcaaagcaaagataataccactcactgagaatgataaaattacaaaaaagaataaagacagcaaagaaccttcaacatgaaaaatatccatttgtttgcaaaaaaagattattaggaaggaaattaatgcaattatcgaaaattcaaaaaatatccaaaaatagtatactttattccagaagagttcaatataatgtttgtcttcaatttttcttacttcagggtaatatagattgctcattacattgtgagcttcatctttatttaattttctgttgactccagctctccgtgataacggttttataattagatgcttatcccaaagatatcgcacccgaagtagtttggctgcattgttatgtaggtctaacgcaccgctaattaaatatgcaaaaatcgcaaaagcacaaggtaatataccaaaagatagtgcccaattaataaagctctcatgatctttaataggtgggacatacttggttggtaatgttattaaagggatgtattcgtaaataactagaagtatgcaatatattagcgtatttaagaaagttgctttatgaagtttaggcaacatttcattataatttttggggggttcgaacatattattcacctgagtcacgctttaggatagtgtaatggtaatatttaattaagtgtcattatatacttttcagtaggttagttacaattttttgtatctgttcaggctgacctagcttcgctgacagacaatattgtgatcagtagcacgtatcgaggaggagtagcgctacaaatttgacgctgggtgagaatctgaaattgatagaaatgaaataatgaaataatgaaatgatgaaatgatgaaatgatgaaatgatgaaatgatgaaatgatgacagagtgtccagtgggcacggatggtgtcttacgacatgcttaccttaatcgttcccagtgtgcctatagcagatattctaaacatgtcgataattcattacgcatatagtatcgaacatagaaaaaactgaagattcatcttattttgtatatactacctagcccaacaatgtagaggttaacgaaaaatgcgctcaccaatttgtcatcttttctcagcaattaattcatcaccatttaagattgcaccagagaaggagcaagatcttaaaacgatagttgacgacaaaaaaattataatttcagttgtgagtgaacctggttttaatatccgagtcaggaagaatgagagtaataattcacatgaaatagttctaacagtagcttcacttgaatatatttgggcattttccaatttcttttgggtttttacgcaagagtactccaaatctcagaaaaataatgatgagcactttgatttaacaggaaaaaataggcttaaaaagtctgatgaacttcttaaatgggcaaggaaaaacttgcaaacaacaggttgcgaatcatggcctaaaaaatgtcccaagccagaagcatatttacaaggaagcgaagactcacaagttgctagcgagatatttctttgtgctattgcttggattcttcatcatgaaataagtcatgttgttttacagcatccattggtcactacagcattctccactcaagaggagcgtgaagcagattcacatgctacaaaatggatattaggcaacctgtatgaatccgctcctgaattaaagaaacgtgcacttggcattgctacggcagtgctttgtatacaaagcttagaagttgaaaattacttctgtttacaaaatacacacccagctgcatatgagcgtatatattcgaatatttcatgctaccctgtcggaaatgaagagttgattgaagctctatgtacagtgatgcttcaatatcttttccatggcaaaaatatcaatgtgaatctagatggggagtccttttcatcgattttaggtgatcttctctgtgatatttcacgtcttaccagtaactgatatggctgtccgccgctcgcttaaagtggactttttagtttttatcatgtgcggtgagaaattcaatgtggcgttgagatgcttaaaggttcacaacgctactttgctccatcctttacctcgatcatcatgataacgatcggtttgttgttgtgttttatgaccaagtagtttttgtgtgtctaacccctgttctttatacagacgttcagataaagacctttgctcatggaatgtcgcaggtgaaccctctccccagtcaattcttgctaaatctctcgctttactaaaattcatcgtcaatgtattggctttaacctgcgctccgcgctctgcttgtgaagttgaacgaaaaaaatgcactaagtatgcactgactgcatagtcacggcagcgggctactacatcgcgtaaactccagttaatcgcattgaggcgaagagaaagaggaattgcgattttgctcccggtcttttcctgaatgacatgaagatgatcatcccaaatatcgctaaatttcatacgcgaaatatcacctaaccgctgaccagtaaccagcgctaacagcatggcatttcccatgtaacgatgagtagcgtctgcgatatcgaagatttttttccattcttcaaggctcagccgttgtcgggtaatttttcttcttggttgtttagtggctaatgctgggttatagccaggaggtacttctccgtagtgctgcgcctctttgaaaacatcaatcaggacggagcgaactacttgtgccattcttggccgcccagcggcgatatactcatcaagcaattgtgctatatctctgacatcaacggctgagatcaacttcattcctgctcgttctctgagcaaggatactggtttagctttttgtttataggtgttgagtcttatatcaccacttttaagcctgtcatcctggatcgcttgatagcgatctaaccaggttgacgttgtgatagcctttcctttgctggttgcgatcctgtcactgatagccagaatctgccgggttctttgttcagccaggcgagtgttggcctcagtggcaatagcgatagcttcagcttcgtttgttcccaaagcatggaattttcctgtcactggatgcttataccgccaatagactttatttaccttcctactataaagcggatataagttagggactgaaacattattcttacgcggtctggctgccattactcaaaatccgttgcaaaagtaatgagtcatttttcttgattacaggtgttaccaactccccaactaactcggcgtcctcacgcactcgccataaccggccttgtttcatggccggtggacaaaataaattctgcttagcataacgacgcaatgtggacacacttggaggattacttctgtatttttcagcagcccattcttcaagagttaacatttgaagcatatgcgatcaccttattactacactaactgcttagtctcagcatatcgaccctgcacggtcggttagtttctccacaaaacagagaagagcacctgtggccacagctatcaggatgggtcgggttattaacccgtcatccggggatactcttctctgttttgtaaaaagggcggtaccagaaaggactaaggaaaaaactggtaccgccaagactacacacagcataaagttgtggtgtcgggtgcccccggtgcctggcgaaggttgcacaccaggcgggtgggtatccacagaaggtcgattgtcagcctcaaccttaacccgcgtgcgctgagccgcattcaccacaacgctaaggattctctctggttgaaaatacttagctgttatgtgcctgtcttttcaccacttcaggctcggtggtatgctggagttctcacacagccagcaagcaaggaaacttaatgaaccagttttatgttcacgttcgtctatttgaagacacagccgaacagaccaaaaaatttgaagaattaatgcttaactttctgtaccagaaaacagttaaagagtctgacgatagctgctgcagactgattccagagggatatatcctcaaaagtacaatgaactgccaacaaatccttgatcaaacattttcaattgctaacagtgccggtgttgacgcaaatatatttgtctgtaaatttgaacaaagcgcatgcttacttccgtctgcttccttagttggtaacgatttcgttcattacgatcttacgcctaagcccatcaagctcgattcttaaagccttaaccattgtgtcgtgataaacacggctcaccttctctccattgcatggcagaggggtgagtgtgttagccatgaaattcatgaactcggttcgaccaggggcttgcgccccgcaagtctttaatgcctgttttgctaacaaaatgcgggcctcagtgcctgcatttggctctatctgctgcaaacgtttagcgtcttccagcaacaatgcgatcacatgcttcaaattctgctcattcatctattctctccactgaaatcatccgctaacgaatcatcccggtcttcgtacgtaccgggcgggctacttcgtgggcgtcctgcctgtttgttgtttctcttgggtacattatgtatctcaaaggtacattgtcaagtataaaaaaacctgccgaagcaggttcataaacattgattaggctttgattttgtatcttcttggttttcctgagaaaatcacagtaccaattatagagcaattaccgttgatcttaatgtaaggctcaggccagtttgggtttaacgctttgagataacgctgtgtcccatcttctatcaaccttttgaaggtggtttcacctgtatcgtgcatcaatgcaataacgtcgtcaccgtggcaggcaggtacttcaggatcgacaaaaatcatgtctcccgggcggtactcatcaatcattgaatcacctattacccgcaagatataagtcatttccccacagggtacagggcagggatacgtttctgctgtgctcaaatcaacctcagaatatccaacttctttccatgctccggcctgtacccatgatatgacagggactaatgtgatttgtttattagtgattgaaacatcaggtttttttgtgatgttcgttgtctggtgttcttgatcgagccatcctacaggcaggtcgaaacatttttcgatgtgtcgtgccatgctgtcaccgatatttttagtagcaccatctcccataaacctgctggtctgggttggctcgcgatcaatcatagtggcaaaggaagaattcccgccaacaccatctctcagttttctggcgttagaccgccggatgtcatggattgttttcataacgaaattaaaacccttgtaccgttaaggtacaagtatcttgaaggttcatttcaatcatgtaatatgtacaccggaggtacatattgtatgaaagcgtattgggactctttaaccaaagaacagcagggcgagttggccggaaaagttggctcaacacctggctacttacggctggttttcaatggctataaaaaagccagttttgtgctggctaaaaaacttgagcaatacacatcaggtgcaattacgaaatctgacttaagaccggatatctatccgaaagattagcagaacactttcaatttttaaccacagaacgatgaggctaatcgtgggtaagcatcactggaaaatagaaaaacagcctgagtggtacgtgaaagctgtcagaaaaactatcgcggcgttgccgagtggttacgctgaagcggctgactggctcgatgtaacagaaaacgctttattcaaccgccttcgtgcagatggcgatcagattttcccgctgggatgggcaatggttttacagcgtgctggtggcactcacttcattgctgatgctgtggcgcagtctgcaaatggcgtctttgtgtctcttcctgacgtcgaggatgtggacaacgccgatattaaccagcgtctgctggaagtcattgaacagatcggcagttattcaaaacagattcgttcagcaatcgaagacggtgtagtggaaccgcatgagaagacagcaattaacgacgagctgtatctctcaatttcgaagctgcaggagcatgcagcacttgtctacaaaattttttgcatttcagaaagtaatgacgcccgcgagtgtgcagctccgggcgtcgtggcgtcgattgcttctggttgtggagaaactaacgcatgaacagtttaacaacacactaccgtcgctcgcaactgattgcgcttcctgtaccgggtggaaaagcgaaggtggaatattgctatgcagtgaatgtaccaggtgacagggaaattgtaacccacagctttgcagagtgggctgtgggtgatttcaaccggcagaaggagacagtcctttgcgacaagttaaccgctggttcaaagatcactacggagtgcccgtcagagtcattcgttgggagccggaaacacaacgggttatctacctccgcgaaggttatgagcatgaatgcttcagcccgctcgaacagtttcgtcgtaaattcagggaaatagaggtcggtcatgagcactaaattaaccggctatgtatgggatggttgcgctgcatcaggcatgaagttatccagcgtggcaattatggcccgcctggctgatttcagtaatgacgaaggtgtgtgctggccatcaattgaaaccattgcccgtcagattggcgcggggatgagtaccgtcagaacggctatcgcacggctggaagcagaaggctggttaacgcgtaaggcgcgtcgccagggtgatggttcatcaccccactgtgccgtggtggatgaatatcacgagcacgccacagatgcgctttacaccacgatgcttaccgggatgggggcgcgacgccagccactgatgtgggccattaccaccgccgggtacaacattgaggggccgtgctacgacaaacggcgggaagtcatcgagatgctcaacggctcggtgccaaacgatgaactgttcgggatcatctataccgttgatgaaggtgacgactggaccgacccgcaggtgctggaaaaagccaatccaaatattggcgtgtcggtttatcgcgaatttttgttaagtcagcagcagcgtgcgaaaaataacgcccgtctggcaaacgtctttaaaacaaaacacctcaatatctgggcgtcggcgcgttcggcgtatttcaacctggtgagctggcagagctgcgaggataaatcactgacccttgagcagttcgaggggcagccgtgcattctggcctttgacctggcgcgtaagctggatatgaacagcatggcgcgactttatacccgcgagattgacggtaaaacgcattactacagtgtggccccgcgtttctgggtaccgtatgacacggtgtacagcgtcgagaaaaatgaagatcgccggacagccgaacgctttcagaaatgggtggaaatgggcgttctgaccgttaccgatggtgcggaggtggattatcgctacatcctcgaagaggccaaagcggcgaacaaaatcagcccggtcagtgagtcacccatcgaccccttcggggcgaccgggctgtcacatgaccttgctgatgaagacctgaaccccgtcaccatcattcagaactacaccaacatgtccgatccgatgaaagagctggaagcggcgattgaatcggggcgctttcatcatgacggcaatcccatcatgacctggtgtatcggcaacgtggtcggcaaaaccattccgggtaacgatgatgtggtgaagcccgtcaaggagcaggcggaaaacaaaatcgatggtgcagttgcgctgattatggcggttggcagagccatgctgtacgagaaagaagacacgctgtctgatcacattgagtcctacgggatccgctcgctttaactgaggtaattatgatcatgctgattctcgcgcctctggtgggcgtgctgggtgcgcttttgctggcgtatggtgcctggctgatttatcccccggcgggttttgttgttgccggggcgctgtgcctgttctggtcgtggctggtggcgcgatatctcgaccgtacacagtcgtctgtcggcggaggtaaatagtgttcttttcgggattatttcaacgaaaaagtgacgcaccggtgaccacgccagcagagctggcggatgccatcgggctgtcgtatgacacctataccggaaagcagatcagcagtcagcgggctatgcgactgacggcggttttttcctgcgtcagagtgctggcagagtcggtcgggatgttgccctgcaatctgtatcacctgaacggcagcctgaagcagagagccaccggcgaacgtctgcataaactgatctccacgcatcccaatggctatatgacgccgcaggagttctgggagctggtggtcacctgtctgtgcctgaggggaaacttttacgcctacaaagtgaaagcatttggcgaagtggctgaactgctgcccgtcgatcccggctgtgtggtatatgcgctgggaaggtgtcagcgatggcctgaaggtgaccgccgggagtgttattcagcgcgatgacctggtgcagtacacgacaactgacgatgcaaccagctccggtggtgtcctgcgcgtgccgatcgcctgctcaagtgcaggtgcggtcggtaacgctgacgacggtacggcattaatcctggtcacgccggtgaatggtctgccgtcttccggtgtggctgacaccctgacaggcggatttgatactgaagagctggaaacgtggcgcgcccgcgtcattgagcggtattactggacgccgcagggcggggctgacggggactatgtcgtctgggctaaagaagtgcccggcattacccgcgcatggacataccgtcacttgatgggaacgggaactgtcggtgtgatgattgccagcagtgacctgattaatcccattccggaagaatcaacggaaacggcggcaagacaacatatcgggccactggccccggtggcaggctctgatttgtatgtgttcaggccggtggcacatacggtggattttcatatccgcgtgacgccggacacaccagaaatacgggctgccattaccgcggagttgcgttcgttcctgctgcgtgatggttatccgcagggagaactcaaggtatcgcgtatcagtgaggcgatttccggtgcgaacggggaatacagccatcagttgcttgcaccggtggacaatatctccattgcgaaaaacgaactggcggtactggggacgatttcatggacgtgacaaacgatgattacatccgcctgttatcggcactgttgccgcccggtccggtgtggtcagccagcgatccggcgattgccggtgcggcaccgtcattaacccgtgttcatcagcgtgcggatgccctgatgcgggagctggatccgcgcaccaccactgaactgataaaccgctgggagcgtctgtgcggtctgccggatgaatgtattccggcgggaacgcagacccttcgccagcgtcagcaacggctggatgcgaaggttaacctggcgggcggcatcaacgaggatttttatcttgcacagcttgctgccctgggcagaccagatgccaccatcacgcgatacgacaaaagcactttcacctgctcatcggcctgtactgacgcggtgaatgcgccggaatggcggtattactggcaggtcaacatgccagccaccaccaactccacctggatgacatgtggcgatccctgtgattccgcactgcgtatctggggtgacaccgttgtcgagtgtgtgcttaacaaactctgcccgtcgcatacctacgtaatttttaaatatccggagtaatccatgcatcgtatagacacgaaaaccgcgcagaaggataagttcggcgcgggtaagaacggttttacccgtggtaacccccagaccggcacgcctgccaccgatctggatgatgactactttgacatgttgcaggaggaactttgcagcgtggtggaggcatccggtgccagcctggagaaggggcggcacgaccagttacttaccgcacttcgcgcgctgctgttaagccgcaagaatccgtttggcgatatcaaatcggatggcactgtgcaaacggctctcgaaaaccttggtttgggagaaggagcaaaactcaatgcagcaacggctacattaggacgcaccggtttcatagctataccggttatgattggtggtattgagcaatcagtaatcattcagtgggggtggaatgccgcaaaagcatctgcctctgggggggatggaaatacagttgtattcccggttgcgtttaataatgcctgtgttgccgttgttgcaaattatgacaatgtcagcgcacctatcaatgcagtggcaacggggggatatacaaccacttcgtttttattacggtgcgcagctcaaacgggtagttattactataactggattgctattgggtattaagatgaaaatatactgttgcttaaataccgttggtttttttatggatggctgtggcgtcattccgccagattctaaagaaataacggcagaacactggcagtcattattaaaatctcaagctgaaggaggcgtgatcgatttttctgtttttcctccttctattaaagaggttatccgtactcatgatgatgaagtcgcagatgcgaactttcaaaagcagatgcttatctctgatgcaactgattttatcaatagcagacagtggcagggtaaggctgcattgggaagacttaaagaagatgagctgaaacaatataatttgtggctggattatctggaagcactggaactggttgatacatccagtgcgccagatattgaatggcctacgcctccggcagttcaggccagatgacatccggcgcggtgctggtatctgttgccgtcaccgcgtcaatgtaatccagcacagcgttaagtctggttgtttctgcctgcgtcagtttacgtccggcctgcaatttcagttgaatcagactaatggaagccattgcagcatcaatcagtgactggcgctgtgcttctgccgcgtctactgcggcgctatgctgtgcttcagtatcggtcacccatttctcaccatcccatttatcgtatggagataaaggggcgatagtggttgtattttcagggtaatcacccggagctttgatttcttttgattctccagttttggtgctatagaccgtttcaccgcgatggtctggcacatattcccatgagttaaaatctgcagaacggcagattgcataaccagccttatgtgtaccaggggcatctaaacaggaacatgccggaatgccgacaccaacggcaagatattcatttgaagtggaaatatattcccgtgtttcaccatcgtagttataaacggtaacatcccctgcctttgttgcaataaggtcactatttaatattgctttatgcatcaggctgccctcacgatatagttaaatgcaatattacgcggacgcgtttctgaggctgcggcacctaaaccatccactgattgtttatatgttttaaaggttccataatccggggctggtaatccggcatcgtttgtgtttcctcttttgataatgtcagtgccactatttacccatatttcatcaaaatagaaattaatcgttgcatcagtcacaatcgtggatcttgacggtaatccatgagcatgatcctccgttgcatacccctgaatacttaaaatagagcgacctgtatcaatcccccgcccgtcatcccagccacgaataaactcaccacgtaaatcaggcaatttatttgtcggataagcctttgccagttccgggtattcttcagcagaaaaagcggcaccattgcatttcagccagcctgttggcggagtggctgaaggccacggaaccgggacaccaacaggtaatgcagagccttctcccaaaccaacgtttatgaaaatgaagaaataacaagcaaatggcatcattcctgcttttaccagggggatttaacatgcttattggctatgtacgcgtatcaacaaatgaccagaacacagatctacaacgtaatgcgctgaactgtgcaggatgcgagctgatttttgaagacaagataagcggcacaaagtccgaaaggccgggactgaaaaaactgctcaggacattatcggcaggtgacactctggttgtctggaagctggatcggctggggcgtagtatgcggcatcttgtcgtgctggtggaggagttgcgcgaacgaggcatcaactttcgtagtctgacggattcaattgataccagcacaccaatgggacgctttttctttcatgtgatgggtgccctggctgaaatggagcgtgaactgattgttgaacgaacaaaagctggactggaaactgctcgtgcacagggacgaattggtggacgtcgtcccaaacttacaccagaacaatgggcacaagctggacgattaattgcagcaggaactcctcgccagaaggtggcgattatctatgatgttggtgtgtcaactttgtataagaggtttcctgcaggggataaataaagttaaagacactttgtgtacaaaagaaagtaaaacaacagcaacttgttgcaattttatcaataaaagtagtattgtcgtgaaaaattgattaaagattaatattatgcatgtttttgataataatggaattgaactgaaagctgagtgttcgataggtgaagaggatggtgtttatggtctaatccttgagtcgtgggggccgggtgacagaaacaaagattacaatatcgctcttgattatatcattgaacggttggttgattctggtgtatcccaagtcgtagtatatctggcgtcatcatcagtcagaaaacatatgcattctttggatgaaagaaaaatccatcctggtgaatattttactttgattggtaatagcccccgcgatatacgcttgaagatgtgtggttatcaggcttattttagtcgtacggggagaaaggaaattccttccggcaatagaacgaaacgaatattgataaatgttccaggtatttatagtgacagtttttgggcgtctataatacgtggagaactatcagagctttcacagcctacagatgatgaatcgcttctgaatatgagggttagtaaattaattaagaaaacgttgagtcaacccgagggctccaggaaaccagttgaggtagaaagactacaaaaagtttatgtccgagacccgatggtaaaagcttggattttacagcaaagtaaaggtatatgtgaaaactgtggtaaaaatgctccgttttatttaaatgatggaaacccatatttggaagtacatcatgtaattcccctgtcttcaggtggtgctgatacaacagataactgtgttgccctttgtccgaattgccatagagaattgcactatagtaaaaatgcaaaagaactaatcgagatgctttacgttaatataaaccgattacagaaataaaattatttattaaagtcacatttaagacgtaataccctacagggtaaaaattttctctgatcttaacttctgcaaatgttaactgctatttttatgctaaaaatggttatcaaaactcaaaaacacatgtttataatcaatgagttatagaaatgctaagggctaatgagttatatgcaaattagtaaaattatgttgctatgtcagatagttacgatttagtcatctaactaatgctgcgccatatgggttggactgaagcggctgacctgattgttaaaggtatggaaggcgcaatcaatgccaagaccgtaacttatgacttcgaacgtctgatggaaggcgctaagctgctgaaatgttcagagtttggtgaagcgatcatcgaaaacatgtaatctctccatgtgttaaatattgaaacgggcgtataacacgcccgttgttttatttatgtggatattattaatagcatatcgagcatatttatatgaagcccattacttgagcccatatgggcatatttttataatgcaactattatgtaaacatttatttgttattttgctttctcctggaggacactcttgactgcttttgagtaaactccataaatccttgttgaatggtgcgatgtgataaatagtaataggatattctttatccttaaggataataccagacttaaccggtgtaaatatactgccaggagggagaaatatagtagattgataccagatgatcattttcatattaccccatatggctgaaaaagatataccacatgtaggttgaattaccgtgtcaattactatccacttcatttgttatgtcttatcccacggtatttaatatggttcattaggatgtttatttcttgattttgcatatgagtatattacccccccctcaaaaaaataaattaattaaaatgatggcttatataaaataaaatttaaagcaaggaatctcaatggatgttaaacaaaatgagattttgtgaaagcaataaattattgacttcgttttagatttgtttagctataatgttatacattcaaatgactgaacatcctgtaattaaaacatagcctttatgctactttgtgccaatttgctaaacattatggttgcctttttatataacgataataatgaatataagcatgacatgagaataaggtttcaatttttgagttatataggaatgatttaacctgttcctggctaaaatacatataaccggatgatgactaaaccaaaatacatgtgcgttaagtattgaaacggacgtgtggcacggccgttgtttttataaatatgttaaccgttataaaataacgtatcaaaagtcaagtgatcacatttcaaatatcaagttgatagtattagtctggtgattatttatgggtgacaataaaaagacagtattaatcatccatagagatagtctctgcacttttatttccattatgctaatgccttactgaattatgaagcatttcttaagtatccaactttagctagattaatggtttattattttctacatcttcaatatataaaagcgtattatcaatggcgtagtaactgcgtttgttatgattaacatcagtaacccaccggaaaacgcccgcgcctgccagtgttgaacagtattcccgaaatgtagattttccgcaaatatgaagcaatgcggcctcttttattttagcagggttcttggtcgtactaacttttaacaggttcctggttcctcttaataacaaaaccgtatcatcgtgagtaataattctgatgttatccgtagccagataataaatgtaatgtgcaatacggtgatgttttaattctgaataaaaccaggagaagttttgctcttttctcacttgctcaaacatcttttgaaaaacaacgacctgatccatcaggataataacctcttgttagttgtgagactgcgtagtgtgcacgatcggttttaccacttcaatctggtctgtcctttggctgtgatatgtacagagtgtgatagagggaatatctgaattctcccggtgagcattttgcaacggaccagctccggtacaaacgctgttgtgggttcagattataacattctgtctaaggggcgggataaaggtgaaattagggggcatgaaagatgactttataaccttgctcaccccagtgttgtaaaagttcgttttgccttctcgttggtgccatgcctgtccagacaatcaatgtttgcgtcgggaacagttccgggcgcggcgattcaatgggatcagcaagaacagaaatgtgccatcctgacaatgataaacgccatgcttccagccacaatcgtgctctctcttcaacattccacgccatcagaatggcttctttaccgggcttacggcgcatttcgaaaagcgaggttgctgcgtattcaattaatgcgccgtcaaacatactgctcataatgcgggaggtgttgtgatcaagcacgagacgctggcgaacaggaaggtaaacatgattaatcaattgatctactgggtactctcgacccagtgaaataattctcgcgcgtagtttggcaggattagccatgcgaagaattgacatcatctcttcttgcaggcggctccagtcatcttccgtatcctggctggtggtttccagtaatgctttaactttgcctacagggacgccattacttatccaacgcttgatctcttcgatgcgttgtatgtcttcttcatcaaagagtcggtgtccgccttcactgcgctgtggttttaacaaaccgtagcggcgttgccaggcccggagagtgacaggattaatcccgcaacgttcagcaacatcaccaatgctgtaataagccacaattcctccttgcggtcacaaatctccgtcgcctgtacacgacccaataatactttgtacaatatacgctaaaattgtacaaagtataaataagatttcagctaaattggatgaaacattatttttaatgtggattaaatttaaacgtaacgtattcattttcacgatgatttactgaaatcatgtgaaagaatgtgctgaaaattattttttctctggccacgctatggaagggataccattcaatttagctttagcaaacagatctccctgaaacatctcaattcctgcggattcaagccacatccactcttctggtgttgccacgcccatagcactgacttgaatttcaagtgatgtacagcattttatgatcgcctgaataattgcctgccgtggcccacttttatgaacattggtaatcaattcctgactgattttaattctgtcaggctggaagcgtgacaggagtaacaaaccagcaaaacctgcgccaaaatgatcaattgctacactgataccagcagcctttagcgatttaatcgcttcggcaaactcatcaaaccgagatatgacttcactttcagtaaattcaacgatgatttgttcaggcaccagagcattggcctttatttcattaagtaaaaaagagactgcgtcaggttcgttaaccagggtcataggtaatagattgattgaaatcattttatcaccgagctcaagtgcgtgtgccatcgtgaatgcaagcgccttacttttgagatccgctgtgtagatttccccgtctttacgctgcccaaccgctatggctgatgggctatcttcatttttttgcacaatggcttcaaaagcgattatccgccgcgataagggatcgacaataggatgaaaggcaaagtggtcgtttatagttggtgaaagggcacaggaatcaagttctttatcagatccgtcagcgataaaaagccaggagtcttcggcagggatctcgaaataggttgattgttcggttgcaaggacaaaagtacgaaaaaattgtagcgctctgtcatcataagttagctgaaattttgatgtgcctttgtcgaatacggcctgtaaaacgtcatctcgctcgtgcaggcgcaaatcaaataattccattcccgctttgccaaaacggcgagcaggcgcgtaatcgcacagcagctcaacaatattatagtgccgtggatcctggcatatagcccgatatatcattttaacctgttcttccggaccttccagaagctggaaaaaatgagaaccattaaacagtaagatccctgttacgtcagactgcatgttcctgcgatttgctatcgaaaccatttcttcgatttttttgacaggttcgtcgtcacgtatatggctacgataaataagggtggtaagcattaacaatccagggtaatgggtgaggcgagagtaagacggtaacagacatatcttcttgtgtctttcttttaataccaaaacataaccgtttctttacattgataaaaaatggaaaaagttgaacactagttggcgaaaaatcttgtatagattgtcagttaaatgatgcaatatgttttatcataacacattgttttatatgcattagcactaattgcaaaaaattaatttatcattctgtacacatatttcgtacaagtttgctattgttacttcacttaacattgattaacatttttaacagaggcgtagcatgcatcaaaattcagtgactttagattctgcgggagcaatcactcgttactttgcaaaagctaacttgcatactcagcaggaaactctcggggaaattgtgactgagattttgaaagatggacgtaatctgagtcgaaagtcgctttgtgccaaacttctttgccgactggaacacgcgactggggaagaggaacagaaacattataatgcactaattgggttgctttttgaataatgcaacagcctgattatttaacaggttagctatgaagtcgttatgaagacatctgataatgaacgtataaaatatgaaattactggccaggcggtgctccagatactgcgcatgaagataaatttttcattgcagactcttattaagcaattactcgtaatgaaatcggctgaggaagatgctttccgacgcgatttaattgacagcataattcgtgattttagcaatagtgattcaggagggccaaaccgaagaacagcgacagctgacaataaaagtatgttcaatggtaagaaaataaacagaatacattaaaatttcataagtaagatgagaggttaccatgcttgaagatactacaattcataatgcaataactgataaagcgttagcaagttactttcgcagttcgggtaatttgttagaagaagaatcagcagtgttagggcaggctgtcaccaatttaatgctttcaggcgataatgttaataataaaaatattatcttaagtctgatacactccttggaaacaacaagtgatattctcaaagctgatgtgattagaaaaacactggaaatcgtgttgcgatacacagctgatgatatgtaacttctaattattaagtataagtttatagaaaactcattcatcttatttttgtctgtcgctttagactatacacagcataattttattgggttaatatttctacgaggctgacatgaataattcaatcccagagagatttatttttcaatgtgctttgtttaaaaatctcgagagggaggtgttcatgacgcatgggtatgttgatagtcatattattgatcaggctttacgcttgcgtttaaaagatgaaaccagtgtgattctttctgatctctatctgcaaatattgcagtacattgaaatgcataagactacactaacggatatcattattaatgacagggaatccgtgctctcttagaacttgagtaaggttttagaataaacatcagctgtatcaccatgctgatgcaaagtgagcatttcaggcgttatgctttcttattatgtccgcaatatcaggtgtcaagaatggagagttctcgctctccattcttgacgcctgatatcccgcctaacttattttgtactgcctacattatgctcaataattaatgggttagatcaagatggagaaaattttatcttcggcgtggatatttcttatgctctctaccatgctctctgtagatgccagcgcgagcgaatgaatggcattttcatgtattaaaccctttggccgggacaagcaaatgcgcaatacactcatacccatcctcgttgcgatatgcttgtttattaccggtgtcgctattttgaacatccagctctggtattccgcaaaagcagagtacctggcgggagcgagatatgccgccaacaatatcaatcatatacttgaagaagcgtcacaagcgactcaaacagcggttaacattgccgggaaggaatgcaacctcgaggagcaatatcagcttggcactgaagcagctctgaaacctcacctgcgcacaatcatcattctcaaacagggaatagtctggtgtacatccctgcctgggaatcgggtcctgttgtctcgtattcctgttttcccggacagtaatttactgttggctccagcaatcgacaccgttaatagattacctatcctgctctatcagaaccaatttgcagatacgcgcattttggttacgataagcgatcagcatattcgtggggcacttaatgtacccttgaaaggggtaaggtatgtattacgcgtggcggatgacattattggaccaacgggtgatgtgatgacgcttaatggacattatccctataccgagaaggttcactccacaaaatatcatttcactattatctttaacccgccgccactctttagcttctacagacttatcgataaaggctttgggattttaatatttattctgttaatcgcctgcgccgctgccttcctgcttgatagatatttcaataaaagcgcaacgcctgaagagatcctgcgacgggcaataaataatggggagatcgtccctttttaccaacctgtggtaaatggtcgggaagggacattgcggggagttgaggtgttagcccgctggaaacaacctcacggtggatatatatcacccgcggcatttattccacttgctgaaaaatccggattaatcgttccgcttacgcaaagcctgatgaatcaggttgccagacagatgaacgctatcgcgagtaaattgccggaaggttttcatattggaattaattttagcgcttcgcatattatttcgccgacgtttgtcgacgagtgtttaaatttccgtgacagttttacccgccgcgatttaaaccttgttctggaagtcaccgagcgtgagccattgaatgttgatgaaagtctggttcagcggttgaacatactgcatgaaaatggttttgtcatcgcactggatgatttcggtactggctactcagggctttcttatcttcatgacctgcatattgattatatcaaaattgatcacagtttcgttggccgcgtaaacgcagacccagaatcaacccgaattctggattgtgtattggatctggcgcgtaaactttcgatcagtatcgtcgctgaaggtgtcgaaacgaaagaacaacttgactatctgaaccaaaattatatcacatttcagcagggttattatttctataaacctgttacatacatcgacctggtcaaaattatcctttctaaaccgaaggtgaaggttgtggttgagtgaaaattgatcagtaaggccatagtgcggtgtaattatagacagctaattagctcgttgcctcttgttactattgttcattattttgtttgctataattgtttgaaagttttgacaggattgccattagtagcatgaacaatagtaataatctggattatttcactctctatatcatattttccattgcatttatgctgatcaccctcctggtcatccttattgcaaaacccagtaccgggctgggagaagtgcttgtgacgataaatttgcttaatgcccttgtttggctggcgatcaatctggttaatcgattaagagaaagactcgtcaaccacagggatcagcaataatctttcagtttctcactgtcagtatgcggctgaatgggttgctggcagtgaacgcctggatcattgaaggaaaggcattattgcgcaaatagttgtcaaccctggtgttatcacggttgtttttatatatcaccgaaataatcctcatcgcaactattaacaattttgatgtcgaagagttatttgttaaacaaaatcgtcacctcaaagtgatcaatgtcatgaaaataaggtgaaaaatgataatgccgacttatttatcatttatatattgtcgctgtttatctatttaaattttttgtgcttttgtttttgtctttaccctccgttttggtaatctgagctcataggttatttgaccaggaatgtttgttaatccaatgaatggatggttaatctatgaaactgaaaaaactccccgggtttagtttgggacttattgctctggcggtgggtaatgcatatgcaacacaattgttggatgattatagtataatttcctatatgactgatgaagaatcgccgattgaaatcaaagataataatccgataagtaatggagagtatctaaccactgaagacgaaagccatgctgtgaaagtggatgacggtgtaactggatatataaataatgccagtgtgatgactagtggtgatggatcttatggtatttctgttgatagtcaaaacaaagtattatatataagcgatagcgatattaagacctctggaagcgtatctgacaaagaaaatggagggataacagccagcgcagtagtcagtgaatttggtggcaccatctttatgaatggtgataattcagtcgagtcgggtggggcatattcagcgggacttttaagccaggttaatgattctgaaaagatggtaaataacacccgtcttgaaaccacagataaaacgaacattgttacctctggggaaaatgcagtaggtgttcttgcatgttcaagtcctggagagtctcgaacatgtgtcgatgctgtagatgatgaagttagtgattctaacagttacgaagttattagccgtgctgatttaaaaatgaatggtggttccataacaactaatggcattaatagctatggtgcttatgctaatgggaaaaaagcatatattaatttagattatgtggcacttgaaactgtggctgatggaagttatgcagttgctattcgacaaggtaacattgatataaaaaatagttctattacaacaacaggcactaaagcccccattgcaaaaatatacaatggtggagagttatttttttccaatgtcaccgcggtatcaaaacaagataaaggaatatcaattgatgcatcaaatatcgattctcaagccaaaatagcactattaagtgttgaactttcaagtgctttggatagtattgatgttaacaaaactacaacggatgtaagtatccttaatcgaagtattatcacacctggtaataatgttctggttaataatactggaggtgacttaaacataatttcgtccgactctattctaaatggagcgactaaactcgtcagcggcacaaccacgctgaagctttcagaaaatacaatctggaatatgaaagatgactccgttgttacccatctgactaattcagacagtattatcaatctttcgtatgatgatggtcaaacatttacccaaggaaaaacattaaccgtaaaaggtaattatgtcggtaataatggtcagcttaatatccgcaccgtattaggtgatgataaatcggctacggacagacttattgttgagggtaatacttcgggttcaactaccgtctatgtgaaaaatgctggaggaagcggcgcggccacgctaaacgggatcgaactcataactgtgaatggcgatgaatctccagcagatgccttcagataaggtgatgcaaggattgcagctggagctttcgaatatcaactaaaacaacaaggcaaaaactggtatttgacaagttatcagtcagtgaatgaggaggataacagctcagagggaaattcagaatcaacagaaacgcctacccccgtcctgcgccccgaagctggaagttacgtcgctaacctggcagctgctaacactctttttgttatgcgtctgaacgaccgtgcgggtgaaacgcgctacatcgatcctgtaactgaacaggagcgttcaagccgactttggctacgtcaaattggcgggcataatgcctggcgtgacagcaacggacagttgagaacgacctcgcatcgctacgtctcgcagttagggggcgatctgttaaccggtggttttaccgatagtgacagttggcgtttgggagtgatggctggttatgcccgcgactacaacttaactcattccagcgtgtcggattatcgttcgaaagggagtgtcagaggctatagcgcagggctgtatgccacctggtttgccgatgacatcagtaaaaaaggcgcatacattgactcctgggcgcaatatagctggtttaaaaactcggtgaaaggggatgaattagcctatgaatcctatagcgcgaaaggtgcaaccgtctcgctggaagcgggttacggttttgccctgaataaatcctttggtctggaagcggcgaaatatacgtggatcttccagccacaggcacaggctatctggatgggcgtcgatcataatgcgcacacggaagccaatggctcacgtattgagaatgacgcaaataacaacatccagacccgactcggcttccgcacctttattcgtactcaggagaaaaacagcggtccgcacggtgacgactttgaaccttttgttgaaatgaactggatccataacagtaaagattttgctgtctcaatgaacggtgtgaaagtcgaacaagatggggcgagtaatttgggggaaattaaacttggcgtaaatggcaacctgaatccagcggccagcgtctggggaatgtgggcgtgcagctgggtgataatggctacaatgacaccgcagtgatggtgggcctgaaatataagttctgatcccgccgttagctaaaaaaccgcgtcgtattcatcgacgcggtacatatgaaatattattttttgccgatagcacgcatggtgtcatcaattgccgtgatcaacagcatttgcgggtctttagcgcaaacctgattcagtttttctaccactttggcgctcagttccggagattgctcaatttttaaatcacggctggcaacgctggcattacccattaccgcaacaatttctgcaacctgtgcgctgtcagtttttgccatttcgttggcttctgcgcaagtaatataggtttctgacggcaaaccgtttttaatattgtagtcctgcgcccaggtcattggtgcgaaaacaaacaggcccgccagtaaagcaaattttttcatcatcattccttatttcattttacccagaattgcaccacccgtaccgccaatcacggcacctttaatcgccccttcgaggccattgccggtcagaacgccagtgacagcaccaacggcggcacccacttttgcacctttacgcgcatttttaccgtcgcggcctttttctgttactgcaccaacaccagcgccaacagctgcacctttcagtacgccattaacaccattgccagtaagtaaaccaacgcctgcgcctagcaatgcacctttcgtggtgcggttcatatccgccatcgctggcgtggagcagaacaatgctgagataagcccgaaggcaagtatttttttcttcaacttagatgtccggtattaagtaagttgcacacacaataatttcgtcttcaattaagatctgcttaactaaagaacgctcgctattattcagataattcaaaatgagcgtggctgtgatgataggaattatgttttttacgtgaatgagaataatcttaaatgaggaataactcattgattgacaatatttttattcaagaagtgtcattgactgttaacgcaatgttgtaaaggtaagataatctgatttatcaatattattgtgtgatttttatgtgagcagaagatattcatcagcaacgattacattagtcattttattttgccgacggcctcattgtcgaaagataagcgtacgacagtattatcagaaaagagtgattttttatccaactacacttcagcgcactgcgtgtaaaaaatgcctctttcttatgcgggatatcatcatttcatcatgatgtctttggtgagcggtgaacacaatacacctgcgctgtctcttcaggatgaatcccctggtctggtgcctgcgggctgatgttgcagcagagcttaggtcacttagacgctactatcatttatccaatggcatggaatcgaaatcagtcgatacccgcagtatatatcgtgaactgggtgcaacgctgagttacaacatgcgcctggggaacggtatggaaatgaaccctggctgaaggcggctgtgcgcaaagaatttgtcgatgataaccgggtgaaggtgaataatgacggtaatttcgtcaatgatttgtcgggcagacgtggaatataccaggcagctattaaagcctcattcagcagtacgtttagcggacatctcggggtggggtatagccatggtgccggtgtggaatccccgtggaacgcggtggctggtgtgaactggtcgttctgaccatcaacgattaaactgcgcttcggcgcagttttcgtttacaggatgttgaaagggaaaattctggggcaaaaaaagcccgccagttacggcgggaaacctcatcctatgggagaacaatgaataatgaaattgcggggttatcatctcccagtatatccatactaacaataaggttatttactcaaccaggcataaacattttgttttgtgcgtgggaacagccttaaggtgtaaagggggaggtggaaatagcaatgaggagtatcagcaagaatactcgccgctttaccacaacgtggatgagagggatgaaaaactcaaggcagagataactctgccttgaagataaatgcgcttttacagcgggcttatttcagctcttctgcttccggtaaggtcacgttcagctcaagaatagaaatatcgccatctttttgctcaagctgtacggttaccatctcaggatcaatttgtacgtatttacaaatgacctcaagaatatctttacgcaactgcggcagataatgcggttctgcatcgctgcgacggcgttcagcaacaataatctgcagccgttcttttgcaatgttggctgtgtttttcttccgcgagagaaagaaatcgagtaatgccataacttatcctccgaacaagcgtttgaggaagcctttcttctcttcttcaatgaagcggaaaggacgttcttctcccaacagacgttctacggtatctgcgtaggctttacccgcatcggcgttaatgtcgagaatgaccggttcaccctggttagaggcgcgcaatactgattgatcctctgggatcacgccgacgagtttgatgcgcaggatctccagcacatcttccatgctcagcatgtcacctctgcttacgcggcctgggttatagcgcgttaacagcaggtgctctttaataggctcttcgccattttctgcgcggcgtgatttcgacgccagaatgcctaaaatacggtcagagtcgcgtactgaggagacttccgggttggtggtaataatggcttcgtctgcaaaatagagtgccattaacgcaccggtttcaatccctgccggggagtcacaaacgataaattcaaaatccatcgctttcagatcatcaagaactttggcgaccccttcacgggtgagggcatctttatcgcgtgtttgcgatgccggcagaatatagagattttcagtacgcttatctttaattaacgcctgatttagcgttgcatcgccctgaatgacgttgacgaaatcgtaaacgacccggcgttcacaacccataatcaggtcgagattacgcaggccgatatcaaaatctatcacgacagttttctttcccttctgggccaaaccagtggcgatggccgcgctggaggttgtcttaccaacaccccctttgcccgaagtaacaacaataatgcgtgccatagaaattccttgttaaaaagggatcaatttaacggttgaacggtcaaagcgttttcgactaactgcagtcgcgccgctttgccataaaattctgctgggatttgatcactcagccagtattcacctgcgatggacaccagttccgccatcaggttcgtacaaaatatttgcgtttcccggtcaccacttgcccctgccagcgcacgaccgcgcatcatgccatagacatgaatgttcccatcggcaatcaattcggccccagcgctaacgtggcttgtaacaatcagatcacattgtggagcataaatacgctgaccggaacgcaccggggtatctattaaacgcgtttttgtgaccggcgttgtattttgcgctggagcctgcggtgtgggagctggacgtggcgctttttcctttccttccgtcaggataggcagccccatcttttcaatttcggctttaagttgcgcatctttgcagccacttacgccaataacccgcaaaccggttgccgaaaccgccttatgcatcgctgaccagtttaccgggtcttccagtgcactgacgttgagtacaacgggggcatgttttaaaaatgcgggggcctgagcgattttgtcttccagcgcctgatggataaccttaggttctgcctcatgcagatgaaccacagataaagtgaagctactgcctttaagctcgattggcgtgtttgacatcctggccttactcaattagctattaatcatcgccagcgcgcgatgatgttccgaagactataaggcatgttatagtctggattatattgaggcaagtcaccctcccatttattcagagtaaaagtctattctgtgataaatggcgctgattcatagcttaaaaaatacccttgtcaatcaacccattgccgtcgtacttttgattgttcttatttacgcttcctttttccgcaccctaatcgtgacagcatctccagacctgtttaaatatccagtattgaggcaagtgtattttttcaccacgccaggctttcttaactttccattttttgcggcatcattaaagaacagatacccgttatcttaatatccgccacagaattgctctatcatagaaaccgcagaagacgtctgatacttctgtcaggtcatcgtaactcgtccaggtcagcggttttgattacggattgatgatgaaatgagcataagtgttgtacggttggattatcaggatgtgctatgaatatgatgcgtattttttatatcggattgtcaggtgtggggatgatgttctcatcaatggcgtctggaaatgacgctggcggacttcaatctccggcgtgcggcgttgtttgcgacccgtatatttgtgtgaactcagatggcatttccccagagttaacaaggaaatatctcggcgaaaaagccgctgaaaacttacaatcattacaaggctacgatcccagcgaatttacattcgctaacggtgtattttgcgatgttaaagaaaaattatgtcgtgatgatcgttattttggtgtggatggtaagcggagtggaaaaatcaatcaaaccaccacaaagatgttatttatgtgtcgtgagtgatgtcttgtttacattatgttctattcgtcattaacctcttgagcgacagagaggagtggggcattaacgtttatgacggggagagtccccgtcggttgacatttacttaatttgaatatcgacgttatattttttagttttgtttttacgggcgtcgtttcgggtttgcaacactcgcagctcatatttgccagaagcagggagtgagtattgtccgtgactatcgagttctggggaatatctggataaatcaactgaatcatcgattcctggcccgaagaggtaagtatcagcgccttcattagagatactcacatgcactttctgaccttttttggcatagaaggtatatgtatcgtaatcgtatccctttatttcgccggagtactgagcgctgctatggccttttctgaactcaacattgacattcttacccgcagcaaagctcgtggaggttagcagtgcaagcagcaatacagccttcctgatgctcttgattttcattggtagtctcctgttcagaatgagtacgatgaactgttataatataacaatccctaacgggagaattccagtggctttcctgcgttcggtaaaatcacgttgcggcatttttgccggggggattacttataaagggggcatggactcaacaaaccgtagaaatctacagctggctggcttgtggcgcgggtttcattgatgttagcttatgccaaaacctggcatcttaaagagtaaaagtatgttttgtgtgatttatcgaagcagcaagcgtgaccagacctatttatatgtcgaaaaaaaagacgatttttcgcgtgttcctgaggaactgatgaaaggttttggtcagcctcagttagcgatgattctgccgctggatgggcggaagaaactggtcaatgccgatattgaaaaggttaaacaggcattaaccgagcaaggttactatttgcagttaccgccaccacccgaagatttgctgaagcaacatctttccgtcatggggcagaaaacagacgacactaacaaataaccgatatccggcggtggcattatctttgtcggcgcgggttttcatatccacgataaggtgaggggaacgttatgtatcaacatcacaactggcaaggtgcgctgctggattatccggtgagtaaagtagtctgtgttggcagtaactatgccaaacatattaaagagatgggcagcgcagtgcccgaagagccagtgctgtttattaaaccagaaacggcactgtgcgatctgcggcagccattggcgatcccatccgatttcggttcagttcatcatgaagtcgaactggcggtgttgattggcgcgacactgcgtcaggctacggaagagcatgtccgcaaagccattgccggttatggcgtggcgctcgatctgacattgcgtgatgttcagggaaaaatgaagaaagccgggcagccgtgggaaaaggctaaagcgtttgataactcttgtccgctttccgggtttattcccgcggcggaatttaccggcgacccgcaaaatacaacgctgagcctgagcgtaaacggcgaacaacgccagcaaggtacgactgcggacatgatccataaaatcgttccgctgatcgcttatatgagcaagttttttaccctcaaggccggtgacgttgtgttgacaggcacgcctgatggcgtcggcccgttgcaaagcggtgatgagctgacagtcactttcgatgggcattctttgacaactcgcgttttgtaatactttttgccgcctgaaagcggcggcaaaacttgcatcgctgtgccagactggttataaggtgcgttttaacgtaatggcggaacacctgatgagcgatgtacctttctggcaaagtaaaaccctggacgaaatgagcgatgcggaatgggagtcgttgtgtgatggttgcggtcagtgttgcctgcataaactgatggatgaagacaccgacgaaatctacttcactaacgtcgcctgtcgccagctcaatattaaaacctgtcaatgtcggaactacgaacgtcgtttcgagtttgaacccgactgcattaaattaacccgtgaaaatctgccaacattcgaatggctgccaatgacctgcgcttatcgtttgctggcggaaggtaaagatttacctgcgtggcatccgctacttactggttcgaaagcggcaatgcatggtgaacgtatctctgtgcgtcatatcgcagtgaaagaatcagaagtgattgactggcaggatcatatcttaaataaacctgactgggcgcagtgataaatttaatagatgctgatgggggctttcttaatatacgtctggatgctcgccatttcgtagccctgtttttgaaagcgctctgtcataatgagagttacccgataccttattatcaacaggtaactctcaatctttaaaaaacgtctgtgtttttaaatgtgataaaccttataccttgagtacatggagagaataatcgcttatcagacttcaggtacctcaaagagtgtctttttaccgtgtcttttctgatactcattacaggtgttaatcatttttttggccgcttcttttagcaaagaaagcattaaatcatcataatcaacgtagaatctggttgtttcagtttccgtttttatctcaccgatggcggctatttcggtggttaatttcaatttggcggcatcgatatctttattcgcttgtttaaccgtgttagacagggtggtaaagaaattctgcacagattttaacttgttcttcaattctggaatcagttttccttcaactacgcccgcagcaatagaataggaaatgattaatccaaatggaccggcgacgacaccggctgcggcaccggcatatgcttccttcctgattttatctacctgtgactggaaatagctgcttttttctgaaaaatcattggttaactggctatctaacgccagcagtttcccggaagcgttgttgaaactttgtgagcttaccagcagggatttttgcgcttcattcagcttcgtgatgccgtcatccagtaccttaatgagaatgtctttctgggcggatgctttcttctcattgtactcatcaaatagcaaaatatacgctgcgagcaattgcgtcgcaacaccacaccattcatacactgtttgggttgcttcaaaatacttatcctggctatccataagtaaggttttaatatcgccgactaaaacggaggctgcctgtgaatactcctgtttaaagcgacttaactcttttatggtttcatcaaaggtctgccaggggatgacctgatcgagatatttattataaagatctaatgctccatctgcggtttcgattgcgtttttaactacttctaccgttttatctgcaacgatttcagtcataatcattcgcctctttaaatatataaattgtaatgaaactcctgttttacaactattaataaattttacttcatctaattcatagttagccgggcgggatgcgtcaatgtctttatttctattaatatgataaatatcaaacaatgtttaatgtcattatggcgaatgcttctattctattttttagccgggtgatatttttcatttctgctggatgagcgtcgtcgccagaaggccacgtgagcacaagataagagaacgaaaaatcagcagcctatgcagcgacaaatattgatagcctgaatcagtattgatctgctggcaagaacagactactgtatataaaaacagtataacttcaggcagattattatgttgtttatcaagcctgcggatctccgcgaaattgtgacttttccgctatttagcgatcttgttcagtgtggctttccttcaccggcagcagattacgttgaacagcgcatcgatctgaatcaactgttgatccagcatcccagcgcgacttacttcgtcaaagcaagtggtgattctatgattgatggtggaattagtgacggtgatttactgattgtcgatagcgctattaccgccagccatggtgatattgtcatcgctgctgttgacggcgagtttacggtgaaaaaattgcaactacgcccgacggtacagcttattcccatgaacagcgcgtactcgcccattaccatcagtagtgaagatacgctggatgtctttggtgtggtgatccacgtcgttaaggcgatgcgctgatgtttgccctctgtgatgtaaacgcgttttatgccagctgtgagacggtgtttcgccctgatttatggggtaaaccggtggttgtgctatcgaataatgacggttgcgttatcgcccgaaacgctgaggcaaaggcgcttggcgttaaaatgggcgatccctggttcaaacaaaaagatctgtttcgtcgctgtggcgtggtttgctttagcagcaattatgagctttacgcagacatgagcaatcgggtgatgtcgacgctggaagagctatcgccccgcgtcgagatttacagtattgatgaggcattctgcgatctgacaggtgtgcgtaattgtcgcgatctgactgattttggcagagaaattcgcgcaacggtgctacaacgtacccatcttactgttggtgtggggatcgcccagaccaaaacgctggctaagcttgccaatcatgcggcaaaaaaatggcagcggcagacgggtggggtggtggatttatcaaatctggaacgccagcgtaaattaatgtctgctctccccgtggatgacgtctgggggattggacggcggatcagcaaaaaactggacgcgatggggatcaaaaccgttctcgatttggcggatacagatatccggtttatccgtaaacattttaatgtcgtgctcgaaagaacggtgcgtgaactgcgcggcgaaccctgtttgcaactggaagagtttgcaccgacgaagcaggaaattatctgttcccgctcgtttggtgaacgcatcacggattatccgtcgatgcggcaggccatttgtagttacgctgcccgggcggcggaaaaacttcgcagcgagcatcaatattgtcggtttatctccacgtttattaagacgtcaccatttgcgctcaatgaaccttattacggcaatagcgcgtcggtaaaactgctgacgcccactcaggacagcagggatatcattaacgctgctacgcgatctctggatgccatctggcaagcgggccatcgttaccaaaaagcgggcgtgatgctgggggatttcttcagtcagggagtcgcgcagctcaatttattcgatgacaacgcaccgcgccccgggagtgagcaattgatgacggtaatggatacactgaatgctaaagagggcagaggaacactctattttgccgggcaggggatccagcaacaatggcagatgaagcgagccatgctttcaccacgttatacaacgcgaagttctgatttactgagggtcaaataaatatagcggcaggaaaaaagcgctcccgcaggagcgccgaatggattagcgaccgaacagatcacgttttttcgctttaaacggctgggaaatcaccaccagcactgcgacaatcaggtaagcgataaaaataccgagcagccactgcggcatttccagacctaaaaaatcccactgacgctcggcgcaatcgccagaggcgacaaacacttgcggcacccacttatccagcggcagccattccgggaaacgaaccataaaatcacaggtggcaaacggcgaaggatagagctgaagcatggtgtgctcgtaagttaactgcacaccgcggaacgcactatacaaccagataaccatcgctacataacgcagcggagttttcggggcgatcgcgccaatcagcgcagcacccagaacgccgaataacgcgcagcgttcataaatacagagcacgcaaggtttcagtaacatcacatgctggaaccacagcgccgtcagttccagtgccagagcagtaaacgccatcaacagccacgcgccccggccttgtgaacattggttcaaaaatcgcaacataatcatttccctgcaatatgcatagagtgcgcagtttaaaccaattcattcgctgcgccaccaggaggcagcaaaaataggacgcaattggacaattatcgggcgaaaaggcaaaccgggcatttatatgcccggtaagttgttatcaaagcgttgctatccagcccatttgcataaaccattcggttacaggggcaagcgtaaactcgacgcagagcaagccgacgagtgtcaggacgagggtgtaaggcagggccatccacaccatgcggccataagagaggcgaatcaatggcgcgagtgcagaggtcagcaggaacaggaacgcagcctgaccgttcggcgtagcgacggagggcagattggtaccggtattaatggcgaccgccagcagctcgtattgcttcaacgtgatagcgccactttccattgccgctttcgcttcgttgatataaatcgtccccacgaagacgttatccgaaatggatgacagcagaccgttgaaaatatagaacagcgacagctgagcatgttccgatgcctgcaacacaaactgaataattggcgaaaacagttgttggtcgataatcaccgcgactaccgagaaaaacaccgtcaacagtgcggtgaatggcagagattcggtgaaggctttaccgatagcatgctcatcggtgacaccggtcaatgatgttgccagaataatgactgacaaaccaatcaagccaacttccgccagatgcaacgccagcgcagtcaccagccagacgccaataatcgcctggacaatcagacggattttatcctgacgggtacgctggtggcggctttgatcgtcaaactgttgcaacacttcgcggactttctccggcagcgtttcaccgtagccaaaccaacgcagcttctctaccagcaggcaggttaacaggccacaaatcagaaccggaacggtcaccggcgacatgcgcaggaagaaatcgccaaaatgccagccagccgctttagcgatgatcaggttctgtggttcgcccaccatggtcattacgccgcctaatgcggtgccgacaccggcatgcatcatcaggctacgcagaaagccacggaactgttccagaaccactttgtaatgcttgtcgatatgactatcgtcttgcaggtcggtgtcttcggtacgggaagaggctacgcggtgataaataccataaaaaccgactgcaacgctgatcaccaccgccacgacggttaaggcatcgaggaacgcggagaggaacgcagccgccacgcaaaaagagagcgacagcagcattttggagcgaatgcttaacagcaaacgggtaaatatgaacagcaacagctgtttcataaaatagatacccgccaccataaacatcagtaacagcaagacttcaagatttgccgccacctcttcacggacgtgttccgcgctggtcatgccgatgaataccgcttcgatagccaacagaccaccggggagcagcgggtagcatttcagggccatcgccagagtgaaaataaattccgctaccagcaaccagcccgcgacgaaagggctgatgaggaaaattaacgggtttacgattaagaaaatgatgagggcgagtttgtaccagtcgggggactggcccaaaaaattgcgccatagcgcgcggccccaggagatctccatgatggtttcccttaccttacaaataatcaatgatgtttttatgtttaaacgcaaagcttaacggtcaggcaggagtgaggcaagtcttgatagtcaaggggaaagagatgcggaaaatgaagccttgatccctttttcttctttttgtctgctatcagcgtagttagccctctggtatgatgagtccaactttgttttgctgtgttatggaaatctcactatggtcattaaggcgcaaagcccggcgggtttcgcggaagagtacattattgaaagtatctggaataaccgcttccctcccgggactattttgcccgcagaacgtgaactttcagaattaattggcgtaacgcgtactacgttacgtgaagtgttacagcgtctggcacgagatggctggttgaccattcaacatggcaagccgacgaaggtgaataatttctgggaaacttccggtttaaatatccttgaaacactggcgcgactggatcacgaaagtgtgccgcagcttattgataatttgctgtcggtgcgtaccaatatttccactatttttattcgcaccgcgtttcgtcagcatcccgataaagcgcaggaagtgctggctaccgctaatgaagtggccgatcacgccgatgcctttgccgagctggattacaacatattccgcggcctggcgtttgcttccggcaacccgatttacggtctgattcttaacgggatgaaagggctgtatacgcgtattggtcgtcactatttcgccaatccggaagcgcgcagtctggcgctgggcttctaccacaaactgtcggcgttgtgcagtgaaggcgcgcacgatcaggtgtacgaaacagtgcgtcgctatgggcatgagagtggcgagatttggcaccggatgcagaaaaatctgccgggtgatttagccattcaggggcgataatcccttccgtttaaagagcaaacccctcaaacgaggggttttttgttgtttttacagatttcccattcttggcgggcaacgttccagcaactcgatgctgccgtcttcgttttgctgttcgagcatcacatcaaatccccacaggcgatgcacatgcttcaggacttctttgcgcccccgatccagcggtgcgcgattatgtggaatataacgcagcgtcagcgaacggtcgccgcgcaaatccacgttccagatctgaatattcggctccagattacttaagttatattgcgacgataaccggttacggatctcccgataaccttcttcattatgaatagcggaaatctccagataattatgccgatcgtcatccagcacggtgaagaagcggaaatcacgcatcactttcggtgacaggaactggctgataaaactctcatctttgaaatcacgcatcgcgaaatgcagcgtttccagccagtcggaaccggcgatatccgggaaccagtatttgtcttcttccgttggcgactgacaaatccgtttaatatcctggaacatggcgaacccgagggcatacgggttgatgccgctgtaccacgggctgttataggggggctggaagaccacattggtgtggctgtgcaaaaactccagcataaaacgttccgttactttcccttcatcatacagatggttaaggatggtgtagtgccagaaggtcgcccagccttcgttcatcacctgagtctgtttttgcggataaaaatactggctcaccttacgcacaatacgcaggatttcacgctgccatgattccagcagtggcgcatttttctccataaaatagagcaggttttcttgtggttcggacggatagcggcgcgcttcagcaaccgttttctcttcctcgcgcttcggcagggtacgccagagcatattgacctgactttgcagatactcttcgcgacttttctgccgggctttctcttcttgcagcgagattttttgcgggcgtttgtaccggtccacgccgtagttcatcagcgcgtggcacgagtccagaagccgttctacttcatcaacgccataacgctcttcgcactcggtaatatatttacgggcaaaaatcagataatcgacaatcgaactggcgtcggtccagctacggaataagtaattgtttttgaagaaagagttatgcccatagcaggcatgagccatcaccagcgcttgcatggtaatggtgttctcttccatcaggtaagcgatacacgggttagagttaatgacgatttcataggccagtccttgctgaccgtgcttatacagccgttcagtctcgataaactttttaccgaatgaccagtgcggatagttaattggcatgccgacgctggagtaggcatccatcatctgttctgaggttatcacttcaatctggtgcgggtaggtatccagccggtagagtttcgccacccggtctatctctgccagataaacatccagcaggtcgaacgtccagtcgggtccatcgctcaaacgtgtggtgtccttattcatagaatcgatcgtcgccatacgcgcacctcattgttgtcggcgctctctgtgtggagcacctcatttcaagcatagaacacctgttaaaaaccgcgtcgccggagaatttttttctttgcgatttcttattatcagagtgccactaatccgcttctgaacggaattttatgctggataaaaagggcgttcagcaggagatactaaagacgccatattgccgcagagtcagggagatgtgagccagctcaccataaaaaagccgcatgttgaataatattttcaactgagttatcaagatgtgattagattattattcttttactgtatctaccgttatcggagtggctatgcgagttgtcatactgggaagtggtgtggtaggcgttgccagcgcctggtacttaaatcaggcaggacatgaggtcaccgtcattgatcgggagccgggggccgccctggaaaccagtgccgcgaatgccgggcaaatctcccccggatatgctgcaccgtgggcggcaccaggtgtgcctttaaaagcgattaaatggatgttccagcgccatgcgccgctggcggttcgtctcgacggtacgcagttccagttgaaatggatgtggcaaatgttacgtaactgcgacaccagccactacatggaaaacaaagggcggatggtgcgtctggcggaatacagccgtgattgcctgaaagcattgcgcgccgaaaccaatattcagtatgaagggcgtcagggtgggacgctgcaactgttccgtaccgaacaacagtatgaaaatgcgacccgcgatatcgccgtgctggaagatgccggcgtaccgtatcagctgctggaatccagccgcctggcggaagtggagcccgcgctggcagaagtggcgcacaaactgacgggcggcctgcagttacccaatgatgaaaccggagactgtcagctatttacccagaatctggcgcggatggcggagcaggcgggggttaaattccgctttaatacgcccgttgaccaactgctttgcgacggcgagcaaatctacggcgtgaagtgtggcgatgaagtgattaaggccgatgcgtatgtgatggcgtttggttcttactcgacggcgatgctcaaaggcattgttgatattccggtgtatccgctgaaaggctactcgctgaccattccaattgcgcaggaagatggtgcgccggtatccaccattcttgatgaaacctacaaaatcgccattacccgtttcgataaccgcattcgtgttggcggaatggcggagattgttggttttaataccgagctgttgcaaccgcgtcgtgaaacgctggagatggtggttcgcgatctctatccacgcggcggtcatgtcgagcaggcgactttctggactggtctgcgcccgatgacgccagacggcacgccggttgtcgggcgtacacgctttaaaaatctgtggctgaataccggtcacggcacgctcggctggacgatggcttgcggttccggtcagttgttaagcgatctgctctctggtcgcacgccagcgatcccatatgaggatctaagcgtagcgcgctacagccgtggatttacgccatcacgtccgggccatttacatggcgcacacagctaaggaaacgagatgacccgtccgatacaggccagcctcgatctgcaggcattaaaacagaatctgtccattgtccgccaggccgcgacgcacgcgcgcgtctggtcggtggtaaaagcgaacgcttacgggcatggtattgagcgtatctggagcgcgatcggggccaccgatggctttgcattgcttaacctggaagaggcaataacgttacgtgagcgcggctggaaaggaccgatcctgatgctggaaggatttttccatgctcaggatctggagatttatgaccagcaccgcctgaccacctgcgtacacagcaactggcagctcaaagcactgcaaaatgcgcggctaaaagcaccgttggatatttatcttaaagtgaacagtgggatgaatcggttgggcttccagcccgatcgcgtgcttaccgtctggcagcagttgcgggcaatggcgaatgttggcgaaatgaccctgatgtcgcattttgccgaagcggaacatcctgatggaatttccggcgcgatggcgcgtattgagcaggcggcggaggggctggagtgtcggcgttcgttgtccaattcggcggcgactctgtggcacccggaagcgcattttgactgggttcggcctggcattattttgtatggcgcttcgccgtccggtcagtggcgtgatatcgccaataccggattacgtccggtgatgacgctaagcagtgagattattggtgtccagacgctaaaagcgggcgagcgtgtgggctacggcggtcgctatactgcgcgcgatgaacagcgaatcggcattgtcgccgcagggtacgccgacggttatccgcgccacgcgcctaccggtacccctgttttagtggacggcgtgcgcaccatgacggtggggaccgtctcgatggatatgctagcggtcgatttaacgccttgcccgcaggcgggtattggtacgccggttgagctgtggggcaaggagatcaaaattgatgatgtcgccgccgctgccggaacggtgggctatgagttgatgtgcgcgctggcgctacgcgtcccggttgtgacggtgtaacttgttgtaagccggatcggaggcaacgtcttctgggtgcaaaaaaatcatccatccggctggtcagcaactgtagttgttaatgtgacagagccattgcccatgatagtgtccattaaaaggatggacactatttccccggaacctgaactcaccgcacaggcgttctacataaaacgcttacgcttcattgttgactcgaactcgacttcagataaatcacgctttacccttgatggagcctgtacatagatttgtgtaattgcctgattttgatatgttcaattcaacatcaaatgaaggttaaattatggacgacaaacaattgcaggctcaggctgcgttcagcaaagcatcgcaaccggcgatagatgcttcattaaatttaagattcagcttcctcttcagccacccgtacgccaatcttcaacacttcattatcttctttctcggccaccgtccagatcatcccggcaaactctacctggtcaccgacaaccggtgccgcgcctaacaactgctggacaatttcacccagcgtttgctgcttatcacgatattctcgcccgtcttccaggccatatatcagcgcaacatcagcatatttggcgctggcttcgagaatgaagtcaccaaagaagcgttgatccagcgcgaccggcggcgactggctgaacagtttaccgagcgccggaagatcgcgttcccgaccaattacacacaacacatcgccttcgcgcagtcgggtgctgccggtaggatgaagcaactggttatcacgaaacagtgccgcaatacgcgtctcttttggcatatgcaaatcgcgcagtgccgcgcccacgcaccatttatcggcactcaattgataaacaaactgctcccacggattttccggatgaatatccaggccaacgcgtgacaccggacgtcccactggcggaaccaccactttggcttttttagccgcccacgagagtgatgttccctgcaagagcagtgaaaccagaaccacaaagaaggcgacattaaagaacagacgtgcattctccagccccgccatcatcgggaacacggccaggatgattggcaccgcgccgcgtaatcctacccagctgataaacacgcgctcacgcagattgaaaccgcggaaggggagcaatccagcaaataccgaaaggggacgggcgaagaatatcatccatgcggacaaaatgagcgccggaatggcaataggcagcagatcgcttgggttaaccaacagccccagcaccaggaacatggcgatttgcgccagccaggcgaggccgtcgaaattttgcaggatgccgtagcggttgcgaatagggcgattacccagcagaaaaccgcacagatacaccgccagaataccgctaccttccagcgcagtagttaatgagaaaatcagaataccgccacttaatgccagcaatggatataatccggcgggcagggcgatgcggttgatcatttgcagtagtaaataaccgccgccaagacctattacaatgcccagaccaaattgttgcagaatatcgacaatgaacatccagctaatattgctctcatgatgctggatcatcgcaattagggtaatcgtcagaaagaccgccattggatcattactgccggattcaatttccagcgtcgagccaacacgttcgttaagccccttaccacccagcagagaaaagaccgctgcagcatcggtagagccgacgatagcgccgattaataagccttcaatcaaatcaagattaaacagccacgccgccatcatgccggttaaaccagaggtgataagcacgcccagcgtcgccagcgacagtgccggtcctaacgccacacgaaaggaactggcctgagtgcgcatcccgccgtcgagcaaaataatcgccagtgccaggttacttaccatgtaggcgaaggggtaattatcaaacgggataccgccgacgccatcgactcctgccagcatgccgatcgccagaaaaataaccagaataggaatgccaagacgggaagaaaatgaactaagtaatatactgctggtgacaaggatggatcctaagatgaaaaggctaattattgttgtggcatccaacggtcggttactcctgattacgctgtctcttatataaaccctaccatattagcggcagagacagcgttttacttagccctgaagcgtgatttttttacattttaagaacaggatgaccgctaatcgtcaactgagtgccttcccgggtgttattcagaatggcatgtgcgcccaacggcagcgtaaccgtgcgttgttcatgaccaaaatcgaggccggtaatgagtggaatcgacaggcgggaacgcaaaaacgcgtacactgactccaggttgtaacctgcgtcataatcattgggcgtgctgccgctaaagctaccgagaataatcgccttctgacgtggcaaaattcccgcatgatagagctgcaacagcatacgttcgacccggaaagggtgctcgttaatatcttccagcaccagaataccgttctcaatttttggcatccacggtgtaccgatcagtgaaatcagcatcgcaagattgcctccccacaacgtgccttcggcccgacatgtcgggccttccccttgccattcaatggtgaaggtttcattgcgtaacgccagccagaaatggtgctcggtaaaggcgttcagttcatccgcgccaaagtttgctaccagcatggggccgctaaaggtgatgacattgccatgcgccagaagaccgcactgaatggcggtaaaatcgctatgtccgcaaatgagcaacgggtcatgttgttggcgagccaccagtgcctgccagtcaatatctgccagtaaacgactggcaccgtaaccgccgcgtacagccagcacgatggtgttgggggtagtcagtctggcaagggaattgagatcttccagacgctctgtttccgtacccgcaaaacgctcacaacgacgggcaataacctcgacgttattgacttgatgccccgcgtcggtaaggcgctggataccacgcagcgcggcgtgctgtttaatgcagtaacccgatggggcaattaagtgaaacagagacatggcaattccttgctgacaacagaaacgaaatgtatatcatgccgcttaggtgtgccgttgtcacctcaacggcgattccaggctataaggatagaagaagtgaaattgagatggtttgcctttttgattgtgttattagcgggttgttcatcaaagcatgactatacgaacccgccgtggaacgcgaaagttccggtgcaacgtgcgatgcagtggatgccaataagccagaaagccggtgcagcctggggcgtcgatccacaattgatcacggcgattatcgctatcgaatcgggtggtaatccgaacgcggtgagtaaatcgaatgccattggtttgatgcagttaaaagcttcaacctccggacgtgatgtttatcgccgtatgggctggagtggtgagccgacgaccagcgagctgaaaaatccagagcgtaatatttcaatgggggcggcttacctgaatattctggaaaccggcccgctggcaggcattgaagatccgaaggtactgcaatatgcgctggtggtgtcatacgctaacggggcaggtgcgctgctacggactttctcgtcagatcggaaaaaggcgatcagcaaaatcaacgatttggatgctgacgagttcctcgaacacgtagcgcgaaatcaccctgcgccgcaggctccgcgctatatctacaaacttgagcaggcactggacgcgatgtaaatcagtcgcgcactttgtccgctttttcccgggcttctcgctcgagagagaaaataatccgctgtaattgccgctccaccgtcgggctgacgttaagaaaacggaagctcagacggggagtggtgatggtttcattcttgccatcaatcactttgcgctcgctgatggagattaactgggcgtcaaagtgaaaaacaccccattgccccatgttgacttcaatctgagcgaagcgcatgccttcttgtaattcggcaggctttgctgtttccagtaatgcgcccatgccgcctaacgacaaatcatacaggcggaaacgtaacgtactgttatccgccagtttggtctggcaaaaataaggcggatggagtggggcggagatgcggaaatatcggcgtcgttgtacaaaccataaggtgggaggcggtacggtaataaatgccggaagctgcaagtattcactctgctgtagttgttcaacagtaaactcgactttcgcaccctgagtttcggcggtaatggtaatgtgctgtgcctttagcacggcgatgttgtcttcggcttgactgccgaaatccagcaccagtttatccggggttattgccagtaatttgctgatcagctgcccgccattccaactgagacgcaaaggaattgcggctttgtgcaaatcgcgtaacacgcccaggacggctaacggattttgtttcaggaactgctcatggtaatgactcacgcggaaaaactcctgactgacaaactgtctttggtttatcggtcacagttaacaaaacttaatacaaatgcgtgaatattttttacatgttgttcttaaatcagccgacatacgcccagcatcgatcccgcccttgcctatacttagagcgttgatgtaagcatttcttgcgtccgattcatcgaaacgagggcctgaacatgggaattattgcctggattatttttgacctgatagccggcattatcgccaagctaatcatgccggggcgtgatggtggtggatttttcctgacctgtattctcgggatagtcggtgcggtggtcggcggctggctggcgaccatgtttggcattggcggctccatcagtggttttaatctgcacagcttcctggtggcggtggtgggagctattctcgttctgggcatattccgcctcctgcgaagagaataagattttcataaggcggatagcgatacagatgccgctatccgctttcacatcagaacgtatactcgacacctgctttacgggtgaaaaaaatcaatatagcacttcgatatccgataaagtcggttcccggtaacaacaacagaatccttttttaattattgtttcgttgtttttggtgtgattcagaaaataaatattttagacagtagccagtcaggcgttaaaaatggggcggatagtgaggcggttttggctgcgcttattgaacatttagaattgatcaatccttctggcagattaagccaaaatacccgttcggcaatgcttcagttacgcgaagaggaatggtctgaattctttttttggttgctaaattctctggagtgtctggattatgtgattattaatttaactccagaaagcaaaaaaacgttgatgagtgaacaccgtaacaatattcaggtagcaattgatgctttatatagccaacgtcggcgtaaatcgccgggtgatgaaagtgaaacacttacccgtagaaatgacgctatcttcggcaaccacgtatggcaaacatttgcgcaatacttcccgccaggacttgaaaaaccgtctgtgtagaaaaaaccatagctatggtgttatctgccgacaacgccatccggagaagccgaatgacgttgtcggagtaagcgctggttaaggtgtgggttgtgcctctttggttgagggttgcgtcgttgctgacttaacggtcggacgcgtcgccggaacattgtcacacggttgctctttcgggcagatcaaatccagcattttcagcgtcacgccattggtccagccaaagccatcctgtaatggatattcgccaccgccgccccccgttccggtggtgctgacatcatatttttccaccagctttttctcccggtcataggtgtgctgaacattggtcaggaagtgccagctaatgtccatcgccacctctttttgcccgtagttttgtaatccttctgtcgcgacccactgtaacggtgcccagccatttggcgcatcccattgttgcccacttttcaccgacgtggtgttcaggccgccgggttgcagcagatgtgttttcgtcgccgtcgccattttgttggcgcgatctttcgctgccgcattgacgtacagcgggaacagggcggccgcggttaactgattgcgcactttatgacttttcaggtcgtaatcggcataccagccttgttgatcgttccacaggtatttttcgatccctttttgacgggcatttgccagcgtttcgtactggtttgccatcgcgttatctccggcagctttgctggcgcgggcgaggattttttccattttaaacatcaggctgttcagatcgaccggtacgatgctggtggtgcgtaaggtatttaactgctgcgggttgtccatccagcgcgagctgaaatcccagccagacgcagcggcagagcgcaggtcgcggtaaatttcagtggcaggtcgattcggattgcttttggcggtggcaatatcttccacccatgactctggtcgtggcgtatcgcgatcgtcccagtagcggttgagaagggtaccatcctgaagtttgacaacgcgtttttcctgttgtccggcttgcaggttttcaacaccgtccatccagtaagcatattctttttgcatttgcggcaggtattgcttcaacgcggcatcgccttcatgctgcgccagtaactctaccatcagggcaaagaagggcggttgcgagcggcttaaatagtaactgcggttgccgttgggaatatgaccgtaagtgtctatttcatgagcaaaattggccaccatatccgcgactttatcccagtgaccgctttcggcaagtcctaacatggtgaagtaactgtcccagtaatatacctcgcgaaagcgtccgcccggcacgacataaggttccggcagcggtaacagagaatcccatttttcggtgttttcggtagaacgcgttaataccggccaaagtccgtcaatatgttcgcgcagtgactgcccctctggcggaacatatttctcgccttctttcggcagggtgaaattgacgttaacgaaatggcgcagatcaaatccgctctggttttgctgcatccgataatcagcaaggatcatcagcggatcgctgttcggcacggcatcggcaaaggttttttggtccggaaaaagtttggcgttttgcacatcattaaacagcggccctaataaaatatcaggcggctgtggtgttaccggtgtttcttctgcctgcaccgatagcgcagcgaaacacaaaaagatacaggctggaattaacgccattttttgcgggcgagaaggtgcgggggatttcatcaatcattctcctttggcgaaaccgaataaaacggtattcaagtatcagaaaaccttagttcaggatcgcactagctgcatgatcgaaatctcattctgcgaactgtcaggcattttagaaaagggaattaaagggataaataacggcgaaatagagtgatcaaataacgtctgtttattagccagccagcggcgttgggttcgtgattagcgaagaaaaatcatcataaattggtgaaaaatataacaggtagttaaaaaccattagtgctgagtaaattgccggatgacatcagaacgatgccatccgaacagtggcttaaccctgacggttgaaacgttgcgttttaacgtccagcgttagcgtttcttctggttgtatcgcatacagtttctcaccctgctggcaaatccagccaatccccagttcacgggcgattagggcgctgtgggataccggacttccggcgctaaggcagataccttttacaaccgccggatccagttgcagtactgtggaaggataaatgttctccgccagtagaatagttggcgagttaaactgcgggagttcttctttcgtttgggtcaggtggaccagggtgcgatgcagaagatcgtccacatcaatatagcgagcttgtagatattcatcatccagttgctggtattgctggctaagttctttaagaacttgctgccaggcatattctgccgtgcaatgttcatgctgaaggagttcgcttgccgccgccagcagttccggatcatctaacagtgtatggtgaccagaaaagattgcggcaatatcgtcaagcccgctggcttctgctttcgctgttaacgtcatcagatctaataacgtgaagtcaatagcctggcgtaatcgatcttgttcttcttccacggtcagggttgattttgcctgtaccgtacataaaactggttgataataaaaggctttacccgaaacaggcggaacgggacgcagagtaggtggagcgacttcctccgtttcaccaaagttatcttcagccagctgacggaaagcgatcagtgcctcttcagcttctggccctttcgcaatcaggcgcagcgtatcgttatagcgaacttgtagtaacgcaatctggttaatactctctggtgtgacgcatttgccgtttttttccagcaacatatcggcattaaatgtcgataaggtataaaccagccgggaggccggacgtacatgcaggccgttacggttttttatgaccaccgccagagaacgggcttcttcatcgtacgcaggacatgtgtcagagatttcagtgtcggaggacggtaaacccagttgttcacgtttggcttccagcgcatgcatggcgtcaaagataactttgtcgatatccgcccccgaggccgcgctgaccgttgctgccagtgtaccttcgaccaacggcgcagcacacaaacgtacttttgcggcgatctcgggagccagcaattccagcgcagtttcagcactcaataatgcgctacccatatccatcatgaccagcacatggtcggcatcagcaacagattcgatggcctccatcactttgacggcatcggtaccaatgggattttgtggatcgtcaattcccgcggcaatggcgattttacaactatcactcattaacatctgacgggctaattcaccgacaccttctcccagtcggctgctatgtgaaactatgaccaggtttaccatcaccaattccttactcttttgcggctaacgccaacatttgcatcataaacatcaccgaggtcgcgccgggatcctggtgaccaatactgcgttcaccgagataactggcgcggcctttgcgggcttgcatcgtaatcgtactttgtgcagcggattcggcgatgctactggcagcttcgagcgccaccggaacagagagattttgctcgctggactgacgtaacgattccaccaccggcacccacacatcacacatggttttatcgccaggttcggctttcccgcgactgattacgccgtccgcgccatcgcggaacatctgataaagctcttccagtgtcaggctttgccgtgcctgggtcgcctgtgcggcgcggataaagaaggtaccgaacagcggaccactggcaccaccgacgctggaaagcagcgtcataccggtattcttgagaatgaaaccgatatctttatctgcgatagcagggagtttttccaccactttgctaaagcctcggttcatatttagcccgtggtcagcatcgccaatttcgcgatccagtccggtaagatactcgctctcggtgctgaaaatatcgccacaacgagtgagccagttaacaatttgagttctgctcagtgacattgctttctccttatttaccccagttaagggccggggtgtggaccggggcgtcccagagtgccagcgtttcgtcatcaactttcagtaaggtgattgagaaaccggtcatatccagtgaggtgcagtacgcgccaattaaattacgttcgatagtcaatcccgcttgctggcaacgtgtggtcaggcggttatagacgccgtacagctcagaaagcggagttgcgccaagattgttaaccagcgcaatcacccgatcgccagactggagcggttgtttggtttgttgttcttcctgccaactgccttgttgataatcccagaaacgcaaagtgcgatggtatgagccatttaccagcagggtgtcgaacatttcatcgacggtttgatcaagggaagagaaggggcggcggtcaatacccggctcaccatgaatgccgacgccaaactccatctcattatccgccagggtaaaagaaggtttgcccgcggcaggaacggtacaggcaccgagagcgatacctattgagtggccttgattattcagcttacgccccagttccgcacaggcgtccagtgagtcgccacgctccgccgctgcgcctacgagtttttcaattaatacggtgttggcaacgccgcgtcgcccggcagtataaagactgtcttttaccgcaacgtcgtcatcaatgaccacagtggtcacttttacgccgctatcgtgcagtaactcggtcgctgtttcaaagttaagaatatcgccggtgtaatttttgataatcaacagtacaccttcgccgccatcaacttgcatggcgcattcaaagattttatcgggcgtcggtgaggtgaaaatttcgcccggacaggcccccgaaagcatcccctgaccgatataaccacagtgcatcggctcgtgtccgctgccgccacccgacagcagggcgacttttcctgcaacaggggcatcagctcgggtgacatacaccggatcctgatgcagtgtcagcgatggatgcgctttcgccagtcctgccagttgttcgtccagtacgtcttgcacatcattgatcaattttttcattattttgctccagcaattacggtagggcatggatgatgttcaacgacacggcgaccactgactgccgatgaatccattgtgcatcaggcaagggaaaagaaaattagcccaaattatgtttcatagtgaaacatatgctttaatgaatgttccatattgaaacttttacgtgtattaatacttaaaattgcgagccggaacaccttttgtcataagggatgcgggatatgagtggcgcttttaacaacgatggtcggggcatatctcccttaattgcaacctcctgggagcgatgcaataagctgatgaaacgggagacatggaacgtaccacatcaggcccagggcgtgacatttgcttctatttatcggcgtaagaaagcgatgctgacgctcgggcaggctgcgctggaagatgcctgggaatatatggcaccgcgagagtgtgcgctgtttatcctcgatgaaaccgcctgcattctcagccgtaatggcgatccgcaaaccttgcagcagctaagtgcactgggattcaatgacggcacgtattgcgccgagggaattattggtacttgtgcgctatcgttagcggctatctctggtcaggccgtgaaaacgatggccgatcaacatttcaaacaggtactctggaactgggccttttgtgcaacgccgttgtttgacagcaagggccgattgacgggaacaatagcgctggcgtgtccggttgagcaaactaccgcagctgatttgccgttgacgttggcaatcgcccgcgaggtcggaaatttactgctgacggacagtttgctcgctgaaactaaccgtcatttaaatcaacttaatgccctgttagaaagtatggatgatggcgtgattagctgggacgagcagggtaatttgcaatttattaatgcccaggcggcgcgggtcttgcgccttgacgcgacggcaagtcagggacgggcaatcactgaactcttaacgttacccgccgtattgcaacaagcaataaaacaggcacatccgctcaaacacgtagaagcaacctttgaaagccagcaccagtttattgatgcggtgataacccttaaaccgataatagaaacgcagggaaccagctttattttgttgctccatcctgtggaacagatgcggcagttgatgaccagtcaattaggaaaagtcagccataccttcgctcatatgccacaggacgatccgcaaacccgccgcttgattcattttggtcgccaggcggcgcgcagtagctttcctgtcctgctttgtggagaagagggcgtgggcaaggcactgctaagtcaggcaattcataatgaaagcgagcgtgctgcaggtccttatatcgccgtcaattgtgagttatatggtgatgctgcgctggcggaagaatttattggtggcgatcgcacggacaatgaaaatggccgtctgagtcggctggaactggcacacggcggcacgctgtttcttgaaaagattgaatatctggcggtggagttacagtctgctttgcttcaggttatcaagcagggggttatcacgcgactggatgcgcggcgtttaataccaattgatgtcaaagtgattgcaacaacgaccgcggacctcgcaatgctggtggaacaaaatcgttttagtcgccagctgtattacgcgctgcatgcatttgaaattaccatcccgcctctgcgtatgcggcgtggcagcattccggcgctggtgaataacaaattacgcagtcttgaaaaacgcttctctacgcggctgaaaattgatgacgatgccctcgctcgcctggtttcttgtgcatggccaggcaacgattttgaactttacagcgtcatcgagaatcttgctctgagtagtgataacgggcgcattcgcgtcagtgatttgccggaacatctgtttaccgagcaggcgacagatgatgtcagcgccacccgcctttccaccagtctgtcatttgcggaagttgaaaaagaggcaattattaacgcagcccaggtcacaggcggtcgcattcaggaaatgtcggctttacttgggatcggccgcactacgctgtggcggaaaatgaagcaacatggcattgatgcagggcagtttaagcgccgggtatgaaagacagaaacgatttctgatacatcagagtgatctgtatttcattccggcgcacgctaacaattttcagcatcgtttaagggcttgtctatcccgcacttaaaagctgaagcgatatcctccgttgacttgcttctgatcaaagaggttaccctgcgtgtaatccgcttcgagatagaatgtgtgctgtttgttatactgtgcactgactcccacgccgttattccagccattacctttgaaactgtacttctcccgggagttgttcaacagatattcggtatcccctgaaaactcgcggatagcgccagtcttcacatagacattcagctggctgttgcctgcggtgatgtcataccccagtatcatgctggcacgccccagcagcgattcgtagtgattcagatgtatattgaggccattactcgccttcatagtcatctcattctggtggctgtatgtaagctgggtttgcggctctatatagaacccataaccagtaggggacaggttgaacctctgcccggcttccagggagatgctcattccattcgcagtgccgttggcgttaacgccgttgttctgactgtccagtacgtggaaactatttttctggcgcgatgcttttataacgagatcgctgtaaaaaccgttttgtgccatgtaactggcgtacattcccatgtagtctgaacgtgcggtaccgtcgcctccgctatagtccggcgatgcatgtgttgagccaatatacagaccgacatacaacggcattacatcagagagacgtttatccccaccaaactggataccgctgtaacccatgtcaaagccgctcagtttgccactggcaaaggagtccaggcttcccccataactgcgcaaccagatattaccgtctttactctgatttcgcaggtcacccatccgttgcatcagcgtacggttttcaacatagttcaataagtaaccgacattgagataattgccgccagcatctgcggtcgtggtgggtttaggcgtgggagcgggttcaggcgtaggatcggggttgactatgggaggctgagcgggagctggtgtgggttcaggattaggagtcggttccggaactgtcccggaagcgtaaagctcccagttagtgccatttttacgcacatcgtacagatatccccccaactcaacctgagaagacgcgctgaacgaggccgcgccgtcagtggtttttaccactgtcagaacttcatttcccgttgtggcctcgctgccctggttgcggatagccaatacgtgattaccagcactactcccgctgatattcaataaatcccctttattattaacgccattaccctcgccaacaacatcagcacgcataataaaggtactgttaccgctcaggttctctacgtttaatgtggcaaatgtgccggcagttgacccgtggctggcaaaatcgacagttgaatggctcagcgccagcgtgtcgagattagaattacttgttacgttccagacgctgttattcattgcaacgtccagttttccgccattgacattatcgctgagggaggaacctgtccaaaccgacccagggtgcatatccagattgattagcccacctttggaaagaacgctaccgttgataagcatacgacccgaggcgttgatgcggctggcggcataaccatcgtcatgttgcgttgcgatggccatctggtcgggtgtactcatatcaatgaccagatcgctcgtgaggtcgatctggctgttggtcatggcataaattcccctggctcctgccgcgccggtgatagccaaactgtctccggttattctaccgccgctgagagcccacaaacccagcgccagactgccattacgatcaactgtaatatcggtattttgcatgttgacaacagccgttgccgtctgggccgaggcaccataagaaccgccggaaaagatgctgtttcgttgcgctgccgtgccagtaaaattgattatcgcgtctgaaccactggtgacgaggccaccgccctgcgcggaagaaatatggctatctgcaccgatagtggttgtaccaccacgaacttcgacgccattggccgcggctccagttacatcaacagtgagtgcattcgcgctaacctggccaaagctccagaggccgtgagcattatcgccattggttttaatggtactgtttgttccgagatcgacaacagagtttttctgtacgtttatccccatggcgctgtagccctgaacatcgattgtcaggtctgtagccgtaaaacgcgcagcaccattggcgttattgccgttgagaccaccgatataaacacctgtacttccatcggtcgtgattttacttccgcttccaagatcgacactggtgccatagtcattgatggttaggcctataccgttcgagttttcaatggtgaattgagtggctgttagtgttgagctatgcccaataatgatgccgtcatcgttactcttaatggtgctgcctgtgcctaagtcagcatgggtatagtcaccaattaagttaatgccgatggcagaggtttgaccaacaacatctactgtgagtcggttagctgtcagggagctgtttttgccctgaataatgattccttttgcatatccagaggcgtcgttgacattgacggtgacatcattacccaggttgatattgccaggcgtgtttcctgctggggtcattacaccatagaggtttcctgatggatcggcggtatctcctgtaattctgtcaccatcattaatagtaatattggtgccatattgacttcctgtatcagcagctatcagcaggggggaaaagataattgcattcaaaccaatagcgccaaattttatcagttgaattgagggcgaacggatttttaattcagcgagacgatctgctttggtattcccattgtgttgtttgatgcccataccactcctatatagtacccagactatgggtctatggattttgtcattttgtttaaatcaatgaataatatcctcttatcatcatgatatttgtatggtgcaatcatgatgagcttctcagagaataattctctattaccgggcaaaatcaggaacacaggaattaatatatatttaacatcccccttacaaaggtgagtttatatcgagttattccctaagttgtcgttacttattccaattcgttactataaatatggcaaaaatattacaacaaacagcggttaaaaaatttggtgaagattttttgtaataatcctaattagttatgggaatttcgcttgatgtatctgcataacaaaaacaatatgcgccatttttgcattactaataagaaaaagcaaaaaacatcgatattcatttttggtcaatgggttttctggcctatcgttgttattgtgctactggttatcattttcatcttgccagcatattggagcgtgatcaattttgatcagctgtgaagggggctgatgtgtagtgatacaaaaacttacgttatatcactgctaatgagatatccggcatctgaacacttatgtctttaattattctcgtggttcactataggcaataagcacaaaagtgtaggatgttacaagaatgattaggactcggtgaaatgaaaaatccacgcaattgcgtggattttatatacttttgcgctcttcatgagatttagcgaaacctcatgagacaataaattaattagacgttgaaaaggaagttcatcacatcgccatctttcacgatgtaatctttaccttctgcacgcattttgcctgcttctttcgcgccttgttcacctttgtaagtgatgaaatcttcaaacgagatggtttgtgcacggataaagcctttttcaaaatcagtatggattttgcccgctgcctgcggcgcggttgctccaaccggaatggtccatgcacgcacttctttcaccccagcggtgaagtaagtttgcaggttcagcagtttataaccggcacggatcacacggttcaggcccggctcttccagcccaagctcctgcataaactcgtcacgttcttcgtcgtccagttcggcaatgtctgcttcaacagcagcacaaaccggaaccacaacagaaccttctttcgccgcgatttcacgcacctggtcaagatatgggttgttttcaaaaccgtcttcgttgacgttggcgatgtacattgttggtttcagcgtcaggaagctcaggtaacgaatagccgctttctcttcagcgcttaaatccagcgcgcgcagcatacctgcattttccaactggggcaggcatttttccaggaccgccagctcagctttcgcgtctttatcgccacctttggctttcttctgtacgcgatgaatcgcacgttcgcaggtgtcgaggtctgccagcgccagttcggtgttgataacttcaatatcgtcagccgggttaactttgccggaaacgtgaatgatgttgtcattttcaaagcagcgaacaacgtgaccgatcgcttcggtttcacggatgttggtcaggaactggttacccagaccttcgcctttcgatgcgccttttaccagaccggcgatatcgacaaattccatggtcgtgggaagcgtacgctgcggttttacgatttcagccagttgatccaggcgaggatcaggcattggtacgacgcctgtgttcggctcaatggtgcagaatggaaagttggccgcttcaataccggctttggtcagcgcgttgaacagggtagatttcccgacgttgggcaaaccgacgataccgcatttgaatcccatgatttaaatcaccttaatatcttaataatcaacctgttattgctaacagattgcagaaatggaaataactttgcctattatacacggcactcggcaaaaatgccgcagacaacgacttattgcgctttaaaggcgtgcaatcggttcgttgctttggtcaagccatctgtaaaccacatttcagtacaacgcgccgcttcgtcaatggcttcatcaattaacttctgttcactaacaggcggtttgcctaacacaaaaccgacaactttatttttatcgcccggatgaccgattccgatgcgtaaacggtgaaagttagggttattacccaatttactgatgatgtctttcagtccattgtgaccaccatggccaccgcccaatttaaatttggcgacgccaggaggcagatccagttcgtcgtgggccaccagaatttcgtccggattaatgcggaaaaaactggccatcgccgcaacggctttgccgctgagattcataaatgtagtcgggactaacaggcggacatcttcgcctccaagagtgactcgcgaagtataaccaaagaatttagcctcttcgcgcagcggagcgcgcaaacgctctgccagtaagtcaacgaaccaggcaccagcattatgtcgcgttgcggcgtattcagcaccggggttcgccaggccgacaatcaatttaatcgtcacgtttttttgtcctgagtgtgtacataactggcgcgtagtttactggttgcggccccgcttgacaaaaaactgcgtatcaaatgcagataacgtaataattgcctgagtggactattagaaagtcaaggtgttcaggcgtttatttgtaaagttttgttgaaataagggttgtaattgtgatcacgcccgcacataacccactgggtgttgtctatactttacacataaggaagaggggtattccctgttacaacccagaaagttccggaggtgacatatgaaacgcaaaaacgcttcgttactcggtaacgtgctcatggggttgggtctggtggtaatggtggtcggcgtggggtattcaatcctcaaccagttaccacagtttaatatgccccagtatttcgcacatggtgcagtgctaagtattttcgtcggtgccattctctggctggcgggtgcccgtgttggcgggcatgaacaggtgtgcgaccgttactggtgggttcgccactatgacaaacgttgccgccgtagcgataatcgccgtcatagctaacaaataatgcagtttgctgaccagtcagtttgcgctgactggtcaatctcgtacttataaatccgccatcgccgcgcgacgattcgggaagaacgccaggcgtcccgggatcggttgaatgccagcgcgagccatagtgcgcagtggctggaattccacgttgcacacgcgcagttcacatccctcgggcagacgcttcacaaaacgctggaacgcatcaagaccaccagcatcaagtaccggaacggcatcccacttcagaatcacaatccgtttgccttcaagacgtgactccaggtccgtgaataagccttcagcagcagcaaaaaacagcgggccaataacgcgcagaaccaggacatcgtctggaacatctacgactaccggtgccaggcgagtcatacgtgcgatacgacgcataaacagcagcgatgccagcacgatccccacgctgatggcaataaccatatcaaacaacacggtcagcgacatgcacagcagcatgacgatgatgtcatctttcggcgcatgacgcagcaagtcgaccactttgtgcgcttcactcatgttccacgccaccatcaacagcagggctgccatggcggaaagcggcagccaggagagcagcggtgccagtaccagcagggcaagaataaccagaatagagtggatcaccgccgagataggggacgttgccccggcacggacgttagcggcagaacgcgcgatggcagctgtagcggtaataccaccaaagaacggagcgataatattccccagtccctgtccaaccagttcgctgttcgccttgtgtttcgtcccggtcataccatccagcaccacggcgcagagcagagattcgattgcgccgagcattgccattgagaatgccgcaggcagcagtgtgcgaatagaatcccaggttagcgtgaattctgaattaggcagatcccacggcagcaccagttgcggcagcagttgcggaataccgttaccctgagaaccatcggccaggacgtagtggaattgcgaaccgatggtagcaacatgtccgccgagcaggttaacaatccccatcaccgcgcaaccagccagcaaggccggaaggtgaccgggtaaacgaatgcccagacgcggccaaaaaacaagaatacctagcgtcacaatgccaatggcagcatcacccacattaatggtcggcagcgccataaataatgcgccgactttttgtagataatgttccgggacatgggccatttgcagaccgagaaaatctttaatctgcatggtaccgatggtgatcccgatacccgaggtgaaacctaaggtgacggaaaccggaatatactcaatcaggcgaccaaagcgtgccagacccatcagaatcaaaaagatccccgacagcaaggtcgcaaccagcagtcctgccagtccaaactgttgcgacacgggatagagaattaccacaaatgccgcagtcggaccggaaacgctaaagcgtgacccacccgtcagagcaatgacaatccccgcaacagctgcggtatataaaccgtactggggtgccacaccactaccaatagccaacgccatcgccagcgggatagcaataatcccgacggttatcccggcaatcaggtcacgggtaaaccgtgcggcagtatatttttctttccagcaagcgtcgatcagagcgcggaaaggcatcacatgtgaggaaaatattttgttcacaataatgtttcatccgtgagcgcatcatctgtcaactaaatggcaggtgaaggaggcataggtcatacaaatggatattacagacaaaaaaacccgccgcagcgggtctttgagccgggttcgattagtgttcgaacatggcagagatcgattcttcgttgctgatacgacgaatcgcttcggccagcatacctgacagggtcagagtacgcacgttcggcagtgatttgatttcatcgctcagcggaatggtatcgcagacaacgacttcatcaattacagagttacgcaggttgttcgccgcgttgccagagaagatcgggtgagtcgcgtacgcaaatacacgtttagcaccacgttctttcagagcttcagcagctttacacagcgtaccgccagtgtcgatcatatcatcgaccagtacgcagtcacgacctgcaacgtcaccgatgatatgcatcacctgtgaaacgttcgcacgcggacgacgtttgtcgatgattgccatatcggtatcgttcagcagcttagcgatagcgcgggcacgcacaacgccgccgatgtccggagaaaccacaattgggttatccagattcagctgcagcatgtcttccagcaggatcgggctaccaaatacgttatcaaccggaacgtcgaagaaaccctgaatctgttcagcgtgcagatccactgtcagcacacggtcaacaccgacgctggagaggaagtctgcaaccactttcgcagtgattggtacacgagcggaacggacgcgacggtcctggcgcgcatagccaaagtaggggataacagcggtgatacgacctgcggaagcacgacgcagggcatcaaccataacgactaattccatcaggttgtcgttagtaggggcacaagtggactggatgatgaaaatatcaccaccgcgtacattttcattaatttgtacgctgacttcgccatcgctaaagcgacctacagcggcgtcgccgagtgaagtgtacaggcggttggcaatacgttgtgctagttccggggtggcgttaccagcaaaaagcttcatatcaggcacgagaagaacctcaggcatgcgtccattggtggaaagaatctgccgaaaactgtgcgggccaggcatgatcctttccaggcggtgtattaaagagcgcgatgcaacgtctggaacaaggtgacgttgtcaccgaaactcagcttgcccggcttaaagcatggctctgtgcaatggggaaagattagcgcctttcgccacaaagccattgagccattccggggcttgctctagcacctggcgggcttcagactctgtatcaaattcagcaaagacacaggcccctgtcccagtcaggcgcgacggggcgtattctaacagccaggaaagcaccgcatcaacctcgcgaaaacgttttcttgcgataacctcgcaatcattgctgaattcacattttagcaacgtttctattgacctttttggcgtattgcgcgggagttcaggatctttaaaaatcaccggagtcggaatacttacaccagggtgcgccaccagataccacttctctggcggatccaccggcgttagtatttcaccaacgccttcggcaaacgcggcatgcccccgaacaaagacaggaacatctgcgcccagcgtcagccccatttccgccagctcatccatgcttagcccgcattgccagagatgatttaatgccaccaggaccgtcgcggcattggatgaaccaccgccgagaccgccgcccatcggcaaacgcttgtcaatgctgatattcgcaccgcttcccgtcggaagacgcccgctgtctgccgcagttttcatcaacaatcgcgctgcgcgaacgatcaggttatcttcatgttccacgccttcaacgggcgttaacagacgaatatccccatcgtcacgaagctcaatgctgatggtgtcgccgtaatcaagaaactgaaacagcgtttgcagcgtgtggtaaccatccgcacgctgaccggtaatgtataaaaacagattaagttttgccggagagggccactgtgtccgcattatttcactatccagttatccatttttaacttgatgcgttgaccaccgtcggtgagttccatattggctggcatcgcaggttgcgttttggtgtcataaccaccataaacaaccttccagtttttgccattctggctgtaggtaatttcgctcaggcggtactggtcgtccagtttgtagtcggttgcatcacccggtaaacctaaaatccactggcgcaagctgttgagcggaattggcattccggtcaatttgccaatcatctcttcggcgtcatcggcggtataacgctgacctttattgtcgactaactgcacgttacccggttgagcattcagctccagttccgtgctgcccaatgggttagtgagcagcagacggtagcgatcctggccggtttgctgccagaaaaagcgggcgtacactttttgttggtcagaaatataagcgaacgcgccgcgagtctgatactgattaagattgcgcacgtcttgctgatgctgacgccattgtggcgaatccgggcttttgccaggacctttgggcgtggtaacggaacaggcagtgagcacaagagcagccagcggtagcaggcggataagacgaaaatcgggcaggggcatagtgatgacaagtccttgagatacgttgcagttataacccttaatgctagcgttaccgtccgctatcgtctatgttcaagttgtcttaattgccagaatctaacggctttcggcaattactccaaaagggggcgctctcttttattgatcttacgcatcctgtatgatgcaagcagactaaccctatcaacgttggtattatttcccgcagacatgacccttttagcactcggtatcaaccataaaacggcacctgtatcgctgcgagaacgtgtatcgttttcgccggataagctcgatcaggcgcttgacagcctgcttgcgcagccgatggtgcagggcggcgtggtgctgtcgacgtgcaaccgcacggaactttatcttagcgttgaagagcaggacaacctgcaagaggcgttaatccgctggctttgcgattatcacaatcttaatgaagaagatctgcgtaaaagcctctactggcatcaggataacgacgcggttagccatttaatgcgtgttgccagcggcctggattcactggttctgggggagccgcagatcctcggtcaggttaaaaaagcgtttgccgattcgcaaaaaggtcatatgaaggccagcgaactggaacgcatgttccagaaatctttctctgtcgcgaaacgcgttcgcactgaaacagatatcggtgccagcgctgtgtctgtcgcttttgcggcttgtacgctggcgcggcagatctttgaatcgctctctacggtcacagtgttgctggtaggcgcgggcgaaactatcgagctggtggcgcgtcatctgcgcgaacacaaagtacagaagatgattatcgccaaccgcactcgcgaacgtgcccaaattctggcagatgaagtcggcgcggaagtgattgccctgagtgatatcgacgaacgtctgcgcgaagccgatatcatcatcagttccaccgccagcccgttaccgattatcgggaaaggcatggtggagcgcgcattaaaaagccgtcgcaaccaaccaatgctgttggtggatattgccgttccgcgcgatgttgagccggaagttggcaaactggcgaatgcttatctttatagcgttgatgatctgcaaagcatcatttcgcacaacctggcgcagcgtaaagccgcagcggttgaggcggaaactattgtcgctcaggaaaccagcgaatttatggcgtggctgcgagcacaaagcgccagcgaaaccattcgcgagtatcgcagccaggcagagcaagttcgcgatgagttaaccgccaaagcgttagcggcccttgagcagggcggcgacgcgcaagccattatgcaggatctggcatggaaactgactaaccgcttgatccatgcgccaacgaaatcacttcaacaggccgcccgtgacggggataacgaacgcctgaatattctgcgcgacagcctcgggctggagtagcagtacatcattttctttttttacagggtgcatttacgcctatgaagccttctatcgttgccaaactggaagccctgcatgaacgccatgaagaagttcaggcgttgctgggtgacgcgcaaactatcgccgaccaggaacgttttcgcgcattatcacgcgaatatgcgcagttaagtgatgtttcgcgctgttttaccgactggcaacaggttcaggaagatatcgaaaccgcacagatgatgctcgatgatcctgaaatgcgtgagatggcgcaggatgaactgcgcgaagctaaagaaaaaagcgagcaactggaacagcaattacaggttctgttactgccaaaagatcctgatgacgaacgtaacgccttcctcgaagtccgagccggaaccggcggcgacgaagcggcgctgttcgcgggcgatctgttccgtatgtacagccgttatgccgaagcccgccgctggcgggtagaaatcatgagcgccagcgagggtgaacatggtggttataaagagatcatcgccaaaattagcggtgatggtgtgtatggtcgtctgaaatttgaatccggcggtcatcgcgtgcaacgtgttcctgctacggaatcgcagggtcgtattcatacttctgcttgtaccgttgcggtaatgccagaactgcctgacgcagaactgccggacatcaacccagcagatttacgcattgatactttccgctcgtcaggggcgggtggtcagcacgttaacaccaccgattcggcaattcgtattactcacttgccgaccgggattgttgttgaatgtcaggacgaacgttcacaacataaaaacaaagctaaagcactttctgttctcggtgctcgcatccacgctgctgaaatggcaaaacgccaacaggccgaagcgtctacccgtcgtaacctgctggggagtggcgatcgcagcgaccgtaaccgtacttacaacttcccgcaggggcgcgttaccgatcaccgcatcaacctgacgctctaccgcctggatgaagtgatggaaggtaagctggatatgctgattgaaccgattatccaggaacatcaggccgaccaactggcggcgttgtccgagcaggaataatggaatatcaacactggttacgtgaagcaataagccaacttcaggcgagcgaaagcccgcggcgtgatgctgaaatcctgctggagcatgttaccggcagagggcgtacttttattctcgcctttggtgaaacgcagctgactgacgaacaatgtcagcaacttgatgcgctactgacacgtcgtcgcgatggtgaacccattgctcatttaaccggggtgcgagaattctggtcgttgccgttatttgtttcgccagcgaccttaattccgcgcccggatacggagtgtctggtggagcaggcactggcgcggttgcctgaacaaccttgccgtattctcgatctcgggacgggtaccggggcgattgcgcttgcgctggctagcgagcgcccggactgcgaaattatcgctgtagatcgtatgcctgatgctgtctccctggcacaacgtaatgcccagcatctggcgatcaaaaatatccacattctgcaaagcgactggtttagcgcgctagccgggcagcagtttgcgatgattgtcagcaatccgccgtatattgacgagcaggaccctcatcttcaacaaggcgatgtccgctttgagccgctcactgcgctggttgcggcagacagtggaatggcagacatcgtgcatatcatcgaacagtcgcgtaacgcgctggtatccggcggctttctgcttctggaacatggctggcagcagggcgaagcggtgcgacaagcatttatcctcgcggggtatcatgacgtcgaaacctgccgtgactatggtgataacgagcgcgtaacgctcggccgctattatcaatgacaagtttttctacactgcttagtgttcatcttattagtatcgcgctttctgttgggctattaaccttacgtttctggctacgttatcagaagcatccacaggcatttgctcgctggacgcgcattgtgccgccggttgtcgatacgctgttactgttaagcggcattgcgttgatggctaaagcgcacatcctgccattttccgggcaggcacagtggctgactgaaaagctgtttggagttatcatttatatcgttttgggttttattgcactcgattatcgtcgtatgcacagtcagcaggcgcgcattattgccttcccgctggcgttggtggtgctgtacatcatcattaaactcgccaccacaaaagtaccgttactggggtaagtcatgagatcgttagctgatttcgaatttaataaagcgccattgtgcgaaggcatgatcctggcttgcgaagcaatccgccgcgattttccctcgcaagatgtttacgacgaactggagcgtctcgttagtctggcgaaggaagaaatcagccagcttctgcctttagaagagcagttggaaaaactgatcgcgctgttttacggcgactggggatttaaagcctcacgcggtgtttatcgtctttccgatgcattatggctggaccaggtgttaaagaatcgacagggcagtgcggtatcattaggtgcggttttattatgggtcgcgaatcgtctcgatttgccgctgctgccggtgattttccctacgcagctgatattgcgcattgaatgtccggatggcgaaatttggctgattaatccttttaacggtgaatcgttaagcgaacatatgctggacgtatggttaaagggaaatatcagcccgtcggcggaactgttttatgaagaccttgatgaagctgataacattgaggtaatccgcaaattgctggatacactcaaagcctcgttgatggaagaaaatcagatggagctggcgttacgcaccagcgaagctttattacaattcaaccctgaagatccctatgaaattcgcgatcgcgggttgatttatgcgcaactggattgcgaacacgttgcgttgaacgatttaagttatttcgttgaacagtgtccggaagacccgatcagcgaaatgatccgtgcgcaaataaataacatcgcgcataaacatattgtgctgcattaattaatcgacattttactcaagattaaggcgatcctatgaaacaaaaagtggttagcattggcgacatcaacgtagcaaatgacctgccgttcgtactgtttggcggtatgaacgtgttggaatctcgcgatctggcgatgcgcatttgcgagcactacgtaactgtgacccagaaactgggtatcccttacgtgttcaaagcctcttttgacaaagccaaccgctcctccatccactcttatcgtggaccgggcctggaagaagggatgaaaatcttccaggagttgaagcagacttttggcgtgaaaattatcaccgacgttcacgaaccaagtcaggcacagcccgttgctgatgtcgtggatgtgattcagttgccggcgtttcttgctcgccagactgacctggttgaagccatggcgaaaaccggtgcggtaattaacgtcaagaaaccacagtttgtcagcccgggacagatgggtaatatcgttgataaattcaaagaaggcggcaacgaaaaagtgattctttgcgatcgcggtgctaacttcggctatgacaacctggttgtcgatatgctgggcttcagcattatgaagaaagtgtctggtaactcgccggtgattttcgacgtgacccacgcactgcaatgccgcgatccgtttggcgcagcttccggtggtcgtcgtgctcaggtggctgagctggcacgagccggtatggcggtaggtctggcggggctgtttattgaagcgcatccggatccggaacatgcgaaatgtgatggtccatccgcgctgccgctggctaaactggaaccgttcctcaagcagatgaaagcgattgatgatctggtgaaaggtttcgaagaactggataccagcaagtaatcttttttgcttgaaaaataaagtattagcgttctgcgttaagacttttttcatgggtgccggatacaaaaaaggccgcaggctgttacccctgcggccggtttcgggcgcatattgccatcacggcagcctgacgcccgttttcaccttacttccggttacgccaccagctgacaatcgctgcggtaataattcccgccaggatcggtgctgccaggtcgtgccagaaaatcatggcaaactgcgcgagcgtcatatagccgccttgttgtaatgacaacattttgcggctattcttgaattgttctggttcaagattagcccccgttctgttgtcaggttgtacctctcaacgtgcgggggttttctctttccagcaaccaatgccaccagggataaagcccccgcaacattgcgcctcaccggataacgccggcttggtgtggatactacgactcaattcatcttcacttcatccctgaaatgtttgcaatgaagagtgcattccggtttttcaacagctgttacagtcatttcatgagtgctctggatgaggcttccagctcgggttgccaatatttacttgtggaagtgataaagacaaaaatggccgcaggctgttacccctgcggccggtttcgggcgcatattgccatcacggcagcctgacgcccgttttcaccttacttccggttacgccaccagccgacaatcgctgcggtaataattcccgccaggatcggtgccgccaggtcgtgccagaaagtcatggcaaactgcgcgagcgtcatatagccgccttgttgtaatgacaacattttgcggctattcttgaagtgtctggtttcaagattagcccccgttctgttgtcaggttttacctctcaacgtgcgggggttttctctttccagcaaccaatgccaccagggataaagcccccgcaacattgcgcctcaccggataattccggcttggtgtggatactacgtctcaattcatcttcacttcatccctgaaatgtttgcaataaagagtacattccggcttttcaacagctgttgcagtcgtttcatgagtgctctggatgatgcttccagctcgggttgccaatatttacttgtggaagagataaagacaaaaatggccgcaggctgttacccctgcggccggtttcgggcgcatattgccatcacggcagcctgacgcccgttttcaccttacttccggttacgccaccagctgacaatcgctgcggtaataattcccgccaggatcggtgctgccaggtcgtgccagaaaatcatggcaaactgcgcgagcgtcatatagccgccttgttgtaatgacaacattttgcggctattcttgaagtgtctggtttcaagattagcccccgttttgttgtcaggttttacctctcaacgtgcgggggttttctctttccagcaaccaatgccaccagggataaagccccgcaacattgcgcctcaccggataacgccggcttggtgtggatactacgtcgcaattcatcttcacttcatccctgaaatgtttgcaatgaagagtacattccggcttttcaacagctgttgcagtggtttcgtgcagggtgtggtacaggctcgcaattctgattaacgacctgtccaggtagtatgaagaaatacaataagcaggaatttatattatctcccccgattaccgtcatcggaggagatataactgtcaggcaaatatcgtcatcaaataggcggcaaacagtgccagatgcgctgcgccattgagcacgttagtacgtccggtggagaaggagatatggcacagcactaaagaggccaccatcaccaccatttctggcgcaccaagtgcaaactgcaattcgttacccgtcataaaggcaattagcgtgacgacaggtacggtaagcgaaatggttgctaacactgaaccaaagaacagattcatcgcgcgctgaacctggttgttcaacactgcttttaatgcacctaaaccttccggcgacagaatcaacagtgccaccaggaagccagtaaaggcgacaggggcattcatgctgtcgagcaatgtctccagcgagctggcgttcattttggtcaccgcaataacggcaatcagatggataatcaaccagatagcatgccacaggctgctatgggcagacggtttaccgtgatgcgggtcgtcatcatcactgtcatcttcgtgctcgtagacaaacaaactttgatgcgttttggtctggatcagcaaaaatacgccatacattgccgcagaaattaatgctaccagtaacgcctgaccggttgaaaaattcgccgcaggcagagccattggaaataccagtacgattatcgccagggggaacagcgcaattaaatactgcttgataccaaacagattcatatattgggtggcaaacttacgaccgcccaacaataatgaaaagccaaccagcccaccggtaacaatcataatgattgaatagagcgtatcacgcattagcgttggcgcggcgtcgccggttgccattaaagctgaaatcaaactgacttcaagaataaccactgaaaggctaagaataagcgaaccgtaaggttctcccaggcgatgggctaatacgtccgcatgacggacaacactaaaggcgctacttaaaataccaataagcgcaagaagattgatggcaatgaccactggtagtgtctggctgcttccccacaggaacagcactaccagcgccagaaccgggaaaataagcgaagtctccttgtggcgggtttttaccgcctcttgagcatttgacattatggttatccctttgcagatgaatttatcgaaaatgtaaaaaataggtaggaaaaataacagaaagtgtctggatatcggtaacattttacgaatttttaccccgctgtcgattttttactcattggggcataaaaataagtattacgtttagacaatgtttgttttagcgtctcttaagaagagtctgacctgaaaattcttatgttttggcaagagtagatattgttgaccacacttaatgttcaactttgtaaaaggagtcaacgatgccgtataaaacgaaaagcgatctgccggaaagcgtaaagcacgttctaccgtctcatgcccaggatatctataaagaagcgttcaacagcgcatgggatcaatataaagataaagaagatcggcgtgatgacgccagtcgcgaagaaaccgcgcataaagtggcctgggctgctgtgaagcatgaatatgccaaaggggatgatgataaatggcataaaaaatcgtaaaaccggtcgcttagttaaagctattcgtgcggtgttgccttgcaagtggtccgtggattgcatattgtcccgttagtggtttcaaaatgagcagtaaaaatgtccggaagacaccaaaaagttgtcgcagggaagtatgcagtggcggaagtgtaaggtgataacgcgtgatttcttgatgaatgccgattgtaaaacggcatttggtgccattgaagaatcactcttatggtcagcagaacaacgggcggcttcgctggcggcgacgctggcttgtcgacctgatgagggaccggtgtggatcttcggctatggatcgttgatgtggaatccggcactggagtttaccgaatcgtgcaccggtacactggttggatggcatcgcgcattttgcctgcgcctgaccgccgggcgcgggactgcgcaccagccgggacggatgcttgcactgaaagagggcggacgcaccacaggcgtcgcctatcgactgccagaagagacgctggagcaggaactaaccctgttgtggaagcgagagatgattaccggctgttatctgccaacctggtgtcagcttgatcttgatgatggacgcacagtaaacgccattgtgtttattatggacccgcgacatccagaatatgaatctgatactcgcgctcaggtcatcgcgccgttgattgcggcggcgagcggtccgctgggaaccaacgcacaatacctgttttcactggaacaggagcttatcaaactgggaatgcaggacgatgggctgaatgatttgctggtatcggtaaaaaaactgctggcggagaattttccggatggtgtgttacgtccgggattcgcctgagtaaacttcccgcatagtggggcgtcagacgccccctcaaacattaaaatgtgagcactttatcggctgacagcgtccattgcgccagttccacaagagtaccgatttccaccccatcaatcagaggaagtgtactaatcccgcgcccgtcggtacaggttttgcacaatttcaccggtacattctgagcggtaaggatctccagcatttgctgaatgttgtagccttcccctggtttttgcccgcgcaacccggctgtgaccgcatcagacatgaggaacagacgcagatccagattgctctcctgctctcgtaacgcaatggccagccgcaagctgttaaacaaggattcgctcccgtaaggtgcgccattggcaacgatcacgattttttgcattatttactcctgtattcagggaattagacactcatcttctatcttactgcttctgcagcgtctgaccaatcggtcacatttttaaggattttcctgaaagcgcgagaaaatacgacaaaagttgccagtaatcgttattctttaaggctatggtttttcattattaccggaagttaccgacgttttgagccgtttcgttcctcgcattatcccgttttatttactcttgcttgtagcaggcggtacagctaacgcacaatctaccttcgagcaaaaagcggcaaatccctttgataataacaatgatggtctgccggatttaggcatggctcccgaaaatcatgatggggaaaaacactttgctgaaattgtgaaagatttcggcgaaaccagtatgaatgataacgggctggatactggcgagcaggcaaaagctttcgcattgggaaaagtccgcgacgcgcttagtcaacaggttaatcagcacgtagagtcctggctatcaccgtggggaaatgccagtgttgacgtcaaagtggataacgaaggacatttcaccggcagtcgtggaagctggtttgtgccgttacaagataatgatcgttatctcacctggagccagcttggtcttactcagcaggataatgggttggtgagcaatgtgggcgttgggcaacgctgggcgcgcggcaactggctggtgggttataacactttttatgacaacttgctggacgaaaatcttcagcgagcgggctttggtgccgaagcgtggggcgaatatttgcgattatcggcaaacttttatcagccgtttgctgcatggcatgaacagacagccacgcaggaacaacggatggcgcgcgggtacgacctgacagctcggatgcgcatgccgttctatcaacacctcaataccagtgtcagcctagaacagtattttggtgatcgtgttgatttgtttaactctggtacgggttatcacaatcccgtcgcgttgagtctgggattaaattacacccctgtgccattagtcactgtgacggcccagcataaacagggtgaaagtggcgaaaatcaaaataacctcgggctgaatcttaattaccgctttggtgtaccgctcaaaaaacaactttctgcgggcgaggttgccgaaagtcagtcgttacgtggtagtcgctatgacaatccgcagcgaaataatctaccgactcttgagtaccgacagcgaaaaacgttaacggtgtttctggcgacaccgccgtgggatctaaaacctggcgaaacagtgccgctgaaattacaaatccgcagtcgttacggtattcggcaactgatttggcagggcgatacgcagatattaagtttgacgccgggcgcacaagccaacagcgcggagggctggacgctgatcatgcctgactggcagaacggggaaggggcaagcaatcactggcgattgtctgtggtggtggaagataaccaggggcagcgtgtctcctccaatgagatcacgctaacgcttgtcgaaccgttcgatgcattgtcaaacgacgaactgcgctgggaaccgtaatcagaaaatgcgctcctgatgcacccataccgctgcttccacgcgagacttgagcttcattttcttcagcatgtgcttgacgtgcacttttactgtgctttcggtgatatccaggcggcgggcaatcatcttgttcggcaaaccctgggcaatcagcttgagaatatcgcgctcgcgtggggttaactggttaacatcgcgctcagtagtggcacggttagcgcgcaagctggcggccagaacaggcgttaatgcttcgcttaataccatttcgccagcagctgcctgatgcaatgctttcagcagatcttccggttccatatcttttaacagatagccatccgcgccgcgtttcagtgcggtgaccacatcttcttcatggttagagacgctgaataccacaatgcgccctgagagggacttttcgcgcagtttatccagcgtttccagaccgttcatgccgggcatattgagatctaacaggatcagatcgggatcaagagactccgccagttcaataccctgttcgccattactcgcttcgccaaccacggtgatatctggtgccatactgataagctgttttacgccagttcgcagcatcgggtgatcgtcaatcagcaggatagtagccggttcctgattactcatgggtatctccttggacgtctgtgaaagttttttcgggaataaaggtgaccaccacttcggtgccacctgattcacgacggcggacgcggcaatcgcctcgtaaactttgcgcacgatcgcgcattattatcatgccgtagtgattgctgcggatggcattttcaggcacgccgcagccgttatcctggacggtcagtttgacctgattatcgttttgcgccaccgtcaccacgacttcactcgcttgcgaatgtttgagggcgttacttaatgcctcacgggcaatttgcaacaagtggattgcctgatgcgaaggcaccaggcgaggcggcaattgataatccagcttcaccgggaagccaaatttggcgctgtactcttcgcaactcgcctccagcgccggacgtaatccaggctcggtgagctgcaagcggaatgtggtgagcaattcacgcaactgcgcccaggatgcattcagttcgttacggatctgacttaacagttcgcggctgctttctggcagcgcatcgccctgcatctgtaaacaactcacctgcatcttcatgcaagagagagattgggcaatagaatcatgcagttcgcgcgcaatggtggcacgctcttccatcacgatcaactgttgctgacgttcctgatggcgatccagcgccagcgtggcggtgagttgttcaaccagggtatccaccagttgttgttgatcatggctaagatgacgcccctgcggcagggtcgccagcaaaataccgtactgcgtatgagagtcagccagccgccacttcagggtcgtgccgcgatcaccaacgggtaatacgccgcgcgggcagagctggcagcctttatcatcacaagtcatatctggctggcaggtaaactcctgatgattctcttcatcatcagtgtcatacacccgcaattcgatatcacgtagcagggttaaattctgtaagccgttgagtacaggtgacaggcgttcacacagcggggcgcgggaatgcaaacggcggttagcctgccataaaaaagagaggatctgatttttatgctccagcccggcggttttctcctgaacccgctgctcaagtacggcataactttcggccagttctgcagacatattgttcaacgcagttccaagcatcgccatttcgttgcgcccgctgatgtttgcgcgttgggtaaaatcgcgatgactgacggcactcgccattgccagcagttgccgccacggttgtagcagtcgcgcccgcaaccagataatagtgaacaccagtaaaagtgccataaataccgccattacccgatggaccagtaccactgtctcgatgcgcatttccgtggtgcggtcaaaaccagataccagttgatcaagcccggcaacaaactggctgacatccgctgacaccgtttctcggttttgtgcacgcatcagcgcagggatcagttcattacgccagtaatcttgtaaaccctgtaattgcgccagttgtccgtctcgttctgctgctcgagtcaactcggcgctaaatgccgtttgttccatctctttaattaagggcttgtctttctcgcttaatggcactgccgccaacagacggtaactttgcatgcgcagcgatcccgctttgttgatcgcatgggcgctgccctgaacgccttgcaccagccagccagaaaccgccatccctgccagtccaatagcagtagaaagcaacacaataagcgcaacctgattaaccagggtgagcggagagagacaacgtttaagcatgtaaacctcttccttcaggctttaaatgagcaataaccttaatgaatgtgacgatacattctggaatggcagtattctcggctattggctgaagtatacccatacccggaaagagttactccttatttgccgtgtggttagtcgctttacatcggtaagggtagggattttacagcaccgtgaaaaatctcataatttttatgaagtcactgtactcactatgggtaatgataaatatcaatgatagataaagttatcttatcgtttgatttacatcaaattgcctttagctacagacactaaggtggcagacatcgaaacgagtatcagaggtgtctatgagtcactcatccgcccccgaaagggctactggagctgtcattacagattggcgaccggaagatcctgcgttctggcaacaacgcggtcaacgtattgccagccgcaacctgtggatttccgttccctgtctgctgctggcgttttgcgtatggatgttgttcagcgctgttgcggtgaacctaccgaaagtcggctttaattttacgaccgatcagctatttatgttgactgcgctgccttcggtttctggcgcgttattacgtgttccatactcctttatggttcctatcttcggtggtcgtcgctggacggcgttcagcaccggtattctgattattccttgcgtctggctgggttttgccgtgcaggatacctccacgccttatagcgtcttcatcatcatctctctgctatgcggctttgctggcgcgaacttcgcatccagtatggcaaacatcagcttcttctttccgaaacagaagcagggtggcgcgctgggtctgaatggtggtctgggaaacatgggcgtcagcgtcatgcagttggttgctccgctggtggtatcactgtcgattttcgcagtatttggtagccagggcgtcaaacagccggatgggactgagctgtatctggcgaatgcgtcctggatatgggtgccgttccttgccatcttcaccattgcggcgtggtttggcatgaacgatcttgctacctcgaaagcctccatcaaggagcagttgccggtactcaaacggggtcatctgtggattatgagcctgctgtatctggcaaccttcggctccttcatcggcttctccgcgggctttgcaatgctgtcaaaaacgcagttcccggatgttcagattctgcaatacgctttcttcgggccgtttattggtgcgctggcgcgttctgcaggtggtgcattatctgaccgtctgggcggaactcgtgtcacgctggtgaactttattctgatggcgattttcagcggcctgctgttcctgaccttaccgactgacgggcagggcggaagcttcatggcgttcttcgcggtcttcctggcgctgttcctgacagctgggctgggtagtggttccactttccagatgatttcagtgatcttccgtaaactgacaatggatcgcgtgaaagcagaagggggttctgacgaacgtgcgatgcgtgaagcggcaaccgacacggcggcggcgctgggtttcatctctgcgattggcgcgattggtggcttctttatcccgaaagcgtttggtagctcgctggcattaacgggttcgccagtcggcgcaatgaaggtatttttgattttctatatcgcctgcgtagtgattacctgggcggtatatggtcggcattctaaaaaataaaccgttactcgtcatacttcgggttacatgtgctgcggctgcgttcattcaccccagtcacttactttagtaagctcctgggattcattcacttgccgccttcctgtaaaccgaattatatagagtaaaatatttgattatcctttgcgcggcatgatgtcgcgctttttttatgcgtcatttagttacaacatactaatgttatatggtttatttcgccggatttcattaagagccattaatatgttacccatggggaatactccttaatacccatctgcataaaaatcttaatagtttaaataactacaggtataaaacgtcttaatttacagtctgttatgtggtggctgttaattatcctaaaggggtatcttaggaatttactttatttttcatccccatcactcttgatcgttatcaattcccacgctgtttcagagcgttaccttgcccttaaacattagcaatgtcgatttatcagagggccgacaggctcccacaggagaaaaccgatgagtaaattcctggaccggtttcgctacttcaaacagaagggtgaaacctttgccgatgggcatggccagcttctcaataccaaccgtgactgggaggatggatatcgccagcgttggcagcatgacaaaatcgtccgctctacccacggggtaaactgcaccggctcctgcagctggaaaatctacgtcaaaaacggtctggtcacctgggaaacccagcagactgactatccgcgtacccgtccggatctgccaaaccatgaacctcgcggctgcccgcgcggtgccagctactcctggtatctttacagtgccaaccgcctgaaatacccgatgatgcgcaaacgcctgatgaaaatgtggcgtgaagcgaaggcgctgcatagcgatccggttgaggcatgggcttctatcattgaagacgccgataaagcgaaaagctttaagcaggcgcgtggacgcggtggatttgttcgttcttcctggcaggaggtgaacgaactgatcgccgcatctaacgtttacaccatcaaaaactacggcccggaccgtgttgctggtttctcgccaattccggcaatgtcgatggtttcttacgcatcgggtgcacgctatctctcgctgattggcggtacttgcttaagcttctacgactggtactgcgacttgcctcctgcgtctccgcaaacctggggcgagcaaactgacgtaccggaatctgctgactggtacaactccagctacatcatcgcctgggggtcaaacgtgccgcagacgcgtaccccggatgctcacttctttactgaagtgcgttacaaagggaccaaaactgttgccgtcacaccagactacgctgaaatcgccaaactgtgcgatctgtggctggcaccgaaacagggcaccgatgcggcaatggcgctggcgatgggccacgtaatgctgcgtgaattccacctcgacaacccaagccagtatttcaccgactatgtgcgtcgctacaccgacatgccgatgctggtgatgctggaagaacgcgacggttactacgctgcaggtcgtatgctgcgcgctgctgatctggttgatgcgctgggccaggaaaacaatccggaatggaaaactgtcgcctttaataccaatggcgaaatggttgcgccgaacggttctattggcttccgctggggcgagaagggcaaatggaatcttgagcagcgcgacggcaaaactggcgaagaaaccgagctgcaactgagcctgctgggtagccaggatgagatcgctgaggtaggcttcccgtactttggtggcgacggcacggaacacttcaacaaagtggaactggaaaacgtgctgctgcacaaactgccggtgaaacgcctgcaactggctgatggcagcaccgccctggtgaccaccgtttatgatctgacgctggcaaactacggtctggaacgtggcctgaacgacgttaactgtgcaaccagctatgacgatgtgaaagcttataccccggcctgggccgagcagattaccggcgtttctcgcagccagattattcgcatcgcccgtgaatttgccgataacgctgataaaacgcacggtcgttcgatgattatcgtcggtgcggggctgaaccactggtatcacctcgatatgaactatcgtggtctgatcaacatgctgattttctgcggctgtgtcggtcagagcgggggcggctgggcgcactatgtaggtcaggaaaaactgcgtccgcaaaccggctggcagccgctggcgtttgcccttgactggcagcgtccggcgcgtcacatgaacagcacttcttatttctataaccactccagccagtggcgttatgaaaccgtcacggcggaagagttgctgtcaccgatggcggacaaatcccgctataccggacacttgatcgactttaacgtccgtgcggaacgcatgggctggctgccgtctgcaccgcagttaggcactaacccgctgactatcgctggcgaagcggaaaaagccgggatgaatccggtggactatacggtgaaatccctgaaagagggttccatccgttttgcggcagaacaaccagaaaacggtaaaaaccacccgcgcaacctgttcatctggcgttctaacctgctcggttcttccggtaaaggtcatgagtttatgctcaagtacctgctggggacggagcacggtatccagggtaaagatctggggcaacagggcggcgtgaagccggaagaagtggactggcaggacaatggtctggaaggcaagctggatctggtggttacgctggacttccgtctgtcgagcacctgtctctattccgacatcattttgccgacggcgacctggtacgaaaaagacgacatgaatacttcggatatgcatccgtttattcacccgctgtctgcggcggtcgatccggcctgggaagcgaaaagcgactgggaaatctacaaagccatcgcgaagaaattctccgaagtgtgcgtcggccatctgggtaaagaaaccgacatcgtcacgctgcctatccagcatgactctgccgctgaactggcgcagccgctggatgtgaaagactggaaaaaaggcgagtgcgacctgatcccaggtaaaaccgcgccacacattatggtcgtagagcgcgattatccggcgacttacgaacgctttacctctatcggcccgctgatggagaaaatcggtaatggcggtaaagggattgcctggaacacccagagcgagatggatctgctgcgtaagctcaactacaccaaagcggaaggtccggcgaaaggccagccgatgctgaacaccgcaattgatgcggcagagatgatcctgacactggcaccggaaaccaacggtcaggtagccgtgaaagcctgggctgccctgagcgaatttaccggtcgtgaccatacgcatctggcgctgaataaagaagacgagaagatccgcttccgcgatattcaggcacagccgcgcaaaattatctccagcccgacctggtctggtctggaagatgaacacgtttcttacaacgccggttacaccaacgttcacgagctgatcccatggcgtacgctctctggtcgtcagcaactgtatcaggatcaccagtggatgcgtgatttcggtgaaagcctgctggtttatcgtccgccgatcgacacccgttcggtgaaagaagtgataggccagaaatccaacggcaaccaggaaaaagcgctcaacttcctgacgccgcaccagaagtggggtatccactccacctacagcgacaacctgctgatgctgactttaggtcgcggtggtccggtggtctggttgagtgaagccgatgccaaagatctgggtatcgccgataacgactggattgaagtcttcaacagcaacggtgctctgactgcccgtgcggttgtcagccagcgtgttccggcagggatgaccatgatgtaccacgcgcaggaacgtatcgttaacctgcctggttcggaaattacccaacagcgtggtggtatccataactcggtcacccgtatcacgccgaaaccgacgcatatgatcggcggctatgcccatctggcatacggctttaactactatggcaccgtaggttctaaccgcgatgagtttgttgtagtgcgtaagatgaagaacattgactggttagatggcgaaggcaatgaccaggtacaggagagcgtaaaatgaaaattcgttcacaagtcggcatggtgctgaatctcgataagtgcatcggctgccacacctgttcagttacctgtaaaaacgtctggaccagccgtgaaggcgtggaatatgcgtggttcaacaacgtggaaaccaagccgggccagggcttcccgactgactgggaaaaccaggaaaaatacaaaggcggctggatccgtaaaatcaacggcaaactgcagccgcgcatgggtaaccgtgccatgctgctgggtaaaatcttcgctaacccgcatctgccggggatcgacgattattacgagccgttcgattttgactatcagaacctgcataccgcgccggaaggcagcaaatcgcagccgattgcccgtccgcgttcgctgattaccggggaacggatggcgaaaatcgaaaaagggccgaactgggaagatgacctgggcggtgagtttgacaaactggcgaaagacaagaacttcgacaacatccagaaggcgatgtatagccagttcgaaaacaccttcatgatgtatttgccgcgcctgtgcgaacactgcctgaacccggcatgtgtggcgacctgcccgagcggtgcgatttacaagcgtgaagaagatggcatcgtcctgatcgaccaggataaatgccgtggctggcgtatgtgcatcactggatgcccgtacaaaaaaatctacttcaactggaagagcggtaagtctgagaagtgcatcttctgctatccgcgtattgaagcgggtcagccgaccgtgtgctcagaaacctgtgtcggtcgtatccgttatcttggcgtgctgttgtacgatgccgacgctattgaacgtgcagccagcaccgagaacgagaaagatctttaccagcgtcagctggacgtgttcctcgatccgaacgatccgaaagtcatcgagcaggcgattaaagacggtattccgctgagcgttattgaagccgcacagcagtcgccggtttataaaatggcaatggaatggaaactggcgctgccgctgcatccggaatatcgcacactgccgatggtctggtacgtgccgcctctgtctccgattcagtctgcagcagacgcgggtgagctgggtagcaacggcattctgccagacgtcgaaagcctgcgtattccggtacagtatctggcgaatctgctgaccgccggtgataccaaaccggtactgcgcgcactgaaacgtatgctggcgatgcgtcattacaaacgtgctgaaaccgttgacggtaaagttgatacccgtgcgctggaagaggtcggtctgaccgaagcccaggcacaggagatgtaccgttatctggcgattgctaactacgaagatcgctttgtggtgccgagtagtcatcgtgaactggcacgggaagccttcccggagaaaaatggctgcggctttacctttggtgatggctgccacggttcagataccaaattcaatctgttcaacagccgtcgtatcgatgccatcgatgtgaccagcaaaacggagccgcatccatgatcgaactcgtgattgtatcgcgtctccttgaatatccggatgctgccttatggcagcatcaacaagagatgtttgaggcgattgccgcgtcgaaaaatctgccaaaagaggatgcccatgcgctgggcattttcctgcgcgatttaacgacgatggatccgctcgatgcccaggcgcagtacagcgaactgttcgaccgtggccgcgccacgtcactgttgctgtttgaacatgtgcacggcgaatcccgcgaccgcggccaggcgatggtggacctgctggcgcagtacgagcagcacggcttgcagttaaacagccgcgaattgccggaccatctgccgctgtatctggagtacctggcgcagctgccgcaaagcgaagccgtggaaggtttgaaagatatcgcgccgattctggcattgctgagcgcgcgtctgcaacagcgtgaaagccgttatgccgtgctgtttgatctgctgctgaaactggcgaataccgctatcgacagcgacaaagtggcggaaaaaattgccgacgaagcgcgcgatgatacgccgcaggcgctggatgctgtctgggaagaagagcaggttaaattctttgctgacaaaggctgcggtgattcagcaatcactgcgcatcagcgtcgctttgccggtgccgtcgcgccgcaatatctgaatatcaccaccggaggacagcactaatgcaattcctgaatatgttcttctttgatatctacccgtacatagccggggcggtcttcctgattggtagctggctgcgttatgactacgggcagtacacctggcgcgcggcgtccagccagatgctggatcgcaaagggatgaacctggcgtcgaacctgttccatatcgggattctggggatttttgtcggtcacttcttcggtatgctgacgccgcactggatgtatgaagcctggctgccgattgaagtgaaacagaaaatggcaatgtttgctggtggtgccagcggcgtgctgtgtctgattggcggcgtgctgttgctgaaacgtcgtctgttcagcccacgcgtgcgtgcaaccactaccggagcggatatcctgatcctgtcgctgctcgttatccagtgcgcgctgggcctgttgaccattccgttctccgctcagcatatggacggtagcgagatgatgaaactggttggctgggcgcagtcggtggtgaccttccacggtggcgcttctcaacacctcgatggtgtggcgtttatcttccgtctgcacctggtgctggggatgacgttattcctgctgttcccgttctcgcgtctgatacacatctggagcgtaccggtggagtatctgacacgtaagtaccagctggtgcgcgctcgtcactaagcgaattttagttcacatagaccctgcttcggcggggtttttttatgggcacggtgcggggtgagttgtcggatgcgcttcgcttatccgacctacaggggaggatattgtaggcccggtaaacgtggtgccatcgggcaaaattagctcggagtaacaggttttgattatttaaggaagcgatggtggtgggggaaggattactcagcgctgcgcgcttcgcccttcgggtcgttgcctgcggcaacgctctctcgctggcgctcaagtcgaaccttggtcgaagcttctcatccttccccgcttgggcagaatatttgattgcggattcgtttgagaattccggggcttttgaaagtgatggtggtgggggaaggattactcagcgctgcgcgcttcgcccttcgggtcgttgcctgcggcaacgctctctcgctgacgctcgagccgaaccttagtcgaagcttctcatccttccccgcatgggcagaatatttgattgcggattcgcttgagagttcagggacttttgaaagtgatggtggtgggggaaggattactcagcgctgcgcgcttcgcccttcgggtcgttgcctgcggcaacgctctctcgctggcgctcgagtcgaaccttggtcgaagcttctcatccttccccgcatgggcagaatatttaattgcggattcgttgggaagttcagggacttttgaaagtgatggtggtgggggaaggattcgaaccttcgaagtcgatgacggcagatttacagtctgctccctttggccgctcgggaaccccaccaggggtaattcaaattttgaggtaatgcttgagatggtggtgggggaaggattattcgtcgcttcgctcctcacccttcgggccgttgcctgtggcaacgttctctcgctttcgctcgaatcgaaccttagtcgaaggttctcacccttccccgatgagtgcaaactttcacaatctcaccgaagttaccacatcgctgtggtgaattatggtggtgggggaaggattcgaaccttcgaagtcgatgacggcagatttacagtctgctccctttggccgctcgggaaccccaccacggggtaatgctttttactggcctgctcccttatcgggaagcggggcgcatcatatcaaatgacgcgccgctgtaaagtgttacgttgagaaaaatgaactggttgcgtaattttcatccgtaacggattaaaggtaaccagttatttttgctggcgattaaagaataatcgttcgattaccgtaaacaaagacgcgctgtgccagtactttgtatagtgcacgacttaagacgtttttctcgacgtcacgacctgcgcgcatcatatcttcagctgtgtaggtatgatcgacatgaataacgtcctgcatgatgattgggccttcgtccagattgtcattcacatagtgagcggttgcgccaataatcttcacaccacgttcataggcctggtgataaggacgtgcgccaataaacgctggcaggaatgaatggtgaatattgatgatcttattcgggaagcgtgccacaaattccggcgttaatacccgcatatacttcgccagcaccacgtagtcaggttgataagcatcaatggcatccgccatcttttgatcgtgctcgttgcgggttaacccttcatggcttaccagctcaaacggaatatcaaaacgctcaaccagagaacgtaaagtatcgtggttaccaataactgccgcgatttcgacatccaggccgccgtaattggctttcatcaacaaatcgccaaggcaatgcgcttctttagtgaccagaatcactatccggcgacgaccggcaggattcagctcacgcacggagccttctggcaatgcgctatcgagatccgccagcagggtggaatcattaaaaatcccttccagttccgtgcgcataaaaaagcgcccggtacggtgatcaacaaattcattgttctgtacgatatttaactcgtgcttgtagcaaatattggtaatacgtgcgatcagacctttttggtccggacaaatagtacgcagaactttacgttggagtgaatgcattgctggaaaaaccttgttgagagtgtttgctaaaccgtaccgtcaaccattattggccgcagcactttttaaattttttacctgaaccacaagggcagggatcgttgcgaccaaactgcggacgtgtaccgtcaatatagtaccattgaccgttttctttcaaaaatcgcgaacgttcaattattgcacctgttttaccaccttcggtaaatcgagcaacaaaactgacaaatccgatattgtcggcgtcctgccaacaatgttcaaatacggtcaatcccaaccattcagtatgcgcaaatccggccatcaattcggcacgtaacgccgctgctccacaagagggatgccaggtctttattaaataatctgcgtcttgcatcacaaaagcgcagtaacgcgaacgcatgagatgttctggatcaggtgcaaccttttcaccagacacataagggtggcaacataggctatactcgacagcactaccacagggacaaagctgagacacaaataatctccctggaaacaataacggcgtattaaccgcctgagtagcactatgttaaccgagcagtagcgatgtggctacgattgcattccaggggaatcttgcgggaataatgagaaagataaaaatagggctggcgctgggatctggcgcggcgagaggttggtcgcatattggcgttattaatgcgctaaaaaaagtgggtattgaaattgatatcgttgcaggatgttcaattggttcgctggtgggcgctgcctatgcatgcgatcgattatctgcgctggaagattgggtgacctctttcagttattgggatgttttacgcctgatggatctctcctggcagcgcggtgggttactgcgcggcgagcgtgtcttcaatcaataccgcgaaataatgccggaaacagagatcgaaaattgttcccgtcgctttgcggctgttgccaccaatttaagtacgggacgtgaattatggtttactgaaggcgatctccatcttgctattcgcgcatcatgcagtattccaggactcatggcacctgttgcacataacggctactggctggttgatggagcagtcgttaacccaattcctatttccctcacgcgtgcattgggggctgatattgtgatagcggttgacctgcagcacgatgctcatttgatgcaacaagatttgctctcctttaatgtcagtgaagaaaatagcgagaatggtgattctctgccgtggcatgcgcgtctgaaagaaaggttaggcagcataacgacacgtcgggcggtgacagcgccaacggcaacagagattatgaccacttctatccaggtgctggagaaccgccttaaaaggaaccgcatggcaggtgatccgcccgatattctgattcaacctgtttgcccgcaaatatctacgcttgatttccatcgcgcgcacgctgccattgcggccggacagctggcagtggaaaggaaaatggacgaacttttgccgttggtacgcaccaacatttgaccagaatttttatctacacttaagttaattctgacaggcgcaggtggcaatagcatgccactattgagtaaagccagtcaggggagagaacatgacgcagccattggtcggaaaacagattctcattgttgaagatgagcaggtatttcgctcgcttctggattcatggttttcctcattgggagcgacaacggtactggcggctgatggggtggatgcccttgagttgctgggaggtttcactccagacctgatgatatgtgatatcgcgatgccacgaatgaacgggcttaaactgctggagcatatacgtaacagaggcgaccagaccccagttctggtgatatctgccactgaaaatatggcagatattgccaaagcgttacgtctgggcgttgaagatgttttgctgaaaccagttaaagatctgaatcgcttgcgcgagatggtttttgcctgtctctatcccagcatgtttaattcgcgcgttgaggaagaggaaaggctttttcgcgactgggatgcaatggttgataaccctgccgcagcggcgaaattattacaggaactacaaccgccggttcagcaggtgatttcccattgccgggttaattatcgtcaattggttgccgcggacaaacccggcctggtgcttgatattgccgcactttcggaaaacgatctggcattttattgccttgatgtcacccgagctggacataatggcgtacttgctgccttgttattacgcgcattgtttaacggattattacaggaacagcttgcacaccaaaatcaacggttgccagagttgggcgcgttattgaagcaggtaaaccatttacttcgtcaggccaatctgccggggcagtttccgctattagttggctattatcatcgcgaactgaaaaatctcattctggtttctgcgggtctgaatgcgacgttaaataccggcgaacaccaggtgcaaatcagtaatggtgttccgttaggcactttaggtaacgcttatttgaatcaattgagccagcgatgcgatgcctggcaatgccaaatatggggaaccggtggtcgactgcgcttgatgttgtctgcagaatgagcaaacgataacgcgggctaaatttgcattacctgctaatgtcggctggtggtactatcgtcgccattcgtataagtaattgtcttaattatgctaactcgcctccttttcagaacttagccccttcggggtgctgatatactgggatgcgatacagaaatatgaacacgttcaaaacacgaacagtccaggagaatttaaatggctgccattaatacgaaagtcaaaaaagccgttatccccgttgcgggattaggaaccaggatgttgccggcgacgaaagccatcccgaaagagatgctgccacttgtcgataagccattaattcaatacgtcgtgaatgaatgtattgcggctggcattactgaaattgtgctggttacacactcatctaaaaactctattgaaaaccactttgataccagttttgaactggaagcaatgctggaaaaacgtgtaaaacgtcaactgcttgatgaagtgcagtctatttgtccaccgcacgtgactattatgcaagttcgtcagggtctggcgaaaggcctgggacacgcggtattgtgtgctcacccggtagtgggtgatgaaccggtagctgttattttgcctgatgttattctggatgaatatgaatccgatttgtcacaggataacctggcagagatgatccgccgctttgatgaaacgggtcatagccagatcatggttgaaccggttgctgatgtgaccgcatatggcgttgtggattgcaaaggcgttgaattagcgccgggtgaaagcgtaccgatggttggtgtggtagaaaaaccgaaagcggatgttgcgccgtctaatctcgctattgtgggtcgttacgtacttagcgcggatatttggccgttgctggcaaaaacccctccgggagctggtgatgaaattcagctcaccgacgcaattgatatgctgatcgaaaaagaaacggtggaagcctatcatatgaaagggaagagccatgactgcggtaataaattaggttacatgcaggccttcgttgaatacggtattcgtcataacacccttggcacggaatttaaagcctggcttgaagaagagatgggcattaagaagtaacatccgtatcggtgttatccacgaaacggcgttgagcaatcgacgccgtttttttatagcttattcttattaaattgtcttaaaccggacaataaaaaatcccgccgctggcgggattttaagcaagtgcaatctacaaaagattattgcttgatcaggaaatcgtcgagggatttaccttgctcatccattgcttttttgattacagctggagtacggccttggccagtccaggttttagtttcgccgttttcgtcaacgtagctatattttgccggacgctgagcacgtttagctttggtgccagatttaacggcagcaaggctattcagcagttcgttcgggtcaataccgtcagcgatcagcatttcgcgatattgctgcagtttacgagtgcgctcttcaacttcagcagcagccgcgctttcttcttcgcgacgttcgttaacaacaacttctaatttttccagcatttcttccagcgtttcaagtgtacattctcttgcctgcgcacgaagagtacggatgttgttcagaattttaagtgcttcgctcattgtagtaatctcaaacttatattggggtggtttgttgaggtaataatagagccttaaattcagttgtgcaatagccaggaatgtaaggaattcaaaattgttctttattttgtgccgccaataaatatcttttcataaaattagccagaaaagacgcggcatatagccctatttacaccgatgatttcgcagcacgtgaggttaaaacttcctgattcatgtcacattttatggggagattatcgtaggctgacgacctttcagtcttctgtattagttgtgtttacgagaattccctattaagcgaatgatgaaaagtagaacagtcgcaataagagcatggacttagtattgcactatctcctggaggtcaacagagggctattacttgcgcaacaggttaaagattgtgaatagttaccagcagtcatttacccgcttataacaagcgaggcagttgtaatgatagctcagaaggattatgcaaggcttcgtaagggagaacgcatatacccacttctgtgcatactgttgagctgaaaaactgacgaattatgataaactccagccaactttatttcatatcattgagggcctgtggctgatggcacagctatatttctactattccgcaatgaatgcgggtaagtctacagcattgttgcaatcttcatacaattaccaggaacgcggcatgcgcactgtcgtatatacggcagaaattgatgatcgctttggtgccgggaaagtcagttcgcgtataggtttgtcatcgcctgcaaaattatttaaccaaaattcatcattatttgatgagattcgtgcggaacatgaacagcaggcaattcattgcgtactggttgatgaatgccagtttttaaccagacaacaagtatatgaattatcggaggttgtcgatcaactcgatatacccgtactttgttatggtttacgtaccgattttcgaggtgaattatttattggcagccaatacttactggcatggtccgacaaactggttgaattaaaaaccatctgtttttgtggccgtaaagcaagcatggtgctgcgtcttgatcaagcaggcagaccttataacgaaggtgagcaggtggtaattggtggtaatgaacgatacgtttctgtatgccgtaaacactataaagaggcgttacaagtcgactcattaacggctattcaggaaaggcatcgccacgattaataagaatttctttactgacagggtgagcagggcacttttatcctgtcagttcgttttacgcacttcttccgggctatatacccttctcggcagttttttaacgccgctatacgcctcacagggctcttaagcaccgacgttgacttgtgacctgtaaagtacaatatccctgtgtttaggcgttatacatcgtcgcaaatatgatgaaggctaatgctgtcggtttatggaaaagttgctttgggtaaacaaaaaatacggccccagaagggcaatgccgttcacttaagaggagcggcactatgtttcacaggataacgggtttttgatatcttaaccgacctcggccttgatggtcgggggcgttttgttatgaacaccacttccagagcaccccgaagatgctccagtcgtttcgggatggtccctggtgacgccgtgtttcccagctctatcatttctgatgcgatattcttccacgcaggcagtagccagtggcggttacaacccttctggttcagcgtcagcagcaggtcttcgctgtaaaaaagtttatcaaacaacgtaatagagttatccgggatggtggcgagcatggagtgggccagcacagtttcgctctgccggtaaggtgcggtcacggcattcagcagaatgtgacttcccaggttcattaaggccaccagacgcataaccgggtaggcgttctgccgcttagtggatgtgttggcagacccataatattcacgcagctcgggtttatcaggtgtcctgaactgtgcgccatcaatggcaaaaagttgcaggccgtgccagtcatccttcaggtaacgttccgcgcccctgtctgtgcggtctggcggaagagccattccactggggcggcccccacgcgctgacgcgcctgggtgacagcgctgcgggccagcaggttcatccccgcttcgccatccgcgctcaggttcagacggcgaacaacatcggtaattggctcattgcaccaccatccagataaccatgtcccccggtaaacgacggcggcgaacggtcgcatgagcagaaagcgtcaggcagtgttgtatccactcggtgggaaggtgttctgcaaatagttgtgcagagggcggaggcataagcggatggtcactgaaatcgagcagatcattgagaagtggcataagaaaacggctccctgttgtggaagccgttatagtgcctcagtttaaggatcggtcaactaatccttaactgatcggcattgcccagaaggggccgtttatgttgccagacagcgctactgattaagcggattttttcgcttttttctcagctttagccggagcagcttctttcttcgctgcagtttcaccttctacataatcacgaccgtagtaggtatccagcagaatctgtttcagctcggagatcagcgggtaacgcgggttagcgccggtgcactggtcatcgaatgcatcttcagacagtttatccacgttcgccaggaagtctgcttcctgaacgccagcttcacggatagatttcggaatacccagttcagctttcagcgtttccagccatgccagcagtttctcgatcttagcagcagtacggtcgcccggtgcgctcagacccaagtggtcggcaatttcagcataacgacggcgagcctgcggacggtcatactggctgaatgcagtctgcttggtcgggttgtcgttcgcattgtagcgaataacgttacaaatcagcagggcgtttgccagaccgtgcggaatatggaactgggaacccagtttgtgcgccattgagtgacatacacccaggaaggcgttcgcaaacgcgatacccgcgatagtcgctgcactgtgaacacgttcacgcgctaccggatttttagacccttcgtggtaggacgctggcagatattctttcagcagtttcagtgcctgcagagcctgaccatcagagaactcagatgccagtacagaaacataagcttccatggcgtgagttactgcgtccagaccaccgaaagcacacagggacttcggcatgtccataaccaggttggcgtcgacaatcgccatatccggagtcagcgcatagtctgccagcggatatttctgaccagtagcgtcgtcagttacaaccgcaaacggagtgacttcagaacctgtaccagaagtggtggtgacagcgatcattttcgctttcacgcccattttcgggaacttgtagatacgtttacggatatccataaagcgcagcgccagctcttcgaagtgagtttccggatgttcgtacataacccacatgatcttcgcggcgtccatcggggaaccaccacccagcgcgataatcacgtctggtttgaaggagtttgccagttctgcacctttacgaacgatgctcagggtcgggtccgcttctacttcgaagaagacttcagtttcaacgcctgctgctttcagtacggaagtgatctgatcagcataaccattgttgaacaggaagcggtcagtcacgatgagcgcacgtttgtggccatcagtaatcacttcatccagcgcgattggcagggagccacggcggaagtagatagatttcggaagtttgtgccacaacatgttttcagctcgcttagcaacggttttcttgttgatcaggtgtttcggaccaacgttttcagagatggagttaccaccccaagaaccacaacccagagtcagggaaggtgcgagtttgaagttatacaggtcaccgataccaccctgagacgctggggtgttaatcaggatacgcgccgttttcattttctgaccgaagtaagaaacgcgagccggttggttatcctggtcagtgtacaggcaagaggtatgaccgataccgcccatagcaaccagtttctctgctttttctaccgcgtcttcgaaatctttagcgcggtacattgccagagtcggggacagtttttcatgtgcgaacggttcgctttcatcaacaacggtcacttcaccgatcagaatcttggtgttttctggtacagagaagcctgccagttcagcaattttataggctggctgaccaacgatagccgcgttcagcgcaccgtttttcaggataacatcctgaacagctttcagctctttaccctgcaacagatagccgccgtgggttgcaaaacgttcacgtacagcgtcataaacagagtcaacaacaacaacagactgttcagaagcacagattacgccgttgtcgaaggttttggacatcagtacagatgcaactgcacgtttgatatcagcagtttcatcgataacaactggagtgttgcccgcgcctacaccgatagctggtttaccggagctgtatgcggctttaaccatgcccggaccaccagtcgcgaggatcaggttgatgtctgggtggtgcatcagtgcgttagacagttcaacagaaggttgatcgatccagccgatcagatctttcggagcaccggcagcgatagcagcctgcagaacgatatcagccgctttgttggtggcatcttttgcacgcgggtgcggggagaagataatggcgttacgggtcttcagactgatcagcgatttgaagatagcagttgaagtcgggttagtggtcggaacgataccgcaaataataccgattggttcagcgatagtgatggtaccaaaagtgtcgtcttcagacagaacaccacaggttttttcatctttataggcgttgtagatatattcagaagcaaagtggtttttgatcactttatcttcgacgatacccatgccggattcggcaacggccattttcgcgagtgggattcgagcatctgcagcagccagagcggcggcgcggaagattttgtctacttgctcttgagtgaaactggcatattcacgctgggctttttttacacgctctacgagtgcgttaagttcagcgacattagtaacagccataatgctctcctgataatgttaaacttttttagtaaatcatctgctcgaatacgagagtatagtcagtgcggtgatgatttgcttaacctatgaaaatcaaaagcttactcgcgctcacactcactgtgatttactaaaagagtttaaacattagagttattatctctaatgcgtcacttccaggtggcgtaagcaagattactcacttctgggtactgattacgtgatccaaatcaaatttttgcaaagctgacacctttcagcatcgcttttcgccattatagctaacagttaataaattgtagtatgatttggtggctacattagcatgttttgcacaactagataacaataacgaatgatagcaattttaagtagttaggaggtgaaaaatgctgtcaaaaggcgtattgtcagcgcgtcttttcaaccttatttatggctaacattatccggcttttgcttcggagctaaccgtgattcagaccttttttgattttcccgtttacttcaaatttttcatcgggttatttgcgctggtcaacccggtagggattattcccgtctttatcagcatgaccagttatcagacagcggcagcgcgaaacaaaactaaccttacagccaacctgtctgtggccattatcttgtggatctcgctttttctcggcgacacgattctacaactttttggtatatcaattgattcgttccgtatcgccgggggtatcctggtggtgacaatagcgatgtcgatgatcagcggcaagcttggcgaggataaacagaacaagcaagaaaaatcagaaaccgcggtacgtgaaagcattggtgtggtgccactggcgttgccgttgatggcggggccaggggcgatcagttctaccatcgtctggggtacgcgttatcacagcattagctatctgtttggtttctttgtggctattgcattgttcgctttatgttgttggggattgttccgcatggcaccgtggctggtacgggttttacgccagaccggcatcaacgtgattacgcgtattatggggctattgctgatggcattggggattgaatttatcgttactggtattaaggggattttccccggcctgcttaattaattcctttcaaatgaaacggagctgccatgctccgtttacttcgtcattatttttactttgttcccgcgcagttatcaaaagcaaaaggaataggtaaaaatattcttctcaaattacagttagttataaggatttccttaactgcttctcctcaccatcatgttattttcgccacatcataatcctgggcttgctgaagaataattgaaatgatattattaattccactgcctttggtagaggaaagtgctaaataataatcaattgttaaattattgtgcatttcactactggaactgtaatcagaaaagatagacatgcttagccaatctctatttgattgaattgaaagatgtttgttaaggcatggatgcaagctatagattctgatacggtcaataaaagagaattgcttaacaattttgcaaaatgtattggcgagtaagaaccgcatttggtactttccgggcaaccgccagacgattctttattggtaatgagaataattaacaattaaagagcgtcgcgaaagaataatgtgtctcgacaggggagacacagtacgaatcgacataaggtgatcgtctgaatcaccagaataaataaagtcggtgatagtaatacgtaacgataaagtaacctgacagcagaaagtctccgagcctgtgcagggtcccaatccgggattacacatgctggttaataccagtaattataatgagggagtccaaaaaacaatgaccaacatcaccaagagaagtttagtagcagctggcgttctggctgcgctaatggcagggaatgtcgcgctggcagctgatgtacccgcaggcgtcacactggcggaaaaacaaacactggtacgtaacaatggttcagaagttcagtcattagatccgcacaaaattgaaggtgttccggagtctaatatcagccgagacctgtttgaaggcttactggtcagcgatcttgacggtcatccagcacctggcgtcgctgaatcctgggataataaagacgcgaaagtctggaccttccatttgcgtaaagatgcgaaatggtctgatggcacgccagtcacagcacaagactttgtgtatagctggcaacgttctgttgatccgaacactgcttctccgtatgccagttatctgcaatatgggcatatcgccggtattgatgaaattcttgaagggaaaaaaccgattaccgatctcggcgtgaaagctattgatgatcacacattagaagtcaccttaagtgaacccgttccgtacttctataaattacttgttcacccatcaacttcaccggtgccaaaagccgctatcgagaaattcggcgaaaaatggacccagcctggtaatatcgtcaccaacggtgcctataccttaaaagattgggtcgtaaacgaacgaatcgttcttgaacgcagcccgacctactggaacaacgcgaaaaccgttattaaccaggtaacctatttgcctattgcttctgaagttaccgatgtcaaccgctaccgtagtggtgaaatcgacatgacgaataacagcatgccgatcgaattgttccagaagctgaaaaaagagatcccggacgaagttcacgttgatccatacctgtgcacttactattacgaaattaacaaccagaaaccgccattcaacgatgtgcgtgtgcgtaccgcactgaaactaggtatggaccgcgatatcattgttaataaagtgaaagcgcagggcaacatgcccgcctatggttacactccaccgtatactgatggcgcaaaattgactcagccagaatggtttggctggagccaggaaaaacgtaacgaagaagcgaaaaaactgctggctgaagcgggttataccgcagacaaaccgttgaccatcaacctgttgtataacacctccgatctgcataaaaagctggcgattgctgcctcttcattgtggaagaaaaacattggtgtaaacgtcaaactggttaaccaggagtggaaaacgttcctcgacacccgtcaccagggtacttttgatgtggcccgtgcaggctggtgtgctgactacaacgaaccaacttccttcctgaacaccatgctttcgaacagctcgatgaataccgcgcattataagagcccggcctttgacagcattatggcggaaacgctgaaagtgactgacgaggcgcagcgcacagctctgtacactaaagcagaacaacagctggataaggattcggccattgttcctgtttattactacgtgaatgcgcgtctggtgaaaccgtgggttggtggctataccggcaaagatccgctggataatacctatacccggaatatgtacattgtgaagcactaatggcaatacgtggggcaggagtgtcctgctccacggtgtctgatttttatcgcattacagaaggcacaggccagaaggtagggcaatgttaaaatttattctacgtcgctgtctggaagcgattccgacgctatttattcttattactatttcgttctttatgatgcgcctcgcgccgggaagcccttttaccggcgaacgtactttaccgccagaagtgatggccaatatcgaagcgaaatatcatcttaatgatccgatcatgacacagtatttcagctacctgaaacaactggcgcacggtgatttcggtccatcgtttaaatataaagattattcggtcaatgacttggttgcatccagttttcccgtttctgccaaactgggagccgcagcatttttccttgcggtaatactgggtgttagtgctggcgttattgccgcattaaaacaaaacaccaaatgggactataccgtgatggggctggcaatgaccggggttgttatccccagttttgtggttgcaccattattagtcatgatatttgcgatcattttgcattggctgccgggcggtggctggaatggtggggcgcttaaattcatgatattgccgatggtggcgttgtcactcgcttatatcgccagtattgcgcgtattacccgtggctctatgattgaagtattacactccaattttattcgtactgcccgggcgaaagggttacctatgcggcggatcattttacgtcacgcattaaaacctgctctgttacccgtgctctcttatatgggccccgcatttgtcggcattattaccggttctatggttatcgaaaccatttatggtttgccggggattggacaactgttcgttaatggcgcattgaaccgtgactattccttagtgttaagcctgaccatcctggttggtgctttaaccattttgtttaatgccattgtcgatgtgctatatgcggttatcgacccgaaaatccgttactgatactggagctcgcgatgatgttaagtaagaaaaacagcgagacgctggaaaatttcagtgaaaagctggaggtcgaagggcgcagcttgtggcaggacgcacgtcgacgttttatgcataaccgtgcggcggttgccagtctgatagtgctggtgctgatcgcgttatttgtaatcctggcaccgatgctttcccagtttgcctatgacgatactgactgggcgatgatgtccagcgccccggatatggagtccggtcactactttggtactgactcatccggtcgcgacctgcttgtgcgcgttgcgattggcgggcgtatctcactcatggtcggtgttgctgcggcactggtggctgtggtcgtcgggacactttatggttcgctttccggttatctgggcggtaaagtggattcggtaatgatgcgtctgctggaaatcctcaactccttcccattcatgttcttcgtcattttgctggtgacctttttcggtcaaaacatcctgctgattttcgtggcgataggcatggtttcctggctggatatggctcgtattgtgcgtgggcaaaccctgagtctgaagcgcaaagagtttattgaggcggcacaagttggcggtgtatcgacatcgggcattgttattcgccacattgtgccgaatgtactcggtgtggtggtggtctacgcatcacttctggtgcccagcatgatcctctttgaatctttccttagcttcctggggttgggtacgcaagagccgttaagcagctggggtgcattgctgagtgatggcgcgaactcgatggaagtctctccatggttattgttgttcccagcgggattcctcgtggtgacgctgttttgtttcaactttatcggcgatggcttgcgtgatgccctcgacccgaaagatcgttaaggagtgcagccatgagcgtaattgaaactgcaactgtgccgctcgcacaacaacaggctgacgcactgctgaacgtgaaagatttgcgtgtcacctttagtaccccggacggcgacgtcacggcggtcaatgatttgaatttttccctacgtgccggagaaacgctgggtattgtaggtgagtctggttcgggtaaatcgcaaactgcatttgcgttgatgggcctgttggctgccaacggacgtattggcggatcggcaaccttcaatgggcgtgaaatcctcaatttgccagagcatgaactcaataaactgcgcgctgaacaaatctcaatgatttttcaggacccaatgacttcgttgaatccctatatgcgcgtcggtgagcagttgatggaagtgctgatgctgcataagaacatgagcaaagctgaggcgtttgaagagtcggtgcggatgctcgatgcggtaaaaatgccggaagcgcgtaaacgcatgaaaatgtacccgcacgaattttctggcggcatgcgtcagcgagtcatgattgcgatggccttgttatgtcgacctaagctgctgattgcggatgaaccaacaactgcgctggacgtcaccgtacaggcgcagatcatgacgctattaaatgaactgaagcgggaatttaataccgccatcattatgatcacccacgatcttgtcgtggtggcggggatctgcgacaaagtgctggtaatgtacgccgggcgcacgatggaatatggcaacgcgcgcgatgtcttttatcaacccgttcatccttattctatcggtttgctcaacgcggtgccgcgtctcgatgcggaaggtgaaacaatgttgaccatcccgggtaatccgccaaacctgctgcgattaccgaaaggttgcccgttccagccacgttgtccgcatgcgatggaaatttgtagtagcgcaccgccgctggaagagtttacgcctggccgtctgcgtgcttgctttaaaccggtggaggaactgttatgaatgctgtaactgaaggaagaaaagtcctccttgaaatcgccgatcttaaagtgcactttgaaatcaaagatggcaaacagtggttctggcaaccgccgaaaacgctcaaagccgtcgatggtgtcactcttcgcctgtatgaaggggaaacattaggtgtggtaggggaatcgggatgcggtaagtccacctttgctcgcgccatcatcggtttggtcaaggcgaccgacggtcatgttgcctggttaggtaaagagttgctgggcatgaaacccgatgaatggcgtgccgttcgcagtgatattcagatgattttccaggatccgttggcatcgctaaacccgcgtatgaccatcggcgagatcatcgctgaaccactgcgtacttatcatccgaaaatgtcacgccaggaagttcgcgagcgcgtgaaggcgatgatgctgaaagtcgggttattgcctaacctgattaaccgctatccgcatgagttctctggtgggcagtgccagcgtatcgggattgcgcgtgctcttattcttgaaccgaagctgattatctgtgatgagccggtgtcggcgctggacgtgtcaattcaggcacaggtggtcaacctgctccagcaattgcaacgtgagatgggattgtcattaatttttatcgctcatgacctggccgtggtaaaacacatttccgatcgtgtgttggtgatgtatctcggccatgcggtagaactggggacctatgatgaggtctaccacaatccactacatccttacaccagggcattgatgtcggcagtccccatacctgatccggatctggagaagaacaaaaccatccagttactggaaggggaattaccgtcgccgatcaacccgccttccggttgtgttttccgtacccgttgcccgattgccggtccagagtgcgccaaaacacgtcctgttctggaggggagtttcagacactccgtttcttgcctgaaagtcgatccgctttaaaaacaataagggctgacagttgtcagccctttttcacgctaaaagcgattatttattcccgccagatgatatggcaaagtttgtgatctttttcgcggcataacagaatgcgggcaaaaacatcgttgatttcaccatcttcactgtccgccagaccaatcaccacttcggcaaaaaagtccgggttcaaatcgaaatcaacatgttcctgccagtcttccgccggatcgaataactccgcgccgccgcgctcttcaaactgaagattgaacagcagaacatcagctggatcgagattgtcggcagccagttcgagaaaaatatcgtaggcctgttcaagcgtttcatcttcagtcaggcgattgtttagatccatatccatagttactacctgtttaacctctgttggcgacgttttacagcaacggactgaagaagtaaaacagtcgctcggcgacacgttgccataatggacgttttagccataaacgggcatcgagcagacgtgaacgcgaaatataatcgtcctgaacggcggcgaggtcagcaccaaaacctttatcgtcgattgccagggtaatctcgaaatttagccacagactacgcatatcaaggttaactgtgccaaccagacttagttcgccatcgaccagcacgctcttggtatgcagtaacccgccttcaaactgataaattttaaccccagcagccagcagttccgtaaagaatgcgcgactggcccagccgaccagcatcgagtcattttttcgcggaaggataatactgacatccaccccgcgctgcgccgccgtgcaaatcgcatgaagtaaatcatcgcttggcacaaagtagggcgtggtcatgatcaaatattcacgcgccgaataagccgcagtcaataatgcctggtgaatgagatcttccggaaagccggggccagaagcaattgtgtgaatggtgtgaccgctggcctgttcaaacggcataatattgacatctggtggtggcggcagaatacgttttccggtttcaatctcccagtcgcaggaataaataatccccatcgcggtggcgatagggccttccatacgcgccatcagatcaatccattgccctacgcccgcatcttgtttgaagtagcgaggatcgaccatattcatgctgccggtgtacgcgatgtaattatcgatcatgatcatcttgcgatgttggcgcaggtccatacggcgtaaaaacacacgcatcagattgacctttaaggcttcgaccacttcaataccggcattacgcattagctcgggccacgggctgcggaaaaaagccacactcccggcggagtcgagcatcaatcggcaatgaatgccgcgtcgcgcagccgccattaatgattcagccacctggtccgccatgccgccgggctgccagatataaaacaccatctcaatattatggcgcgcgagctggatgtcgcggattaacgcctgcatcacatcatctgactcggtcatcagttgtagctgattccctttgaccccagcgatcccctgacgacgctcgcaaagcttgaataatggcgcagcgacactgctattttcttcggcgaagatatgcttacaggctttaaggtcgttaagccattttgcggtggaaggccacatcgctctggcgcgctcagcgcggcgtttgcctaaatggagctcgccaacggcaagataggcaataattccgactaacggcagaatgtaaataatcaacagccaggccatcgcggagggaactgcgcgtcgtttcattagaatgcgtaaagttacgcctgcaatgagcaaccagtatcccagaatggccaaccaactcaccaacgtataaacggttgtcatagattagaaatccttttgaaagcgcattgttatgagtttacgcatatggattcatctggcaaataaaaacgcgggaaaagcactggtcagcgtcgggggtgggggtataatgaccattctgttattgcatagagtagttaacatgaagcggagtagaacggaagtggggcgctggcgcatgcagcgtcaggctagccgacgtaaatcgcgttggcttgaggggcaatcgcgccgaaatatgcgtatccacagcatcaggaagtgcattctaaacaaacagcgtaactcgttattgtttgcgatctacaatatctaaatgtactgggcaccattgcggtgcccaataagtttactcttccgtctttaaactctatttttgcgccgattctttactgtcagctttcgtttctagttcatcgttatcgctgaaaataccatgacctgagttcaacaacattgaaacgagcatatcattattaatctcttcaccatttaaaactcgcgccagaatttcgctgccaaacagttgcggtgagagaatgatatccggatgtaccatcttaatcttattcaggtttttgctatcactgacggcgagaactgttttgacatcactgctcatatcttttgccgagagtacaacaaacgcgttatctgcatcgttatcactcagcgccagaatggcccggcaacgatcgattcccgctttctttaatacagaactgtcattactgtcaccggggataacatcagcattatcgcctaagcgttgctcaagttgcttgatatcatcttcaggcaagttgctgataaccgttacgttttgtccgcgttgattcagttgcaggatcgtattgatggcgagaatcgaatgtccgcaaacaataaaatgatctttacgatgcattgtatgattgtttccttttacaagtttgttgaatcccccgcggataagcggaccaaaaattgaggtcatagatgtggcaaaaacggtaatgccggaaataatgaccgaaatagtgaacaatcgtgctgattcagaaacagggacaatatcgccatagccgacggttgacatggtttctatcgaaaaatagaacgcggtcatcaaactttctattcgcggattaaaaccttcgcttaaataaagcgcaccgtaggttgagtaaaacagtaatgtcgtgaaactaataaatgcaaaaattgtcccggctgcggcgctactgtgggagaagtctttgcgcagtatcagcaaaaacaccagcgtaaaaatgcaaaatccaatactaaatttcagccagggataaaaatgcagggtgtaaattagcgctatcaacaacaaaatgatactgattgcccatgcgagctttgcccggaacagtaagccaatggagttcaggacaagaaagacgccgagcataaagagtggggcgtttgccagcaaggagagatccaactctgaaaatgctttgatatggaaaatatcaagcaaattgaccgacataccatagattgttttaaaaataagcaatccatttaaaaagacggccagcgcgagaatgtcgtgccgaagggtcacccataaatttgttgctgtttgtttgaatgtagcccagtgactcactgatacctctgtaaccacaattttgtttaattatcttagcgtgcacattttctgaacatacatgcagcgcgtgaatgtgttaaacaatagtagatgactttatccgcagtaatcaaaggatttgagcgagcaactgtacctcaggaaaggtcatttttcctgaatatgctcacatcatataaagaaatacagataaagttattatctgcttgtggtggtgaatgcactgaccggctataaggaaaggccaaacaagaacacggttgcaaaaaccgtgcccttaaatattgaatctctattcagaacactttcttaaatggtttcactgaaacgtgttcatagactcctgccgctacgtacgggtcagcatcggcccaggcctgagctgcttccagcgattcaaattcagcaataacggttgagccagtaaatcccgcagcccctggatcgttactgtctaccgctggcattggaccagctgtcaacaaacgaccttcatcatgcagtaactgtaaacgtgctaaatgtgccggacgaacggaaaggcgtttttcgaggctatcagctttgtcttgagcgtaaataacatacaacacgggcacaactccttgttcgggaaagttgtaaagtacgttatttgaaagggcgaagatctgcaacggaaagatgatgtctttgttaaggccatgcataaagtaagggtaattacgccaaaaatgacattttcactgatcctgatcgtcttgccttattgaatatgattgctatttgcatttaaaatcgagacctggtttttctactgaaatgattatgacttcaatgacccttgatttacctcgccgcttcccctggccgacgttactttcggtctgcattcatggtgctgttgtggcgggtctgctctatacctcggtacatcaggttattgaactacctgcgcctgcgcagccgatttctgtcacgatggttacgcctgctgatctcgaaccgccacaagccgttcagccgccaccggagccggtggtagagccagaaccggaacctgagccgatccccgaaccgccaaaagaagcaccggtggtcattgaaaagccgaagccgaaacctaagccaaaaccgaagccggtgaaaaaggtacaggagcagccaaaacgcgatgtcaaacccgtagagtcgcgtccggcatcaccgtttgaaaatacggcaccggcacgcctgacatcaagtacagcaacggctgcaaccagcaagccggttaccagtgtggcttcaggaccacgcgcattaagccgtaatcagccgcagtatccggcacgagcacaggcattgcgcattgaagggcaggttaaagttaaatttgacgttacgccggatggtcgcgtggataacgtacaaatcctctcagccaagcctgcgaacatgtttgagcgtgaggtgaaaaatgcgatgcgcagatggcgttatgagccgggtaagccaggcagtgggattgtggtgaatatcctgtttaaaattaacggcaccaccgaaattcagtaagcagaaagtcaaaagcctccgaccggaggcttttgactattactcaacaggtaaggcgcgaggttttccttcaggatcaaccgcgacatacttaaataatgcttctgtcgctttatagcgttgcccaattggttcagacgctacttttttcacccacacttcaatattaatgctgaccgatgtcgtccctttctggacacagcgtgcatagcagcacaccacatcgccgaccgcaaccggccgtaagaaagtcattccttcaacccgcacagtcactacgcgaccgtgggcaatttcttttgccagaatagcgccgccaatatccatttgtgacattaaccaaccaccaaagatgtcaccattggcattggtatcggcgggcatggctaaagtacgtaaaacaagatcgccctgagggacgttatgtgttgtagacatggtaaaaccgacttaaaaggaaaatcacaggcgcgatgctactatgattttcctgaggagaacagaggagatacagcgccagccccgaaggactggcagtctggttaggatttatcttcctgcggcatgtggcggtagatatagataccgcttaacaatgtgaagattaaggtaagggcggtcaggccaaagactttaaagttgacccaaatattttgcggcagccagaatgcgatgtagatgtttgccagaccgcaaaggataaagaaaacagcccaggccagattcagcttcgaccataccggttgcggcagcgtgagttctttacccagcatccgctgaattagcggctttttcatcacccattggctgactaacagggctcccgcaaatagagcataaatgacagtaaccttccatttaataaactcatcattgtggaagaacagcgtcaagccaccgaagacgaccaccagaacaaaagtgatcagggccatcttctcaaccttacgaaagcgaacccagctatagataagcacaatcgccgtggcgacgatcagcgccgcagtagccgcatagatgtcataaatcttgtaaaacgcgaaaaagacaaccagcggtaaaaaatcaagaaactgcttcattttacgattccgtaatcaaatgcttaaggttattggcgaatcaacatatacaggcggaacagatagatgagcaatatggctgaaatcaggttgctcaaggtgttcgccagtacggcaccaatttccggggttaatgcggcaaaagaagaggcaaaaagcagcaacagtgtttttgccagcaaccagctcagtactgcgggtgccaccagacgcatattcgcccaagtcagccgcatactgctacgcatcgaggcaaaaacgcccattttgtcctgtaccaacatcaccggtgccagggccagtaaaatggccatgataattcccggaacgaccaccagcatgatgccaatctgtactaaaagggtagtcagaaaaatcagaataaataactttggcaatatcggcgcactggcaccaatagctcgcagcgcactgactctctgacccgcagacaccagctggataattaatattacgcctccggcgagaatggcgttaccgattaatcctgaaaaagtggacgccgctgaagcctgcagcaaaatttgttgctgttccggtgacatattctgaaccaggtcgaacaacccactactgccgctaacgggcacgccgtcattgagctgcgcaagctgtgcatcactgggtgagaaaacatgccctaacaccactgtgataaacgcacatagcaacgataccaacagaatggtcataaattgattacggaagaaatttccggtgtcacggtatacggactgcgccgtgatagacatgcactctccttgagttttatgcaggtgttaattagcgggcaattgtaccctggttaagcctcgggtggcagcatcaggtcttgtatggaaaagcatatctttgtaaagcggaggtaattgctggccttcaggcatgggcaaatcgcggcaagtggcgaccgagttaatatttgcgtagcgaaaatatttaaaaattgatttaaatcacattaaccaggattctcaatgcaacttctaaattaatccagatcaataaagggtgaattatcatatgtaatgtgatctatgtaggatcatttgttactccaatgtaggtatattcgtcacgtttttataaccataacgacggagcggatatgaaaaagttaacagtggcggctttggcagtaacaactcttctctctggcagtgcctttgcgcatgaagcaggcgaattttttatgcgtgcaggttctgcaaccgtacgtccaacagaaggtgctggtggtacgttaggaagtctgggtggattcagcgtgaccaataacacgcaactgggccttacgtttacttatatggcgaccgacaacattggtgtggaattactggcagcgacgccgttccgccataaaatcggcacccgggcgaccggcgatattgcaaccgttcatcatctgccaccaacactgatggcgcagtggtattttggtgatgccagcagcaaattccgtccttacgttggggcaggtattaactacaccaccttctttgataatggatttaacgatcatggcaaagaggcagggctttccgatctcagtctgaaagattcctggggagctgccgggcaggtgggggttgattatctgattaaccgtgactggttggttaacatgtcagtgtggtacatggatatcgataccaccgccaattataagctgggcggtgcacagcaacacgatagcgtacgcctcgatccgtgggtgtttatgttctcagcaggatatcgtttttaattccgcacaaaaacgaccccgtaatatacggggtcaataaggacatggtataaagggtattatttcttcgcttctacgccatcagtttcagagcgaattaaaaatttctcagttgtttgcggaatattctgaatcagccagtcggccatttgcttttcctcatttaaaatcgcttcgatggttggaattgaagctgtatcaccggcattttttgctgctgctaatagtgaggtgtaacaggcgatttcaaattgctcgaagacatatccgctaatagagcctttgactatttcatcagaagggaatataccaccgattgactgcccaagcgcagccattttactcatggaatctttaatgactgaacgtgaaatgtcattacgatcaagaatagtttccagttgaacaatctggtttttggtttcactaagatgttgttcaatacgagcgcgtagttcaggataattatctatacggctggccatggattcaagcatagattcggcttgcttttccattgcgtgggcgtcacgtaaccagtcatgataatgttcaatacgattcatgaaaatgtcctctttataaaatgactaaaagttaaaattcatatttcaggctttattttcggctttcttatttacgttattaatggccagatcagtcagtttgatgtcggtggccttttcttcttccagggtttctttcagaagcttcgctgctttacggtaacctaattgttcagccagcgtcgctaatgtcccgtaactggcaatctcataatgctcgactttctgtgctgcggcaatcagtgcggcatcacgcacttcgtttttctcggtactttcgatgacctcattagcttcttcaataagaccttccattgccacacatttcatgcgcttaattttcaggttcgattcggactccacaacttgatcaatacgttcaatctgtccatgagtttcctcgaggtgcgcatgaaaagcctgacttaatttttcatttgatgttgctcttgcgagttttgccagtgcccgggttaattgtttttctgcgctgtaggtatctgaaagcaggtgaataaatacatcttcaatggtcttcatattcatatttttctccagtgaaatcactgcgagccatacggcccgcagatgcaattatctttatcagctgatattaataattaacggtgaatcaggatttgcctgatttattaccaccgctttgttgaccgccttttttacccgcttcagatgcgcgttgcggatcatttttaaaattaccgccgctatgctgaccgcctttacggcctgcgtcggatgccttctcacggtcttcggcgaaatttcctgaaccaccacgatgttcggccatgttatttctcccgttgcgttgcattgtttcattaatatgagtgttgtgtgtcgacactcattaaaattagtcgctaatgagaattagtcaaattaagcgcaacgagaagatagagggaaaatatattttgaggaacattctggatatattaacaattacctgaggaataagtgacttagagaaaattattgattttactggtgttatgttgcgggattaatttgtttgattatattactgttgggcggaaaaatgacgtaagttgacgttcgaccggggtaagcgaaacggtaaaaagataaatattaaatgaatttaggatttttccggcttcattaaagaaagttaaaatgccgccagcggaactggcggctgtgggattaactgcgcgtcgccgctttcatcggttgtacaaaaactttcagtgccgccagcattttctctggctcattaatatgttgctcgatgattttaacaatggccgaaccagaaatcgcgcccgcagctcctgcatcaatcgctgcttttacctgatccggggcggaaataccaaatccctgcaatggaggtgcagcgttgtactctttcagcttcgcaaccagatgattgaggggtaacgcggcgcggttttctgcgccggtcacgcctgctcgtgacagcaaataggtgtaaccacgaccgtaagaggctatctggcgcagcaggtcgtcatcggcatttggcgggcagatgaagataggtgcgacattatgacgcaacgcggcctggcggaagggcgcggactcttcaactggcacatcggcaaccagcaccgaatcgacgccgactttttcgcactgggcataaaactcatcaatgcctttgttaaacaccagattggcatacatcaacaggccaatgggaatggtcgggtgtttctggcgaatcagtgccagcatttcaaaacattgtgccggagtcacacctgccgcaaaggcgcgcagagtggcgttttgaatcgtcgggccatccgccagtgggtcggagaaggggatacctaactccagcgcgtcagcaccggcttcaattagcgtatcgataattttcaatgactgctcaatgcccggatcaccgagcgtgacgaaaggaacgaatgcgccttctttgcgctccttcaactgggcaaacagagattcgtagcgttccatcagatttcccctcgtgctttcaaaatatcgtgaacggtgaagatgtctttatcgccgcgaccggaaaggttaaccaccagtagctgctctttatccgggttttcgcgcatcattttcaacgcatgggccagggcgtgggaggattccagcgccgggatgatcccttcgtgcaggcacagcgttttgaaggcttcaagggcttcatcatcggtaatagacacgtaatcagcgcgtccagtgctgttaagatacgcgtgttgtgggccgacagacgggaaatccagtccggcggagatggagtaagattcttcaatctgcccgtcttcggtttgcatcatcggcgctttcataccgaaatagatacccacgcgaccatgttttagcggtgcgccgtgctcgccagtttcgataccgtgaccacctggctccacaccaatcaggccgacgttggtttcattgatgaaatcagcaaacatgccgatggcattcgaaccgccgccaacacaggcgataacggcatccggcaggcgaccttctctttccagaatctgcgctttggtttcttcgccaatcatccgctgaaactcacgcacaatggtcggataaggatgcgggccagctgcggtgcccagcatatagtgcgcggtttcgtaactaccggaccagtcgcgcagcgcctcgttacaggcatctttcagcgtcgcggaaccgctatgcaccgggatcacttccgcacccattaagcgcatacgaaaaacgttaggcgactggcgttcaacgtctttggcacccatataaatacggcatttcaggccgagcagggcgctggcaagggccgacgccacgccatgctgaccggcaccggtttcggcgatgatttcggttttacccatccgcttcgccagcaacgcctgccccagcacctggttagttttatgcgcgccgccgtgcagcaaatcttcacgcttgagatacagcgtggtgttcgtcccggctgtaatgttctggcatttggtcagcgcggttggacgcccggcatagtttttcagcaggtcgttgaactgagcctgaaattcaggatctttttgcgcactgacaaaagcttcttccagctggcgcagagcaggcatcaggatttgtggcacgtacatgccgccaaactcaccaaaataggggttaagtaatgttgtcattgttcctttccttaatatgcgcgcagcgtctggaaaaccgaggccaaaagacgtgcgtctttgatgcccggttgcgactctacagcagaattaaaatcaagtccggcgcagccggtttgtgccgcttccacgcagttatctgcgcctaagccccccgccagcagaacgttgccaagcgattgaccatttaatagtgaccagtcaaaacgttgcccgcttccaccctggccgttgtctaaaacatatttatcaacgtgctgaaactcgcgggcgggcagggtttcaccgacgcttaatgctttccagatggcaacatgtgctggcagagcttcacgcagcgtatcgatatacagctgttcttcattaccatgcagttgcactgccgccagcgataacaccttagctttgtccaccacatcggcaatatcgtgattgcggaacacgccaacatactgcaacggtgccgcagccatcacttcctgcgcctgttcaacgttgacgcaacgcggtgatgtcgcaacaaaaatcaacccaccgtaaatcgcgcccgcgtcataagctgctttagcatcttgcccacgcgtcaggccacatactttattctcacccagcaacacccggcgcacggcggcgtgcaaatcgtcatgggccatcaacgccgaaccaatcagaaaaccgttagcgaagtggcttaactcgcgcacctgagcgtaagtattgatgccggattcgctgattaccgtcacgttgtgccccagtttcggcgcaagctcgcgggtacggttgagatcaatcgacaaatcacgcagatcgcggttgttgatgccaacgacctttgctcccaatgcaatggcgcgctcctgttcctcttcattactgacttcggtcagcacccccatctccagactgtgagcgacggcggcaagctggcgatattggtcgtcatccagtactgaaagcattaataagcaggcatcggcctggtaatagcgcgccagatagatctggtaagggtcgataatgaagtctttacataaaatcggctgcggggcgatttggctgacgatggggaggaaattaaagctcccctgaaaatatttctcatcagtcagcaccgaaattgccgaagcgtaatgtttataaatggcggcaatgcgtgctggatcgaaatcatcacggatcacgccttttgacggcgacgctttcttgcactccagaataaacgccgtgcgcgcaccctgtagcgcatcataaaaatgtcgcgtgctcggctgaacctcattctgaaaactggccagcggttgctgctgtttgcgggcttctacccaaatcgccttgtctgcgacgattttcgctaaaacggtttgcatcatttaccctcgtgccgccagtgcggtgactctgtcgtaagcggaaccactgcgcagtacctcaagaacggtttgcgcattggcttgcagatcttcatggccatgcaggcgcattaacatggcgacgttcgcagcgacggctgcttcatgggcggcgtcgcctttaccttgtaacaaacgtgttaaaatgtcacggttttcttccggtgttccgcctgccagttgctcctggtggtagggtgtcaggccaaagtcttctgcggtgagctgatagcttttaatttcgccgtcatgcagttcggcaacgattgtcggcgcgtgtaatgaaacttcatccatcccgccgctgtgcaccaccgccgcgcgttgataccccagcacgcgcaaggtttcggcaatcggcagcaccagttccggactataaacaccaattaacgccagcggcggatgcgccgggttaatcaatggccccagcacattgaacagggtgcgggttttcagttgctggcgaaccggcatcgcgtggcggaatccggtgtgatacttcggcgcaaagaggaaacatacacctaactcatccagcgcctggcgcgatttatcggcgttcatatcaagattaataccgaacgccgccagcagatcggacgaaccagatttactggagacgctacggttgccgtgtttcgccactttcagcccacaggccgcggcgacaaacgcactggcggtagaaatattgatactgttgctgccgtcaccgccagtaccgacgatatcagcaaacagataatccgggcgcgggaacggcgctgcgttttccagtagcgcggttgctgccccggcgatctcgttcgggtgctcaccgcgaattttcatgctcaccagcgccgccgccagttgttccggcttcagctcgccacgcaccaccgctgaaaacagctggtggctttcttgttggctaagcgtctgcgcctgatacagtttttccagaatcggttgcagcgtgttggctggctctagtttctgctgcgcccaggccagcgtttgttccagcaggcgagcgccctgggtggtgagaatggattccggatggaactggaatccacaaacgcgatccgcatcgtgacgtactgccatcaccatgccattaaaatgggcgttgatggttaaaccggccggaatgttactgccaaccagcgagtgataacgcgccaccggcagcgggtttgttaatccggcaaacatcgcctgaccgtcatgttcaatgctggaggctttaccgtggagaatttcgcccgcctgaccgacatagcccccgtaagcttcgacaatcgcctgatgtccgaggcaaatgccaataatgggcagcttgccacgcaagcgggtgaggagttccggcatacaaccggcttcgctcggcacaccggggccaggagaaagcatcagcaccggattgctcatggtcgccaggcgttcaattaaggtttgcgccggaatatggttgcggtaaatcaccacgttatgcccattgctgcgcaactgatctgccaggttgtacgtaaaagagtcgatattatcgagcagcagaatgtcagccatcagaaagtctcctgtgcatgatgcgcggtggcaatagcgcgcagtacagcgcgggctttgttacgggtttcgtcggcttccgactgcggaacagaatcaaggactacaccagcacccgcttgcacggtggcgataccgttttccaccagcgccgagcggatcacaatgcaggtgtcgagatcgccatgcgcggtgaaataacctaccgcgccgccgtagctgccgcggcgacgaccttccgcctcggcaattaactgcatagcgcgtactttcggcgcaccgcttaacgtccccatattcatacaggcgcgataagcgtgcagggcgtcaagatcgtgacgcagttcgccgactacgcgagagacgaggtgcatcacataggaataacggtcaactttggtgagatcggcgacgtagcggctgccgggggtgcaaatgcgtgccagatcattacgggcgagatcaaccagcatcagatgttcagacagctctttatgatcggtacgcatttccagttcaatacggctgtcgagatctctgtccagtgaaccatcggcgcgacgaccgcgtgggcgtgttccggcaatcgggtagatctcaatctggcggctggtggcatcatacttgagcgagctttccggcgacgcgccaaatagggtgaaatcattatcctgcataaaaaacatgtacgggctgggattactctttttcagcacgtaataggccgccagcggtgacgggcagggcagagagaaacggcgagatggcaccacctggaaaatttctccagcgcgaatcgctttttgcaacaaacgcactacgccaccgaactcttcatcgctctgattacattcacaacgcatatgcggcacggaaaccactggcagcggcggcgcggcttcggtcagttgctgacgtagttcgttcaggcgagcagtgagacgttgtttttcttcttcattcggagcaaacaggctggcctgaatacgggtgctttttttctgatggtcaatcaccatcagcgtttcagcgagataaaaacagaaatcagggcagttattttccgctgacagttgcggtaaatcttcaaatcccgccacaaggtcataagagaacaggccgccgaagaacatggcttctcgttcttccttcggtacattcaacagattctgcaataaacggaaagcgtcaaaaaccgaaagggagcataagcgggcgtcttcatccagcagtggactgacaggggggaagcgcagcacacggcagtttggtgattgttcactttccacacccgcaggcagggcgttatccagtagtgccaggagggcttcgccgttgccggaaagtgcctggattgtgacagtgtcacctaaagctgtaatgcgcagcgcactgtctaccagcagcaggctttttaaatcatctttgctgtcgatatctgcggattccagcagcagcgttgccggacgatccccacacaactggtgaaaaagcgcggtgggattgtcgcgataagcgccttcgcaggttagcagttcgagagtcggtttttgtgtttgcattgttattctctaattttgttcaaaaaaaagcccgctcattaggcgggctgggtatctgattgctttacgcatggtgaatacactgcccgtttcaggaagtgcgccaccaacctttcagtacgaaaattgctttcattgtcgataccctttttacgtgaacttgcgtactagttaactagttcgatgattaattgtcaacagctcatttcagaatatttgccagaaccgttatgatgtcggcgcaaaaaacattatccagaacgggagtgcgccttgagcgacacgaattatgcagtgatttacgacctgcacagccataccacagcttccgatggctgcctgacgccagaagcattggtgcaccgtgcagtcgagatgcgcgtcggcaccctggcgatcaccgaccatgacaccacagctgcaatcgcgccagcaagagaggaaatttcacgttcgggactggcgttgaatcttattcccggcgtggaaatttccacggtctgggaaaatcatgaaattcatattgtcgggctgaatattgatattactcatccgctaatgtgtgagttcctcgcgcagcagacagaacggcgcaatcagcgggcgcagctgattgccgaaagacttgaaaaagcgcaaatacctggggcgctggaaggcgcacaacgactggcgcagggcggcgcagtgacgcgcggtcattttgcgcgtttccttgttgagtgcggcaaagccagttcaatggcggatgtctttaaaaagtatctggcgcgcgggaaaaccggatacgttccgccacagtggtgtacaatagaacaagctattgatgtcattcatcattctggcggtaaggcggtgctagctcatcctgggcggtacaatcttagtgctaaatggctgaaaagattggttgcgcattttgccgaacaccacggtgacgcgatggaagtcgcgcagtgccagcaatcgcccaatgaacgtacccagctggcggcccttgcgcgtcagcatcatttatgggcatcacaaggatctgattttcatcagccatgcccgtggatcgaactgggtcgtaaactctggctgcccgcaggcgttgaaggcgtctggcagctatgggaacagccgcagaacaccacagagagggaattatgagccagtttttttatattcatcctgataacccacagcaacgtctgatcaaccaggcggtggagatcgtgcgtaaaggcggggtgattgtttatccaactgattccggctatgcgctcggctgtaaaattgaagataaaaacgcgatggagcgtatttgtcgtattcgccagctgccggacggtcacaactttaccctgatgtgtcgcgatctttctgaactctcgacctattcatttgttgataacgttgcgtttcgtttaatgaaaaacaacacgccgggcaactataccttcatcctgaaggggacgaaggaagtgccacgccgtctgttgcaggaaaaacgcaaaaccatcggtatgcgtgtgccttctaaccctatcgctcaggcgttacttgaagcattgggcgaaccgatgctttccacttcgctaatgctgccaggcagcgaatttaccgaatcggacccggaagaaattaaagatcgtctggaaaaacaggtagatttgattattcacggcggctatctcgggcagaaaccgacaacggttattgatcttaccgatgatacgccggtcgtggtgcgtgaaggcgtaggtgatgtgaagcctttcttataacaaattgcgttccacggatggaagactatggcagggaagtttcgctgcattttgctgttgatagcagggctgtttgtatcatctctaagttatgcagaaaacacggagatcccttcttatgaagaagggatctcgctctttgatgttgaagccactctgcaaccagatggggtgctcgacatcaaagaaaatattcattttcaggcgcgaaatcagcagattaagcacggcttttatcgtgatttaccacgactatggatgcagcctgatggggacgctgcactgctgaactatcatattgttggcgtcacccgtgatggtattcctgaaccctggcatcttgactggcatatcgggttaatgagtattgtcgtgggcgataaacaacgtttcttgcctcaaggcgactatcattatcaaattcattatcaggttaaaaatgctttcctgcgtgagggggattctgatctgctaatctggaacgtgaccggtaaccactggccgtttgaaatttataagacccgtttttctctccagttctctaatattgcgggtaatccatttagcgaaatcgatctttttaccggagaagagggcgacacatatcgtaatggccgcatccttgaggacggaagaattgaatcccgcgatccgttttatcgtgaagatttcacggtcctctaccgctggcctcacgctttacttagcaatgcctcggctccgcaaacgacgaatattttcagccatcttcttttaccctccacgtcatcgttgttaatttggtttccgtgtctgttcctggtttgtggatggttatatctctggaagcgcaggccgcaatttacgccggtagatgtgattgaaaccgatgtcattccgccagattacacgcccggcatgttacgtctcgatgcgaagctagtttacgacgataaaggtttttgtgccgatatcgtaaatctgattgtgaaaggaaaaattcatctggaagatcagtctgacaagaaccagcaaatcctgattcgtgttaatgaaggcgcgaccagaaataatgcggtattactgcccgcagagcagttattactggaagcgttatttcgtaaaggcgataaggtcgttcttacggggagacgcaacagagtcttacgcagggcatttttacggatgcagaaattttatctgccgcgtaaaaagtcttcgttttaccggtctgatacttttttgcaatggggtggactggcaatattggcggtcattctttacggtaacttgagtcctgtaggctgggcaggaatgagtctggtgggcgatatgtttattatgatctgctggattattccttttttattttgttcccttgagcttttgtttgcccgcgatgatgacaagccttgcgttaatcgtgtaatcatcactttgtttttaccactgatttgttcaggcgtggccttctattctctctacatcaatgtcggagatgtattcttttactggtatatgccagcgggttattttaccgctgtttgcctgaccggttatctcactggcatggggtatatttttctgccaaagtttacccaaactggacagcaacgttatgcccacggtgaagctatcgttaactatcttgcgcgtaaagaggcagcaacacacagtggacgtcggcggaaaggggaaacacggaaactggattacgcgttgctaggttgggctatatcggcaaatttggggagggaatgggcgttacgcattgccccttcgctttcttcggcgattcgcgctccagagattgcccgtaacggcgttttattctcattacagacgcacctaagttgcggggccaataccagtttgttggggcgaagttattccggtggtggtgctggcggcggcgcgggtggcggaggcggtggtggctggtaattaagctgatgttaatcgaaacaagctttaaccataaagatagtgtagtatgttgcgcctcaaagccaggccgataaacgtcgagtcgtttacttaaggcctgaagagttcaaacagactttactatcagtgagtcagatgtaagttctgactcactgttgcacaaaagcatatcagacgcctgggaaggcgacaccaaaaggaagctctatgagcgaaaagctacagaaagtgctggcgcgtgccggccacggttctcgccgtgaaatcgaatctattattgaagccggtcgtgtgagtgttgatggcaaaattgctaaactcggcgatcgtgttgaagttacccctggattgaaaatccgtatcgatggtcacctgatttcggtacgtgagtccgctgaacaaatttgtcgcgttctggcctattacaaaccggaaggtgagttgtgtacccgtaacgatccggaaggacgtccaacggtgtttgaccgtctgccaaaactgcgtggcgcacgctggattgccgtgggtcgcttggacgttaatacctgtggtctgctgctgttcaccaccgatggtgaactggcaaaccgtttaatgcacccaagccgtgaagttgaacgtgaatatgccgtgcgtgtatttggtcaggttgacgacgcgaaactgcgtgatttgagtcgtggcgtgcagttggaagatggtccggcagcttttaaaaccatcaagttcagcggcggcgaagggatcaaccagtggtacaacgtgactctgaccgaaggccgtaaccgtgaagttcgtcgtctgtgggaagcggttggtgtgcaggtgagccgcctgatccgtgttcgttacggtgatatcccactgccaaaaggtctgccacgcggtggctggacggagctggacctcgcccagactaactatctgcgcgaactggtggagctaccgccagaaaccagctctaaagtcgctgtagaaaaagaccgtcgtcgcatgaaggcgaatcagattcgtcgtgcggtgaaacgtcacagtcaggtgagcggcggtcgtcgttctggcggacgtaataataacggttaatcaaagtatgccggacgtcatatccggcatttttacagattaataatcgatccctatctgcgcttttacaccggcatcaaacgcatgtttgacggggcgtaattcacttaccgtatctgccagttcaagaatatcccgatgacaaccacgacccgtgataatcaccgtctgttgatgtggacgttcatttaacgcctgcaccacttcttccagtggcaaatagtcatacgccaccatatacgtcagttcatcaagcaaaaccatatccagtgaggaatcagcaagcatccgctttgcatgttgccagacttcgcggcaggcggcggtatcagactcgcggttttgtgtatcccaggtaaagcccgttgccatcacctgaaactcaacgccatgtggctccagcagattgcgttcgccattaggccaggtgcctttaataaactgcacgacgcctactttttttccgtgaccaactgcgcgtgttgccgtaccaaatgccgcggtggttttgccttttccattgccggtaaagacgatgataataccgcgttcatcctgggcctgggccacacgagcatctactttttctttcactcgctgctgacgctgttggtagcgttcatcactcattgggaaattcctggtttacggcccggttgggcgtcaaaggtcatgccggttttacggcggctgtcatcgcccatcagccagaggtagagcggcatgatatcagcgggtgttttaagtttctgtggatcttcggtcgggaaggcgctggcacgcattgcggtgcgcgtaccgcctgggttaatgcagttgacacgcaggcgctgctgatattcatcggccagtacctgcatcatcccttcggtggcaaatttcgacgctgcatatgcaccccagttggctcgtccctgacgtccaacgcttgatgaagtaaagaccagtgaaccggcgtccgatttgagtaataaaggaagcagtgcctgggtgagcataaaggtggcattaacgttgacctgcatgacgtcctgccagacctgcggattttgttcgctcattgggcaaacatcgccgagcaatccggcattatgcaaaacaccatccagacgcggataattaacggcaatgcgctgtgccagttgttggcaattttcggacgtgcaggtcagcaaatcgagaataaaccactgtggctgacgcccagtttcttcgtttatgtggctggctacctgacgtaatttttcttcattacggcccaacagaatcactgtcgcaccatagcgtgcatacgtcatcgcggcttcacgaccaataccatcgctggctcccgtcaccaggataatgcgatcattgagtaaatcttgttttggctggtaatgcatggctactcctcaacgacgttgtctgtcgcgctgccagtgtactttatgactttggggctttatgcctgaaacagaagggcatttcaatcagcctggggcgataacaccgcaaaatggatactttgtcatactttcgctgcaataacatctctgcgagacggcttaacatgcctgttgtaaactgtgagccaaagcgttgtttaaccaaggtggggactcgtggaattgttgtctgaatatggtttgtttttggcgaaaatcgttaccgttgtgctagcgattgcggcgattgccgccattattgtcaatgttgctcaacgtaataaacgccagcgtggcgagttacgggtcaacaatctcagcgaacagtataaggagatgaaagaagaactggccgcggcgctgatggactcacatcagcaaaaacagtggcacaaagcgcagaagaaaaagcataagcaagaagcgaaagcagcaaaagcgaaagccaaactgggcgaggtggcaactgacagtaaaccccgcgtctgggtgctggattttaaaggcagcatggacgcccatgaagtgaactcgctacgtgaagagataacggctgtactcgcagcattcaaaccgcaggatcaggttgtgctccgtctggaaagccctggtggcatggtgcatggttacgggctggcggcttcgcaactgcagcgtctgcgcgataaaaacattcctttaactgttacggtagacaaagtcgctgccagcggcggttacatgatggcctgtgtggcggacaaaattgtttccgcaccgtttgctattgtgggttccattggcgtggtggcgcaaatgcccaactttaaccgcttcctgaaaagcaaagatattgatatcgaactgcacactgccgggcagtataagcgcacgctgacgttgctgggtgaaaataccgaagaagggcgggagaaattccgcgaagagttgaacgaaacgcatcagttgtttaaagattttgtgaagcgtatgcgtccttctctggatattgaacaggtggcaacgggtgaacactggtacggacaacaggcggtagagaaaggcctggttgatgaaatcaacaccagtgatgaagttattcttagcctgatggaaggccgtgaagtggtcaatgtacgctatatgcagcgtaaacgactcattgaccgattcaccggcagcgcggcagagagcgccgatcgattgttgctacgctggtggcagcggggtcaaaagccattgatgtaaaagacaaacgcgaggctaagacctcgcgttttgctttaatcaaccagatgatatttttctgaaagcacatgggccaggtgtttgaacatattaaacaccgcggtgcttttggctgttggcaatccttgttcatctaaaaagtagtcgccggtaaataccagcacgccattacgctgcgtgacgccggtggcttcaatccctgcgagcgtatcctcatgctcacgaatgattttgttggcctctttcaacagcgtttcgcggtcgatgggttgtgtctctttgttcattatttactccttaaacaaggacattagtctacgccaggcatggcttgcagacaaatataccacgctggtggcaagagcgccttactggcaactttggattttgcatgctaataaagttgcgtatcggattttatcaggtacagtgtgacgctttcgtcaatctggcaatagatttgcttgacattcgaccaaaattccgtcgtgctatagcgcctgtaggccaagacctgttaactcagtcacctgaattttcgtgaacagagtcacgacaaggggttgatatccgcagagagcgagtccatatcggtaactcgttgccagtggaaggtttatcaacgtgcgacgcattcctggaagaatcaaattaggtaaggtgaatatgggtaaagctcttgtcatcgttgagtccccggcaaaagccaaaacgatcaacaagtatctgggtagtgactacgtggtgaaatccagcgtcggtcacatccgcgatttgccgaccagtggctcagctgccaaaaagagtgccgactctacctccaccaagacggctaaaaagcctaaaaaggatgaacgtggcgctctcgtcaaccgtatgggggttgacccgtggcacaattgggaggcgcactatgaagtgttgcctggtaaagagaaggtcgtctctgaactgaaacaactggctgaaaaagccgaccacatctatctcgcaaccgaccttgaccgcgaaggggaagccattgcatggcacctgcgggaagtgattgggggtgatgatgcgcgctatagccgagtggtgtttaacgaaattactaaaaacgcgatccgccaggcatttaacaaaccgggtgagctgaatattgatcgtgttaatgcccagcaggcgcgtcgctttatggaccgcgtggtggggtatatggtttcgccgctgctatggaaaaagatcgctcgtggcctgtctgccggtcgtgtgcagtcggtggcggttcgcctggtggtcgagcgtgagcgtgaaattaaagcgttcgtgccggaagagttctgggaagtcgatgccagcacgaccacgccatctggtgaagcgttggcgttacaggtgactcatcagaacgacaaaccgttccgtccggtcaacaaagaacaaactcaggctgcggtaagtctgctggaaaaagcgcgctacagcgtgctggaacgtgaagacaaaccgacaaccagtaaacctggcgctccttttattacctctacgctgcaacaagctgccagcacccgtcttggatttggcgtgaaaaaaaccatgatgatggcgcagcgtttgtatgaagcaggctatatcacttacatgcgtaccgactccactaacctgagtcaggacgcggtaaatatggttcgcggttatatcagcgataattttggtaagaaatatctgccggaaagtccgaatcagtacgccagcaaagaaaactcacaggaagcgcacgaagcgattcgtccttctgacgtcaatgtgatggcggaatcgctgaaggatatggaagcagatgcgcagaaactgtaccagttaatctggcgtcagttcgttgcctgccagatgaccccagcgaaatatgactccacgacgctgaccgttggtgcgggcgatttccgcctgaaagcacgcggtcgtattttgcgttttgatggctggacaaaagtgatgcctgcgttgcgtaaaggcgatgaagatcgcatcttaccagcagttaataaaggcgatgctctgacgctcgttgaacttacaccagcccagcactttaccaagccgccagcccgtttcagtgaagcatcgctggttaaagagctggaaaaacgcggtatcggtcgtccgtctacctatgcgtcgatcatttcgaccattcaggatcgtggctacgtgcgagtagaaaatcgtcgtttctatgcggaaaaaatgggcgaaatcgtcaccgatcgccttgaagaaaatttccgcgagttaatgaactacgactttaccgcgcagatggaaaacagcctcgaccaggtggcaaatcacgaagcagagtggaaagctgtactggatcacttcttctcggatttcacccagcagttagataaagctgaaaaagatccggaagagggtggtatgcgcccgaaccagatggttctgaccagcattgactgcccgacttgtggtcgcaaaatggggattcgcacagcgagcaccggggtattccttggctgttctggctatgcgctgccgccgaaagagcgttgcaaaaccaccattaacctggtgccggaaaacgaagtgctgaacgtgctggaaggcgaagatgctgaaaccaacgcgctgcgcgcaaaacgtcgttgcccgaaatgcggcacggcgatggacagctatctcatcgatccgaaacgtaagttgcatgtctgtggtaataacccaacctgcgacggttacgagatcgaagagggcgaattccgcattaaaggttatgacggcccgatcgttgagtgtgaaaaatgtggctctgaaatgcacctgaaaatggggcgtttcggtaaatacatggcctgcaccaacgaagagtgtaaaaacacacgtaagattttacgtaacggcgaagtggcaccaccgaaagaagatccggtgccattacctgagctgccgtgcgaaaaatcagatgcttatttcgtgctgcgtgacggtgctgccggtgtgttcctggctgccaacactttcccgaaatcgcgtgaaacgcgtgcgccactggtggaagagctttatcgcttccgcgaccgtctgccggaaaaactgcgttatctggccgatgcgccacagcaggatccggaaggtaataagaccatggttcgctttagccgtaaaaccaaacagcaatatgtctcttcggaaaaagacggaaaggcgactggctggtcagcattttatgttgatggcaaatgggttgaaggaaaaaaataacctttaattctgtcaggtttttataaacaaagggtcgcgaaagcggcccttttttattgcatattattttttcttcacacctatacactaaggctataaatgatatagtggttatagttagcaccttttttattattaaatcgtattagtcacccgccaggtgtgacgaaaaaacgatgttctgatggcgtctaagtggatggtttaacatgaaattacaacaacttcgctatattgttgaggtggtcaatcataacctgaatgtctcatcaacagcggaaggactttacacatcacaacccgggatcagtaaacaagtcagaatgctggaagacgagctaggcattcaaattttttcccgaagcggcaagcacctgacgcaggtaacgccagcagggcaagaaataattcgtatcgctcgcgaagtcctgtcgaaagtcgatgccataaaatcggttgccggagagcacacctggccggataaaggttcactgtatatcgccaccacgcatacccaggcacgctacgcattaccaaacgtcatcaaaggctttattgagcgttatcctcgcgtttctttgcatatgcaccagggctcgccgacacaaattgctgatgccgtctctaaaggcaatgctgatttcgctatcgccacagaagcgctgcatctgtatgaagatttagtgatgttaccgtgctaccactggaatcgggctattgtagtcactccggatcacccgctggcaggcaaaaaagccattaccattgaagaactggcgcaatatccgttggtgacatataccttcggctttaccggacgttcagaactggatactgcctttaatcgcgcagggttaacgccgcgtatcgttttcacggcaacggatgctgacgtcattaaaacttacgtccggttagggctgggggtaggggtcattgccagcatggcggtggatccggtcgccgatcccgaccttgtgcgtgttgatgctcacgatatcttcagccacagtacaaccaaaattggttttcgccgtagtactttcttgcgcagttatatgtatgatttcattcagcgttttgcaccgcatttaacgcgtgatgtcgttgatgcggctgtcgcattgcgctctaatgaagaaattgaggtcatgtttaaagatataaaactgccggaaaaataatttcttgcgttattttcggcaccttttatgtagcgaaggtgccggaatatattctcttttgttacttatttctataccgtgcacaatatttttatccctcatatttatagggtaaattacctgtaaagtagtgtctaattacccgcctcgcaaactccagttttcaaatatctatttcaggtcaaaagattgaattattcactggagacgattcgtaaattcgctggatttttgactaaagtttctttaggatttgtctcatcgtatgattaattacaccaatcgttcaacgtcttgctgataagtgatggcgattatatgaggttagcaatgccttctggaaatcaggaaccccgccgcgatcctgaattaaaacgtaaagcctggctggcggtttttcttggttctgcacttttctgggtggttgtcgcactgctgatttggaaagtgtggggataactatggtcggtcaggagcaactggagtcgtcaccattatgccagcatagtgacaatgaaacagaaacgaaacgggaatgttccgtcgttattccagacgactggcaactaacatcgcagcagcaagcctttatagaactgtttgctgaagatgatcagccgaaacaataattatcatcattcttattacccatttttaatgaattaaagggcttttaatacaccgcagcaataacagcttgagttatctcaacacaaaataataaccgttaagggtgtagcctatgatcaacacaaatatgaaatattggtcctggatgggcgcgttttctctgtcgatgctcttctgggccgaactcctctggatcattactcactgatccttgaccccgctgcggcggggttgtcatttgctttgccacaaggtttctcctcttttatcaatttgggttgttatcaaatcgttacgcgatgtttgtgttatctttaatattcaccctgaagagaatcagggcttcgcaaccctgtcattaaggaggagctatgtcgtcaaccctacgagaagccagtaaggacacgttgcaggccaaagataaaacttaccactactacagcctgccgcttgctgctaaatcactgggcgatatcacccgtctacccaagtcactcaaagttttgctcgaaaacctgctgcgctggcaggatggtaactcggttaccgaagaggatatccacgcgctggcaggatggctgaaaaatgcccatgctgaccgtgaaattgcctaccgcccggcaagggtgctgatgcaggactttaccggcgtacctgccgttgttgatctggcggcaatgcgcgaagcggttaaacgcctcggcggcgatactgcaaaggttaacccgctctcaccggtcgacctggtcattgaccactcggtgaccgtcgatcgttttggtgatgatgaggcatttgaagaaaacgtacgcctggaaatggagcgcaaccacgaacgttatgtgttcctgaaatggggaaagcaagcgttcagtcggtttagcgtcgtgccgccaggcacaggcatttgccatcaggttaacctcgaatatctcggcaaagcagtgtggagtgaattgcaggacggtgaatggattgcttatccggatacactcgttggtactgactcgcacaccaccatgatcaacggccttggcgtgctggggtggggcgttggtgggatcgaagcagaagccgcaatgttaggccagccggtttccatgcttatcccggatgtagtgggcttcaaacttaccggaaaattacgtgaaggtattaccgccacagacctggttctcactgttacccaaatgctgcgcaaacatggcgtggtggggaaattcgtcgaattttatggtgatggtctggattcactaccgttggcggatcgcgccaccattgccaatatgtcgccagaatatggtgccacctgtggcttcttcccaatcgatgctgtaaccctcgattacatgcgtttaagcgggcgcagcgaagatcaggtcgagttggtcgaaaaatatgccaaagcgcagggcatgtggcgtaacccgggcgatgaaccaatttttaccagtacgttagaactggatatgaatgacgttgaagcgagcctggcagggcctaaacgcccacaggatcgcgttgcactgcccgatgtaccaaaagcatttgccgccagtaacgaactggaagtgaatgccacgcataaagatcgccagccggtcgattatgttatgaacggacatcagtatcagttacctgatggcgctgtggtcattgctgcgataacctcgtgcaccaacacctctaacccaagtgtgctgatggccgcaggcttgctggcgaaaaaagccgtaactctgggcctcaagcggcaaccatgggtcaaagcgtcgctggcaccgggttcgaaagtcgtttctgattatctggcaaaagcgaaactgacaccgtatctcgacgaactggggtttaaccttgtgggatacggttgtaccacctgtattggtaactctgggccgctgcccgatcctatcgaaacggcaatcaaaaaaagcgatttaaccgtcggtgcggtgctgtccggcaaccgtaactttgaaggccgtatccatccgctggttaaaactaactggctggcctcgccgccgctggtggttgcctatgcgctggcgggaaatatgaatatcaacctggcttctgagcctatcggccatgatcgcaaaggcgatccggtttatctgaaagatatctggccatcggcacaagaaattgcccgtgcggtagaacaagtctccacagaaatgttccgcaaagagtacgcagaagtttttgaaggcacagcagagtggaagggaattaacgtcacacgatccgatacctacggttggcaggaggactcaacctatattcgcttatcgcctttctttgatgaaatgcaggcaacaccagcaccagtggaagatattcacggtgcgcggatcctcgcaatgctgggggattcagtcaccactgaccatatctctccggcgggcagtattaagcccgacagcccagcgggtcgatatctacaaggtcggggtgttgagcgaaaagactttaactcctacggttcgcggcgtggtaaccatgaagtgatgatgcgcggcaccttcgccaatattcgcatccgtaatgaaatggtgcctggcgttgaaggggggatgacgcggcatttacctgacagcgacgtagtctctatttatgatgctgcgatgcgctataagcaggagcaaacgccgctggcggtgattgccgggaaagagtatggatcaggctccagtcgtgactgggcggcaaaaggtccgcgtctgcttggtattcgtgtggtgattgccgaatcgtttgaacgaattcaccgttcgaatttaattggcatgggcatcctgccgctggaatttccgcaaggcgtaacgcgtaaaacgttagggctaaccggggaagagaagattgatattggcgatctgcaaaacctacaacccggcgcgacggttccggtgacgcttacgcgcgcggatggtagccaggaagtcgtaccctgccgttgtcgtatcgacaccgcgacggagttgacctactaccagaacgacggcattttgcattatgtcattcgtaatatgttgaagtaacaactatttgcttgccggttattttgcttccggcaagcaaatgaattacacaatgcaagagggttatttgttcagcaaatggcccattttctcggctttggtatcgagataatgttcgttattggggttacgacctacaatcaatggtacgcgttcaacaatattaatccctgcttcggtcagaatttcgacttttttcgggttattggttaacaagcggacttcattgacgccaaggagtttgaacatatcagcgcaaagagtgaagtcgcgctcatcagcggcgaagcctaactggtggttagcctctacggtatcgtaaccttgatcctgcagtgcgtaagcgcggattttattcagcagaccaatgttacgaccttcctgacggtgatacagcaaaataccacggccttcctcggcaatttgcgtcaatgccgcttcgagctggaagccacaatcgcagcgcaagctgaacagggcgtcaccggtcagacattcggaatggacgcgcgcaagtaccggggtatgcccggaaatatcgccatagactagcgcgacatgatcgtgtccggttgccagttcttcaaatcccaccatcaggaaatcgccccatggggttggcagtttggcttctgccacacgtttaagctgcatgaaattctccagataatgctggttctgtattggcttattttgccataacgagaaggggttcacctaatcacgacgcgtcgatcgttcacggaatggcacaaatctgtcaatttttcctggaactggcgttttcagttatgattgtgggacttatcaaaaaggagaggccatgcgttcgattgccagacgtaccgcagtgggagctgcactattgcttgtcatgccagtagccgtatggatttctggctggcgttggcaacctggagaacaaagttggctactaaaagcggctttttgggttactgaaactgtcacccagccctggggcgtcattacacatttgattttattcggctggtttctctggtgtctgcgttttcgcattaaggctgcctttgtattatttgccattctggcggccgcaatccttgtgggacaaggcgttaaatcctggatcaaagacaaagtccaggaaccacgaccttttgttatctggctggaaaaaacacatcatattccggttgatgagttctacactttaaagcgagcagaacgcggaaatctagtgaaagaacagttggctgaagagaaaaatatcccacaatatttgcgttcacactggcagaaagagacggggtttgcctttccttccggtcacacgatgtttgctgccagttgggcactgctggccgttggtttgctgtggccgcgtcggcgaacgttaaccattgctatcttgctggtctgggcaacgggagtcatgggaagccgcctgctgctcgggatgcattggccacgcgatctggtagtagctacgttgatttcgtgggcgctggtggcggtggcaacgtggcttgcgcaacgaatttgtgggccattaacaccacctgcggaagaaaatcgcgaaatagcgcaacgagaacaagaaagttaacgctggttgattttccgaatttagcccttaaatcatcaacaatgcgtgtggatgccatttcgcagacggcgcgaaaatggtactttaaagggctattgcggtaagttgaccataatttattcgctctaaccacataacgggaagtaatgtgaaatatttactcattttcttactggtgttagcgatcttcgtgatttcggtcacgttgggtgcgcagaacgatcaacaggtgacgtttaattatctgttagcgcaaggggagtaccgtatttccacattgctggcggtattgtttgctgcggggtttgctatcggttggttgatttgtggcctgttctggctgcgagttcgtgtttccctggcgcgcgctgaacgtaaaataaagcgactggaaaaccagctttcacccgcgactgacgtggctgtagtgccgcactcgtcagcggcgaaggaataactttctatgctggagttgttgtttctgcttttgcctgtagccgctgcctatggctggtatatgggccgcagaagtgcgcaacaaaacaagcaagatgaagccaaccgcttgtcgcgtgattacgtagcgggggttaacttcctgcttagtaatcaacaggataaagcggtagacctgtttctcgatatgcttaaagaggatacaggcaccgttgaagcccaccttacgctcggaaacctgttccgttcgcgtggcgaagttgatcgcgctattcgcatccatcagaccctaatggaaagcgcctcgctgacctatgaacagcgtctgttggcgattcaacaactggggcgtgattacatggccgccgggttatatgaccgcgcggaagacatgttcaatcagctgaccgatgaaactgacttccgcattggcgcgctgcaacagttgctacaaatctaccaggctaccagtgagtggcagaaagcaattgatgttgccgaacgcctggtgaagctgggtaaagataaacagcgcgtcgaaattgcccatttctactgtgagttagccctgcagcatatggccagcgacgatctcgatcgtgccatgaccttgctaaaaaaaggggcggcggcagataaaaacagcgcccgcgtatccataatgatgggacgcgtgtttatggcgaaaggagaatacgccaaagccgtcgaaagtctgcaacgcgtgatatcccaggacagagaactggtcagcgaaacgctggaaatgttgcaaacctgctatcagcagttgggtaaaactgccgaatgggcagaattcctgcagcgtgcggtggaagagaacaccggtgccgatgctgaattgatgcttgctgatatcatcgaagcgcgcgacggtagtgaggccgcacaggtctatattacgcgccagcttcagcgtcatccgaccatgcgtgtgttccataagttaatggattaccacttaaatgaagcggaagaagggcgtgccaaagagagcctgatggtgctgcgtgacatggttggcgagaaggtacgtagtaagcctcgttatcgttgccagaaatgtggttttaccgcatacaccctctactggcattgtccgtcttgtcgggcctggtcaaccattaaaccgattcgcggtcttgatggcctgtaatttttaaaaaaaatccgactttagttacaacatactaattattaatgttccattgtgctccggcaacgacggcgcagaaaaagcctgccaggggagaaatcgcaactgttaattttttatttccacgggtagaatgctcgccgtttacctgtttcgcgccacttccggtgcccatcatcaagaaggtctggtcatgacgttaactgcttcatcttcttcccgcgctgttacgaattctcctgtggttgttgcccttgattatcataatcgtgatgacgcgctggcctttgtcgacaagatcgacccacgcgattgtcgtctgaaggtcggcaaagagatgtttacattgtttgggccacagtttgtgcgcgaacttcaacagcgtggttttgatatctttcttgacctgaaattccacgatatccccaacactgcagcgcacgctgtcgctgctgcagctgacttaggcgtgtggatggtgaatgttcatgcctctggtggggcgcgtatgatgaccgcagcgcgtgaggcactggttccgtttggcaaagatgcaccgcttttgattgctgtgacagtgttgaccagcatggaagccagcgacctggtcgatcttggcatgacactgtcacctgcagattatgcagaacgtctggcggcactgacgcaaaaatgtggccttgatggtgtggtgtgttctgctcaggaagctgtgcgctttaaacaggtattcggtcaggagttcaaactggttacgccgggcattcgtccgcaggggagtgaagctggtgaccagcgccgcattatgacgccagaacaggcgttgtcggctggtgttgattatatggtgattggtcgcccggtaacgcaatcggtagatccagcgcagacgctgaaagcgatcaacgcctctttacagcggagtgcatgatgagtgattccaacagccgtctggtctactcaacggaaaccggacgtattgatgagcccaaagcggcccctgtacgccctaaaggcgacggtgtggtgcgtattcagcgtcagaccagtggacgtaaaggtaagggcgtttgcctgattaccggtgtcgatctcgatgatgccgaactgacaaaacttgcagcggaactgaagaaaaaatgcggctgcggcggagcagttaaagatggagttattgaaatccagggcgataagcgtgatttattaaaatcactacttgaagcgaaagggatgaaggtaaaactcgcaggcggttaacataaaaagccacggatatatccgtggctttcgaatattttactgtgcgtattattcagttatttcgtactgaacagaatcaagcgtattataattgcgagtcgataatcgacatttatttacgattatttaccgacctggtgaccaataacacctccgacagctgcaccacctaatgtacccaacgtactgccatcggtcagtactgcaccgcctaatgcccctgcacccgcgccgattgcggtgttgcggtcccgtttagaccagttagaacaggcactcagagacattgccaaagtaattgccagaacagccgcggtcatttttttgctcgttacaaacataatactctctcctgaatttatgattcacggaagtaagctctctataactataatagctaagaataagtctggtgaaattattccgtgaaatctgctcgcgcgcagggttatatcacgcaggtgataatgacttcctgttatatcgctgataataattttatatcttgagagtgttaataacaggtaaatagtcttaattatcaaccaggaatcatcttagagcggatgatttgccaaactgcaaatcatccgtagagaagggaaatggttaaatgtcaacgacgtgaatggtgagtttactgtgctcaagatgcatcagatcgctggcgcgtattttcgaatcggtaatcacgcgattgaatcgctcaacgggaccgatggagtatgaatgtacagcaccaaatttcgagctgtcagtcaggactatcgcttcgcactctttttccagcacggcattgaccacatcggtacgcatcatatcgcgaccggtaaatccagtttcaggttgccagccatcaataccaataaatgctttgctgaaatgcacctgttggatgcactggcgtgtcaaagggccaaccatactttcgctttttttctgatacacgccaccgagcaaaataacttcacaaggcgcgtctttcagcaaatgcgcgatgtagctgctgaccgtgatgatagtgacatttttcttctgctcgcccagagtccgggcgagtagggcattgctgctgccattttcgataaagatggtttcgcccggttgaaccagcgacgcggcaaactcggcgagttcacgcttcagcgtatagttgctcatcatacgggtttcgacgtcatcactatcaagcgaaacagcaaagccatgtgcacggcggaggtaactcagtttttcgagtgtgttgagatcctggcgaatggtaacttcagaaactccagtggcttttgccagatcggttacgctaacctgaccctggtcaatgaccatctgtagaatagtttgttgtcgggaattcatcgctgtaattcttataacgttataatacttaataaaaaaatactgacgcgccgggcatcctcaaataggaaaacctgaaggcacgattgttaaatctcccacggtgccttcgggatgtctggcgtagattcagcaacctggcgcaagagttctgctttaagtatctcgagattatggatcgcagagtggtaatcgcctgccacaaggatatctaacacaatatcaatacgttcggcaacgcgctgggcatcaaattcagacatcaaggacatccttatagcaaaagggggaaaatgaataatgcaaaaattgccgctaaaagagaagtgtttaacagcaacggctaattatcatccaggaatacgatatataatgacgggatatagcgctaagtatatatattcatctacttatgcgcgcttcagatagcgtttataccagcgttcgaaggcgacggcgggcatcggtttggcaaacaaaaatccttgccgctcattgatcccgttcttggttaaaaaagcatcttcctttgcactctctacaccttcggcgatcacctgaagattcaatgcctgggccacagcgacgatcgcccggaccagtgactgcgagacaggttgtttgtgaatatctcgaacaaaaacctggtcaagtttgatggcatcgatcggaaagcgcgccagttgcgaaagtgaagagtagccggtaccaaaatcatccagatgcacttgcgcacctagttggctaaattgttgaataacagacagtgccagttcatcattctcaatcagacaactctctgtcagttcaacatctatagggcagtattcaaaattgagttcctggagaacctgtttcagggcggtgaaaatggtttgatcggcgagctgacgtgcagaaatatttaccgccactcgcaggtttatgcctttatcccgccactttgccacctggcgtacgacatcgagaatcacccaacggcctaaaggcacaattagccctgactcttcggcgtaggaaatgaagtccaacggtggaatcaacccacgttcaggtgactgccaacgtactagtgcttccagactgcgcacttcgccacgccaggtgattttcggttgatagtgaataaccaactgatcgttttccagtgctttacgcaagttggtatccagccagagatattcaaatacccgttgattcatttctggggtaaaaacgcaaaattgtcctcgtccgccttccttcgctgtgtacattgctgtgtcggcgtgacgaataatagccgtgctgtctgaaccatgttcgggagagagtgcaatacctactgaacagctggtataaacttcaattaaaccaatgcgaaaggggagccgtaagcgggtcaaaattcgtgatgccattgcttccagcgcgctttgtgaggtgttggatgccagtaccagaaactcatccccacctggacgcgccaacacctggtcatgttcgagacagcttaaaatagccaatgacacgtcgcgtaataactggtcaccaaacaaatgcccataggcgtcgttgacctttttgaaattatccaaatcaagatacacaaccccaactttattgttatctgcatgattaatagcgtgatcgattaaatcctgcattgcgttacgattcggcagtccggtgatactgtcggtatttgccagaatacgcagtcgctcctgagcgcggcgctcttcggtaatgtcggtgccggaacagattaaaaaaatctcgtttttgccactgccgctgtggacaaatttattgcgaaacagaaacagccgctggcctttacatgttggtatccacagttcgacttcatatgcattgccgcttcgaaaaaatacacggttattgcgcctggatgccgcagcttcacgacggctcataaacagtttaaacacgctttgcccaatgacgtcgtgttctttcaaccctgtgtaatcttcacataaccgattgaagcgttggatattcccccggctgtcgagaatcactattgcggaatgtgcttcagaaactacctgctcagcaaaggaaagcccgtgtgataaatcacgagcaaccgccggtgtgtcatgccatgcagacgcgttgccagcccattcccgtttattgatttttcgtcctaccagatgcacagaaagatcgctttcatcgacggtcagactcatcatcaggctggaggtgatgaccgtcatttccctgatgcgagcagcctgttcggcagataactgcaatgtacgatcaggttctgtggtttcggtggtagaaaagcgcaaaacatcgctgctttccgtcaaccgccagtatggattgtgcgatccgagaaagttgtacaacgttgtggactccctaacggttttcatgatgcatatcctccggttaacagcggagtccgcggttaaataaaaggaacaacatgacttacatgaaattaacggcggctaaacgcattgttttttttatatatttatttgtaatccagttttggaaaaacgccagttttcaaacgaaagtcagttaaaaaatctgcctggatataacgaaggtagagcggggaaataaacggcccatccatgaggaatgggccgtgaaaggagattacgcgaccgggcgcgcaataatgctgcgggtttccatgcggacttcggcaatagtgacgtcaataacgtcagtcactttgtaaaccgtttcacctttaatttgtacagtgccgttttcctggctgcaaaccagttcatcgcgcacagcgtgtaagaaaggtgccggaataaaggcgatagcgccgttatcaaccaaacgaacacgcatgccgccacggctgatatcgacaatttccgctgcgaaacgggtgtcggtcccggctttgtctttcaggaagcgtgcgtataaccagtcaccaacatcacgttctgccatccggttgagacggcgacgctcggccatttggacagtgatttcatcctgtgggcgcgtcgcagtttcgcctttgataaccgctttcagcagacggtggttgatcatgtcgccatatttacggatcggcgaagtccaggtggcgtatgcttccagaccgaggccaaagtgaggaccgggttcagtgctaatttcagcaaatgactggaagcgacgaatgcggctgtcgaggaaaccagttggttgcgcgtccagttcacgacgcagtttgcagaaaccgtccagcgtgagcacttcttcggcatcgacatgcagaccgtgcgttttcagcaacgctgccagcgcgtcggcattcgccggatcaaagcccatatgcacgttatagatgccaaaaccgagcttatcgcgcagtacgcgggccgcacaaatgttagcggcaatcatcgcttcttcgacgatacggttggcaatgcgacgaggctcggcgacgatatccagcacttcacctttttcaccgagaataaagcggtaatccgggcgatctttaaacaccagtgcgtggttatgacgccactcgccgcggcgttggcaaatttgcgctagcaaacggacttgttcggcaattgcttcactttcaggctgccagtcaccggtattttccagccagtcagaaacctggtcatacaccagctttgctttggattcgatggtggcggcaaagaattcgatattatcttcaatggtgccatcagcggagagcgtcatgcggcatgccagtaccgggcggacttcattggcgcgcagtgagcagagatcgtcagaaagctcgcgaggcagcatagggatgttgaagccaggcagatagttggtgaatgcgcgaattttcgcggctttgtccagcttgctgccttcagcaatccacgcggttggatcggcaatcgccacaatcagctgaagtttgtcatccggcaacgccttagcgaaaagggcgtcatccatatcttctgtgctggcactgtcgatggtgacaaaatccagcgcggtcagatcttcacgaaccagaccttcatcgagcatttcggtagcgacgccgtctggtgcttctttttccagattatggcgtgcaagggtaacccaccacggtacaaagtgatcgtcaccaaaagtgatgtattgtgtcagttctgcatagaaagaacgatcgcctttcagcggatgacggcgcatttcggcaaccgcccagtcgccttctttaaactcgtggttcaggccacgggctgcgcggcaaggaatggcgtcttttaagagtggatgatcaggaacgatggccagacggtcatttttgccctgaaccttacccacgaaacgagtcaggaacggttcaaccagttcttctggctctgcggattcacgttctttttcactgtggatcaccgcgataattcggtcgccatgcatgacttttttcatctgcggcggcggaatgaaataacttttttgcgcgtcgacttccaggaagccaaagcctttttctgtggcttttaccaccccttcagcgcgtggcgtctgggaatgcagttgctgtttaagctgcgctagcagcgggttgtcctgaaacataattgtctattttggtggccattagagcggctgacagttttacgcgaatctgtctgacgcggcaaggttaatatgtctcacccaacgcgatttttaagcgatttatccagccacacagcccgctccataccagcagattaataatctgcgttgatgatttttcgtgttcgagtaaagggctgaactgggcggcgctaaagcgatcgggtgctcgggtcagccattgtatcgcctgaacggtagcgcgctcaacagaatgacggtcagcccattggttaatttcattttcgcccttgcgcataagggtgctgatttttttatattcatttgatgaatccatacaggtggcaaaacaagcaggactgccatttatacgcgcgcataacaacgccgcaagctgattatccggctgtgtattgccccgtgtgctgtttaacaacttttcgagaagggaaagtgaaatagggtggagagagagtatttcggccagttggcaaagttctgcagttgaactttttgtgtgctcttcaggtagtttttccacctcatagctgcttcgccagcgtaatgattcatcagcaaacagtgacgcgtcggcgtagttttgtatctccagcccgggtaaccagcgtaccggatgcccgagataagcctgaaatgtcgcaattgtccgcgcctgaaagccaataaaaccaatgatttggctaatgatcacacagtcccaggcagtaagaccgacgtcattcagatgctggcgcgatcggttgtcgataatagaaggcgagctagccagttggcgggcatattgcgtgatttgtgccaaccgatgattactttccctggtggaatcaggcccggggagcggcgtaagtcgcgccgaatagtagttacataaccgctggacgccgcaaacctgagcaaccgtcagggccgtcgacaagcgttcataagcggtgaaggtctgtgaacgggtcacggtaagctggtcagggaacaaatccactgcaagaacacgcgcagggtccagccatgaaaggaagggggccagcgtttctttttcaaggatcacgtcgagtagaaagggatcgctgacctttgcggcttccgggaccagaggcagaacgtcatactccgtagtactggattgcgtttcatgataccagtggcttttgccggtgatgtggcgttgttccatgggcgctccttggtcgtaaaggaaatcgttatcctgacgcaaggcgggaaggggagaaagacggatcggcgataacaaatatcagaaaggtataacagagataacgggcggcagaacgccgcccatctttaccaacagaacgattatttcagttcgagttcgttcattgcagcaatgctgaaaccgccgtcaacgtggaccacttcaccggagataccggcagagagatcggagcacaggaatgccgcagagttacccacatcttcaatagtaacggtacggcgaatcggggtaacggcttcgcaatgagccagcattttgcggaagtctttgataccggaggccgccagagtacggatcggaccagcagagatggcgttaacacgcacaccttccggacccatcgcgttcgccatatagcgcacgttcgcttccagagacgcttttgccagacccataacgttgtagttcgggatagcgcgctcagcgccaaggtaggaaagggtcagcagggcagaacccggattcagcatggagcggcaagcttttgccattgcaacgaagctgtaggagctgatgtcgtgggcaattttgaagccttcacgggtaacggcgttaacatagtcaccatccagctgatcgccaggtgcaaaaccaatagagtgtacgaaaccgtcaaatttcggccaaactttccccagttcagcgaacatggtgtcgatgctggcatcttctgcaacatcgcactgcagaacgatgtcagaacccaattgagcggcaaattcttctacgcggcctttcagtttgtcgttctggtaggtgaatgccagttcagctccttcgcggtgcatcgcctgagcgataccgtaggcgatggatagtttgctggcaacaccggttaccagaatgcgcttaccggaaagaaaacccatagctttaatccttattgttgatgcttgttgtgcctgaaaatcaggcgattcgtcgttttagtaaacagtacgaacagataaacggttattataatcaacctggctgtgagtagctatagttgccaggtccgaccggagcaggctgcggcagggggggcgcttttcccctcaccctaaccctctccccagaggggcgaggggaccgtattgtgcaaatattgttaccccagcaacaaacaggctcatacagcccctaaccctttcatggcgatggctgggacggttcagaccttgccgaatattctccagcaccgtctccatgttttcaccacaacagctattcggctcggtctgccccctcgctctttcagggagagggtgaccggcggttcagttcctgcagaatattctccagcaccgtctcctcattacaatcaatctcgttattccagaaacgcagcacggtccagccctgcgactcaagccagctagtgcgcctggaatcataggcaactgctaaatcatgctgcccaccatccagctcaacgactacacgcgccgagcagcaagcaaaatcgagaatgtagctccccactggatgttgacggcgaaatttgaaatcactaaaacgtcggctgcgaagatatcgccagagctttcgttcctgcaaagtgagattgcgtcttaaatcacgcgcatttgatttaattttatctatcacctcattctgacaagatttaatcttttgtcagaatgaggtgaataatctggaaggaggattcagaaaattagcgatctttacgccacgcatccgccgtcaatgcctcgccaaaatgaccggcaatcagccgtttggtgagttcatgcagcggcgatgccagcacatccgcggtgctgcctcgctcgacaacctcgccctgatgcatcaccagcacctggtcgctaatgtgcttcatcattccgatatgctgggtaacataaatatacgaaatgccctgtttttcctgtaattccagcatcagattaatcaactgcgaacgcatcgacatatccagtgaagcgagggcttcatcggcaataatgacttttgggcgcaatatcagcgcgcgcgccagacccagacgctgtttttgtccgggtgccaacatatgcggatagtaactgacgtgatccggtagcagcccaaccatacgcatcgtttcaataatctgtttgcgacgctgttccggttccaggtcggtgttcaggcgcagtggaaaatccagaatttgcgagatacgttgacggggattcaacgaggtcgaaggatcctgaaaaatcatgcgaatacgctgactgcggaaggaataatcgccaaaatgcagtggatgatcgtcaatcaataactcgccgctggtaggctctatcattcccgccagcatttttgccagcgtggatttacccgaaccattctcgccaataatcgccagtgtctggccttcacgtagcgtaaagctcaagggttttaccgcttctacggtctgacgacgaaaccagccggtccggtagcggaacgttttacttaaattacgcacttcaagcagcgtttcgatcatctcactctttctccatgttcagcgggaaatgacaggcatagagatgatttttcgcccccgtcaaacgtggcgtcacaatgcattctcgttgtgcatacgggcaacgtggccccagacgacaaccaatcggtaactgttccagcagtgggatagcgccgggcagcgtattgaggcgacttttatgcggcatcgcgctgccgaagtctggtatcgcgcggatcagcgcctgggtataaggatgatgtggcatcgtcaccaactccttactcggcgcggtttccactgtttgaccgcagtaaagcacgttaattttatccgcccattggctaagcatttgtaagtcatggctgataagcaaaatagtggtattgctgttttggttgagacgcgtcagcaggcgaaagatttgcgcctgggttgttggctccattgagttggtcggttcgtcagcaatcagcagacgcggttgattcgccagtgcaatggctatcatcactttctgacattcaccttcggtcaactcatagggaaaactgcgcatcgcatctttgtgatctttaatccccacgcggtgcagcagttcaatggcacggcgtttgcgccagccaaaacgctgccaccaacggcctttataggtccaggctgggatgttttgcatcaactggcggcccacacgttctgaagggtcaagacacgactgcggttcctggaaaatcatcgacacgttatggccaaccagtttgcgccgttcgcgtgcggagagacgcagcaaatcgatatcatcaaaacgcatacggtcagcagtaacacgccagttatctttattcaccccacaaatcgctttcgcaatcaaactcttgccggaaccggattcaccaacaagaccgcggatttcaccttcggttaaggtcatacttacccggtcgacggctttaacccactcatcaccggttttaaattcaatggtcaggttacgaatatcgagtaatggcattattccacccccgcaataatcgcacgacgaacgccatcgccaaggaggttaaccaacaacacgctaatcataattgccgcacctggcagcatgacagtccacggggcgacataaatcagttccagcgcatcaccgagcatcgctccccattcaggcgaggggagttgtgcgccgagatcgagaaagcccagcgcggcgatatcgagaattgccatcgacagtgcgcgggtgatctcggtgaccagcccggcggtgatgtttggcatcacagcaaaccagagaatattcagcgttgatgcgccatccagacgggcggcgataacgtactctttttccagttcgtcatgcaccatgctgtaaatcgaacgtaccatacgcggcagcaatgccagccagacagcaaacatagcgtgggacaaactcggtccggcaaacgctacaacgataattgccaacagcagcgaagggatcgccagtaaggtatccagaatatggttaagcaccgctgagcggaggccgtgtgtcgccccggcgaaggtgcccagtaccaggccacagatcgtcgcggcaagcgtcaccacaaatgcgccacccacggttggcgcagctccgctcagtaaacggcttaaaacatcgcgtccgaggtcgtcagtccccaggaagaaagaaacttcgccatagcgcgaccatgacggcggcaataattgataaccgagaaattgctggtcgatgccgtaaggcgcaaaccagccgccaaaaatacacagtacagccagccccgcgcagccgtacaggccgaccatcgcagaggcgtcactataaaatttgcgccaggcggtacgcagcgtgcccggcgggcgcttttcgctgtatacgctatcgtaaggcataccattccttatgtttcagagggttagccatggcacccaaaatatcagaaatcacgttaacaataatgaccagtgagccacacaccatcactccggcggaaatggctgcgtaatcctgctggcggatggcgttaattaaccagcgccctaaacccggccagctaaaaaccatttcggtgatcatcgccagcgtcagcatggtggaaaactgtaagcccaggcgaggaataaccggcggtaacgcgttatgcagaacgtggcgacgcaaaatagtaaagcgcgacaaaccgcgggtcgccgccgcttttacatagttctggtcatacacttcgatagtgctgatacgcatcaggcggatcacttcagttgttggcgcaaccgacagggtgatcacgggcaatatcatatggcggattgcgctcatgatcatttcatcccgccatggtgagtccgaaagccaggcatcaatcaacgcaaaaccggtaatcggtttcacttcgtagagcagatcgaaacgccctgaaacgggcaaccaacctagcgtgagtgaacaaaacagcgtcaacagaagcgccagccagaacaccgggattgaaaagcccagtaaggcgatggcgttgatcaagttatcctgccacttatggcgcgtaatcccggcaatcatccccacggggatgccaacaatcagcgcaaaaccgaaggcgaggatgcacagttccatcgtcgccgggaagacctcttttaactgttcggcaatcggttgaccgttaatgctggaaacaccaaaatcccagtggatcaggccgttaaaccagaacacccaggcattccacagtgacgcgccttgtaacggcgcatgaggggtgaaatagctcaagctgaagccaacgaaggtcagcaggaacaaggtgacaatcaataacaaaatgcggcgtaaggtgaagataatcatggttttttcacctcatcctgtttctcgcgatacaccccagcaaaggaggcgttaccaaacgggctaagtaccagacctttgatatcgtaccgataggcctgcaaacgcaatgacgacgccagcggcaaaatgggcaattcctgcgccagaatactctgcgcttcgtcataggcttcaatacgcgccgccagctgctgcgaagagagcgccttacgcaatacgctgtcgaatttcggatcgcaccagtgggcgaggttggtctgcgaatgaattgccgcgcagctcagtaacggacggaagaaactgtccgggtcgttactgtccgtcgcccaaccggataacgtcagatcatggctcatatccatcaaccgcgcctcctgaaagcgaccttctaccggcacaatcaccacttttacgccaacctgcgccatatccgcctgaatcagttcggcagttttcagtggactggggttccacgcctgcgaacgtgtgggcacccacagtttcagcgttaaattttccagccccaacgacttcaactgttcgcgcgatttcgccggattgtattcagtaattttagcctcgttgtcataggcccacgaggcgcgcggtaaaatagaggccgccgtttcagccgtaccataatagatggattgcatcaggcgctggttattaatcgccagtgccagcgcatggcggacagcgggattatttagcggcggtttggcggtgttaaatgccagataggcgacgttcatcccaggacgcagcgttaaacgcaagcgcgggtcgtcacgcaaaatggatagctggctggcagcaggccaggccagaacgtcgcattccccggtcaggagtttcgacagacgtccggtgccgccggagcctaaatccaccactacctgcggcattaacggtttaccgcgccagaagtcatcatgacgttgtaggcgaataaattgcccggcgcggtattccgacaactgatacggaccggtgccgaccggttgacggtcgagttgctcctggcgatcttctttctctaacttccgggcatattctgccgacatgaccgaagcataatgggttgcgaggtgccacaaaaaagaagcatccggctgggcgagtcggaactcaacggtatgattatccagtttgcggacgcttttcacgttatcggcaaattgcaggctgtcgaagtaggggaagttgctgccgttgacgttatgccacgggttgttgcggtcaaaaattcgctggaaggtaaacaccacatcgtcggcattcattttacgagtgggagtaaaccagtcggttttttgaaacggaacatcgcgacgcaggtggaagcgataggtcgcgccgttgtcgagtacttcccagctttcggcaagttccggcatcaggcgataggtatagggatcgacatccagcagtcgatcataaaactgggcggcaagggtatcgacaattaacccactgctcgctttggatgggttaaaggtgttgacttgcccgctgacgcaatagacaaaaccgctgtcgcggatatcagcatgcgggggagattcaggcgcggcgattgcctgaccactcacaagtccagcaatcaccaaaagagacgataatacctggcgcataatattaagggattttatgtaaagaggctatcttactaatatttaatgacatttgccattaccgtttgtgttcaggggtcgtaatgagggccgtgtggttggtcgttgaacaggtgacgtcgccatctgttcaacattcgtacccgtgatttctctataactataactcacagaacaacttagcgaggagcagagcggtacgatcgtgagaaacccattaaagcacgctgcagtgcgtgtcattgttagccagatgcggcgtgaacgctttatccggacaacgatactgaccgatcgtctgcaattaaatcattactcattaccccattgattcaaaaactctgcgatctcatcaatgcgtacgggattaatccccgcttcagcagccatttcatgttgggcttcttcgctgatctcttcattgttcatcaaacgggtgagcagtaactggaagtagtgggccagcggtgtgcgttcagcctctgcgacaggctctgcgcattcggtcgcgtactcatcggcaatatcaaaatattttagcgggatatcgtggttcattatttgcccctggggttaatgcgctaagcataagggcggatgatagcactcgtgatccgggtcatacatctttttatagttaatggcgcggcgcgttaccctcaggcaggataatgcgccgcgcatccgactattacgtttcactcaccggcgttctgtcaccatcatacaacggcactttgcgatagcggcggatcagataccataaatatgcgccgcctaacgaagcccataccagaccgagtgtcagtgacgttgactcgaggttaacccacagcacacccaccgtcagcgcgccaaccagcggcatcagcaaatagtggaagtgatccttccagcttttattcattcctttacgccgccagaaatgattaaacaccgacagattcacgaaggtaaacgccaccagagcaccgaagttaattaacgctgtggcggtaactaaatcgaagaacagcgccgacaacgcgacaatcccgaccataatgacgttgagtgccggagtccgccattttgggtgcacatagccaaacacgcgctccggaaacacattgtcacgccccatcacatacagcagacgcgacacgctggcatgtgaagccaggccagaggctaacgtgttcacaaacgtggtgcagaggaaaatcgactggaagagcttgccgccgacgtacagcgcaatttcaggcagtgcggcatccggatctttaaagcggctgatatcgggaaagaacagctgcataaagaacgacgccgcgataaagataacgccaccgtagaccgccgtcaggaagatggctttcgggatcacgcgtgcggcgtccggcgtctcttccgaaagcgtggtcaccgcatcgaaaccgaggaaggagaaacagacaatcgtcgccccggtaataatcgggatcaggtgcgcgttctcgctgataaacggctgaagtgaccagacggtgccaacgccttctcctttatgcagtccctgaactaccaggaagataaacaccaccatgatggagatttgcaccagtacaaacagggtattgaagttagcgaccaggttgacgctcttcagattcgcggcggttaaaatggcgacgaaggttaccacccacacccacggcggcacttccgggaagagggcggagagatagattttcgccaacaagacgttaatcatcggcaaaaagagataatccagcagcgatgaccagccgaccataaatccgacgtgcgggttaatcgacttttgcgcgtaggtataggccgaaccggcctccggaaactggcgaaccagtttgccgtagctgatagcggtaaacagcacacccgccagcgccagcaaataggacgccggaacgtgaccgtcgctaatgccggagacaataccaaaagtatcaaatacggtcatcggcgtgagataggccagacccatcatcaccacctgccacaatttcagtgattttcgcagacgggttttgccgggttgcgcagcaatattcagtggtgaattaatagccataattgctgcctcccctgcgtaataaggtttgcggtcgtgtcgacctgaaatcaaacctgtttagcaagggaagcaaagggggcggagtccagtcagtagcaggaggggcgcatacgcagcctccctcgccatgcggggatttaatcatcggcatcatctcatttcctcgtcacagtcttaatcgttaacggaagcccgttgccgcccgcgctccataacgcgacatccgggaaatgtctggattaccagcaaatgtcaggcctggctccgctcaggccgatgaaacaaccccgcaaggggtattacgcgtttttcaacatccactcaatttctgtttctgtgatgaggcgctcaaactgcaacagctcatcatttttacaggcgtgatagacatggcagaagcgttcgcctaaatagcggcgcaggtgatcattctcgataaactcacccagggcatcgctctggcgaatcggaaagggtaagccttcctgttccagcccgttgccttcgacttcttcctgcaacggcagctcgttatcaaggccatgcaaaataccggcaaaaatcgctgccatcaccagatatgggttggcatcggcacccgccacgcgatattccacgcggtgattatgacggtcgccgcacggaatacgcagggcgacggtgcggttgttatggccccacgacgcctgcgtcggcacatacattcccggctggaagcggcgatacgagttcacgtttggtgccagcaacgccatcgacgacggcatcaggtcaatcatcccggcgagcatctttttcagcagcggcgaatcttcgccttccgcgtcagaaagcacgttctcgccacgattattttgcatactgatatggatatgcattccgctgcccgcgtgctcttcatacggcttcgccataaaagtggcgtgcatcttatgcttttctgccatcagacgcaccaggcgttttagtgccagcgcatcatcgcaggcttccagcacgttatcagtatggtaaaggttgatttcaaactgacccggcgaggcctcagcgaccgcgccatctgccggaatcagctgtaactgcgccagttcatcaatatcattgagcacgtcggcgaagtggttgaggttatcaacggagtaaacctggctttgtgtattgcggtcatcggtgccaggcgcgcagggcggttgcagatacccttcagcgtcgcgctggcgatccagtaaatagaactccagctctaccgctacgaccgggaacaatccgcgctggcgcagctgctgccacaggcggttaagaacgttccgcggctcaacgtcaaagggagcgccatcttcatcgaccatggtcaggagcatctgaccgataaactctggatcggcggcagaaggagttaaggaaccgagaacaggaacacaggtacgatccggctcgcccatttcctgacccagacctgcttcttctactacgttgcccagaatatccattgcaaataccgaggccgggaaataacaccctttctcgagcttcttcaggcttgaaacaggaatacgctttccacggaagcaaccatttaaatcggtaagtaaaacatcaacatattgcgtattcgggtagcgctccaggtagcgtttcacttcctgcgtaaaggcgctaccccgcctctcttctgactgctgaacaaagttctctacttcaacgatattggtttccatgattcttcgcctttggtttgttttccgctcgttatcaaagcgtaaaatataatgaccaccattcgaatctgtatgcaaactaaatgtttgtcaaatgttaaattgagtttgcaaaaatgaaaacccactgctagattgaaaaaatattgaacataaaggtcatttaaagcgcagtaatggcgataatttagtccactttgtgagattgagcatggaaaatataatgaacaatccggttatcggtgtcgtaatgtgcaggaacaggcttaagggtcatgcgacccagactctgcaagaaaagtacctgaatgccatcatccatgcaggcggcttgcctattgcgctaccacatgcgctggcggaaccgtcattacttgaacaacttttgccgaaactcgatggcatttatcttcctggtagtcccagcaatgtgcagccgcacctatatggtgaaaacggcgatgagcctgacgccgatcccgggcgtgatcttctgagcatggcgataattaatgccgcactcgaaaggcgcatccccattttcgccatctgccggggtttacaagaactggtggtggcaaccggtggttcgttgcatcgcaagctgtgcgaacagcctgaattgctggaacatcgggaagatcccgaactgccggtggaacagcaatatgcaccgtcgcatgaagttcaggttgaagaggggggattactgtctgcgttgttacctgaatgtagcaacttttgggtaaactctctacatggacaaggggcgaaggtcgttagcccacggttgcgtgttgaagctcgctcgccggatggcttagttgaggcggttagcgtcatcaatcatccttttgcgctgggcgtacagtggcacccggaatggaacagtagcgagtacgcgctttcgcgtatattgttcgagggctttatcaccgcttgtcagcaccatatcgctgaaaaacagcgactctgaccactacagtttaaggaaatgcaaatatgagtgatgagggactggcgccaggaaaacgcttgtcggaaatccgccagcagcaggggctttcacaacgtcgtgccgccgaactctccgggctgactcacagtgctatcagtacgatagaacaagataaagtcagccctgccatcagtacgctgcaaaagctgctgaaggtgtatggtctgtcactctcggaattcttttccgagccggaaaaacctgatgagccgcaggtcgtcattaatcaggacgacttaattgagatgggtagtcagggtgtgtcaatgaagctggttcataacggtaacccgaatcgcacgctggcgatgatctttgaaacgtaccagccgggcacaaccactggggaaagaattaagcatcagggtgaggaaataggcactgtactggaaggtgaaattgttctgacgattaatggtcaggattaccacctcgtcgcggggcaaagttatgccattaataccggcatcccgcacagtttcagtaatacgtcggcaggtatttgccgaattatcagcgcccatacgcccaccacgttttaatctttttgttctgtaagccgggtaagcgcaatgcgcccggcaatctatacacaaaatcattcaagttgcatcaaggcggcaagtgagcgaatcccgatgagcttactcaggtaagtgattcgggggagcgaacgcagccaaggcagaggcggcttgaaggatgaagtgtatataaagaatgtcgccagaaataaacgggcatacggcccggggatctctgcgccctgacgttcacaaactgcatatatctgatagacgtgaaacaggagtcataatgaattttcatcatctggcttactggcaggataaagcgttaagtctcgccattgaaaaccgcttatttattaacggtgaatatactgctgcggcggaaaatgaaacctttgaaaccgttgatccggtcacccaggcaccgctggcgaaaattgcccgcggcaagagcgtcgatatcgaccgtgcgatgagcgcagcacgcggcgtatttgaacgcggcgactggtcactctcttctccggctaaacgtaaagcggtactgaataaactcgccgatttaatggaagcccacgccgaagagctggcactgctggaaactctcgacaccggcaaaccgattcgtcacagtctgcgtgatgatattcccggcgcggcgcgcgccattcgctggtacgccgaagcgatcgacaaagtgtatggcgaagtggcgaccaccagtagccatgagctggcgatgatcgtgcgtgaaccggtcggcgtgattgccgccatcgtgccgtggaacttcccgctgttgctgacttgctggaaactcggcccggcgctggcggcgggaaacagcgtgattctaaaaccgtctgaaaaatcaccgctcagtgcgattcgtctcgcggggctggcgaaagaagcaggcttgccggatggtgtgttgaacgtggtgacgggttttggtcatgaagccgggcaggcgctgtcgcgtcataacgatatcgacgccattgcctttaccggttcaacccgtaccgggaaacagctgctgaaagatgcgggcgacagcaacatgaaacgcgtctggctggaagcgggcggcaaaagcgccaacatcgttttcgctgactgcccggatttgcaacaggcggcaagcgccaccgcagcaggcattttctacaaccagggacaggtgtgcatcgccggaacgcgcctgttgctggaagagagcatcgccgatgaattcttagccctgttaaaacagcaggcgcaaaactggcagccgggccatccacttgatcccgcaaccaccatgggcaccttaatcgactgcgcccacgccgactcggtccatagctttattcgggaaggcgaaagcaaagggcaactgttgttggatggccgtaacgccgggctggctgccgccatcggcccgaccatctttgtggatgtggacccgaatgcgtccttaagtcgcgaagagattttcggtccggtgctggtggtcacgcgtttcacatcagaagaacaggcgctacagcttgccaacgacagccagtacggccttggcgcggcggtatggacgcgcgacctctcccgcgcgcaccgcatgagccgacgcctgaaagccggttccgtcttcgtcaataactacaacgacggcgatatgaccgtgccgtttggcggctataagcagagcggcaacggtcgcgacaaatccctgcatgcccttgaaaaattcactgaactgaaaaccatctggataagcctggaggcctgaaatgaccgaacataccagcagttactacgccgccagtgcgaataaatatgcaccattcgacacgctgaatgagtcaatcacctgcgacgtttgcgtggttggcggcggctataccgggctctcctccgcgctgcatctggcggaagcgggctttgacgtagtggttctcgaagcctcacgcatcggctttggcgcaagcgggcgcaatggcggacagcttgtgaactcctacagccgcgacatcgacgtgatcgaaaaaagctacggcatggacaccgcccgtatgctcggcagcatgatgttcgaaggtggtgagatcatccgcgaacgtatcaaacgttatcagattgactgcgactaccgccccggcggcctgtttgtggcgatgaatgataaacagctcgccacacttgaagagcagaaagagaactgggaacgctacggcaataaacagctggaattgctggacgccaacgccattcgccgtgaagtagccagcgatcgctataccggtgcgctgctggatcacagcggtgggcatattcatccgctaaaccttgccattggcgaagcggacgccatccgcctcaacggcgggcgcgtgtatgaactttctgccgtgacgcagatccagcacaccacgccagccgttgtgcgaactgccaaaggtcaggtgacggcgaagtatgtgattgtcgccgggaatgcgtatctgggcgataaagtagagccggaactggcgaaacgcagcatgccgtgcggcacgcaggtgatcaccaccgaacggctgtcggaagatttagcccgttcgctgatcccgaaaaactactgtgtggaagactgtaactatctgcttgattactaccgtcttaccgccgacaaccgcctgctgtacggcggcggcgtggtctacggcgcgcgcgacccggatgacgttgagcgccttgtggtgccgaaactgctgaaaaccttcccgcagctgaagggcgtgaaaattgattaccgctggacgggcaacttcctgctgaccctgtcgcgtatgccgcagtttggtcgcctcgataccaacatctattacatgcagggctacagcggccacggcgtgacctgtactcatctagccggacgtttgattgccgaactgctgcgcggcgacgccgaacgtttcgatgccttcgccaatctgccgcattacccgttccccggcgggcgcacgctgcgtgtgccgtttaccgcgatgggcgcggcgtattacagcctgcgcgatcgtctgggcgtttaatttccgattaaccgtgaagagtcaaaaggtgtgaaacatgagcaacaatgaattccatcagcgtcgtctttctgccactccgcgcggggttggcgtgatgtgtaacttcttcgcccagtcggctgaaaacgccacgctgaaggatgttgagggcaacgagtacatcgatttcgccgcaggcattgcggtgctgaataccggacatcgccaccctgatctggtcgcggcggtggagcagcaactgcaacagtttacccacaccgcgtatcagattgtgccgtatgaaagctacgtcaccctggcggagaaaatcaacgcccttgccccggtgagcgggcaggccaaaaccgcgttcttcaccaccggtgcggaagcggtggaaaacgcggtgaaaattgctcgcgcccataccggacgccctggcgtgattgcgtttagcggcggctttcacggtcgtacgtatatgaccatggcgctgaccggaaaagttgcgccgtacaaaatcggcttcggcccgttccctggttcggtgtatcacgtaccttatccgtcagatttacacggcatttcaacacaggactccctcgacgccatcgaacgcttgtttaaatcagacatcgaagcgaagcaggtggcggcgattattttcgaaccggtgcagggcgagggcggtttcaacgttgcgccaaaagagctggttgccgctattcgccgcctgtgcgacgagcacggtattgtgatgattgctgatgaagtgcaaagcggctttgcgcgtaccggtaagctgtttgccatggatcattacgccgataagccggatttaatgacgatggcgaaaagcctcgcgggcgggatgccgctttcgggcgtggtcggtaacgcgaatattatggacgcacccgcgccgggcgggcttggcggcacctacgccggtaacccgctggcggtggctgccgcgcacgcggtgctcaacattatcgacaaagaatcactctgcgaacgcgcgaatcaactgggccagcgtctcaaaaacacgttgattgatgccaaagaaagcgttccggccattgctgcggtacgcggcctggggtcgatgattgcggtagagtttaacgatccgcaaacgggcgagccgtcagcggcgattgcacagaaaatccagcaacgcgcgctggcgcaggggctgctcctgctgacctgtggcgcatacggcaacgtgattcgcttcctgtatccgctgaccatcccggatgcgcaattcgatgcggcaatgaaaattttgcaggatgcgctgagcgattaatagcccaacgcaataatgtctgatgcgctgcgcttatcaggcctgcaaacgacgtattgattatgtatgccgaataaagcattcacgccgcatccggcaagttgtattgctcaacttcgctaaatctggtgctttttcaacaacgcgcggaactgatgataagttaaccccagtaattcagccgcgcgcttctggttatatttcccttgttgcaaactgagttgcagcaactctttttcctgctgcatctgaaactcacgtaaatccagcggcagtgttggaagcgaggtggtttctgaaacggcgatagcgtcttcaggcggacgccgtttaaagggatcaataatgatgtcatcaagcggataatcgctggtgccgtggcgatacactgaacgttccaccacgtttttcaattcacgaatatttcccggccaacgataattcagcaatgtttctctggcgcgctccgtaaaccccgggaacagaggcagcttgatttcccgacacatctggatggcaaagtattctgccatcaacattatgtcgctttcgcgctcgcgcagtggtggcagttgtacaacatcaaaagccagtcggtcgagcaggtcagcgcgaaaagtgccttcattgaccatcgccgggagatcggcattcgtcgcgcataccaaccgcacattcacctgcaatggttggctgccgccaacgcgctccagttcaccgtactcaatcacgcgcaataatttctcctgcaccatcatcggtgccgtagcgagttcatcaagaaatagcgtaccgccgtcggcacgttcaaatctccctggatgacgtttttgcgcaccggtaaacgcccccgcttcgtgaccaaacagttcggaatccagcagattttcatttaacgccgcgcagttaagggaaataaacggcccttgccaacgggaggagagataatgcaggcggctggcaatcagctctttaccggtgccgcgttcgccgatgatgagcaccggtttgtccagcggtgcgagatgcgaaacctgttccagcacttcgagaaagctgttcgcctcaccaagtaaattatctttgtattctgccatgatgaaattcgccacttgttagtgtaattcgctaactcatcctggcatgttgctgttgattcttcaatcagatctttataaatcaaaaagataaaaaattggcacgcaaattgtattaacagttcagcaggacaatcctgaacgcagaaatcaagaggacaacattatgggtattttttctcgctttgccgacatcgtgaatgccaacatcaacgctctgttagagaaagcggaagatccacagaaactggttcgtctgatgatccaggagatggaagatacactggttgaagtacgttctacttcggcgcgcgcgttggcagaaaagaaacagctgactcgccgtattgaacaagcgtcggcgcgtgaggttgaatggcaggaaaaagccgaactggcgctgctgaaagagagagaggatctggcacgtgcagcgttaattgaaaaacagaaactgaccgatctgattaagtccctggaacatgaagtgacgctggtggacgatacgctggcacgcatgaagaaagagattggcgagctggaaaacaaattgagcgaaacacgcgctcgccagcaggcattgatgttacgtcatcaggcggcaaactcgtcgcgcgatgtgcgtcgtcagctggacagtggcaaactggatgaagcaatggctcgtttcgaatctttcgaacgtcgtattgaccagatggaagcggaagcagaaagccacagcttcggtaaacaaaaatcgctggacgatcagtttgccgaactgaaagccgatgatgcaatcagcgaacaactggcacaattaaaagccaaaatgaagcaagacaatcaataataacatccaggcggcgtccgaacgcgccgccgctcatcgtctaaggagtacttatgagcgcgctatttctggctattccgttaaccatttttgtgctgtttgttttaccgatctggttatggctgcattacagcaatcgttctggtcgcagtgaattgtcgcaaagtgagcagcagcgattagcgcaactggctgatgaagcaaaacggatgcgcgaacgtattcaggcgctggaatctattcttgatgcagaacatccgaactggagggatcgctaatggcgggcattaatctcaataaaaaattatggcgtattccacagcagggcatggtccgcggcgtctgcgccgggattgccaactattttgatgtaccggtaaaactggtgcgtatcctggtggtgctgtcgattttcttcggtctggcgctgtttaccctggttgcttacatcattttgtcatttgcgcttgatccaatgccggacaacatggcctttggtgagcagctaccttccagcagcgaattgctggatgaagtcgaccgtgaactggcggcaagtgaaacgcgtttacgcgagatggaacgttatgtcacttccgatactttcacgttacgtagccgtttccgtcaactgtgaggaaagttatgaatactcgctggcaacaggccgggcaaaaggtaaagcctggtttcaaattagcaggcaagctggtacttcttaccgcactgcgctatggcccggcgggtgtggcgggctgggcgataaaatcagttgctcgccgaccgctgaaaatgttgctggctgtggcgctggaaccgctgttaagtcgggctgctaataaactggcacagcgttataaaaggtgaggggagtttcgcaaaaattgttaaatctcaggcgtataatggatggcaattttcatccatagaaggacgcttacatgtttaaaaaaggcttacttgctctggcactggtgttttcactgcccgttttcgccgctgaacactggatcgatgttcgtgttccagagcagtatcagcaagagcacgttcagggggccatcaatattcccctgaaggaagtgaaagagcgcattgccaccgccgttccggataaaaacgacaccgtgaaagtgtattgcaatgccggacgccagtcagggcaagcaaaagagatccttagcgagatgggatatacccacgttgagaacgccggtggcctgaaagacatcgcaatgccgaaggtcaaaggttaaaagaattcaccatgagcggcgcttatgcgccgtttttttttctgtcacaccttatttacatccccatagattatttgcgtcagctcacaaatacgctttttccctggtaaaaaatgatttcctgcgtgactaaaacccttgtgctcaattgacagtttattttctgcggagtagtctctcgtttcatgggaccgctaccacggaaaggcaacatgaaacagaaaattacggattacctggacgaaatctacggtggaacatttaccgcaactcatttacagaaacttgtaacgcgtcttgagagtgcgaaacgattaattacacagcgacgtaaaaaacactgggatgaaagtgatgtcgtgttaattacctatgccgatcaatttcacagcaatgatttaaaaccattacccacatttaatcagttttaccatcaatggctgcaaagcattttttcacatgttcatttgttgccgttttatccatggtcatctgatgatggcttttcggtaattgattatcatcaggtcgccagtgaagcgggggagtggcaggatattcagcaactcggtgaatgcagtcatttaatgtttgattttgtctgcaaccatatgtcggcaaaaagtgaatggtttaaaaactatttacaacagcatccaggttttgaagatttttttattgccgttgacccgcaaaccgatctcagcgccgtcactcgcccgcgtgcgttaccgttattaacgccattccagatgcgcgatcattcaacgcgccatttatggaccacctttagtgacgatcaaattgacctgaattaccgtagccctgaagtgttgctggcgatggtggatgttttactctgttaccttgcgaaaggtgctgagtatgtccgcctggatgccgttggctttatgtggaaagagccgggaacaagctgcatccatctggaaaaaacacatctgattatcaaactgttacggtcgattattgataacgttgcgccaggtacagtgatcattaccgagaccaatgttccgcataaagacaacattgcttactttggcgcaggcgatgacgaagcacatatggtgtaccagttctcgctgccgccactggtgctgcatgcggtgcaaaaacagaacgttgaggcgctttgtgcgtgggcgcaaaacctgacactaccttccagcaacaccacctggtttaacttcctcgcctctcacgatggcatcgggctaaacccgctacggggcttgttgcctgaaagcgaaatattagagctggtcgaggcgttacagcaggaaggtgcattagtaaactggaaaaataatcccgacggtacacgcagtccgtatgaaataaatgtgacctatatggatgcgttaagccgccgtgagagtagcgatgaagaacgttgcgccaggtttatccttgcccatgcgattttgttaagtttccccggtgtgccagcgatatatattcaaagtattcttggctcgcgtaatgattacgcaggtgtcgaaaaactcggatataaccgtgcgattaaccgtaaaaaatatcacagtaaagagataacccgagaactgaacgatgaagctacattaaggcatgcggtatatcatgagttgtcgcgtttaattacacttcgtcgcagccataacgagtttcatccggataataattttaccattgatacgattaattcatccgtaatgcgtattccaagaagtaacgctgatggtaattgtctgactggattgtttaatgtcagtaaaaatattcagcatgtaaatattactaatctgcatggtcgggatctgattagtgaagttgatatattgggtaatgaaataacgctgcgcccctggcaggttatgtggattaaataaaaaggaacatctcatgattaaatcaaaaatcgtgctgttatcagcactggtttcatgcgccctgatttcaggctgtaaagaagaaaataaaacgaatgtatccatcgaatttatgcattcttcggtggagcaggagcgccaggccgttatcagtaaattgattgcccgttttgaaaaagaaaaccctggcatcaccgttaagcaagtgcccgtggaagaagatgcctataacactaaagtcattactctttcacgtagcggttcgctgccggaagtgatcgaaaccagccatgactacgccaaagtgatggacaaagagcagcttatcgatcgcaaagcggttgccacagtcatcagcaacgttggtgaaggcgcgttttacgatggcgtactgcgtattgtgcgtaccgaagatggtagcgcatggaccggtgttcctgtcagcgcctggattggcggtatctggtatcgcaaagatgtgctggcaaaagcggggcttgaggagccgaaaaactggcaacagctgctggacgttgcacagaaactgaatgacccggcgaataaaaaatacggcattgcgctgcctacagcagaaagcgtgttgacggaacaatccttctcccagtttgcgttatccaaccaggctaacgtctttaacgccgaaggcaaaatcacccttgatacaccagagatgatgcaggcactgacctattaccgcgaccttactgccaacactatgccgggttctaacgacatcatggaagtgaaagacgcctttatgaacggcaccgcgccgatggcgatttactccacctatatccttccggctgtgattaaagaaggcgacccgaaaaacgtcggtttcgtggtgccaaccgagaaaaactctgcggtctacggcatgttgacctcgctgaccattaccgccgggcaaaagaccgaagagacggaagcagcagaaaaatttgtcacctttatggagcaggcagacaacattgccgactgggtgatgatgtcgccaggtgctgcgctgccggtgaataaagcggtggtgactaccgccacctggaaagacaacgacgttattaaggcgctgggtgaactaccgaatcagctaatcggtgaactgccaaatattcaggtttttggcgcagtaggggataaaaactttacccgcatgggtgatgtgacgggttctggcgtggtgagttcaatggtgcataacgtcaccgtgggtaaagccgatctctctactacgctgcaagcgagccagaaaaaactggatgaactgatcgaacagcactaaacccaggacaggaatccgcaatgaacaggcttttttcaggtcgttccgatatgccctttgcgctgctgcttctcgcgcccagcttattactgctgggcggtctggtggcgtggccgatggtgtcgaatatcgaaatcagttttttacgtctgccgctcaatcccaacatcgagtcaacgtttgttggggtgagcaactatgtgcgtatcctctccgatcccggcttctggcattcgctgtggatgacggtctggtataccgcgctggtggtggcgggcagcaccgtgctcgggctggcggtggcgatgtttttcaaccgcgagttccgcctgcgcaaaaccgcgcgttcgctggtgatcctctcctacgtaacgccgtccatttcgctggtgttcgcctggaaatacatgttcaacaacggctacggcattgttaactacctcggcgtcgatcttctgcatctctatgagcaggcaccgctgtggttcgataatccgggcagtagctttgtgctggtggtgctgttcgccatctggcgctacttcccgtatgcctttatctcgtttctggcgattttgcagaccatcgacaaatcgctgtacgaagcggcagagatggatggcgctaatgcctggcaacggtttcgtatcgtcacgctgcccgcaattatgccggtcctggcgacggtggtgacactgcgcaccatctggatgttctacatgttcgcggatgtttatttgctgacgaccaaggtcgatattctcggtgtatatctctacaaaaccgcctttgcctttaatgatttaggaaaagcggcggcgatctcggtggtgctcttcatcattattttcgctgtcattctgctgaccaggaaacgggtgaacctcaatggcaacaaataaacgcacactcagtcgcatcggtttttactgcgggctggcgctgtttctcatcatcacgctgtttccattttttgtgatgctgatgacctcgttcaagggcgcgaaagaggcgatctcactgcatcctacgctgctgccgcagcagtggacgctggagcattacgtcgacatttttaacccgatgattttcccgtttgtcgactacttccgtaacagtctggtggtgtctgtggtttcatccgtggtggcggtattcctcggcattcttggggcttacgcgctttcccgcctgcgctttaaaggtcggatgaccatcaacgccagcttttacacggtgtatatgttctctggcattttgctggtggtgccgcttttcaaaatcatcaccgcgcttggcatttacgacactgagatggcgctgatcatcaccatggtgacgcaaactctgcccaccgccgtgtttatgctgaaaagctacttcgacaccatccccgatgagatcgaagaagcggcgatgatggatggcctcaaccgtctgcaaattatcttccgcatcaccgtgccgttggcgatgtccgggctgatatccgtgttcgtctactgctttatggtggcgtggaacgactatctgtttgcgtcgattttcctctccagcgccagcaatttcaccttaccggtgggcctgaacgcgctgttcagtacgccagattacatctggggacggatgatggcggcctcactggtgaccgcattgccggtggtgattatgtatgcgctttcggaacgttttattaagagtggtttgaccgccggtggcgtgaagggctaaagcggccagtttctttacaaggagttttaaatgaaaaagttagtagccacagcaccgcgtgttgctgcgctggttgagtatgaagatcgggcgattttagctaatgaagtgaagatccgcgtgcgtttcggcgcaccgaaacacggaacggaagtggtcgacttccgcgccgccagcccgtttattgatgaagactttaacggcgaatggcagatgttcactccgcgtccggcagatgcgccgcgcggcattgagtttggcaaattccagcttggcaacatggtggttggcgacattatcgagtgcggcagcgacgttaccgactacgcggtgggcgacagcgtatgcggctacggcccgctctccgagacggtcatcattaacgcagtgaataactacaagctgcgcaaaatgccgcaaggcagctcctggaaaaacgccgtctgctacgacccggcgcagtttgccatgagcggcgtgcgcgatgccaacgtgcgcgtaggggattttgtggtggtggtagggcttggcgcaatcggtcaaattgccatccaactggctaaacgcgctggcgcttctgtggtgattggcgtcgatcctatcgcccatcgctgtgatattgcccgtcgccacggcgcggatttctgccttaaccccatcggcactgatgtaggtaaagagatcaaaacgctgaccggcaagcagggtgccgatgtgattatcgaaaccagcggctacgccgacgcgctgcaatcggcgctccgcggtctggcttatggcggcaccatctcctatgtcgcgtttgccaagccgtttgccgaaggttttaacctcggacgcgaagcgcatttcaataacgccaaaattgtcttctctcgcgcgtgcagcgaaccgaacccggattatccgcgctggagccgcaagcgtattgaagaaacctgttgggaactgctgatgaacggttatctcaattgcgaagatttaatcgacccggtggtgacctttgccaatagcccggaaagctatatgcagtatgtcgaccagcatccggaacagagcatcaaaatgggcgttacgttttaattcaaaggaatgaaaaaaatgaaaatcggcacacagaatcaggcgttctttccggaaaacattctggagaaatttcgttatatcaaagagatgggcttcgatggttttgagattgacggcaaactgctggttaacaacatcgaagaagtcaaagcggcgatcaaagaaaccggtttaccggtgaccaccgcctgcggtggctatgacggatggattggcgactttatcgaagagcgtcgtcttaatggcttaaagcagatcgagcgcattctcgaagcgctggcagaagtgggcggtaaaggcatcgtcgttccggctgcgtggggcatgtttaccttccgcttaccgccgatgacctcgccgcgtagcctggacggcgaccgcaaaatggtgagtgattccctgcgcgtactggaacaggtcgccgcgcgtaccggaaccgtggtgtatctcgaaccgttaaaccgctatcaggatcatatgatcaacaccctcgccgatgcccgccgttacatcgtcgaaaacgatcttaaacatgtacagattatcggcgatttctatcacatgaatatcgaagaagataacctggcgcaggcgctgcatgacaaccgcgacctgctcggtcatgtgcatattgcggataaccatcgctaccagccgggcagcggcaccctggatttccacgcgctgtttgaacagctgcgcgcggataactatcagggctatgtagtgtacgaagggcgtatccgggcggaagatcctgcccaggcgtaccgtgattcgttggcctggttgcgtacctgctaagaggtctttgtgaaaagtgcaatgacaagctctccgctgcgggtcgcgataataggcgcaggccaggtggcggataaggttcatgcttcgtactactgcacccgcaacgatctggaactggtggctgtctgtgacagccgcctttcccaggcgcaggcgctggcagaaaaatacgggaatgcatccgtgtgggacgatccgcaggccatgctgctggcggtgaaacctgatgtggttagcgtctgctcacctaaccgttttcattacgaacataccctgatggcactggaagcgggctgccatgtgatgtgcgaaaaaccgcccgccatgacgccagaacaggcgcgggaaatgtgcgataccgcgcgcaaactgggcaaggtgctggcctacgactttcaccatcgttttgcgctcgatacgcaacagctgcgtgaacaggtgaccaacggcgttttgggagagatttacgttaccaccgcccgcgccctgcgtcgctgcggcgttcccggctggggtgtctttaccaataaagaactgcagggtggtggcccgctgatcgacatcggcattcatatgctggatgctgcgatgtatgtgctgggctttccggcggtgaaaagcgtgaatgcgcatagctttcaaaagatcggcacgcaaaagagctgtggtcaatttggtgagtgggatccggcaacttacagcgtcgaagattcgctgtttggcaccattgaatttcataacggcggcattctgtggctggaaacgtcatttgcactcaacatccgcgaacagtcgattatgaacgtcagcttttgtggtgataaagctggtgcgacgctgtttccagcacatatctacaccgataacaacggtgaattaatgacgctgatgcaacgggaaatagcagacgacaaccgccatttgcgcagcatggaagcctttatcaatcacgtacagggcaagcccgtgatgatagccgacgccgagcaggggtacatcatccagcaactggtggcggcgttgtatcaatccgcagaaacagggacgcgtgtggaattatgaccaggccagtaacgttatcagaaccccatttcagccagcataccctgaacaagtatgcatcgctgatggcgcaggggaacggctatcttgggcttcgcgccagccatgaagaagattacacgcgccagacgcgagggatgtatctggcggggctgtatcatcgggcgggaaaaggtgaaatcaacgaactggtgaacctgcctgatgtcgtggggatggagattgccataaatggtgaggttttctcgttatcccacgaagcctggcagcgtgagcttgactttgccagtggcgaattacgccgcaatgttgtctggcgtaccagcaacggctcaggttacaccatcgccagccgtcgctttgtttcggcagaccaactgccgctcattgcgctggaaatcactattacgccactggacgccgacgcgtcagtgctgatttcaacaggcattgacgccacgcaaaccaatcacggtcgccaacatctcgacgaaacccaggtgcgggtgtttggtcagcatctgatgcaggggagctacaccacccaggatggacgcagtgatgtggccatcagctgttgctgtaaggtgagcggtgatgtgcagcaatgctataccgccaaagagcgccgtttactgcaacataccagtgcgcagcttcatgcaggcgagacaatgacgttgcaaaaactggtgtggatcgactggcgggatgacaggcaagctgctttagacgagtggggcagcgcgtcgcttcgccagcttgaaatgtgcgcgcagcagagttacgaccaacttcttgcagcatcaacagaaaactggcgtcaatggtggcagaaacgtcgtatcacggtaaatggcggcgaagcgcacgatcagcaagcgttagattatgcgctttatcatctgcgcatcatgacgcctgcccacgacgagcgcagcagcattgcggcaaaaggcttaaccggcgaaggctacaaaggccacgttttctgggatacagaagtatttttgttaccgtttcatctgtttagcgatccgacggttgcccgaagtttactgcgttatcgctggcacaacttgccaggcgcgcaggagaaagcgcgacgcaacggctggcagggcgcgctatttccgtgggaaagcgcgcgcagcggcgaagaagagacgccggaatttgccgccattaacattcgcaccgggctgcggcaaaaagtggcctcggcgcaggcggaacatcatctggtggccgatatcgcctgggcggttattcaatactggcagaccacgggggatgaaagtttcattgcgcatgaaggcatggcgctacttctggagacggcaaagttctggattagccgcgcggtgagagttaacgatcgtctggaaattcatgatgttattgggccagacgaatataccgaacatgtcaataataatgcatacaccagctatatggcccgctacaacgttcaacaggcgctgaatattgcccgccagttcggctgtagcgacgatgcgtttatccatcgcgccgaaatgttcctcaaagagctatggatgccagaaattcagcccgacggcgttttgccgcaggatgattcgtttatggctaagccggcgattaatctggcgaaatacaaagcggcggcggggaagcaaaccatactgctggattattcacgcgcagaagtgaacgagatgcagatcctcaaacaagctgatgtggtgatgctcaattacatgctgccggagcagttctcagcggcatcgtgtcttgccaatctgcaattttatgaaccgcgcactattcacgactcgtcattaagtaaagcaatccacggcattgttgccgcacgctgtggcctgctgacccaaagttatcagttctggcgcgaggggactgaaatcgatcttggtgctgatccgcatagttgtgatgatggtatccatgctgccgcaactggcgctatctggctgggggcgattcagggttttgccggggtgagcgtgcgtgacggtgaattgcatctcaatccggcgttacctgagcagtggcaacagttgtctttccctctgttctggcagggctgcgaattacaggtcactcttgacgcgcagcgtattgcgattcgaacttctgcgcccgtttcactgcgtttgaacggtcagcttataaccgtggctgaagaatctgttttctgtttgggtgattttattttgcccttcaatgggaccgctaccaaacatcaggaggatgaatgaaactgcaaggggtaattttcgatctggatggtgtaatcaccgataccgcgcatctgcatttccaggcgtggcagcagattgccgctgaaattggcatcagcattgatgcgcagtttaacgaatccctaaaagggatcagccgcgatgagtctctgcggcgcattctgcaacacgggggcaaagagggcgactttaactcgcaggagagggcgcaactggcgtatcgcaaaaatctgctctatgtccactcactacgcgagttgacggtcaacgctgttctacccggcattcgctctttgctggcagatctccgtgcacagcagatctcggttgggctggcttctgtctccctgaatgcgccgacgattttagcggcgctggagctgcgcgagtttttcaccttctgcgcggatgcttcccaacttaaaaactcgaaaccggacccggaaatctttctcgccgcctgtgcagggctgggcgtgccgccgcaggcatgtatcggcattgaagatgcgcaggcgggcattgacgccattaacgccagcggtatgcgctcggtggggatcggcgcgggcttaaccggggcgcaattactgttgccttcaacggaatcactcacctggccgcggttatcggccttctggcaaaacgtatagcaaaggaatcaacatggctcagctttcgttacaacatattcaaaaaatctacgataaccaggtgcatgtggtgaaggacttcaacctggaaattgccgataaagagttcatcgtgtttgtcggcccgtcgggctgcggtaagtcgaccaccctgcgcatgattgccgggcttgaggagatcagcggcggcgatctgttgatcgacggcaaacgaatgaatgacgttccagccaaagcacgcaatatagcgatggtgttccagaactacgcgttgtatccgcatatgacggtttacgacaacatggcgtttggtctgaagatgcaaaaaatcgccaaagaggtgattgatgagcgggtgaactgggcggcgcaaattctcggcctgcgtgagtacctgaaacgtaagccgggggcgctttccggcgggcaacgtcagcgagtggcgcttgggcgggcgattgtacgcgaagcgggcgtgtttttaatggatgaaccgctctctaaccttgatgccaagctgcgcgtgcaaatgcgcgcagagatcagcaagctgcatcagaaactgaacaccaccatgatctacgtgacccacgatcagaccgaagcgatgaccatggcgacgcggattgtgattatgaaagacgggattgttcagcaagtaggtgcgccgaaaaccgtttataaccaacccgcgaatatgtttgtttccggatttattggatcaccagcgatgaattttattcgcggcacgatcgatggcgataaattcgttacggaaacgcttaaattaaccattcccgaagagaaattagcggttctgaaaacacaggaaagtttgcataagcccatcgtgatgggaatacgaccggaagatattcatccggacgcgcaagaggaaaataacatttccgccaaaattagcgtggcagaattaaccggtgcggaatttatgctctacaccacggttgggggcacgagttagtggtccgtgctggtgcgttaaatgattatcatgcaggagaaaatatcactattcattttgatatgacgaaatgtcatttctttgatgcagaaacggaaatagcaattcgctaaatacagggggaaggcattcccccaggataatacaaggaacaataatgaaaaagttattaccctgtaccgcactggtgatgtgtgcgggaatggcctgcgcacaggccgaggaaaggaacgactggcactttaatatcggcgcgatgtacgaaatagaaaacgtcgagggttatggcgaagatatggatgggctggcggagccttcagtctattttaatgccgccaacgggccgtggagaattgctctggcctattatcaggaagggccggtagattatagcgcgggtaaacgtggaacgtggtttgatcgcccggagctggaggtgcattatcagttcctcgaaaacgatgatttcagtttcggcctgaccggcggtttccgtaattatggttatcactacgttgatgaaccgggtaaagacacggcgaatatgcagcgctggaaaatcgcgccagactgggatgtgaaactgactgacgatttacgtttcaacggttggttgtcgatgtataaatttgccaacgatctgaacactaccggttacgctgatacccgtgtcgaaacggaaacaggtctgcaatataccttcaacgaaacggttgccttgcgagtgaactattatctcgagcgcggcttcaatatggacgacagccgcaataacggtgagttttccacgcaagaaattcgcgcctatttgccgctgacgctcggcaaccactcggtgacgccgtatacgcgcattgggctggatcgctggagtaactgggactggcaggatgatattgaacgtgaaggccatgattttaaccgtgtaggtttattttacggttatgatttccagaacggactttccgtttcgctggaatacgcgtttgagtggcaggatcacgacgaaggcgacagtgataaattccattatgcaggtgtcggcgtaaattactcgttctgataatgggctaaattgccggatgcggcgcgagtactttatccgatctataaatgtaggccggataagatgcgctagcatcgcatctggcattcaggcaaggtagctggtatttatttcagcgtcatatgcgtggcaacggtaatattctgtggtgacggttttccagaaattaagcggaataataactcgcagctttgttgacctaactcctgcgtcggaacatcgatgccgcccggtgcaggcgttaaaataaatgacagcgtttcattgctataacccaccaccgctaactgctgcggaatagcaatatttttctctgctgccgcacgataaatgctcattaatttcaggctgtcagtggcaaacaccgcctcaggcaacggtgactggcttaataattgccgtgctgcttttaatgcagtttcatgggtataaccgccatcaacaatccattcatcacgcactgcaatattatgcgcagccaggctctgcttataaccattaacgcgatcaaccgaaacatggacatcaagcggagcatgcaggcaggcaatattttgatgcccactttcaattaatgcatcggtcaacgcaatgctgtcgccaaaattatcggtatcgacagaataaacatgggcatattgaccttcaactttgccaatcaccaccaccggaatatcatatttatcgagttgggcaaaaaatgactcatccgctggcgaactgagcataataatgcctttaatcattttctgcttaattttgctttcgcatttttgcagatcttctgccggattgtgcgacgtttgtaatatcacgtcgaaaccttcttcttcagctttggcggtgatggcatgcaaaacttcagagaaaaacggattacccgccgtagttttggtcgaacgggtagaaatcaccataatggcatcaaaacccgaagaggtcagcgcgcgggccagcttgtttggctgatactgtaattcttcaatggcccgtaacactttttcgcgcgcttccggggagatattagtttgcttattcagcacgcgtgatacggtggattttgatacgcctgcaaccctggcaatatcataaatagtaggggacataggtcaggaactccgtccgaacgtgaatgctgcacatcttatggagttcgccggtcgatgacaacacgggcagttgataatcaatggcctggcccccacattcatatccttacgaatgattttttttctggtcttcagagcagcacaggacagcaatgaagcgacttaaaaatgaactcaatgcgctggtgaatcggggtgtcgacagacatctgcgcctcgctgtaaccggacttagccgcagcggcaaaacagcgtttatcaccgcgatggttaatcagttgcttaatattcacgccggagcacgtttgccgctgttaagtgcggtgcgtgaagagcgcctgctgggcgtgaaacgcattccccagcgtgactttggcattccgcgcttcacctatgacgaagggctggcgcagttatatggcgatccacccgcctggccaacgccaacgcgcggcgtcagtgaaatccgcctggcgctacgttttaaatcgaatgattcgctgctacgccactttaaggatacctccacgctgtatctggaaattgtggattatcccggcgaatggttgctcgacctgccgatgctggcgcaggactatttaagctggtcgcgccagatgacgggcttactcaatggtcagcgcggagaatggtcggcgaaatggcgaatgatgagcgaagggctggacccgctagcgcctgccgacgaaaaccggctggcggacattgccgccgcgtggaccgattatctccaccactgtaaagagcaggggctgcactttattcagcctgggcgctttgtcttgccgggagatatggcaggtgcgcccgcgctgcaattcttcccgtggccggatgtcgatacctggggcgagtccaaactggcgcaggccgataagcataccaatgccggaatgctgcgcgagcgctttaattattactgcgagaaggtggtgaaggggttctataagaatcattttctgcgctttgaccgccagattgtgctggtggattgcctgcaacctctcaacagtgggccacaggcatttaatgatatgcgtctggcactgacgcagctgatgcaaagttttcactacgggcagcgtaccctgttccggcgtttgttttcgccggttatcgataagctattgtttgctgccactaaagcggaccatgtgaccatcgatcagcacgctaatatggtttcattactgcaacaactgattcaggatgcctggcaaaatgcggcgttcgaagggatcagcatggactgcctggggctggcgtcagttcaggcgaccaccagcggcattattgatgttaacggtgagaaaatcccggcgctgcgtggtaatcgacttagcgatggcgcaccgctcactgtttatcctggcgaagttcccgcacgtttgcctggtcaggcgttctgggataagcaaggcttccagtttgaggcatttcgtccgcaggtgatggatgtcgacaaaccactaccgcatattcgtcttgatgctgcgctggaatttttaataggagataaattgcgatgaccgaaccgttaaaaccacgtattgatttcgacggtcctctggaggtcgatcagaatcctaaattcagggcgcagcagacctttgacgaaaatcaggcgcaaaattttgccccggccacgctcgacgaagcgcaggaagaagaggggcaagtcgaagcggtaatggacgcagcgttacgtccgaaacgcagcctgtggcgcaaaatggtgatgggagggctggctctgtttggcgcaagcgttgtcgggcagggtgtacagtggacaatgaatgcctggcaaacccaggactgggtggcgctgggtggatgtgccgctggggcattgattatcggcgctggcgtaggttctgtggtaacagagtggcggcgcttatggcgcttgcgacagcgcgcccatgaacgcgacgaagcgcgtgatttattgcatagccacggcacgggcaaaggccgcgcattttgcgaaaaactggcgcagcaggcgggtattgatcagtcgcatccggcgctgcaacgctggtatgcctcaatccatgaaacgcaaaacgaccgtgaagtggtcagcctgtatgcgcatttggtccagccagttttagatgcccaggcgcggcgcgaaatcagccgttcggcggcggaatcaacgttgatgattgcggtcagcccgctggcgttggtcgatatggcgtttatcgcctggcgcaatctgcgtttaattaatcgcatcgccacgctgtatggcattgaactggggtattacagccgtttgcgtctgtttaagctggtattgctgaatatcgcttttgccggagccagcgaactggtgcgcgaagtggggatggactggatgtcgcaagatctcgctgctcgtttgtctacccgcgcagctcaggggattggtgcaggacttctgacggcacgactcgggattaaagctatggagctttgccgcccgctgccgtggattgacgatgacaaacctcgcctcggggatttccgtcgtcagcttatcggtcaggtgaaagaaacgctgcaaaaaggcaaaacgcccagcgaaaaataatgcaatatcgggtgctgaccggatatctttacgccgaagtgcccgtttttccgtctttgtgtcaatgattgttgacagaaaccttcctgctatccaaatagtgtcatatcatcatattaattgttcttttttcaggtgaaggttcccatgcgtctggaagtcttttgtgaagaccgactcggtctgacccgcgaattactcgatctactcgtgctaagaggcattgatttacgcggtattgagattgatcccattgggcgaatctacctcaattttgctgaactggagtttgagagtttcagcagtctgatggccgaaatacgccgtattgcgggtgttaccgatgtgcgtactgtcccgtggatgccttccgaacgtgagcatctggcgttgagcgcgttactggaggcgttgcctgaacctgtgctctctgtcgatatgaaaagcaaagtggatatggcgaacccggcgagctgtcagctttttgggcaaaaattggatcgcctgcgcaaccataccgccgcacaattgattaacggctttaattttttacgttggctggaaagcgaaccgcaagattcgcataacgagcatgtcgttattaatgggcagaatttcctgatggagattacgcctgtttatcttcaggatgaaaatgatcaacacgtcctgaccggtgcggtggtgatgttgcgatcaacgattcgtatgggccgccagttgcaaaatgtcgccgcccaggacgtcagcgccttcagtcaaattgtcgccgtcagcccgaaaatgaagcatgttgtcgaacaggcgcagaaactggcgatgctaagcgcgccgctgctgattacgggtgacacaggtacaggtaaagatctctttgcctacgcctgccatcaggcaagccccagagcgggcaaaccttacctggcgctgaactgtgcgtctataccggaagatgcggtcgagagtgaactgtttggtcatgctccggaagggaagaaaggattctttgagcaggcgaacggtggttcggtgctgttggatgaaataggggaaatgtcaccacggatgcaggcgaaattactgcgtttccttaatgatggcactttccgtcgggttggcgaagaccatgaggtgcatgtcgatgtgcgggtgatttgcgctacgcagaagaatctggtcgaactggtgcaaaaaggcatgttccgtgaagatctctattatcgtctgaacgtgttgacgctcaatctgccgccgctacgtgactgtccgcaggacatcatgccgttaactgagctgttcgtcgcccgctttgccgacgagcagggcgtgccgcgtccgaaactggccgctgacctgaatactgtacttacgcgttatgcgtggccgggaaatgtgcggcagttaaagaacgctatctatcgcgcactgacacaactggacggttatgagctgcgtccacaggatattttgttgccggattatgacgccgcaacggtagccgtgggcgaagatgcgatggaaggttcgctggacgaaatcaccagccgttttgaacgctcggtattaacccagctttatcgcaattatcccagcacgcgcaaactggcaaaacgtctcggcgtttcacataccgcgattgccaataagttgcgggaatatggtctgagtcagaagaagaacgaagagtaagcgcgaatatgcctgatggtgcaacaccatcaggcatattaaattatgctttcagtacagccagagctgcttcgtaatccggctcggtggtgatttcatccaccagctggctgaaaatcacattgtcattttcgtcaataaccacaacggcacgcgctgccagacctttcagtgggccatcagcaattgccacaccgtaagcttgcagaaattcagcgttacggaaagtggagagggtgataacgttgttcagaccttctgcgccgcagaaacgagactgggcgaacggcagatcggcagagatacacagcacaacggtgttgtcgatctcagttgccagttggttaaacttacgtactgatgcggcgcaaacaccggtatcaatactcgggaaaatgttcagcactttgcgtttacccgcaaactgaccgagggtgacgtcagacagatcttttgccacgagagtaaaagtctgcgctttgctacccgcctgcgggatggaattggcgactgtaaccgggttgccctggaaatgaacggtttgtgacatgattatctttcctgtttacatatagttaacgtcacacctagtttatgctaactgtcaataacacagcaaacgctatttgcgcttaatccgcagaccaccgcgacaacaaggagtaaagatgagaaccgttaaggtattcgaggaagcctggcccttacataccccgtttgtgattgcccggggaagtcgcagtgaagcgcgcgtggtggtggttgaactggaagaagagggtattaaaggcaccggcgaatgcacgccgtatccgcgttatggggaaagtgatgcctcggtaatggcgcaaattatgagcgtcgtgccgcaactagagaaagggctgacacgggaggagttgcaaaaaattctccctgccggcgcagcacgtaatgcgctggattgtgcattgtgggatctggccgcgcgaagacagcagcaatcgctggctgatttgatcggcataacgcttcccgagacagttatcactgcacagacggttgtcatcggtacgcctgatcagatggccaatagtgcatcaacactctggcaggcaggcgcgaaattactgaaagtgaagctggataaccatcttatcagtgagcggatggtggcaattcgcacagctgtgcccgatgcgacgctgatcgttgatgcaaatgaatcctggcgtgcagaagggttggcggcgcgttgccagctattggcggatttaggcgttgcgatgcttgaacaaccgcttcctgcgcaggacgatgcggcgctggagaattttattcatccgttgccgatttgtgctgatgaaagttgtcatactcgtagcaatttgaaggcgctgaaagggcgctatgagatggttaatattaagctcgataaaaccgggggtctgacggaagcgctggcgctggcgactgaagcgcgtgcacaaggtttcagtctgatgctgggctgcatgttgtgtacctctcgtgccattagcgccgctttaccgctggtgccgcaggtcagtttcgccgatcttgacggaccgacctggctggcggtagatgtggaaccggcgcttcagttcacgacgggcgaattgcatctttaggatgccagcgcagcaagtttgccatcgcaaagagatatttttcgctggcttcgtcggaggagatgggcggaaactctgcggtgatgcaatgcaagttcagatctgcacaccaactgccgaaagagccaggcgtttcataaccgacgctggttaccagaggcaattcaaacgcctgagccagccattcgcctaattcgctgtgtctgggatcttcaatacaggccagtggatcgtggaatgagaccacccaggcaggttgaatgcggtgtataagctggcacagcgcctgggtttcaggttcggagccaggtttgtcacctgtcagtaatacgacatcgcgttcttcagcggcgctgttccagcgataaacggtttcaccttccttccagttcgccgccggaaagtttctgtttaaatccacaccattagcattggcccgtaaccccaactggcagccgtcaggattcacacacagcaccacatgatgacggcgcaaagaaggtgtcaacgtccgcagagcacaggagagcgtgacgaccgaagagttttcatcaccgtgagtgccagccagaatcaaaccactttcgcggctggctgcaggggcaggaaaccagattaacggcgcgcccaataatgaacgtccgtaatgttctgttccgggcggaaatgcgccgcgttcggcgcgtgggcgggttacggtcatgatcgtctctggttcaggaagtattacaggcagtgttgtgcaaattttgcggattatcaaatccttttcttcaacgctatgtcatcgatcttgtatcacttttttgccggaagttgtttgcattttattagttggatagggtttgtggatttttgctggctgacgggcaaataaagtttgtttaatggtttgcttatctgccagttgattaatcacatggcgggctatctgaccgccagcaccaagaatcagtacatttttcatgaaaattatcccagattattggcagcaatatgccagtccatatcactattgcggatttgaatatgtttcattacagagtttcctcaaagaacggagctaatactgaaattgcttcagccacataggctttgccgtcataaagatccatatggtttgcgccttcaacaatgtgatagcgtttatcctggcttgatgctcgatcgtacaggtcgtcactcatccatttgctccctgcctggctgcccgccacaatctgcgtcggctgagtcaggtacacttccgccatatggtaagcatcataggtaataatctggttaaggctgcgcaaagtagcgtaacccggtgctgttggatactgcgcgcgaggggtgtggtaatactcccaggcctgacgcagttcttcgttcggcgcatcggactccttcattggtgccagtggcataatggcgtattctccgctgctaatatcgctggttctggcgtttgaacccgcttcaacgtatggcagggcatcaatagatttcacattgttttcccaaccattacggaatatcgaaccaatattgaccgcactaacggtaccgatggccttgatgcggcgatcctgaattgcagcattggctgtatatcctgcaccggcacaaattcccatcgcaccaattcgggtattgtcgacataagaaagcgttgtcaggtaatcaatcacggcactgatgtcttcagtacgaatgtatgggttttctaactgacgcggctcgccgccactttcaccttgataagatgcgtcataagcaatagtgacaaatcccttttccgccagttttttggcataggttccggccgtttgttctttaacgcccccacctgggtgagataacacaattgcctgatactgacgggtttcatcaaattttggagggaaatagatcactgcagacaaagagatggttggattattgctgttagtgaagctgactttattattcatcattccgttcctcatggagttgtcggttcgttttaacggttggtgatatcactatagatattgatcattaagttgattagacccaaaatcatgattagacctatcatttaaatgattaatagattgcatggagatactgaatgaagcgtgaagaaatcgctgatctgatggcgtttgtcgtcgttgcagaggagcgtagcttcactcgtgcagcagcccgcctgagcatggcgcagtcagctttaagccagatagtgcgtcgtatagaagaacgattgggattgcggcttctgacgcgaaccacgcgcagcgttgttccaactgaagcgggcgagcatcttttgtctgttcttggccctatgttgcatgacatagattcagccatggcatccctgagcgatctgcagaaccgcccatccgggacaatacgtattactactgtagaacatgcagcaaaaacgatattgttaccagcaatgcgcacattcctgaaatcgcatcctgaaattgatattcagctcaccattgattatggtttgaccgatgtcgtttctgaacgttttgatgcaggcgtccgtctgggtggggagatggataaagatatgatcgccattcgaatcgggccagatataccaatggctattgttggctcaccggattatttttctcgccgaagtgttccaacgtcagtgtcacaattaatagatcatcaggcaattaatttgtatcttcccacatcgggtacagcaaatcgctggagattaatacgcggtggacgtgaagttcgtgttcgcatggaaggtcagcttttactgaatacgatagacctgatcattgatgctgcaattgatgggcatggattggcgtatctaccttatgatcaggttgagcgggctattaaagaaaaaaaactgatacgtgttttggataaattcacaccagatttacccggttatcacctgtactatccacaccgtcgacatgctggctcggcattctcattatttatagataggctgaagtataaaggtgctgtttagcactacttgctgatacattaatttaattcttctcttaacgtattctcagttcctttcaacgttttggtcattttttattcttcgtacaatggcgacagatgctgattatgataccgaaaacgggtttgaacgtgcgaagcccgaacgtagtgttcggagttctatgtgctttaccgcattttggagactattatttacactaaatctgatttgatatattgatacttaaaacatttgatgcttcctttgtcacttttttgatggaagttgtttgcatttctttaaggcgaaacaaataattacgcatcaattttaatgtcggttagagggaaacttatgaagcactctgtttcagtcacgtgttgtgcgctgttggtcagcagcatttctctttcgtatgctgcagaagttccgagcggcacagtactggcagagaagcaggagctggtgcgccacattaaagatgagcctgcgtcgctggatcccgctaaagccgtgggcctgccagagattcaggtcattcgcgatctgtttgaaggtctggtgaatcagaacgaaaaaggggagattgtccccggcgttgcgactcagtggaaaagtaatgacaaccgtatctggacttttaccctgcgcgataacgcaaaatgggcggatggcacaccggtaacggcgcaagattttgtctacagctggcaacgtctggtggacccaaaaacattgtcgccatttgcatggtttgccgcgctggcgggaatcaacaacgcacaggcgattattgatggtaaagctacgcctgaccagcttggcgtcaccgcagttgatgcccatactttgaaaattcagcttgataaaccgttgccgtggtttgtgaatttaaccgctaactttgccttcttcccggtgcaaaaagccaacgtagaaagcggtaaagagtggacgaaacccggaaatctgatcggcaatggcgcttatgttcttaaagagcgcgtagtcaatgaaaaactggtcgtggtaccgaatacccattattgggataacgccaaaacggtactgcaaaaagtgaccttcctgccaattaatcaggaatccgcagccactaagcgttacctcgcgggggatattgatatcaccgaatccttcccgaaaaatatgtatcagaagctgttgaaggatattccggggcaggtttatacgccgccgcagctcgggacctattattatgcgtttaacacgcaaaaagggccgacggcagatcagcgcgttcgtctggcattaagtatgacgatagatcgccgcctgatgaccgaaaaagtattagggacgggcgaaaagccagcgtggcattttacaccagatgttaccgcgggatttacgccggaaccttcgccgtttgaacaaatgagtcaggaagaactgaatgcgcaggcaaaaactttgttgagcgcagctggttatggtccgcaaaaaccgctgaagctgacgcttttgtataacacttcagaaaaccatcaaaaaattgcgattgctgtagcatcgatgtggaaaaagaaccttggcgtagatgttaaattgcaaaatcaggaatggaaaacctatatcgatagccgtaacaccggcaattttgatgttatccgcgcctcgtgggtgggggattataatgaaccctccactttcctgacattattaacgtcaacgcattcaggaaatatttcacgctttaacaatccggcatatgacaaagttctggcccaggcatcgacggaaaataccgttaaagcgcgtaatgccgattacaacgcggcagaaaaaatcctcatggagcaagcaccgattgcaccaatttatcaatataccaatggacgattaatcaagccgtggctgaaaggttatcccattaataatcctgaagatgtggcgtacagtcggactatgtatattgtgaagcattgatgtgatgggaactggcgttacccttgtgcataacgccagtgatgtctgatttagcgaccctgttccggcggtgtaatgttatccatatacagcgtctggctggggaaggcaaagtccgcgccgtgtgactgtacaatatcgataatcttcaaataaacgtcttgctgtgcagcaagccattcagcccataccgtggttttggtaaagcaataaaccataatattcaatgaagagtcagcaaactggttgaaataaaccagtaaggtttgtcgctggtcgatggccgggtgatttttcagcatctcacgtacagcttcgacaataacgcccacttttgccgcatcctcataacgtaaaccaatggtcgtggtaatgcggcggttggtcattcgtcctgggttttctacgctgatcgacgaaaacagcgagttcggtacgtacaatggacgattatcaaaggtcgtaattttggtaattcgccagccaatttccgctactgtaccttcgatatttctgtccggtgaacggatccagtcgccaatactgaaaggacggtcgaaatagagcataatcccggaaaagaagttactcagaatatctttaccggccataccgacagccagaccaccaataccaccaaaggtcagcaagccagaaaggctcatgccgaaatgttcgccataaagcagaacaagcaccacaataatggtgattttgatgatacgcgacataatccgcgcactggtgatatcgcgaccttttttaatctgctgtttttcaaactgattaatcagcagaaatagcttaatcgtcagaataaccgcaatcagggacgtacagataaaatcgataacgcctggggtgataaatttgagtttatagttttctataacataattaataatgctaccaacagcactgataattatggtgtagattaaaaattgcaccgcatggaataaaaatccttttcttttacgatttccacggcgaaaccaaaagctcatcagaatcaatgctgcgcagctaccgaaaataatgaccagattaagcgcattatttgtaaacagttcagcgatcattgttttatcaggctcctccagataattgtcgtcatgccggaaacccctggcggggctattttaccgcgacaattcattcagatcatcaatagtcagggaaggaagtagcaacattagctaaggaaggtgcgaacaagtccctgatatgagatcatgtttgtcatctggagccatagaacagggttcatcatgagtcatcaacttaccttcgccgacagtgaattcagcagtaagcgccgtcagaccagaaaagagattttcttgtcccgcatggagcagattctgccatggcaaaacatggtggaagtcatcgagccgttttaccccaaggctggtaatggccggcgaccttatccgctggaaaccatgctacgcattcactgcatgcagcattggtacaacctgagcgatggcgcgatggaagatgctctgtacgaaatcgcctccatgcgtctgtttgcccggttatccctggatagcgccttgccggaccgcaccaccatcatgaatttccgccacctgctggagcagcatcaactggcccgccaattgttcaagaccatcaatcgctggctggccgaagcaggcgtcatgatgactcaaggcaccttggtcgatgccaccatcattgaggcacccagctcgaccaagaacaaagagcagcaacgcgatccggagatgcatcagaccaagaaaggcaatcagtggcactttggcatgaaggcccacattggtgtcgatgccaagagtggcctgacccacagcctggtcaccaccgcggccaacgagcatgacctcaatcagctgggtaatctgctgcatggagaggagcaatttgtctcagccgatgccggctaccaaggggcgccacagcgcgaggagctggccgaggtggatgtggactggctgatcgccgagcgccccggcaaggtaagaaccttgaaacagcatccacgcaagaacaaaacggccatcaacatcgaatacatgaaagccagcatccgggccagggtggagcacccatttcgcatcatcaagcgacagttcggcttcgtgaaagccagatacaaggggttgctgaaaaacgataaccaactggcgatgttattcacgctggccaacctgtttcgggcggaccaaatgatacgtcagtgggagagatctcactaaaaactggggataacgccttaaatggcgaagaaacggtctaaataggctgattcaaggcatttacgggagaaaaaatcggctcaaacatgaagaaatgaaatgactgagtcagccgagaagaatttccccgcttattcgcaccttccctaactaatcaatgcgttgattgtaaatccagctaagaggtgaggttttcagagcagacaacggtgaaatgtcatggtattgttacgtttaggtaacaagaaatttgtctgcacaaggattacatcatgattatggcgaaactgaagtcagcgaaagggaagaaatttctctttggtttgttggcggttttcattattgcggcgtcggttgtgactcgcgcgaccatcggcggcgttatagaacagtacaatattccgctgtctgagtggacgacatcaatgtatgtgattcagtcatcgatgatttttgtttatagcctggtctttactgtgttgctggcaatcccgttgggaatttatttccttggcggcgaagagcagtaagtaaaaaataggcccgataactcgggccttgtcagttattgaagagtcgttaatcgtcttcttcgtcatccagttcaacgggtgtctgatactggtcaggtttaatgaccagcaggtcgcagcgaagatgatcaatcacctgttccgccgtgttgccgaggaatgctgctgaaataccggtgcgtcctaccgtgcccagaaccacaatccccgcctgtaagtgctccgccaaatcaggaatcacctcttctggcagacctttttctacgtgcgtcatgttttcattaatgccgaatttctgccgcagggctttcattgccagcaaatgttgcccacgaatggcatcgttataaacgctcgggtcaaattccggcagttcaatcgcgatattaattggcgttaccggataagcgccaaccagatgaacttcggtatggttgacttgttctgccagttcgatcgtctctttgaccagtttttcattgagcgcattatgatacggctcttcactggcgagattcaccgccaccagcgccttgcctccttccggccacggctggtctttcaccatccacaccgggcttgggcatttgcgtaacagatgccagtccgttggcgtaaaaatcaccgcttccagacggtcatgttggtgcgccatttttagcaccaaatcgtgtccgccgctgatcacttcctgaatgatggcttcgaaaggacggttatgccagaccactttaatttcaatgggaacgccagcattgagataatattttgcctgctcgtggatccaggctgtacgctggctgatgacgccctgacgcatagcggtacgttcgtccggggagagcagggtggtcatttcgtatgagaagtcatagatcggcaaaaaggctttaattttgccaccaatccgttgatgtaaataaacagctcgccgcaatgctggttggtcgtcctggttaggatcgataacaacgagcatgttctgatacatagccatacagggtctccttacaacaactgtcaacgcagtttgtaattaaaagattaacccatatctggtgaatgaaacagtgatgaaccttctgccagatcaataaatcagaaaaatttaatgatatgacagaaggatagtgagttatgcggaaaaatcaggcaacgttacgcgtatgaccagcaagctgggccagcgcatcgttattttcgatggtgatgtatttacctttgactgccagcatgccgcttttctggaagcgacccagcagacggctgatggtttctaccgtcaggcccagatagttaccgatatcgccacgagtcatcgtcaggcggaattcacgaggggagaagccgcgttgggcaaaacgacgggacaggttgtagatgaatgcagccagacgttcctcggcatttttcttcgacaacagcaggatcatgtcctgatcgcctttgatttcaccgctcatcagacgcatcatctgctgacgcagattcggcattttaccggacaaatcgtccagcgtttcgaacgggatttcacataccatcgaggtttccagcgcctgcgcgaagctcgggtgatggccgctgccgatggcgtcaaatcccaccaggtcgcctgctaaatggaaaccagtgatttgctcgtcgccttgctcagtgatggtataacttttaatcgtaccggagcggatggcataaagcgatttaagttcatcaccagccttaaacagcgtctggcctttctgaataggcttcttccgctcaatgatattatcaagctgatcaagctcatgttcgttgagtgtgaacgggatgcaaagctggctgatgctgcaatcctggcaatggatagcacaaccgccagactgaatgcgccgtataattcgcttttccgggatcataggtctgctcaagccgtaattgatatttgtcaattttaacatctttttagggagcaagtaagtctaagcaaaccttaacagcagagaattccgatattagatgtaaatatatgtctatctatttgaaaacccttaagttgttaagggtaactttacataaaagtgtgaacaagctggcacaaattgtttaatgtttacagcaaaagataaccttcatggcgcaataaccactcttttcgctgaactccgcctgcatatccggtcatggtgccgtttcggccaataacccgatggcaaggtacgacgatgctgatgggattcgatccgtttgccgcaccaacggcacgcgccgcgccaggacggcccaattgctcagccagttggccgtaatgcattacctgcccgcaggggatagtgcgtagtgttttccagacttcgcgctgaaatggcgtcccccccgtagcagtgggaagcgtatcaataatgctaagattaccggcaaaatattcacgaagcttgtcgcttaaaccgcctggattggtggcagaaatgcgctcatagccttctttgcgataatggatgtccagcagctgcaccatgcgttcgctgtactcttcccattcaaccgcccgcaggcgaaattgctcatcgcaaatcacccacagtggacccagtggcgtggcaattttttcttcaagtaatctcagcatccgttctctcttaagacaaacgtgggtaaatacccggacctatcggcagaccgacaagataccacgccagcaacatcagcagccataccaccaaaaagataagtggatagggcaagactaacgaatagtaagtacccagtttcgcgtctggtttgtagcgttgcaggaatccaagaaacagtggaacaaaaggagataccggcgctaaaggcaatacggatgagtcggcaatacgaaagaggatttgcgcaaatgccgggtgaaagccaagtagcataaacattggtacgaaaatgggggcgagaatcgaccagattgcggaaccgctggcaataaacatgcataagaaagaggaaagcaacgccagaccgacaaacgccgggatgccgctaagccctgaactttccagtatatcggtcagccccacggcgatgaatttccccatgttgctccagttaaacatggcgacaaattgggcgaggggaaaaaccatcacgataaatcccgccatctctttcatcggttcaatcattaaatgcggtaaatccgcctgacgtcgaattgtgcgggtagcgatgccataagccagcgagacaacaaagaaaaaaagaatgatcagtggcacgatacctttaataaagggtgatggcatcacggtgtgattaatcggatcgcgcaatatcccgttttgcgggatcaccatcagcgcaatcgcagcaataaaaagtagcgatacgacacctgctatgcgtaaaccaaaacgctgactttcggtcaatgtctgcagtttctcatcgctgtttccctgccattgacctaaccgtggctcgatgattttgtcggttatcaggccgccaacaatcgtcagtacgactacggagctggccataaaataccagttatcaattacactgacgtgcatttgcggattgaacgcagctgccgcttccgtgctgatccccgacagcaacacgtcggttgtgacaatcagtaaattagccgtaaagccgcaacctacgcctgcaatggcagccagtaaacctgcaactggatgcctgcccaccgccagaaaaatcagcgcacccatcggtggcatgatcactaacgccgcatcggaagaaatgtggctgaaaaaagcaataaacagcaccatataactggcgtagcgggcattaacatgcgatgccattttaaccattagtgctggcagtaagccgacgcgctccgccagaccggcacctaaaaccagcgccaggatcgcaccaagtggagcaaaaccgctaaagtttttaataacattgggtaaaaaccagtgtaatccttccacactgagcaggtttttcaccacgaccggcgtaccatcggtcgggtttttcgcactgacgccaaaggccgacaaaattgccgtcgtcaccatgagtacgataatcaaatagataaagagcagaaaaggatggggaaccttgttaccaattctttcgacccagccatagagcttcccggattgggaggacgacggtatggatgacatactcatgggcattcctcggttgttgtgtttgcgttgttgttgttattttaaaggtgacggtgtcacgtttttcgggatagggcagtgatacggttgcgtgtccgttacttgctgatgctcttgttggcattcttgcaatagccctgaatcaaggaagagattgactgtggttgctgccatagttttcgccgccagcagcattcctttatgagcaatagatgttcgcccctggctaaccagttgccacgtatgtagcggtgtaccgacggcaaaacaggggctgaaacactgggcaacaggcagtttccaactgacgtcgccgacatcagtcgatgccgcaagcacgttatcggtggcggcatatggagcgacttcattcgccagtaccgtttcacgatgacgtagtgcaaaaaccttgccgttttcgccaccggttgcggcgatattattcagactgttttgccgatcgttggaggtgagcgtagcctgaatttgtttcgcaaaagccagttcttcggagttccattccggggtaccaaaatgggatagggcctggtacatggcattttctaaggtgcgattcgggagataactggaacaggctttgtcgaagcggcattcaaccgtggtttcggtcatcaatgccgcaccttcggcgattttggcgacccgatcataaatatgctgcacgtcggtcatttcgggggcgcggataagataaagcacttctgcctgcgcctggaccacgttgggcgagatcccgccgctatttgtgatggcatagtgtacgcgcgctttttcaataatatgttcgttgaggaagttggtgccagtggtcatcaacgttacggcatcaagggcgctgcgtcccaaatgaggggaattcgcggcatgtgctgcgatccctttaaagcgccatgatgcctgaatgtttgccagcgtgcgggtattgaacataccggcaaaggcttccgggtgccaggtgagtgccgcatccacatcatcaaataccccctcgcgaaccatgaacgttttacccgagccgccttcttcgccaggacaaccataaaagcgcaccgtgccgccttgcccatattgttccagccatttcttgacggctattgcagcggcaaaggcggcggttcccagcaaattgtgtccgcaaccgtgaccattttcaccgggcgtcacggatgtaggttgcgcgcaacctgcttgctgacttaaacctgccagggcgtcatattctcccagcagggcgataaccggtttgccttgaccaaacgaagcaataaaggcatttgggatattgcctacgttgcgggtaacggtgaagcctgcagattccagcgccgaagccagatgctccgctgaccagaactcttcaaaacgtgtttctggatgatcccagatttgatcggcaatatcggtataacgttggcgatcggcttcaatcgcatcgtcgataaaacgatagatttcctgcatcagatacctcgcgtccagggaaaattgagcgcggtgcgcgccagcgtttcgacggcaatagcgagaacctgctcgtcaaaatcgaatttttcgttgtgatgacctgccgccagctgtgtgccaaacaccacgtaggaggcttgcccttgatgttgctgcacgcgggccatcattaatgtggcatcttcggaacccgcaggcgcttcaacacgttcaatggcctgattgacccccgcgacctgagccgcctgactttgcaaccatgcgacccattgcggcgaaggagaactggcggtagctgcacccatcagacgagtttcaacgccgacaccatacatggttgctgcgccctgaatcgcttgttgtgcacggtcaaaaacatattgattaatgacgtcgctggccccgcgtgtttccactttcagcaacgccgaggcaggaacaacgttacgaccgcttcctgcctgcataacgcccacgtttactctggaagctccttcgctgtgcggggcgattgcatgcagtgcaagagtggcttgtgctgccgccaacaaggcattgtgaccgtcttctggttttgcgcctgcgtgagcggcggtaccggtgaagtgcgcgtcaaatttggtggttgccataaaattatcactgccgcacaccacggtgcccgcaggtacgccagtgccaatgtgcacggcagtaaaataatcaacatcatctacgacacctgcatcgaccatcgcccgcgcgccacgcgtaccttcctctgcaggctgaaaaatcagtttgatgacgccatgtagtccggactcgaactgtttaagggtatgcgccagcccaagcccaatggcggtatgtccatcatgaccacaggcatgcatcattccggcgttacatgacgcaaaaccgtcgcggtaggggcgatggctgacatcctgctcttcactgagatccagcgcgtccatatcgacacggaaagccatcaccggaccggggcgaccggtatccagggtggcgacgataccagtgaaaccaccttcaaaagccgcaatccattgtgctagcgcaccctgttgacgagcgcgctcgaattcgcgttgtagagtgaattcatcaggtaatcccatccggctactttcattaactacttcgcgacccagcgccagtgaatagccgagctggtgcaattcttccgcaacaagggtggcagtgcggaattccacccagccagactctgcatagtgatgaaaatcacgtcgccagtgcgataattttggggcaagcgaattaacaaattgattcaaagactccataacctttcccgtcatcagtaaaaagtgtgacccggttcacgtagcgatagtttttacttatcactaactgatttttcacagttttaaccgttcataaattaccctgacacaatcatctgcattaaagtagatgccagtttctttggtctgataaataacggttatcggtggcgtcatggcttttcaggtaaaaattcatcaaattcgggcttttgttgaagtggctcgtcagggcagcattcgcggagcgagccgaatgttgaatatgtcgcaaccggcactgagtaaatctattcaggagctagaagaagggttagcggcgcaactcttttttcgccgtagtaaaggcgtgacgttaactgatgccggtgaaagtttttatcagcacgccagtctaattcttgaagagctgcgcgcagcccaagaggatattcgccaacgacaagggcaactggcagggcagattaatatcggcatgggggccagtatttcccgcagtctgatgccagctgtcatatctcgttttcatcagcagcatccgcaggtaaaagtacgcattatggaagggcaactggtgtcgatgattaatgaattgcgtcagggagaattggatttcaccatcaatacctattatcagggaccgtacgaccacgaatttacttttgagaaattactggaaaagcaattcgcgatcttttgccgcccgggacaccccgccattggtgcccgttcgatcaaacagttactggattacagctggacaatgccgacgccacacggcagctactacaaacagttgagtgaattgcttgacgatcaggcgcaaacgccacaggtcggtgtagtctgcgagacgttctcagcctgtatcagtctggtggcaaaaagcgattttctcagcaaactgcctgaagaaatgggctgcgatcccttgcacggacaggggctggtgatgttgccggttagcgaaattttaccgaaagcggcctattatttgattcagcggcgtgatagtcgccagacaccactgaccgcgtcattaatcacgcaattccggcgagaatgcggctatctgcaaagttaaaactgcataaaaaaatagagtctgtcgacatccgccagactctacagtacacacagcagtgcatccgcgtcttaaatccggcattgtctcctctgcgccggtgactgtgttataacggttttaacctttagttgccaattttcttcagtgacagatttcacgaaaatataagttacattattaatatcgtgaatgaataatcatgcataagtattttgcttaaaatatcggcaatatttggaacttattactggaaatttgggtaatacgttgttggaccgacccggtctggttatcatatcgcgctcttaattgcgggaggatgtaacatgaaccttgacgacaaatcgctgtttcttgacgccatggaagatgtccagccgctgaaacgtgctaccgatgtccactggcatccaacgcgtaaccaacgtgcgccgcagcgtatcgacacgctgcagcttgataatttcctcaccaccggatttctcgacatcatcccactaagtcagccgctggagtttcggcgggaagggttgcaacatggggtgctggataagctgcgcagtggtaaatatccgcaacaggcgagcctgaatcttttgcgccagccggtggaagagtgccgcaaaatggtgttcagttttattcaacaagccctggcggatggtttgcgtaacgtgctgattattcatggtaaagggcgggatgataaatcgcatgccaatattgtccgcagctatgtggcgcgctggctgaccgaatttgatgatgttcaggcatattgcaccgcgctaccgcatcatggcggcagcggggcgtgttacgtcgcactacgtaaaacggcgcaggcgaagcaagaaaactgggagcgccacgctaagcgcagtcgttgatctcgagacgcatccgcggcttatgccgccagcacgcggttgcgtccatcatttttcgcccgatacaaagcatcatcaacgcgtttaaacagttcatcgatgctttcatttccttcgtgatgcgccacaccaatgctgacggtaaagcgtggtaagcccgaaatactcacttttgccacgcttacgcggatagtttcagccagcgaaagcgcggtatccagtggggttcttggtagcaataagacaaactcttcgcctccccaacgaaacaccaaatcgcctttgcgagcgcaactttcgagggtgcgggcgagggcgcataacacctcatcacctttagaatgcccatagagatcgttaatgtgtttaaaacgatcggtgtcgatgagcaacaagctgtaatcctgagcgatggcgagatgctgcatttggcctggttccgtaatgtgataaaactgtcgccgattcagtaatccggtcatcgcgtcatggtgagcagcatgttccagctgctcctccagccgtttttgctcagtaatatcatgcacaatacataacatgagcttgtcgccataaatttcaatcggtccggcataggtctgcacatgacgagtcgaaccatccgccagtttatgaacaaaattcaaaggtttatgaccaccgggtaaatgcgagatttcatgcatgataggcatgacgcgacgcccgagcatatttatttcccaggtatgtttctggcacatcgtttcatggttataaccatagaaattgagcgcggcgaggttagcatcgacgatttgtccatctcgtgacgggtcaatcaacaacattggtgcagagttagtcagaaaaaagcgcgcataaaaaccttgttttttgcgctgataatttgccgagcgactggcttttaaacccagcgttgccggcgcttcgataccttcgaaaataatcaccggttctgtttctgtcagctttcgcaaaacaagccgacagctcaatgctgtttcctcttctttacgctgaacagtgaggatttcgataatatcgtgttggttttgcagatcggagaggtatttcggcagttctttttgtgaggagacggaatagggtccggttcgtagctgactaaacgtgaggtcttgcatcaacagtttcgccgcgctattggcataaattaactgttcctcaaagggcgaaacgatccagacaggactggtgagtaagtccagggtattgaagttgtgcgtaatcattgagatcccgttatttttatcaatttttgttgctatccgatcgcaaaaaagccacgtcatatgatcagataattctgataatgatagacgctatttaacacttcacacggtttgtatacggaaaagcattttgctttttgtattcaatttagacagaattttattaatcatttcagggtaatggggtgatgagatgttgcgtaacagggccagaaggctagactacaaaataatgcgttgatgatggaggcactgtggaagcgattaagggatcggacgttaatgtcccggatgcagtatttgcctggatgctggatggtagaggcggcgttaaaccgctggaaaatacagatgtgattgatgaagcgcatccctgttggctccaccttaattatgtacaccatgatagcgcccaatggctggcgacaacaccgctgcttcccaataacgtacgtgatgcgctggcgggcgagagcacgcgtccccgagtcagccgtctcggtgaaggcacgctgattacattgcgctgtataaacggcagcaccgatgaacgccccgatcaactggtcgccatgcgtgtatatatggacgggcggttaattgtttcgacccgacaacgcaaagtgctggcgctggacgatgtggtgagcgatctggaagagggcacgggtccgaccgattgcgggggatggctggtggatgtgtgcgatgcgttgaccgatcattccagtgaatttatcgagcagctgcacgataaaattatcgaccttgaagataatctccttgatcagcaaattccaccgcgtggattcctggctctgctgcgcaaacaattaattgtgatgcgtcgctatatggcaccgcaacgtgatgtttatgctcgtcttgccagtgaacgtttgccgtggatgagcgatgaccaacgccgtcggatgcaggatattgccgatcgccttgggcgcggccttgacgaaatcgacgcctgtatagcacggactggcgtgatggcggatgaaatcgctcaggtgatgcaggaaaatttagctcgtcgtacctatacaatgtcgttgatggcaatggtctttttacccagtacctttctgaccgggttatttggcgtcaaccttggtgggatccctggcggcgggtggcaattcggattttcaattttttgtattctgttagttgttcttattggtggtgttgctttatggttgcatcgtagtaaatggttgtaacaaaagcaatttttccggctgtctgtatacaaaaacgccgcaaagtttgagcgaagtcaataaactctctacccattcagggcaatatctctcttgcaggtgaatgcaacgtcaagcgatgggcgttgcgctccatattgtcttacttccttttttgaattactgcatagcacaattgattcgtacgacgccgactttgatgagtcggcttttttttgcctgttatttatcagcgtctaccctttaagagtccacccaatgaccagagggaaatatgacgacacttatttatttgcaaattcctgtccctgaaccgattcctggcgatcctgttccagtgcccgatccgatccctcgcccgcaacccatgcctgacccaccacccgatgaagaaccgattaaattgtcgcatcgtgagcgtagatctgcgaggatacgcgcctgctaactttgcgtcgatgaccacgagaatagattgtgaccgctttttctaccctgaatgttttgcctcccgcccaactcacgaaccttaatgagttgggttatttaaccatgacgccggtgcaggccgccgcgcttccggcgatccttgccggaaaagatgttcgcgtgcaggcgaaaaccggcagcggcaaaacggcggcttttggcctcggcttgttacagcaaattgatgcgtcgctatttcaaacccaggctttagtgctgtgtcctacgcgtgaactggcggatcaggtggcaggtgaattgcgtcggctggcgcgttttctgccaaataccaaaattttgacgttgtgcggtggtcaaccgttcggtatgcagcgtgattcgttgcaacatgcgccgcatattatcgtggcaacgccggggcgtttgctggatcacctgcaaaaaggcacggtatcactggatgcgttgaatacgctggtgatggatgaggccgaccgcatgctggatatgggatttagcgatgccattgatgatgtcatccgttttgcgcctgcatctcgacagacgcttctgttttcggcaacctggccggaagccatcgctgcaatcagcggacgagtgcaacgcgatcctttggcgattgaaattgactcaacagatgctttgccacccattgaacaacaattttatgagacatccagcaaaggcaaaattcctctgttgcaacggttattaagcttgcatcagccatcctcttgcgtggtgttttgcaataccaaaaaagattgccaggctgtctgcgacgcgctgaatgaagtagggcaaagtgcattgtcattacacggcgatttggagcaacgcgatcgcgatcagaccctggtacgttttgctaacggtagcgcccgtgtactggtcgcgactgatgttgctgcgcgtggtctggatattaaatcgcttgagctggtggtgaactttgagctggcgtgggaccctgaagttcatgtacatcgcatcggtcgtacagctcgtgcaggaaatagcggtctggcgatcagtttctgtgctccggaagaagcacagcgggccaatatcatttctgacatgttgcagataaaacttaactggcaaacgccgccagctaatagttccattgcgacgctggaagcagaaatggcaacgttgtgtatcgatggcgggaaaaaagccaaaatgcgcccgggtgatgtattaggtgcactgacaggagatatcgggcttgatggcgcagatattggcaaaatcgccgtgcatccggcgcatgtctatgtcgcggtccgtcaggctgttgctcataaagcatggaaacagttacagggcgggaagattaaaggaaaaacgtgccgggtgcggttattaaaataatgaaatgttgaattgccgggtgcaagagtaaacatcttattcgggattgccggatgcgacgctggccgcgtcttatccggcctccataagagtagcccgatacgcttgcgcatcgggcgctatcctggttatttcacttcaaccacattcagccgtaactcatccaactgattttcatcttcttctggctgccagcacgccggttgtagtgggatctcttcgcgatcaaacgccagatcacccccgttaaccacttcagaaccgtgggtgatgcctttgaaatcgaacaggttggtatcgcacagatgcgacggcaccacattctgcatcgcgctgaacatcgtctcgatacgccctggataacgtttatcccagtcacgcaacatgtcagcaatcacctgacgttgcaggttaggctgtgaaccgcacaggttgcacggaataatcgggaacgcttttgcatcggcaaatcgctgaatatctttctcgcggcagtaggccagcggacgaataacgatatgtttgccatcatcgctcatcagtttcggaggcatacctttcatcttaccgccgtagaacatatttaagaacaacgtttgcaggatatcgtcacgatggtgacccaacgcgatcttcgtcgcccccagttccgttgcggtacgataaaggataccgcgacgaaggcgagaacacagtgagcaagtggttttgccctctggaatcttctctttcacgataccgtaagtattctcttcaacaatcttgtactcaacgcccagcttttcaagatactcgggcagaacgtgttccgggaagcccggttgcttttgatcgaggttaacagccaccagcgaaaaattgattggcgcgctttgctgcaaattgcgcagaatctccagcatggtatagctgtctttacccccggagaggcaaaccatgatgcgatcgccttcttcaatcatattgaagtcagcaatggcttcgcccacgttacgacgcagacgtttttgtaatttgttcaggttgtattgttctttctttgtaatttgttgattttcttgcattatttcagttctctggtactaaatggggcaaattgggggcaaactttgcaactacgataaccgcgcattcaacatggctatctgttcgtcgttcatgtcatcaatccacataccgtaaatttcatacaccatctgcgcagtttcatgccccatttggctggctataaatgccgggttcgctcctgccgtcaacagccagcaggcaaaagtatgccgcgtatggtacggattacggcggcgaataccagcacgttttactgctgcattccaccttgcccccaaactgcttaccgagtaataaggtttttgttttccgttacacaccctgggcatgaaaacaaaatgcagtttttgcttttcggttctgccgtactcccgatgataaaaggtgatttcgcttttgcgatgatgcccggtcagtttgtattgctccttcagtgcttcaagagcaggctgcagtagtgttactgttcggatcccggcatttgtttttgggggaccgaacatatcaagtatcgtcaggtttcttctgacattcactattcccttttcgagatccacatcctcccacgccagagctgccagttccccgtgacgaagtcctgagtaaacggcaaatttccacaagttctggctctgtcctttttcactttccattaatgcattgaattctgttttagataacggatcaggctttattctgtttcgctgtaatttttttactccttcaaatggtttggttgatataaatcccgactgatacgcaaaacgcaacagcgaacagagcagggcgatatagttatcaactgtgcgcacggttcttccttttttgttggatcttggattatccaggtaaagcgtttctccatgcagcagttcattccggtagtttaagatatcgctataacgaatatgtgatatcggggtactttcacaaattattattctgagtgtttttaattgtgatttcgttttcttcattgtgtttgttgttaactctgtctctttaatttttgtccagatatcacaaagctctccgaacgtttttatgactctcgttgtcaccatttttgccccagtgctggactggggaaaacgtcttaaatactcaaattcaccggagtttatttcatgaactatcagcgctcttaaatttccggcctttttaatattactgtttgtaatctcccagccttttaatgtttcccgacatcgttttcctcgaaacatgaaccagatgcgaatgtatctacctctaatctcgacacctgttggtaatttagacatatcatgagtctttgataaactgatttatctttggatagttgtaccagataatccctcgtttgctgtctggcttacctaaaggagatactcgtttgaagtggaagccctccacccaacagttctggcggtatgcttcaatttgtctggcccccagaccagtgcgaagcatcaggccgtattcaaccatccactcttcattaaagattacttgtgccatcgcatcacctctggcaggcgccaatgttagactgaaattgacgcccgatgttgattattaataatcagctatgaagttttaatttgaatacaatgcaattctcgaggactgaagtttctcgcaattaaaatttatcagttttactttctgctctctggaaacgcctgcttcttttttacctgagagcattttttcgcattctgatttcgttagtttagattttgaatatcttgtccagttagtaggagtgccaccttccttttcaatagtggcggtaattttatacatgaacacctccattattatttccagtggttcgtttattccatctttcgagtgcttctttttcacttccaccataaccggttcgggattcgcatccgttacacttcgctcggtaatatcctgaaatggctttcaccgttactgatggacaaccacaaaatggacatggtttaacattgtcatatctcataatttttctcataaaaaatatttcaagttggcggtgcattacaccgccaggctgaattattcctctgaattatcgattacactgtattccccggttaatacagaggaatctgcaggatcgattgtcagtggttccttttcatccattgatactgcacgctggatctcaattgatacgggcaaatatttgaacaggcgacgaatagccgttttctttgccatttcttcccagtgagttacccacggcccgttattaccagctttactcaggctgcgcaccagctcaatctgtttgcgcgtcataacttcaaactgagtacctccgtctttcagtcttgcgacagcatagacgtgggtaaccggggcatcttcgttttctcccgggcggtgtattaacttttcatcaaggccaaattcgaagctaaactcgtcaccttcacggacaacacgggctgacaggctggcgatttgaccagaacggcgagccagatcaatcatgccgcgatagccaatgattagctgaacgttctttttaccgctcttttcgtttttattaccaaaaggcagtaaatatgcatgaccgagggcgctacctggctcaagtccgagctgtgaacactgtacgatcgcactgacaaaactcatagtgtcacagtttcctaacgccggaactttacgaatttctgtggtggcgatacggatcatacgttcagccgtcatatggcgtggaagagctgctgccagttgctctttcattgatggctggttaataaaactaatcacgtcgctatttttaactgctgctggtgcacggtttccctgagttttttgcagatcggcttttgcgattggtggttgcttagtcatttgcatattccttagcccagcggggcagtgataatgtcttaatagctggccattcatcggtattcaggcagtcagacagggttcgcagattgcggtgatattcctgttgacctgccagttttgcttcttcgcccatcatgaaaatttcaaccggataacgtccgcattcaatagttgtgctggcaaccagaaaaacgaaagttggctgcactccaaactgtgcttcataaccgtcactgtagaatgcatcctgaacgtgatagcggtagtcgtaataagcggttttgaatcgttgaatatccgccgtagttttcacgtccatgatccagtgaaattcagggataattttgtccggacggcaccgacacaaaattcctgtttcaggatcttcccagtaaattgatgattcagcgtgtccggcgctttcaacaagccattgccccagcggcaaagccataacgctttgatacatgagttcaattttccggccttcttccgcagtgataaccgtttttcctgtgcttgcgcattccatcagaaacgctttctcttcttcttttccggcgtttgtacggcggttaaattcaggtgctacgataaagcggttactgaattcttccggttcaagtacccggcagtggaaagcagttcctaaatcgagcgtttttgtctttgtggtgtccacgggggcatttttacgccacaaatatagtgccggagtatcagcaatgtcatcgagctgagacttactgataccgggacccgcgtggtaattctcattcgaaattccgtaataaatacctggctctatgtcttctacgattacgggatctgcgacttcgccagtttcatcactgcaatcgcgatgcggatcgctgccagcattctcattgtgcggatgttcagcgccttccatttcctccggatcattttccttagcttcaacctgactctcttcatcgaatgtttcctggtatgttgcgtcgcccatcaccgcaccacagtcagggcagttatccccgccagtctggccgcaggcattgcaggctatttccggttcctgttgcactactggctcaggttgattcatatctgggctggttttttccgtttctggctggttctggtacacacaatcgcgagtctggatcccctttacccatttcggatcgttcgggtcgctaattccgtcaacaaattcaccacgtgatgcagcaagcaatttatcgtcatcgacaggattttttgatggaatgtttttccgggcttcatggagttctgcccgcagttcctgatatttcgcatcaacagaatttacctgtgactgagcatccagcggctgcgtgtcctgatgatgttcagttgcgtccggttccattgtttcagcctctccctgttcaactgccgttgttccagatggttgcggtttttcttcatcatcctgttttccttcttctgttactcgctgcggcatcggggcagaggagcgaccgcaggcaatatccacgatttccggatcagggttggcatgatcggtttcagtcagtactttgttcagatattcagtgacgtgcgcggggatgacctcgatcccaattggtgcttcttttacggacgcaaccacgatggcgcgggaataatccagcccgccaggcatggtgatgaatttgtcgcggaaaacagaaaagggcggtttattttcagcgataatttcctcaatgcgtttagcgtgtgccggatgaaggttatagatgtccagatccattgaacgggccagtacgccagtggctacgtcgcgcgccagtgacgtcagatcgtgtacgaaaccttcgccgcgatcggtgaggtttccgccgccagcattagcaccggaagccgtgcgagtgatgtgtgaaacacgattacccttcatccactcttttgtcagcagtcctcgatcggtgtagtcagcgttcaggtatgcttcgaaaaaagcagttatcagtcccaggtttgaattaccaggattagggaaaactttgtcagtgtcacgaaccagtttgtggagttcgcgaatttccagcgggtcgagcaggctggttttgtgggaaacagccagggcagtaacagccggtagttcttcagcccgagcaatgtgtaatgcctggagtccgtcgcgtgaaacgtgcgttaccggtttttcgctgccgtgttgagcaagccaacgaatgggcagttcctggccagaaattgggagtagcatattctcctcaatctcagtcatgtcttcgccgttgacgttggtattgccttgatagtgagcgttgtctggtgctgctcccggttttagttcccatgtcatggagtctttgctgagttgatagcgttcactccaggtaaaatcgatctcaccttcagcgggcaggtcattaacgacaggaaaattcgtggcaacagctttaaaatagctgctcagttttttacctgacttaacgatcaggtagtccagagtggcacaggtcgattcaaaatcgttgcttgcccacaggacgacgtcaggttcaccggatgattttttcgctttccgtaacaggaagagtggttttgtgctcattgttttttaacctcaactcagattaaaattcgttttgttcagtgaatgatcttgccggatacacactgttcatagcctgcgccatacgcaggctatttctttcagatttcaccttttaatttcattgcaattagagttgccagaaattcggcttttttttctgcgggcagattctttccgatatgcaccaggcacatttttttgacaccttcatcaagtgtttttacgttgcctgatggaccatcgatatcaaccacagtgaatggggtttctttattttctgttttaattacgtagccaatgcgctttccttccagattcacctcgtgaacaatgtcatcggtagttacaacagtggcttcataattggtaatcatgtttttctccttaattaaggttgagcgaatacctgccatttctggcataaattcagtttcgaatagtcaattaattaaagttcatgtgccatctggtctttttcggcacaagcttcactgcaatattttctcggttcgtcttttgataaaatcccgtgcatgaagtgaagcattctttcaatagctttgctttcttcaacgtcttttttgcaaaggtggtaagcacattttattttcttagtcatcaccatgactccgcctttacaggtaaaccatcacgaccgaggaagactttaatcatgcggtcagtaatgaatgtttttgtggtcaggttacgaatatatagttttcgctttttaatattgtttgccgaggcaatatatgtccggccttcatgaagaacataatcgccaggagtcacacactgacgtggtatttcatcagttccgaagtgatgtgcaatcataattatctccatttttacaaatgaactttgttgatgcggtgtctggtgcctccaggtgactgcaaccagttaacaattacagtcggctttcccacccaaaccaataaggactaacatgacttttaactgtgccacgtgcgcttagccgcattcaccgcatcacaaaattcactttaaaaagggcggacatcagccgaacttcaagaaaaaaactgatgccgccaggactacacacagcaatgtcgttatttacaaccggaggcgcactcccaccatttaaatttaacagacaagaccgactctttatggatatcggaaatgcgccttcgtgttgtgcccggttttatttcaccacctccgggcttcggtggtctcggctatacccctacagcgagagcttgtgttaacatttcaatacccttacagttgagagttattgatatgttggatgtatttactccattgttgaaactttttgctaacgagccactcgaaagacttatgtatacgattatcatttttggtctcactctctggctgataccgaaagagtttactgtcgcattcaatgcttatactgaaataccttggctctttcagattatcgtttttgccttttctttcgtggtcgccatttccttctcaagattgcgagcacatattcaaaagcattattcattactaccagagcaacgagtattgcttcgtttatctgagaaagaaatcgctgtatttaaagatttccttaaaacaggaaatcttattatcacttctccttgccgtaacccggttatgaaaaaattagaacggaagggcatcattcaacatcagagtgatagcgcaaactgttcttattatctcgtcaccgaaaaatactcccattttatgaagttattctggaacagcaggagtagacgttttaatcgttagcttactgtgtgcttctccaaccatcggcgcgcaccagtttcggttttaaatgttttgcttttggtatacgtcatggcagtgaacgttccatcctggttggggaacacgccgcacaccagggattcgttgttgccgaggtcgattttttgcattttgcgaatctcacatcttgttgctacgtatagcgacttctgcctgccagagatcccagtcgttgctgcgtaaagcctgcacagcctggttgtaagtgataccgcaacaatccatcaaatactgaactacttcgtaatgcaccatcttatctctccccttaacgccgggtggcggaactaactgctgcactgcaaaatttgaatcccgccgtcatgttcatacgcctcgggctggctacttaaccccttaccactgcctggtaactcgaagtattgcccggcgttctgtggggcggggtgggtggtatgctggaactataggtaatgcctaattgattgtcaataggctatgcctaatgttttgagcgtaacctaataggtgatggcgacagcagaaagtgatgggggggttaaataacggaatccaggagttttccgtcagaccatataagtttaagttccagtttttgtgatgttctggcttttccgttcagattcaagagctttcagatacttacccactttcatttccatcgctgctatgtaggcgcgaacatcgtggtcaacccaatctggttctgtagcatttccagataacaggaaagctacaatcgctcttatttcatcagaggctgcttgataaaggttgtttatatctaaaagttcactttttgtatctgaattggtgggggttggtatggggtattcgttaagcccccaatgctctggaccaacaacatcagaaaagaaacgccataattctggaagtttatctttacttatagagcctttcttaatccagtcataaattgatggtggttggactttaaagtggcgtgcgacctccgcctttgatttgacggatcccgatgcgatttttttgttaatggcctgctctatcgctcggcctaagtctttaccactaagcattgcttaatattctcctatgcgcattacattaggcaatccctacccttactgcattaggcacagcctattgacaattgcgttaggcgtcgcctaatatttctgtgtgtttttggagttcattcgatgaaaaaagagaactattcattcaagcaagcttgtgctgttgtcggtgggcaatcagcaatggctaggcttttaggtgtatcacctccaagcgtaaatcaatggatcaaaggggtacgtcaattgcctgccgagagatgtccagcaattgaacgtgcaacaagaggtgaggttctgtgcgaagaacttcgtcctgatattgactggtcatatttacgacgttcggcatgttgttcgcagaatatgtcagtgaagcaactaaatgacagtaacaaatcctcatttgatcatacctgaaacatcaagaggcaaatgattcatgaaaatcaagcatgagcacatcgaatcagtgttgtttgccctagcagccgaaaaagggcaggcatgggtagccaatgcaattactgaagaatatctgcgccaggggggcggcgaattgcccctggttccaggcaaggactggaacaatcagcagaatatctatcaccgttggttgaaaggtgaaacgaaaacgcaaagagaaaaaattcagaagctgatcccagcaattctggcaatccttccgcgcgagctgcgtcaccgactctgcatcttcgataccctggaacgccgtgcattactggcggcgcaggaagcgttaagtacggcaattgatgcgcatgatgatgcagtccaagccgtttaccggaaagcgcatttcagcggcggcggttcttccgacgattctgtcattgttcattaagcaaaagtttccatgctgtttgtgcttattctaagccaccgggcagcatcatacggggcaattatggccgcattaccatacatgcaactgtacatagctgattacctggctgacaccatgcatttgtcagcagaggagcatggtgcgtatttgttgctgatgttcaattactggcaaacaggaaagccaatacctaaaaacaggctggcaaaaattgcccgtctgactaacgagcgatgggctgatgttgaaccatccttgcaggagtttttttgcgataacggcgaggaatgggtgcatcttcggattgaggaagatctggcatcagtcagggaaaaattaaccaaaaaatcagccgcaggaaaagcatctgttcaggccagaagaagcagaaaggaagcagatgttcaaacaaaacaagagagaaatttaacaggtgttcaaacagatgttgaagtggtgtttgaacatgatgtcaacacaaaggcaactaataaagatacagataaagatctaaaaacagatccccccctaaatcccccccgggggaatcgaggtgtcaaaaagtttgaccctctggatattactttgccgaactggatttctgtctcgctttggcgtgagtgggttgaatttcgccaggcattgcgaaaaccgattcgaacggagcagggcgctaacggggcgatacgggagctggaaaaattccgccagcagggtttttcacctgagcaggtgattcgacacagcatcgccaatgaataccagggcttgttcgcgccgaaaggtgttcgacctgagacgttactccgacaggttaacaccgtctcgttaccggatagtgcgatcccgccaggcttcagggggtaactgaccatgaaaaatattgcgacaggcgatgttcttgaacgtatccgcagactggccccgtcacatgtaaccgcgccattcaagacggtagcggagtggcgcgagtggcaactttccgaaggccagaaacgttgtgaggagatcaaccgtcagaatcgtcagttgcgggtggaaaaaattctgaatcgctctggcatccagccattgcaccgcaaatgctcgttttcgaattaccaggtgcagaacgaagggcagcgatacgcgttgagtcaggcgaaatccatcgctgatgaactgatgaccgggtgtacaaattttgcgttcagcggaaaacctggtaccgggaagaaccacttagcggcagctatcgggaatcgcctgctgaaagacggtcagacagtgattgtggttaccgtggctgatgttatgagtgccctgcacgccagctatgacgatgggcagtcaggcgaaaaatttttgcgggaactgtgcgaagtggatctgctggttcttgatgaaattggcattcagcgcgagacgaaaaacgagcaggtggtactgcaccagattgttgatcgccggacagcgtcgatgcgcagcgtggggatgctgacaaacctgaactatgaggccatgaaaacattgctcggcgagcggattatggatcgcatgaccatgaacggcgggcgatgggtgaattttaactgggagagctggcgtccgaatgtcgtccagccaggaattgcgaagtaatttttaccgggagaaaaatttaatggagactgtttttgacgcactgaaagcaatgggaaaagccacatccatagaacttgctgcgcgacttgatatcagtcgtgaagaagtgctgaacgaactatgggaactgaaaaaggctggttttgttgataaaagcgcgtacacctggcgtgtggctgataacaatgttcagcaggaacagccagcgcaggcagaactgccggaagaaatcaccacagcaacagtagcgaaaatctcagagtgcgatttaaccgcgacgattgaacaacgaggaccacaaacggctgatgagctggctacattgtttggtaccacatcacgcaaagtggcttcaacgctggcaatggcaatcagcaaaggtcgtctgattcgcgtaaatcagggcggtaaatttcgttactgcataccgggcgataatttaccagcagagccgaaagcagcatcggtatctccgctctggttatctgcatcgtcgtctgcctgtcatggggtgttaatcattaccgtgataacgccatcgcctacaaagaacagcgcgacaaaaatgccagagaactgaagctggcgaacgcggcaattactgagatgcagatgcgtcagcgtgatgttgctgcgctcgatgcaaaatacacgaaggagttagctgatgcgaaagctgaaaatgatgctctgcgtgatgatgttgccgctggtcgtcgtcggttgcacatcaaagcagtctgtcagtcagtgcgtgaagccaccaccgcctccggcgtggataatgcagcctccccccgactggcagacaccgctgaacgggattatttcaccctccgggaacgactggtaatgatgcaggcccaacttgaaggtgctcagcaatacataaccgagcagtgtttaaagtaaaatcttaactacaatatgattcattttgatgattgtttcataaggaacagtgaagtaagatctaagaggagttaaattttatacagtataatcataatattgcagcaaggtggttataattgaaagaatatttagatatgaatacatctcatgtaagagttgttactcatatgtgtgggttcctggtttggctctatagtctttcaatgttgccaccaatggttgtagcattgttttataaagaaaaaagcctgtttgttttctttataactttcgttatatttttttgcattggtggcggagcgtggtatacaactaagaaatctggcattcaattacgtacccgtgatgggtttattataattgtaatgttttggattttgttttctgttattagtgcattccctttatggattgactcagaacttaatttaacgttcattgatgctctgtttgaaggggtttctggaataacaacaacaggagcaactgtaattgatgatgttagttcattacctcgggcatatttgtactatcggtcacagttaaattttataggtggtttaggagttattgttctggcggttgctgtattgccattattgggtattggtggtgcaaagctttatcagtcagaaatgccggggccatttaaggatgacaaactcactccccgcctggccgatacgtcacggacactgtggataacttattctttattaggtattgcttgtattgtctgttatagacttgcaggaatgcctttgtttgatgctatttgtcacgggatttccacagtttcgcttggtggtttctcaactcatagcgagagtatcggatattttaataactatttggttgagctggtggctggttctttttccctgctatcggctttcaacttcactctttggtatattgttattagcaggaaaacgataaaacctttaatcagagatattgaacttcgtttctttctgttaatagccttaggggtgatcattgttacctctttccaggtctggcatataggtatgtatgacttgcatggaagttttattcattcgttttttcttgccagctccatgctcactgataatggtttagctacgcaggattatgcaagttggcccacgcacacgatagtgtttttgctgttgtcaagtttctttgggggatgtataggttcaacttgtggtggaattaagtcacttcgatttcttatacttttcaaacaaagcaaacacgagataaatcagctttctcatcccagagcgttgttgagtgtaaatgtaggagggaagatagttacagatcgtgtaatgaggtctgtatggagtttcttttttctttatactctcttcacggtgttttttatactggtgttaaatggtatgggatatgattttcttacatcatttgcaacagtggctgcatgtattaataatatgggattaggttttggggctactgcatcgtcattcggagtgcttaatgacattgcaaaatgcttaatgtgcatagctatgattcttggtcgccttgaaatttatcctgttattatattgttttcaggttttttttggcgctcctaatatatggctgatttataattgtgagtttaatattatgttgactcactcattgatccaatacctaactttaccagcaacacctccgtccccagtagcactggctgctggggtgcgttttattcataaagcaaggctgtatgagcgagaaattaaagatagtctatcgcccattacaagaattgtcaccgtatgcgcacaacgccaggacgcacagtactgagcaggtggcacaactggtagaaagtattaagcaattcggctggactaatccggtgctgattgacgaaaagggcgaaattattgcgggtcacggtcgtgttatggcggctgaaatgctcaaaatggattctgttccggtcattgttctgtctggcctgacggatgagcagaagcagcgataacgatcagtatcgctcccgtaatgcattaatccgtcgccacattgagaaaatggatgccagtttgcacgtcggaacgaaggagtttgatatttcaaaggtttccgaggtggattctgttgatgatttactcattgataatgccgctcgttatctgctgaaagactggaaaggggttggtgaactggttaatggtgttgaggttgcactggaatatacggcagaacgagggatcgcgctgcttaagcagaatccagagttgtactggcagatccttgcagaagcagccagcatcgcccagggtaaagagcagcagaagcaggatacgataaaaaagccatagctgcccagcggtggttatcggagttcgggggagaaaggggggaaaaggcaagatggaagcgagaaaaactcaggttgccaccgataccggaaccagaaatagacccggtgcttaaggagttgttgtacgcctattcggtaatatcccgtgcccgacgttatgctggaatggctggggtgcctttgcctttatctctgacagagataaatgaatatttagccactcatccggtattgattgagcgcgatgaatttgaagcagtgatctttgcactggatgaccagtattttcaggagcagtgtgtgtagttgttaattacgtacactctgttacagagatgtgatggtgtctttaattaaatcgatgatgctcctggagaaaagcattgcgtggcctcgtaatcgctatatctactattatgtcgcctgaaacccacttcgcggtgggttttttgttgtcaggagttttaataaatggcagagcaaacctcgcgtctcgcaataattattgatagcactggagcgaaaaataatgctgacaatctgacctcctcattagtcaaaatgacgcaggctggggaaactgctgcaaatagcgcagggaaagtgactaaggcaacagaagatgagaagaacgcgctcgcaaaattaaaagcagctattgatccagttggtgccgcaattgatactgtcggtcgacgctattctgaattaaagaaatttttcgataaagggcttattgataaagaagaatatgaatttcttgtccgtaaacttaatgaaaccacagaggaattgagcggggttgcgcaagcgcagagagaagccgagaaggccggaaaacttgctgccgctcagcaggaagcgcaggctcaggcctttcaaagaatgctggacaagatcgaccctctggctgcggcgctaagaaatcttgaacaacagcatgatgaacttaatgctgcgtttgcatccgggaaaataaatggttctcagtttgagaattatagccgaaaaatacaggaaacacggcgagagcttaccggagaggctcaggcagagcgagaagcagcaaaagcgcatgatgaacaggttgttgctttgcaacgtctgattgctcaacttgatcctgtcggaactgcttttaatcgtctggtagaacaacagaaacagctcaatgaagcaaaagctaaggggatgctttctcctgaaatgtatgaggagctttctggaaaacttcgtgctatgcggagtgagcttgaggttactcaatcacaattaagcaaaaccggaatgtcggcaaaacaaacggcttttgctatgcgcatgttgcctgcacaaatgacggatattgttgttgggttgtccactggtcagtcgccatttatggtgttaatgcagcagggcggccattcagctatgcaggagacaagaatcgccagcttacccgttacagcgatacccgctggcatgaagattccgtgcgtaaccgctggttcagcgtgatggtggggccgtctgtgcgcgtgaatgaatggttcagcgcgtatgcgatggcgggtatggcttacagccgtgtgtcgactttctccggggattatctccgcgtaactgacaacaagggaaggtgcgaataagcaggtcatttcttcccaagctgactcgctgattaaaatttcgcggatctgggccgatttttttcccgcaaacacatcgaatcagcctatttaggctattttttccaccatttctggcgttatttccggtttttactgagatctctcccactgacgtatcatttggtccacccgaaacaggttggccagggtgaataacatcgccagttggttatcgtttttcagcagccccttgtatctggctttcacgaagccgaactgccgcttgatgatgcgaaacgggtgctccaccctggcacggatgctggctttcatgtattcgatgttgatggccgttttgttcttgcgcggattctgcttcaaggtttttaccttgccgggacgctcggcgatcagccagtccacatccacctcggccagctcctcgcgctgtggcgctccttggtagccggcatcggctgagacaaattgctcctctccatgaagcagattacccagctgattgaggtcatgctcgttggccgcggtggtgaccaggctgtgggtcaggccactcttggcatcgacaccaatgtgggccttcatgccaaagtgccactgattgcctttcttggtctgatgcatctccggatcgcgttgctgctctttgttcttggtagagctgggtgcctcaatgatggtggcatccaccaaagtgccttgggtcatcatgacgcctgcttcggccagccagcgattgatggtcttgaacaattgacgggccagttgatgctgctcgagcaggtggcggaaattcatgatggtggtgcgatccggcagggcgctatccagggataatcgggcaaacaggcgcatggaggcgatttcgtacagggcatcttccatggcaccgtcgctcaggttgtaccaatgctgcatgcagtgaatacgcagcatggtctccagcggatagggccgtcggccattgcccgccttgggataaaacggctcgatgacagcggtcatattctgccatggcagaatctgctccatgcgggagaggaaaatctcttttcgggtctgacggcgcttagtgctgaattcactatcggcgaaggtgagttgatggctcatgatgtccctctgggatgcgctccggatgaatatgatgatctcatatcaggaacttgttcgcaccttcccaaggggaaaacgcacgacgtgctgaccggaagtgatgacggtcgccacagcaacacgtctctggcgtggggagctggcgtgcagtttaacccgaccgaatccgtggccattgatattgcttatgaaggccccggcagtggcgactggcgcactgacggtttcatcgtgggtgtcggttataagttctgattagccaggtaacacagtgttatgacagcccgccggttcaggcgggcttttttgtggggtgaatatggcagtaaagatttcaggtgtactgaaagacggcacaggaaaaccggtacagaactgcacaatccagctgaaagcaaaacgtaacagcaccacggtggtggtgaacacgctggcctcagaaaatccggatgaagccgggcgttacagcatggacgttgagtacggtcagtacagcgttattctgttggtggaaggattcccgccgtcacatgccgggaccattaccgtgtatgaagattctcaacccggtacgctgaatgattttctcggtgccatgacggaggatgatgcccgtccggaggcactgcgccgttttgaactgatggtggaagaggtggcgcgtaacgcgtccgcggtggcacagaacacggcagccgcgaagaagtcagccagtgatgccagcacatcagcccgtgaggcggcaacccatgcggctgatgctgcggactcagcacgcgcagccagcacgtcagccggacaggccgcgtcgtcggctcagtcagcgtcttccagcgcaggaacggcatcaacaaaggccactgaagcatcaaaaagtgctgccgctgcagagtcctcaaaaagcgcggcggccaccagtgccggtgcggcgaaaacgtcagaaacgaatgcttcagcgtcactacaatcagcagccacatctgcatccaccgcgaccacgaaggcatcagaagctgcgacctcggcccgggatgcggcggcctcaaaagaagcggcaaaatcatcagaaacgaacgcatcatcaagcgccagtagtgcagcttcctcggcaacggcggcaggaaattccgcgaaggcggcaaaaacgtccgagacgaacgccaggtcttctgaaacggcagcgggacagagcgcctcggctgcggcaggctcaaaaacagcggctgcgtcgtctgccagtgcagcgtcaacaagtgccgggcaggcctcagccagtgccaccgccgccggaaaatcggcagaaagcgccgcatcgtctgcttcaacagccacaacgaaggctggcgaagccactgaacaggccagcgcagcagcgaggtctgcttccgcagcgaagacatccgaaacgaacgcgaaagcgtcggaaacaagcgcagaatcctcaaaaacggctgccgcatcgtcagccagttcggcggcgtcatcggcatcatcggcgtctgcttcaaaagatgaggcgaccagacaagcgtcagcagcgaagagcagcgccacgacggcatccacgaaggcgacagaggctgctggcagtgcgacggcggcagctcagagcaaaagtacggcggaatccgcggcaacgcgcgccgagacagcagctaaacgggcagaggatattgcatccgccgtggcgcttgaggatgcaagtacgacgaaaaaggggatagtacagctcagcagtgcgaccaacagtacgtctgaaacgctggcggcaacgccaaaggcagtaaaatcagcctatgacaatgcagagaaacgtctgcagaaagaccagaacggcgctgatatacccgataagggatgcttcctgaacaacattaacgcggtcagtaaaacagactttgctgataagcgtggtatgcgttatgtgcgggttaacgctcctgcaggtgcaacatctggaaaatattaccctgttgttgttatgcgttctgctggctcagtaagcgaactggcatcaagagtcattatcaccacggcaacgcgaaccgcaggcgatccgatgaataactgcgagtttaacggatttgttatgcctggtggctggactgacagggggcgttatgcttatggcatgttctggcaatatcaaaacaatgaacgagccattcactcaataatgatgagtaataagggcgatgatttgcgctctgtgttctatgttgatggcgctgctttccctgtttttgcgtttattgaagatggcctgtcaatatccgcacctggtgctgatctcgttgttaatgatacgacctataagtttggggcaacaaatccggcgactgaatgtatcgcggcggacgttatccttgattttaagagtgggcgtggtttttatgagtctcattcgttaatcgttaacgataacttgtcgtgcaaaaaactttttgccacagacgaaattgtagcgcgtggtggtaatcagattcgaatgataggtggggagtatggtgcattatggcgtaatgatggcgctaaaacttacctgctgcttaccaatcaaggtgatgtttatggtggctggaatacattaagaccgtttgctattgataacgcaaccggcgaactggttattggaaccaaactgtccgcaagtctgaacggtaatgcattaacagcaacaaagctgcaaacgccaagacgggtttctggtgttgagtttgatggttccaaagatattactttaaccgccgcgcatgtggctgcttttgccagaagggcaacggatacatatgccgatgcggatggtggcgttccatggaatgccgaatctggcgcttacaatgtcacccgctctggcgacagctatattctggttaacttctataccggagtcggaagttgccggaccctgcagatgaaggcgcattacagaaatggtggtctgttctaccgttcttcaagagacggttatggttttgaggaagactgggcagaagtttatacctcgaaaaatcttccaccagaaagctacccagtcggcgcaccaatcccgtggccatcagataccgttccgtctggttatgccctgatgcaggggcaggcttttgacaaatctgcttacccgaaacttgcagccgcttatccgtcaggcgtgatccctgatatgcgtggctggacgattaagggcaaacctgccagtggtcgggccgtattgtctcaggaacaggacggcattaaatcgcatacccacagcgccagcgcatccagtacagatttggggacgaaaaccacatcgtcgtttgattacggcactaaatccacgaataacaccggggcacatacacacagtgtgagcggctctacaaactcggctggagcacacacacactcactagccaacgtgaacacggctagtgctaactccggtgctggtagtgcatcaacaagattgtctgttgtgcataatcaaaactatgcaacatcatctgctggcgcacatacccactcactgtccggcactgctgcaagcgcaggtgcacacgcgcatactgtcggtattggtgctcatacgcactccgttgcgattggttcacatggacacaccatcaccgttaacgctgctggtaacgcggaaaacaccgtcaaaaacatcgcatttaactatattgtgaggcttgcataatggcattcagaatgagtgaacaaccacggaccataaaaatttataatctgctggccggaactaatgaatttattggtgaaggtgatgcatatattccgcctcatacaggtctgccagcaaacagtaccgatattgcaccgccagatattccggctggcttcgtggctgttttcaacagtgatgagtcatcgtggcatctcgttgaagatcatcggggtaaaacggtttatgacgtggcttccggcaacgcgttatttatttctgaactcggtccgttaccggaaaatgttacctggttatcgccggaaggggagtttcagaagtggaacggcacagcctgggtgaaggatacggaagcagaaaaactgttccggatccgggaggcggaagaaacaaaaaacaacctgatgcaggtagccagtgagcatattgcgccgcttcaggatgctgcagatctggaaattgcaacggaggaagaaatctcgttgctggaagcatggaaaaagtatcgggtattgctgaaccgtgttgatacgtcaactgcacaggatattgaatggccagcactgccgtagggtaaaacatataaattctataattagatgtatctttccatttacggcaaggaagggggcttggaagacgtaaagcatctcacaccgagattattttttatatgtcaggtgtctgaagttttgctttggctcttaaaatggtttgccgcgaggttttgaattcccgggcaatggcacttatacttacacctgacttaattcgttcgaataccacctgtttctgttcttcatttaacacaggaggtcgaccaaaacgtttccctgcgccgcgggctcttactatcccggaatgagtgcgttcaagtaaaaggtctcgttcaaattcagcgactgctgaaattacttgcatcatcatttttcctgttggactggtcaggtcaatgccacccaatgctaagcaatgcactctgatacctgtttcggtcagttgttccactgttttcctgatatccattgcattacaaccaaggcgatccagttttgtcacaatcaattgatcaccacatttcaggcgagcaagcaaccggttaaaaccaggacgctcactggttgctgctgagccgctaatgtgttcttcgattatttgctgaggtttgattttaaaacctgcactttcgatttcccggcgttgattttcggtggtctgatccagcgttgatatccgacagtaagcaaaaattcgagacatagtgagactctatacgaaattggtgttcatatcataatgcatctcagaaaataattatgattatttttgtgcatatttgtatgtacacgttcgaaaataaacgaatgcgtatgcaaccccgtaattttggtgagacccaaaatcgattttgtgaaaaatggctttaactcggtttgtttttcgagttccgggcggactcaaggaagaagaatagtgttgcgtgttattttaaccagatttcaagttgtttggtcgtggaaaagtggagcaaaatgttgttaaagtggaaaaatgataaaaaagtaagtttattatattacattttaccatttaaattttggttgtctttaagaactgatatcgctgtttgtaataattctttgttatccagccatgatgttttctttatgtttccttcaatgtaatcaagcaatgttctggtattgataggtcttccctgttttgctacttccactacagcatcccctaggataattcttacttcaggaagctgcgcagggaaccactttagggtgtcttttgatttcatgaagatattccttaaaatattattgattttcattgcgatattgtatgtctgattcaggatatgttgacttatacatcggttttgtctgggttattggatatgccaatccctaattttattagagcatgactaaaaatgctgaatatgataaggagcgaagtgattatcagtatgctgttcatatagcctcgaattagtaatgtgttatatatgatatagttgacaatttttatcctgggtgttcttaaagttcgtagataaacattgtcgtttcaggtatacaggaatgctaacaggtggcggcaaaaatcaggcggtttatggcgcaagctgaagtggcaactgcaaactatcttatgcagagactctacacggattgggtttaaaagtatacatagataacagtttttatctgaagaagaaaaatatcaaggtgatatagcctatatgcctttgatgcggaggaatgaatgtgatgggagtgatgtatctgaatagttgaaaaaccgcagtcacgtcgtatgcaagaacgtgctgcggttggtttgactttgattgagacgttttggaatttttttcggtggcaaaaatggggcaaaacgctgcaaaaggggcaaaaaaggggcaaaaaaagagtggattatcgtagcttattgttgtcgctgatgatatttaacacattgaaaaataagtaaaatacttatgagtcagagagttgtgatttttgcccttacttgttcaggttgtattgttctttcttactaatttcttgattttgcgacatttaaaagcgactcaattcgttatatggcatcagaagagtatgcgtcatgccggaacgcccagcataagaaatctgatataaaaaactgtggcgtgtatggtacggattagaggggaaaatgtcagcacatttgcgaaatgaatcaaaaagcccgcagcaatgtgcgggcgttagtgtcagcgcacaaccagcacggagcactctgcgtgacgcactacagctgcggcgttggaaccgagcagataagtggtgatatccggtcgatgggaagcaatgatgatcatatgagcggggatcttcttcgccaattccagaatgcggtctttgggcgagccttcctcaacatggacatgcactctgtcggttggcagtttaaattttttaatgatctcttccagttgcgatttggcttccgctttcaggtcatccattgccggtaattctgcggaatacgctaaacccagagaggcatagtagggcagtgaaggtattaccgtcaggaaatgaacctctgcatcatcaatctttgcctcttcctcaacgtggctaatcacgcgttgagttaattctgaatcggaaatatcgatagggacaagaatcgttctgttcataaaacctcctgttttagtatccgcataaagtgtaacgccagatgacactttttgtgtaatgacggagttcacatttttaatttagatcaaaggaggaagaataagcagaaaaagcccgccataacagcgggcaggaggatttagaactgataaaccagacctaaagcgacaatatcatcggtagagatgccattggcagcgtagaagctgtcatcttcatccaacaggttgattttatagtcaacgtaggtggacatgtttttattgaaatagtaagtcgcgccaatatcggcgtatttaaccagatctttatcatcaacacctgccgggttgtctgcaccacccgcagcgtgcaggtcacggcctttagacatcaggaaagagactgccggacgcagaccaaaatcaaactggtactgtgcagtgacttcaaaattctgggttttgtttgccacagcataatcgctgtcgccaaacggggtcatattacgcgtttctgaatacatggttgccaggtaaatattgttagcatcgtattttagcccagcagtccacgcgtctgctttatcaccacccgccgcagtatggttaacctggtcattggtgcggtcagaagaggtgtatgccgcaccagcgctaaagcccatgcctaaatcatatgttgtggaaagaccccagccgtcaccgttttcatggcgaacatcacgtccgttgttggtgccttcctgaccattactggctccttcgttgttaccttgatactgcaccgcgaagttcagaccatttaccagaccgaagaaatcagtattacgataagtcgcgacgccattggctcgaccagtcataaagttgtctgcattggtataagagtcaccgccaaattcaggcagcatatcggtccagccttcgatgtcgtacattacgccataattacgtccgtaatcgaaagaaccgtaatctgcaaatttcagcccggcaaatgccagacgggtccatgactggttttttgaagattcagtgttgtttgcctgaatattgtattcccattgaccgtagccagtgagttgatcgttaatttgggtttcgcctttaaaacccagacgcgcatagctctggtcgccatctttcgctgaattatcagaaaaataatgcaggccatcaactttgccatacagatctaatttgttgccgtctttattataaacttcggctgcatgtgcagcacctgcggcgagcagggcaggaattaaaagtgccagtactttgcttttcattgaataaatcctttagttattttatttgccttttatccccatttcggggagtgaaaacatcctaaaggagaagttcagttagccgataaatatcatttgttacgccttaagtaaaaccttaatcaaataattcctctgaaatgataataagtctggtgaatgtatcgaagataatacatacaaaataaaaattatacttttaatttgctatacgttattctgcgcgggttatatgcctttattgtcacagattttattttctgttgggccattgcattgccactgattttccaacatataaaaagacaagcccgaacagtcgtccgggctttttttttagaattggataatccttatccagagcatttaatcggtgttgcttttttccgcttttccggccatttgtgccaggaagtcatagcgtttttgcaaatcagctgcagcatctttccataactgttctgccacttctggctgctgcgaattcagccgacggaaacgttgctcgtgaagtaacgtttcttccggtgcttctgacggcgggcgtgaatccaaggccagcggcagtttgccttcatcggcacgacgcggatcaaagcgatatagcggccagaagccggtagctgtgagttggcgcatctggtcgtggctgagtgccagatcgtaaccatgctcttcacacgggctataagcaatgatcagcgatggccccggatacgcttccgcttcctgaatcgctttcaccgtctggttcagctgcgcgccgagagaaatctgcgccacataaacatgaccgtacatcatcatactgacgccaagatctttacgcgctttacgtttgccgtgctcgccaaatttagttactgcacccagcggtgtcgctttcgacgcctgaccaccggtgttggaatagcattgcgtatccagcaccagaatgttgacgttttccgtcaaactcaatacatgatccagaccgccaaagccgatatcgtaagcccagccatcaccaccaatcagccagattgatttttccaccagtgcatctgcatcacgtagcagttcatgtgcttcggcaacatcgttgagttgctggcgtaaagctgcaacctgttcacgacgaacctctggcgtggcgtctgatttcaacgccgtcagtaattccgccgggattttatcggcaaattgatccagcagacgcagcacgcggacacggtgttgatcgaccgtcaggcggaaaccaaggccaaattcggcattatcttcaaatagagagttcgcccatgccggcccacgaccgttggcatcggtggtatacggtgtagagggcaggttaccgccataaattgaagaacagccagtggcgttagcgatcaacatccggtcgccatagagctgagtcagtaatttaatatacggcgtctcgccacaaccggagcaagcacctgaatattcaaacagcggtgtaatcagctgcgatgtacgaatatcaatacgttccagtttgctacggtcgatttctggcaggttgaggaagaaatcgtaattgattttctcttcttcgacatgttccaggcgagacatcatattgatggctttaatctctggattctgacggtctttcgccgggcaaacttcgacgcacaggttacaaccggtgcaatcttccggtgccacctgcaagacatatttctgcccgcgcatatcacgcgatttcacatccagcgaatgcaggctggcaggggcgttttccatcgcttcaggcggcaccacttttgcgcgaatagctgagtgtgggcaagcggcaacgcagtggttacattgggtacagagttcctctttccagatggggatctcttcggcgatattgcgtttttcccagcgcgtagtgcccatcggccaggtgccgtctggcggcagcgccgaaacggggagggcgtcaccaagcccggcgagcatcgcagcggttacggttttcacgaaatcaggggcggcatcggaaaccactggcggtcgattggcgctgtgcggatttaccggttgcaacggaacttcttctacggattcacgcgccagcgccagagcctgccagttgcgttccaccagatcctggcctttgctactgtaacttttggcaatcgcaccctgcaattctgcgagggcgctatcgccaggcagaatttgcgtcagatggaaaaaagccatctgcatgacggtattaatacgggccgccaggccacattcgcgggcgattttcgccgcgttaatcacatagaagcgcgcttttttctggtttaacacggcctgaacttcttgcggcaagcgcgaccacacttcatctgcgctgtacggcgtgttgagcaggaaaatgccgccaggttttaaacgctcagccatctgatatttatcgataaactgcaactggtggcagccaacaaaatcagcctgggaaatgagataagcggaacgaatcggctgttcgctcactcgaaggtgagaaaccgtcaggccgcccgcctttttggagtcgtaaacaaaatagccctgtgcgtaccacggcgtggaattaccgataatcttgatattgtttttggtcgcggaaacgctgccatcactaccaaggccataaaacaaggcttccagtttcgccgagtttggcagggtgttttccggcaacggcagtgacagattggtcacatcatcgtaaataccaaccgtaaagcgcgctttcggtttagccgcgttgagctcggcaaataccgccagtacacagtctgggccaaattctttggatgaaagaccatagcgcccaccaatgacacggggcagagtttcgcgctcgccattattaaaggcttctgccagtgcggtcattacatccagatagagcggttctgcctgggcaccgggttctttggttctgtccagtaccgccacgctgcgtacggatcccggcagagcttgcagtaaatgtttagcggagaaggggcggtacaggcgaactttcagcacgccaactttttcgccacgggttagcaattcatcaaccacttcttcacaggtgccaatggcagagcccatcaggataatcacccgttccgcttgcggatgcccgtaatattcaaacggctgatactgacgacctgtcgcggcagagaaatcattcatcgcctgttcaacatggtcatagaccgcgttgtaccatgggttggtggcttcgcgagactggaaataagtgtcaggattggcggacgtaccgcggatcaccggatgttccgggttgagtgcccgggcgcgatgagcatcaatttcgacctgcggcatgagatcaagaatcgtgtcatcggccagcgggacaattttattgatttcgtgggacgtgcggaaaccatcaaagaaatgaataaatggcacgcggcttttcagcgtcgcgatttgcgaaatgagagcaaagtcttgcgcttcctggacgtttgctgcacacaacatcgcgcaacccgtctggcgcaccgccataacgtcggaatgatcgccaaaaatagagagtgcatgtgtggcaacggtacgtgccgctacatgcaggacaaacggtgttagttcgcctgccagtttgtacagcgtcgggatcatcagcagcaaaccctgcgatgacgtaaacgatgttgaaagggcacccgtctgcaaagcgccatgcacggtagcgatagcacccgcttccgactgcatttcaaccacgcgtggtgtgtctccccaaacgttctttaagccgtttccggcccaggcatcagcctgttctgccatcgtggaactgggggtaatagggtagatggcgataacttcactggtgcgaaatgcgaccgaagcaaccgcgccattaccgtcaatagtaatcatatgacacccttacattgcgcaaatgaggggcgcacgaaattgctgcgcgcccagtagtaatctttcaattttagcaaatggctttcttctgcattttcgcttttgtgtcccccacatcagcgtaatgaatgttttgatcaaacagagggcaaaaaaatagccataaaaaagtaaaaatgcggggcaacgcgcaggacagctctcgacgccgccctctgtgctgcctattatttatggcggtgtcgtttggcttgaagatcagaggaagaaaagatgcgagcagcgttttgggtagggtgtgccgctttattgttgtcggcgtgtagtagtgaacctgttcagcaggcgactgccgcgcacgtagcgccaggtttaaaagcgtcgatgtccagtagtggagaagcaaattgtgcaatgatcggcggttcgctttctgttgcccgtcaactggatggtacggcgattgggatgtgtgcattacccaacggcaaacgctgtagcgaacagtcacttgccgccgggagctgtggcagctattaattcattaaatccgccagcttataagttaatgtctgttttgcggtcgccagcgttaactggttcgcggtcagatccacttgtgcaccttctttcagcatttcgctaatggtgttatcgagttcattaagctgcgggttagcgcacatcatacgggtcattgccagccctttggctgtcagttcaccattagacagtttgccttcaccgctaaagcggttacacatgctgccggaaatcatcattttttcaccaaagctgatttctggcggatttttatcgctggtcacgggcttaccgtttacgctttccagcacaaagcgatgatgctgtagctgttctggcgtaacagcaattttgtcattacttacacatcccgccatcagcaggcttagcgcaacaaacgcggctactttcttcattgtggttctcaattacagtttctgactcaggactattttaagaatagaggatgaaaggtcattggggattatctgaatcagctcccctggaatgcaggggagcggcaagattaaaccagttcgttcgggcaggtttcgcctttttccagattgcttaagttttgcagcgtagtctgagaaatactggtcagagcttctgctgtcaggaatgcctggtgcccggtaaacagcacgttgtggcaggcagacaggcgacggaatacgtcatcctggatcacgtcgttggatttatcttcaaagaatagatcgcgttcgttctcatacacgtccatacccaacgaaccaattttctgatttttcagcgcttcaattgctgcctgagaatcaatcaatgcaccgcgactggtattgacgatcatcacgccatttttcatctgttcgaaggcggcttcgttcaacagatgatagttttccggtgtcagcgggcagtgcagagagataacgtctgattcagagaacagggttggcagatcgacatactccacaccgagttccagcgccgctgcacttggatacggatcgaacgccagcagacgcataccaaaacctttcagaatgcgcagcatcgccacaccgattttaccggtaccgataacgcctgccgttttgccatacatagtaaagccggtcagaccttccagagagaagttagcatcacgggtacgctgatacgcgcggtgaatacggcggttcagcgtcatcatcataccgatggcgtgttcagcaacggcctctggatcataggctggaacacggactactttcagccccagttcttttgccgcgtcaaggtcgacgttattgaaaccggcacagcgcagggcgatatatttaacgccgtgctttttcagctcttccagcaccgggcggctgccgtcatcgtttacgaaaatacataccgcttcgcagccattggcagttttagcggttttttccgtcagcagaaagtcaaaaaattccagctcaaagccaaaggactcgttcacctgttgcaggtacttcttgtcgtactgttttgtgctataaacggcgagtttcataagactttctccagtgatgttgaatcacatttaagctactaaaaatattttacaaaatttcaaatttaattgaaagctatggcgatattgaaaaattcatcaacaactatgcttagtgtaggcgcaaccttcaactgaacggttaaacatgccacaatacccgtattgaatgcttaatttttcgctaaatcaggatattaactacccatgctgggtaaatataaagccgttctcgcgctgttattactgattattcttgtgccgttgacgctgctgatgacgctcgggctgtgggttcccacgctggcgggcatctggctaccgctcgggacacgtattgcattagatgaaagcccacgcattacgcgtaaaggtttaatcattcccgatctccgttatctggtgggagattgtcagcttgcgcatatcaccaacgccagcctttcacatcccagccgctggttattgaacgtcggcacggtagaacttgattctgcttgtctggcgaaattgccgcagacggagcaatcgccagccgctccaaaaacactcgcgcagtggcaggccatgctgcctaacacctggatcaatatcgataaactgattttttctccctggcaggaatggcagggaaaactctctctcgcattaacctctgatatccagcaactgcgttatcagggcgaaaaagttaaatttcaaggccagctgaaagggcaacaacttacagtcagcgaactggatgtcgtcgcgtttgaaaatcagccgccggtaaaactggtgggggaatttgctatgccgctcgtgccggatggacttcctgtaagtgggcatgctactgcgacgttaaacttgccgcaggaaccgtcactggtggatgccgagctggactggcaggaaaatagcgggcaattgatcgtgctggcacgggataacggcgatccgttgctcgatttgccgtggcaaattactcgtcaacaattgaccgtaagcgatggtcgctggagctggccgtatgcaggttttcctttgagtggccgactgggtgtcaaagtcgacaactggcaggcagggcttgagaacgctctggtcagcggacgactgagtgtgctgacccaggggcaagcgggtaagggcaacgcggtgcttaattttggcccaggaaaattaagcatggataacagtcagctgcctctgcagctgaccggtgaagcgaaacaggcggacctcattttatatgcccgtttacctgcgcagctaagtggaagtctgtctgacccaacgctgacctttgagccaggcgcgttacttcgttcaaagggaagagtcatcgattcgctggacatcgatgaaatccgctggcctttagcgggtgtaaaagtcacccaacgtggtgttgacggacgtttgcaggccatcttgcaggcgcatgaaaatgaactgggcgatttcgtgctgcatatggatgggctggcgaatgattttctccctgacgctggccgctggcagtggcgctactggggaaaagggagttttacaccgatgaatgccacctgggatgtcgcaggaaaaggtgagtggcatgacagcacgattacgctgaccgatctctccaccggtttcgaccagttacaatacggtacgatgacggtagaaaagccgcgattaattctcgacaagcccatcgtctgggtacgtgacgcacagcatccctcctttagcggcgcgctgtcactggacgccgggcaaacgctgttcactggcggcagtgtgttaccgccatcaaccttaaaatttagcgtcgatgggcgcgatcctacctatttcctctttaaaggcgatttacatgctggtgagattggcccggttcgggtaaatggtcgctgggacggtattcgtctgcgcggtaacgcctggtggcctaaacaatcactgaccgtattccagccgctggtgccacccgactggaagatgaacttacgcgatggtgaactgtatgctcaggttgcattttctgctgcgcctgaacaaggattccgcgcgggaggacacggcgtgttgaaaggcggtagtgcctggatgccagataatcaggttaacggtgtcgattttgtcctgcctttccgttttgccgatggagcctggcatctggggactcgcggccccgttacgttgcgaattgccgaagtgattaatctggtgacagcgaaaaatattacggctgatttgcaagggcgttatccgtggactgaagaagaacccttgctgttgactgatgttagcgtcgatgtgttaggcggtaacgtactgatgaaacaattacgtatgccgcaacatgacccggcgctgttgcggctgaataatctctcatccagcgaactggttagcgccgtcaatccgaaacaattcgccatgtccggggcatttagtggtgcactgccgttatggctgaacaatgaaaaatggattgtgaaagatggctggctggcgaatagcgggccgatgacattgcgactggataaagacactgcggatgcggtggtaaaagacaatatgactgcgggttcagcaattaactggttgcgctatatggaaattagccgttcatcgacaaaaattaatttagataatctcggtttattaaccatgcaggccaacattacaggtaccagtcgcgttgatggtaaaagcggtacggtaaaccttaattaccatcatgaagagaatatttttacgctgtggcgcagtttacgctttggcgataatctccaggcatggctggagcagaacgcacgtctgccgggaaatgactgtccgcaaggaaaagagtgtgaggaaaaacaatgaaaattttactggctgcgttgacgtcatcttttatgctggttggctgtacgcctcgcattgaagtcgctgcacctaaggaaccgatcactatcaatatgaacgttaaaattgagcatgagatcatcatcaaggcagacaaagatgtcgaagagctgcttgaaactcgtagcgatcttttctgaggtgatgatgaagaaaacattacttctttgtgcgtttcttgttgggctggtaagcagcaatgtaatggcattgactctggatgaagccagaactcaggggcgggtaggtgaaacattttacggttatctggttgcgctgaaaacggatgctgaaacagagaaattagtagccgacattaatgccgaacgtaaagcgagttaccaacaactggcaaagcaaaataatgtgtcggtagatgatatcgcgaaactcgccgggcaaaagctcgtagctcgggccaaaccgggggaatatgtacaagggataaacggtaaatgggtgcgaaaattttaatagcaaaaccgcaatatcgggataacgctacaggagaaggcgattgatctattttcctgaaacaaggtgaatattcaaaaactcctgtcaaattgccttttgccctgaaaaatgcatagtcaaatatctgttttaactaattggcgttgcagtacatgcaacgccaattagttagcggaatttacgtcgatactcgcctggcgtcatcccaaagcgttgcttaaataccgttgaaaaatgactctggtcagaaaatccccaatgaaagccgatgcctgccagtttttcatcatctgcggcatggcgaatcgcatctgcacaaaaatcgagacgacggttacgaatatattgcgcgactaccaaacctttatcggcaaacattcggtacaaactacgtactgacatacctgtctctccggctatccactccgggcgtaatatctcttcgcgaatattatcgtctatcaacgtaaccactttttgaaactgacgttcacgacgaggttgaacagattcccgctgatgaagtaccgggcgcagcagacacaccatcgcctgtagcgcagcttcactttctgtttcagaaagtgccggattattcatgctctcctgtaacaggcgatgactgagttgcaccatgggtaagtcagcgtccagtctttctgcgcagataggtttttgatggggaaaatattgttccagcagagtgcgtggcaaaagtaatgaaatctgtttagaagactcctgccagtaaagcgaacaggggcgtgaggcatcgagtaacgtaatatcgccagcgccaatctgcacctgacgctcatcctgctccattattgcctgaccactaagctgaaaaacggtgtaaaaccaggcatcgtcgctgccttttacttcctgccaggtgcgggataaattcaccccgctggttgtcacggtactcagctttagtcctttggcaaaatgcgtgtccagtacacccgtgtaacgctcagtcagcaggcgtccggtaaaatttccgcatacctgattgatttgggaaagccattgctgaaactcattatccactgcggggttcatggcacgttttcgctctgtgaaatgtatttttattgttgcatttgtgttgcaataaacgaagctaatgagcctgactataggaaataagtcttgtcaggcatagagacataagcggttattgtcacgatttgcggagcttgtcacagctgacaaagcgaatgtcacagcgaaaaaagtgacttttcttgtcgctgcgtacactgaaatcacactgggtaaataataaggaaaagtgatgacagagccgcatgtagcagtattaagccaggtccaacagtttctcgatcgtcaacacggtctttatattgatggtcgtcctggccccgcacaaagtgaaaaacggttggcgatctttgatccggccaccgggcaagaaattgcgtctactgctgatgccaacgaagcggatgtagataacgcagtcatgtctgcctggcgggcctttgtctcgcgtcgctgggccgggcgattacccgcagagcgtgaacgtattctgctacgttttgctgatctggtggagcagcacagtgaggagctggcgcaactggaaaccctggagcaaggcaagtcaattgccatttcccgtgcttttgaagtgggctgtacgctgaactggatgcgttataccgccgggttaacgaccaaaatcgcgggtaaaacgctggacttgtcgattcccttaccccagggggcgcgttatcaggcctggacgcgtaaagagccggttggcgtagtggcgggaattgtgccatggaactttccgttgatgattggtatgtggaaggtgatgccagcactggcagcaggctgttcaatcgtgattaagccttcggaaaccacgccactgacgatgttgcgcgtggcggaactggccagcgaggctggtatccctgatggcgtttttaatgtcgtcaccgggtcaggtgctgtatgcggcgcggccctgacgtcacatcctcatgttgcgaaaatcagttttaccggttcaaccgcgacgggaaaaggtattgccagaactgctgctgatcacttaacgcgtgtaacgctggaactgggcggtaaaaacccggcaattgtattaaaagatgctgatccgcaatgggttattgaaggcttgatgaccggaagcttcctgaatcaagggcaagtatgcgccgccagttcgcgaatttatattgaagcgccgttgtttgacacgctggttagtggatttgagcaggcggtaaaatcgttgcaagtgggaccggggatgtcacctgttgcacagattaaccctttggtttctcgtgcgcactgcgacaaagtgtgttcattcctcgacgatgcgcaggcacagcaagcagagctgattcgcgggtcgaatggaccagccggagaggggtattatgttgcgccaacgctggtggtaaatcccgatgctaaattgcgcttaactcgtgaagaggtgtttggtccggtggtaaacctggtgcgagtagcggatggagaagaggcgttacaactggcaaacgacacggaatatggcttaactgccagtgtctggacgcaaaatctctcccaggctctggaatatagcgatcgcttacaggcagggacggtgtgggtaaacagccataccttaattgacgctaacttaccgtttggtgggatgaagcagtcaggaacgggccgtgattttggccccgactggctggacggttggtgtgaaactaagtcggtgtgtgtacggtattaatctggttcgctcataagtaaaaaacggcacctggtgccgtttttttgtctgaaacaatcacttatctttcttcagcgcccctagcgttggcgtttcgtcaaagaagttccatggtttcagcagagtatgtacccattcggtcggcataatcggccactcttcggcgcgggccacatgtgtggtgccggtggtcatccagacaacggcgtcggtgttgtccagcgactcgttatccttactgtattgtccaagaccggtgtcatgagtagaacggttcggatatttgccttccgggaaacgctcgccaggatgataacgcgttacccagagctgcttgtccataaagcttaaacgatgatagatccactcgtccggcgcgaactgggcaccttttgctaccgggtgagtaccacctgcataaggaataatttgataggaaaccggattgcccatgcggttctctttgttcgggttactcaacagacgaatcgtgcccggatcaaatttctgtgcggcatcctgttcattgccgatgttgtactgattaacttgcatggtactggtgcgtgggccaccggcagtattcggttttaccactgggtccatcgccaccaggctgttattctcgccatctacatccagatcgaggcggaaattataaatatgttggtgtgtagtacccacgatattgtgatcgataagcgtgccgtagcgcgtgtcatctttcgccgtctcatcgtgcatggttttcgctttaacacctttcaccgcttcgatgcccgtagcaccggcatcgatgccaatagtgccgttttcatggaagatccagtcaaaaatgtagtcatagttacccactgtactgatccagcgcaccactaactcccggcgttcggtactgacgttgggctggcccatttcctgatgcttatactccggcccggcataacgttcaaataccgcgatagcgcgagggatctccatcggcacgccagtgtagtcggcgatggtttcattaaggagcactgcgttagacggggcatctttaccacgagcaattggtgaggttagcgtgcccataccgtagtcaccagagtccagatacgctttaaagtaccagccaatatcaggatcaccgtaaggcacaatcatgccgccgagagaaccttcgtacatgactttgcgtttggtgccattgtcgttataagtcacggtggagatcatcggcccgacgcgagagttcatgctgaggtgaaaatcccagttccgccagtgaatcatatcgccagtaatggtgtaatttttaccttcaggctcaatgatttgcataggcttaactgccggagcaacgcggtcacggccatcaaatgggcgtgcggtcattggcaccggaactaccggaccttcttcaatcttaacgatttttttctgttctaaatcaacgaccgccaccaggttttcgatgggatgtgcccagtagttgccatcaccgacatcaagatagctgatgactttgagcaaccgggcatcttgtttcaggccatctttaccatcgaaataacctacggtcagcggcgtggtaatcacttttttcgcatcagtaataccgcgtttcttcacggcagcggcaaattcttcactgttgttaataatgttctgcacactggcgaaatcatccagcaacaccataccgtgggcgtctttaatgggttgccaggagagcagtttgttgttttgcagatccaccaccgcttcgatgatatgtttgccgtcgagcataatgacgtcggctttgcgcggctggtcaaccggtttgttttccagcgcaaacgcccagacagcttctttatctggcggtagcagggagatctcagtaaaacgggtattgggtttgaagtccgcggaagctttaacaatttcaacggcctgtttaatttcgtccgcagttagcgcattaagtgggtgagggcgcttttctacctgaaaggtttgatccagcccggactggaaaacatcgttaataaaggtgtcagaaacccaggctttattgtctttcatcactaccggtacttgcagtgccagaggctgaccattaacaattgctgtttgcgcaccaggcttcactttcacgtacgcgccatctttaatcagggtaaagagctgggcgtagtcgtcccactgcacatcggcaccaaattctttaagcgttttatccattggcaccatatgcgcttcaccaccgtgggcaaataccggcgcttgccaggcgaaacttaaggcgactgccaacgccagggttgttttacgggcagaatacagagaggggcttcccattattaacctcgtcagatgttgtgttcttgttagcaaccgcgctctgtgggcggtttagtcaggttcacattatcagtactgatgcaaaggggattgcctgcacctgccaggttgtttggcaggtgtgccagcttttcatacagtggatgccctgaaaatagatgtacacatcatgcataatgtgacaacgtcacaaaacttagtgaaataaaagggcaactattcgccgttgcccttcattcaccgattaatcgacaaaatcaccgtgctgcctggccaccagcgtcagaattgaatacagcgccaccggggtttgatgctgattgaatacctctacagcccattccaccacacctgttggtttttcttctgcgctacgctgttttttcagcgtcttgcgcttacaggtgagacgcacctggatggtatcgcctggctttacgggttcgataaaacgcaagctttccagcccgtagttagcaatgaccggaccgacaccggcatcgacaaacagacccgcagccgcagaaagcacaaaatacccatgcaccacccgctcaccgaaaatagattcggcagcagcaatcttatccatatgtgcatagaaatgatcgccgctgaggcaagcaaagttaacaatatcggcctctgtcattgtgcggcggggagtcaacaggctgtcgcctggttgtagctcctcaaaatatttgcggaacggatgaatacgatcttcttcgactttcgcaccgcgcacccactgtttactgatagcggcaagcatcgtcggactaccctgaacagcggttcgctgcatgtaatgtttcaccgctcgtaaaccgcctaattcttcaccgcctcctgcgcgaccaggcccaccatgtaccagttgtggcagtggggagccatgcccggtggattcttttgccgactcttcattgaggatctgaattcgcccatgcgtacgtgccgcgtcggcaataaactgacgcgcaatttgcggatcagccgtcaccagcgttcccgcaaggctaccgccgcctgcacaagccagttgcagagcatgtcgctggttttgtgctggcatcagcgttgcgacagggccaaaggcttctgttgcatgtaccgccggtgtttcatccggctgcggacagtacaataaggttggcgggaagaaggcacccgcagcagataaatccgcctgaccaccgaggcgaatctcgcatcctgcagccagcaatatgttcactttttcctgcacatcggcacgctgctcagcatttaccagtgcgcccattttcacgccttcctgagcaggatcaccgaccacgactttctgtaatcgcgcaaccagagcatcactgacagcattaaccaatgcctgcggcacaataatccgccggattgccgtacatttttgcccggcttttgtggtcatctcacgcacaacttcacgaataaacagcgcaaactccggttgatccggggtgacatcttcgcccagtacgcagcagttcagggaatcagcttccatagtgaaggggatagatttggcgacgatatttggctgaactcgcagcatctgtccggtcgccgctgaccccgtgaaagtcaccacatcctggctgtccagatgatccaacaagtcgccagcactaccgcagatcagactaattgcgccttcgggaacaagaccactatcgacaattgatttcaccatcgcctgagtcagttgggccgtcgcggtagctggtttgatgatggctggcattccgcccagccacgttggtgccagcttttccagcattccccagcaggggaagttaaaggcgttaatatgcactgccacgcctgactttgaggtcagtaaatggcgcgcggcaaatccaccttctttcgataaggggatcaattcatcttccggccacagcgtatcgtcaggcagctcccggctaccgaggctggcgtaagtaaataacgtcccaatgccaccttcaatatcaacccaactgtctgcccgcgttgcgcctgtttgcgcagaaagagcatagaaacgctctttttcactcagcagatgtttagcgaccgctttaagcatcgccgcacgttcgataaaggtcatagcgcgaagggcgggggcacctttttcaatggcaaactggcgggcagccgccatatcaagaccttcactggtcacttcccataacgcctcgccgctaatagcgtggtgaatcaaacggctacggccccggccagactgccaggtaccggataagaaactggctaactgctgcatcgctactctccagatgtttcacatttctgttgctaatagttaaatcgcgaatcataaaaagcaaaggatcttttaacgaaatgttaactatgcgatctgtatagcaactgcggaaaacattaatgcactgataaataatgatttataaaaatagggtgcgaaatccgtcacagttcaaacatacaaaatttgtgattttacttaactattgtgtaactttcataaaacaatgtgattcgtgtttttaattaattcacgaaaactggaatcgtaaaggtgatgacgtgacccaagaagaacgctttgagcaacggatagcccaggaaacggctatcgagccacaggactggatgcccgatgcttaccgaaagacattgatccgccagattgggcagcatgcgcactccgagattgttggtatgttgcctgaaggtaactggatcactcgcgcaccaaccttgcggcgtaaagccattctgttggccaaagtgcaggatgaagccggtcatggtctgtatctctatagcgccgccgaaacactgggctgcgccagagaagacatctaccaaaaaatgctcgacggacggatgaaatattcctccatctttaattatccgacattgagttgggctgatatcggtgttatcggctggctggtggatggcgcagcgatcgtcaatcaggtggcgttatgccgcacttcttatggcccgtatgccagagcaatggtgaaaatctgcaaagaagagagttttcaccagcgtcaggggtttgaagcctgcatggcactggcgcagggcagcgaagctcaaaagcagatgttgcaagacgccattaaccgtttctggtggccagccttaatgatgttcgggccaaacgatgataactcgccaaacagcgccagaagtctcacctggaaaatcaaacgtttcaccaacgacgaactccgccagcgtttcgtggataacaccgttccacaggttgaaatgctcggtatgaccgttcctgacccggatctgcattttgacactgaaagcggtcactaccgctttggtgagatcgactggcaggagtttaacgaagtaattaacggtcgcggaatttgtaatcaggagaggctcgacgccaaacgtaaagcctgggaagaaggtacctgggtacgggaagcagcgctggcccatgcacaaaaacaacatgcccgtaaggtcgcataaggagattcaaaatgagtaatgtttactggccgttatacgaagttttcgtgcgtggcaaacagggcttatcacaccgccatgttggcagtttacatgctgccgatgagcggatggcactggaaaatgcccgtgatgcttacacccgtcgtagcgaaggatgttcaatttgggtggtgaaggcgagtgaaattgttgcctcgcaaccggaagaacgcggtgaattttttgatccggctgaaagcaaggtctatcgccatccaacgttttacaccatccctgatggcattgagcacatgtgaggtcggaaatgaatcagttaacggcttacaccttgcgcctgggcgataactgcctggtgctctcccagcggttgggtgaatggtgcggtcacgcaccggaactggaaatcgatctcgcactggcaaacattggcctcgatttattaggtcaggcacgcaacttcttatcgtatgccgctgaattagcgggagaaggcgatgaagataccctggccttcacccgagacgagcgccagttcagcaacttattgttggttgaacaaccaaacggcaattttgccgacaccattgcacgccagtatttcatcgatgcatggcatgtggcgctctttacccgtctgatggaaagccgtgatccgcaactggcggcgatttctgccaaagcaattaaagaagcgcgctatcacctgcgttttagtcgtggctggctggagcgactgggcaatggtactgacgtatcagggcaaaagatgcagcaggccatcaacaagttgtggcgttttaccgccgaactgttcgatgccgacgagattgatattgcactgagtgaagagggtattgcggttgatccacgcactttacgcgcagcgtgggaagccgaagtttttgccgggatcaacgaagccacattgaacgtaccgcaagagcaggcgtatcgcactggcggtaaaaaaggactgcataccgaacaccttggacccatgctggcagaaatgcagtatctccagcgtgtcttgcccggtcagcaatggtaacagaggagatgggtatgcaacgtctggccaccattgcaccgccacaggttcatgagatatgggcgctactcagccagatcccggacccggagatcccggtgctgaccattactgatttaggcatggtgcgtaatgtgacacagatgggagaaggatgggtgatcggctttacgccgacatattccggttgtccggcaacggaacatttgattggcgcgatacgtgaggcaatgacaaccaacgggtttacccccgttcaggttgtgctgcaactcgacccggcatggaccaccgactggatgacccccgatgcccgtgagcgtctgcgagagtatggcattagcccgcccgccggacacagttgccatgcccatttgccgccagaagtacgttgcccgcgctgcgccagcgtccataccacacttatcagtgaatttggttccacggcctgcaaagcattgtaccgctgcgatagttgccgcgaacctttcgattatttcaaatgtatttgaggatgccatgacaacgtttcattccttaacagtggcaaaagtcgagtcggaaacccgtgatgcggtgaccattacctttgcggtgccccagcctttgcaggaggcgtatcgctttcgccccggtcaacatttgaccttaaaagccagctttgatggtgaagaattacgccgttgttactccatttgccgcagctatctgcctggcgaaattagtgtggcggtgaaagccattgaaggcggacgtttctcccgctatgcccgcgaacacatccgccagggtatgacgctggaggtcatggtgccgcaggggcatttcggctatcagccgcaggccgaacgccaggggcgctatctggcaattgcagcaggatcaggtattacgccaatgctggcgattatcgccaccactttacaaaccgagcctgaaagtcagttcaccctgatctacggtaaccgtaccagccagagcatgatgtttcgccaggcactggcagacctgaaagacaaatatcctcagcgtttacagttgttgtgcattttcagtcaggaaaccctcgacagcgatctgcttcacgggcgtattgacggtgaaaaattacagtcacttggggcctcgctcattaattttcgtctttatgatgaggcatttatttgtggtccggcggcgatgatggatgacgcggaaaccgccttaaaagcactgggaatgccagataaaaccattcatctggagcggtttaatacgcctggcacgcgcgtcaaacgtagcgttaacgtgcaaagtgacggacaaaaagtgactgtacgtcaggatgggcgggatcgggaaatcgtgcttaatgccgacgatgaaagcattctcgatgcggcattgcgccagggggcggatctgccctatgcctgcaaaggcggcgtctgtgcgacctgcaaatgcaaagtgctgcgtggcaaagtggcgatggaaaccaattacagtctggaaccggatgaactggccgcaggttatgtgttgagttgccaggcactgccgctgaccagcgatgtggtggttgactttgacgcgaaggggatggcatgagcgaactgatcgtcagccgtcagcaacgagtattgttgctgacccttaaccgtcccgccgcacgtaatgcgctaaataatgccctgctgatgcaactggtaaatgaactggaagctgcggctaccgataccagcatttcggtctgtgtgattaccggtaatgcacgcttttttgccgctggggccgatctcaacgaaatggcagaaaaagatctcgcggccaccttaaacgatacacgtccgcagctatgggcgcgattgcaggcctttaataaaccacttatcgcagccgtcaatggttacgcgcttggggcgggttgcgaactggcattgttgtgcgatgtggtggttgccggagagaacgcgcgttttgggttgccggaaatcactctcggcatcatgcctggcgcaggcggaacgcaacgtttaatccgtagtgtcggtaaatcgttagccagcaaaatggtgctgagcggagaaagtatcaccgctcagcaagcacagcaggccgggctggttagcgacgtcttccccagcgatttaaccctcgaatacgccttacagctggcatcgaaaatggcacgtcactcgccgctggccttacaagcggcaaagcaagcgctgcgccagtcgcaggaagtggctttgcaagccggacttgcccaggagcgacagttattcaccttgctggcggcaacagaagatcgtcatgaaggcatctccgctttcttacaaaaacgcacgcccgactttaaaggacgctaatgatggaattcatcctcagtcatgtagaaaagggcgtgatgacactaacgctcaaccgcccggaacgcctgaacagttttaatgatgagatgcacgcacaactggcagagtgcctgaaacaggtcgagcgcgacgacactatccgttgcctgttacttacaggtgccgggcgcggattttgtgctggtcaggatcttaacgatcgtaacgttgatcccacaggccccgcaccggatttagggatgtcagttgaacgtttctataacccactggtacgtcgcctggcaaaactgccaaaaccggtgatctgtgcagtcaatggcgtggcggcaggggcaggcgcaacactggcactggggggcgacatcgttattgctgcccgttcagcaaaattcgtcatggcgtttagtaagttaggcttaatacccgattgcggtggaacctggttactgccacgcgttgccggacgagcgcgcgccatggggctggcactgctggggaatcaactgagtgctgaacaggcgcacgaatgggggatgatctggcaggttgttgatgatgaaacgctggcagataccgcgcaacagctggcacggcatctggcgacacaaccgacatttggtcttggacttatcaagcaagcgataaatagcgctgaaaccaatacgctcgatacgcaactggatctggaacgtgactatcagcgacttgccggacggagcgcagattatcgtgaaggtgtcagtgcgttcctggctaaacgctcaccgcagttcacggggaaatagcatgatgataaatgtgcaaactgtggcagtgattgggagcggcaccatgggggcaggcattgctgaagttgctgccagtcatggacaccaggttttactgtatgacatttctgctgaagcgctgacccgcgcaatcgacgggatacacgcgcggctaaattcacgcgtgacgcggggaaaactgactgctgaaacctgtgaacgcacattgaaacgcctgatcccggtgaccgatattcacgcgctggcagctgcggacctggtcattgaagcggcgtctgaacgtctggaagtcaaaaaagcgctctttgcacagctggcggaagtttgcccgccacaaacgctattgaccactaacacttcgtcaatctctataaccgcgattgctgcggagataaaaaatcctgaacgtgttgcggggctgcatttttttaacccggcaccggtgatgaagttggtggaggtggtcagtgggctggcaacggcggcggaagttgttgagcagttgtgtgaactaacgttgagttggggtaagcagcctgtgcgctgtcattcgactcctggatttatcgttaaccgtgttgcgcgtccttattattccgaggcctggcgggcactggaagagcaggttgctgcaccagaagtgattgacgctgcacttcgcgatggcgctggtttcccgatggggccgctggaattaaccgatctgattggtcaggacgtcaattttgctgtcacctgttcggtgtttaacgctttctggcaggagcgtcgttttttaccttcgctggtgcaacaggaactggtgattggtggacggttgggcaagaaaagtgggctgggcgtgtacgactggcgcgcggaacgtgaggcagttgttggcctggaagcggtaagcgacagttttagcccaatgaaagtagaaaagaaaagtgacggtgtcacggaaattgacgatgttttattgattgagacacaaggcgagacggcacaggcgctggcaatacgactggcacgcccggtggtagtgatcgataaaatggcgggcaaggtggtgaccattgctgctgcagcggtgaacccggactcagcgacccgcaaggccatttattacctgcaacagcagggcaaaacagtgctgcaaattgcagattacccaggaatgctgatttggcgaacggtagcaatgatcatcaatgaagcccttgatgcgcttcaaaaaggcgtggcctctgaacaggatatcgataccgccatgcgtcttggggtgaattatccatatggcccacttgcctggggagcgcaacttggctggcagcgaatattaaggctccttgaaaatctacagcatcactatggcgaagaacgctatcgcccatgttcattgctgcgccaacgggcgcttctggagagcggttatgagtcataaggcctggcaaaatgcccatgcaatgtatgagaacgatgcctgcgccaaagcgcttggcatcgacattatctcaatggatgaaggctttgctgtagtgaccatgaccgtcactgcacaaatgcttaacggtcatcaaagttgccacggcgggcagctattttcactggctgatactgcctttgcctacgcctgcaatagccaggggctggcagccgtcgcttctgcctgcacgattgattttttgcgtccaggctttgccggagacaccttaactgctactgcgcaggtacgtcatcagggcaagcaaaccggtgtttacgacatcgaaattgttaaccaacaacaaaaaacggttgcgctgtttcgcggtaaatctcaccgcatcggcggcaccattacaggagaagcctgatgcgtgaagcctttatttgtgacggaattcgtacgccaattggtcgctacggcggggcattatcaagtgttcgggctgatgatctggctgctatccctttgcgggaactgctggtgcgaaacccgcgtctcgatgcggagtgtatcgatgatgtgatcctcggctgtgctaatcaggcgggagaagataaccgtaacgtagcccggatggcgactttactggcggggctgccgcagagtgtttccggcacaaccattaaccgcttgtgtggttccgggctggacgcactggggtttgccgcacgggcgattaaagcgggcgatggcgatttgctgatcgccggtggcgtggagtcaatgtcacgggcaccgtttgttatgggcaaggcagccagtgcattttctcgtcaggctgagatgttcgataccactattggctggcgatttgtgaacccgctcatggctcagcaatttggaactgacagcatgccggaaacggcagagaatgtagctgaactgttaaaaatctcacgagaagatcaagatagttttgcgctacgcagtcagcaacgtacggcaaaagcgcaatcctcaggcattctggctgaggagattgttccggttgtgttgaaaaacaagaaaggtgttgtaacagaaatacaacatgatgagcatctgcgcccggaaacgacgctggaacagttacgtgggttaaaagcaccatttcgtgccaatggggtgattaccgcaggcaatgcttccggggtgaatgacggagccgctgcgttgattattgccagtgaacagatggcagcagcgcaaggactgacaccgcgggcgcgtatcgtagccatggcaaccgccggggtggaaccgcgcctgatggggcttggtccggtgcctgcaactcgccgggtgctggaacgcgcagggctgagtattcacgatatggacgtgattgaactgaacgaagcgttcgcggcccaggcgttgggtgtactacgcgaattggggctgcctgatgatgccccacatgttaaccccaacggaggcgctatcgccttaggccatccgttgggaatgagtggtgcccgcctggcactggctgccagccatgagctgcatcggcgtaacggtcgttacgcattgtgcaccatgtgcatcggtgtcggtcagggcatcgccatgattctggagcgtgtttgagcatatcaacctgcgagtaccctacaatgataaccaatacaaagcttgacccgattgaaaccgcgtctgttgatgagttacaggcgttgcaaacacagcgtctgaaatggacgctcaaacacgcgtatgaaaatgtgccgatgtatcggcgcaaattcgacgcagcaggcgtacatcctgatgatttcagggaactttcagacctgcgtaaatttccctgtaccaccaaacaggatctgcgcgacaactatccctttgacacctttgccgtgccaatggaacaagtggtgcgcattcatgcttcttcgggaaccacaggtaaaccgacagttgtcggctatacgcaaaacgatattgataactgggccaatattgtagcgcgttctttgcgtgcggcagggggctcgcccaaagacaaaattcatgttgcctatggttacggcctgtttactggtgggctgggtgcgcactatggtgccgaacgtctgggcgctacggtgatcccgatgtctggcgggcagacggaaaaacaagcgcaactgatccgtgattttcaaccagatatgatcatggttacgccatcttattgccttaacctgattgaagagctggagcggcagttgggcggtgatgccagcggttgctcgctgcgggttggagtatttggtgctgagccgtggacacaggccatgcgtaaagagattgagcgtcgcctggggatcaccgcactggatatttatggcctgtcagaagtgatggggccgggggtggcgatggagtgtctggaaactaccgacggcccaaccatttgggaagatcatttctatcctgaaattgttaatcctcatgacggcacaccgcttgccgatggtgaacatggcgaactgttattcaccacgctgaccaaagaagcattgccggtcattcgttaccgcacgcgtgatttaacccgactgttaccaggaacggcgcggactatgcgccgcatggatcgcatcagcggacgcagcgatgacatgttgattattcgcggtgtaaatgtctttccgtcacaactggaagaagagattgtcaaattcgaacatttatcgccgcattaccaactggaggtgaaccgccgggggcatcttgattcactttctgtgaaagtggagttgaaagaaagtagcctgacattgacgcatgagcagcgttgccaggtatgccaccagctgcgccatcggattaagtcgatggtggggatctctaccgatgtgatgatcgttaactgtggcagtatcccgcgttcagaaggcaaggcgtgtcgggtgtttgatctgcgcaatattgttggtgcctgacgtatcgtctggccctggtggggtaaagcgccagggccagaagtcgatacgacctgtgctatgattcataaatcacaacaataacaacagactgaagcgaatgagtaaacttgatacttttatccaacatgctgtaaacgctgttccggtcagtggcacatctttgatctcctctctgtatggtgattcgctttcccatcgtggtggtgaaatctggttgggtagtctggctgctttgctggaagggctgggatttggtgagcgtttcgtgcgcaccgctttgtttcgtcttaataaagaaggctggctggatgtttcccgcatcgggcgacgcagtttctatagcctcagtgataaaggcttgcgcctgacgcgacgggcagaaagtaaaatttatcgcgcagagcaacctgcatgggatggtaaatggctcctgttgctctcggaaggtttagataaatcaacgctggctgatgtcaaaaagcagttgatctggcaaggttttggcgcactggcacccagcctgatggcatcgccgtcgcaaaaactggccgatgtacagacacttttgcatgaagcgggtgtggcggataacgtgatttgttttgaagcgcaaataccactggcgctttctcgcgcagcactgcgtgccagagtagaagagtgctggcatttaactgaacaaaatgccatgtacgaaacctttattcagtcattccgcccgctggtgccgcttttaaaagaggcggcagacgagttaaccccggagcgggcatttcatattcagcttttactgatccatttttatcgccgtgtcgtccttaaagacccattgttgccggaggagttgcttccggcacactgggcagggcatacggcgcgtcagctgtgtatcaacatttatcagcgcgtagcgcctgctgctttagcgttcgttagtgaaaaaggtgaaacctcggtcggtgaactgcctgcgccgggaagcctgtattttcaacgttttggcggcttgaatattgaacaggaggcgttatgccaatttatcagatagacggtctgactccggttgtgccagaagagagttttgtccatccgacagcggtattgatcggcgatgttattctcggcaagggcgtttacgttgggccaaatgccagcctgcgtggcgattttggtcgtatcgtggtgaaagatggcgcgaacattcaggataattgcgttatgcacggttttcccgagcaggatactgttgtaggagaagatggacatattggtcatagcgctatccttcacggctgcattatccgccgcaatgcattagtgggaatgaacgcggtagtgatggacggtgcggtgattggcgagaacagcattgttggtgcatccgcatttgtgaaagccaaagcagaaatgccagctaattacctgattgtcggcagcccggcgaaagcgattcgtgaactcagtgagcaggagttggcatggaaaaagcagggtacgcatgagtaccaggtgctggtgacacgctgtaagcagacgttacatcaagtcgagccattgcgggaaattgaacctggcaggaaacgcctggtatttgatgagaatctgcgaccgaaacagtaacagatgtaaaattattttgtccctttaattataaagcagagttatgtttaagctctgctttatttatttgagtattaattcataccgttttttcatcatataattatttataatgagaatgtggttttaatttgtaatttatattatatacacaatttatatatttcatggtctttttttattcacctgaattataattgtgaattataggaaagtatgtttgattagataataatctactggcaatattggatgtcttctatgttttaaataactaattggtcgggttagtgcatccggctttctttatattcgccagaaggatttattatgcaaaggaaaactctattgtcggcctgtattgcattagctctgagtggtcagggttgggcggcagatatcacagaggtagaaaccaccacaggtgaaaagaaaaataccaatgtgacttgtccggcagacccaggaaaactcagtccggaagagcttaaacgcttaccctctgaatgctctcctttagtcgaacaaaacctgatgccatggctttccacaggcgctgctgcgttaatcacggccttagccgtagtggaactaaacgacgatgatgatcatcatcatcgcaacaattctccactcccaccgacaccccctgatgatgaatcagacgacactccagttcccccaactcctggcggagatgagataataccggacgatccggatgatacgcctacacctcccaaaccggtttcgtttaataatgacgttattctcgataaaacagaaaaaacgttaactattcgcgattcagtttttacttataccgagaatgctgacgggactatatctctgcaagatagcaatggtcgtaaggcaacgattaatctttggcagattgatgaagcgaataacactgttgcccttgaaggggtgagcgcagatggcgcaacgaagtggcaatataatcacaacggtgagcttgttattacgggtgataatgccacagtaaacaacaatggcaaaaccaccgttgacggtaaagattccaccggtacggaaatcaacggtaataacgggaaagtgattcaggacggcgatctggatgtcagcggcggcggtcacggtattgatatcaccggtgacagcgcgacggtggataacaagggcaccatgaccgtcaccgatccggagtccatgggtatccagatcgacggtgacaaggccatcgtcaataacgaaggcgagagcaccatcaccaacggtggcaccggcacccagattaatggtgatgacgccacggcaaacaacaacggcaaaaccaccgttgacggcaaggattccaccggtacggaaatcaacggtaataacggaaaagttattcaggacggcgatctggatgtcagcggcggcggtcacggtattgatatcaccggcgacagcgcaacggtggataacaagggcaccatgaccgtcaccgatccggagtccatcggtatccaggttgacggcgaccaggcggttgttaacaacgaaggcgagagcgccatcaccaacggtggcaccggcacgcagattaacggtgatgacgccacggcaaacaacaacggcaaaaccaccgttgacggcaaggattccaccggtacggaaattgctggcaataacgggaaggtgattcaggacggcgatctggatgtcagcggcggcggtcacggtattgatatcaccggcgacagcgcaacggtggataacaagggcaccatgaccgtcaccgatccggagtccatcggtatccagattgacggcgaccaggccatcgtcaataacgaaggcgagagcactatcaccaatggcggcaccggcactcagatcaacggtaacgacgccaccgcgaataacagtggaaaaaccactgttgatggaaaagattccacgggtaccaaaatcgcgggcaatatcggcattgtaaatctggatggtagcctgactgttacaggcggtgcgcatggtgttgagaacattggtgacaacggcacggttaacaacaaaggagatattgttgtttccgatactggatcgattggcgtgctcatcaacggtgagggggcaacagtatccaatacgggtgatgttaacgttagcaatgaagcgacagggttcagcatcacaaccaacagtgggaaggtttcgctggcaggcagtatgcaggttggcgatttctcgaccggggtagatcttaatggcaacaataacagcgtgacgctggcggcaaaagatctaaaagtggtcgggcagaaagcgacgggcataaacgtttctggcgatgcgaatacagtgaatatcactggtaacgttctggttgataaggataaaaccgcagacaatgcggcggaatatttcttcgatccatccgtgggtatcaacgtttacggcagtgataataacgtgacgctggatggaaagttaactgttgtatcagacagtgaggttacttctcgtcagagtaatttatttgatggcagcgcagagaaaacgtcaggtctggttgtgattggcgatggcaataccgttaatatgaatggtggacttgaactgattggagagaaaaacgcgcttgcagatgggtcgcaggttacttccttgcgcacaggatatagttataccagcgttattgtcgttagtggtgagtcgtcggtatatctgaatggagatacgacaatcagcggagaattccctctggggtttgccggggttattcgggtacaggataaagctttgctggaaattggcagtggcgctacgctaacaatgcaggatattgacagttttgaacatcatgggacaagaaccctggatttgcccctatatttccagacatctgttatcacttaacccattacaagcccgctgccgcagatattcccgtggcgagcgataacccagcgcactatgcggatgccattcgttataatgctcgaacgcctctgcaaggttctttgctgccgttaacccgtctggtttgggcatgatactgatgtagtcacgctttatcgttttcacgaagctctctgctattccgttactctccggactccgcaccgccgtgttcttcggttcaagtcccaacatccgggcgaactggcgtgtttcattagcccggtagcatgaaccattatccgtcagccactccactggagacgacggaagatcgttgccgaagcggcgttccaccgctcccagcatgacgtcctgtactgtttcactgttgaagccgccggtagtgaccgcccagtgcagtgcctcacgatcacagcagtccagcgcgaacgtgacacgcagtctctctccgttatcacagcagaactcgaacccgtcagagcaccatcgctgattgctttctttcacggccactctgcctgtatgtgcccgtttcgatggcggtacagcaggttttcgctcaagcaacagcgcattctggcgcatgatccggtaaacacgtttggcattgatcgcaggcataccatcaagttctgcctgtctgcgaagcagcgcccatacccgacgataaccatacgttggcagctctccgataacatggtgtatacggagaagcacatccgtatcatcagtgtgacgactgcggcggccatccatccagtcatcggttcgtctgagaatgacgtgcaactgcgcacgcgacacccggagacaacggctgactaagcttactccccatccccgggcaataagggcgcgtgcgctatccacttttttgcccgtccatattcaacggcttctttgaggagttcattttccatcgttttcttgccgagcaggcgctggagttctttaatctgcttcatggcggcagcaagttcagaggcaggaacaacctgttctccggcggcgacagcagtaagacttccttcctggtattgcttacgccagagaaataactggctggctgctacaccatgttgccgggcaacgagggagaccgtcatccccggttcaaagctctgctgaacaattgcgatcttttcctgtgtggtacgccgtctgcgtttctccggccctaagacatcaatcatctgttctccaatgactagtctaaaaactagtattaagactatcacttatttaagtgatattggttgtctggagattcagggggccagtctaaaccccagaacttacttatgctgattccggtgcgaaaattgttaataaaggtacttgtagattcaattggtcaacgcaacagttatgtgaaaacatggggttgcggaggttttttgaatgagacgaacatttacagcagaggaaaaagcctctgtttttgaactatggaagaacggaacaggcttcagtgaaatagcgaatatcctgggttcaaaacccggaacgatcttcactatgttaagggatactggcggcataaaaccccatgagcgtaagcgggctgtagctcacctgacactgtctgagcgcgaggagatacgagctggtttgtcagccaaaatgagcattcgtgcgatagctactgcgctgaatcgcagtccttcgacgatctcacgtgaagttcagcgtaatcggggcagacgctattacaaagctgttgatgctaataaccgagccaacagaatggcgaaaaggccaaaaccgtgcttactggatcaaaatttaccattgcgaaagcttgttctggaaaagctggagatgaaatggtctccagagcaaatatcaggatggttaaggcgaacaaaaccacgtcaaaaaacgctgcgaatatcacctgagacaatttataaaacgctgtactttcgtagccgtgaagcgctacaccacctgaatatacagcatctgcgacggtcgcatagccttcgccatggcaggcgtcatacccgcaaaggcgaaagaggtacgattaacatagtgaacggaacaccaattcacgaacgttcccgaaatatcgataacagacgctctctagggcattgggagggcgatttagtctcaggtacaaaaaactctcatatagccacacttgtagaccgaaaatcacgttatacgatcatccttagactcaggggcaaagattctgtctcagtaaatcaggctcttaccgacaaattcctgagtttaccgtcagaactcagaaaatcactgacatgggacagaggaatggaactggccagacatctagaatttactgtcagcaccggcgttaaagtttacttctgcgatcctcagagtccttggcagcggggaacaaatgagaacacaaatgggctaattcggcagtactttcctaaaaagacatgtcttgcccaatatactcaacatgaactagatctggttgctgctcagctaaacaacagaccgagaaagacactgaagttcaaaacaccgaaagagataattgaaaggggtgttgcattgacagattgaatctacactgttgaaattcagaatttaggttttgcttttgttactggtgaaaatacaacaggtataaatagtggcacgatctcgttattacaaaatggtaaagatccggcaccgtctcccattgttttactggctactaacggagggagcgccactaatgcaggtacgatcacaggtaaagtgacggaacaacatagcgtatttaacaagtattcaacgggcacatcgaattcatttatttttaataacgatgtcagtagcataacagggttagtcgctcaatcgaatagcacaattatcaatactgacagcggcatcattgatttgtatggtcgtggtagtgtcggcatgcttgctatagcagattcaacagcagaaaatcagggtaaaattacactggattctatgtgggtagatgcaaatgacactaccgcaatgcgagatatagctagcaacagcgccattgacttcggtacaggtgtgggagttggtactgatagttatagtggtgcagggaaaaatgcaacagcaattaaccaattgggcggtgttataactatttataacgccggcgcaggtatggcggcctatggcgccagcaatacagttattaaccaggggacgattaacctcgaaaaaaatggtaattatgacgatagtctggcagcaaatactctggtagggatggctgtttatgagcatggtactgctatcaacgaccagacgggtgttatcaatatcaatgttggtactggtcaggcgttttataacgatggcacaggaacaattgttaactatggtacaatctgcactttcggcgtgtgccaatcggggaatgagtacaataatacagatgatttcacctcactgatctataccggtggcgatacgattacacgaagcggagaaactgtaacgctaaataaatctgctgctgtgactgataagctggctgggaatgttgttaatagcggaacgctttccggtgatcaaattacggtatcaagcggtcttctggaaaataccagcggtggcatcatcaataacttagtaaaacttgacaagggtgccgtcattaaaaatgccggggtgatgacgaataacgtcgatgttagcggtggaatcctcaataatgccggagaaatgactgcgcaaattaccatgaatgctggtgctgatagttcgttagtgaacaacaccggaaccatcaataaaatcgtgcagaacgcgggggtattcaataatagtggcagtgtaacagggcggatgatgtcggctggcggggtctttaataatcaaactgacggggcgattatgagaggtgctgcgctgacaggtactgcagtggcaaataacgaaggaacctggaacctcggaagtagtagtgagggtaacaacaccgggatgctggaagttaataataattcagctttcaataaccgcggcgagtttattcttgataacgacaagaatgctgtgcacatcaaccagtccggtacgctttataataccggtcacatgaacatcagtaattcttcccacaacggagccgttaatatgtggggcggaaatggtcgttttatcaatgacggaacgattgatgtttctgcgaagtcactggtagtcagcgctaataatgccggcgatcagaatgccttcttctggaaccaggataacggggtcatcaacttcgatcacgacagcgccagtgccgtgaaagtcacccacagcaactttattgcccagaatgacggcatcatgaacatcagcggcaccggtgctgtggctatggaaggtgataagaacgcgcagctggttaacaatggcaccatcaacctcggtaccgcaggcactactgacacgggtatgatcggtatgcaactcgatgccaacgccacggcggatgcggtaatcgaaaacaacggcaccatcaatatcttcgccaatgactcgtttgcatttagcgtactgggtacagtaggtcatgtggttaacaacggcacggtggtgattgccgatggggttacgggttctggactgatcaagcagggcgacagcatcaatgttgaaggtatgaacggtaacaacggtaatagcagcgaagtgcattatggcgactatacgttgccggatgtgccgaagcccaatacggttagtgtaacgtcgggaagtgatgaggctggtggcagcatgaacaacctcaacggctatgtcgtcggtaccaacgttaacggcagcgccgggaagctgaaggttaacaatgccagcatgaacggcgtggagattaacacgggctttaccgctggtacggcagacaccactgtgagttttgataacgtagtggaaggtagcaacctgaccgacgctgacgccatcacctcaacgtccgtggtatggactgccaaaggcagcaccgatgccagcggtaacgttgacgtcaccatgagcaaaaatgcctacaccgatgtggcaacagatgcctcggtgaatgacatcgcgaaagcactggatgcgggttacaccaacaacgaactgtttaccagcctgaacgtcggcacgactgctgaactgaacagtgctctgaaacaggtcagcggtagccaggcgaccacggtattccgcgaagcgcgcgtgttaagcaaccgctttagtatgctggcagatgccgcgccgaaagtgggtaacggtctggcgttcaacgttgtcgcgaaaggcgatccgcgtgccgagttaggtaataataccgaatacgacatgctggcattgcgtaaaactatcgacctgagcgaaagccagacgatgagtctggagtacggtatcgctcgtctcgatggtgatggtgcgcagaaagcgggtgataatggcgttacaggcggttatagccagttttttggcctgaaacatcagatgtcgttcgataacggcatgaactggaataacgccttgcgttacgacgttcacaaccttgacagcagccgctcgattgcatttggcaacacgaacaaaacggctgataccgacgtgaaacagcagtacctggagttccgcagcgaaggggcgaagactttcgaaccgagcgaaggactgaaggttacgccatatgcgggtgtaaaactgcgtcacacactggaaggtggctatcaggagcgcaatgccggagactttaacctgaatatgaacagtggcagcgaaacggcggtggacagcatcgtcgggctgaaactggactacgcaggtaaagacggctggagcgctagcgctacgctggaaggcgggccgaacctgagctacgcgaagagccagcgtacggcaagcctggcaggcgcaggcagtcagcactttaacgtcgatgacggtcagaagggcggcggcatcaatagcctgacaagcgtcggcgtgaagtacagcagcaaagaaagttcgctgaatctggatgcgtacaactggaaagaggatggcatcagcgataaaggcgtgatgctgaacttcaagaaaacgttctaatttttagcatgtgatccctaaaccgcaacgctgatacaggttgcggtttttttattgccggatgtggtacgtgacgcgttttgttttgtgtctttcaggacaatagagcaactcatccagtaatcttgtttacaccttcgcattatttatctcttttcgtttctatactgatttttcttaatccgttttattacagggcagggtgcgatgagcagcaatacatttactctcggtacaaaatccgttaaccgtcttggttatggcgcgatgcaactggcaggtcctggagtttttggccccccacgagatcgccacgtcgctataaccgtgctgcgtgaggcgctggcattgggcgtcaatcatattgataccagcgacttttatggtccgcacgtcaccaatcagattatccgcgaagcgctttatccttactctgacgacctgacaattgtcactaaaattggtgcgcggcgtggagaggacgcatcctggttgcccgcattttctccggcagagctgcaaaaagcggtgcacgataatctacgtaatctcgggctggacgtgctggatgtggttaacctgcgcgttatgatgggggatggtcatggcccagcggaaggatcgattgaggccagcctgaccgtgctggcagagatgcaacaacaaggcctggtaaaacatattggcctgagcaacgtcacaccgacgcaggttgcagaggcgcgcaagattgccgaaattgtctgtgtgcaaaacgaatacaacatcgcgcaccgtgctgatgatgcaatgattgatgctttggcccacgatggcattgcctacgtgccgttcttcccgctcgggggctttacaccgctgcaatcgtccacactttccgatgttgctgcgagcctgggtgcaacaccaatgcaggtggcgctggcgtggctgttacagcgttcaccgaatattttgctgatcccagggacgtcttcggttgcgcatttacgggagaatatggctgctgaaaaattgcatctttctgaggaagtgttgtctacgttggatggtatttcgcgagaataacgaatatacaaaagggaaagatgcatttccctttttttcttttttaatggcatggagtgcatatgttgaaggccaggaattgcggctggatacgtttactgcccctgtttatgctgagtctaccagtacaggcggaacttcgatgtgttgcaaatgcagttgatattgaatcatttttttctgcggctaccgctgaagataaacaacaagttgaacaagctatcaacagtagcgtgaatcttgtccccttcggtttatctgcatcgaactggaaagtgcatcgtggcgatttagtggtagaaggtaatatagagagtaatcaaaaattgattgttcttgggaatttgacagtcaaaggtaatatttccactttctctctttctaatccatgggttattctcggtaacgtgacggcaacgaatatagttgcggattcaccactgttaattaccggttcgataaatgcaagtggactggtatttatcgactcatattacgataatccgtctacgattaaggggagtattaatgcgcgtgggatatttatcaatgacataattgcacctgttgttgcgtcttcgacaaatagtgaattcatggtccgtgcgagtgacaaacatgacactgaaaatgtcaaaaaagcgctgatgataataaatcctgatgcatattattgggggctaattaatgatgaagatgctctgaaagaaatttttaagcgaagcaatattcgcatggcagggaatgtctgtaatcagatgaaaaaagaagcgctgtttcgccctaagccttctcctgagttagtgcaagaattgcaaatgctggatgaaggcaaagttgctgcatttgaaggacgagacattgcgacatttgatcttgccgtaatgcgaactctcccaaggcttaaaggaatttcagctaacctacgcaaacaacttattaatagcaatgatgaacaaacgattgaaagtatggcgagatatatgcctgacaatgagattctggagttgaccgatcagcaattgggttaccagcctgttgttctggggttgctcgaccgtgaaccgctctctgtcgaaataatgacgcgaatgagtcgtctacctgatggtgtcggtccgttgaatcttgcgctacgtgaaaatctccctctggatatcgtcatgactctggcgaaaagagattgggatatgatcattcaggagctttataaagatgcgtggttattgcctgaatccattattgatggctatatccgcagtgatgattcctctattcgtcaggtcggtgctggaggacaactcacctacaatcaggcaatgcagttggcgaacgattcatcaaacaatgttgtcacaagcttagcgttcaagctggcagagatgaaacaccatggtcaattgttgcggatgacgccacaagagagtgacaaagttgcaggctatttataccaaaaattcgagaatgacgatgatctaatacgtgtgttatttttagcattgccagataacttacagtttaattttgttaaaaggatggagaaaaaatccccggcctacttttgctgtcgggatatgcaggtaattcactctgacgctgctttacaacggttattgacacgtttcaacgatcctgaagggtggagtaatctggcgaaaaatcagtatctgagcacgtcgatgaaacaaaaaatttggcaacgtgctttatcgcatcggaaaaataatccgaaagcagattcagatgcatatgaaaccagcgctgatatgattttgtctgagctgattagccacggcgaagttgatgaccagatgctattaaatgccaccgccctgatacgttcggacgactgggactttttagagagtgcattaattagttgggataatttacccgctgttgttctcaaggaattacagcaaaacacgccacgcaatgatatttgggcgaagttttttctgaggcaggaaaacagttcccgtgcgcaggttgacgaagcgttacgtgtttattatgcactagaccccgatgcgttagcacaactggatgtactggcaaaacaaccggatcgtatatggtggagtacactggcgaaaagcaatctcacatttttcaagttcggcgcacttaacaaccgccacacaccgcctgcagtactggcggcagaaattgatcccgagtggtggattgtggcgatgaataatccccgttttccagttgatgtattaaaggcgaggctgaaacgtgatcctttgctggcgttagagcttgttaaccctgaactggatttagtccgccagctggcgcttaacggtaagacgcgcgcaatacgggaacaagcgatgagaaaacttgatgagttgtattgatccacaacgtaatgttttttaactatctgattaattggggataatcattcctgacagtgagtccccaataccttgatatattctgaatttttaatgaaacggcgtgttgcgatatctccgtcaggggaattgatgcaccatagcgcaaaccgaattatcaaggattgataatgacgctctaccagataaaaccgctctttcagtcgctgttaaggccgacgatgttttggctttataagcaccacgttacagcgaatcacatcactcttgctgcactggcgctttctcttcttaccggattgctgttgatgttggcggcacaacccatcctctttttgctattgcccatcgtgctttttatccgtatggcgctcaatgcgctggatggcatgttggcgcgtgagtgcaaccagcaaacacgtctgggggcgattttgaatgagactggcgatgttatttccgatattgcgctctatttaccatttttatttttaccggaaagtaacgcatcactcgtgatactcatgttattttgcaccatattgaccgagttttgcggtttactcgcgcagacgattaacggtgttcgcagttatgccggtccatttggcaaaagcgatcgcgcgttaatatttggtctgtggggtctggccgttgccatttatccacagtggatgcagtggaataatcttttatggagcattgcttcaattctgcttctctggactgcgattaatcgttgtcggagtgtgcttcttatgagcgctgaaatataatgctggaaaaatctctggcaacacttttcgcgttgttaattttagcaacgctgataaaccgttttctgctatggcggttaccggagagaaaagggggtgaggttacattacgtattcgtacctggtggggcatcgtcatttgtttttcaatggtgatttcaggtccacgctggatgacgttgacgttttttgcgctgataagttttctggcattgaaagaatattgtacgcttatatctgtacattttccgcgttggttatattggggtattcctcttaactatttgcttatcggttttaattgctttgagctgtttctgttatttatacctttggctgggtttctgatattagccaccgggcaagttttagtgggtgacccctctggttttctgcataccgtgagcgccattttttggggctggataatgaccgttttcgccttgagtcatgccgcctggttattaatgttgccaaccacaaatatccagggcggggcgttactggtgttatttcttttggcattaaccgagtcaaacgatattgcacagtatttatggggaaaatcctgcggcagaagaaaagtggtccctaaagtcagcccgggaaaaacattggaaggtctgatgggcggcgtcatcaccatcatgattgcgtcactgattatcggaccgttactgacaccgctaaatacattacaggcattattagcgggtttgttaattggtattagtggtttttgcggcgatgtcgtgatgtcagccatcaaacgagatattggtgttaaagatagcggaaaactattgccaggacatggcggactccttgacaggattgactcattaattttcaccgctccggtatttttttattttatacgctactgctgttactgaaggaaaatagagaaaatggaaaattcacgcatccctggggaacatttttttaccaccagtgataatacagcgttgttttatcggcactggcccgctttacagcccggggcgaaaaaggtcatcgtcttatttcatcgcgggcatgaacattctggtcgtctacaacatctcgttgatgaactggcgatgccagatactgctttttatgcctgggatgcccgagggcatggaaaaagttcggggccgcgtggttatagcccatctcttgcgcgttcagtgcgggatgtcgatgaatttgtccgttttgctgccagcgacagccaggttggactggaagaggtggtagtgatcgcgcaaagcgtcggcgcagtgctggttgccacatggattcatgattatgcacctgcaattcgcgggctggtgctggcttctccggcctttaaggttaaattgtatgtgccgctggcacgtcctgcgctggcgttatggcatcgtctgcgtggtctgttttttattaattcctatgtgaaaggacgctatttgacccacgatcggcaacggggggcgagtttcaataatgatccgctgatcacacgggcgattgccgttaatatcttgctcgatctctacaaaacgtctgaacgtattattagagatgcggcggcgattacgctccccacgcaacttctgatatcaggcgatgactatgtggtgcatcgccaaccgcagattgatttttatcagagattacgtagccctctgaaagagctgcatctgctgccaggcttttatcacgacacgttgggtgaagagaacagggcgctggcatttgaaaaaatgcaaagctttattagtcgtttatatgctaacaaatcgcaaaaatttgattatcagcatgaagactgcacaggaccatcagcggatcgatggcggctactttctggtggacccgtgccattatcgccggttgatttagcgtatcgctttatgcgaaaggcgatgaaattgttcgggacgcactcttcgggcctgcatctcggaatgagcaccggctttgattcaggcagttcgctggattatgtctatcaaaatcaaccgcaaggtagtaacgcattcgggcgtttagtcgacaaaatctacctgaacagtgttggctggcgcggtattcgccagcgcaaaacccatttacaaatactgattaaacaagccgttgccgatctccacgccaaaggtttagccgtccgcgtggttgacattgccgcagggcatgggcgctatgtactggatgcgctggcaaacgagcctgccgtaagcgatattttgttacgtgattacagcgagttaaatgttgcacaggggcaagagatgattgctcaacggggaatgtctgggcgggtgcgttttgaacagggcgatgcgtttaacccggaggaactcagcgcgttaactccgcggcctacgctggcgattgtctctggcctgtatgagctttttcccgaaaatgagcaggtaaaaaactcactcgcaggtcttgccaatgccatcgaaccgggcggcattctcatctacaccgggcagccgtggcaccctcaactggagatgattgccggggtgttaaccagtcataaagatggtaaaccgtgggtaatgcgcgtgcgttcgcaaggggagatggattcactcgtgcgtgatgccggatttgataaatgcacacaacggattgatgagtggggtatttttacggtttcgatggcggtgcgtcgtgataactgaacgtcggaacgtattgctacaaggcgctggctggttattgttgctggccccgtttttcttcttcacctatggatctcttaatcagttcaccgcggttcaggaccttaacagccatgatatccccagtcaggtattcggttgggaaacggcgatcccttttcttccctggactattgttccttactggagtctggatcttttatatggattttcgctgttcgtttgtagcacgacattcgaacagcgccgacttgtccaccggcttattctggcaacggtaatggcctgctgcggttttttgctctatccgctgaagtttagttttatccgtcctgaagtgagtggggtgacgggatggctattttcgcaacttgaactgtttgatctgccttataaccagtctccttcgctgcatattattctctgctggctactttggcgtcactttcgtcagcatctggctgagaggtggcgtaaagtctgcggcggatggtttttactcatcgccatttcgacgctgacgacctggcagcatcattttattgatgtcatcacagggctggcggtaggtatgttgattgactggatggtgcccgtcgaccgtcgttggaattatcagaaacctgatcaacgtcgaatcaaaatagcactgccctatgtcgtaggcgcgggctcgtgcattgtattgatggagctaatgatgatgattcagttatggtggtcagtctggttatgttggccagtattatcgctactcataattggccgtgggtacggtgggcttggcgcgataacaacagggaaagatagtcaggggaaactaccgcccgccgtttactggctgacattgccctgccgcatcgggatgtggctgtctatgcgttggttttgtcgtcgcctggagccggtgagcaaaatgactgctggtgtttatttaggggcgtttccacgacatattccggcacagaatgcggttctggacgtcacctttgaattccctcgcggacgagccacaaaagatcgactctatttttgtgtaccgatgctggatctggtggttccggaagagggggagctccgacaggccgtggcgatgctggaaacattacgcgaagagcaaggcagcgttctggtccattgtgcattgggattatcgcgcagtgcgctggtggtggcggcatggttgttatgttacggacactgtaaaaccgttaatgaagcgattagctatattcgagccagacgcccgcagattgtgctgacagacgagcacaaagcgatgctgagattatgggaaaacaggtaagtggattgagatgtggactgaatatctacagtccacatcaagaccgtgtccggttatgcagaaacaatgctgtcgatggctgcttttgcgtcagactgtgctttcgctgccatttccggaccgtatgcgatcccttcggcgaagacaaatttcacatcggtaatgccgataaagccgaggaacgtggacagatacggcgtcaccaggtccgttggtccatctttgtggatcccgccgcggctggtaataacgatggcttttttacccgttaccagaccttccggaccgttctcggtatagcggaaagtaacgcctgcgcgggcaaccaggtcaaaatagtttttcaactgagtcgagatgttgaagttatacatcggtgccgcaataacgataacgtcgtgggctttcagctcggcaatcaactcatcggaaagtgccagagcttcctgctgacgcggagtcagcggcgcatcgctcggacgcagagcgccaaccagttcgccatccagtaccggaatcggatttgcagccaggtcgcgaacggtgatttcatcagcggagtgcttttcgcgccattgttcaacaaaataatcggacaactgattagactgagagtaccctgccaggatgctggatttaagaactaataccttgctcatggtgtttccttatagatgtttgaatgggcgatgccccgttgcttgttgacactttattcacaatcctgccacagagatagcgcaataaatcgaagcctatgttcgaatttattgaacaacgcatagaaagccgcgatgtggtactctatatctatcatttaaaagaaaattaatcaggcagactactgcccactaacgttatgacagaacaacaaaaattgacctttacggccttgcagcagcggctggattcgctgatgctgcgtgacagactgcgtttttctcgccgtctgcacggcgtgaagaaggttaaaaatcctgatgcacaacaggccattttccaggagatggcgaaagagattgaccaggcggcagggaaagtcctgctgcgtgaagcggcacgaccggaaattacttatcctgacaatttaccggttagtcagaaaaaacaggacattctcgaagcgattcgtgatcaccaggtggtgatcgtcgccggggaaacgggttctggtaaaacgactcagttaccgaaaatctgtatggagctggggcgcgggattaaaggactgatcggccatacccagccgcgtcgtctggcggcaagaacagtggcgaaccgtattgcggaagagctgaaaacggagccgggcggttgcatcggttacaaagtgcgtttcagcgatcacgtaagtgataacacgatggtcaagctgatgaccgacggtatcctgctggcggagatccagcaagaccgcctgctgatgcagtacgacactatcattattgacgaagcgcacgaacgcagcctgaatatcgattttttgctcggctatttgaaagagttgctgccgcggcgtcctgacctaaaaatcattatcacttccgcgactatcgacccggaacgcttttcgcgccactttaataatgcgccgattattgaagtctccggtcggacctatccggtggaagtgcgctatcgcccgattgttgaagaagccgatgacaccgagcgcgatcagttgcaggcgatttttgacgccgtagacgaactgagtcaggaaagccatggcgacattctgatctttatgagcggcgagcgggaaatccgcgataccgccgatgcgctgaacaagctgaacttacgccataccgaaatcttgccgctttatgcgcggctttcgaacagcgaacaaaatagggtattccagtcgcacagcggacggcgcattgtgctggcgaccaacgtcgcggaaacgtcgctgaccgtaccggggattaaatacgttatcgaccccggtacagcgcgtatcagccgctacagctatcgcaccaaagtgcagcgtttgccgattgagccgatttcccaggcgtctgccaatcagcgtaaaggccgctgtggtcgtgtgtccgaagggatctgtattcgtctctattccgaagacgatttcctctcgcgcccggagtttaccgatccggagattctgcgtaccaacctggcctcggttattttgcagatgaccgcgctggggctgggcgatatcgctgcgttcccgtttgtcgaagcaccggataaacgcaatatccaggatggcgtgcgtctgctcgaagagctgggcgcgatcaccactgatgaacaggccagcgcctataaactgacgccgctcggtcgccagctctcgcagttgcctgtcgacccacgtctggcgcgtatggtgctggaagcgcaaaaacatggctgcgtgcgtgaggcgatgattatcacgtccgcgctctccattcaggatccgcgcgaacgtccgatggacaaacagcaggcatcggacgaaaaacatcgtcgcttccacgacaaagagtctgactttctcgcgtttgtgaatctgtggaattatcttggcgagcagcaaaaggcgctttcttccaacgccttccgtcgcctgtgtcgtaccgattatctcaactatctgcgcgtgcgcgaatggcaggatatctacacccagttgcgtcaggtggtgaaagaacttggcattccggttaacagcgaaccggcggagtatcgcgaaattcacattgcgttgctgaccggtttactttcccatatcggcatgaaagatgccgataaacaagaatataccggcgcacgtaacgcgcgtttctccatcttccccggttctggtttattcaaaaaaccgcctaaatgggtaatggtggcggaactggtagaaaccagccgcctgtgggggcgcattgctgcgcgtatcgacccggaatgggtggagccagttgctcagcatttgattaaacgcacctacagcgaaccgcactgggaacgggcgcagggcgcggtgatggcaacggaaaaagtcactgtttatggtttgccgattgttgccgcgcgcaaggtcaactacagccagatcgatccggcgttatgtcgtgaactctttattcgccacgcgctggtggaaggtgactggcagacgcgtcacgcattcttccgtgaaaacctgaaactacgggcggaagtagaagagctggaacacaaatcacgtcgccgcgatattctggttgatgacgaaacgttgtttgagttctacgaccagcgcatcagccacgatgtaatctccgctcgccacttcgacagctggtggaaaaaagtcagccgcgaaacgcctgatttgctcaactttgaaaaaagcatgttgatcaaagagggcgcagaaaaaatcagcaagctggattacccgaacttctggcatcagggcaatctcaagctgcgtttgagctatcagtttgagcccggcgcggatgctgacggtgtgaccgtacatattccgctgccgttacttaaccaggttgaggaaagcgggtttgaatggcagatccccggtctgcgccgcgaactggtgattgctctgattaaatcgttgccgaaaccggtacgccgtaattttgtacccgcgccaaactatgccgaagcgtttttaggccgcgtcaaaccgctggagttaccgttgctcgacagccttgagcgcgagttacggcggatgaccggcgttaccgttgaccgcgaagactggcactgggatcaggtgcccgatcacctgaaaattaccttccgcgtggtggatgacaaaaacaagaagctaaaagaagggcgctcgctacaagatctgaaagatgcgctgaaaggcaaagtgcaggaaacgctatctgcggtggcggatgacggtatcgagcagagcggcttacatatctggagttttggtcagctgccggaaagctacgaacagaagcgtggcaactacaaagtgaaggcgtggccggcgctggtggatgagcgcgacagtgtggcgatcaaactgtttgataacccgctggagcaaaagcaggcaatgtggaacggtcttcgccgtctactgctgctgaatattccatcgccaatcaaatatttacatgaaaagttaccgaacaaagccaagctgggactgtactttaacccgtatggcaaagtgctggagctgatcgacgactgtatctcctgcggtgtggataaattgatcgacgccaatggtggcccggtctggacggaagaaggctttgctgcgctgcatgaaaaagtgcgtgccgaactgaacgacacggtggtggatattgcgaagcaggtcgagcaaatccttacggcagtgttcaatatcaacaaacgtctgaaagggcgggtggatatgaccatggcgctggggctttctgacattaaagcgcagatgggcgggttggtatatcgcggttttgtcactggtaacggcttcaaacggctgggcgacacgctgcgatatttgcaggcgattgaaaaacggctggaaaaactggcggttgatccacatcgcgaccgtgcgcagatgctgaaagtcgaaaacgtccagcaggcgtggcagcaatggatcaacaaactgccgcccgcacgtcgtgaggatgaagacgtgaaagagatccgttggatgatagaagagttgcgcgttagttacttcgctcaacaacttggtacgccttatccgatttcagataagcgtattttgcaggcgatggagcagattagcggttaaccctgctatttgcctgataaagaaaaaacccggtaagcatttagcgccgggttttttattaattctaaaacggtaagggtaaaaattcaggaattcagaaaaatacaattctctgctgcaagatgaataatgtttatctacagcatttccttaaaagatatgtcaggcttgcggagtggcggttaaggacatacgatttcctcctttcagagtgctccgcttctcactattatctcacgcagtattcttaagggaacgataaggaggaaccatgaacattaccccgtttccgacgctttcgccggcaactatagatgccataaatgttatcggacagtggctggcgcaggatgatttctccggtgaggtgccgtatcaggccgattgcgtgatccttgcaggcaatgcggttatgccgactatcgatgcggcatgtaagattgcccgcgatcagcaaattcctttactgattagtggtggtatcggtcactcgacaacttttttgtatagcgccatcgcacagcatccgcactacaacactatccgcaccactggcagagcagaagcgaccatcctggcggatatcgctcatcagttctggcacattccgcatgaaaaaatctggattgaagaccagtcaacaaactgcggtgaaaacgcacgctttagcatcgcgctattgaatcaggccgtagaacgagttcatacggctatcgttgttcaggaccccaccatgcagcggcgcacgatggcgacgttccgccgtatgactggggacaatcccgatgcaccacgctggttaagttatcccggattcgttcctcagttaggaaataacgcagacagtgtaatctttattaatcagttacaaggattatggccagttgagcgttatctctcactactcactggcgagctgccgcgtttacgcgatgatagcgatggctacggtccccgcgggcgagattttatcgttcacgttgattttccggcagaagtcatccatgcatggcaaacgctgaaacatgatgcggtgctcatcgaggcgatggaaagtcgctcgttacgttaaaaattgcccgtttgtgaaccacttgtttgcaaacgggcatgactcctgacttttatttctgccttttattccttttacacttgtttttatgaagcccttcacagaattgtcctttcacgattccgtctctctgatgattgatgttaattaacaatgtattcaccgaaaacaaacatataaatcacaggagtcgcccatgtcagtacccgttcaacatcctatgtatatcgatggacagtttgttacctggcgtggagacgcatggattgatgtggtaaaccctgctacagaggctgtcatttcccgcatacccgatggtcaggccgaggatgcccgtaaggcaatcgatgcagcagaacgtgcacaaccagaatgggaagcgttgcctgctattgaacgcgccagttggttgcgcaaaatctccgccgggatccgcgaacgcgccagtgaaatcagtgcgctgattgttgaagaagggggcaagatccagcagctggctgaagtcgaagtggcttttactgccgactatatcgattacatggcggagtgggcacggcgttacgagggcgagattattcaaagcgatcgtccaggagaaaatattcttttgtttaaacgtgcgcttggtgtgactaccggcattctgccgtggaacttcccgttcttcctcattgcccgcaaaatggctcccgctcttttgaccggtaataccatcgtcattaaacctagtgaatttacgccaaacaatgcgattgcattcgccaaaatcgtcgatgaaataggccttccgcgcggcgtgtttaaccttgtactggggcgtggtgaaaccgttgggcaagaactggcgggtaacccaaaggtcgcaatggtcagtatgacaggcagcgtctctgcaggtgagaagatcatggcgactgcggcgaaaaacatcaccaaagtgtgtctggaattggggggtaaagcaccagctatcgtaatggacgatgccgatcttgaactggcagtcaaagccatcgttgattcacgcgtcattaatagtgggcaagtgtgtaactgtgcagaacgtgtttatgtacagaaaggcatttatgatcagttcgtcaatcggctgggtgaagcgatgcaggcggttcaatttggtaaccccgctgaacgcaacgacattgcgatggggccgttgattaacgccgcggcgctggaaagggtcgagcaaaaagtggcgcgcgcagtagaagaaggggcgagagtggcgttcggtggcaaagcggtagaggggaaaggatattattatccgccgacattgctgctggatgttcgccaggaaatgtcgattatgcatgaggaaacctttggcccggtgctgccagttgtcgcatttgacacgctggaagatgctatctcaatggctaatgacagtgattacggcctgacctcatcaatctatacccaaaatctgaacgtcgcgatgaaagccattaaagggctgaagtttggtgaaacttacatcaaccgtgaaaacttcgaagctatgcaaggcttccacgccggatggcgtaaatccggtattggcggcgcagatggtaaacatggcttgcatgaatatctgcagacccaggtggtttatttacagtcttaatgagtgaaagaggcggaggttttttcctccgcctgtgcgcgtcagagtttagcgaatttttcgagggtgcgaataagctgtgtgacgaagccatattcgttatcgtaccaggcgaccgttttcaccagttgtaaatcgcccacggcggtaatttccgtttgcgtggcatcaaacaccgaaccgaaatggctgccaatgatatcggaagagactatttcttcatcggtataaccaaatgactcgttattggtggttgcttgtttaagtgcgttattcacctcttcggcagtcacttttttccgagaatcgataccagttcagtgaccgaacctgttttcaccggcacgcgttgcgcatgacctttcagtttgccgctcagttccgggatcaccagaccaatggcttttgccgcccccgtagtgtggggaatgatattttctgccgctgcgcgtgaagcacgtaaatctttaccacgcgggccatccaccagtgactgggtgccagtataggcatgaatggtcgtcatcgtgccgacttctatcccgaaactgtcatgcaaggctttggccatcggcgcaagacagttagtggtgcatgacgccacggaaacaatggtgtcgttgccatccagagtgtcgtcattgacgttataaacgatagttttcatttcaccggcaggggcggaaatcaacaccttcttcgcaccagcatcaagatgcgcctgcgatttctcggcggaggtataaaagccagtacattcgacaatgatttctgcacctttcgctttccacggaatatttttagcctctttttcggcgtaaaccgcgatacttttcccatcaacgataagtgaatcttccgtaaaatcaacgctccaggggaatggtccgtagtttgaatcatgtttcagcaggtaggcgagaatttatggggaagtgagatcattaatagcgacaacgtctatgttgcttttgacttcaagtaatcgacccaacaccagtcgaccgatacgaccaaaaccgttaataccaactttactcatggttttctcctgtcaggaacgttcggatgaaaattgatcctttccaagcttagaccaggatggcgggatgggcaatctccattctcacagtgaaacgtaacgtactgaaaacgggtgaacaatatttaatgaaattttgagaaaagcccgttatgttaacggaaaattatgttaaagcaggaaatgttatggaaaataaatattcaaggttacaaatcagcattcactggctggtctttttactggttatcgcagcgtattgcgcaatggagtttcgtggtttcttcccacgtagcgatcggccactcatcaacatgattcatgtttcctgtggcatctcaattctcgtgctgatggtcgttcgtcttttgttaaggctgaaatacccaaccccgccgattatacctaagccaaaaccgatgatgacgggactggcgcatttgggacatttggtgatttatctcctgtttattgcgctgccagtgattggtttggtgatgatgtataaccggggcaacccgtggtttgcgtttggtttgacgatgccttacgcttcagaggccaatttcgaacgggtagatagcttaaagtcgtggcatgaaacgctggcgaatctgggatattttgtcatcgggttgcacgctgcggctgcactggcacaccactatttctggaaggacaacacacttctacgcatgatgccgcgtaaacgttcctgaaggatatttaaagaaaacgcctgtactaaaaccgacccgtggtacaggcgaagaatacgggtctacatcggaagcgcctattatatttatttgtatgataaataaaaccataatccttgcccatacgtccatctggcttatttttaatcaattcacccgatctttgatctcatcaacggtatcaaaataaaccagcgtataacgttcaaatcgaacataagattcgataaaccatggaggttatatgaaaaaactggcacttattttgtttatgggaacgcttgtttccttttatgccgatgccgggcgcaaaccctgttctggttcgaaaggggggatctcacactgtacggcaggcggcaaatttgtctgtaatgatggttctattagtgcatcgaaaaaaacatgcactaactgaagtgtaaaaggggtgccatgagaaaatgaatctgctagtcaaatgcgcggggaaaatccccgcgcttgcccttacctggacgtgcaggccatgagcgcagcaacctccttatcaccgtcccggaaccgcagttcgtagagcgtttgtcgggtcaggagtgtgaatgtcagaatcgtaatgcagataatgagcagacacaccaccagagggttgtgcttcatagcctttctccttgccggatggcgggtaagaggctaagatctgaattgctaggttcattcgttggcctcggttgatagaaatatcggtcggggccttcgtctttctgattcccggttagcctgaaaacagaaagtctcaggcacccgcaggcatcctatgaggtttccttagggacgaaaataatcacttcacgaaattgcgtgctgttttccagaatttttcgtcattcgggttagccagtttagccattcgttactctcttcattccaatagcattaattttctatgcaataattgttgtaaaaatgtgacgcaaagaggtttttggtcataagtaattaccgtcaagtgccgatgactttctatcaggagtaaacctggacgagagacaacggtaatgaatacaactccctcacagcgattaggttttttgcatcacatcaggttggttccgttatttgcctgcattctaggcggtatcttagttctattcgcattaagttcagccctggctggctatttcctctggcaggccgatcgcgatcagcgtgatgttactgcggagattgagattcggaccgggttagcgaacagttcagattttttgcgttcagcccggatcaatatgattcaggccggggctgcgagtcgtattgcggaaatggaagcaatgaagcgaaatattgcgcaagccgaatcggagattaaacagtcgcagcaaggttatcgtgcttatcagaatcgaccggtgaaaacacctgctgatgaagccctcgacactgaattaaatcaacgctttcaggcttatatcacgggtatgcaacctatgttgaaatatgccaaaaatggcatgtttgaagcgattatcaatcatgaaagtgagcagatccgaccgctggataatgcttataccgatattttgaacaaagccgttaagatacgtagcaccagagccaaccaactggcggaactggcccatcagcgcacccgcctgggtgggatgttcatgattggcgcgtttgtgcttgccctggtcatgacgctgataacatttatggtgctacgtcggatcgtcattcgtccactgcaacatgccgcacaacggattgaaaaaatcgccagtggcgatctgacgatgaatgatgaaccggcgggtcgtaatgaaatcggtcgcttaagtcgtcatttacagcaaatgcagcattcactggggatgacagtagggactgttcgacagggcgcggaagagatttatcgtggcaccagcgaaatttcagctggcaatgcggacctgtcatctcgcaccgaagaacaagcggcggctatcgaacaaactgccgccagcatggagcaactcactgcgacggtgaaacagaatgcggataacgcgcatcatgccagcaaactggcgcaagaggcttctattaaagccagcgatggcgggcagacggtttccggtgtagtaaaaacgatgggcgctatctccacgagttcgaagaaaatttctgagatcaccgccgtcatcaacagtattgctttccagacgaatattctggcactgaatgctgccgttgaagccgcgcgagcgggtgagcaagggcgtggatttgccgttgtcgccagcgaagtacggacactcgcaagtcgcagcgctcaggcggcgaaagagattgaaggcttgatcagtgaatcagtcaggttaattgacctggggtcggatgaggtggcaacggccgggaaaaccatgagcactattgttgatgccgtcgcgagtgtcacacatatcatgcaggaaatcgccgccgcctcggatgaacaaagtagaggcataacgcaggttagccaggcgatttctgaaatggataaggtgacgcaacagaatgcttctctggtagaagaggcctcagcggcggcggtgtcccttgaagaacaggcggcacgattaactgaggcggtggatgtattccgtctgcacaaacattctgtgtcggcagaacctcgcggagcgggtgaaccagttagtttcgctacggtgtgaaaatgttcaaggagggatcgacagatcccttcacctttcagaacggcattgattttcgaatagcgttaatcatcaactggcaaccagaagagaacgtcgcatctacgcgggtcagtattccaatcggttcgcctgcaccatgtcccggaacaggcagggccaccagcgtggcatgacgcaggtcgtcttttacagcgccagaagggacaaaccacacgtaatcgtattcaaccgtaagttgacgagatagcgaagcagacagcgtttcgatacaacccgaaggaattttacagccctggctctgcactaatgcatctgaatgctggcgtggcgcagtgccttctggtgatacaacgaccggccattccagcacccggcttagcgttacgttctcctgaagtagcgggtgattagggcggacaaccagcttcaacgattcaagaaacagcagttcgtaattaagcccggtcatcagttcaggatctgacatccgaccaatgccgatatcgatttccccggtttttaaacccgccagaatcatagggttactcattgtcgcaacttgcaaggtcgtctctttttgttgctgatgaaactgacctataaccgaaggtaatatccccagtgccgcagtaggtagtgcaccaaccctgacgacatcattattaagaccttctttacgatgaagcgaccgtccggcagtgttgatggcgtcaagaactctgactgcatgcgttaaaaattgttcgccgggtaaggtaagttgcgccccctgacgaccacgctcaaacaagcgagcgccagtcagctgctccagttcattcaatgtcttagagagcgcaggttgactcaaattaagggtttcagccgcgcgccccaaagttccttgttgtgcgacagctacgaatgtatgaaggtggcgcaaacggatgcgctgactaaacagactatttttttccataagcgatgttaaaaacgaagcggtgtcgctgacaagtgaagttgtttgattatgataacttgattgcaaaatattattaacaattaaagcaattatgttacagcaaaatggataatattgatgttttcgcggcgagatcacagtttgtaaattcttcccgcaagagtgaatgcggttacctacactccagattactgaccactggaggcagacactatggcgaacagcatcacggcggatgagattcgggaacagttttcgcaggcaatgtcagccatgtaccagcaagaagttccgcaatatggcacgctgctggaactggtagctgatgtgaatctggctgtgctggaaaacaatcctcaactgcacgaaaaaatggtaaatgcagacgagctggcgcgactgaatgttgaacgtcatggggcgattcgcgttgggactgcacaagagcttgctactcttcggcggatgtttgccattatggggatgtacccggtgagctattacgatctctcgcaggcaggggtgccggtacattcgacagcatttcggcccattgatgatgcttctctggcgcgtaatcccttccgcgtttttacctccttactccgccttgagcttatcgagaacgaaattttgcgccagaaagcggcggagattctgcgtcagcgcgatatcttcaccccacgttgtcgacaactgttagaggaatatgagcagcagggcggttttaacgaaacacaggcacaggagtttgtgcaggaagccctggaaacgtttcgctggcaccagtcagcaacggtagatgaagaaacctatcgcgcattgcacaacgaacatcggttgattgctgatgtggtctgttttcctggatgccatatcaaccacctgacgccacgtacgctggatattgaccgggtgcagtcgatgatgcctgaatgcggaattgaacccaaaattctcatcgaggggccgccgcgccgcgaggtaccgattttactacgccagaccagctttaaagcactggaagagacggtgttgtttgcggggcagaaacagggcacgcataccgcgcgctttggtgaaattgagcagcgtggcgtggcattaacgccgaaagggcgacaactgtatgatgatcttctgcgtaacgctggaaccgggcaggataatctcactcaccaaatgcatttacaggaaaccttccgcacttttcctgacagtgagtttttaatgcgtcagcaagggttggcatggttccggtaccgtctgacgccttcgggtgaggcgcatcgtcaggcgattcatcctggagacgatccacagcccttaattgaacgtggttgggtagtggcgcaacccatcacctatgaagatttcttgcccgttagcgcggcggggatcttccagtcaaatctgggtaatgaaacgcagacacgcagtcacggtaatgccagtcgcgaagcatttgagcaggcgttgggttgtccggttttggatgagttccagctttaccaggaagcggaagaacgcagtaaacgtcgctgtggtttgctttaaaatctgaccatccgcctttgcaaaaatttgcctgattttacaaacgaatcaggctcatcccatcgacataaaaaaaatgccgatttatgcatattctctcagttcaacaattggattattaataaatattgtctagagtgagcggtcataaataagcactttcttgccgctgaaaacgaccagcgcgggaccattcacaacaccagaaggactcactttcaggtatggatcgtagacgatttattaaaggttcaatggctatggccgccgtgtgcggtaccagcggcattgcttctcttttttctcaggcggcattcgcggcagattctgatattgccgacgggcaaacccagcgttttgacttctccattctacagtcaatggcgcacgacttagcgcaaacagcgtggcgtggtgcgcctcgtccgttacctgacacgctggcgacaatgacgccgcaggcttataacagtattcaatacgacgccgaaaaatcgctctggcataacgttgagaaccgtcaactggacgctcagttcttccatatgggaatgggattccgtcgccgcgttcgtatgttttctgtagatccagcaacacatctggcgcgtgaaattcactttcgcccggagttgttcaaatacaacgatgcaggtgttgatacaaaacaattagaagggcaaagcgatctcggctttgccggttttcgcgtgtttaaagcccccgaactggcgcgccgtgatgtagtatcatttctcggcgcgagttatttccgcgccgttgatgatacatatcaatacggtttgtcggcccgcggcctggcgatcgacacttacaccgacagtaaagaagagttccccgactttaccgccttctggtttgatacggtaaaaccgggggcaactacctttaccgtttatgcgttgctcgatagcgccagcattactggtgcctataagttcactatccattgtgagaaaagtcaggtgattatggatgtggaaaatcacctgtatgcgcgcaaagacattaaacagctgggcattgcgccgatgaccagtatgttcagctgcggtactaatgaacgtcggatgtgcgatacaattcatccgcaaattcatgactctgatcgtctgtccatgtggcggggcaacggcgagtggatttgccgtccgctgaataatccgcaaaaattgcagttcaatgcttacaccgacaacaacccgaaagggtttggtttattgcaactggatcgtgacttctcccattatcaggacattatgggctggtataacaaacgcccaagtctgtgggtggaaccgcgtaacaagtggggtaagggcaccatcggcctgatggaaatcccaacaacgggcgaaacgctggataacattgtctgcttctggcagccagaaaaagctgtaaaagcaggtgatgagtttgcattccagtatcgtctgtactggagtgcgcaaccgcctgttcattgcccattagcgcgcgttatggcgacgcgtaccggcatgggcggtttctcggaaggttgggcgccaggtgaacactatcccgaaaaatgggcgcgtcgttttgccgtcgatttcgttggtggtgatctgaaagctgccgcgccaaaaggcattgagccggtgattacgctttccagtggggaagcgaagcaaatcgaaattctctatattgaacccatcgatggttatcgtattcagtttgactggtatccgacttcggactccactgatccggtcgatatgcggatgtatctacgttgtcagggggacgctatcagtgaaacatggctgtatcagtatttcccgccagcgccggataaacgtcagtatgttgacgaccgcgtgatgagttaatcgttttttcttcggcaccttcttcgggaggtgccgtctggttaaacacgatcccgctcgcatttttccctaagttaaatgagtaatctgatggtgtgtatttcagatacaccttgtcagccactaacagggagtgcgtatgtttccagaataccgagatttaatatcccgtctgaaaaacgaaaatcctcgctttatgtccttgttcgataaacacaataaacttgatcatgaaattgccagaaaggaaggttccgacggtcgagggtacaatgcggaagtggtccgcatgaaaaaacaaaagctacagttaaaagatgagatgctcaaaatcctgcagcaggagagcgtcaaagaggtgtaaactttcctaagccgccagccaggcggcttttttaacaactgcatggattgactggagataagatgactgaaacgataaaagtaagcgaatcacttgaattacatgctgttgcagaaaatcacgtcaaacctctttatcagttaatctgtaaaaataaaacctggttacagcagtcgctaaactggccgcagtttgttcaaagtgaagaggacacgcgaaaaacggtgcagggtaatgtgatgttgcatcaacgcggctatgccaaaatgttcatgattttcaaagaagatgaacttatcggcgttatctcgtttaatcgtattgaaccactgaataaaaccgctgaaataggctactggctggacgaatctcatcaggggcaggggatcatttctcaggcgctgcaggcattgattcatcattacgcccagtctggtgaacttagacgcttcgtgatcaaatgtcgggtggacaatccgcaaagcaaccaggtcgctttgcgcaatggttttatccttgaaggttgcctgaaacaggctgagttcctgaatgatgcctatgatgatgtgaacttatacgcgcgtattatcgattcacaataaccctgccagcggcgttcgcgtaatgcgctcctcgccgttaatgacttttggaccacggacatgaaccgtgtcgccatcaaaggcttcaacgacggcgtggtcggttaactccacatggttttcaattatcaccgcacctgtaatacggctctcaccttgtatgacaacgtgctcgtcgagcagaatcggtccgccacgtaccacggcatttccgccaaccaagacatgatgttttaacacacaattaccttccacaatggcatattccgccacctgcgaactgtaatgaatcgtcggaatggcatcttcttctatgccagctttcacctgcgcgtgaccgtagactttagcgcaatcgcatagccagacattgttctcttcattaccttcaatactggcaaaatcaaaaacttcggcgcgatgttcaataaaagcataccggacgacggcatcgccataaatttgtgcctggtggacaatacgcgaggcgctaacccttgcgcgatcataaatttggagcaggagttgatggtcgggcgttaagccttgtgcggcgacgatcatagaatgttgatcaattaaggcgtgaccaaatattctacattgcccgtaaactaatgagtcatgaatggtgacgctgtcacttatatatgcaccctggctgatttcactattatcgatccagacgttatccgttgcgtaaacctctccccacagcacgctggtgccggtgatacgcgtattaccggaaatcaccgctccgccgaacgcaatagcattctggtcgtaaatccagcaatttccttcttgtgctaacaccgtttcgcgatcgatccagccgccagcggttcctgctatcacatcgttaaaatcgctaatggcgataatctgccgtaataacacattttttttagtgccatcttcctgataactaaaggctcgctgttcttcacttagacgatatttgcgcatagcgttttcccacaggtgacttactataaccgtagcaaattctgcggctctggctatgctcgagaaaattccataaaatgcatttcaaatatactttataaattaaacaaaatgagtaagaagatgcagagcgataaagtgctcaatttgccggcaggctactttggtattgtgttggggacgatagggatgggatttgcctggcgctatgccagccaggtttggcaggtcagccactggttaggggatgggctggtgattctggcgatgatcatctggggattattgactagcgcatttattgcccgactcatacgctttccgcatagcgtgctggcggaagttcgccatccagtgctgagcagttttgtgagtttgtttccggcaacgacgatgctggtggcgattggttttgttccgtggtttcgcccactggcggtgtgcctgttcagttttggtgtcgtggttcagttggcttatgccgcctggcaaactgcgggattatggcgcggatctcaccctgaagaagctaccacgcctggactgtatctgccgacagttgccaacaactttatcagcgcaatggcctgtggtgcgttgggctacaccgacgccggtctggtgtttttaggcgcaggcgttttctcatggctaagccttgaaccggtgatcttgcagcgtctgcgcagttcgggagaattacccacggcactgcggacatcactcggcattcagctcgctcctgcgctggtggcttgtagtgcctggctgagcgtcaacggcggcgagggtgacacgctggcgaaaatgcttttcggttatggactgctgcaactgctgtttatgctacgtctgatgccatggtatctctcccagccatttaatgcttcattctggagtttctcgttcggcgtatctgcactggcaaccaccggtttgcatctggggagtggcagcgataatggatttttccatacgctggcggtgccgctgtttatctttaccaattttattattgcaatactgctcatccgtacttttgcgcttctgatgcagggaaaattgttagtcagaaccgagcgcgccgttttaatgaaagcagaggacaaagaatgatcattcgtgacgaaaactattttactgataaatatgaattaacccgcacacactctgaagtactggaagcggtgaaagtggttaaaccgggtaaaacgctggatctgggctgtggcaatggtcgtaacagtctttacctggcagccaatggttatgatgttgacgcatgggataaaaatgccatgagtatcgccaacgtcgagcgcattaaatccattgaaaatctggataatttacacacccgagtcgttgatctgaataacctcacatttgatagacagtacgattttattctttcgactgtggtgctgatgttccttgaggctaaaaccatccccgggttgattgccaatatgcaacgttgcactaaacctggtggttacaacctgattgtggcggcgatggataccgctgattatccatgtaccgtcggcttcccgtttgccttcaaagagggagaattacgtcgatattacgaaggctgggagagggtgaaatacaatgaagacgtcggcgagctgcaccgcaccgacgccaacggtaatcgtattaaactgcgtttcgccacgatgctggcacgtaaaaaatgacccggtaagcacaaaacgcgtgaaaattccccacgctgagatgatttactgttcttcttttcggtaagcatattttttatcgaagggatgtgaaattaatcacagtagtcgaagtttttagcagcttaacttactgaaatttaagtactgatgattgacttagcccctttttcggcattgactatgtcgtctgaaaaggggctgaaaaatttattttcaccaacactttttttgccacaacacgaagcggcgctttttgctataacttagaaagtaatataatcatctcaggaaactattcatgcgtaccacatcatttgcgaaagttgcagctttatgcggcttattggctctgtctggttgtgcatctaaaatcacccagccagataaatattctggttttttaaacaattactctgatttaaaagaaacaacctcggctacaggtaaacctgttttacgttgggtagacccgagttttgatcaaagcaaatatgacagcatcgtctggaacccaatcacttattatccggtaccgaaaccgtcgacccaggtagggcagaaagttctggataaaattttgaactataccaacaccgaaatgaaagaagcgatagcgcagcgtaaaccactggttaccaccgctgggccgcgtagtctgattttccgtggggccattaccggtgtagataccagcaaagaagggctgcaattctatgaagtggttcctgttgcattagtggttgcggggacgcaaatggctacaggccaccgtaccatggatactcgcctctattttgaaggtgagctgattgatgcagcgactaataaaccggttatcaaagtcgttcgtcagggcgaaggtaaagacctgaataacgaaagtacgccaatggctttcgaaaatattaaacaagttattgatgacatggcgaccgatgccaccatgtttgacgttaacaaaaagtagttccagacgcgccatcgttagatggcgctttttatccggtgcgccgtaaaaccccatccttcagggcggggatataaggcgcggttttccacctgaccaggtgtttgctgttgttcaatgtattggcggatgacggatattggcgcacctccgcagctactggcaaaatagccaggactccacaaaacgcctttgtagtaatacctgaatgcaatatctggtcgatctcgtcgcagtcacctacccgatacgcctttgaggctgtttaccagactggatatcgccagtttgggaggatagttaattaacaaatggacgtgatctggttcgccatccatttcaaccagttcagcttcaaaatcagcacatacatttgaaaagtaagtgcgtagtttttctgtcgcgtcatggtcaaaaatctggcgtcggtatctggtgacaaagagcaggtgaacatgcatcaggaaaacacaatgccttccacgccggatatcggtttcttttttcacagaccaaagtatcatttgacctgtgaaacgattacaggcatttaaattccagttaagacccggtggtcaacaggagtgtgaaatgaggcgcttcgcaggcgcatgtcgtttcgttttcaatcgtgctctggcacgtcagaatgagaatcatgaggccggtaataaatacatcccttacgggaaaatggcttcctggctggttgagtggaaaaatgccactgaaacgcaatggcttaaagattctccctcacagccattgcaacagtcactgaaagaccttgagcgggcttacaaaaacttcttccggaagcgggctgcttttccccgattcaaaaagcggggacagaatgatgcattccgctacccgcagggcgttaagctcgatcaggaaaacagccgtatttttctgccgaaactgggctggatgcgctaccggaacagccgtcaggtcacgggtgttgtgaaaaatgtcactgtcagccagtcctgcggtaagtggtacatcagtattcagacagaaagtgaagtatcaactccggttcacccttcagcatcaatggtcgggctggatgctggcgtggctaaactcgccacgctgtcagatggcacagtctttgagcctgtaaacagttttcagaaaaaccagaagaagctggcgagacttcagcgacagttaagccgcaaggtcaaattcagcaacaactggcaaaagcagaaacgcaaaatacagcgactgcattcctgtatcgcaaatatccgcagggactaccttcacaaagtcacaacggccgtcagcaaaaaccacgcaatgatagtcattgaggatttgaaggtcagcaacatgtcaaagtcagcagcgggtacggtcagccagccggggcgcaatgtccgggcaaaatcaggtttaaaccgttcgatactggatcagggctggtatgaaatgcgccgccagcttgcgtataagcagctctggcgtggcggtcaggtgcttgctgttccgccagcgtatacaagccagcgttgcgcgtactgtggtcatacagcgaaagagaaccgcctgtcacaaagtaaattcagatgccaggtatgtggatatacagcgaacgccgatgtaaatggcgctcgcaacattttagcggcggggcacgccgttcttgcctgtggagagatggtgcagtcaggccgcccgttgaagcaggaacccaccgaaatgattcaggcgacagcctgaacgtagcagggatccacgtccttcagggcgtggaggatgtcaatatcggtttctgtcagcgattaaattcaacaccacgtaacaaacgcctccggcaattaatccccaaaacgcagaaccaatcccgaccagcgtcaatccacttgccgttaccagaaatgccaccaccgccgcgtctcgctcacgctcattatgcagcgcctgatacaaactgccgccgatggtacttaacagcgccagacctgccagcatctggatccaacttacgggcagggcagccatcatcccggtaatggcactaccaaacagacctgcgagcaaatagaaaatgcctgcaacggcagcggccagccaacgttgatctttatccggatgcgcttccgggctttggcaaatagccgcggtgattgccgcaataccgacggaataaacgccgaaaggggaaaaaaccagtgccagcaatccagtaaatacaattaatggcgaaacaggagccgaatatccagctgctttcattgctgcgatacccggtgcgttttgcgatgccatcgtcaccagaaaaagggggagtgcaacgctcaggctgtgagcaaacgaaaaatcaggggtaatataagtggggagaacgggtttaaagacaacatcagttgtgacaacgtcaccttgcgcgatgacgatcacgatcccaataatcatcgcggcaattaccgcatagcgcggcgcaacggccttggttgccagccataccagcaacatacttccacacaacgtaaattgaccgtccagactggcaaacgcctgtaaaccaaagcgtaataaaatcccggcaagcattgccgccgcaagcgagtgcggaataatgcgcatcagacgagcaaagagtcccgttatgccgcagaggactattagcgcgttggtgacaataaaaacgccgatggcttcgttaagtgttagtccctgcaatccggtgaccaacaaagccgcgccaggcgttgaccatgcggtgagaacaggtacgcgataccataatgtcagagtcagcgtactgacgcccattgccagccccagcgccgtcatccagccagagatttgtgcagtggtggctccggcgacaatcgctgcttgccagattattgccgctgaactggcgtagccaattaataccgccagaaaccccgccagtagcgtgggtggaggaatagaaaacagacgcatagtcacctcgtgcgttatagcgtacaggcaccgtagcatttgtccgttataacgcacaagtgataaacttccgttttgccggaggagtcgcatggaaaatctcgctcgctttttatccaccacacttaaacaactacgccagcagcgcggctggagtctttcgcgactggcagaagcgacgggcgtttctaaagcaatgttagggcagattgagcgtaatgagtccagtccgacggtcgcgacattatggaaaattgccaccgggttgaacgtaccattttcaacatttatttctccgccgcagtccgctacgccttcagtttatgatccacaacagcaggcgatggtgatcacttcgctgtttccttatgatccacaactctgctttgaacacttctcgattcagatggcatctggtgcaataagcgaatcgacgccccatgagaagggggtaatcgaacatgtcgtcgtcattgatggacaacttgatctgtgcgttgatggggaatggcagacccttaattgtggggaaggcgttcgatttgctgcagacgtcacgcatatctatcgtaatggtggggagcaaaccgtacattttcattccctcatccattacccgcgcagttaagcgggaaaactatttcgcaacgtcgcgcttgtggctaaaatagccgccatttttcagctactggataagaatgtgaccgtatcttctcatcgacttgaactgttaagcccggcacgcgatgccgccattgcccgcgaagctattttgcacggtgccgatgctgtttatatcggcggccctggttttggtgcccgtcataatgccagtaatagcttgaaagatattgccgagctggtgccgtttgcccatcgttatggtgcaaaaattttcgtcacgcttaacaccattttgcatgatgatgagctggaacccgcgcaacggctgattactgacctctaccagaccggtgtcgatgcgctgattgttcaggatatggggattctggaacttgatattccgccgattgaactgcacgccagtacgcagtgcgacattcgtacagttgaaaaagcgaagttcctctctgatgttggcttcacgcagattgtgctggcgcgagagctgaatcttgatcagatccgcgcgattcaccaggctacggacgcgaccattgaattctttattcatggggcactgtgcgtggcctattcgggtcagtgctacatttctcatgcgcaaacagggcgtagcgccaaccgtggcgattgctcgcaggcgtgccgtttgccatacacattgaaagacgatcaggggcgggtggtttcctatgaaaaacatctgctgtcgatgaaagataacgatcagactgccaacctcggcgcgctgattgatgctggtgtacgctccttcaagattgaagggcgttacaaagatatgagctacgtgaagaatatcaccgcccattatcgccagatgcttgatgccattattgaagaacgtggcgatctggcgcgcgcttcatcaggtcgtactgaacatttctttgttccatcgacggaaaagactttccaccgtggtagcacagattattttgtgaatgcccgtaaaggcgatattggcgcgttcgattcgccgaaatttatcggcctgccggtaggcgaagtagtgaaagtggcgaaagatcatctcgatgttgccgttaccgagccactggcaaatggcgatggcctgaacgtgttgattaaacgtgaagtcgtcggttttcgtgccaatacggtcgagaaaaccggagaaaatcagtaccgcgtctggcccaatgaaatgccagcagatttgcacaaaattcgtccacatcacccactaaaccgtaatcttgatcataactggcagcaggcactgacaaaaacctccagcgaacgtcgggtggcggtagacattgaactgggcggctggcaggaacaactgattctgaccctcaccagtgaagagggtgtcagcatcacgcatacgctggacgggcagttcgacgaagccaataacgccgaaaaagcaatgaacaatctgaaggatggtctggcaaaactggggcaaaccctctattacgcccgcgatgtgcaaattaatttgccgggggcgctgtttgtaccaaacagtctgttaaaccagttccgccgtgaagctgctgacatgctggatgctgcgcgtcttgccagttaccagcgcggcagccgtaaaccggttgctgatcctgcgccggtttatccgcaaacgcatctgagtttcctcgcgaacgtatacaaccagaaagcgcgtgaattttatcatcgctatggtgtgcagctgattgacgcggcgtatgaagcacatgaagagaagggcgaagtcccggtgatgatcaccaagcattgtctgcgctttgcctttaatctgtgcccgaaacaggcgaaaggcaatatcaaaagctggaaggcgacgccaatgcaactggttaacggcgatgaagtattaacgctaaagtttgattgccgcccatgcgagatgcacgtcattggcaaaatcaaaaatcacatactgaaaatgccgttaccgggaagcgtagtggcatccgtaagtccggatgagctgctgaaaacattgccgaagcgaaaagggtaaaacgccagttttctggttactcacaacttattgaatctgcatgatattgcctgccgggtaaggcgttacgccgcatccggcatcaaatgactcaacgttgtcccgcttctggtttgcgcgatttttgccagtaaaaatgctcgcgcaaaccttccgccgactcttccgccacagcacgcaattcatcgctgtccgcttcatgacgcagctgatgatccacattctttacccacacaaattcatgtcctttgtgccctgccatgagttgtcctgaaaacagagcacacgttaataagacaaccgataacgccttcgtaaacatcctgccacctttttcttaccttttgccgctatgatgccgatcgtttcttgaggttattattcagttttgcaaattagcgcaaagaaattctggaatcttccttcctgattttgcattgcattctgccgttgcggcgatttagtgctattttcgagcaaattacacacggaggtaaacactaatgtttactttgttgatatactcagcggcagggaggcgatgtgaaacaaagcgagttcagacgttggctcgaatctcagggcgtcgatgtagcgaatggcagcaaccatttgaaactcaggtttcatgggaggcgcagtgtcatgccgcgtcacccctgcgatgagattaaagaaccattgcgtaaagcaatcctgaaacaactcggtttgagttaatcgccaattaaaaaggttaatgacatgcgagagacagtcgaaattatgcgttatcccgtcactcttacacccgcgccggaaggcggttatatggtttcttttgtggatatccctgaagcgttgacccagggcgaaactgtcgctgaagcgatggaagcggcaaaagatgctttactgaccgcatttgatttttattttgaagataacgagcttatccctttaccttcgccattaaatagtcacgatcactttattgaagtacctttgagcgtcgcctctaaggtattgctgttaaatgcttttttacagtcagaaatcactcagcaagagttagccaggcgaattggcaaacctaaacaggagattactcgcctatttaacttgcatcatgcgacaaaaatcgacgccgtccagctcgcggcaaaggcgcttggcaaagagttatcgctggtgatggtttaattacagttaacgaaaagttgtcatttttaacaactgatatagactgccgaatcatctgcacataattacgattcgataatgaaaaaataccagcagcttgcagaacaattacgcgagcagattgcgtcgggtatctggcaacccggcgatcgtttgccttcgttgcgtgaccaggtggcgctttcaggcatgagctttatgactgtcagccatgcctatcagttgctcgaaagtcagggatatattatcgcacgaccgcagtcgggttattacgttgcgccacaggcaataaaaatgccgaaagcgccagtcattccagtcactcgagatgaagcagtcgatatcaacacttatatttttgatatgttgcaggccagtcgcgatccgtcggtcgttccgtttgcctcggcctttcccgacccgcgacttttccccctccaacaactaaaccgctcgctggcgcaggtaagcaaaaccgccacagcgatgagcgtgattgaaaacttaccgccaggaaacgcagaactgcgtcaggctattgctcgtcgctatgccttacagggcatcaccatttctcctgatgaaattgtcattactgccggggcgttagaggcattaaacctcagtttgcaagcggtaactgaaccgggcgattgggtgatagtagagaatccttgtttctacggtgcgttgcaggcgctggagcggctacggctgaaggcgttatcggtggcgacggatgttaaagaagggatagatcttcaggcgctggaactggcgttgcaggagtatccggtgaaagcgtgctggctgatgactaatagccagaatccactcggatttaccttaacgccgcaaaaaaaagcacaactggtggcgttgctcaatcagtacaacgtaacgctgattgaagatgacgtttacagcgaactttattttggacgggaaaaaccgctgcctgcgaaagcgtgggatcgccacgatggcgttttgcattgctcttcgttttcgaaatgtctggtgcctggttttcgtattggttgggtcgccgccggaaaacatgcacgtaaaattcaacgcttgcagttgatgagtacgctttccaccagctcaccgatgcaacttgcgctggtggattacctttccacgcgccgatacgacgcccatcttcgtcgcctgcgtcgccagcttgcggaacgtaaacaacgtgcctggcaggcactgctgcgttatctgcctgcggaagtgaaaattcatcataatgacagtggttactttctctggttggagctccccgagccgttagatgccggcgaattaagcctggcggcactgacgcatcatatcagtattgcgccgggtaaaatgttttctaccggtgaaaactggtcacgttttttccgttttaataccgcgtggcagtggggagagcgtgaagaacaggcggtaaaacaattaggcaaacttattcaagaacggctgtaatagcgtttaatttaattcctcttagattgggtaatatgaatttcgaatagcagtcatatttcctaactccttgactatactccagaagataaccttacagacggcataatgcgcggtagctcacaacctgaataaattttctcaggggcgaaggtgtgcctgcaagccgccgtctatggttaaacaaggagatatttttacggcacggcggctgaacaattaattacgacaggagtaagaccttatgagcaagacatttgcccgcagcagcctgtgtgcgctcagcatgacaataatgaccgctcacgccgccgaaccgcctaccaatttagataaaccggaagggcgactggatattatcgcctggccgggatacatcgaacgcggacaaactgataaacaatacgactgggtaacgcagttcgaaaaagagacaggctgcgcggtgaatgtgaaaaccgccgcgacttccgatgaaatggtcagtctgatgaccaaagggggttacgatctggttacggcatccggcgatgcctcgctgcgtttgattatgggtaaacgcgtgcagccgattaataccgcattgattcccaactggaaaacgctcgatccgcgcgtggttaaaggcgactggtttaatgttggcggcaaagtttacggcacaccttaccaatgggggccgaacctgctgatgtacaacactaaaaccttcccgacgccgccggatagctggcaagtggtttttgttgagcaaaatctgccggacggcaagagcaataaaggccgcgttcaggcttatgatggccctatctatattgcggacgctgcgttgttcgttaaagccactcagccgcagttgggcatcagcgatccgtatcaactcaccgaagaacagtaccaggcggtgctgaaagtgctgcgcgctcaacacagtttgatccatcgctactggcatgacactaccgtgcaaatgagcgatttcaaaaacgagggtgtggttgcttccagtgcctggccctatcaggccaacgccctgaaagccgaaggccagcctgttgctaccgttttcccgaaggagggtgttaccggttgggctgataccaccatgctgcatagcgaagcgaaacatccggtttgcgcctacaaatggatgaactggtcattaacgccaaaagtgcagggcgatgtggcggcctggtttggctcgttaccggtagtgccggaagggtgtaaagccagtccgttattaggcgaaaaaggttgtgaaaccaacggttttaactatttcgacaaaatcgccttctggaaaacgcctatagcagaagggggcaagtttgttccctacagtcgctggacgcaggattacattgccattatgggcggtcgctaacttcgctggggtgctttatgacgtacgcagtggagtttgacaacgtctcgcggttgtacggtgacgtgcgcgcagtagatggcgtcagtattgcgataaaagatggtgagttcttctctatgctggggccgtccggctccggcaaaaccacctgcctgcgcctgattgctggcttcgaacagctttccggcggggctatctctatctttggtaaacccgccagcaatctgccaccgtgggagcgggacgtgaatactgtctttcaggactacgcgctatttccgcatatgtcgattcttgacaatgtcgcctatgggctgatggtcaaaggcgtgaataaaaagcagcggcacgcaatggcgcaagaggcgctggagaaagtggcgttggggtttgtacatcaacgtaaaccgtcacaactttctggtggtcagcgccagcgggttgctatcgccagagcattggtgaatgaaccgcgcgtattgctgttggatgaaccgctcggcgcactggatctcaaattgcgtgagcagatgcagctggaactgaaaaaactgcaacagtctctcggtatcacttttatcttcgttacccacgatcagggcgaagcgttatcgatgtccgatcgtgtggcggttttcaataatggacgcattgagcaggtcgattccccgcgcgatctctatatgcgcccgcgcacgccgtttgttgccgggttcgttggtacatcgaatgtttttgatggactgatggcagagaaactttgtggcatgacgggaagcttcgccctgcgaccggaacatatccgcctcaacacccctggtgaactgcaggccaatggcacgatccaggcggtgcaatatcagggcgcggcaactcgttttgaactgaaattgaacggcggtgaaaaactgcttgtgagtcaggccaatatgacaggcgaagaactgcctgccacgctcacgcccggacaacaggtgatggtttcctggtcgcgtgatgtgatggtgccgctggttgaggagaggtgaatggcgatgaatgtattgcaatcaccttcacgtccaggtctgggtaaggtgtccggtttcttctggcataatccggggctggggctgtttttactgctgcttggcccgctaatgtggtttggcattgtctatttcggctcgctgctgacactgttatggcagggattttatacttttgacgatttcaccatgtcggtaacgccggaactgacgctggcgaatatccgtgcgctgtttaatccggcgaattacgacatcattctccgcacgctgactatggctgtggcagtcactatcgccagcgccattctggcttttccaatggcgtggtatatggcgcgctataccagcgggaaaatgaaagcgtttttttatattgcggtaatgttgccgatgtgggcgagctacattgttaaagcctatgcctggacgttattgctggcaaaagatggcgtggctcagtggtttttacaacatcttgggctggaaccactgctgactgcgttccttacattacctgcggtgggcggaaatacgctgtcaacttccgggctggggcgctttctggtgtttctctatatctggttgccgttcatgatcctgcccgttcaggcggcgcttgagcgtttgccgccgtcattgttgcaggcgtcggctgatctcggcgcacgtccacgacaaacctttcgctatgtggtgctgccgctggcaatcccgggtattgccgctggctctatctttaccttctcactcacactgggcgattttatcgtcccgcagctggttggtcctccaggatattttatcggcaatatggtttattcccagcagggggcgattggcaatatgccgatggcggcggcattcaccctggtgccgattattctcatcgcactgtacctggcgttcgtgaaacgtctgggagcgttcgatgcactctgaacgcgcaccgtttttcctcaaactggcggcctggggcggcgttgttttcctacattttcccatcctgataatcgccgcctatgcgtttaacactgaagatgcggcgtttagttttccaccgcagggcctgacgctgcgctggtttagcgtggcagcacagcgtagtgatattcttgatgccgtgacactgtcacttaaagtggcggcgctggcgacattaattgcgctggtgttagggacgctggcagctgccgcgctgtggcgacgagactttttcggcaaaaacgccatttcgctgttactgctgctgcccattgcgctgccgggcattgtcactggtctggcgttattaaccgcctttaaaaccatcaatctggagccgggatttttcaccatcgtggtcggtcatgcgactttttgtgtagttgtggtgtttaacaatgtcatcgcccgttttcgccgcacctcctggagtctggttgaggcgtcaatggatcttggggccaatggctggcaaaccttccgctacgtagtgttgccgaatctcagttcggcgttactggcaggaggaatgctggcgtttgccttgtcgttcgatgaaatcatcgttacgacctttacggcaggtcatgaacgaacgttaccgttgtggttgctcaatcagcttgggcgaccgcgtgatgtaccggtaactaacgtggtggcactgctggttatgttggtaacaaccttgccgatcctgggggcctggtggctaacccgcgaaggcgacaatggtcaataaccactgatacaggaatatgctatgcaacataagttactgattaacggagaactggttagcggcgaaggggaaaaacagcctgtctataatccggcaacgggggacgttttactggaaattgccgaggcatccgcagagcaggtcgatgctgctgtgcgcgcggcagatgcagcatttgccgaatgggggcaaaccacgccgaaagtgcgtgcggaatgtctgctgaaactggctgatgttatcgaagaaaatggtcaggtttttgccgaactggagtcccgtaattgtggcaaaccgctgcatagtgcgttcaatgatgaaatcccggcgattgtcgatgtttttcgctttttcgcgggtgcggcgcgctgtctgaatggtctggcggcaggtgaatatcttgaaggtcatacttcgatgatccgtcgcgatccgttgggggtcgtggcttctatcgcaccgtggaattatccgctgatgatggccgcgtggaaacttgctccggcgctggcggcagggaactgcgtagtgcttaaaccatcagaaattaccccgctgaccgcgttgaagttggcagagctggcgaaagatatcttcccggcaggcgtgattaacatactgtttggcagaggcaaaacggtgggtgatccgctgaccggtcatcccaaagtgcggatggtgtcgctgacgggctctatcgccaccggcgagcacatcatcagccataccgcgtcgtccattaagcgtactcatatggaacttggtggcaaagcgccagtgattgtttttgatgatgcggatattgaagcagtggtcgaaggtgtacgtacatttggctattacaatgctggacaggattgtactgcggcttgtcggatctacgcgcaaaaaggcatttacgatacgctggtggaaaaactgggtgctgcggtggcaacgttaaaatctggtgcgccagatgacgagtctacggagcttggacctttaagctcgctggcgcatctcgaacgcgtcggcaaggcagtagaagaggcgaaagcgacagggcacatcaaagtgatcactggcggtgaaaagcgcaagggtaatggctattactatgcgccgacgctgctggctggcgcattacaggacgatgccatcgtgcaaaaagaggtatttggtccagtagtgagtgttacgcccttcgacaacgaagaacaggtggtgaactgggcgaatgacagccagtacggacttgcatcttcggtatggacgaaagatgtgggcagggcgcatcgcgtcagcgcacggctgcaatatggttgtacctgggtcaatacccatttcatgctggtaagtgaaatgccgcacggtgggcagaaactttctggttacggcaaggatatgtcactttatgggctggaggattacaccgtcgtccgccacgtcatggttaaacattaaggataatattgcagatcgtaagagtatgagatgatcttgcgtactgtcagagcactgatttctctgacagtacgtgctgcgtgcaaaatcactacatcaaataaaccagccaaatctcatagagataagagtaaacaaaccaacagcagcaaagaaatttatcagtactacagttctactggaaacattcatttttgccaccttttatcattgcccctatgtgtatagtacgggttaagaaaatccgcaataatactcattctgaagatggataagggcaagttgctgtttgatgattttttctcaaactggtgaaaaaacttgatgcacgtcaaaaaatgacgcatatttgcgcgcgttttattcatctggctggacgcccgtacatgtctctctatcaacacatgcttgttttttatgcggttatggcagcaatcgcatttcttatcacctggtttctttctcacgataagaaacgcatccgtttcttaagcgcctttctggtgggggcaacatggccgatgagtttcccggtggcgctgttgttttcactgttttaaatcttactcactggcttgacggcaccacgcagacttatatcatttggatgaatcgataaatttcacaagtggctaaggagaaagtatgtcgcatctggatgaagtcatcgcgcgcgtggatgccgcgattgaagagagcgtcattgcccatatgaacgaattattaatcgccctgagcgatgacgcggagttaagtcgggaagatcgctacacccagcagcaacgtctgcgcacagcgatcgcccatcacggtcgcaagcataaagaagatatggaagcgcgccacgaacagttaaccaaaggcggcaccatcctctgattaaaatgagcgtctggctaccaaccaggcgccaaccacaagtaaaattgcgccacaaattgggccgaacaacgcccgtagtggtacgccatgactgcggaagatatccagcatcagaccgccaatcagctgactggcgaccagtacagcaatagttgtcgccgctcccacattctgatatccgctgatactggcgaagacaaaaaacgatcccagcaagccaggtataagtgtccaccagcgcacgctggacaccagttcgccaaaccccgccatgccttgtttaaaccataaaatagaaacaaagagcacaatccccaccagtgagttcagcaacatggcgatgagaatggtagaggaggtctgggtgatgcgcaccatcagcgtgttctggacaaccagaccaattccggcggcaatcaaaaaagcaagggtgagcgactgattcatccaatcgcgtccggttcagtgcgctcgtcgagttgcaactgcataaatgtcagatccagccaacgaccaaatttagtgcctacctgcggcatttgcgcggtgacgacaaatcccagcgactggtggagatgcagcgaggcctgattttgcgattcgatcccggcgaccatgacatgcttcccgcaatcccgcgcttcatcaatcaatcggcttaacaatttacgccccagacctttgccctgatgatcgggatggacataaaccgaatgttccacggtatggcgaaaaccatcgaaactacgccagtcgccaaacgaggcatatcccgtcactacgccgttttcctcgctcaccagcactggataacctgctaaagtccgcgcttcaaaccaggcaatgcggttatcagcatccaccgtttggtcattccagatagccgccgtatacaacacggcgtggttataaatttccgcaatggcagcacagtcggctttgcgggcaaaacggatggacatgtctggcctcaataaaataatgatgatgatgttatcaatactatcgaaaacagcccgaagcaacggattcctcgatgaaattattgcgtgttgcagaggggatgtgacggctgcaaacaaaaccaatcccgtgagcctgctactattgatggattcatgccaaaagcacaggagagcattatggggcaacaaaagcagcgtaatcgacgttgggttctggcctcgcgtccacatggcgcacctgttccggagaatttccgtcttgaagaagatgatgtcgccacaccgggtgaaggacaggtgttactgcgcacagtttatttgtccctggacccgtatatgcgtggacgtatgagcgatgagccatcttattcaccgcctgttgatattggcggcgtgatggtcggcggtacggtgagccgtgtcgtggagtcgaatcatcctgattatcagtctggcgactgggtgctgggctacagtggatggcaagactatgacatatccagtggtgatgatctggtgaaacttggcgatcatccgcaaaatccatcgtggtcgctgggtgtgctagggatgccaggctttaccgcttatatgggcctactggatatcggtcagcctaaagagggcgaaacgttggtggtagctgcggcgacaggaccagtgggggcgacggtggggcaaatcggcaaacttaaaggttgcagagtggtgggggtagccggtggcgcggaaaaatgccgccatgctaccgaggtgttaggcttcgatgtttgtcttgatcaccacgcggatgattttgccgaacaactggcgaaagcgtgcccaaaaggtattgatatctattatgaaaacgtgggcggtaaggtattcgatgcggtgctaccgttacttaatacatctgcgcgcattcccgtctgcggattagtgagcagctataacgctacagagctaccacccggtccggatcgtttacctctgttgatggctacagtgctgaaaaaacgtattcgcttgcaaggttttattatcgctcaggattatggtcaccgcatccatgagtttcagagggagatggggcaatgggtgaaagaggataaaatccactaccgcgaagaaattactgacggtttagagaatgcgccacagacgtttatcggcctgctgaagggtaaaaacttcggcaaagtggtgatccgcgtggcgggtgatgattaaagtttcaacggcggcgtaagccgccataaaaatccaggcaaaaagcttattttcagctttaattaactaaccacatcattgttctgctgctaataacaacaaaggtgagtggtttatgattattcactttaatacaccaggtgaattccttctgccatgcaggcagggttggacagaaaacacgcgaaggaattaaaatgcctggaacgggaaaaatgaaacatgtcagtttgactctgcaggttgagaacgacctgaaacatcagcttagtattggcgcattaaaacctggcgcacgcctgattactaaaaatctggcggagcaattaggtatgagtattacacctgtgcgtgaagcattattacgtctggtttcggtgaatgcgctttctgtcgcacctgcacaagcatttacagttccggaagtggggaaacgtcaattagacgaaatcaatcggatccgctacgaactggaattaatggcagttgctctggctgttgaaaacctcaccccgcaagaccttgcggaactccaggaattgctcgagaaattacagcaggcgcaagaaaagggcgacatggaacaaatcattaatgtaaacaggctatttcgcttagcgatttatcatcgctcaaatatgcccatcctgtgtgagatgattgagcaactgtgggtcaggatggggcctggtttacattatctctatgaagcgattaatccagcggaattacgggagcatatagaaaactatcatctgttactcgctgcgttaaaagcaaaagacaaagagggatgcagacattgtcttgctgaaattatgcaacaaaatattgctattttataccagcaatacaatcgttaaagtaaatgcccggcaaataccgggcatcaaggtaattactcaaatctccacgcaatattcatgccgacaccataatttcgtccgggcgaaggttcgtaatatcgcccgtttgactcattgacaatgacagaaccaacgtattctttatcgaataaattatcgacacgaccaaataaatccacagttaaattgtggtaattgtatttatacccggtgaataagccgacgagagtataagacggcgcttttgccgtattttcatcatctgccataatatcgcccatataacgcgcttccgtgcctgcataccaaccatcttccggtacataacctatcgacgcaaagcccatattacgggcgatccctggcatccgattaccgttacaatcctgttcattgcaaacattgctgcgataggtcgcatcaagccaggtccaggacgcgtttacgcgaaaatctcctgcgaaacgttgatcccatgccagttcagcgccttgacgacgggtctttccggcatttttgtaagtcgtacgcccaccgctactgctatcgacaacaatttcatcatcagtgtcggtctgaaacaatgcgagactaagcagcccatcaccaatacgcgttttactgccgatctcaattgtatcgttggtggatggttttaaacctaagttcataccgctttgcccatcagcacgataagacagctcattaatcgtcggcgtttcaaaacctcgcccggctgccagatagatattccaggcatcggtcattgcatattttaacgaaccggcaggtagccatttatgataactggcatcaccgctgtcatcgccgttacccggagtaacgtaatggtcgttggaatcaaaccacacggagctgtagcgcacgccagcatccagcgacagtttttcgctcagctgccactgcgtctgtaaatagggatcgatgttccacatcagattgcgttcgtcgcgacgcaactcacctttttgcccgtactccggcatgccgctattcaggcggaagttattgtagcccttgcggttttcactcatgttttcgtagttcaggccggtagtgaacgtgaccggaacgcccagttcaccacggtgtgtccagcggctgtctattccctggtaatggcgttgcagggtaatcacgccgcccgcatgtgacgggttaagttgtggtgccatgggtattgactggtactgggtcgtttctcgctctccggcatacatcatcacactcatatcatcccgcgaactcaggctacgctcatagcgcaacccagcctgagtttgcttgatggtttttcgcgtgtcgtactgttctgcacgaggcgcttgttgtggattagccttccattctgctttggttagcccacctgggtcatctgctttgatatccacactattgaaaatcagacttaatttgctggcttcatcaatgcgtacgcccagtttggcattggctaaatttttctgtgcgccactatggtcacgatagccgtgggtcgtaaaacgcgtggttgagacggtgtaatcgacatcgccaggctgtgtgccgtctcccgttgcgcccgttgctttcagcccatagcgccagctgccaaaactgccgtagtaactactggcttcaatggttggtggctgttgtccggtctgggtggtgacattcattaccccaccagacgcgttgccatacagggcagagaaggggccacgcagcacttccacattttgcacactgcttaaatcgatgttggatgtttgcccttgcccgtcgggcatggtggcgggaataccgtccacatacaggcgaataccgcgaataccgtaagtggagcgggagccaaatccgcgaatcgacagctgtaaatcttgcgcatagttctgccggttttgtacctgcaaaccaggcacgccggtcagtgattcggacaagttaatgcgcggtgttgccaggcgcatctcctcgccatccaccacgcttactgctgctggggtatccagttctgaaaccacctgcggtgcggcactgacaatcatagtctgttcatcagcggcaaaaacaacgggggaaaggacaagcagtgcgggcaaaacggtctgtcggacggaaaaaatcttcatgaaaaaagccaggttaagaatgggaaaacgccgtcatggtaatgaaattgtaaatttatggaaaatgaaacggcacaatacgttaagtaattgagaaaattgtagtcgtaacggcaagaaatgctccacatttgagaaaataatgattaccattcccatttataacaagagcgtaacgatgattacgcttagcgaagcattgtgaagcagcaaaaatatcggttcatcaaagggagtcgtcatgcatttacgtcatctgttttcatcgcgcctgcgtggttcattactgttaggttcattgcttgttgtttcatcattcagtacgcaggccgcagaagaaatgctgcgtaaagcggtaggtaaaggtgcctacgaaatggcttatagccagcaagaaaacgcgctgtggctcgccacttcgcaaagccgcaaactggataaaggtggcgtggtttatcgtcttgatccggtcactctggaagtgacgcaggcgatccataacgatctcaagccgtttggtgccaccatcaataacacgactcagacgttgtggtttggtaacaccgtaaacagcgcggtcacggcgatagatgccaaaacgggcgaagtgaaaggccgtctggtgctggatgatcgtaagcgcacggaagaggtgcgcccgctgcaaccgcgtgagctggtagctgacgatgccacgaacaccgtttacatcagtggtattggtaaagagagcgtgatttgggtcgttgatggcgggaatatcaaactgaaaaccgccatccagaacaccggtaaaatgagtaccggtctggcgctggatagcgaaggcaaacgtctttacaccactaacgctgacggcgaattgattaccatcgacaccgccgacaataaaatcctcagccgtaaaaagctgctggatgacggcaaagagcacttctttatcaacattagccttgataccgccaggcagcgtgcatttatcaccgattctaaagccgcagaagtgttagtggtcgatacccgtaatggcaatattctggcgaaggttgcggcaccggaatcactggctgtgctgtttaaccccgcgcgtaatgaagcctacgtaacgcatcgtcaggcaggtaaagtcagtgtgattgacgcgaaaagctataaagtggtgaaaacgttcgatacgccgactcatccaaacagcctggcgctgtctgccgatggcaaaacgctgtatgtcagtgtgaaacaaaaatccactaaacagcaggaagctacccagccagacgatgtgattcgtattgcgctgtaatagatatggcgagggtgaaaacggtgagacttgcctgccttttatcacggcgtatccggcactttcgtcagtaatctgaatttgcccggcacgtagccgggcaattttgcaattaactcgccgtttcaggcttaaacacaatttcctgtttttcttcatcttcctcgacgactggcgcagtgctgtgaatttcagcaacgcgtttgcgcacaccaaaccagcctataaccagcaaaataccgataatcggcagcgccgcgatagtataagtcccgttcgggtaatcgaacgccatcagcacaaggacactcagtaaaaacagtaatgtcagccaggaagtgaagggcgcgccaggcagtttaaaactgacatccgctgctttgccttctttaatcgctttacgcaggcgcatctggcacacgatgataaacgcccatgaagcgatgattcccagcgacgcgaagttcaacacaatctcaaatacgcgcgacggcaccagatagttgaggaatacgccgacgacatacacaactagtgtcgccagaatcccggcatacggcacatgctgacgactcattttcgccataaaactcggtgcggaaccgcccatcgccattgagcgcagaatacgtccggtgcagtacagacctgaattcaggctggagagggcagcggtcagcaccacaatgttcataatgctgccgatatatggcacacccagtttagagaaaaacgtcacgaacggactttgccccgcctgatacgcgctccacggcaataacataaccagcaacaccacggagccgacgtaaaacaggccaatacgccaaatcacactgttaatggctttaggcaccatggtctgcggatctttacattctccggcagctgtacccaccatttcaatggaggcaaaagcaaacactacgccctgaatcaacaccagcgcaggcagcaaaccgtgggggaagaagccgccattatcggtgattaaatgaaagccagtggtgttgccatccagcggctgaccactaccgaggaacactgtacccacgaccaaaaaggtcacaatggcgagcactttaataagcgcaaaccagaactccatctccgcaaaccatttcacaccgatcatattcatggtgccaacgatggtaagtgcagcgagcgcaaagacccactgcggcacgccgccaaacgcaccccagtaatgcatatacagagcgacggcggtaatatcaacaatccccgtcatcgcccagttgatgaagtacatccagccagcaacataagcggctttctcacccaaaaactcacgggcataagaaacaaaactgccactggaagggcggtgtagcaccagctcacccaatgcacgcagaataaaaaacgaaaacaagccacaaattaaataaaccagtgccagtgcgggccccgccatttgcagtcgggctcctgcacctaaaaacaagccggtgccaatcgcgccgccaatggcgatcatctgcacctggcgattgcccatcgctttgtgatacccctcttcgtgggcattaagccagcggcgtttcgcggcgtgttgatctgaagtgtcggtgtcgtgtttactcattgctctccctgattgctttaatgaaaaagtcatataagttgccatgaacaatgtttattcatcctggcgatgatagttatcaccattattctttatgggtataaaactatcggcgcagcatcctacccgttatcgataaacgatgcaaaacatccccttacaatcctgaaggggattaatacaactgacgaaaaaatgacaaatccttttgctggttaacctgtgtactgtcctacacttaatctttaaaagattgtgaggggcatatgattaaggtgtatggcgtacccggatggggctctacaatcagtgagctgatgctaacactggctgatattccttatcagttcgttgatgtcagtggttttgaccacgagggagcttcacgcgagttattgaaaaccctgaacccgttgtgtcaggttccgacactggcattggaaaatgacgagattatgacggagacagcggcgattgcattgatggttctcgatcgtcgcccggaccttgcgccaccggttgggcgcgccgaacgtcagctgtttcaacggctattggtctggctggttgctaatgtctatccaacattcactttcgccgattaccctgagcgttgggctcctgacgcacctgaacagttaaagaagaatgttattgaatatcgaaaatcgctttatatctggttgaattcgcagctcactgctgaaccttatgcgtttggtgagcaactaacgctggtggactgttatctttgcactatgcgcacatgggggcctgggcatgaatggtttcaggataatgccacgaatatcagtgcgattgctgatgctgtatgtcagttaccgaaattacaagaagtattaaaaaggaatgaaattatttgagtgggataccagaagattatgttatttattattcagtaactttatccacaatgatgggcgtaattaattaaattcatggtatgttttttaatttatatcactctccttttcattcagcgtgtctatttcatttcctctgaaaagaaactaactattcacatcgtgcagatgtttcagttgttatcacaggcattctataatctcaaaatgtttttaatgatggatatgctcggagttggagatgcaattaatattaatacaaataaaaatatccggcaggtatgctaaaaggataaatggcgttctctgtatttattcgcaattatctgtaggacaaatatggagagcttgatgagtcagagctaaaacagcaattgattaataaacatgttgatttattcaagaaaatggatgtattttaaatgttgattcttaatataacctaatcaatagattatcaagtgagagctacacattattggaggggcaggggaaaacaccattttgggaacaatgcatcaggtactcttaccactgaagcaagatcatccggcaccaggtggtggtgcagtgctttggaaatggtcccctcgggggagttgtcattattttctatgctatttgcttattatattcatcaggtgaatttaataaattcctaatttgaaatatccactattaagctagtgtttaacgacgttaagatggcaatgtgcagatcatgttatcagggtggggcggtagcgtatattccttatacaaaccatcattcatttcaatgattgttattgaattatttattgttgtgaataaaaagacattatgaatattggtttgactttgcatatcaggttttttattactcgctgtaatgtacgagcctgtcgtgaataacgtcgagaacccatccgttgcgtttgtgattattttgttgactaaacagacacccgtttctctgaagtaaaatcccagactaaatcatcacataaccatgacatttttctgatattccccggtaacgccagatgtcgactcgcttaaccaccctcagccataccagtgaaggccaccgcgtgtcggtccactacggctatgacgataaaggccgcctgaccggcgaacgccagacggtggagaacccggagacgggggaactgctgtggcaccatgagaccggacatgcgtacaacgaacaggggctggcaaaccgcgtcacgccggacagtctgccgccggtggagtggctgacctacggcagcggctatcttgcgggcatgaagctgggcgggacgccgctgctggagttcacgcgcgaccgcctgcaccgtgagacggtgcgcagcttcggcagcatggcaggcagtaatgccgcatataaactgaccagcacatacacccccgcaggccagttacagagccagcacctgaacagcctggtgtatgaccgtgactacgggtggaatgacaacggcgacctggtgcgcatcagcggcccgcgacagacgcgggaatacggctacagcgccacgggcaggctggagagtgtgcgcaccctcgcaccagacctggacatccgcatcccgtatgccacggacccggcgggcaaccggctgccggacccggagctgcacccggacagtacactcacagtgtggccggataaccgcatcgcggaggatgcgcactatgtctaccgccacgatgaatacggcaggctgacggagaagacggaccgcatcccggcgggtgtgatacggacggacgacgagcggacccaccactaccactacgacagccagcaccgcctggtgttctacacgcggatacagcatggcgagccactggtcgagagccgctacctctacgacccgctgggacggcgaatggcaaaacgggtctggcggcgggagcgtgacctgacggggtggatgtcgctgtcgcgtaaaccggaggtgacgtggtatggctgggacggagacaggctgacgacggtgcagactgacaccacacgtatccagacggtatacgagccgggaagcttcacgccgctcatccgggtcgagacagagaacggcgagcgggaaaaagcgcagcggcgcagcctggcagagacgctccagcaggaagggagtgagaacggccacggcgtggtgttcccggctgaactggtgcggctgctggacaggctggaggaagaaatccgggcagaccgcgtgagcagtgaaagccgggcgtggcttgcgcagtgcgggctgacggtggagcaactggccagacaggtggagccggaatacacaccggcgcgaaaagttcatttttaccactgcgaccaccggggcctgccgctggcgctcatcagcgaagacggcaatacggcgtggcgcggggagtatgatgaatggggcaaccagcttaatgaggagaacccgcatcacctgcaccagccgtaccgtctgccagggcagcagcatgatgaggagtcggggctgtactataaccgtcaccggcactacgatccgttgcaggggcggtatatcaccccggacccgattgggttgagaggtggatggaatatgtatcagtatccgttgaatcccatacaagtgatagacccaatggggttagatgcgattgagaatatgacatcaggtggactaatttatgccgtatctggtgtacctggattgattgctgcaaacagcattactaacagtgcttaccagttcggttatgatatggatgctattgttggcggagctcataatggggccgccgatgcaatgagacattgttacttgatgtgtcgaatgactaagacatttggatcaacaatagctgacgtgataggtaaaaatcatgaggcggcaggggatagacaaggtcagccagctaaagaaagaatcatggatcttaaaaataacactgtcggtattgcttgtggcgatttttctgccaaatgtagcgatgcatgtattgaaaaatataacactgggcaactcttcgggttagatggtataaaagcagataatccaataaaagcaaagcaagggagttcagatgcttcaaattattagaggcaaacttgtcatttttttaattaccctttgtttatttgttgtttaccttgggtttgataacaattcaaattctgacatcgtattttatggacataaaacaccaaagagcgttgagatatatctttctgaaaaaaatattatttataaaataattaatgaccaaaaaattagtagagggaatggtcattttataagtataatggttaataattacaggacgcactgtggagtggttgatataaatcttaattttttcaatgatattctttatagcgtgcgattaaaaaacattagtaaactggagaatatggagttctgcgctacaaaacaacgggtgtattttagtgataaaaacaagaaggctagttataaaataattaattatggagactattatgatgttgattattatgataacaatttgaaaaatgaagtttttgactggattggtaaatggtcataatgaacaacaccagaaagagaaaaatataaaatacatacagaaagacatgagagcaagggacggggcagggcaagatcatgaaaattgtgatgtaaatcacgattttcatctttgctttaacgcctacaggtgatcaaaatttaacctttggaataactaaaaagataaaaaaggacgccaggtgagtattcaaagtttgcttgattatatttcagtgacccctgatatacgacaacaaggaaaggttaaacataaattatctgctattttgtttctcaccgtatgtgcagtaattgcaggtgccgatgagtggcaggaaattgaagattttggacatgaaagacttgaatggctaaagaaatatggtgattttgataatggcattccggtcgatgacaccattgcacgcgttgtgagtaacattgacagtttggcctttgaaaagatgtttattgaatggatgcaggagtgccatgaaatcactgatggtgaaattatagcaatagatggaaagaccataagaggctcctttgataagggaaaaagaaaaggagcaatccatatggtgagtgcattctcgaacgaaaatggtgttgtactggggcaggtgaaaacggaagccaaaagtaatgagattacagccattccagagttgcttaacctactgtatttaaagaaaaatttgataaccattgatgctatgggctgtcagaaagatatcgcttcgaagatcaaagataaaaaagcagattatcttctggcagtaaaaggcaatcaggggaaattacatcatgcattcgaggaaaaatttcctgtaaatgtgttttctaattataaaggcgattcgtttagtacgcaggagataagtcatggaagaaaagaaacacgtttgcatattgtcagtaacgtaacgcctgaacttttgtgattttgaattcgaatggaagggattaaaaaagctttgtgtagcattgtcattcaggcagaagaaagaagataaatcagcagaaggtgtaagcatccgatattatatttcatcaaaggatatggatgctaaagaatttgcacatgctatcagagcgcactggctgatcgagcacagtcttcattgggtgttagatgtaaaaatgaatgaagatgccagccggataagaagaggaaacgcagcctaaataatatctggaataaagaagatggcactgaatttattaagagattgcaaagacattaagggtgaagaggaaaagaaagaaggctgcgttaaacacagggaaagatcatcagaagttcactttttgtactaaacaattcgcattttatgtttaaaaattgagatattccttattacctaaagctgttttttattgcttacacatgatcaaatactccttacataattaaggagaacaaaatggaacttaaaaaattgatgggacatatttctattatccccgattacagacaagcctggaaaatggaacataagttatcggatattctactgttgactatttgtgccgttatttctggtgcagaaggctgggaagatatagaggattttggggaaacacatcccgattttttgaagcaatatggtgattttgaaaatggtattcctgttcacgacaccattgccagagttgtatcctgtatcagtcctgcaaaatttcacgagtgctttattaactggatgcgtgactgccattcttcagatgataaagacgtcattgcaattgatggaaaaacgctccggcattcttatgataagagtcgccgcaggggagcgattcatgtcattagtgcgttctcaacaatgcacagtctggtcatcggacagatcaagacggatgagaaatctaatgagattacagctatcccagaacttcttaacatgctggatattaaaggaaaaatcatcacaactgatgcgatgggttgccagaaagatattgcagagaagatacaaaaacagggaggtgattatttattcgcggtaaaaggaaaccaggggcggctaaataaagcctttgaggaaaaatttccgctgaaagaattaaataatccagcgcatgacagttacgcaatgagtgaaaagagtcacggcagagaagaaatccgtcttcatattgtttgcgatgtccctgatgaacttattgatttcacgtttgaatggaaagggctgaagaaattatgcgtggcagtctcctttcggtccataatagcagaacaaaagaaagagctcgaaatgacggtcagatattatatcagttctgctgatttaaccgcagagaagttcgccacagcaatccgaaaccactggcatgtggagaataagctgcactggcgtctggacgtggtaatgaatgaagacgactgcaaaataagaagaggaaatgcagcagaattattttcagggatacggcacattgctattaatattttgacgaatgataaggtattcaaggcagggttaagacgtaagatgcgaaaagcagccatggacagaaactacctggcgtcagtccttacggggagcgggctttcgtaatcttgccctgggcattattgtcgtataaacgctttaccggacacatgacattcacaatgtgtgttaattttactgacatctttcaaaaggagcgtaatcatgccgcacatcgacattaaatgttttccgcgtgaactggacgaacaacaaaaagcagcacttgctgcagatattaccgacgttattattcgtcatctgaacagtaaagacagttcgataagcattgctctacagcagattcaaccagaatcttggcaagctatctgggatgccgaaatcgcgccccaaatggaggctttgataaagaaacctggttatagcatgaatgcttaacccgccgtaacacgcttgccgctggtaacaaacgtcccagcacctaaatgatgcaacgtattgagcttatcatcatcaaactgccagcggccttcgacaaatacccgtgcgtctgccgctgctgatactacttcgccaaacagcgtgtcgtattcttcttgcgcagaagtcgcaggtagcaatcgacactccatccacgccagacatttttcctcgaccagaggcaaaccaaataccgggcctctcacaaccggaatgccatagcaattaaatttatcttcatcacgccccgacacacttcccaccgcccacgtccagttagttgctgcaacgcccgggataacgatgccaaatttaccgttatgttcaatcaactccctggtccatgtcgatttatctaccacaatcgccacgcgtggaggttcaaactccaccggcattgaccaggctgcagccataatgttacgccgctgggattgctcatcgaaactggtgatcaagaccgttgggccatgatttaacagacggctggcatggtgtaattctatggggatgaatcggctcatggtatcgcctcgcgaagaaggtttttttaagcgtagtccgtaacgcaataagtaacgaaattaacgggattggcgatttgcgaacgtgatgcatgtccgcgatcgcacaaaatagccggtgcggcgtctattccaggttataagttgagaaaaccactaagggaaacgcctgatgacgcccattctgaatcactattttgcccgtattaactggtcgggagctgctgcggtcaatattgatacgcttcgtgcattgcacctgaaacacaattgcaccattccgtttgaaaacctcgacgttttgctgccgagggaaatacagcttgataatcaatcgccggaagagaaactggtgatagcccgtcgtggcggttactgttttgagcagaatggcgtgtttgagcgggtgttacgcgagctggggtttaacgttcgcagcttgttagggcgcgtagtgttatcaaatccgccagcattaccgccgcgcacccatcgtttgctgttggtggaactggaagaggaaaaatggattgctgatgtcggtttcggtgggcagacgctaaccgcgccgattcgtttagtttccgatctcgtgcagaccacgccacacggagagtatcggttgttgcaggagggtgatgattgggtgttgcagtttaatcatcatcagcattggcagtcgatgtaccgttttgatctctgcgagcagcaacaaagcgattatgtgatgggcaatttctggtcggcgcactggccgcagtcgcattttcgccatcatttgctgatgtgccgccatttgccggacggcggcaagctgacactgaccaattttcattttacccattatgaaaatgggcacgcggtggagcagcgaaatctaccggatgtggcgtcattatatgctgtgatgcaagaacagtttggtctgggcgtggatgatgcgaaacatggctttaccgtggatgagttagcgctggtgatggcggcgtttgatacgcacccggaggcgggaaaataatttatgtcaggttgccggatgcggcgtaaacgccttatccggcatacattagcccggttgtagacctgacaggcgaagcgcatcagacaacggtttcagagttcaattgcccattcggcatgaaacaaaatcaccgctgtgcctgaaatggtgactttttccggttggttatcacgaattgtcaccgtcacttcaatcataccgtcacgccccaatgcgcgcccctgatggcctttaacacgcaacacgttgccatcgtggggcaatacgttgtgatgtaccaaccatgcacccatcgggccattggcattgccagtcaccggatcttccacaataccaatcgcaggcgagaacatgcgaccatcggtttcgtttttgcctgggcggatctggaacgggaagaaaccattgcagccaatctttttgctgatagcggtcagcgcattaaggtcaggcgaaagggcgtcgatatccacttccggtttcagtgggatcatcacttttgagtgtcctgttgttgccacctgaattggcaagcctggcagaatatcgtcctcagtgagatgaagcgcgttgataatcgccgcacgtgtttcaccttccagcggtggctcaaagcccggcgtaccttgttccagcgaaatacgataatcatcgttgtgcttttcgatagtcacgcgatgttttcctgccagcgatgtttgccagatcgtgcaatttcctaaacctaacaccttcgcacgtacatagtgcgcagctactgtcgcgtgaccgcaaatcggcacttcaaccgttggcgtaaagtagcggatgcgcacatcgctgtcgtcgctgtgcagcagaaaagcagtttccgaatggcctaactcgcgggcgataagctgcatttgcgcttcgctaagattatcggcggggaaaacaacaccggcagaattgccgcgaaacggttgtgaggtaaaagcatcgacgtggtacacctgcggtttcattaacgttctcctgtgactggagaactatcatagcctgcaagtggccggagagcgaagggctatccggccagggtgaaattatcgccgcgaacgcacaatttgatatcgacgagtaaagtactcaaacggcgcgctccacacatgcaccagtcgggtgaacgggaagagcaggaagatggtcattcccaacaccagatgcaggcggaagacgaacgctacgccgttgagcatctctgacgatccaccacggaaagtgacaatgctttgcgcccaacccaccagcttcatcatttcgctaccatcaggatactgtgctgaaaacggtatggtacttagccccaacagacactggatcagcaaaatgctcatgatgatgatatccggcgtagtggaagtggcacgcacgcgctgatttgtcagcctgcgccacagcagtcctgcgccgccaatcaacgtcaacacaccgcaaataccgccgagcaccatcgccatgagttgtttcgctgccactggcaaaaaccacgcgtacatccagtgcggcgttaacatgccgaacaagtgcccgaagaaaatccccaaaatgccgatatggaacagattcgaccatatcaccatcccgcgtttatcgagcatttgacttgaggaggcgcgccaggtgtactgcccgtagtcgtagcgcagccagctgccgaggaaaaacaccgtcgcacaaatgtacgggtagatatcgtaaaaaaagacgttcagatactgaatcatttcccacctcccgcactgatgtcgacatattgcggcgcgacatcctggctaaagcgtcgctgatattgattaagcggcgagctgtcacacgccgtggcgttatcttcaataaacttcacctgttcctcttcccacactgcatcaagcgcctggcgggtgtcatcgcgctcttcgctgtttacttgttttgtgacactgtcacttgaaagggagcttcccgccagttgcagcagagcatcaaacaacgcgtaccacggtgcctcgcgttgttttaagcgaccgccaagcagggcgaggatcggcgcaacattgagcaatccttctttcgcctgatcgtcaggcagtacgcttaaatactccagatacagcggtagataatcgggcagttcccgacaatccagctgcaggccgaccttttcatactccgccagcaggtccaccattgcctggccgcgatcgcgggactcggcatgaacatgttcgaacagcagcagcgacgtggtgcgcccgcggtcaaacacttcgcaccattcggcctgtttatccagcagcggcgcgttaagcaggttgtgggtgaaatccgtaagcatcggcgcgtcgcggcggatcaacgccagcgcgtcctccttgcattcccacaacagctcgtccggatactccatcaacaggccgatcactttgaggatctgcattattcgccctccgctttgtcgcgcacttcggtgatgttgatggcatcgatacggctactgttgaacaggttgaatttactgtccgaaccgtggcaaccgtcgccaaaggtaaaaccgcagccgttgcgttctgcgaaggcatcgcccgccatttcccgatggctggtcgggataacaaaacgatcttcatagttggcaatggcgagatagcgatacatctcttcgacctgggcgacgctcaggcctacttcgtcgatggcacgagtatcagtaacgccttccacggtttgtgaacgcatatagtggcgcatcgccatcatccgtttcagcgcccgcagtaccggaccggtatcgccggcactcaacatattggcgagatattgcaccggaatacgcaggctttcgatggcgggcagcacgccttcgcttttcggcaaaccgcccgcatctgcgtaggactgaatcggtgacagcggaggaacgtaccagaccatcggcagggtgcggtattcagggtgcaacggtagtgccagtttccagtccatcgccattttgtagactggcgaacgctgggcagcgtcaatcacattttgtggaataccttgtttcagggcttcctcgatcactgagggatcgtgtggatcgaggaacacttcgcactggcgttcatagaggtcaacttcgcgctcggtgctcgccgcttcctcgatgcggtcggcgtcgtaaagcagcacgcccagataccggatgcgacccacgcaggtttctgagcacacggtcggttgaccggactcaattcgtgggtaacagaagatgcatttttctgacttgccgcttttccagttgaagtagatttttttgtacggacaaccgcttatgcacaaacgccagccacggcatttatcctgatcaatcagcacaatgccgtcttcttcgcgtttgtagatagcgccgcttgggcaggtcgccacgcagctgggattgaggcagtgttcgcacaggcgcggcaggtacatcatgaaggtgttttcaaactgcccgtacatctccttttgcatggcctcgaagttgcggtcgcgggcacgtttttcgaactcaccgcccagcagttcttcccagtttggcccccagatcactttgtccatccgtttgccgtcaatcagtgaacgcgggcgagcagtaggaatatgtttgccttccggtgcgctatgcaaatgttcgtagtcgaaggtgaaaggttcgtagtaatcatcaatctgcggcaccaccgggttggcgaagattttggttattacgcccatcttgttgcccagacgcgggcgtatcttgccattcacatcacgcacccagccgccttgccactcttcctgatcttcccagtttttcggataaccaatgcccggtttggtttcgacgttgttaaaccatgcgtactccatgccttcgcgcccggtccagacgtttttacaggtcaccgaacaggtatggcagccgatacatttgtcgaggttaagcaccatgccgacttgtgaacggattttcattttttcgcctcctgtacctgatcgcgaccttcatcatccagccagttaacgttcttcatcttgcggatcatgatgaactcatcgcggttcgatccgacggtgccgtagtagttaaagccccaggccagctgcgcgtaaccgccaatcatatgcgttggtttcgggcaaacgcgggtaaccgagttatgaatgccgccgcgcatgccagttacttccgaaccaggaatattcataatgcgttcctgggcgtgatacatcatggtcatgcccggcggtacacgttggctgaccaccgcgcgggcagtcagcgcgccgttggcgttgaatacttccacccagtcgttatcgacaatggtcagttctcgggcatctgtttcgctgatccagacaatcggtccaccgcgagagagcgtcagcattagcaggttttcactgtaggttgagtgaatgccccatttctggtgcggcgtcaggaagttaagtgctttttccgggaagccgtttggcggtatctggcgcatctcactgacgctacgggtgtcgataggcgggcgataagccaccaggctttcaccaaaagcacgcatccacggatgatcctgatagagctgctggcgtcccgacagcgtgcgccacggaattaactcatgaacgttggtgtatcccgcgttataggagacgtgatcgctttccagaccggaccaggtggggctggagataattttacgcggctgcgcctgaatatcgcgaaagcgaatcttctcgtcctctttgtgcagcgccagatgggtatgttcgcgcccggtgatctcgcccagcgcctgccacgctttgactgcaacatgaccgttggtttccggtgccagtgccagaatcacttctgaagcgtcaatggcggtgtcaatcagcggacgcccctgtgccgggccatcacgcttggtgtaattgagtttgccgaggaaatcgatttcatcctgggtattccacgaaatccctttaccgccattgccaagtttgtccatcaatggcccgagcgaggtaaagcgttcatacgtagcagggtagtcgcgctccaccgccacaatattcggcgcggttttgcctggaatcagatcgcattcgcctttgcgccagtcgagcacttcacacggctgtgagagctctgccggagagtcatgcagtaggggttgtaataccacgtcggtttctttgccaagatgacccacgcacacttgcgaaaatgctttggcgatacctttgtagatttcccagtcgctgcgtgattcccacgccggatcgaccgccgcagaaagcggatgaataaacggatgcatatccgaggtgttcatatcgtctttttcgtaccaggtggcggtgggcagaacgatatcggagaacaggcaggtactggacatgcggaagtcgagcgtcaccagcaggtcgagcttgccttcaatcgctgcagtttgccactcgacttcttccggtttgatcccgtcgctggcaccgagttcctcgccctgaatcccgctttcggtccccagcagatacttctgcatatactcgtggcctttgccggaggagccaagcaggttagagcgccagacaaacaaattacgcggatgattgctgctgctatctggttgttcgcaggccatacgtaaatcgcccgatttcagcgcctgggcggtaaattctgtgggggataatccggccttgtcggcttcagctttaatcccgagcgggttacgccccagctgcggcgcagaaggtagccagcccatacgttcggcgcgaacgttgaaatcaatcagatgaccgctgtacttactggcatcggcgagcggtgaaagtaactcctgagcagagactttttcatagcgccattggctggaatgattgtagaaaaacgaggtgctgttcatttggcgcggtggtcggttccagtcgagcgcaaaggccagtggcaaccagccggtttgtgggcgcagtttttcctggccgacatagtgtgcccagccgccaccgctttgcccgacacaaccgcagaagatcagcatattgatcatcccgcggtagttcatgtccatgtgataccagtggttaacacctgcgccgaggataatcatcgagcgcccatgcgttttatgggcggtatcggcaaattcacgggcgatggtttcaatatactggcgcggcacgccggtaatttgctcaccccaggctggggtgtacggtttgatttcagcgtaatctttcgcactgttttcatcttccagcccgcgatcgaggccgtaattcgccagtaccaaatcataaacgctgaccaccggacaggtgttgccatcgactaacgtcaggtttttaacgggcaattggcgcaccagcaccggattgtgttttacgctgcgaaaatgcggattttcaatgccgccaaagtaggggaaggccacgcctgcaacagcgtcatgttgaccgagcagggttaacgacaattcggtttccgtaccggcggcaatggattccagattccatttgcctttttctccccagcggaaaccaatcgaaccgttcggcactaccaattcacctgcggtattaactgctacggttttccactgcggattgttgctttcgcccagtccatccaccaggtcagatgcgcggatcatgcgcccgggaacgtagctaccatcgtcgcgaggctccagcattaccagcatcggcatgtcgctgtagcggcggcagtagttgataaagtagtcgctgggattatcgagatgaaactcttttaaaatcacatggcccattgccatcgccagggcgctatcagtgccttgtttcggtgccagccactggtcgcacaatttggccacttcagagtagtcaggggtaatggcgatggttttagtgcctttgtagcgtacttcggtaaagaagtgggcgtccggcgtacgtgtctgcggtacgttagacccccaggcgatgatgtagctggagttataccagtcggcagattccggtacgtcggtttgctcgccccaggtcatcggcgaggcgggcggcaggtcgcaataccagtcgtagaaacttaaacaggtgccgccaagcagcgacagataacgcgttccggcggcgtaagaaaccatcgacatcgccgggatcggcgagaaaccggcaacgcgatccgggccgtaggttttgatggtccagacgttagcggcggcaatcagctggtttagttcctgccagttggagcggataaacccgccgcgcccacgcacttgtttgtagctcaggcacttttgcggatcgttcataatcgatgcccacgccagtaccggatcgctgtgttgcttgagggcttcgcgccacagttcaatcagtcgtttacgaatgagcgggtatttcaggcggttagcgctgtaaagataccaggagtaacttgcgccacgcgggcagccgcgaggttcatgattgggcaggtcagggcgagtgcgcgggtagtcggtctgttggatttcccaggtcaccagaccatttttaacgtagattttccagctacaggagcctgtacagttaacaccgtgggtggaacgcacgattttgtcgaactgccaacgctggcgatagctgtcctcccagtcgcggttgctatgcatcacctgtccgtgaccatcggcaaaggtttcgcccttttgtttgaagtagcgaaagcgatccaaaagtttactcatgacatgactcctgctccaggaatgaattgggatctgatgccttgtcggatgcgacacggttgtacatcaggcatcgatctcttatttttggctgaacttccgccgaccataaaccagccaggtcagcagcacacaaacgatgtagaagattaaaaacactttcatcgcgccgaccggagagccggtcatattgagcgacatgccaaacgcctgcggaataaaaaagccgcccactgcgccaatggctgagataaagcccagagccgccgccgtttcggtgacggcttctttatgagcttgctcatcactaccgcctttcatctttacccgataaatggttatctggcgaaagatgacggcgatcatctggaaagtagaaccacttcccagacccgcagtcagaaacagccccataaatacggcgtaaaaggcgatgaaattaccggagcctgtgcccggtaaggtaaggaacagcagggcactgaaaatcgccataaaaataaagttgatcaacgtcacccgcacgccgccgaacttatcggaaatagcaccaccaaccgaccgcgcgatggcaccgataaatgggccaaagaacgccaggcgcagaatattcacatccgggaactgggtttttgccagcatggcaaaacccgcagaaaaaccgataaacgaaccgaaggtggcaaggtaaagcaggctcagcagccagagatgcaggcgttgtaagacagggagctggtcggcaattgaggcgcgtgaactggcgatatcattcatccctgaccatgcggcgatcgtggcaatcgccagtagcggtacccaaatccatgcggcattcgccagcgacatcaccgaaccgtcggcctgcggtacgccattgacgccgagaaaggcaaatacaggtacaaaaatgaccagcggtgcaaccagctgcattacacttacacctaagtttcctaatccgccattaatcccaagagcgctcccttgtttggcttttggaaagaagaaactgatattgcccatgctcgaagcaaagtttgcacctgcaaaaccgcatagcaaagcgataacgataaatatcccaaaaggagtattcggattttgcacggcaattccgagccagacgcaaggaataatcaggattgcagtactaaaaaccgtccatcggcgtccaccgaatataggcaccataaaggagtagggaacacgcaataatgcgccagaaacggagggtaatgcggttaataaaaagagttgatcggtagtaaaattaaaaccgattttattgagattaacggtaactgcgctaaatagcatccagacacagaaggcaagaagtagacaactgactgatatccagagatttcttcgagcaatatgttttcctttattttcccagaaggccggattttctggtttccagtcgcgcaaaagataacgactatttttctcattttgcagtgccatattgttcctcacatgcacacattggtaatgaaaaaaagacaaaacacgaggtaaggcgcaatagccagttattagaattaaggatgaattgggtgaagtgctgattgaaagaatagataagaaagcgtaaccgcgggggcagaatggggattaagtagccagatatgtgttactaaatgtaactaacaagctaaccttcaaacggggttaatctttgaacgtatgtcatgtttcaacccttcagatcgtgaatctaaagggttacatattaactatattatcaacaagaccagacacttatagaattagtgatgatttattcactaaaaaggccatgaactggaggaaaacgatctgtccagaaggtctatcggttcctctcttattgcctgattgtaataatcgttattacagtaagtattgtttatttcatctaaggtcatgtttttaacttttatattcatctggtttacaacttcctctgtcttgtaagtgtgtatattatatggggtatatgcttttttaataggatagtgaaacaattcgttatccacatctattccgtcagagtgaacttcaaatgcaccaggcgaaagaattgccaggccagtattaagcttaagtgctggggaaaacaaattaaataacatgagctgcatagtagggcaattgttcttcccagaaacatttaaaaaatttaagttttgctctgttttattatggggaataaagttccaatatcggatgtattattagtatcaatgtgggttattttattattgtccagtcttaaacttttgatagatggaagataagtcaggaaatcaagatttatatatttcaactggttgttagcagcgtttaatgtctgaacattgcagaagttgctatagaatattttaatttcagaaagcaaattgttgttaataagtaacgtattcaagttgggaaataagtcattgtgtaaacttgttagtttattatgggatagatccagcagtaagagttcatttttattacctgcaacaatatcagttaattgattatggctgagattcaggtattgcagccattcgcaagattctaattgcacaaactctagttgattatgtgccgcactaaaataagtaactgatgaaagcctatctatatcaatatttctgagagcattattattcatagatatatgtgtaatacttacatttctgccttgaggaaaatttattgactcaagagcattactattcagacttagctttacgagtctatcgtagttggttgcatcaaaatgtgtgaattggttattatcaagattgatagatgtgaagttttgcagccctggtggttgagtggttaaattaagtcctgataaatcaatggtcacttcattagtgtcatcaattatatttcttactgcagtccagtactgcatttgtgcaagtggatcattgttgatgccgttaactaatacatgccaaagatgttttgatgatattagttgatcaatgtcattggttggcagtaaattgttattgcttaagtttaaatattccagttttgtagtgtttttggcgtttaaatgtgcaatatggttgtcgtttaaagtgattgttttcatcctgggatgattgtgtaatataaggtcagtgatcatattgtgatgggcacttaactcaatcagagattcttgccgcgcgagccgttggcttcatcgttatagcctttaaaatcatattcccagtgaccaaaaccaatcatttgatcattgatttgcgtttctcctttaaagccgagacgggcataagttttatcaccatcgtcacgcttatcatcagtaaaataacgtagagcggtaaccttgccataaaggtcgagtttattaccatccttgttatagacttcggcagcgtgtgctacgttcgcagctaacaaaccagttacaaccaccgcaactatttttaatttcatttaacagaatccttttaattatcgttaaacgtattttctaaacgaattttaaacggcgtcatttataaatgacatactgtttttaaaatagaatggtgattaaaaacaatgagaaaaatagatgaaataatattatttatcgatatgtgatcgaagtcgaaatgagatataaggtgaattactggtatttgaaatttatttttttaatattgtcggaatttatctgattaactaccgggccgtagacccggcagttattttaaccacgacgtgtcgccagccagcagagcagggaaccgccgcagaccatcagcgcgccttgccagaacgagaacgacagcggggcgctgagcagcacggctgcaagcgctgaggaaagtacaggcgtaaaatacgaacctaccgccataatggtgacattgccatgcaatataccgacattccatgcagcataagcaaatcctaaggtaaatgccgcagagatgagtttaatcatgacgggcgtgctaaatatcatttctggttgtggcgtaagaaaatagtaaacccacagacttgctcccgttagcaggacaaaaacggtaattccattaaatccgcgtgcgtatttattcgttactgtgcaataggctgcccagataaacgcaccaatgaacgccaggaaataactcaatgggctggtggtgatattattgatgatttcatcataatgtaacccattgtcaccgcctaacacccaacagacgccgacgagggctaataataatccaggtacaatcaaccagttggttttctgaccattaaacagaatggcaaagagaattgtcaggctgggccacagatagttcaccatacccacttcaatcgcctgatgatgggtcgccgcataccctaaggaaagcgccagacagatttcatagctgacgaataacagactcccggcgagtaaatagcctttcgggatttgccgaatacgcggaaatccaaccgtgaagattaacagcagcccgcttaatgaatagatagcagctgcgccgccgaccgggccgagcccctcactgacaccgcgaatcaatcctaccatcgtgctccacaggacgatcgctatcagccctatgagcgttgctttttgtcgtgtcatgctcgctgttttgtctctcttgccgttaaaaattaagctgaattttatagcatttttttaactggcctgtcaggcagtggtgcgtttttctaccgctattgaggtaggtcaatttgcgaaggcggattattttgtggcaaacagatgttctttttgatttcgcgcaaaaagattcagaattttactgttagtttcctcgcgcagtaatacccctgaaaaaagaggaaagcaatggacgtcagtcgcagacaattttttaaaatctgcgcgggcggtatggctggaacaacagtagcggcattgggctttgccccgaagcaagcactggctcaggcgcgaaactacaaattattacgcgctaaagagatccgtaacacctgcacatactgttccgtaggttgcgggctattgatgtatagcctgggtgatggcgcaaaaaacgccagagaagcgatttatcacattgaaggtgacccggatcatccggtaagccgtggtgcgctgtgcccgaaaggggccggtttgctggattacgtcaacagtgaaaaccgtctgcgctacccggaatatcgtgcgccaggttctgacaaatggcagcgcattagctgggaagaagcattctcccgtattgcgaagctgatgaaagctgaccgtgacgctaactttattgaaaagaacgagcagggcgtaacggtaaaccgttggctttctaccggtatgctgtgtgcctccggtgccagcaacgaaaccgggatgctgacccagaaatttgcccgctccctcgggatgctggcggtagacaaccaggcgcgcgtctgacacggaccaacggtagcaagtcttgctccaacatttggtcgcggtgcgatgaccaaccactgggtggatatcaaaaacgctaacgtcgtgatggtgatgggcggtaacgctgctgaagcgcatcccgtcggtttccgctgggcgatggaagcgaaaaacaacaacgacgcaaccttgatcgttgtcgatccccgttttacgcgtaccgcttctgtggcggatatttacgcgcctattcgttccggtacggacattacgttcctgtctggcgttttgcgctacctgatcgaaaacaacaaaatcaacgccgaatacgttaagcattacaccaacgccagcctgctggtgcgtgatgattttgctttcgaagacggtctgttcagcggctacgacgctgaaaaacgtcaatacgataaatcgtcctggaactatcagctcgatgaaaacggctatgcgaaacgcgatgaaacactgactcatccgcgctgtgtgtggaacctgctgaaagagcacgtttcccgctacacgccggacgtcgttgaaaacatctgcggtacgccaaaagccgacttcctgaaagtgtgtgaagtgctggcctccaccagcgcaccggatcgcacaaccaccttcctgtacgcgctgggctggacgcagcacactgtgggtgcgcagaacatccgtactatggcgatgatccagttgctgctcggtaacatgggtatggccggtggcggcgtgaacgcattgcgtggtcactccaacattcagggcttgactgacttaggcctgctctctaccagcctgccaggttatctgacgctgccgtcagaaaaacaggttgatttgcagtcgtatctggaagcgaacacgccgaaagcgacgctggctgatcaggtgaactactggagcaactatccgaagttcttcgttagcctgatgaaatctttctatggcgatgccgcgcagaaagagaacaactggggctatgactggctgccgaagtgggaccagacctacgacgtcatcaagtatttcaacatgatggatgaaggcaaagtcaccggttatttctgccagggctttaacccggttgcgtccttcccggacaaaaacaaagtggtgagctgcctgagcaagctgaagtacatggtggttatcgatccgctggtgactgaaacctctaccttctggcagaaccacggtgagtcgaacgatgtcgatccggcgtctattcagactgaagtattccgtctgccttcgacctgctttgctgaagaagatggttctatcgctaactccggtcgctggttgcagtggcactggaaaggtcaggacgcgccgggcgaagcgcgtaacgacggtgaaattctggcgggtatctaccatcatctgcgcgagctgtaccagtccgaaggtggtaaaggcgtagaaccgctgatgaagatgagctggaactacaagcagccgcacgaaccgcaatctgacgaagtggctaaagagaacaacggctacgcgctggaagatctctatgacgctaatggcgtgcttattgcgaagaaaggtcagttgctgagtagctttgcgcatctgcgtgatgacggtacaaccgcatcttcttgctggatctacaccggtagctggacagagcagggcaaccagatggctaaccgcgataactccgacccgtccggtctggggaatacgctgggatgggcctgggcgtggccgctcaaccgtcgcgtgctgtacaaccgtgcttcggcggatatcaacggtaaaccgtgggatccgaaacggatgctgatccagtggaacggcagcaagtggacgggtaacgatattcctgacttcggcaatgccgcaccgggtacgccaaccgggccgtttatcatgcagccggaagggatgggacgcctgtttgccatcaacaaaatggcggaaggtccgttcccggaacactacgagccgattgaaacgccgctgggcactaacccgctgcatccgaacgtggtgtctaacccggttgttcgtctgtatgaacaagacgcgctgcggatgggtaaaaaagagcagttcccgtatgtgggtacgacctatcgtctgaccgagcacttccacacctggaccaagcacgcattgctcaacgcaattgctcagccggaacagtttgtggaaatcagcgaaacgctggcggcggcgaaaggcattaataatggcgatcgtgtcactgtctccagcaagcgtggctttatccgcgcggtggctgtggtaacgcgtcgtctgaaaccgctgaatgtaaatggtcagcaggttgaaacggtgggtattccaatccactggggctttgagggtgtcgcgcgtaaaggttatatcgctaacactctgacgccgaatgtcggtgatgcaaactcgcaaacgccggaatataaagcgttcttagtcaacatcgagaaggcgtaagggggcgaacagatggctatggaaacgcaggacattatcaaaaggtccgcaactaactccatcacgccgccttctcaggtgcgtgattacaaagcagaagtcgcaaaacttatcgacgtttccacctgtatcggctgtaaagcctgtcaggtggcgtgttcggagtggaacgacatccgtgatgaagtggggcactgcgtcggggtttacgataaccccgccgatctgagcgccaagtcctggacggtgatgcgctttagcgaaaccgaacagaacggcaagctggagtggctgatccgtaaagacggctgtatgcactgtgaagatcccggctgcctgaaggcgtgcccgtctgctggtgcaatcattcagtacgctaacgggattgtcgatttccagtcggaaaactgcatcggctgtggttactgcattgccgggtgtccgtttaatattccgcgcctcaacaaagaggataaccgggtatataaatgcacgctctgcgtcgatcgcgtcagcgtcggccaggaaccggcttgtgtgaaaacctgtccgaccggggctatccacttcggcaccaagaaggagatgctggagctggcggaacagcgcgtggcgaaactgaaagcgcgtggttacgaacatgctggcgtctacaacccggaaggggtcggtggtacgcacgttatgtacgtgctgcatcacgccgatcagccggagctgtatcacggtctgccgaaagatccgaagatcgacacctcggtaagcctgtggaaaggcgcgttgaaaccgctggcagcggctggctttattgccacttttgccgggttgattttccactacatcggtattggcccgaataaggaagtggacgatgacgaggaggatcatcatgagtaagtcgaaaatgattgtgcgcaccaaatttattgatcgcgcctgtcactggaccgtggtgatttgcttcttcctggtggcgctgtccgggatttcgttcttcttcccgacgctgcaatggctgacgcaaaccttcggtacgccgcagatgggacgcattttgcacccgttcttcggcattgcgattttcgtcgcactgatgtttatgtttgtgcgttttgtgcatcacaacatcccggataagaaagatattccgtggctgttgaacattgtcgaagtattgaaaggcaatgagcataaagtggcggatgtcggtaagtacaacgccgggcaaaagatgatgttctggtcgatcatgagcatgattttcgtgctgctggtgaccggggtgattatctggcgtccgtactttgcgcagtacttcccgatgcaggttgttcgctacagcctgctgatccacgcggctgcgggtatcatcctgatccacgccatcctgatccatatgtatatggcattttgggtgaaaggatcgattaaagggatgatcgaagggaaggtaagtcgtcgctgggcgaagaaacaccatccgcgctggtatcgtgaaatcgagaaggcagaagcgaaaaaagagagtgaagaagggatataatctcttttgaactttaagctgaaaatggcgctgtaaaaggcgccattttcatattgtagacaacgtaggctttgttcatgccggatgcggcgtgaacgccttatccggcatgaaaacccttcaaatccaatagattgcagtgaacgtgtaggcctgataagcgtagcgcatcaggcaatgttgcgtttgtcatcagtttcaaatggcgctgtaaaaggcgtcattttcatattgtagacaacgtaggctttgttcatgccggatgcggcgtgaacgccttatccggcatgaaaacccttcaaatccaatagattgcagtgaacgtgtaggcctgataagcgtagcgcatcaggcaatgttgcgtttgtcatcagttctaaatggcgctttataaagtgccatttttttattgcgtaaccagacggcgtaatcgcgacacatccactgttttttctgcctctgccagactccaggcgttttgcagattcagccacatttgcggcgaactgccgatcaccacggaaagtttaatcgccatttctggcgtcaaagctgcttttcctgtcagcaatcggcttgccgttgagggagcaatttccattgctctggcaaactcgcgcaggctgacattaagttcgtccagtgattcctgaataatgtcccccgggcggggatgattggccattttcattagtgtctttactctcagtagcgttccttcactgggaacactatcattattgttccttcctacgcaacaataatccatttagccatttcatgttggagagtgtgcgatgctgcgacccgaacatggcagtcgcagcaaaggcctcttagtgacggaaatcaatcaccatgcggccacggattttgccttcttccatctcagtaaagatggtgttgatgtccgctaacggacgcagggcgactttcggcaccactttaccttcggcggcaaactggaaggcttcagttaaatcctggcgcgtgccgaccagcgaaccgaccacttcaataccatccagcacaagacgtgggatatccaggctcatagactccggcggtagaccgacagccacaacacgaccgcctgcacggacagcatcaactgccgagttaaacgcagctttagctaccgctgttaccaccgcagcgtgagcgccaccagttttctcctgcacaattttggcggcgtcttcggtgtgtgagttaatcgctaaatctgcgcccatttcggttgccagttttaactgctcatcattgacatcaatggcgatcactttggcgttaaagacattcttcgcgtattgcagggcgaggttacccagaccgccaagaccgtagatagcaatccactgccctggacgaatttttgacagcttaacggctttgtaggtggtgactcccgcacaggtaatgctgctggccgccgccgagtccagaccatctggcacttttaccgcgtaatcggcgaccacgatgcactcttccgccatcccgccatcaacgctgtatccggcatttttaactgaacggcagagcgtttcgttaccactgttacagtattcgcaatgaccgcatccttcgtagaaccacgccacgctggcacgatcgcctggttttaatgaggtgacacctggacccacttctgccaccacaccgatgccttcatggcccagaattacgccggttttgtcaccaaaatcgccattcttaacatgaagatcggtatgacatacaccacaacactccattttcagcagggcttcgccatgtttcagtgagcgcagtgttttatacgtaacgtcaacatgatgatccttcgtaacaactgcagccttcatagttcctccttttcggatgatgttctgcatagcaggtgaggcaaatgagatttattcgccactacccagtatggatgagatctgaaaaagggagagggaaatagcccggtagccttcactaccgggcgcaggcttagatggaggtacggcggtagtcgcggtattcggcttgccagaaattatcgtcaatggcctgttgcagggcttcggcagaggttttcaccgccacgccttgctgctgcgccattttgccaaccgcaaacgcaattgcgcgggagactttctgaatatctttcagttccggcagtaccataccttcgccgttcagcaccaatggtgaatactgcgccagcgtttcacttgccgacatcagcatctcatcggtgatacgtgacgcgccggaagcaataacacccaggccgatgcccgggaaaataaaggcgttgttacactgggcgatagggtagattttatctttccataccactggattaaacgggctgcccgtggcgaccagcgcgttaccttcggtccaggcgataatgtcctgcggtgtggcttccacgcgtgacgtcgggttagacagcggcatcacgatcggacgcggacagtgtttatgcatctcacggatgatctcttccgtaaacagcccggtctgtcctgagacgccaatcagaatatctggttttacattgcgcaccacatccagcagtgacagcacatcgctgtcggtatcccagtcactgaggttttcgcgcttctgcaccagtttggtctggaaaggcagcaggttcggcatcttgtcagtcagcaagccaaagcgatcgaccataaagactttctgccgcgccgcttcctcgcttaatccttcgcgctgggtctgggagatgatcatttcggcaatgccgcatcccgctgaacctgcgccaaggaagacgatttttttctcgcttaactgaccacctgccgcgcggcttgctgcgatcagtgtgccgactgttaccgccgcagtgccctgaatgtcatcgttaaaagaacaaatttcattgcgatagcggttaagtaacggcatcgcatttttttgagcaaagtcttcaaactgcaacagcacgtctggccagcgttgtttcacagcctggataaattcatcaacgaattcatagtattcgtcgtcagtgatacgcggattacgccagcccatatacagcggatcgttaagcagctgttggttgttcgttccgacatccagcaccaccggaagggtatacgccgggctgatgccgccacaggcggtatagagcgacagtttaccgatcggaatgcccatcccgccgatgccctggtcaccaagccccagaatgcgttcaccgtcagtcaccacaatcactttaatattatggttcggcacgttttgcagaatatcgtccatattgtgccggttctggtaagagataaacacgccgcgtgaacggcggtagatctcagaaaaacgctcacaggctgcgccgacggttggggtataaataacaggcatcatctcatcaagatgattgtttaccagacggtagaagagggtttcgttagtgtcctggatgttacgcaggtagatgtgtttgtcgatttcggttttgaatccctgatactggatccatgctcgttccgcttgttcttcgatggtttcgaccacttccggcagtaaccccagcaggttgaagttacggcgttcttccatgctgaaggcactgcctttattcaacaacggaaattccagcagtacagggccagcgtaagggatataaagcgaacgctgtttttttgtttttggttccatgtcactcactcttttttgaatatccatccctggggggcttttatcgtctttgctttaccgccagggcgtcggcctcaagtataaagcagataaaaacaaaaacaccattgcgcaggcaatggtgtttaatcgtcattgaggactgatggttatgaattacttttcagcggggcgttttctgccggttgggttatttactacgctggatttgtcaccttcggtaactattttgcgctggttagaaattttatggtccagtccaagaatatgacgtgcctgacggttcgatttcattttaactcctcaatcctgtagctagttttaaggacaacatcgccgtagcgaagaaacacgtgctaaacccctaaattaggttgccgatcaagcatagcaccttaaagcgtagggtgctggccactgaccacataattgatcgtttgctggtagatatcactgaggatgtcgttatcagaagcttcaacccatttggtcagctccatgagaatgtcatcttcagtgacaacaccatgctgtgcccgaaggccttgctcaatggcattaaccagagcgggttctgctgttgaattttctgcctgataataagtaaacatagtgattctccgtgtctgtgtatttatggtgtctgctacggatcgcagatttataaagcacattcagcatggcaaatatttgccgcttcgttgttaagattagtcctggttgatgatttttatattttaacaccatgatattcatagggattgtgattggtatgatccgattaatattgatacaatatcttttgggttatatattcccggtaatctattgtgggaatttaatttaagtgcagaagtaatattttcgccggattttattcggaatatcctgcttatcctcgtgctgtttctcacgtagtctataatttcctttttaagcccacaggagagcaacaatgacaatccataagaaaggtcaggcacactgggaaggcgatatcaaacgcgggaagggaacagtatccaccgagagtggcgtgctgaaccaacagccgtatggatttaacacgcgttttgaaggcgaaaaaggaaccaaccctgaagaactgattggcgcagcgcatgccgcatgtttctcaatggcgctttcattaatgctgggggaagcgggattcacgccaacatcgattgataccaccgccgatgtgtcgctggataaagtggatgccggttttgcgattacgaaaatcgcactgaagagtgaagttgcggtgccgggtattgatgcctctacctttgacggcataatccagaaagcaaaagcaggatgcccggtctctcaggtactgaaagcggaaattacgctggattaccagttgaaatcgtaaagcattgccggatgacgcgtcaggcgcgtgaatgcctgatgcgttgttagcatctctacagcgcccgccagcaccggagctcacgtccgtcctcccttattgctaatgattgccggacttcacatccgtgggttgccagcgggcaacgttcgtagaaaaaacagccttgcggcaacgtgcggtttcccggcagatccgttttacgtaatgcccattcttcctccagcggtttatcaatggcggggagggaatccagcaataatcgggtgtatggatgtgcaggtgccgtcagcacctgctgcgcgtcgcccagttctacaatctgcccgagatacatcaccgccacccgatcgctcatatgacgtatcaccgagacattgtgtgaaatcagcacataggtcagcccgtgattttcctgtagcgttaccagtaaattgaggatctgcgcctgaacggagatatccagcgcagaggttggctcatcaagcacaatcacgtcaggctgcgaagagagtgctctggcaatggcgatacgttgccgctgcccgccggagaacgcatgaggcaggcggtcgagatactccggacgaatacccacctgcacagccaactcctctgccaacgctcgccgctgttgttcactactacgcttagctatccagagcggttctgtgatgatgcgccacaccggtaagcgcggattaagcgaagagagcgggtcctgaaacaccatctgcataatgcgttgtgagccagaacggatgtactgcccgtggctcggttgcagcatacccattaaaagctgtgcgagggtgcttttgccgcagcctgactcgccgacgatccctaaggtttcaccacggcggatctgtaaatcaataccattaatggcatgaacatgttccgtagttttaccaagccagtttttacgggccgggaaattgatatggacgtcgcgtaacgttaataacgtgtcagacacttataacctcctgctgcggataccaacaggcacagcgctggttgttgtcaccacacgctgtcagcgccgggacgttttcacactgtgcacctgccgcatagcaacgatcgcgaaaagcgcagccgtcaggcaaatgggtgaggtttggtaccgtccctggaatggcgggtaatagctggcgtggtactccatgttctggtgcgcattgcagcaaaccaatggtatacggatgccggggatgatggataacgtctgccgtcacgccgctttcaattacgcttccggcatacatcacgtaaacgctatcgcacagttgcgacaccacggccatatcatggctgatgaacagaaccgcagttccactggcgcgggctttatgtttaagcaaacgcagtacctgcaactgcaccgtgacgtccagcgccgtagtcggttcgtcggcaataatcaattgcggctcgcaggagaatgccagcgcaatcattacccgctggcgcataccacctgaaagctcaaacggatagcgcgacataacttccacggcatccgggatttgcatctcttccagcaggtcaatcgctttagctctggcttcccgacgacttattggttgatgatggcggatcacgtccatcatctgaagacctattcgacgtgtcggattgagggcggtcatcggttcctgaaagatcatcgccactcgtgcgccgcgccactgacgaagctgtttttcccgcgcgttaagaacatcttctcccagcagggaaatctgcccccgatgtacgcaataactgcccgtcggtagcagacgcataatcagcattgcggtgactgatttacctgagccggattctcccaccagaccgacaatttcaccgcggttaatctgcaaggacacattgttgagcgcgtgaacatcaccgttaaaaccggggaaactcaaatgcagttgttgaatgtccagaacgggttgggtcatgactgctttcctcctgctttcgggtcaagcagatcgcgaataccatcaccaaagagattaaacccgacggcggtaagcaaaatcgctgcccccggaaatgcgcaataccaccactgatcgagtacatagttgcgaccatttgctaccatcgcgccccattcagcactcggttgttgagcacccaggccaataaatcccaacgtggcggccattaaaatcgcgctaccgatatccagcgatgcctgcacgatcagcggcggtagggagttacgtaaaatatgccagttgatcagatgccaacgagacgcgccaaaggttttcgccgcctgaacataggtatactggcgtacaactaatgcttgcccccgcgccaggcgcacataaaagggaattcgcacaatagcaatagccagcatggcgttaaacaaactcggcccgagagcggcagccagtgccattgtcagtaccaacgaaggaatcgacagcataatgtccatgatgcgcatgatgatggcgtctgcgcgtccaccaagcacaccggatagacatccgagtagcgaaccaatcatacccgcaatggcaaccacgactaatccggcgagaattgattgctgactgccgaccagtacgcggctaaacagatcgcgtcccacttcatcggtgccaaaccagtgcgccgcagaaggcggcaaaaggcgggcggttaaatcaatggcgttgggatcatgcgtcgccagccacggtgaaaaaatcatcatcaatagcattaatacaatgatgactgcgctggtcacggtgagcggactgcctttcagcatccataccagttttgcaccgttaaatcgcgtttgtttttgtgggcgtacggcggacgtttcctcgcttagcatcattcaccacctccacgtccgatacgcggatcaatccacaaatagagcaaatccaccaccaggttgaccagcacataagcaaatgaaaccacgacggcaaagcccatcactgccgggaagtcgagcgcctgtattgatgttactacccatgcacccattccgggccaggcaaaaacggtttcggtgagcactgcgccatacaacaaatcgcccagcgccaaacccaatacggtaatcgatgggatcaacgcattgggtagcgcataacataaaacgatataccagccgggcaagccgctggcccgggcggtacgaatgtagtcttcactcaattgttccagcatcgctgagcggatctggcgagcgacaattcccaggtgaacgaacgccagcgttaatgccggtaagatgagatgttgcaacgcattgaagaagacttcaccgttgccttcaagcagcgcatcgagcagataaaagccggtaacgtgcgttggtggatccagccagtcatcaagccttccgccgccgggaagaatttgcagatgaccataaaacagcacaatgacgcccagcccaagccagaacgcaggtgtggagattccggtaatggccattattcgcaccagatgatccagccagcgatttcgccagactgcagagagtatgcccagcgggatgccaatcaggagtgccagcagcagggcaccaaaagccagctccagcgtcgccgggaaaaatatacgcaactcttccagcaccggacgcccggtacgaatggatgttcccaggtcaccatgaaacaggtcgctgacgtagcggtaaaactgtacatacagtggctggtccagtcccagttgctggcgaatattttccacgatagcatcgctggcgcggtcacccgccagtaaccgcgccggatcaccagggatcagatgcgagataataaacgtaatcacgcagacgcccgccaccacgagcaccagcccccagcagcgttggcgtaaaatactccagaaggtcacgttatttactcatggtattgatattgaagacctgttccagcatgggattgaacacaaagcctttcacctctttgttcatcgccagttggtagtttttctggaacaggtacacataagcagcgtcatcaatgacgattttctgtgcctgctggtagtcccgggtacgctgcgtctggtcggtggtcgcaagcgcattgcgcagtaacttatcgacctcactgttttcatagaacgagcggttacccggcagaccttttttgtctgactcaaaccagtaattcataaacatatacgggtcggcaaaatccggactccagttgccaatcgcaatgtcgtaatcacctttacccactctgtcgcgcatggtggcgttcgccagcttttccagcttcacaatgatgcccagcttgttgagactggattgtgtcgccagagcaataggctcccagttcggatcgttatcggagtagagaaacgtcaggctggtgggtttgctcgtcactttatcccattcggctttggctttcgtttcgtcatggttgtattgcattgccgtcgcatcgtagccccacatgccttccggaatcgggccgcgcatctgttttccgttaccactcagaatgccgttaaccatgccctgataatcggtagaccaggaaatggcccgacgcagatccgcctgattaagaggcgctttgctgttattcagatacagataggtaacgcgcagtgacggatactctgccacattgactttattttcctgcttcagggcgttgagttgatccaccggcagcgcatcggcaatgtcaatgtcgccacgggagagctgcaggcgacgggaggcactttcaccaataatttttaccgatacccgtttgaagttcggtttattgcctgggtaatgcggatttggcaccagaactaattgctgacctttttgccagcttttcagcataaatggtccggaaccggcggtattttgcgcgaggaagccgcgagcatcatccgctgcatgttcctttaagaccgccggattgataatggatgcaccgtcattcgccagcgtgtagaggaacggtgcgaatggttggctaagggtaaacttcaccgtatgttcgtcgggagcatcaatctttaaatctttgggaaatgcttctgctggcccctggccgatttttagtagccgctcaaaagaaagttttactgcttcggcagtgacaggtgtgccatcggcaaatttagcattatctttcagggtgaacgtccactctttttgatcgtcagacgctttccagctacttgccagatcgccttcaacgtcggttgagcctttatcaccgtccgttttgtactgaaccagccgctgataagacgggtaggtcactgtccagtcgttattatctattgttaccgccgggtcgagggtttgtggatcggcggccttaccaatcaccagcatatcttttggtacggcggcgtgcgcaaccgggaaatttgtggcaaggacgagcgcgagcaatgtgggacgaaacgatatcgatctcttcatgacagtttcctgattaactgacgtgctgtgtgccaggggatataaaacaagagaattgatcagcgagcagagggtaactcgctgcctggggtaattcgaagtgccaccattcgctggagataccgacaaaaccgccaccagtcattatcgcattcagcaacagccgattgcgctgagcggcgggcgggacggaagggtgataggcatgggagcgctcgtgcatttcatcgaaccctgcgcccatatcgaggatgttcccgtgctcatcacgaagcgtcaggtcgatcgccgtgccacggctgtgattagaaccgaccgtcacatcaacaacatattgcgggtctgggcaggcttgccacaacatcgcctgtgcttgttgtgggcgatacgcatcgtaaatcaccagttgtaaccctgacagctgggcgatgctgatacttttcgccagcgcggtaatcgcatccttgtgtaacagacaacgcgcttgctgataaatagctttacctgtgatgttatcagcgcaggcgtatttcaattcgatctccagatcagggaagattacggctaaatcaaccagttcggtggtatccgacataaacggttcctgtataagacaaaaattgctgcgctttccgcttatgcagatctcatgccatgccgggataagcgccagaatgctggcttaaagttatattttttaacttttgatcaacatttgtgcagcgtagtgcagttttggtgcaagaggggaagttaaggaaggaatctcccggaatcgtagctgaaatcacagtatttaagtgacagtgtcacgttaaatgaaaacccgcgagtgcgggcgagaggaatttgtcagattttcagcggtaacacgctgctcatccagcctggaatttcttcggcgggtagggggcgggaaaagaaatatccctgaataacgcgacagtggatcttgcgtagcatctcaaattgctctttggtttcgacgccttccgccacgacggttaaattgaggctttgcccaatgctggtaatggcttcaagtaaggcaaggatgcgtttttcggtcagacaacgatcgacaaaacttttgtcaattttgatttccgttaccggaagactgactaagcgggataatccggaaaagcccgtaccaaaatcatctaccgataagcccacgcccatatcacgcaggatctgaatgcgcttaaagatttcggtatcgtgttccatcatcatgctttccgtgatttctaccgtcagctggtggccgtcaataccccaggcgtgcattgcatcagacacctgattaggcagttgattactgcgaaagtgcagcgccgacaagttcacggataacgccgggatatgaatattctggctacgccattctgctaactgacggcaagcttccgcgatgacccagcgcccaatattttcgatttcaccaatctcttctgcgagaggaataaaccgtgaagggggcacatgaccatgcaggggatcgtgccagcgagcaagggcttcgatgccgtacagttcacccgtttctgcgaagatttgcggctggtaaaccagtttcagttggttattgctaatcgcttctttcagcgctgcgcctaaaaccaaacgctcttttaccatttcgttcatcgccgggctgaagaactgccagccgttaccgccattcttgcgaatataatccattgcattgtgagcagtggagagcaagtaatcgcggtttttacccaggtcgtagctgatgccaatactcaaggtaagcgggaagggtttatcgtcaatcattatcggcttgctgaccacattccgtagctcatcggcgatttgggtaatgttactgacgtcgttttcgaggctcacgaggacaaactgcgtaccttcgatacgacagagatactgatccggtttgagtttttcacgaaagcgattgaccacttccagcaatgcctgatcggcccacgcatagccaaggctatcaatcacatcctgaatatggtcaacaccgatgagatacaccacgggagagacggctttgtcgaccaggtcatcgaggtaattgtgcaggttattgcgatttggcagaccggtcatcggatcaaattggatgagttgttcaatatgctgacggcttttttcctgttccagcgccagcgcggccatatgctggctgatatctgccacgcgttcgataaaggcgctggtttctgctcctgacgaggttttaatttgcaggatccccgcaggcgcgccatcacgctgacgaatggtcgctgaccagctttgcgcattttgaatttctgcaccgtgggaagatgacgcccagtgtatcggcatcccgttgcgcagtgcgaacagcgaaacatgcgattcgttgagtacagattcgatgttacgacaaatgatttcccccatttcatgaaatggcgggctgctgcacatggcggcgagaatattgccttcaagctggcgaatctgccgttcttcggtgatatccgagaaagtcattaccaggttctgcagatgcgcgagcacgtcataaaccgggctgatagaggctttaatccagattttttcaccggtgcgcgtcaacagcagaaattcgtcctgatcgcgggcggttttccatagcaactgttgtaaacgaatgcggttatcggcagggaattcaggaatgttcaggagtgtatcgggctgcataccgctggcttcgctaatgcagtaaccaaacatttcggtaaatgcgcgattgcactgcacaatatggcgttccggatcgaggacaatcaccggtcggtcgagatggtcaacggcaataatcaattgtcgggtctgttctttttgcgccatttctacgctggcatcccgtaccagcgccaggtaataaactttcccctcggcgctcactttcgatagcgcaaaacgggtccagattttactgccgtcttttttctccagctgcagctcccgactcatcccctcaacacgcgctttaccgccttcacggttgtgacgaatgtattcaggatgcgcaggacgcaaatcccgcggaatcagcatatcaatgttattgccaatgacttcttcacgtttgtatccccagagcttctctgcggcggggttgaaaaacatcacttcatcattttcgttaattaacaccgcacccatcatattttgctcaagggcggggaaaaaaatgccatcggcggcattatccgcatcggttagcttcatgattacctctgcatcctggcgcatctaaagactggctttccagagttcaacacggtttctacctcgtcttttggcgatatacagagcttcatcggctatttgaatgaggcgctcatagtcaggatgaccattaaacatggcggcaccgatggaaagtgagagggcaatatcttcgccgtttgcggctttcagtttggttttctccacccgactgcgaatacgttctgcggtacgtaacgtttcgttttcagaagcttcagtcaaaacaatgataaattcatcgcccccgtagcggaaaacataatcactactgcggacgttgtcataaaaggcctgagagactttacgcagaatttcatcaccagtgttatggccccacgtatcgttgatctctttgaatttatcaacgtcaataatcagcactgacagcggtgtaccggtccggttggcatgggcaatttcgcgtttgaagatagtcggtaggaaacggcggttaagtaatttcgtcagtacatccataccgacttcgtggcgcgatacttcttcaaacaattcacgcagcaaggtaataatttgcgatacggtatttcttatctgtaataaaaatttcacccgcagacttctgttattcaaatttctggtgttacgcatggtttgattgaaaataccgtcgaaatcctgaatcagacgggagatatggcctacttcggcaataccactaaaataatgtcgacctttatggttaaaccacaggccaaaatcagcctggcttaaaggcaaactactgcctaaatcagaatccagcaggattttatagataatatctatttcccatgaaagtattgaggctatttgccgttctttttcttcttcggcgttttccagtaacgagaagatacgatagttttcatcttcctttgaggcactactgtcactaaaggtaaacgcgcgagtcatcacttccatcgcgatatcaatactgttaatcgagaaatggtagacctgaagtttttctgcggcggaataatccgaagagaagatcaccggatagaggatttttttcagcacccgaaaccccatctcgacaatttctaccggaattcctatgcgggcatgcacttccgcgacggtatgctggatttgtattagcctttcgacatcgtcaacctgggcagaaagcacgttaataatccagcgttccatcgcactcttcaactgccgctcaacttgttcattactcaagaattcttcggcatgcgggtcgatgcggacaattcgataaaactcgatactcagataatgagcatgcgcaacggcaatttccgcggctttagcacgaatgggcggatctgcctgttcgacaagtccggtccactcatctttcattcttttaaaatacatctccataattcacacccttataaggctgggaaatcagacggaatcaaaatgaaacgcaacgtgcgagatcgactaactgcaccatattctcctgaaatatgaagatatactgaaaagaaataagcgatttaggacagtttcaatctacgctactgttcttcagaagagtatagcccatcgtaattatttttcggtgacagcgaatatcgtatggtttttcatattcatacatttttattagggatttatggctgtttaactaagtgtggttaatttgacttaagtaagcatgattattagtgggatagtttaagagggtaacaagccggtgggtaaagcaccggcttgttacaaagtaagaatgggagtttaactgccccagcgactttgcagatagctgaccgcttgttgagtctgcggtttattcagatagtcctcacggaacaagatggtgccgctaatttcgggcacagcatcgttaagatcgagctgctttttcagttccggtacgccgccgttaatcatccagtctggctctatctttgaaggttcacccactttatagaaggcgataccgatatacaggcgggtcctggtcggtttaacgacatccgcccaccattttgccaacacgtcataacgcgcggcactccgtgagaacggccagtaaatttggggagcaatgtaatccagcaatccttgttccacccatcgacgggtgtcagcgtaggattcgtcataggctgccgcgcctcgggtatcggaaccgagcggatcgtgtgatcggttacgccacacgcctgccgggctaacaccaaattcgactcccggcttaatgcttttaatggtgtgcgatacctttgcaattaactgctgagtattgttgcgccgccagtctgcttttgacgcaaatgcgcctccgtatttacggtacgtttcgttatcatttagccgtgaacccggtgactccgtatagaaatagtcgtcaaactgcacgccatctacgggatagcgggaaaccacttctgcgactattgatgtgatccagtcctgaacctcagggatgcccgggtcgaggacaaagcgatcgccagacgttctgatccagtcgcggtgttgcacatagacgctcgccggttgttgagacagagtgctattcagttccctgatagtaccgggcttcgtattaaccgatacgcgataggggttaaaccaggcgtgtactttcatcccacgcttgtgggcttcgtcgagcataaattgcagcggatcgtaacccggattttcaccaatcttaccggtcataagatcggaccacggcaaaattttcgatggccacagggcggtaccgtccggcttgacctggaaaaagaccgtgtttatgccgagacgttgcagatgatccagtttgtcgatcatcgcctgttgttgtacacgggcccggctggtggggttactaatgttaaccgaggaaaccggtggccagtcgagccgagaaaccgtggccagccagatgccacgcatcggttgtgacgattgttgcgtcgtggctggtggctttgaacctgctggtggtgtcaccatggactctggaggcgtgcttttacaactacacagtaaaagtgccagtgcaactagtatcgctggtcttctaatcgttaatttcttgtttcgggagcagatatccatatgtgctggtttccggtaaacagatgtgcgctcattctcgtacttatccccgttaagtcaatacgacagcaagcacgaaaaagggagcgatgaattatcgctcccttgtcttataaccattcagacatggttagtgtttcttgtcattcatcacaatatagtgtggtgaacgtgcacgcgggtgcaggaagaagtgaccttttggtgcgttctgactgttgattggctccagagtgacgccggtatttgctttgcctttacgatcatgaacagcatagagaataaagggcagggcaagtaccaccaggaaactaacaaccagtaattcaacatacatatcggtagaatcaccctggatgttatccggcggcaggaaggaaacaataaacgccataattgaagtcagcagaccgacaattgccacgaccagtttcacccctttaccaccagggatattaaatgtgcgttttaagtcaggatgtttaagaaccaacacaatgtagccaataaacagcatgaaataagcacacagataaatcaccaccgtcagcgccagtgcgatcaggaaggacatgttgttaccgccaccggtattggtgaggatgatcaacgcgatagacgtaatcaccagctgcgaaatgaccagcgttaccggtacgccatttttgttcattttagcgaatgccgctggcagcaggtttttctgcgctgttacatacatcccgcgagaaggaccaacaatccaggaggcgatttccgccagaacacccagcaacagcagtgcggagatcacgcgaaccgtccactcaatttctggtgccacatgggacatcagaacggtaaaggtttgcattacccctgcggagaggttgatttcattacccggaatgaccatcgcaatagacaaaccaccaacagagcttaagcagattgccgccaccatcagcagtaacatagccaacggatagtcgcgccctgggttgctcatttcattgacgtgggttgcggatgcttctacgcccatataactcaaaatgaaggcaacaaatactaccagggtgcccactttagagaagtcagggaagaaggtcttcgaatccatttcgatagcaacgggggcaccggagtgcagataaatagccgctaatgcgatcaaaataaatgcaggtaacaggataccggcgaagaagccaactttagcaattcgcgccgtgtatttcgtgccaccaaactgcgttaatgccagcgcccaaagaatgatgagtgctgcaatagttttggtaatggggtcttcattcagcgctggccatttcaggatgtaggagagtgcccctaacacgaaatagagcatcggaataaaaccaatggcgatttgcagatagccaaatgagatcgctgcaaatccccatctcggccccagagtatttgatacccaggcgaagacaccaccttcttcccagccgtcgacggtggccatttccgcagcacaaagtcccacgggaataaaccataaaatcccgcctaatagcaggaagaagactaatgaaaagcccgatgttgcgaaggtagggtattcataaacagccattaccatcgatgccgttatggcaaagaatccaagtaatgtgagctgcttagctttacctgtctgtactgatgtagccatattatccccctaaaacggtattcctgtcggaaccgcacctgttttgttctgaagcgtattcagaacaatattttccgttgctaatgccagtgaacagactttggaaattgtcccgaaacgggttcgtttcgggacaccgttaccgttaaacgttatcaggtatgtttaaagctgttctgttgggcaataccctgcagtttcgggtgatcgctgagatatttcagggaggctttgtagtcttccagcaacagttcagcaaagtccatttcgaagccgcgacgacacataatgcgcatcaccacgatgtcggtggcttcaccgccgagagtgaaggccggaacctgccagccgcgcagacgcagacgttcagagaggtcatacagggtgtatcccggatcttcaccatctttcagtttgaagcaaaccgccgggatgccttcgtccgggcgacccgtacagatgaactcatacggccccagtttggcgatttcatccgccagataagcggcaacctggtaagaggcgttctgtactttggtatagccttcacgaccgaggcgcaggaattcatagtactgtgcaattacctgacccgccgggcgggagaagttgatggcaaaagtaccaatttgaccacccaggtagtcaacgttgaacaccagttcctgcggcagcgcttcttcgtcacgccagataacccagccgcagcccagcggagccagaccgaatttatggcctgaagcactgatcgatttcacacgcggcaggcggaagtcccagacgatatccggggcgacgaacggtgccaggaagccaccgctggcagcgtcgatgtgcatgtcgatgtcgataccggtatcggcctggaatttatccagcgcatcgtgcagcggttgtgggaactcatagttaccagtgtaggtcacgccgaaagtcggcaccacgccgatggtgttttcgtcacaggcttcaatcatgcgtttcgggtccataaacaactgaccggggcgcatagggatctcacgcagctccacatcccagtagcgggcgaatttatgccagcagatttgtaccggaccgcacaccaggtttggtttatccgttggtttgcctgcagcttccatacgcttgcgccaacgccatttcatcgccatcccgccgagcatacaggcctcggaagaaccaatggtgttggtgccaacggcctgaccatttttcggcgcaggcgcatgccacagatcggcaaccatatttacgcaacgcaggtcgatggctgcggattgcggatattcttctttgtcgatccagtttttgttaatggataaatccatcaatttgtggacattttcgtcgtcccaggtctggcagaaagtggccaggttctgacgagcgttgccatcaagatataattcgtcattgataatctggaatgcgacatcgtcgcgcatttcgtgcagcggaaaacgttttgattctgcgatagtggaaatagacttcgcaccaaaacgtgaatcgagtagttccgaccttaaatccgttacttgcttcttatccattttaaactccttaaaatgattggatcgcattaaaaaagtaggatttatcgataaagtaagcaagtgcaaaggactcgtgtttaaataacaaaatcctaatgttatttatcgtgagatattacgcgaataatattttttcattgaaaaacaatacaatatgaaattcttgggtggtggtaaggtgttttatgctgttatttttatgcgcattctgtgtctcctgaattatcacgtaaaaatcagaccttaaaatatcactattagtacttgattattattttgaacgcatttataaaattattacataaaaatagcgaatattgctaaaatccccgccaacgatgtgttgacggggctgttattattttggcaataatactccggtataagtatttaccggatgagaaagatattgtttaacggcagtgttaacattctctaccgtcatttgtttcaacaattgctcctgctcagtccatgctgcaggatcgtcatattgaataagactatttacaatagtgttcgctaattgttgaacgctacgctgttggatatcgaggctgcgctgaacgttttgctggtattcattcagttcttgctcactgatccctttagccagacgcttaaccatcacttcattcgctaacgttaacagttcatcatgtcgttctggttgacaagtaaaagccagcaaatgactgatatctttggcctgaggatcaaccgagaggcgagaagaaacgctgtatgctccagatgcctgttcacgaatattaacacgtagatcttttgccagtgcgacgttaaaagcatcgagcgccatacgcgtcggcagattaacaggtgtccgggaatcataacgcttccactgtgaaacctgtgccacaggttcattttgttcttttacagtaaccgatgcgttgtccgtcgcgcgagttaatggtttacctgcggctaatggcgaatcagagtgtttgattgatcctaagtaacgcgtaattaacgccacgagtttgtcttctgcgacattaccgacaatgacaaacgtgatatccgctggagatgaaaacaattggcgatcggcagccagcgcatctgcggcagtaaactgtgcaatctgattttcttgcagtaatttcgtgcggtcatcagcatagcgcgtctcatacatctgctgggcgaatttctccgctggacgctggtcgagcgttttcaacgcctgaatttgagcattttgtagcgatgcccaaatattatcgttaatcgtgctgtgggtgattcgctggttaatcaactgaaaaccaggttcagggttattagtccgcgcgctaacggagagcaacgtattcatgccactgactttactgctcatggttaccgaattttccgcactccagcgtttcaggctggaagaggagagttcgccaacgccgcttccgctaactgctttatttgccagcgcgataagtgatttttgctgcgcagggaaacttaaatcgcctttattcgatacggcaataatttgtagcttttgctcttcacccgcggattttgccagaataaccctggcaccattggaaagtgttaatgatgtcagattctccgccagcgtttctttgctgctaatttccgcctgtgggtctgcgtctactgttaacgataaatttctgcctgggaagacgtaagccgccagctttttgttggcgtactccttttccagcgccaggatagccgcaggagacaatgcttttttggcggcaacctcattgtttaccatttgctcccaaaatgcgtcctggttctttcttaactgctgccatttttccgccagactttgcacggtaatttgctgccacagacgtttcgaaagttgatatgtctcttccggcgacaagaacggcgtattatttaatgagctggatgccaggcgactggtcagcatacgtaaatcacgttcagcttgctgatcaaccgcatttttcagccaggtgaggcgggtagatttgacatcatcgagttcttcagcagaaaaaccatgctgatcaatggttgccaactctgccattaatgcattcgcagcatcctgcatattatcgtctcgtgcatttacacggaaaaacagcgactgataatcgggtgcaattttaacgctgcgcgcagtgccgccagaaatagtcttcaactcgcccgactgtatgcgttcctgcagacgttgattgaacagctgaactaacatgctccattcagcttgttcgataaagctttgctcatcgttcacttgtaccattggcaggcgataatagagtgcgatgccgttcacccggttttctttatcattaatgatattaaagcgcaggtggttttcggcttttgtcggccagacgcgattttcagctgctttgttagccggaagcttacttaaattatcctttatcagcgccagcgcttctttactgtcgatatcgccgaccacgataaaggtcatattatttggttgataccagcgttgataaaattggcgcaattgtgccggtgtgaccgtggcgacagtatccatcaggccgataggttcacggtctaaattacgggtatttgccagcaggaaagggcggcgcgcctgagaggtgcgccatttcgcatcctgatgggcacgccattcctcagtaattacgccacgttcagcgtctacttcgagtttttcaaaggttgcggcattactccattcactgaagattgccatcacttgttgcagattttgtttctgcgtagtcggcaaactcacctgatacaccgtttcgtcatagctggtataggcattaacatcgcgaccaaaacgcaggcccattgactcaaatgtttcgatgactttattacccggccatgtttttgtgccgttaaacatcatatgttctacaaaatgagccacgccgagctcattgtcttcttcctgcaatgaaccggtatgaatttgcagccataaatttacctgatcctttggatgagcatgcggataaatcatatatcgcaagccattgtccagttgcccggtaattaacttttcatcctgcggtaaggcggcggcaatcagccgcccggggagcaacagagttgccactaacgtcagtaagaaacagaggtttctcataattatctccatgcgaaaaccgggcgaatttacccggttaagtaaaatccgaactattaaaatttcatgctgacatcaagccagaaagtacggccactggcgtaggtcgccacaccggtgttcgttgtatcaacagcggttttgctatccagtacattgagaatatcggcactgatcgtcaggttttgttgttgcagaaattgtggcgtccaggacaagcgggtgtcccaggtcaggctgctatccagtttttcgtcaacatactgcttgtaatctgaatattcgctgatgtattgcgcatttgtcttaccaaggataatgcgagctttacgcgcttcttgccaggccagcgtattcgcccacactaacccgctcggttgatgcgtgaaatccatgtttaaggagatctttaatgggttattaaaatctgccactggaacgctatcgtaagagaccagattaccgttataaaccacctggttatcaccggtattgctctcctcataaccattgtttaacgacaagttgcccttgctcttgatatagctaaagacaatttgtgggttaatatctacctggcggatatgcaggggttcggccagttcaaaactgaggctgaacgaatgcgttttggttttgccatcgttgttatattcagtaatggtggttttagtcgcgctgtcggtacgactgcttttgctgatttgatcatgcgcttcacggtaaacatagtttgcacgcgcaataacgttcttaccgattttctgctgcaatcccattgccagttcatcgttataaggcgttttcaaatcctgataacgcgtcagagttttattacctgataccgattccgtccagctattgcggatatcacgtaatcccatatcaagaatattcccgccatagtaacggttataacctgctgtaatcattgaggtttgattagcaaaaatatcccattccgtcataaagcgcggggagatattgtggtttgacagatagttgtcatagtcataccgcacgccgggcattaatgacacattacgccagctaatgcgatccgccatatacagcgtgtagttgtcaattcccaggcggcctttacctttatggtaaatggtatggttagttttctttccggcagcattaatcacataggattcagactggttatggcgttcagtccacgcatcggaatagatgtattccgcgccgaagtagggttgatgcgaaacattacccacggcgaatttttgccagtccaggcgtgttttgaaggtgtaattatctacagcctgggaaatgtgtcctaatccgccacgggtgcaacgccctgtaatatcaccatatgtacatgaaagttcggtgtaccagatgtcatgatcgtgacgggtataatcactaatatgatcccaaccaacggtggtacgcagtttggcccatgcgagctgcgtatccatatcccatgccagaccataggatttattacccatttcgcgatcagactgcgggaaggtgctggtattataatcacggctggagccggtatattttaaggttaaatcgtgggtaaagcggtcgctggcaaaccaggtaaatttgcttaatgcagtatcgataacgtttttatactgtgcccgaccggcgacaatgccgtcattcgaaacataatccgcgcgggtgatatcagactggcggcgcgataaaccggcggtaacgccgaagttatcagcgagttcctgattaaacgacaaggtataaaagttctttttaaaatctggggagtaataagtacttcctgaagagccttgattaaatgcgctcttgttattctcatcgatatgcgatgttaaccagtccgaacgcgtagtgcgataacccaatttcaccttgctatcatcagcgttgaagcgtttgatctttgcatcaattaccccgccattgaagcgaccaaattcaaccggcacaaaactgtcataaagcgtcacattgtccagtaagctgacatcaagataatacccctgtgacatcccgctaatattggttgcactactggcatcggactcattcgctgggttcaggttattagttgcactaataccgtcaatcaaataggcattctggtagggcgacgcaccgtgaatagagattttctcagggcgaatatctccctggttcaacgaggtactttgcgttgaatccatgcgtaccgcagggttggttctcagcagatcgctgatattgccattcccggtcggtaaacgctcgatgctttcactggtgtaatgcgtgttgccgtttacgggtacagggacaggagcatagaccgtcatctcttcaaaaaaatgcatgtacatgtttttgtcatcgacggcctgcgccacatcagcgccacataaaatgacgccaggaataagaactcgcttcatttatttatatctccgtacagcagggcttttattgtttttataaaaccgcgctaatgtcacaaatatcatcggccaggttccagacaccgggttgatgtgtaaccataatgacgccgcttgtgggtagtttttcacgcactaaacgcagtaagcggatagcctcttgttcctcaagatgagaggtagtttcgtcaagaaatatccatttcggacgtcgtaaaattaatcgtgccagggcgatacgttgtttttcgccgctggaaagaatatctccccagcgatcgtggtcatgaatacgcgcagccaatttcccaagaccaacctgatgcagtacttcgctcaacgatttatcgtctacgggcaggggaagtgctttacaaataatctctttcagtaagccggttttgattaacggtgtttgtgacacataccaactgtcagcaggagaagaaatatcacctttaaaccacggccagcagtgggataatgttttaagcagtgtggtttttcccgcgccagagtagcctttcagtaatagccatttgcctggcgaaacatgaaagttcaggttctctaatatgatcttattatcaggcgtacgaatactcgcatcagccacttgtaccgcatgttggcaatttttaggcttattcgtagggcgctgttcagtgagttgatggaactcatacaagcgatcgataaccgcagccagttcagcaagttcgtcatatttataaataaaccagcttaaattgttcgataccagcataaatgcctggcgcgatttcatcagtccgcccagattgatctgcccgctaataaactgcggcaataacagaaagtagggaagaacgctaagcgagcgcgaataaatattctgccagtaatcaagccaccgctgacgattcattaaacgatgccagttctctttaatggtatgaaaattgtcgctcaactcctggcgttgtagagactcagcattgcttagcgcaatcagttctgcctgcttattatgctgcacaagatttgttcgaaatgtcgcttcgctacgttgtttttccacattaagcggacgaatacgtttacccaccttatgggtaaataaagttccaccgatcacaatgagcacgacggtatagaccatatacccctggatattccattctgttccaccaacagtgaatgagagcgtacccgcgctttcccaaagaataacggtaaaggtgatcagcatgctaagtgactggatgaagccaaatgaaagactgagcgttttgctgatcagtaagagaatgtcttcagcgatacgttggtcagggttatctgtatttttatgctcgccgtagatctgcgtgaagtagtagtttttatctgcaaaccaccgattaaggtagtaatctgttaaccattcgcgccagcgaatagtcagtagtttaattaaccatgttttgtttacggatattaatacaaagatccccagcagggcagggaaccaaaggacaagctgccaaagcttatcggtttctttctggcttagcgcattgaaaaaatcattattccagtcgtttaaccagacctgaattttaaccacgccaaggatcatggcgaggataataatgattaacaacactgaagttttattattcttacgcagccaaaagggcttcaacagacagagatactttgctatcaacatacgaagcgtaatgggaatggttatcattagcgaaaattgattgtgccatccaatgattatctatggcaatgatttactgatgaaatttatttaagtatcatttaacaatatgaaatataaaggaatatttcattttcagtggttatggttatgctattgataatcaaggatattgctaatgccctgatgcataccacgtaagccaggattttcgcaagggaagatgatgatgacgaaacacccgacaggaatttatgtcgggtgccttgttaaggtcataagaaggaggctaagaatggagttaaaagagagcgttattaattattctccatttgttttgcaacatccataatgtggtaaagcggtactctgttcttagctaactctaccatggcgttcatataaggtaccatggttgaaaaaaggattttataaccttcgcaaaaataagaaacagtctcattgtttactttagtaatacgatgcttaggacaaccgccattgcagataggtttatatgcacattgctgacatttcgctggaatccgttttttttgcgctgtcagttgtacactgttcatcgttttgagttcagatttattaatgtttccaattttgtactgtggatagacaaaatggtcgcattcgtaaatgtctccattactttcaacaaccagattatccttgcaggactcctggaaaatacaactggtatgcccattccccaaaaaacggctgacaaagctttcaaactgacggatgaaaatttcacccacatcgtttttaacccattgcataaaaatggttgacataaacttgccataagccgtgggaggcacagaaaaatcaatgatacggaatgtgttctcactatgaccactgaaatcaatattcggcgtcccggtttctagcaattcgataaattgcatatgtttactgccgatagattttaaaaaatgataaacctcaagagggtaatggacattaacgttattaatgacggttaacgtattaaactctacttgatatgatttcagacgctcgatggctgctatcacttttgcaaaagtaccgttacctgaattactgcgtctgtaacggtcatgtaactcctgggggccatcgatcgagataccaaccagaaattcatgttctttgagaaaggcacaccattcattattcaataaaatgccattcgtttgtaatgcattaaaaatacgtttttggcctgcatagcgttgttgatagtgaataactttacggaaaaaatccaggccagccagagtgggttcaccgccttgccaggtaaaatagacctgattgccagacgctgcgatatattgtttgatgaactctttcagagtgctgtcatccatccatttttcatgagtaaactgcgactctttttcaaggtaaaaacagtaatcacatttgagattacattgaaaactggagggcttggctgtaacgtgcatcgctatctcgctcaataaggcggcggaaaaatccgccgcatgaaggtttagttatttcgcttcgcttagtgctttcttgatattgttaaacttctcctgatttacctcgctaagcggtggctggctgctgtcgataaactctcttaccacgccttgcatctctttaacgacctgcggattggcggcggcaaggttatctttttgctgtagatccgtcagtttgtagagacctaactgattgttttctactgtatagacaagcgaataatcgttatttctcaccgtataagagaattggcttaagtcctcagtgttggggttatgcgggtaatcgtctgactgatggcgaacaaatttgtggtaattatcccagaatggaatattttcctcgtcaaaccagtgagaataagaggttatccaggtcagatttttatgtggctcgccttgtttcttatcttgcaaccagggcagcaaggaaacgccatccagcttaaggtcttttggaatgctgatatcggctgcatcaagagctgtcgggtagaaatccattgcggaaatcagcttgtcataattaccgggttgaagttttcctttccaccacataaacattggggtgtgagtaccgccaggataggtctgactcttatagcctttttgcgccccgttcagcggcagaggaccatcgataaccgcaccattatcggaggtaaagagaataattgtattgtcatactgtccgtttttcttcagttgttcgagaatgcgttttacaccctgatcaacagaataaacggaagcgtagtagttatctgctgtttgactaccggtattaaattgcttctgatattgatccggtgcaggattatcatttggcaggtgcggagcattataagccaggtaaagcataaaaggctggtcaagtgttttggcacgatcaacaacgccaattgcctcatcggttaactgatcgctgatataaccttttgcggggacacgttcacgatttttgaacagtgaaggggagttgtaatatgccgttcctgcagcgtggaatcccataaagtaatcaaagccacggttttgaggttgccattcttccgcagaaaatgtggtgaagttgtcatgatagtcacgcgtttgtttatcttccggtaccggcacattactgatttttgacaagtgccatttacctactgctgcagtgtaataaccatgattctggaataattcaggcaagaaagtttctgttagcggaataccatcctgagcatcggtattggaatagacaccaaagcgggcgggagctcgaccggtcattattgcggcgcgggaggggccggaaacaccgtgtgccacatagccgttagtaaaacgtacgccttcatccattaatgaaaggagcgtcggcgttgatttttgtgcagcttcaatggctttatctatccctattttgtaggtatcgacaacttcacgattttccattgtttttgggtcaaaagatcccttatcaaaaggaagttgtccataaccaagatcatccatggtcagtacgataatatttggctttcctttggtactgtattctgtcggcgtaaagtctgagaaagcaacgtttgttttggttgctttcagctttacatcatctgccgcatgagcagcaaatgcagccataccagatgccagtatcaaagatatcgaggtacttacgacacttttctttaatgcagacttcataaatgttcctcttcttattgtacttaattccaaagtaattttacgaagagaaataagtggatgtaagtgaagttagtcacataaagagatagcagatttagctaaaaaaagggaaaaaacagtccataaagcgttgacattactttctgttctattaagtaatttctcgccgataaacaactaatttattgatatttaataaattattgcattttactgacaaaatgcagaattgagatcataaataatcatgcaacaggttatgcaagtgcataaatatgtgatggatgtcacttatttatttcaataaatatatcgcctaaaaacaacgcggggcagggaatggctgccccatttaattcttacgcagcgtgtgtggttgactactcgttagcaaataatcaaatagctaaagcattcatcgtgttgcccgtattcatacccgtgtgactttgacaacggtactccttagaaactctcttcggactgttgccgaaatgtttgcggaacgcataaataaaataagatgtactggcataaccacattgttcggcaattttattgactgaaccttctacgcgtatcaaattttttgcgtgctgcattcttgcatctaaaagaatctgtgagaatgtcgtttgctcttgcttaagttttttcttcaacaggctttcactgatgtacaggcagtcacaaatatctttcagcttccatgggtgcgccggcttcatgttgacaatatttctcactttcccagaaacggatagcacaccgttagttaatagtgtaatgaaacctttgcatgcggcaaaaatagacaggcaagaaaaaagcaaaagttctgaaaaattatgatgattgcgttcttccgagttgagataagcaatcatttcattaagcaatccagtcggtacatttgaagcacgtaaaaacttcgcaggaacaggcaccgtcactgtctggatgttagtgcattgtagatattttttaatggtattttcagtaaatccgatctctttaaaatgccgctcataaggttcaaaatgcgtacgaacagcgttatctaccatcaggatctcgccgtcagagaaggcgtaatctttatctaaaatgttagcgttgaaggcatgatgaataaatataacagaacaaacgagcgacattttatctccttaaaacaataaagtttttatcgatacttttttaacatttcatatttataatttgctgtttgttttcagccttgcaaactattgataatgaaatgtgtaagatctcttgcaatgcgacccatttctgaaatactcagctgatcaattgccgaaaaaatggctatcaacgtaagtgtcagtaataagacaaccacaattgcagacatgatttctttatagttgtctctttgcgtgattttgtttttcactgtggtcgcatgcatttcaaatatgtttatttagcggataacgttaaaaatcgttaatcagtatgcttaatataacaggctggagaaaagaggaaataggactggtgcttcagtactgagcggagtttcttacagctgtaggcagaagtttatatcttatagtatgtagtttaatttaatccatgtgagcaaattgcgaaataatagtcaatgaggaattcttctgctgtgcggatgacagcagaagaaatgagaagaggcattaatttgatggttctaattcaaccggaatacttttatagccaggaatgccacttaatggatcgtggttatcaagtgttagcatgtgattcgattctggaaaataggtcaccagtgagcggtcagccatagggtaaatgaccacttttaatctatccatgcggcgtgagctgcgcttaccgtctggcgtaagcgcaataagattaactctttcgccgttttttacacggcaaattttagcttgtttagcactcataaagaccacatctcgttgaccgaatacccctcgatagcgatcatccataccataaatcgtcgtgttgtactgatcgtggctgcgtactgtcgccatgaccagcttactgttaaacgctgaagagggatcttctaacagccctttgctggtaatgaaattagccttacctgacggcgtcatccagcgcctttcagcagctgcatttatcaggtgaaaaccaccgggatgacggatgcgctggttatagtcggcgaactctggcagcacagcttcaatgtcattgcgaatgcgatcataatcttccaccagatactcccaggctaccacgctctggggtagtgctgcctgcgcgattcccgcgaccactgcacactctgatttcagcattacaccggcgggttttaacacgccacgcgaggcatgaatcatcgacattgaatcctcaacggttaccgcctgcgcaccgtttttttgcatgtcaatctcgctacgtcccaggaccggcagaatatagctatgccgtgcggtcaacagatgagagcggttaagcttagtggctacgtgtaccgccaaatctaattgcgttaacggtacagcgctcgcttcccgatctggcattgccagcgcaaaattgccccccatgcagatcaatgctcgagcctgccccgtacatattgcttgcatgctggcaattgcagcatgtccaggtgcatgaggtggggtgaagccatagcgctcacccagacgagccagaaactctgcagacggtttctcggtgataccgacggttcggtcgccctgtacattagagtgtccacgtagtgggcagatacccgcaccaggcttgccaatgttacctttcatcaacagcagattgaccagttgctgtacgttctgggtaccatgttcgtgctgagtgatccccattccgtaacagataatggtgcgttcggcagcggcatatgcgtcagccagttcggcgatttgtgtctgacttagtccagaaatacgttcgatatctttccactcggaattgagaacgtcacggcgtagctcgtcaaagccgacggtatgcgtttgaataaactcgtcatcaagcaatgaaggccgacctgcggcgcttgcagcatcatcgcgctcaattaacaggcgcatcatccccttgagcaacgccatatcgccaccaatgcgcacgttatagtaggcactggccaactgagtctcagagttcgtcagcatttcaaacgggttttgcggtgcggtaaatcgctccaggccacgttcctgtagaggattgatggcgatcattttcgctccccgtttcactaaagcgcgcaacgaagtcagcatgcgagggtggtttgtaccagggttatgcccaatgcaaatgactaaatcgcacttctcaaagtcttccagcaacacggtccctttacctacaccgatactcgctgccaaacccacgcttgtcggttcatggcacatgttggagcagtcgggaaagttattgctcccgtattcacgggcaaaaagctgataaagaaaggcagcttcattggaagtgcggcccgaagtatagaattcaacctgattgggatcactatagctttgaaggcgtgcgccaatttcgtcgaaagcttgttgccagcttaatggcttgtaacagtcgctgacggcatcatatttcaaaggctgagtgagtcgccccgcagcctcaagctcgtggtctccccaggtaagtaatgattgaaccgtattctcagcaaagaaagaggcgtttacctgcttatccgtgacttcccaggcgattgcttttgcgccgttttcacaaatgtcgaatgacgcactgtgcttaggatctggccatgcacaacccggacagtcaaagccctctggcttattcatgtcaaacatggcaataacatcctggcgtatatccatctgcttacgtactgcattcgctacggatttaacagcaccccaaccacctgcagcaccctggtaggattcaatttttttcttcatctacttatcctgtgtggaaatgaattattaggatttgtaatagcgatgatgcacagtacatacaaagggattatcgccaacatggatatataagagtaggggactactctctttctatttttaatctattatcgttaaacaatagattaaatacgataagttaagcatcatctctcatagtgtttaaattaacatatttttcaatataaaaaataagactctggcttcaattgtgcgcggattttcttacaggtgtaggctaatagccttcacaaaataattatccgcgcaattttcgtgaatggagcgcatagactaaggtcaaaatcacaattattcatagataaaagtgacaccaatgactgactggacggttccggctgaaaccttgtttcctgtttgtccataggttgcgcttaaacccagaggtactttgcttttatttactgtccccagggagacattttctcccgtagccagtatttttccattacgcattagagtgacacccactcccgatgcttttgttgcatcaggtgctgtgttagcaaacacttgtcggctactgtcagtggtggcacccgaaagataaaatgagagcttttgttcgcttgagcaatatacgccaaggggtatttctgcgcttccaggaaagtccgggagatccacggtgacatttcgactatcaacggtgcagccgcctgttggcataacaacattgttatttgaaataatattccacgtaaaattacgcggatttccgcttcctaatgttgcaattttatacatatgaatacgggcaatgacttcccccgcttttatgacaactccaccggccgccccaactggggtaatatagagttttaacggtaatggcatcggtgtcttatcaccaatatccaatacgttggtatttgtcgtcaacgggaaggggtaggtcacattattccagtacagcgatcctttatatgactgtagggagcctgcgaaagctgagccttgtaccaggtttatatgatcagtgtcgtaccagccgccgtaatcattccagcaacttatatgctgagacaagtctacaaccagattctggcccggctgtattacagggtcgagattaacataaacagaggttgtacctgctccaatacttgacccgccatcgacattacaactgaaggcaaaaactttgcctgccattaatagaagataaataccgaacaggacctttatactgattgttttacccatgatatatcctaaggttaaaaattgatttaaaaagaaggctaagaaaatcgaatcgacgttattgccaggtgtagatcacattgattagcgcctcgatcgttccctggcttgcgtttccattcaccgtgatagctcttgccttaagtggaaactgtgcattacgagtgatctcatcaacaataaccgttttgctatcgccattttttaacgcagcatcctggtcatccctcagctctatctgaatattttcggcagtaccttcatttttgtaataacccgtattgtcagttgaacctgtcacgattgccgtcactgcacttgtttcaaccggacaatcggttaatgacaaagtaatattgtgccagccagatgcagaaccaggttgttgcagattgcgcgtataaagatccccgagattaacgttagcttctttggtttgaatagtgcagggtttagcgactacccgaccattaacagtgatagtgacatcggcggcctggagagttgctgtgaataacgcgcaaaacgtagctaacaggaacctcttgtgaagtcttttcatatctgactctgattattgaaattcaagggtaaaggttgccgaagccctcaccagtcccggattgacggacttctgagttgacttcagacgagcggagtaaggcaaaatattgttctgttctggtaccagtgggatccactgcatcccggcatgaagatcattcagtttcaccggacgcatatttgcgtccaatatttctatacccaaaccggaggccgtattgcttccttcatccagtttcaacaaagtattattttctgcatcctcaataccgttaaatgcaacccgaacccccgttgtccctttgctgcattcacttaacgtaatctgaaaagggacggctggacttgtgctaccggtcgttggaaattgtctggcactgtttttttggagatctacggtaaaattaagcgaatccgatgagactgtgcagccataatcgaggacgcgcccgctaattttaataacgctatctgcggataaagcagaataggtggttaaccccagacataaaccgaggaaaataatgttattgtatttcataatctattgttccttagcgacagattgctgtctgctggttcagtaaggtaccaggagaaacttcaggaagcttgtactcgacaatacagtttgagtttttatctttgccccatgaaacctgtaattgccctgactgtggaagtccagtcagataaacctgaccattttccgcgacaatgctgccatttttattctctccgtgtgtgacaattgcaccgaatggaacgctcttattaccgtacttcaacgtcattaatactttcccgccgatttgtgcattaaatgttgctctggcaatagcaccgtgagttgggatgacagtgaccacggtttcatccagttcaacattatctgcaagggaattcgcgttaagagcaacacggttttctctatattctgtcgcaaatggtaatatggcatagccacgccagtcggtatgaattccggtctggttctctattttgacattatcagcaccaggagccttaaccagaaccattgtgtcgcccagcggctgtccaaaggtgatgccatcagcatgagcaataatcccaccactcattccgtaataaatctggctgctgtcaccactccgactgtaaccgacattagtattaccataagctccacgataattaagagaactgtaaccactggtgccagacgatgtattacctccgtgggtgttaccgacctgaacgctataattcaggttattatccggcagcagagtgccataaacccccgatagattggtcatgccgcctttcaaatcgtttgacatactgtaactggcgtttgaattacgaaatgccgactgactgtctgtacgcatccaatgactgaagggaacattaagcgtaaaagcgagtaaatgatcccgatcgttttgccatatattattggaatagctgtaattcagcgaagtcgtaatatcaccaaacggcacatttaatccaaatgatatttgctggtcgctgcgtgacgtgttccagtaactttggcgactggcactgaaaaatgtcgtaccgtaatttccaagctgctgagagatgcttatttgttcctgaccacgcttactgtagaacagattaaaataatcaataaattgtgtctgctcattggtgtctccggtaggaggcttgacggtgtaaccactcattcgactgtaggcactgtcggataagttataaaaaccttgcgtagaatagcgatatcctgcgacctggatattggttccacaacaagtttattgctgcacttgttgaagagagtatttgcaaaaacattttatgtcgctaaataacatgacgatttcattatgcatgttatttataaaccgtgactaaacagaatattattgcgaacaagggaagtgtcaggaaaggtcaagagctaccaatggttaatatggctataaatcattagctatggttaatgtttgcttgctgaaactaacaccgaattgctctaaacagataagtgcagggtttattaaagctgtccgacagactttcttaacctggtaatatctctcttgggtgactctccaaacatccgcgaatattcccgactgaaatgggatagctttcgtaaccgacagcataggctgctgtggtgacatcgtaatgttcattcagcatctgtcgcctgacttcattgagacgtagccatttctgataccggagtggactcattcccgcttgatccgtccttaaataagtaacagcaccctctggtgttttcgtatgcagtgtctatgcgacagacactgcgctcttagcatggggcagggaataaccaggctatttctccatgcacaggccaattatgaaagaggagaggcttaagttcttgaaccctgaacgaataacgactaccagaaaagcacttcgcatcactcagacatgatttaacataatatacattatgcgcaccaatataaaccaaggaagaatccagtcgttggcggtcatgattgtcatgctcattaacaatgaccaaaccccatatctcacttactaccgtattctcggcttaaccgtccatgcaacctcaacacattgctttcaactgccgtcaccacgttctccggaaaatctgtcggtaatgaagtcttcacgttatccagtgctgctggaatcattctggcaaagtcactcaggatttcatgcatctgcacttccgggaatctcagcacctttgctgtcgccaaaaaatgtcgcggataaattttatcgattgccgtttttttgcctttggatgcgttaagccccattgccagtttgagatcgctgatgtgtattcccgtaccgccaaggaccggaaatgctgaaatgatgtcgtaaaatggcgtgagtcgataactgccgccagcctgaataaatacggagaagttttttgcatgaccgtccgttgcgccaatcaaccactggaagacctggaatttcataaaatcatagcgatctttcagcgcctcgctggaccccatcaaaaaagccatgatccgcgcgatgcctgggcctccatctgattcatatttcaccgatgaaggtaaaccgaatgtctgacacatatcctcctgtggcaagcgaagtaaaaccgttcgctcagcattccaacgcctgtcaaaacgttcgaccgctaacgcgcgcacatttcccgctttaatgatttctgcgtccggaacattcaacccaagttctttcgccagcagcagacagtaatactcattatcaacgctttggctgagatcgagcgtcgcattgggctgcctgatttcgccaatcggtaatttaatgatgtgcgtcgtcggcgttattcctttcggaatgcaccagtcattgcctattctgagcagtgctgtcttctcctgtgcgccagcaaccgagatgcgaaagtcattttcttctctaatcatgcctagcgggatatctgctttataagccgttaatacttcttcaagtctggcttcagtaagcttttcccatgccattatcggatgcgttacggtttcgtcttcgggtattaacgtcacggcaccaacgctgtctcgccctatttctgacaataaatcaaacggttgtctggatttggcatgataacgtttaacgatccggtcacgtacaatcgggctatcgggtaacaggttatcgaagaagttaaatacggcatcagaggtgatattccccctctgcaatggcagcgaaagtgacaacggtctggcataacggcttgctaaccactccggtgcatacttaaaggtgtgcgcgccgttggctaacttcgttaactcgcctacccgctggttgttcatccaagtgacaagtttaggcattaccactccagattttgctgttctgttgattctggcgaggcatttttcgcgtcgcatagcgtcattgagagttcaagcgactgtaaaatcttaaaaaatgtcgtgagcgtggtattgtcagggttgttttcgaaattggaaatcgtcgcctgcttaataccaatttttttcgccagctcgctctgcgtccagccattttgctggcgaaccagtttcattgcattcgccaattgcgttgggctatagatcttctgaaagctcatcatgtcatacgtccacagcaagtttatccgcttaaggggatattataagttttatcctttagtgaggataagtcaatctggaaacacatcttatccgctctacgggataaacgctgcgatatccgcgatcgcggataaaaaggaggatttaaataaggcgttgatgcgccgtttgaagtcggcaatattaagccgcatgccatctcgacatgcggcttatacggtttaccagctatatttcactcccagcatgccctgagtatcgctatagcctttatcacctagttgcacaccgacattcccccacaggctaaggttgttatttactttcgcctcaaccccggtacgtacttcaccgagattacgcgcaccttcacggcctacggtttgaccattcatcttcacggcgtagactttgctattgttgatccagttcgcttcaatgtaaggctggaactcacgctgtttaccatcgtcacgctggtgatggctgttcaggtaggttttcaccccaagtcgcgtttgcacatttccgtcgccttccgtttcaatgcgcgttccgtctttccgggtatggtcggaatctttcacacccatccaggtgatttgcgcctgtggctggacgtaccaggtattcagcgtcccttcgctgccgctaaatgttcccgcttcaaaggtatacccaccctcaacagaggccgtcacaccgcgagaatcatagtcgtcagcagaacggttatcggaactgacgctgttatcaaaccagttatacagcgcccagctgtcaacataagcgccggtcttattcgcatcgttctgataccaggtcgcgtacagcccagcgctgtaaccgctgatgcgcccatccgatttataacccacacgattactctgagtattactgtgctgattggcgtagcctgccatcacgccaagatgccagcgatcctgcgcgttgctactccactgcgccaaatcgccgcctagctgcaatacatagcggttagcctgagtatttagctgaccgtcaccggcccttgaacgttcgtgccctccgacatgacgcatccacatactgcttgccgacccctgagaatgcagtgaatctgtatactgcggctcacccagacggtcgtgtaaacgatggctaaacagcgagttggctgcggcaatgttgctgatatagcttccggcctccgggcgataaactgatgggccttccggatccacaacagggggattattgatgggatcgggtgtatccgctggcgttacgccgtcccatttactggtcagataccagtttttctcgtcattccccttccctttagccagcgtgtagacgtaagccccagcttcgacagttccggtggtcagcgcgaagttacctgcagaattaccgccaacctcaatgagttcaataccgttgaccgtttgtgcaccgacgccgccaatgttatcaacccgaacgcgagtgttcccttgggtatcgcctttcacgttcatcttatcggtgggcgaattatcgccgcccagcgtcgcgttgaacgtcatcaggccattgtttccggtatagttgccgttaacggtcagtacattccccggtttccccccttcgctattcatttgaaccgtgccgccattctccaggttgccgccgatagtggttttagcgacacgcagtgccccccccaggcataacgttcatatcacctgcagtggtgacatttcccgacatcacaccgctgttatggatattaatgtgttgacttgccatattaatggcagagtcggaaccgaaagcaatttccccccccacgatatccgtcgtaccctgatacgccgcggaatcgttgttaagagtcaggatcccggtacccagttttgtcacatcaccgctaccgctgatactgtgcgtcatcgcccagctacgctcagtggagatggtgagcaggccattattgataacggaagcatcacccaggtttttctgctcgttgacgctgagcgcgctgcctgtatcaatgttgaattgccccacaaagcggctattatcgccatccaactctacatctgtcctggcggttgcgctcacgatacccttcccgcttatgctattacgcagttcgccagtcacgttttttagcgttaacagaccgtcattggcaatatttcctctgcctaacccctgagtattatcgaggctgacttccgcatttgggctaatgctggttaacgcattgtagcgtgcattaagcccctcgatagccagcgttccccctgtaacattcaggtttccgccacctgtcagttcaccctgactgatcccacctttatttaccgtcagcgccccctctttgaacaaaacagtcgaacccatctgcccggtgaatgtctctaccgtctgcgtcgatccattaagatcgacgatggccgcgttgctgatgttcagttcccgggtgttgccaagtgcaccatccgcatcggtacgtaatgtccccatctgaacgtaggttgccccctgatagtcgttctgaccgttggaaagcgaaacctgtcgcaccgtattgattgccagatccccttcaccaccgatttttgccgacatatcggccgttgcgccataggctccgccatgttcggctaacgtcagcttttgcccaccatggatgttcagcgctttcagcccatagttaacgtacaaaccattacctggtgcggtcgtgaggcggaatccataatcaccctcggcgaccaccgttccgttttgcgcaatgtgtaacgttttgtccgcttccacctcgtcgccctgtaaatcacgtaacgttaatgagccacccgacccaataaccgtttgcgccttcaccagttgaacgccgacatggctatcgtcgtgttccagcaaattgagcgtcgtcagagggttattcgccatgggatcattccacggtttaggcacgtcgataagcacgtcgcccgtcccgtttacctgatagttacggcctttccaggtgtagtcacccgcgccgacaaccagcgtatcgacgctgatatatccctccgcgagcgtcgcagcaggaatatccgtatcgaaaatgatggtacctccattcatggccagtccaccaatggattgctctccaacttttaccgatgtggtattttcactgtcagactgcaacatcgcgtgagtaagcgcagcggtgttgtcgcgttccagagtgaaggtactgtctttcagttgggcaacaccggcgaattcagtccctgttgcatgggtaaagccaaacatcttgtcggaggatgacagctgcactcgcatcaagccatcgcctttgagcgcattggtcagcgtgtaatctcctgcactgttcgttgatgcgagaatgtcgagcgtaccggggtttgcaatggttacttcactcgaccccatgcccgttaccccatctgccgtatgagacgcaatggtcaggaggccgtcattgaccagcgttttaccgctataagtattccctgcattgaacaccgtatggcctgcatcatggatcacttttccgtctttatcgtcacctgtaatcagcatatcgacctggtagccggcatcactgttattggtatgattaaagacaaaaacgccttcgccaagaccaaactccactttcgtcgcattggtgataaatccggcatctgccgccgcctcaccgtgagcagcaccaatgtttagcgttcctacagcaggctcaaaaacacctaagtaaacttctccaccttcgacattcagcgtaccgttattcgtcagggttaacgtacccgtaccagatgtccctacgtacatattgaatgtttcaagaagagagttctgcccatccaccctcacgtcgcccttacttttgtcattgagagctatctgtgtatcacgcgctttaactatacctccggtggtaatattcagttcacccgtgcctaatacaccgacctgtagcaattgtgcgttagtagatgatgtctttaaattccagagactgtccgttgaaatattaactatccccttaccggaggcatttcctccgataaatccatagcccgttgaattaagggtggcaccattactgacatttacgataccgctaccaaaattaccgacattgatacccacagtatcgaacgatgatgtcgcatccatcaggttcagtgtgccgataccgcttgctttatcgcccaaaaaagtaatattttgcgatacgaacttaccgccatcgctaatattgaggtttccgacgcccgcaacaccaatggtggtatagacattcttattgacctcccacattccccccgtggtgatgctgacattcccgacgccggtttctccataaccgagtgaacttcctccgttgctgacaacaagcccctgattactgatattcatttcgccgtggccgtcataaccaagattagttccgagattagtgataacggagttcttatccttaacagtaatgttgcctgtgcctgtttctttcatccccgcagtgataattcccgaatctactttgccttcactcgagacattaagttcaccgtcgccagcatcaccgatatagatatagcggaaagcttcgcccgttccgaggaaattccaatgccctttatcggtcacgttgacgacaccgtgggaaccgtcctgaacgcccaccaatgaatattctttgttattaatcagtccattattggaaatattgactgtgccattaccgaaatatccattatagagtctgcgtaccgtgatgacagagtcttgatcctgcacattcagggttccgataccggtggcattgccaccgataatcgtattttcagccgtaaccaaccccccctcgcgaatagtcgcctccccagttccttgattaccaatttgaaattcaattgaggaatcattattttttattagccactcgccacccttttcaacgacaacctggccattactgcccgcctgatagcctaaaatggcgacgattgaactcgtgacgtaacccttatccgtaatatttaatgaacctgtgccatagctacctatttcgaataattcggtcgtcagaacagagtcctctccctcaacattgaccgtcccgacgcctcctgtcgaagaacctaatcttaaatagcctccatcgacgtgacccttctgtttaatattcagcgtccccgttccggattgacccacatttaaaggccttgcattatttccgctatcatacaatcgccaggtgccacccaaaacattaacggtgccctctgagtcctcattagcgccaatgacgctggtagtaatagtggttaaggaggcattaccgccagccaaaatattaagcactccagtgccataccagccaaccaggtaggcatcataagcaacatcagtatcaatattggtaatctgatcattatcaacttccagacttgcaccagacgctgaaccgcttagtgccagcaaaacacccagcgtcaatctactgaatttcgttgtcagtccagaggatttacgcaaattaaccgtcgatgttttacctgccctgcgagttaattccgagcaggcctgaaatacctgtagagtgcaattccatatcacgcgatagattctattcatataaacgctccatatacaaacaatacagccacgaaagagatgagtcgtcagacattaaaaatgaaacttattaaattgtcagaggtctgtattgagtgttagttggaggtgggaaggtgtcaatttggctaatttgctaatgctttcgaattgatagattaaaaattgcatagttcttattttatttaaatatgaactatgagttattgttgcttaataagaaaactgtttctttcaataggaaaattatcatcatcatatttaacaaagaatagcactaattgctaaaaatcgaagtttattaaaccccttttgcatccattagtgtctttaggaatattcgctataaaataagggttgtgcttaatgctttaagaaaaatagcaattttcccttgaatatcgtactggtgatggaacgatgaatctgcaagctggcttttaacaagccagctctaaaagaagggaaataagaataactatactcaaaaactaacagccacggtcatcatgatgtggctgtcaatgaaactataacccaggcgctttccataacgacgtcgtcagtccatgatcaaccagccccagctgatcctgataaactgcctgccacttatcgcgtgaatcctgataaagttcatgcttttccgggtctggtgtgtgcgtccgttcccagcgaaccaggcgttctccggtttctgccattgatgaaaaaattccggcaccgacgccagctgcaatggcacatcctaatgcagtggcttctttgaccaccggaatattgacgggtaatcccgagacatcagcgagaatttgactccataatttcccttttgaacctccgcctgcaaagactaacgatgaaggatgaatattcgagaaatcagcaatttgctgcaagttacacgctgatacaatcgccgcattttcttccagcgcacggaacaatgtcgctttgttacatttatccgggtcaatggacaagttaataaaggaaggcgcagcgtgataccaggttttaaagcgcattctgtcggagaagatcggcattacgccccacgacccaggcggcacccgactggccatctcttccagcagcgtataggtgtcgatgcctaaacgttcggcaatcagtttttcttcggcacagaaagcatcgcggaaccagcgcatggtgagtccggtaaaaaagcttatagattcagcttgtaccatgccaggaataacatgaggattaacgcgcacgttcatttctgggtctgtcaccggcgcggctaaatttacaacttgctgccagaatgtgccgccaagaaccgcggtttgtgccggacgcacaacgcctaacccaaggcaaccaagctgcacgtcgcctcctccaacgaccaccggagtgcccgccttcagaccgcagagttccgccgcttgtgaacttaccacgcccagcaatgtgccggtttctttgacaggagaaagaatatcggcacgtaggccagccatatccagcaatgcaggtttccagtcacgggtggttagatcaagaagtcccgtggtgccagcgttagagggatccaccgccagttcgccgctgagcatataggccagccagtcgctgatcatggtgatggttgatgcctgacggtaaatatcggaacgatggtgcgccagccaaagtaatctggggatggcacttaaagccagtgtttgtccggtcgcgcgataaacttcgttttcaaaggtattgttgtgcagttctttaagttcgctaacttcgcgtgccgctctggcatccacattggcgcaggcccagatcggggctccttcattattatataaaacaatgccttcacgcatcgaacatgccgaaacggcagcgatatactccggggctatgccggcgttgtgcagcgcctggcgcatacactcacacgccagttgccagtttttgttgagatcaaattccatagaaccaggaacgtccggtactgccagatgccgccactccgcctgtcccactgctatttgattgccttccaggtcgaatatcacagcccgaatacttccggtgcctgcatccagcgccatcaggtagtactttgattctgaaagggtaaagagtcgagccattagattatcctcggcttatgcgttctgtctgttcctctatacgttctccatcattcccggtaataaggtcatgcaaatttaactacgtaaaatcgccgctgctgtgtcctgatcggtaaccagtgcgttgatataaccgcctttcattgcagcggcaattgcttcggctttattttctccccctgccacgccaacccggacgggtatggtcttcagcgcgcttaaaggtaagccaatcagttcgttatgtattttgatattcgtgacaacgtcaccttttgcatcaaaaaagtagcctaaaatgtcgccaaccgccccttttcggccaatcattaactgttcgccctggctgatataaccggagcgaatgattgtcgcatcgtcctgttgactcacagcaccaatgccgacaatcgccacatccgctgcttgcgcggctaacagaacatctttgacgcaattttcattttttagcgtacgggcaatgtcagcggaggatgcccgcaacggagccggaataatattcacactgcacgccgcgttaagctgcccgattcccgtcatataagaaccgacgccaccggagagcgtgaccaggcgaatttgctgtgacgaaataaaaccacttaagcgttgcagcgtattcatggttgcctcgccaaaaccaatcgccagcatctgttgtggttgaagtaaactcatcaacatatgcgccgcgcctatccccagtcgcccaccgacatcagcatccgcaagcccagggatcacccggacatgttgcagcgaaaactgacgacgtaattgagtttcatattccagacagccttcaaagcgagaattaatctgtacgcgaataatgccggactgatgccctttctccagcaatcgcgacactttcaaacgtgtcaggccgagacgatcgctgatctcgctctgggtcagcccgtcgtgatagtaaaaccacgcgatccgcgcgacctgttcttcttcacacattccctgttctgaaattgccgaatcgttgattgtcataattcattcttcactttgaacatatttaaatctttaatgcaattgttcagttcttgctcatttatatctgtgatggcaaccacagtttgactctacgagcatgaacaaacgcaaccgtgaaaatcaaaatagcataaattgtgatctattcgtcggaaatatgtgcaatgtccacctaaggttatgaacaaattaaaagcagaaatacatttgttcaaaactcacctgcaaaactgaacgggggaaatatgcaaacgagtgatacccgcgcgttaccgctactttgcgcccgctcggtttataaacagtattcaggggtcaatgtcctgaaaggcatcgattttacgttgcatcagggggaggtccacgccctgctcggcggcaatggtgccggtaaatcgacgttaatgaagattattgccggtattacccctgctgatagcggtacgctggagattgagggcaacaactacgtcagattaacgccagttcatgctcatcagctgggtatttatctcgttccccaggaaccgctgcttttcccaagcctgtcgataaaagaaaacatcctgtttgggctggcaaaaaaacagctctccatgcagaaaatgaagaacttgctggcggcgctgggctgccagtttgatctgcatagtctggcaggatcgctggatgtcgccgatcgccaaatggtggaaatcctccgcgggctgatgcgcgactcgcggattctgatcctcgatgaacctaccgcctcgcttacccctgcggaaaccgaacgcttgtttagtcgcttgcaagagctgcttgctactggcgtgggtattgtttttatctcgcataagctgccggaaattcgccagattgccgatcgaattagcgtgatgcgcgacggaaccatcgccttaagcggcaaaaccagcgaactgtctaccgacgacattattcaggccatcaccccagcggtacgggaaaaatcgctctctgccagccaaaaattatggctggagttacctggtaaccgcccacaacatgccgccggaacgccggtgctgacactggaaaatctgaccggcgaaggtttcaggaatgtcagcctgacgctcaatgccggagaaattctgggcctggctgggctggtgggggccggacgcacagaactggccgagacgctctatggtctgcgtactttgcgtggcggacgcattatgctgaatggtaaagagatcaataaattatccactggagaacgtttactgcgcggtctggtttatctgccggaagatcgccagtcatccggactgaatctcgatgcttcgctggcctggaacgtctgcgcccttactcataaccttcgtggattctgggcgaaaaccgcgaaagataatgccaccctggaacgttatcgtcgggcgctgaatattaaattcaaccaaccggaacaagctgcacggacattatccggtggcaaccagcaaaaaatcctcattgccaaatgcttggaagcttcgccgcaagtattgattgtcgatgagccgacgcgcggcgtggatgtctcggcccgtaatgatatctaccagctgttgcgcagcatcgccgcacaaaatgtggctgtgctgcttatctcctccgacctggaagagatcgaactgatggcagatcgtgtgtatgtgatgcatcagggcgaaattacccactctgcactgaccgagcgcgatattaatgtcgagactattatgcgcgttgccttcggcgatagtcagcgtcaggaggcgtcatgctgaagtttattcagaacaaccgtgaaatcacggcactgctggcggtggtgctgctgtttgtattacccggttttctcgaccgccagtatttaagtgtgcaaacgctgaccatggtttatagcagcgcgcaaatcctgatcctgctggcaatgggcgcgacgctggtaatgcttacgcgcaatattgatgtttcagtgggttcgattaccggaatgtgcgcggtgctgttggggatgttactgaacgcaggatattcactacctgttgcttgtgtcgcgactttactgcttggtttgctcgcgggatttttcaacggtgtcctggtcgcgtggctaaagatccctgccattgttgccacccttggcacgttagggttgtacagaggcatcatgttgctgtggactggcggcaaatggattgaagggttacccgccgaactgaaacagctctccgccccgctgctgcttggcgtttcagcaattggttggttgacgataattctggtggcatttatggcctggctgctggcaaagacggcgtttggacgcagtttttatgccacgggcgataatttacagggcgctcgtcaactgggcgttcgtactgaagccattcgcattgtggcattttcgttgaacggctgcatggcggcactggcgggaattgtgtttgcttcgcagattggttttatccccaaccagaccggtaccgggctggagatgaaagcaattgcagcctgcgtgctgggcggcattagtttgctcggtggttccggtgcgatcattggtgcggtactcggcgcatggttcctgacgcagatcgatagcgtactggtgctgttgcgcattccggcatggtggaatgattttatcgcgggtctggttctgctggcggtgctggtgtttgatggacgcctgcgttgtgcgctggaacgtaatctacggcggcaaaaatatgcccgctttatgacgccaccgccatccgttaaacccgcttcgtcaggtaaaaaacgggaggccgcataatgcgtattcgctacggttgggaactggctcttgccgcactgctcgttattgagattgtcgcatttggtgcaattaacccgcgaatgttagatctcaatatgttgctgttcagcaccagtgactttatctgcattggcattgtcgccctaccgctaacgatggtgattgtcagtggcgggatcgatatttcgtttggttcgaccatcggcctctgcgccattgcattgggcgtactgtttcaaagtggtgtgccgatgccgctggcgatactcctgaccttactgctcggcgcattgtgcgggctgatcaacgccggattaattatctataccaaagttaacccgctggtgattacgcttggcacgctgtatctgtttgccggaagcgctctgctgctttccggtatggccggagcgacggggtacgaaggtattggtggattcccgatggcgtttacagatttcgctaacctggatgtgctgggactccccgttccgctgattatcttcctgatatgtctcctcgttttctggctctggctgcataaaacccatgccggacgtaatgtgtttttgattgggcaaagcccgcgcgtggcgctttatagcgcgattccagttaaccgtaccttatgtgcgctctatgccatgacggggctggcgtctgcggtcgccgctgtgctgctggtatcgtattttggttcagcacgttccgatctcggtgcgtcgtttctgatgcccgccatcaccgccgtggtgcttggcggggccaatatttatggtggttccggttccattatcggcaccgccattgcggttttattagtgggatatttgcaacaaggtttgcaaatggcaggagtgccaaatcaggtgtccagcgccctttccggtgcgctacttatcgtcgttgtcgtaggtcgttccgttagcctgcatcgccagcaaattaaagagtggctggcgcgtcgggccaataacccattgccataaaggatatcttcatgacacttcatcgctttaagaaaatcgccttacttagcgctcttggcattgccgcaatctctatgaatgtgcaggccgcagagcgtattgcatttattcccaaactggttggcgtgggattttttaccagcggtggcaacggcgcacaacaagcgggtaaagagctgggcgttgatgtgacctacgacgggccgacagaacccagtgtttctggtcaggtacagttgattaataacttcgtcaatcaaggttataacgccattatcgtttctgcggtttcgcctgatggcttgtgtccggcactgaaacgcgccatgcaacgtggtgtgagagtgctgacctgggactctgatactaaaccggagtgccgctcttactacattaatcagggaacgcccgcccagttaggaggtatgttggtggatatggcggcgcgtcaggtgaataaagacaaagccaaagtcgcgtttttctactcaagccccaccgttacggaccaaaaccagtgggtgaaagaagcgaaagcgaaaatcgccaaagagcatccaggctgggaaattgtcactacgcagtttggctataacgatgccactaaatcgttacaaaccgcagaaggaatattaaaagcgtatagcgatctcgacgccattatcgcccccgatgccaacgccctgcccgctgccgcacaagccgcagaaaacttgaaaaatgacaaagtagcgattgtcggattcagtacgccaaatgtgatgcgcccgtatgtagagcgcggcacggtgaaagaatttggcctgtgggatgtggttcagcaaggcaaaatttcagtgtatgtcgcggatgcattattgaaaaaaggatcaatgaaaacgggcgacaagctggatatcaagggcgtaggtcaggttgaagtctcgccaaacagcgttcagggctatgactacgaagcggatggtaatggcatcgtactgttaccggagcgcgtgatattcaacaaagagaatatcggcaaatacgatttctgatgtgcattacttaaccggagtaagttatggcagatttagacgatattaaagatggtaaagattttcgtaccgatcaaccgcaaaaaaatatcccttttaccctgaaaggttgcggtgcgctggattggggaatgcagtcacgcttatcgcggatatttaatccgaaaacgggtaaaaccgtgatgctggcttttgaccatggttattttcagggaccgactaccggacttgaacgcattgatataaatatcgccccgctgtttgaacatgccgatgtattaatgtgtacgcgcggcattttgcgcagcgtagttccccctgcgaccaataggccggtggtactgcgggcgtcaggtgcgaactctattctggcggaattaagtaatgaagccgtggcgttatcgatggatgacgccgtgcgcctgaacagttgcgcggtggcggcgcaggtttatatcggcagcgaatatgaacatcagtcgatcaaaaatattattcagctggttgatgccggaatgaaagtgggaatgccgaccatggccgtgactggcgtgggcaaagatatggtgcgcgatcagcgttatttctcgctcgcgactcgaatcgccgctgaaatgggggcgcaaattatcaaaacctattatgtcgaaaaaggttttgaacggattgttgccggatgtccggtacccattgttattgctggcggtaaaaaattaccggagcgcgaggcgctggaaatgtgctggcaggctatcgatcagggcgcttctggtgtggatatggggcgtaatattttccagtctgaccatccggtggcgatgatgaaagccgtacaggcggtggttcaccataacgaaacggctgatcgggcatatgaactctatctgagtgaaaaacagtaactgcggatctaaggagaagaattatgcacgtcacactggttgaaattaacgttcatgaagacaaggttgacgagtttatcgaagtttttcgccagaaccacctgggctctgtacaggaagaaggcaatttgcgcttcgatgtcttacaggacccggaagtgaattcgcgcttttatatctacgaagcctataaagatgaagacgcagtggcgttccataaaaccacgccccactacaaaacctgtgtcgcgaaactggaatctttaatgaccgggccgcgtaaaaaacgtctgttcaatggtttgatgccgtgaggcgaatttatcaattttatctacaattggggtaacgcgctgacgggagtaaaaaaatgtctgactggaacccctctttatatctacacttttccgctgaacgatcgcgtccggcggtggagctgcttgccagagtgccgctggaaaatgtcgaatatgttgccgatcttggctgtggcccaggtaacagcaccgcccttctacaacaacgttggcctgcggccaggataacaggcatcgactcgtctccggcgatgattgctgaagcgcgcagtgctttgccagactgccagttcgtggaagcagacatccgcaactggcaaccggtacaggcactcgatctgatttttgctaatgcctcactgcaatggctgcccgaccactacgaattgtttcctcatctggtttctttacttaatccgcagggcgtgctggcagtacagatgccagataactggctggagccgacccatgtgctcatgcgcgaagttgcctgggaacaaaactacccggatcgcgggcgtgagccgttggctggcgttcatgcttactacgatattttgagcgaagccggatgtgaggtcgatatctggcgaaccacctactatcaccagatgccgtcacaccaggcgattatcgattgggtgactgccactggattacgtccgtggttacaggatctgaccgagagcgaacagcagctttttcttaagcgctaccatcagatgctggaagagcagtatccactgcaagagaacggacagatactgctggcatttccgcgtctgtttattgttgcccggcgtatggagtaaatatcacgtcagctggtaatgacgatcgggaagaatttttgctggaatttcggcttcatcgttcatctgtaacaggtcaatttcaatagcgttgcagatggcatccagtggtaaatcattgttttcagtaccgaacggatcttccagttcttccgccagacaatccagcgaaataaaagtgtaggaaatcagcacagagataaaaggcgtcatgtaatgcaggtccacgaccagcgcgaacggcagcatgatacaaaacagataaacggtacgatgcaaaatcagggtgtaggcaaagggaattggcgtataggcaatgcgctcgcatcctgccaggaccgctgaaatatcattaagccgatcgttgaggctaataaacaggatatctgaaagctgtccattgcggcgctgaaccgccaaccattctcccattattaacaagatacggttagctggagagttcgaagccagtacacgctgaagatcttcagtcttgagataatgagccagcacttccgcctgtggctgtttgcgtaatgtcatgcgtaaacagtgggcgaaagcgatttgcagccgggcaaactcccttacacttgccgaatccggcaatgtcgtttttacctcgcgcagtaacgaccgtgaggcaatcatcaactgcccccaaagttttcgcgcttcaacgtaacgggcgtacccggcattattacgaaaaccaagaaaaatggcgatggcgacaccgagaatgctgaacggtgcgagggtgaatttgatgcccagatgcgtgtaccagggcagcatgaaaataacagcgatagaaaagagaaaattgagtagtaagcgcgaggatatcttggataatactgagccgtgccagacaaaaatacggcgcagccagtgttgttgtggacgaacaatcatggttatcttcaggcgtggaaaagtcgccctattaaacgtgattacgatcacattctcaagacgctacttacaaattacctacaagcttacaacattagcaggcgctgcatgtggcacctgttaatgataaaggcatataggatgttgtaactaatatggtgaaataagaaacccggtcgaaaccgggttcagaagtaacggtgttattagcacaacggacgtacagcttcgcgcatccctttttcgagaatcgcatccaggtcattagcaacctgctcgaccagaccaggcacttgcgtcaggtcctgctcccagtggtctttttctgccaaaacaatcgctaccagttcctgggtgccgataacacggtcacgatgctggctccagagttgctgataacgttccagccagtgtgcatcgtcctgtaccggatatgtttcgccgttacgctcaccacgatagaacgcaatcaatgccgctaatgcgaaagtaaggcgcgccggaagtgtgccgtttgccttctgccctgccagcagctgtggcaggatgcgggtgcggaacttggtcataccgttgagcgcgatagacagcagctgatgcttaatgtacgggttacggaaacgcccggtgactgcactggcgaaagattccagttcatcacgaggcaaatccagtaccggaataatttcttcgtagatagctttttcaacgaatgcgcaaatttcagcatcgttcatcgcttcacctacggtatccagccctgcctggaacgccaccggcaccagcgcggtgtgcgcaccgttgaggattgccactttgcgttctttgtacggtttaatatcgtcaacaatcagcacgttgagcggatatttgtccagacgcagttcagtcgctaaggatttcggtccctgaatcacaaacaggtaaaagtgttcagcggtgtcgagaaaaccatcgtgataacccagttcttcttccagtttagccacttcatcgcgcggataaccggtaacgatacggtccaccagcgtagaacagaagctgttagcctgatccagccattgaataaatgcttctggcagtgcccactcttgcgcatagcgcagcaccagttcacgcaacgcgtcgccattgtagtcaatcaactcacacggaatgatgatccaacctttatccagcgcaccgttgaaatggctaaagcgttcgaacagcagacgggtcagttttgccggatagcttaccgctggcgcgtcatcgaatttatcgcccgcatggtagctgatacccgcttcggtggtgttagagaaaacaaagcgcatttccgggttgtgcgccagtttcaggaattcatcgtattcactgtagacgctgatttcacgattaaccgagcgaatcagacgcgcgtcgctgaccgcttcccccttctcattcaggccacggataatggtggtgtacagaccatcctgcgtgctcagtgacggcgggaatgaagtttcaatcggacgaacaacgaccacgccagaattcagatcggtgtgctcattcaggagatcgatttgccagtcaacaaaggcgcgcaggaagttaccttcaccaaactgaatgatacgttctggatactgtgcaccgggaaaatcgcgacgatttagtgttttcacaatgggttcccttctgattagtcatacaacctgtttgaattggtacgacaggttagcaaactttaatacgccgaacccctgttttgatcaactcctgatgattaatgagcagttttatgagaaaagtgtggcgcggatcatggtttaatcgaggaaaaacgccttttcctggatcataaagtggtagaacacattgcattcaaatcgcgcgtaatgaataaagatgtcagacaacttcctcaccgtaacgcatagtgctggtacggttgcgcccatctttcttcgagcgatacagacacgtatcggcttcgaccatcaatttattaaagtcatcggtcagcgttaggtacgatgcgcgaccactaccgacgccaatacttaccgtgagataaagcgttttttgttgccaggtgaatggttgcagttcaacgcctttacggattttttccgccattagcagaccatcgacaggattcaccgacggcactgcaacagcaaattcttcgccgcccattcgcgccaccagccccttatcaccgacaatcttctgaatatgccgggcaaacacgcttaacactttatcgccacattcatgtccatagttatcgttaatgcttttgaaatagtcgatatcaagcagcatgacagtcagatgttgtgtctgtttcagcgatggacttttcagcgcctcataaagaccggaccgtgagtaaacctgagtcagaaaatcaaagtcggctcgcagcgcaacttgcttcattagcgaattgatcgctgccacgctaaaagaaaccataattgggcatatcgccatcgtggcaataccgagacgtgcggagaacatttgcggaatggagaacggcgaaccgaccgagatatcaatcaccgaatttgccaccagtacgatttccaccgcaccggtgacaaaggtcaacagacatgttacctgcggcgtatagcgcactgcacaccagattaatgcaggcagcgggaacgccagactccccgctccgccaatgactaccgaggcaataaccgacacaataagcgcgatggcgggcatcatctgttctgctttaaagcgcggcagcactccaggaatagccaacgtcagcatacaaggcacgatcaacacgcccgttgagaattgctcactgaaccagtccgcaagcaaaggccagaaatccagactatcaatactgaccgaaccaagatagcatgttcgctgacagcggcggcaaataaaggtaccctgggaatgctattttgtcgttttccgcaattctcatggctgattcatctgtacaaccagccagtgatagattaccgccacgatataacgttgttgttcttcgcttaacgaaacaccctgcggaatgttatgccacttagccagacaaccgcgacagcaggtcgcggtggcgtgctgagcgataaacaccggatgcccgcgcatgggggtttgcttaccgtcattagccggtaatgccggagcaagacgtttagcgacaaaatccgccgcatgttgttcgatgactggcgcgcctttctccaggcaatactgacgctctttcatgcccagacgaaagcgagagcgaaattttgaacgggataaacgcgcgaagagtggatcgagagactgcattaataaaccgaacgccctaactgtttcgtcaattgttcaagaacggcaatacccgcaagcgagttacctgcatcatccagttccggactccagacagcgatggccatttcatgcggaacaatcgccacaataccgccaccaacgccagatttcgccggtagccccacccgccaggcaaactcccccgcgttctggtacataccactggtcgccatcagcgcgttaatttgccgcgcctgcattggcgtcaccactggttcatcaatatgaatagctttcccctgattagccagaaagacaaacgtccgggccagctctacacagctcattttcagagcgcagtaatgaaagtagttttgcagaacggttgtcacgtcatgatggaaattgccaaacgacttcatcagccaggcgatagccgcatttcgcgcggaatgttcaaattcggaacgcgctaccaccgtatcgtaggaaatatcagacacaccgcttaagccgcgcacgacttccagcatacgttgccgtggtgcgcttaatcgcccttgcaacatatcgcagaccaccagcgcaccggcattaatgaacggattacgcggtataccctgctccatttccagttgcactaaggaattgaacggtgatccagacggatctttgccgacgcgttgccagatttcctcttcggagtaatgacgcatggcgacaacgagactcagcactttggaaatagactgaatggaaaaacgttcttgcgcgtctccggcctgaaaaagctgtccgtcaacggtacagatagcaatccccaatcgggaaccgtctactgtagccagcgccggaatataatccgcgactttaccctgaccaatgagcggccgcacttgccgcaagatgttttctaaaattgcattatccatggcgactgccactttctactcctggaccgcaggtctgaaaagacctgcgagtatatcagagctgaatatgtcgcgtcagatccggtctttccacaccgtctggatattacagaattcgtgtaagccgaaatgggaaagctcacgaccaaagccactctttttcacgccaccaaaggccactcgcgcgtcgctggcacaataaccattgataaacaccccaccgcattccagacgtgccgccatctgtctggcctgtgtttcgtcagtggtaaaaatggtcgctgaaaggccgaactcactatcattagccagttccagtgcatgttctgcatctttcgcaatggtgattgccgcaacggggccaaacatttcttcccgaaacgcggtcatttctggggtaacattcgccagaaccgttggcggatagtagttacctgccccagccatcttttccccgcccagtaacaaacgcgcaccctgcgccagggttttctccacctgatgatgcagctcatcacgtaaatcaaaacgagccattggtccgagagcgttctcttcgtcacggggatcgcccattttcaaggctgccgcagctgccacaaaacgttcggtaaatgccgaagcaattccctcttcgataataaagcgttttgccgctgcacatacctgtccggtattctgataacgtccggctaccgccgctttcaccgccagttccagatcggcatcgttaagcacaataaacggatccgaaccgcccagttccagtacgcattttttcagtgccgctccagcctgtgcgccaatagccgctcccgcacgaacacttccggtcaccgtgacagcagcaatgcgcgagtctttaatcatctgactgacaccgtcgttgtcggcattcagccagccatatacgccttgtgggatacccgcatctttaaacacctgggcaatgagctgtgcacagcccatcacattcggcgcatgtttaagtaagtagccgttacctgcaagaatgatgggaacagcgccacgcatcacctgccataacggaaaattccacggcataatcgccagaatcgtccccaacggtcgatactcaataaccgcctgctgattttccaccagcgtaggttccgccttcagcattgccggaccatgttctgcataccagtcacacaaattcgccgatttcgccacttcagcgcgcgcctggttgattggtttgcccatttcgcgggtgatcatttgcgccatttcttcgctacgagcgcgcagagccttaccgatatcacgcagtttttcagcacgataatctatatttgtctcgcgccagtcgcgaaagcctgctgccgccagctgaagtgcgttttcgatatcgtcagcgccagcccacggcagcacagaaagttgttcacccgtggcaggatttatcgaaattgcatgagttgccggagtaatggtcatcggggtatctcctttatgagtcatggtatgaagatacgcagatttactcttgctttaaaatgaataatattaagccacttattcacgaatcgagaatgctatggatctgacccaactggagatgttcaacgcggttgccgaagctggcagcataacccaggctgcagcaaaagtgcatcgcgtgccgtcgaatctcactacccgtctgcgccagctggaaacagaactgggggttgatctgtttattcgcgagaatcagcgtttacgtctctctcctgccgggcataactttttacgctatagccaacaaattctcgcgttagtggatgaagcgcggagcgttgtcgctggcgatgagccgcaaggtttattttctcttggttcgctggaaagcaccgctgcagtgcgcattccagccacgctggcggaattcaaccgtcgttatcccaaaattcagttttcactttccaccggcccttccggcactatgctggatggtgtactggagggaaaactgaatgcggcgtttattgatggacccattaaccatactgccatcgacgggataccggtataccgcgaggaactgatgatcgtcacgccacaaggatatgcgccagtaacccgtgccagtcaggttaatggcagtaacatttatgccttccgcgccaattgttcgtatcgtcgccacttcgagagctggtttcatgctgacggtgccgctccgggaactatccatgagatggagtcttatcacggaatgttggcctgtgtgatcgcaggagcaggcattgcgcttattccgcgctctatgctggaaagtatgccggggcatcaccaggttgaagcgtggccgttagctgagcaatggcgttggttaacaacctggctggtctggcgtcgtggtgcgaaaacacgtccgctcgaggcatttattcaactgctggatgtgcctgactcggcaagacagggatatcaatgagctatttttgatagttcttgcggttaatatgctctatatagtgatgttccgatgacttatgactatatggggcaaatatggttacgccagtaagcatcagcaattacatatctcttcctgatgattttcccgtacgtaatattgcaccgcaggtaaaagaagttttaaaggattttattgatgcacttagtacaataatatgtaatgaagagtggcgcacgtctttaaacatcaactcagccacaaaaaagatatttaataaccttgacaacttatcatatattcagaggacttcttttcggggtaacgacacgctatacaatgaaaaggttcagtttaaactcacttatcccgccaggaatggaagacacaaagaaaatattgaatttcaggtagtaataaatttaagccctatttatttagataattttcgccatgatggagaaattaatattttttgcgctcccaacccaaagcctgtcactatggggcgcgtatttcagaccggcgtcgagcgtgtactctttctgtttctgaatgattttattgaacaatttccaatgatcaaccctggtgttcccatcaaaagagcgcatacaccacatattgaacccctgccttcggatcaccataccgctgcagattacttacgccagtttgatttgcttgtcctgaattttatctctcgcggtaattttgtcatactcccccgattatggaataactctgaggttcacagatggttcgtcaataaagatcctaacttgatcaccgccattctcgacataacggacagcgaattaaaagaggatttgttgcaaagcctgatggattcattaggttctaacaaacatgtactacccgaagtctgcatctgctttttatcccttttagcagaacaagaatctcctcattttcagaacttgtttttatttttcgccaatatgttattgcactatcaccaatttatgaatcccaatgaaagtgatttgaatgacgtgttgatgccagcatcattaagtgatgataaaattatcaaacatatggcgcgcaggaccctcaaactgtttgtaaaaaatgaaacaccgccaaaagttactcacgaagacctggtgaaaaacaggcctcgctcccctgtcagaccacctatacccgcaaccgccaaaacgccagacctccctgaacgtcattaaaccgtgatgttaccgactctctgacgcgtgaaagaatcagcgtcagagaaacggaaaacgcgatccagatcacaaatgcattgtattcacatcattaaccgttttaagatcatttcatcactttttcgcaactcacccgataatctgttatgacaacaaacactgtttcccgcaaagtggcgtggctacgggtcgttacgctggcagtcgccgccttcatcttcaacaccaccgaatttgtccctgttggcctgctctctgacattgcgcaaagttttcacatgcaaaccgctcaggtcggcatcatgttgaccatttacgcatgggtagtagcgctaatgtcattgccttttatgttaatgaccagtcaggttgaacggcgcaaattactgatctgcctgtttgtggtgtttattgccagccacgtactgtcgtttttgtcgtggagctttaccgttctggtgatcagtcgcattggtgtggcttttgcacatgcgattttctggtcgattacggcgtctctggcgatccgtatggctccggccgggaagcgagcacaggcattgagtttaattgccaccggtacagcactggcgatggtcttaggtttacctctcgggcgcattgtgggccagtatttcggttggcgaatgaccttcttcgcgattggtattggggcgcttatcacccttttgtgcctgattaagttacttcccttactgcccagtgagcattccggttcactgaaaagcctcccgctattgttccgccgcccggcattgatgagcatttatttgttaactgtggtggttgtcaccgcccattacacggcatacagctatatcgagccttttgtacaaaacattgcgggattcagcgccaactttgccacggcattactgttattactcggtggtgcgggcattattggcagcgtgattttcggtaaactgggtaatcagtatgcgtctgcgttggtgagtacggcgattgcgctgttgctggtgtgcctggcattgctgttacctgcggcgaacagtgaaatacacctcggggtgctgagtattttctgggggatcgcgatgatgatcatcgggcttggtatgcaggttaaagtgctggcgctggcaccagatgctaccgacgtcgcgatggcgctattctccggcatatttaatattggaatcggggcgggtgcgttggtaggtaatcaggtgagtttgcactggtcaatgtcgatgattggttatgtgggcgcggtgcctgcttttgccgcgttaatttggtcaatcattatatttcgccgctggccagtgacactcgaagaacagacgcaatagttgaaaggcccattcgggccttttttaatggtacgttttaatgatttccaggatgccgttaataataaactgcacacccatacataccagcaggaatcccatcagacgggagatcgcttcaatgccacccttgcccaccagccgcataattgcgccggagctgcgtaggcttccccacaaaataaccgccaccaggaaaaagatcagcggcggcgcaaccatcagtacccaatcagcgaaggttgaactctgacgcactgtggacgccgagctaataatcatcgctatggttcccggaccggcagtacttggcattgccagcggcacaaaggcaatattggcactgggttcatcttccagctcttccgacttgcttttcgcctccggtgaatcaatcgctttctgttgcggaaagagcatccgaaaaccgataaacgcgacgattaagccgcctgcaattcgcagaccgggaatcgaaatgccaaatgtatccatcaccagttgcccggcgtaatacgccaccatcatgatggcaaatacgtacaccgaggccatcaacgactgacgattacgttcggcactgttcatgttgcctgccaggccaagaaataacgcgacagttgttaatgggttagctaacggcagcaacaccaccagccccaggccaattgctttaaacaaatctaacattggtggttgttatcctgtgtatctgggttatcagcgaaaagtataaggggtaaacaaggataaagtgtcactctttagctagccttgcatcgcattgaacaaaacttgaaccgatttagcaaaacgtggcatcggtcaattcattcatttgacttatacttgcctgggcaatattatcccctgcaactaattacttgccagggcaactaatgtgaaaagtaccagcgatctgttcaatgaaattattccattgggtcgcttaatccatatggttaatcagaagaaagatcgcctgcttaacgagtatctgtctccgctggatattaccgcggcacagtttaaggtgctctgctctatccgctgcgcggcgtgtattactccggttgaactgaaaaaggtattgtcggtcgacctgggagcactgacccgtatgctggatcgcctggtctgtaaaggctgggtggaaaggttgccgaacccgaatgacaagcgcggcgtactggtaaaacttaccaccggcggcgcggcaatatgtgaacaatgccatcaattagttggccaggacctgcaccaagaattaacaaaaaacctgacggcggacgaagtggcaacacttgagtatttgcttaagaaagtcctgccgtaaacaaaaaagaggtatgacgatgtccagacgcaatactgacgctattaccattcatagcattttggactggatcgaggacaacctggaatcgccactgtcactggagaaagtgtcagagcgttcgggttactccaaatggcacctgcaacggatgtttaaaaaagaaaccggtcattcattaggccaatacatccgcagccgtaagatgacggaaatcgcgcaaaagctgaaggaaagtaacgagccgatactctatctggcagaacgatatggcttcgagtcgcaacaaactctgacccgaaccttcaaaaattactttgatgttccgccgcataaataccggatgaccaatatgcagggcgaatcgcgctttttacatccattaaatcattacaacagctagttgaaaacgtgacaacgtcactgaggcaatcatgaaaccactttcatccgcaatagcagctgcgcttattctcttttccgcgcagggcgttgcggaacaaaccacgcagccagttgttacttcttgtgccaatgtcgtggttgttcccccatcgcaggaacacccaccgtttgatttaaatcacatgggtactggcagtgataagtcggatgcgctcggcgtgccctattataatcaacacgctatgtagtttgttctggccccgacatctcggggcttattaacttcccacctttaccgctttacgccaccgcaagccaaatacattgatatacagcccggtcataatgagcaccgcacctaaaaattgcagacccgttaagcgttcatccaacaatagtgccgcacttgccagtcctactacgggcaccagtaacgataacggtgcaacccgccaggtttcatagcgtcccagtaacgtcccccagatcccataaccaacaattgtcgccacaaacgccagatacatcagagacaagatggtggtcatatcgatagtaaccagactgtgaatcatggttgcggaaccatcgagaatcagcgaggcaacaaagaagggaatgattgggattaaagcgctccagattaccagcgacatcaccgccggacgcgttgagtgcgacatgatctttttattgaagatgttgccacacgcccaactaaatgctgccgccagggtcaacataaagccgagcatcgccacatgctgaccgttcagactatcttcgattaacaccagtacgccaaaaatcgctaaggcgatccccgccaattgtttgccatgcagtcgctccccgaaagtaaacgcgccaagcatgatagtaaaaaacgcctgtgcctgtaacaccagcgaagccagtccagcaggcataccgaagttaatggcacaaaaaagaaaagcaaactgcgcaaaactgatggttaatccataccccagcagcaaattcagtggtactttcggtcgtgcgacaaaaaagatagccggaaaagcgaccagcataaagcgcaaaccggccagcatcagcggtggcatgttatgaagccccactttgatgaccacaaaatttagcccccatacgaccactaccagtagcgccaacaccccatcttttcgcgacattctaccgcctctgaatttcatcttttgtaagcaatcaacttagctgaatttacttttctttaacagttgattcgttagtcgccggttacgacggcattaatgcgcaaataagtcgctatacttcggatttttgccatgctatttctttacatctctaaaacaaaacataacgaaacgcactgccggacagacaaatgaacttatccctacgacgctctaccagcgcccttcttgcctcgtcgttgttattaaccatcggacgcggcgctacgctgccatttatgaccatttacttgagtcgccagtacagcctgagtgtcgatctaatcggttatgcgatgacaattgcgctcactattggcgtcgtttttagcctcggttttggtatcctggcggataagttcgacaagaaacgctatatgttactggcaattaccgccttcgccagcggttttattgccattactttagtgaataacgtgacgctggttgtgctcttttttgccctcattaactgcgcctattctgtttttgctaccgtgctgaaagcctggtttgccgacaatctttcgtccaccagcaaaacgaaaatcttctcaatcaactacaccatgctaaacattggctggaccatcggtccgccgctcggcacgctgttggtaatgcagagcatcaatctgcccttctggctggcagctatctgttccgcgtttcccatgcttttcattcaaatttgggtaaagcgcagcgagaaaatcatcgccacggaaacaggcagtgtctggtcgccgaaagttttattacaagataaagcactgttgtggtttacctgctctggttttctggcttcttttgtaagcggcgcatttgcttcatgcatttcacaatatgtgatggtgattgctgatggggattttgccgaaaaggtggtcgcggttgttcttccggtgaatgctgccatggtggttacgttgcaatattccgtgggccgccgacttaacccggctaacatccgcgcgctgatgacagcaggcaccctctgtttcgtcatcggtctggtcggttttattttttccggcaacagcctgctattgtggggtatgtcagctgcggtatttactgtcggtgaaatcatttatgcgccgggcgagtatatgttgattgaccatattgcgccgccagaaatgaaagccagctatttttccgcccagtctttaggctggcttggtgccgcgattaacccattagtgagtggcgtagtgctaaccagcctgccgccttcctcgctgtttgtcatcttagcgttggtgatcattgctgcgtgggtgctgatgttaaaagggattcgagcaagaccgtgggggcagcccgcgctttgttgatttaagtcgaacacaataaagatttaattcagccttcgtttaggttacctctgctaatatctttctcattgagatgaaaattaaggtaagcgaggaaacacaccacaccataaacggaggcaaataatgctgggtaatatgaatgtttttatggccgtactgggaataattttattttctggttttctggccgcgtatttcagccacaaatgggatgactaatgaacggagataatccctcacctaaccggccccttgttacagttgtgtacaaggggcctgatttttatgacggcgaaaaaaaaccgccagtaaaccggcggtgaatgcttgcatggatagatttgtgttttgcttttacgctaacaggcattttcctgcactgataacgaatcgttgacacagtagcatcagttttctcaatgaatgttaaacggagcttaaactcggttaatcacattttgttcgtcaataaacatgcagcgatttcttccggtttgcttaccctcatacattgcccggtccgctcttccaatgaccacatccagaggctcttcaggaaatgcgcgactcacacctgctgtcacggtaatgttgatatgcccttcagaatgtgtgatggcatggttatcgactaactggcaaattctgacacctgcacgacatgcttcttcatcattagccgctttgacaataatgataaattcttcgcccccgtagcgataaaccgtttcgtaatcacgcgtccaactggctaagtaagttgccagggtgcgtaatactacatcgccgattaaatgcccgtaggtatcattaaccaatttaaatcggtcaatatccaacaacattaaataaagattcagaggctcagcgttgcgtaactgatgatcaaaggattcatcaagaacccgacgacccggcaatcccgtcaaaacatccatattgctacggatcgtcagcaaataaattttgtaatcggttaatgccgcagtaaaagaaagcaacccctcctgaaaggcgtcgaaatgcgcgtcctgccagtgattttcaacaatagccagcattaattcccgaccacagttatgcatatgttgatgggcagaatccattagccgaacgtaaggtaattcatcgttatcgagtggccccagatgatcaatccaccgaccaaactggcacagtccataagaatggttatccgttatttctggcttactggcatctctcgcgaccacgctgtgaaacatactcaccagccactggtagtgggcatcgatagccttattgagatttaacaagatggcatcaatttccgttgtcttcttgatcattgccactcctttttcacagttccttgtgcgcgctattctaacgagagaaaagcaaaattacgtcaatattttcatagaaatccgaagttatgagtcatctctgagataacattgtgatttaaaacaaaatcagcggataaaaaagtgtttaattctgtaaattacctctgcattatcgtaaataaaaggatgacaaatagcataacccaataccctaatggcccagtagttcaggccatcaggctaatttatttttatttctgcaaatgagtgacccgaacgacggccggcgcgcttttcttatccagactgccactaatgttgatcatctggtccggctgaacttctcgtccatcaaagacggccgcaggaataacgacattaatttcaccgctcttatcgcgaaaaacgtaacggtcctctcctttgtgagaaatcaaattaccgcgtagtgaaaccgaagcgccatcgtgcatggtttttgcgaaatcaacggtcattttttttgcatcatcggttccgcgatagccatcttctattgcatgaggcggcggtggcgctgcatcctgttttaaaccgccctggtcatctgccaacgcataaggcatgacaagaaaacttgctaatacaatggcctgaaatttcatactaactccttaattgcgtttggtttgacttattaagtctggttgctatttttataattgccaaataagaatattgccaattgttataaggcatttaaaatcagccaactagctgtcaaatatacagagaatttaactcactaaagttaagaagattgaaaagtcttaaacatattttcagaataatcggatttatatgtttgaaaattattatattggacgagcatacagaaaaagcaaatcacctttacatataaaagcgtggacaaaaaacagtgaacattaatagagataaaattgtacaacttgtagataccgatactattgaaaacctgacatccgcgttgagtcaaagacttatcgcggatcaattacgcttaactaccgccgaatcatgcaccggcggtaagttggctagcgccctgtgtgcagctgaagatacacccaaattttacggtgcaggctttgttactttcaccgatcaggcaaagatgaaaatcctcagcgtaagccagcaatctcttgaacgatattctgcggtgagtgagaaagtggcagcagaaatggcaaccggtgccatagagcgtgcggatgctgatgtcagtattgccattaccggctacggcggaccggagggcggtgaagatggtacgccagcgggtaccgtctggtttgcgtggcatattaaaggccagaactacactgcggttatgcattttgctggcgactgcgaaacggtattagctttagcggtgaggtttgccctcgcccagctgctgcaattactgctataaccaggctggcctggcgatatctcaggccagccattggtggtgtttatatgttcaagccacgatgttgcagcatcggcataatcttaggtgccttaccgcgccattgtcgatacaggcgttccagatcttcgctgttacctctggaaaggatcgcctcgcgaaaacgcagcccattttcacgcgttaatccgccctgctcaacaaaccactgataaccatcatcggccaacatttgcgtccacagataagcgtaataacctgcagcatatccgccaccaaaaatatgggcgaaataactgctgcgatagcgtggcggtatagcaggaagatccatattttccgccaccagcgcccgcaattcaaaatcatcgacatcctgcattgcttcgttttcttccaggcaatgccagcgcatatcgagaagtgcggcgctaagcagttcgctcatctcataccctttgttgaacaggctggcattacgcattttctgttgcagttcgtcaggcattgctgccccgctctgataatgccgggcgtagcgagcgaatacctgcggatgcgttgcccagtgttcgttgatttgcgacggaaattcgacaaaatcacgcggcgtgttggtgccggaaagcgtggcataacgctggcgggcaaaaaggccgtgcagcgtatgaccaaattcatggaataaggttatgacatcatcccagagtaacaacgcaggctcaccggcagcgggtttctgataattgcagacgttataaattaccggatgtgttttattaagcgttgattgctcaacaaaattgcccatccatgcaccgccgctttttgaatcacgggcgaagaaatcaccgtaaaataacgccagccccacgccattatgatcaaaaatttcccacacacgaacgtcaggatggtagacaggaatatcaaaacgttcgacaaacttaataccgaagagctgattcgcggtccagaatacaccttcatttaacaccgtgtttaattcaaaatatggcttgagctgcgcctcatcaagatcaaatttctcccgccgtacctgttccgcataaaatgcccagtcccacggctgcgcgctaaacccgccctgctgcttatcgataaccgcctgtatggaggctaattcatcgctcgcacgttgacgcgccgctggaacaatttcccgcataaagttaagtgctgcttcaggtgtttttgccatctgatcggcgattttccatgcggcataatgaggaaaaccaagtagtgttgcctgttgtgcacggatctccaccagacgttgaatgatagcgcgggtatcattggcatcatttttttccgctcgcgtccagcccgcaataaacagtttttcacgcgtcgcacgatcgcgcatttcggcaagcgccggttgttgggtggtattcagcagcggaatcagccatttgttatccagacctttctcgcgagccgcctctgccgccagcgcaatctcttgctcactcattcctgccagctgcgcgatatcgttcacaaccagaccgccggatttatttgctgccagtaatcgctggttaaactggctggtcagggtcgcagcttctgtattcagtacttttaattttgctttatcagcttgcgcaagtttggctccggcaaggacaaaacgttgatgaatcacctccaccaggcggatggattcactatcaagccccagggattcacggcgctgccagacagcatctacccgcgcgaataattcaccgttcagatagatatcattagccagttccgccagttcagcggaaaactgctcgtcaagacgctgtaattcatcattggtatgcgccgcagtcatcgcaaaaaagacgctggtaacgcgggtaagtaattctccgctttgttccagtgccagaatagtattgttgaaatcaggcatttgcgggttaagcgcgatggcagcaatttctgcccgcttttgctgcattccctcatcgaatgccgggcgatagtgatgattggcaatttgatcaaaatggggagccagatacggcagtgtgctttgcacaaggaaaggattcattgttgtcattttcttctcctgaacgcgaggtgttccatagcgtaggcttactgataacggagtgcaatcttgcaatccagtattacccgctcttaagcatcccgtgctatgttattgacacacaaaagcgttgaggaacagtgagatgatcgttttagtaactggagcaacggcaggttttggtgaatgcattactcgtcgttttattcaacaagggcataaagttatcgccactggccgtcgccaggaacggttgcaggagttaaaagacgaactgggagataatctgtatatcgcccaactggacgttcgcaaccgcgccgctattgaagagatgctggcatcgcttcctgccgagtggtgcaatattgatatcctggtaaataatgccggcctggcgttgggcatggagcctgcgcataaagccagcgttgaagactgggaaacgatgattgataccaacaacaaaggcctggtatatatgacgcgcgccgtcttaccgggtatggttgaacgtaatcatggtcatattattaacattggctcaacggcaggtagctggccgtatgccggtggtaacgtttacggtgcgacgaaagcgtttgttcgtcagtttagcctgaatctgcgtacggatctgcatggtacggcggtgcgcgtcaccgacatcgaaccgggtctggtgggtggtaccgagttttccaatgtccgctttaaaggcgatgacggtaaagcagaaaaaacctatcaaaataccgttgcattgacgccagaagatgtcagcgaagccgtctggtgggtgtcaacgctgcctgctcacgtcaatatcaataccctggaaatgatgccggttacccaaagctatgccggactgaatgtccaccgtcagtaatttttatacccggcgtaactgccgggttattgcttgtcacaaaaaagtggtagactcatgcagttaactcactcacaagcaagaacgaatgaccgtcgaaacgcaacttaatcccacacagcctgtcaatcagcagatttatcgtattcttcgtcgcgacattgtccattgcctgattgctccaggcacaccgttgtcggaaaaagaagtttctgttcgtttcaatgtgtcacgccagccggttcgtgaagcctttattaaactggcggaaaacggcctgattcaaattcgtccgcaacgtggcagctacgtcaacaaaatttccatggcccaggtgcgcaacggcagttttatccgtcaggccattgagtgcgcggtggcgcgtcgggcggcgagcatgattaccgaaagccagtgctatcaactggaacaaaatcttcaccagcaacgcattgccattgagcgcaagcaactggatgatttttttgaacttgatgacaacttccatcaactcctgacgcagattgccgactgtcaactggcgtgggataccattgagaacctgaaagcgaccgttgatcgcgtgcgctatatgagtttcgaccacgtttctccaccagaaatgctgttacgccagcatcttgatattttctctgccctgcaaaaacgtgatggcgatgcggtagaacgtgcaatgacgcaacatttgcaggaaatcagcgaatccgtgcgccagatccgccaggaaaacagcgactggtttagcgaagagtaattcatttcctctcatcccatccggggtgagagtcttttcccccgccttatggctcatgcatgcatcaaaaaagatgtgagcttgatcaaaaacaaaaaatatttcactcgacaggagtatttatattgcgcccgttacgtgggcttcgactgtaaatcagaaaggagaaaacacctatgacgacctacgatcgtaaccgtaacgcaatcaccactggcagccgtgttatggttagcggcaccggtcacactggcaagatcctgtcgattgatactgaaggtctgaccgctgagcaaatccgccgcggaaaaaccgtagttgttgaaggttgtgaagagaaactggcaccactggacctgattcgtctcggcatgaactaagcgtgtgaatgccgccgatggcggcattgcttttttacttcacggaatattttgccacggtcgctttcgcgccatgcgctaataaagacaagtacgtttccgtcactcttgcagtaaacaaactattgtctggcaaatcatcaccaaagatcgccttaatcgccagcaatgactggacgcgcgctttcccttcggcactactttgtacagccttctgaataacaggtaacagtgggtcactgatttctatcggatttccctgttcatcaacaccaccgacataacgcatccaacccgcgacgcccagcgccagcagatcgaacttgctgtcatgcgccagatgccagcgaacagaatccaacatccgctgtggcaatttctggctaccatccatcgcaatctgccaggttcgatgacgtaacgccgggttgctatagcgtgcaattaatcggttagcgtaatcttgcaaatcaacgccctgcactttcaacgtcggcgcttgttcctgcaacatcaagccatacgccgcataacgataatgttcatcttccatacagtcattaatgtgctgatatcctgcaagataccccagatacgccaggaatgaatgactgccgttgagcatgcgcaacttcatctcttcataaggcagcacatcgctaaccagttcggctcccgctttttcccattccggacgtccggcaacaaagttatcttctattacccactggcggaaaggttcacaggcaacgcccgcaggatcgcgcacaccggtaagttgttcgattttcgccagcgtatcctctgtcactgcgggcacaatacggtccaccattgttgatgggaaagtcacgttatcttcgatccattgtgccagttttacatcaacggcttgtgcgtaggaagtgacaacgtcacgcataacatgaccgttttctggcatgttgtcacatgacatgacggtaaatgcgggaagtcctgccgctttacggcgagccagcgcctcaacaatcacccctgttgctgttttcggctggtggggattttgcacgtcggcagctaccatcgggtgatcgagcattaactgtccggtcgccggagagtggaaataccctttttcggtgattgtcagagagacaatcgcgatttgcggttcacacatcgctgccaacacggtttctaagccatctatctgtacgtgcaaggcttttttaacgacgccaacgacgcgagccgtccacacatcggccgacatttccgcaacggtataaagattatcttgctgttgtaaatcggcaatttgctgttcgccgccgattaagttgacctcataatatccccagtcactgaaatgttccgtagcaagaatatcggcatacacaccctgatgcgcacggtgaaatgcaccaaagcctaaatgaacaattcttggagccaggttattaagatcataaacagggagtgtcgcttttgctgataacaaattatttcccataacaattccttaaatataaatatggcaagctatatgttttgttatatgaataaaaatcccctctccggtaagagaagggattaagggtttacagacttctggaaggttgcgcagctcttacaacacgcggttgatcttccgcagcgtcttccagcgcacttaaatcacggtctttcacctctggcattttcagcgcagagattaaaccaatcactgaatatgccatgatcataatggcgatcggataccaggattccgtcatggtgcagaaaatacccgccaggataggaccaaaaccggaagcgataagaccaccaatttctttagaaatagccatccgggtaaagcggtttttacagccgaacatttctgccatggtaatgttttccagagcaaataatcccagcaccgcacagttatgaatcacaatcagtgcaaccataatggtgctcggggcatagcttttatctacaatgatagaaagcattggccatgccagcacaatcgcggaggtattcataataatatacgggatccggcgaccaattttatcggataaccaaccaaggaacggaatggtcataaagccgagaatcgaactgatcatcaatgcatctgttggaattgctttgttaaacaataacgtctgcactaaatagcctgcaaggaaagtctgaattaacccggagttacccgcctgaccaaaacgcagccctgttgccagccagaaggatttgctctggaacatgctaccagcaggtgcaggttttgctgtcggttggttactgtcgttaaccttctcaaagaccgggctttctttcagattcatacgcaaccagatagcaaagaccatcacgacaacactcgccaggaacggtatacgccatccccacgccagcagttcctctttactgagaatgaagaacataaaggcccagattgccgttgcgctcaaggttccgcagttagttcccatagccacaaatgaggagataattccgcgcttaccttttggcgcatattccgccagcatcgtaccggcaccggaaatttccgcacctgcacccaacccctgaataatacgcaacgtcaccagcaagatgggtgcaaaaacaccaatctgtgcataggtcggtaacacaccaattaaggtggtacagatccccatcatggtgatggtaataaagagcacttttttacgccctattctgtcgcccattttgccgaaaataaatgctccgacaatacgcgccacataacctgcaccgtaggttcccattgccagaattaacgccattgccgttgatgattcaggaaaaaatatttcatgaaacactaacgctgcgccgagcgaatataactggaaatccataattcacaggtgttttttcccatcctgtggtttccttggcgttttctaggttttttcagatagttgcatttttttaaaaagcatcctaagttcgatctcagtgtctatctggggcctatttctgtcccatatatgccccaaaaaaactccccaacagataagtagttttttcatggatttatgcgtaaaatcaagaacggctggaaatcattcaatactcacactatcgaaaaatttaccagccaatcgcagcacgttcttgcataaggtgtgtctgcggtttttcaactattcagatacatcactcccatcacattcattcctccgcatcaaaggcatataggctatatcaccttgatatttttctttttcagataaaaactgttatctatgtatacttttaaacccaatccgtgtagagtctctacataagatagtttgcagttgccgcttcagcttgcgccataaaccgcctgatttttgctgccacctgttagcattcctgtatacctgaaacgacaatgtttatctacgaactttaagaacacccaagataaaaattgtcaactatatcatatataacacattactaattcgaggctatatgaacagcatactgataatcacatctctccttatcatattcagcatttttagtcatgccctaataaaattagggattggcatatccaataacccagacaaaaccgatgtataagtcaacatatcctgaatcagacatacaatatcgcaatgaaaatcaataatattttaaggaatatcttcatgaaatcaaaagacaccctaaagtggttccctgcgcagcttcctgaagtaagaattatcctaggggatgctgtagtggaagtagcaaaacagggaagacctatcaataccagaacattgcttgattacattgaaggaaacataaagaaaaaatcatggctggataacaaagaattattacaaacagcgatatcagttcttaaagacaaccaaaatttaaatggtaaaatgtaatataataaacttacttttttatcatttttccactttaacaacattttgctccacttttccacgaccaaacaacttgaaatctggttaaaataacacgcaacactattcttcttccttgagtccgcccggaactcgaaaaacaaaccgagttaaagccatttttcacaaaatcgattttgggtctcaccaaaattacggggttgcatacgcattcgtttattttcgaacgtgtacatacaaatatgcacaaaaataatcataattattttctgagatgcattatgatatgaacaccaatttcgtatagagtctcactatgtctcaaatttttgcttactgtcggatatcaacgctggatcagaccaccgaaaatcaacgccgggaaatcgaaagtgcaggttttaaaatcaaacctcagcaaataatcgaagaacacattagcggctcagcagcaaccagtgagcgtcctggttttaaccggttgcttgctcgcctgaaatgtggtgatcaattgattgtgacaaaactggatcgccttggttgtaatgcaatggatatcaggaaaacagtggaacaactgaccgaaacaggtatcagagtgcattgcttagcattggggggcattgacctgaccagtccaacaggaaaaatgatgatgcaagtaatttcagcagtcgctgaatttgaacgagaccttttacttgaacgcactcattccgggatagtaagagcccgcggcgcagggaaacgttttggtcgaccacctgtgttaaatgaagaacagaaacaggcggtattcgaacgaattaagtcaggtgtaagtataagtgccattgcccgggaattcaaaacctcgcggcaaaccattttaagagccaaagcaaaacttcagacacctgacatataaaaaataatctcggtgtgagatgctttacgtcttccaagcccccttccttgccgtaaatggaaagatacatctaattatagaatttatatgttttaccctacggcagtgctggccattcaatatcctgtgcagttgacgtatcaacacggttcagcaatacccgatactttttccatgcttccagcaacgagatttcttcctccgttgcaatttccagatctgcagcatcctgaagcggcgcaatatgctcactggctacctgcatcaggttgttttttgtttcttccgcctcccggatccggaacagtttttctgcttccgtatccttcacccaggctgtgccgttccacttctgaaactccccttccggcgataaccaggtaacattttccggtaacggaccgagttcagaaataaataacgcgtcgccggaagccacgtcataaaccgttttaccccgatgatcttcaacgagatgccacgatgactcatcactgttgaaaacagccacgaagccagccggaatatctggcggtgcaatatcggtactgtttgctggcagacctgtatgaggcggaatatatgcatcaccttcaccaataaattcattagttccggccagcagattataaatttttatggtccgtggttgttcactcattctgaatgccattatgcaagcctcacaatatagttaaatgcgatgtttttgacggtgttttccgcgttaccagcagcgttaacggtgatggtgtgtccatgtgaaccaatcgcaacggagtgcgtatgagcaccaataccgacagtatgtgcatgcgcgcctgcgcttgcagcagtgccggacagcgagtgggtatgagcaccatctgatgatgtcttccctgcattacgagtctggccactaccgcttgttgtgctcataatccccgcgcttagatttgaaatcgcggtataaccattagggaaaatgctcgtgttcgtgccaccaaatgcaccggaactcttgtgttggtgcgcaccggcactatttgcggtcccgctaatactatgggtatgcgccccggtgttattcgtggatttggttccgtaatcaaacgacgatgtggtttccgtccccaaatccgtactggatgcgctggcgctgtgggtgtgcgatttaatgccgtcctgttcctgagataatacggcccgaccactggcgggcttgcccttaatcgtccagccacgcatatcagggatcacgcctgacggataagcaactgcaagtttcgggtatgcagatttgtcaaaagtctgcccctgcatcagggcataaccagacggaacggtatctgatggccacgggattggtgcaccgactggataaaactctgcaggaggatgagccgaggtgtaaagctgcgcccacggcgaccagtttgcgtcggtcgtatcccgtcgtgaacgaataaatgccggagcatgagcaccgcttgtaccactccagccgatgagtaactcaccttcgccaacggctgtcatccctttcaggtgaatgatatttccatacgctgttggatatccgttgttatacacctcgtataactcaagacctgctgccccctgcgtattgtctgtcagcgcggttatattcactcagcaaccccggtatcagttcatccagcgcggctgctttgttcatggctttgatgatatcccgtttcaggaaatcaacatgtcggttttccagttccggaaaacgccgctgcaccgacagggggatcccgtcgagaatactggcaatttcacctgcgatccgcgacagcacgaaagtacagaatgcggtttccaccacttcagcggagtctctggcatttttcagctcctgtgcgtcggcctgcgcacgcgtaagtcgatggcgttcgtactcaatagtccctggctggagatctgtctcgctggcctgccgcagttcttcaacttcccggcgcagcttttcgttctcaatttcagcatccctttcggcataccatcttataacggcggcagagtcataaagcacctcattacccttgccaccgcctcgcagaacgggcattccctgttcctgccagttctgaatggtacggatactcgcaccgaaaatgtcagccagctgctttttgttgacttccattgttcattccacggccaaaaacagagaaaggaaacgacagaggcccaaaagctcgttttcagcacctgtcgtttcctttcttttcagggggtattttaaataaaaacattaagttacgacgaagaagaacggaaatgccttaaaccggaaaattttcataaatagcgaaaacccgcgaggtcgccgccccgtaacctgtcggatcaccggaaaggacccgtaaagtgataatgattatcatctacatatcacaacgtgcgtggaggccatcaaaccacgtcaaataatcaattatgacgcaggtatcgtattaattgatctgcatcaacttaacgtaaaaacaacttcagacaatacaaatcagcgacactgaatacggggcaacctcatgtcaacgaagaacagaacccgcagaacaacaacccgcaacatccgctttcctaaccaaatgattgaacaaattaacatcgctcttgagcaaaaagggtccgggaatttctcagcctgggtcattgaagcctgccgccggagactgtgctcagaaaaaagagtttcttctgaagcaaacaaagaaaagagtgacattactgaattgctcagaaaacaggtcagaccagattgaagcaatttagataatcgtgcagactacgccccctcatatcacatggaaggtttatctatggatcaggtagtcatttttaaacaaatatttgataaagttcgaaacgatttaaactatcaatggttttattctgagctaaaacgtcacaatgtctcacattacatttactatttagccacagagaatgttcatattgtattaaaaaatgataatacagtgttattaaagggcctaaaaaacattgtgtctgtcaaattttcaaaggataggcatcttatagaaacgacctctaataagctgaaatccagagagatcacatttcaggaatacagaagaaaccttgctaaagcaggagtttttcggtgggttacaaatatccacgaacaaaaaagatattactatacctttgataattcattactatttactgaaagcatccagaaaactacacagatcttaccacgctaaaccataacgtccggcttctctcactcctgagccggactgcattggtttaataaaaaccatcaacaattgtgatttagatattcggaaccattcaaatataacaaaaccccgtaaaaacgaggtttatggataaattttattattgaatacatcagattaaattaatcttgacatcatagctttcaagacccgtcattttttcccgtgcggtaaactgaatactggtaacttctttcccggtctttttcttaagttcaataattttttttgttatatattcagaaatatctgcttctgcttttgtttttaagttttcaatattcatcatttcctcttttagtctgttatgactttccagttacacagtaagtcgattatatggtgcaaacgtgtaaaagataagatgaaacatcgcaataatcaacatacgatagtctaaattttacacaaacagacaaagagaattttcctgaattatcaatgcaatagcatcaaatcaactcaagagccttattgctgcttccagaatttcttctgaagtaacatgtcgatccgcggctacataaatgactttatgatctccggtcagagatggaaaccctgcggccattacagtaaggtgtgttttttcgccatttggatattcacgcatgatggtgttaactccagtcatcgctggcactaccactgctggttcagagttaaaaaaactatgatttttttcatgatgttaccgtagtatgtgagtatccatcgaatagacaccaagcaaaaaagctcccgaaggagccttcattttcacttttttaaatccaacgacagacggctggcatttaagtattgtgaaatattatcaaatgtaatcatcattgatttacaaaagatacattttgccccgaaaggattcatgtcagaaacatcaaaagatgatgttctatactgggaaccatgacaacacgggcatctaaagtgaatatggtttgtaatattgtctacctcaaagcgccactacatgaacagcggcaggacctttaggtccgttctcaataccaaattcaacttcctgattctcagttaatgttttgaaatcgttgctctgaattgctgagaaatggacaaacacatctttgctgccatctttcggcgtgatgaaaccaaaacctttttcagggttaaaccatttcactaaaccagtcattttgttagacataattattaccttttgaagaaattagcccttgggcagaatggtccgaaaaaaaatatcagagagaaaaaccaacaaggaaatctcaagaggtacaaataataaaattataacaatgactgcttcagataaatttgtaacaaaccagaacaccattaacgcatgattaaccacccatagcaaggattacttttgtaaagaaaaacacagcaatgaaagaatagctttatttattaataaaacgtgtcattctgattaagaccttttatcttacccttaagatttcaggaattttggctcatggaagagtcctttttatttaaattttacattccgcgatgtaaatgttccgatttaatattaccctacatttgatgctttttatctcttaaagattcatagatctgttgacaagtcactcctgcgatgtagcgttcgtcagcaatttcagcataaagctgagcttctgctgcaatatctccgagcatgttggtgagcattccttcggcggttttggttgttttgcctctgacggcagcggcaagatctgcggtatgcttcgctgcgtcaaggcgtatggcatatttttttgcttcggcacgcaactggttaacactatcagacagataagcagccctggcagaaatttcagcagatttctgttgcgcatctttaacagcctcatcacgggctatagttcgcccctgttcaattattcgagcagcaaattgagcatttacctcttgtgataatgcggcagcatcacgttccgcccattttttttgccatcctcggtcgctccagacatttccgacgataaatcctgacaacacgagaaaaatcaccatgaatatctgattcactgttctatcccccagcaggttaatgcgctctcctggtcacgacgaataacctgaccgtaacagttatttgaacgaatgcggcaatcgcgtccgccatccttaatccaccagcgaatcgcttcgcatgcacctttacgatcaccagcattcagccgcttataaaacgtcgacgggaaacacttaccggggccaatgttatagggacaaaatgacgcgatacccgctttttgtggttcggtcagtggtactttaatattgcgctccacccatgccagcgccttatcacgctcaatggcgttgacctggtcgcatttttccttcgacagtttcatattgggaaaaacggtttttccatccaccactgtggcaccccgacagatggtccatatgccagaaccatcgcggtatgccattgtgtggttaccttctttttcgtccagaaactggtcaagtatctgaggagcagatgcgccagcaccaatcagcgccagaacggcagccgacaggccgtatctgatttttgtgttcatagatatttatgatgaggacgctcgtgcttattggcaggattttcaatcttaaaggagtactgatgctgcagataagactcaactttttctgacaatttttctgctacttccaggaagacttgccggacgctccttctggctgctgcctcataaaactccagcgcagctccttcaacacggtccatggcgacatccaggtcaaaaatttcaccgtcaaagcgttctttgtcctgtaaggctacagttaccgtaactttattctcaaaattacggactcctttcacaaccagttcatagtcttgagtcattggattactctcctctcgcagccttacgcctgtcttctttaatcttgaaataaagatttgtcagatacgtcagcaggccaaaaaccaggctacccagcacaccgattgcagcccactgtgacggagttactttatcgagtaactgcaatgcccagaaaccagcattacccgccgatgtgccataggcaacacctgttgttaacttatccattgatttcatatcctcaccccgatgtacacggatggtgcaatatgtttgaaaagatcggagtctacggggtagttttgacagcacacgttgttctcaacggcgctaaaaaaacatacacattaaaaatgtgggtaattattttgaaagaaagtcatatataaaataataatacgagaaatgttttcatatttagtgtactgtatacggccatttatacaggaaaagcctatgtcagaacgtaaaaactcaaaatcacgccgtaattatctcgttaaatgttcctgcccaaactgcacccaagagtcagaacacagtttttcaagagtacaaaaaggtgcccttttgatctgccctcattgcaacaaagtattccagacaaatcttaaagctgtagcctgattgattttattagtaacaagtattttttatattttaataatatatttaaagcagataataaaaaacccgcctgagcgggtttgagattgtggtgctttttgtgggagtcatccacttacgcactttgttttgccatgccagcagttagcttctgctgtaaaactattcatgcagcaaacctgcacttcaccacaatggttagcatacttttcctgattaagattttgccaaatatgctagccattgtttcatgtattggacctccttactttttattaaagagatccaatattcactactctgtccgtatctctactcaggcatcagccttcttcgttatcgtatacagacgagcgatgaattttaatcagtaatgatgacatttgctgctgcaggacctttagcaccactctctatagagaaggtaaccttttgaccttcaaataaggttcgataattatcattctgaatcgcagaaaaatgcacaaacacatctttactaccatcaacaggagaaataaagccgaaacctttatcagcgttaaaccattttactaaaccagtcattttatttgacattctacattccttaacttgagcctttcggcataaatggtttgcataacagaaacgacttcgtacttaattggagagactcaaagaaggaataagtgaataacacctgaaatgagaactgctttagtaaactacttcgtatatcgtctgttcttcaaaccgacgcaatcattaacgcatagttgaacatatgaagcaatgtttattttagacatccagccatcttcaaccccatcaaaaaactatagctttcttcaggaacgtgtgtatagtgcgccaagttatcagtattaaggaatttttttgtcccgtaaaatgacaggaattgtcaaaacctttgacggcaaaagcggcaagggtcttatcaccccatccgatggtcgtatcgatgtccagcttcatgtttcagcgctcaatctccgcgatgcagaagaaattaccaccggattacgcgtggaattttgccggataaatggtctgcgtggcccttcagctgccaatgtttacctttcatgagctatattaaagctttaatttcaggccccatcggatcacacatggagagtttttatgaataaccccgtctgtcttgatgactggttgattggctttaaaagcttatgctgtactttggccgtaatagctctgctaataatataataagcagactcattgtgtttagggacattgtactggaagaaaacattttaaacatcaggcaaataaccaagtcaccagctaaataataagttaacagacatgagtcccgggatgagattcaacattaccattgccccatttaaagcacaaaacccgctcatcagcgggttttctactttttcttaacgtcgggtatacaaagcccatcgttgaaaaaattttatccatattttttgaaaaatgcaaacatcatgtcgccatcttcagcaaaaatcatttatctcgtcaccttcctcaattgcgcttccgcgtatgcttcttcctgccagcactttgttaccagtttaccaatgacgtccgcataccccttataccactgataatcggtcaggtctggtaccagcttctggacatgacgtcgtgccagcgtggtcggtaaacgactaaaccggtttccattacaacgcccacaaatcttatataccggtacgccatgaaaccgggttcttttttcatccagaacaatccctttacccttacaccctctgcacgctgtgctggcttcgcccttaccatggcaatgctgacatagttccttcacccattcttccttgattacagattccccgcgtctgtagtgtttcaccacttcgcgcaatacattataaaatcccgtacctgaacaatgctcacagcgagccttacttgccgcagacctggagtaatcagcaaaggcaaaactcacgaggtaaggaataatctgtaaccggatttcttcactcaatttgttcaatgtcgggttatccagtgccatcgcgtaatttagcaggccttcaatcgcaaactgagggtcctgaacaccaacttttgccagaaataaggccaacccaagtggtgctttcgactgcaccatcccctgcgctgccattacatccgtaattgttaaacaaccggtgcctgtcgctggagcgtcatcgctcaattttggagattttggggagtaatattttggtaaggcttcaaggttcatgctcgttctccacttacgccagtacgccaattgccagcgcgcgatcgataaaacgaaatatcagctccagttgggagccatacttatcttcaaatgccactgtatccgtatgcagctcgttgtgatgctttctgcacaaaggcaacacaaagagatcatgtgcttttgttcccattccgccctgcccgtgaccaatcagatgatgcggatcgtcggctggcataccgcagcaagcacacggctgtgtcttaacccaacgtgtgtatttctccttaacccagcggcgacgtttaggcagcttcatgaaagattccggagactctggatcaacggtgatgcttaccaccgtcttttcctgtggtgatttttgttgctggtgggcgtaaggcaacggtgcaagattttttgtgcgttgtttcaatatgctggtggcggtcagctctcccggtacgatgtcgctttcgcggtacaccgagcagattttttccgctggtaatcccagcgaacgacgcgatacagcctcaggtagtgcatccaccacctgattgcagaccgcccaccaggataattcagccaaagataattcccgctcctgcgtaccgcttattgcgtgacggatgacgtcaatcacccatgctgtcagattttgttgagcaagcagctccagtgattccgatgtctggtcacgcagttggttgtcgcagtgccagcacaacaccattgcgccggtaccataacggtgaatgactgtttcagtgtgatggtaatcgccattaggccactggcaggatgtaacatgacgtaatagccagtcggacaatgcgccaacgccgccagcagcacgaatcacccgttcgttactaaaaaacggcagcaatgttttgtcttccgccagcggctggcgaacggcaggaacgactccggatggcagattacgcatgctttttggttccggttccaccagcactcgaggattatgaaatatctgtatggattcacggcccggcttaaggaccaccagcccaagctcaggcaccagaacaggtctaagtaatacccgcacgttacctccagatccgttgctggaaagtgcgggacgcacgtggtgggcgttcggaataaggcagcctgacagagattatccagtgccgatagtcgagactgagagctttcttaacctcgaacccgcgcctgcggtaagaatgaatcagccattcggcctgttctgcagtgcatggagggtgctggaaccattcagacttgaatgcgtgagaataccgcccgtgcgtgcaggcaagaacgggcgaattatcagaattgtaatattttgcgttgcgtgccatcggttttctccggtggcacggtgttactcagcgggagttcagccccgcgcaagattgtagatgagtttattctcctgaaaaagcagaaaagccagcttttattccgatctctttcaatgcctgtaatgaagtgacaaactcaccttcgcgcaagataaatccgtccgtgacccgagcatccacaaaattaattaacgcagccccattctttcgcaaacacataatgcggtaatgactaacaagatttccattttcaacgcacacagcatagaggccatcttcacaaaaaattttacgcagttcttcgatgttcatcatcagaatccttccggataattagctctcccctttaagggaccatccctcttatccctgcgcgctacttaagtatttttgattctattccggcaccgtccagaacttcaaacgcgttgaaaataaaaacaaaaacccgccgaagcgggttaagtgcgggtgcgttgaggatgcctgccacatcagaggtggcgagggatttctcccccgccgggtctcttactcctcaggttcgtaagctgtgaagacagcgacctccgtctggccggttcggattcgtacctcgcagaggtctttcctcgttaccagtgccgtcactatgacggttaaacagatgacgatcagggcgattaacatcgccttttgctgcttcatagcctgcttctcctgtcaacgcaaagcagaagtgtcaccttcggtgcgaaacagagatgtcatgctttggttcagagaatgcgtttgaccgcctcgctatatacttccgagcgttctcttttcccaacagaaatcacgaaaacgacaactttctcgtctataacctggtatacaaggcgatagcctgaagaccggagcttaatcttgtaacaatcaggcataccacggagcttgtttgcttcaatccggggtgactcaagtacttcaaccagcttctttttcaactgttcacgtaccgtcgagcccagctttcgccattcctttagtgcccgctcgtcaaaatccagaaaatacgccatcagagttcatccagcgtcacacgtactggcttaggattacgaagccgttctttcactatctccacaagttcagcatcttcatcactcaggagtgtctgtttgaacggcaagcgttcattgtcagcgatatactcgagcatgagacgaagcgcttcagaaggagttacacccattttttcaagcgcggcgtaagaacgcgctttaagttcatcgtcaatacgcaggttaatgctacccatgtcttacacctcttgtaattacaaatgtcattacaagtatcgcactacaacatgcttagggcaagtcacgaaggaagtcagaaagtagtcgtaagaacggtgatcactgtccgctttgtgccaggagcagccattgctaagtccatcctgtattgtgcaggtcagctcgtttttaaagagtccggccatcatcttactggtacagacaccatatactttgtgacggtcaggctacatatgcacaactcaacttattcatctattttttgctttagcatgtcagtgttgctttctcgtcggcgggtgagcggtgacctgacctgtcgataaaggaacgtaacacgttttatgcaacacccgcatgcggcagaaaattattgccgaacgtttacccctgtcaacaagctttactttctgaggcgcgccagcccgcgaggaaaacaatctgaacatcaaacaattaatgacacaagaaatacgattaaagatttttttgtgcatgccgatagtgcttttttaaaaggagaaatctatgtctgtcacaattcagggaaatacctcaaccgttatttcaaacaactccgccccggaaggaacatcagaaatagccaaaatcacaagacaaattcaggtgctgactgaaaagcttgggaaaatctcatcggaagaggggatgacgacacagcagaaaaaagaaatggctgcattggtacagaagcaaattgaaagcctctgggctcaactggagcagttgttaaggcagcaggcagagaaaaagaatgaagacgcgacagttcagcctgataaaaaagaagagaaaaaagacgatacaaataccgctggcaccattgatatttacgtctaagtgacagccgtattgtggccctcatcgggccacttttcgccatcagccttttctttaaagacatattatctttgtatcatttctgatagttaacattacaagatataagtaatggacgcactcccaattagtctatttaaatcgccacgagtttaactgacaacccatgatcaattatgaattgcaactatttctgtagtcacttttgtggggacagtccacaaaactgccaacttccgcttcttgctcttagcggacattagcataggctatttaccataacgcctcattacgcgcaccgcccagactgactcagcgcgtttctggcatatccccggtaaaacaagtaacaaaccacccgaaaatgaacaccagaaacgcgacttaagaatctaccctatgaatggatatgcactcaaccgaatcgatcttggtttcaatcttttttatcgggatcaggcttctttttaggtaacttcgggggcttaacttgctgatgactttgcgttcggcgcgtaagccagggatggtcagctttaggtttaacatagtattttgagcgtaaatcaatacgggcattatccactcgttcatggacactcttttcatcatccagtggtagcctccataattgcaggcactagcgccgtgaacttttcacgcttatccctggtgtcgatagccttccagcgttcaaatatcttcactcgattaacgccaagcgctcgctgatcaatcgcgccaccttcatatgtgacacgctgaacatcgatgttcgggcgctctttcaaagcccagaatgcttcagtgattaatatcgtcgcctgctcctgtgtcattcctggtcgacatatccaggcatccagagcctcacgagcctgttcaggagtgattttcattgttcaaccgccccgcccgcttcgtcttacgatattcatcataaactttgggatcatactgaagctccccgccagatgcctcctgtagacgcatcgcgcgaccttcgggaactaaatcccctttccagctataaagcgaagccaaacgaatacctgctgcttgtgcaagttttgtttttgaaccgaaatacaaaagagcgtcagttttaagcatttaaaacacctttattgttagtcataactaacaagatagatgttaacaaaaacatagtcaatacgatttagcattagctaactatggaaacaaaaaatttaactatcggcgaacgcatcaggtatcgtcggaaaaacctcaaacacacccaaaggtctcttgctaaagccctgaaaatctcccatgtgtctgtatcacaatgggaacggggtgatagtgaacctacagggaagaacctttttgccctcagtaaagtattgcaatgctcaccaacatggattctatttggcgatgaagacaagcaaccaacaccacctgttgagaagccagttgccttatcccccaaagaactagagctccttgagctgtttaatgcactgccagaatcagaacaggatacccagctcgccgaaatgcgagctcgagtaaaaaacttcaataaactctttgaagaattactaaaagcccgtcagcggacaaataaaagataacatcatcaatgagttatcttttaccacatcaattatgttagctatagcatacaaaatcacttgaccgatatgttagtcatggctaatcttgtttgcatcaacacaccgcacggtgttctcagcaaacagttccgctaccccagcgttaaggggaaatgaggtcagcatggatactatcgatcttggcaacaacgaatctctggtgtacggcgtgtttccaaaccaggacggcacgttcaccgcaatgacgtataccaaaagcaaaacgtttaaaaccgaaaatggtgcccgtcgctggctggaaagaaactcaggtgagtgatatggatttcgacacaatcatggaaaaggcttacgaagaatacttcgaaggccttgccgaaggcgaagaagctctcagcttcagtgagtttaaacaggcgctttccagttcggcaaaatctaacggctgataagcgaaacagcaccgcgaggaatcagtatgcagaaacgagaacccgtcatcatcgcgccagactataccgatgatgaactttatgagtggatgcgccagaaaattaatgcagcgcaggatctgaaatgggctaatgaagccagggctaagcaggctgaaaatctgtccgctctggagcaggatatcaccaatctggaaaaagcagcggcattaagcattgccagaatgattacatacccgcgttagtagctaatcaacaaagctaaggttagtaattaaggagttctccacgggtgaggtggagtgcgtgcgccggacacgggtgcgcatccggaactgacagtttactgaaaggatatttccctgaaaagtcagaccataacgcgaaagcgcatggcgaggtagctggttcatagatagcctgtcgttaaattttcgtcgaccgtgcgcttccggttgtggcaacccgcgaaatggcgcggcggtaagtatggcggggttattccttccccgttgaggacaccgggttgtcaggttgaccatacgcttaagtgacaaccccgctgcaacgccctctgttatcaattttctggtgacgtttggcggtatcagttttactccgtgactgctctgccgccctttttaaagtgaattttgtgatgtggtgaatgcggctgagcgcacgcggaacagttaaaaccaaaaacagtgttatgggtggattctctgtatccggcgttaattgttaactggttaacgtcacctggaggcaccaggcactgcatcacaaaattcattgttgaggacgcgataatgaaaacgttattaccaaacgttaatacgtctgaaggttgttttgaaattggtgtcactatcagtaacccagtatttactgaagatgccattaacaagagaaaacaagaacgggagctattaaataaaatatgcattgtttcaatgctggctcgtttacgtctgatgccaaaaggatgtgcacaatgaattcagcatttgtgcttgttctgacagtttttcttgtttccggagagccagttgatattgcagtcagtgttcacaggacaatgcaggagtgtatgactgcagcaaccgaacagaaaattcccggtaactgttacccggtcgataaagttattcaccaggataatatcgaaatcccggcaggtctttaaaacagttccgtaataaatatccggtttcattcttatatgccagcaatggcagggatttgttcatccttaaatctgtcatgaggttaaaacaaatgagtaaagtctttatttgcgccgctattcctgacgaactggcaacaagggaagaaggcgctgtggctgtagccacagccattgaagctggcgacgaacgccgtgctcgagcaaaatttcactggcaattcctggaacattatccggctgctcaggactgcgcttataaatttattgtctgcgaggataaacctggcataccccgccctgccctcgattcatgggatgctgaatatatgcaggaaaaccgctgggatgaggagtctgcttcttttgtcccggttgagactgaatccgatccgatgaacgtcacttttgacaagctggcccctgaagtacagaacgctgtcatggttaagttcgacacatgtgaaaacatcaccgttgatatggttattagcgcacaggaattgttgcaggaagacatggcaacattcgacggacatatcgttgaagcgttgatgaaaatgccagaagttaacgccatgtatccggagcttaagttgcacgccattgggtgggttaagcataaatgtattcctggtgctaaatggcccgaaattcaggcagagatgcgcatctggaaaaaacgtcgcgaaggtgaacgcaaggaaaccggaaaatacacgtctgttgttgatctcgcccgcgccagagccaatcaacagtacactgaaaattcaacaggaaaaatcagcccggtcattgctgccattcatcgcgaatacaagcagacatggaaaacactggatgacgaactggcctatgggcgctgcttcgcagacaggcagaacttgatggtatgcctgcgatcaatgccaaacgtgtttaccggatcatgcgccagaatgcgctgttgcttgagcgaaaacctgctgtaccgccatcgaaacgggcacatacaggcagagtggccgtgaaagaaagcaatcagcgatggtgctctgacgggttcgagttctgctgtgataacggagagagactgcgtgtcacgttcgcgctggactgctgtgatcgtgaggcactgcactgggcggtcactaccggcggcttcaacagtgaaacagtacaggacgtcatgctgggagcggtggaacgccgcttcggcaacgatcttccgtcgtctccagtggagtggctgacggataatggttcatgctaccgggctaatgaaacacgccagttcgcccggatgttgggacttgaaccgaagaacacggcggtgcggagtccggagagtaacggaatagcagagagcttcgtgaaaacgataaagcgtgactacatcagtatcatgcccaaaccagacgggttaacggcagcaaagaaccttgcagaggcgttcgagcattataacgaatggcatccgcatagtgcgctgggttatcgctcgccacgggaatatctgcggcagcgggcttgtaatgggttaagtgataacagatgtctggaaatataggggcaaatccacaggtgaactacgctcctctgtttgttacgcaataaaaactggtgttttcgactatgcaaaacagtttccctcctcacgcaatctggaaaaatttggtgaggcccgacaagatttaaccataaaagaactggctgaaaaatttctggcactgaaagaaactgaagtcgccaaaacatcactcaacacataccgtgccgtcatcaaaaatatcctgagcataatcggtgaaaaaaatcttgcctcatcgattaataaagaaaaattactggaggttcgtaaagagttactgactggataccagatccccaaaagtaactatattgttacacaaccagggagatcggctgtaactgtaaataattacatgacaaatcttaacgccgtgttccagtttggtgttgataacggttacctggcagataatccgtttaaggggatctcgccattaaaggaatcaagaaccattccggatcctctttcgcgggaagaatttatccgtcttatcgatgcgtgcagaaatcagcaagcaaaaaatttatggtgtgtttctgtttatactggagttcgccctggtgagctgtgtgcacttggatgggaggacatagatctgaaaaatggaacaatgatgatcaggagaaatttagcaaaagaccgtttcacggtaccaaaaacacaggcgggaaccaatcgggtcattcatcttattaagccagcaatcgacgctctccggagtcagatgacattaacgagactgagcaaagagcatatcattgatgttcacttcagagagtatggcagaacagaaaaacaaaaatgcacctttgtttttcaacctgaagtgtcagcgagagtaaaaaattatggtgaccattttaccgttgactcaataaggcagatgtgggacgcagcgataaaacgtgccggactccgccatcgaaaatcatatcagtcgagacatacttatgcctgctggtcgctgacagctggtgctaacccggcatttatagcaaaccagatgggccatgcagatgcgcaaatggtatttcaggtatacggaaaatggatgtctgaaaacaataatgcacaggtagctttgttaaatacacagttaagcgagtttgccccaaccatgccccataacgaagcaatgaaaaattaatttaatatttatcaaatagttaacacgcatgactcttgaaatccataaattcaagcgcagtgcccagccatcccgatactgctgctttcaccaaatccttagtgcttctttcgtgtttttctattgtcataatggttatctctaaaaaagaggtaagatgcgtactacttactcgccgttattggtattattcagaaaaagtgagtaagactttgcagcaatgtttttgatcctgttcaaataaactaatggcatcagcaacatgctggaaatcaaacgtatgggtaattaatttttctggtttaattaaccctttacttaaccagtcgataacgatcgggaatttatttgcatttaagcgtgaagagaaaatagagagttcttttccggtaattccttgctgaatcacttcagacggttcactggagaaccccatcaatacaatacgtgccgctggagaagccagcgttacggcctctttcaggatagaaggatgacaagccgcatcgataattaatgtcggcttgatgcctttttcagtgaaaatctcgccaagcggtgtctggctgttattaatcgcccagtcagccccgctctctttcgctttttccagtcgttcatcaatgcgatcggcaacaatcacatttttaacgttatagacgccttttaatacctgaacgatcgtcaggccgattggaccggcaccataaaccagaacggtatcattttcagtcggttgaccatgtccggttacgttagccgcaatggtaaaaggttcgatcattaccgcatattgatcggccactgcttcaggaattttccacgcattttttgccggaaccacggcatattcactgaaaccaccgtcagcgtgcacacctaatacagccagtgtcgtacaaacgttcggtttacctatagagcacggatagcaatgcccacagctgaccaccggatcgacagcaacacgttcaccgactctggcgctttccacgccttcacccactgcatcaatgacgccaaagaattcatgaccaatgacgcgcggatatttcgcaaaaggattatgcccacgataaatatggctatctgaaccacaaattccggcaagtttcacttttactcgtacttcacccgctgacggggtgggtatttcacgttcgacaatcgccagttgattcggtttttcaattaatatgcttttcattatcttactccttaccagttccacagcgtgccatcttccagacgtgcgactggtagataagcaggttcatagggatatttcgccgccagcttttcatcgaattcgataccaagacccggtttgtctcccggatgcatatagccgttatcgaaagtccagttgtgcgggaagacttcgagcatttgttcggaataacccatgtattcctggacaccgaaattggggacccacagatcaaagtgcagcgccgcagccatgcagactggtgacaaatcggaaggaccgtgtgagccagtacgtacctgatacagcgaagcaaaatcggcaatccggcgcataccggtaattccgcctgcatgggtcagcgtggtgcggatataatcgatgagttgctcttcaatcagttgtttgcagtcccagatgctgttgaagacttcacccactgcgatgggtgtgacggtatgttggcgaatgagacggaagcattcctggttttccgcaggcgtcgggtcttccatccagaacatgcgataatcttcaatgcttttaccaaagcgcgccgcttcaataggcgttaagcgatggtgcatgtcatgcagcaaatgttcattaaaaccaaacttgttacgtaccgcgtcaaacaatttcggcatgaaatcgaggtatttctccgtcgaccacagctgctcttccggccactgtcctttggttgcgggttcataagccagacctttacctttcgacatgccgtaggtggttttcataccagggattccgcactgcacgcggatggctttgaatccaagctcttgatgacgggcataatcatccagagcttcatcaatactgtgaccggtggtatggcaataaaccatcaccccttcacgagacgcgccgccgagtaactggtaaagcggcatgttggcagctttggctttaatatcccacagcgccatatcaaccgctgaaatggccgacatcgtaaccggaccgcgacgccagtaagcacctttatagaaaaactgccagatatcttcgatacggtgcgcatcgcgaccaataagctgcggacaaaggtgatcctgcaaataagaggccacggaaagctcacgtccattgagggtggcatccccaaggcccgtaataccgtcctcagtggtgatttttaatgtgacgaaattacgccccggacaggtaacaaaaacttcagcctttacgatcttcatgttcgattccttgcatcgcttgtcgtgatgcatgaaatctacgcaactgagctactaccatacaagtataaagatcgaaaaaagccggagtgatcacaaaaaaaggcgtatatttgcgctgtgaatggttgacaaaagatgaaatagaataccttttgtcagctgacacttcctcttatcttattgataaaatggatttatgttcctacgtgcgcccccagcccgcaacaatgatcaacatgccgcaaagcgcaatcaacgcacccgtccagtcataaagagtcagtttcacgccatccacaacgcgcagccacatcaacgccgtgcagacataaacgccaccataagccgcgtaaacacgcccactcgccgctggatgcaacgttaacaaccagacaaacagcgccagtgaaatccccgccggaagcaacagccagatactggcgtttcgttttaaccacaaccagggcagaaagcatccaataatttcacacagcgcagtagcaaaaaatagtaacgttgttttaatcatctttgtctcttattgacatcatgtatagttatagggcgacataatatcatcaatataaacaccctcctggtacgttttgcgtccgcagtggatggtgtagaatcacctttaatcattcatacagggaatgaattatgaaaatcactctcagcaaacgaatcggcctgctcgctattctgctgccttgcgcactggcattgagcacaactgttcatgccgaaactaacaaactggtgattgagtctggcgacagtgcacaaagccgccagcacgccgctatggaaaaagagcaatggaatgacacgcgcaatctgcgccagaaagtgaataaacgcactgaaaaagagtgggataaagccgacgccgcttttgataaccgcgataaatgtgagcaaagcgccaacatcaatgcctactgggagcccaatactttgcgctgcctggaccgtcgaactggccgcgttattaccccctaacctgttattgatttaaggaatgtaaggacacgttatgccaagcgcccacagtgttaagctacgcccgctggagcgtgaagatttacgctatgtacatcaactcgacaataacgccagtgtgatgcgttactggtttgaggaaccctacgaagcctttgttgaactctctgatctgtatgataagcatattcacgatcagagcgaacggcgctttgtggtggaatgtgacggcgaaaaagccggtctggtggagctggtggaaattaaccatgttcatcgccgcgcagaatttcagataattatctccccggagtatcaggggaaaggtctggcaacccgtgccgccaaattagcaatggactatggctttaccgttctcaatctctataagctgtatctgatcgttgataaagagaatgaaaaagcgattcacatttaccgcaagcttggcttttcggttgaaggtgaattgatgcacgagttctttattaatggtcaatatcgtaatgccattcgcatgtgtatattccagcatcagtatctggcagagcacaaaacaccgggtcagactctcctgaagccgaccgcacaatagcattaataataatcgatcgtatttttgatggtgtaaacccgttcgacggcgggttttactccttcatcaacaatgattagctgacagtccaccggattagcgtgactgtcatattcacagctctgttttacattaccaacccgttgattattcagtaaagtaaccgctgtgtaatctaattttttgatcggatccgttgatggcgtggcgctgacagataatgttttgtcgttacttttcgtggttttacccagcggataaccctgatcatcatagcgatattccatctgcatttgtttgctgctggctttaatcacgaagccattatcatcggtttcccaactcaccccggcagaaggtaattctgctagctggcattttccctgtaaacgtactctcttctccagcgtctcggcatcacggtaataattggcgtccagtaccagagcgaccacggtattattttccagatccagtaattcgagtgaatcaaaacagccttcttccgacaaagtcccagaaacacgtttcgtcacttcaccttgctcatccattaatgtctgagtgaaatcttttaccggaccacgcagcggatcaaaatcgaattcattagagaaactggccatctcaggggtaaatgaaagtgttacctctgtgcggtcacatcctgtgaggaatatcgcgagtaagcatggtagtaatttgtatttcacaacagtcaccagagagtagagatgattctcaatcatagtagcaaatacagtactttacacgttaaatgctatgcttaaagaagttatcttcgcgtaaggagcttatgatgaaactctcaacctgctgtgccgcgcttctgctcgccctcgcctcacccgcggtactcgccgcgccgggatcctgtgagcgcatacagagcgatatatcacagcgcattatcaataatggcgtacccgaaagcagcttcacgttaagtattgtacccaatgaccaggttgatcagcctgattcccaggtcgtcggccattgcgctaatgatacgcataaaattctctatacccgcaccaccagcggtaacgtctctgctcccgcgcagtctagccaggatggcgcgcctgccgaaccgcagtaacacattatcgactgaacgccggatatgacaaatccggcgatttgaacatacaacataatcccaccttattactcatacccttctattgatatggattaataattcttaacccaaaatgggtagactccctctattgttagcgcgctaaatattcaatatataaacttttatataacgataaagaacagggagtgagttatgtccaaaaatgaacgaatggtgggcatcagccgcagaacactcgttaaatctaccgcgataggttctctggcgctggctgcaggcggtttttctttgccgtttaccctgcgcaatgcagcagcagcggtacaacaggcccgcgaaaaagtggtctggggtgcctgttccgtcaactgtggtagccgctgtgcacttcgtctacatgttaaagataatgaagtgacctgggtggaaactgacaataccggcagcgatgagtacggcaaccatcaggtacgcgcctgtttgcgcggtcgctccatccgccggcgtattaatcatcccgatcgcttgaattacccaatgaaacgcgtgggcaaacgcggcgaaggcaaattcgaacggattagctgggatgaagccctggatactatcgccagtagcctgaagaaaaccgtcgaacaatatggcaatgaggctgtatatattcagtactcttcggggatcgttggcggcaatatgacccgctcttcgccatcagcctcggcggtcaaacgcctgatgaactgctacggcggttcactcaaccagtatggctcctacagcactgcgcaaatttcctgtgccatgccctacacctacggcagtaatgatggcaacagcaccacggatattgaaaacagcaagctggtcgtgatgtttggtaacaacccggcagaaacccgcatgagcggtggtggcatcacttatcttcttgaaaaagcgcgcgagaaatcgaacgccaaaatgattgttatcgatccgcgatataccgatacggctgccggtcgtgaagacgaatggctccctattcgcccgggcaccgatgccgcgctggttgcgggtattgcctgggtattgattaacgaaaatctcgttgatcaaccttttctcgataaatactgcgtcggctatgacgaaaaaaccttacccgcagatgcacccaaaaatggtcactataaagcctatattcttggtgaaggtgacgataaaacagcgaaaacgccgcagtgggcttcgcaaattaccggtatcccggaggaccgtatcatcaaactggcgcgtgaaattggcacagcaaaacccgcttatatctgccagggctgggggccacaacgccaggcaaacggcgaactgactgcacgcgctattgctatgttacctattttgacgggcaatgtcggcatcagcggcggaaatagtggcgcgcgtgaatcgacctataccattaccatagaacgcctgccggtgctggataatccggtcaaaacgtcaatctcctgcttcagctggacagatgctatcgatcatggtccgcaaatgacggcaatccgcgacggcgtccgcggcaaagataaactggatgtgcccattaagttcatctggaactacgcgggaaataccctcgttaatcagcattctgacatcaacaaaacgcatgaaattctgcaggacgaatcgaaatgcgaaatgattgtggtcatcgaaaactttatgacctcatcggcaaaatatgccgacattctgctgccagacctgatgaccgttgagcaggaagatattattcctaacgactacgccggtaacatgggatatctcattttcctccagcctgtcaccagcgaaaaattcgaacgcaaaccgatttactggatcctgagtgaagtcgcgaaacgtcttggacctgacgtctatcaaaagttcacagaaggtcgcacgcaggaacaatggttacaacatctgtacgccaaaatgcttgccaaagatccggcgttaccgtcttacgacgaactgaaaaaaatgggtatctataagcgtaaagatcccaatggccattttgtcgcctacaaagcatttcgtgacgaccccgaggcaaatccacttaaaacgccttccggtaagattgaaatttattccagcaggctggcggaaattgcccgtacctgggaactggaaaaagatgaagtgataagcccattgccagtttatgcctcaacctttgaaggctggaactcccctgaacgtagaaccttcccactgcaactgtttggtttccattacaaatcccgtactcactcgacctacggcaatattgatctcctgaaggctgcctgccgtcaggaggtgtggatcaaccctatagatgcgcagaaacgtgggattgccaacggcgatatggtgcgggtgtttaaccatcgtggcgaagttcggctaccagccaaagtaacaccacgtattctccctggagttagcgctatgggccagggagcctggcacgaggccaatatgtctggcgataaaatcgaccatggcggctgtgtgaatacgctaaccactctgcgcccttcaccactggcgaagggaaacccgcagcacactaatctggtcgagatcgaaaaaatataacccacgacaaccataaattctggcatgacattttgtttgaaaagcaataagtgagtaatgatgaaaatccataccacagaggcgctcatgaaggctgaaatcagccgtagaagtctgatgaaaacctccgcacttggcagtcttgcgctggcaagcagtgctttcactctgccattttcccaaatggtccgggcggcagaggctccggtagaagagaaagcggtctggagttcctgcaccgttaactgcgggagccgctgtctgttacgtttgcatgtgaaagatgacaccgtgtactgggtggagtctgatacgacaggtgacgacgtctacggtaatcatcaggttcgagcgtgtttacgcgggcgctctatccgccgacggatgaatcatcctgataggttgaaatatcccatgaagcgcgtcggcaagcgcggtgaaggtaaatttgaacggataagttgggacgaagccctggataccatcagtgataatcttcggcggatcctgaaagattacggcaatgaggctgtacatgtcctgtacggaacaggcgtagatggcggaaacatcaccaactcaaacgtcccgtaccgtctgatgaactcttgcggtggttttctcagtcgctatggcagctacagtaccgcacagatcagtgccgcaatgagttatatgttcggtgccaatgatggcaacagcccggatgatatcgccaatacgaaactggtcgttatgttcggaaataacccggcagaaacgcggatgagcggcggtggtgtcacttactacgtcgagcaagcccgcgaacgttcaaacgcacgcatgatcgtcatcgatccacgttataacgacactgctgccgggcgtgaagatgaatggctgcccattcgccctggcaccgatggcgcactggcctgtgcgattgcctgggtactgattactgaaaacatggtcgatcagccatttctcgacaaatattgtgttggttacgatgaaaaaacgctgcccgccaacgcaccacgtaacgcgcattataaagcctatattctgggcgaagggcctgacggcatagctaaaacgccggaatgggcagcaaaaatcaccagcatcccggcagaaaaaattatccagttggcacgagagatcggttcagcaaaacctgcttatatttgtcagggttgggggccacaacgacattccaacggcgagcaaacatcccgcgctattgccatgctttccgttctcaccggcaacgtcggcataaacggcggcaactcaggcgtacgcgaaggtagctgggatctgggggtagaatggttcccgatgctcgagaatcctgttaaaacgcagatttccgtctttacatggacagatgccatcgaccatggtacggaaatgaccgcgacccgtgatggtgttcgtggaaaagaaaaactggatgtccccatcaagtttttatggtgctacgccagtaacacattgatcaatcaacatggcgacatcaatcacacccatgaggtgcttcaggatgacagcaagtgcgagatgattgttggcattgaccacttcatgacggcctcggctaagtattgcgatatcctgttgcccgacctgatgccaacagagcaagaagaccttatctctcatgaatctgcagggaatatgggctatgtgatcctcgcccaacccgcaacctcagcaaaatttgaacgcaaacccatctactggatgctgagtgaagtcgccaaacgcttaggaccagacgtttatcaaacctttactgaaggtcgcagtcagcatgaatggatcaaatatctccatgcgaaaacgaaggaacgtaaccctgagatgcccgactacgaggagatgaaaacgaccgggatctttaagaaaaaatgcccggaagaacactacgtcgctttccgcgcattccgtgaagatccacaggcaaacccgttgaaaacaccttcggggaaaatcgaaatttattctgaacgactggcgaagattgcagatacctgggaattgaaaaaagatgaaattattcatccccttcctgcgtataccccaggttttgatggctgggacgatcccctgcggaaaacctatccactgcagttaacgggcttccattacaaagcgcgtacccactccagctacggcaatattgatgtgttacagcaggcctgcccacaagaggtgtggatcaaccccattgatgctcaggcacgcggtatccgtcatggcgataccgtgcgggtatttaacaataatggagaaatgctgattgccgcaaaagtgactccgcgtattctgcctggcgttaccgccatcgggcaaggtgcgtggcttaaagcggatatgtttggtgaccgggtcgatcacggcggcagtatcaatattctgacctctcaccgcccttcaccgctggcaaagggaaacccgtcgcacagcaatcttgtccagatcgaaaaggtttaaggagtagcccatgaccacacaatatggattttttatcgattccagccgctgtactggctgtaaaacctgcgaactggcgtgcaaagattttaaagatcttggcccggaagtcagtttccgccgtatttatgaatacgctggcggcgactggcaggaagataatggcgtctggcaccagaacgtgttcgcttattatctctccatctcctgtaaccattgcgatgaccccgcatgtacaaaagtctgccccagcggcgcaatgcataagcgtgaagatggctttgtggtggttgatgaagatgtttgtatcggctgccgctactgccacatggcttgtccgtacggcgcgccacagtacaatgctgaaaaagggcacatgacgaagtgcgatggttgttattcgcgcgtcgccgaggggaaacaacccatatgtgtcgaatcctgcccgctgcgtgcacttgagttcggtccaattgaagagctgcgccagaagcacggcactcttgctgccgtcgcgccactgccgcgcgcgcatttcacaaaacccaatatcgttatcaaacctaacgccaacagccgcccgaccggcgataccactggttatctggctaatccggaggaagtgtaaaatgggaaatggatggcatgagtggccactggttatctttaccgtattgggtcaatgcgtagtaggcgcgctgattgttagcggaattggctggttcgccgccaaaaatgacgcagaccgtcagcgtattgtccgtggcatgtttttcctctggctgttgatgggcgtcgggtttattgcctctgtcatgcacctgggatcgccactgcgggcgtttaactccctgaatcgaatcggagcttctggtctgagtaacgagattgctgccggttccatattttttgccgttggcggattatggtggctggtggcagtcatcggtaaaatgccgcaagcgttggggaaactctggttacttttcagcatggcgctcggcgtcattttcgtctggatgatgacctgcgtgtatcaaatcgacaccgtgccaacctggcataacggttacactacgctggctttcttcctgacggtattgttgagcggtccaatacttgctgccgcaattctgcgggcagctcgcgttacatttaataccacaccatttgccatcattagcgttctggcgctgatcgcttgtgccggggtgattgtgctgcaaggtttgtctctggcgtctattcactcatccgtgcaacaagccagcgcactggtaccagattacgcctccttacaggtctggcgtgtggtattgttatgcgcaggtcttggatgctggctttgcccgctcattcgtcgccgtgaacctcacgttgccggacttattctggggctaatcctcatacttggcggtgagatgatcgggcgtgtgctcttttatggcctgcacatgacagtaggaatggctattgcaggttaacaaattggtgcggggcaacccgcacatttcaggatgttaggaatgacccatttttcacagcaagataatttttctgtcgcggcgcgcgtgttgggcgcgctgttttattacgctccagagagtgcggaagccgcacctctggttgcggtactcaccagtgacggctgggaaactcagtggcctctaccagaagcgtcattagcgccgctggtgacggcttttcagacacagtgtgaagagactcacgcccaggcctggcagcgtttgtttgtcggcccgtgggcactgccgtctccgccgtgggggtcggtctggctggatcgcgaatctgtgctgtttggcgattcaacattggcacttcgtcagtggatgcgcgagaaaggcattcagtttgaaatgaagcaaaacgaaccggaagatcattttggttcactgctgttgatggctgcgtggttggcggagaatggtcgccagacagaatgcgaagaattgctggcatggcacctttttccgtggtcaacacgttttcttgatgtttttatcgaaaaagcagaacaccctttctaccgtgcactgggtgaactggctcgcttaacgctggcgcaatggcaatcacaactgttaattcctgtcgcggttaaaccgctgtttcgataggatcaccgtaatattgccggatggtgacgattacgcgcaatccggcaataataggttacagtgtcacgtttttttatctcttaaagcacgcactgcttttgcggctggcctcttttgccgcaaaatagtcgcccgtgtttcattgcccatttctgctcatgcatcatctacacatctatccggatctgcgcactatgttccaccgtctgcttatcgcaacagtcgtcggtattctcgcggcctttgccgttgccgggtttcgtcatgcgatgctgctactggagtggttgttcctcaataatgactccggcagtctggtcaatgcagcgacaaacctttccccctggcgacggttgctaactccggcgctcggcggactggcggcgggtttgttgctgatgggctggcagaaatttacccaacaacgccctcatgcgccgaccgattatatggaagcgttgcaaaccgatggacagttcgattacgcagcaagcctggttaaatcgcttgcctctctgctggtagtaaccagcggcagtgcaattggtcgcgaaggtgcgatgattcttttagctgcccttgccgcctcctgttttgcccaacgttttacgccacgccaggagtggaaattatggatcgcctgtggggccgcggcgggaatggctgcggcctatcgtgccccgcttgctggcagtttatttatagccgaagtgctgtttggcactatgatgttggcctctctcggcccggtgattatttccgccgtcgtggcattgctggttagcaatctgattaatcatagcgacgcgttactctacaacgtacaactctcagtgacggttcaggctcgtgactatgcgctgattatcagtacaggtgtgctggcaggtctgtgcggaccactgttgttaacgttaatgaacgcctgtcatcgtggatttgtgagtctcaaacttgcgccgccctggcaactggcactaggcgggttgatcgtgggtctgctttccctgttcacacctgcagtgtggggcaacggctatagcaccgtacaatcctttttaaccgccccaccactgttaatgatcattgccgggatcttcctttgtaaactgtgtgccgtgctggcgagtagcggttccggcgcacccggtggggtctttacaccgacgctatttatcggtcttgccattggcatgttgtatggtcgtagcctgggattatggttccctgatggcgaagaaattacacttttactcggattgaccgggatggcgacactgttggcggcgaccacgcacgcgccgattatgtcgacgttgatgatatgtgaaatgaccggggagtatcagctactccccggtttattgattgcctgcgtaattgcgtcggtaatttcgcggacgttacaccgtgactctatctaccgccagcacactgcgcagcatagctaagcggatgtattgccccagttcacgctgttcggcgcgcggcagataaggcagttcaccaatgagcggtgccggaagttttttacccagcacatcaatgatttccgcataatgcgccagtcctgggttgattcggttagccacccagccaatgagcggcagcccgtcgttggcgatcgcctgagctgttagcagtgcatggttaatgcaaccttcctgaataccgacaaccatcaacaccggcagttgttcctgcactacccattcagagagtggacgcaaatcattcatcagactgcgccagccgccagtcccttctaccacgacatgatcgactttttcggtcaggtttgccaggccgtttgaaatgagggtgtaattgattgggcaactgtgcgccacgctactttcttcttcgcttaacgcgataggattaactgcttcataaggcagttcgatggttgaaacactctgcaacaccagggcatctttattacgcagcccttcgggtgtctctttgctccccttcgctacgggtttatatcccgcaaccgtttttccctgggaggctaacgcttgtagcaatgcgcgggaaaccaccgttttccctacagaagtgtctgtaccggtaataaagaaacgcttcagcatcactaactccaccgttatgcttcacaaatataaaccaggaaaataattaaccttgaaagtctaagttatgctttcctggcccaaattgagatagcgcaaattttggtagaacagttaaaaaatgttaaccctgcaacagacgaatcaacaaagaaccgttatacatcgcgtcttttaccagtgcagcgcctgccatcgtgccctggttagaaaactgagtactctcaacgctgatgtgctgactatacgcaggaagggcctgctgacggatgctgtctgagatgaccgggaagaggatatctgccgctttacttaacggtgagccaatcagtattttttgtgggttaaataaattcaccatgatggcaagaatgcgcccgacatgcgcgcccaccccggtaatgatgtcttttgccagtagatcgccgcgcaatgccgcctgacacaatgagtccacggttaacggttgtccatgtaacatcgagctcatggattgattaagacgcagctgtgccagctcaagaatactgtccacgctggcgatggtttcgaggcagccgtgattcccgcaataacagcgtttcccatacgggtcgacctgtgtgtggcctatttccacgagactactgctgcctgcgtgtagcagatgaccatcggtaatgacgcccgcccccacgttgtgatcgataaccacctgaatcacatcgcgcgccccgcgtgaggcaccaaacaaggcctctgccatcgtccatgcgctgatatcatgctgaatataaaccggaacgccggtatgctgctccagcgcctcgccgagcggcatctcttttacatcctcgtagaacggcatgcgatgtacaataccattttccgtatcaataattcccggcaaggttatggcaatcgaagttagacgctcaagttttttctggtggcggataaaaaactgatcgatatgggaaataatacgatccagcaatggcaagtcatcttttaacgccagttcctgcgactcttccaccaccagtttgctgctcagatcgcgcagagcaaggaaaatctccccgcgactaatgcgcagagaaagatagtgccaggcttcagtttcaaccaccagccccaccgccggacggccacggttccccgcttctttgatttccagctcttgcaccaggtgtgcttcgagcatctcacggacaattttagtgatactggcaggagccagttgcgccagacgggaaagatcgatacgcgagactggaccaagctgatcaatcaggcgataaaccgcgcccgcgttggtctgctttatttgatcaatgtgcccaggctggttttcagcaaccaccgcatactccctatattttcgcgctccgaaataatctgtaggctatggtgaagcacttcaatacgtgtcgtcaaatttttacttaggcatgtgattaacagcacatttttcgggctttttcgctgaaatttccctcacctgagagcattcagcagatgaatacgaaagttacgcgcagccggactttgttcatgatgtttcggccagaccaaccacatttcagaaaccgcatcctcttcagcaatcggcacccagcgcatttcgttgagctgaacacgtttaaatgacgcaggcaaaattgaaacacccagaccggcggaaaccagaccgatgatggtcattgcctcgcccacctcctgagtgatgacgggcgtcaaatggtaacgtcgcatcagcccgagaatatcgtcatacagccctgtcccgacgtgcggatcaaaaaagacaaagggttctttcgccagttcagccagcgttacattcgggttatttgccaggggatgatcgtgcgggatcatcgccataagcggttcatggacgatgactgcgtgttcaagcgactccggtaacgctgtgttacgcagcaatcccatatccagcgttccttcaatgagcggagcgatttgctcgcgagtgttcatttcgcgggtttgtaaatggacatcaggataatcacggcgaaacagcgataacgtatcggacaccgcccgaataaaaggagccgacgaagtaaaaccaatgcgcaactcccccgcttcaccctgatgcagcctttcagcgcgagcggcagcgtcatccaccatagacaggatttgccgactatctgcaagaaactgttttcctgctgccgtcagcaatacactgcgattggttcgtgccagcagtcgggcaccaatttgttgctccagcgcctgaatctgctgacttagcggcggttgcgaaatattcaggcgggcagcggcgcgcccgaaatgcagctcttccgcaacagcaacaaagtaacgcagatgacgaagttcaatattcatatttaaaacatcttatttgagattattaatatattagacagaacaattcgattttcctaccctatgtataagcctgatctacaggcatatttagcaaggatttcaagtgagccgtactacaactgttgatggcgctccggcaagcgacactgacaagcaaagcatttctcagccaaatcaatttattaaacgcggtacgccgcaatttatgcgcgtcaccctggcgctgttctctgccggactggcaacatttgcacttctctattgtgtgcagcctatccttccggtgctttcgcaggagtttggcttaacccccgcgaacagtagtatttcactgtccatttccacggcgatgttggctattggtttgctgtttactggcccgctatccgatgccattggtcgcaaaccagtgatggtcacggcgctactgttggcctccatttgtacgttactttcgacaatgatgaccagctggcacggcattttgattatgcgcgccttgattgggctttcgttaagtggcgtggcagctgttggcatgacttatcttagcgaggaaatccatcccagtttcgtggccttttcaatggggttgtatatcagcggcaactcaattggcggcatgagcggacgcttaattagcggtgtcttcacggactttttcaactggcgaattgctctggcggcaatcggttgtttcgcgctggcctcggcgttgatgttctggaaaatcctccctgaatcacgccattttcgcccgacttcgctgcgccctaagacgttgtttatcaactttcgtctgcactggcgtgaccggggattaccgttattgttcgcagaaggctttttgctgatggggtcgttcgtcacgctgtttaattacatcggctatcggttgatgctctccccctggcatgtcagtcaggccgtggttggcttattatcgctggcttatttgaccggtacatggagctcacccaaagccggaaccatgaccacccgctatgggcgtggtccagtgatgttgttttcgacgggggttatgctgtttggtttactgatgaccttattcagctcgctgtggctgatctttgccggaatgttactcttctcagcaggattcttcgcagcccactcagtagccagcagctggatcggcccccgcgcaaaacgcgctaaaggccaggcctcctcgctgtatctgttcagttactatctggggtcgagtattgccgggacgctgggtggtgttttctggcataactatggctggaacggcgtcggcgcatttattgctctgatgctggtcattgctctgctggtcgggacgcgtttgcatcgtcgtctgcacgcctgaaaaataagtccggactgcggtaaatacccgtccggacttattgccagctcaaaccaacgttaatagccatcctaaaatagacgaagcgccagccaattcccgcagcgcgtctagcgtcatcaggattataagtacccaaataaacggattcattttgctgtgtgtcatttattactgatgcgcagttattctactgctttgtaagtagtaaaatagttaacccgatcaagactactattattggtagctaaatttcccttaagtcacaatacgttattatcaacgctgtaatttattcagcgtttgtacatatcgttacacgctgaaaccaaccactcacggaagtctgccattcccagggatatagttatttcaacggccccgcagtggggttaaatgaaaaaacaaattgagggtatgacaatgaaaaaagtattagctctggttgttgccgctgctatgggtctgtcttctgccgcctttgctgcagagactacgaccacacctgctccgactgcgacgaccaccaaagcagcgccggcgaaaactacacatcataaaaaacagcataaagcagcacctgcccagaaagcgcaggcggctaaaaagcatcataaaaatacgaaagctgaacagaaagcccctgaacaaaaagcgcaggcagcgaagaaacacgccaagaaacacagccatcagcaaccggcaaaacctgctgcacaacccgcagcgtaagttttcaacagtaatgctggcgcgccccctcgcgcctgaaaattacggtgctaagcgggtaacgtttagcaccgcctttagcggagggtagtatggtgggccgttatcgctttgagttcattctgatcatccttattttatgcgcactgattaccgcccgtttttatctttcctgattgtagttatctgattttactcccactttcatcccgtcccgtctatagtatttatgagggtttgcttttaataatcataattacccaccagagtgtgatatgcgtacaaccattgctgtagtgttgggtgcaattagtttgacgtctgcttttgtgtttgcagataaaccagacgttgccagatcggcaaacgatgaggtcagcaccctgttttttggtcatgatgatcgtgtgccagtgaatgacacgacccaatcaccgtgggatgcggttgggcaactggaaacggccagcggcaatttatgtacggcgacgctgattgcacccaatctggcattaacggcaggacactgtttattgacacctccaaagggtaaagccgataaagcagtggcgctgcgttttgtgtcaaataaaggtctttggcgctatgagatccacgacatagaaggccgcgttgatccgacactgggaaagcggttaaaagcagatggggatggttggattgtacctcccgcagccgcgccgtgggacttcggattgattgtgctacgtaatcccccttctggcattacgccgttgccgttatttgagggagataaagccgcgcttaccgccgcattaaaagcggcaggtcgtaaagtgactcaggcaggctaccctgaagatcatctcgatacgttgtacagtcatcaaaactgtgaagtgactggctgggcgcaaacgtcggtgatgtcacatcagtgcgataccttgccgggtgacagcggttcgcctctgatgttgcataccgatgacggctggcaattaattggggtgcaaagttcggctcctgccgcgaaagatcgctggcgcgccgataaccgggccatttctgttaccggttttcgcgacaagctggatcaactgtcgcaaaaataatgttcaaacgctgcccgacagcgcgggcagcgtcttcatcaggcaagtttcaccatgatcattccagccaacagcaagaccaggccaatccagcctttacgatttaaccgttgaccaaacaagatccaacctgcggctaacgtggcggcaataccaaacccgccccacaatgcataagcgacagacaagtcgatccctttaacggcttgagaaagcgcactaaaggcagccagcaccgccgccagggagagcaagccaaatattttgcgacgaaagccgtcagaaaatttcaaaaagacgttagcaacgatttccagcacgattgccaatgccagccaggcggcgtgaacccattcaaactgcgccatggttcacctccagttcaggtttacgcgctttacgggtacctgattttatcaacacaatcccggcgaccagggtggttaacccggcaattttcatcagcgataaactttcgtcgaataacaaaacgctaaacaaggtaataaataaaataccgataccttcccacagcgcataagctacgcctaaggcgatttttttaacggcgaaagagagaaatatatacgacagagaaatcatcaccagcattaaaataaagccgccatttccctcactgacgctcgcccatttcattgacagcgtaccggtaatttctgtagcaatagccagacctaataaaatccaataaatatacattgtccttctcctgcaagagaattattttaattttcgcttaattcagcgaaaccaaagtaaagtggtcaagccccgcgcatagcgcaagctttggcagaagaaaggactaaagcgcgttgcgccagtgctgctcacctacgagcaagatagtggatgaggtacgaagatgggtaaatgtagaaaataacgtcctgaacaaattgtccataatattacaattatccgcagtgttgcttctcgtcatcgcggatgataattgtcctcggtagttgaacacgcctgatttgtatcatagcttaagaattaactcaaaatattttcacttctttacctgagcggtttgattttcgttatgatgacggagcgaaaaagacattattattagcaaaggaagaaaaaacggggacaagcatggcaaagccgatcatcacgctcaatggcctaaaaatcgtcattatgttgggaatgctggtcattattctctgcggtatccgttttgccgccgagatcatcgtgccgtttattctcgcattatttattgctgttattcttaacccgctggtgcaacacatggtccgctggcgtgtgccgcgtgtactggcggtgtcgattttgatgaccatcatcgtgatggcgatggtgttgctattagcttatctgggttccgcgctcaacgagttgacgcggacgttaccgcaatatcgcaactctattatgacgccgctgcaagcgcttgaaccgttgttgcaacgcgtagggattgacgtctcagttgaccagctggcgcattatattgatccgaacgcggcgatgacgttgctcaccaacttattgacgcagttatctaatgccatgtcatcaatatttttattgctgctgacggtgctgtttatgctgctcgaagtgccacaattgcccggaaaatttcagcaaatgatggcgcgtccggttgaagggatggcggcgattcaacgtgcgattgacagtgtttctcattatctggtgctgaaaacagccatcagcatcatcaccggcctggtcgcctgggcgatgctcgccgcactcgatgttcgcttcgcttttgtctggggattgctggcctttgcgcttaattacatcccgaatattggttcagtcctcgcggcaatcccccctatcgctcaggtactggtgtttaatggcttctacgaagcgttgctggtgctggcgggatatctgctgattaatctggtcttcggcaatattctggagccgcgtatcatggggcgtgggctggggctttccacattggtggtatttttgtcgttgattttttggggatggttgttaggaccggtgggtatgctgctttccgtgccgttgacaattattgtcaaaattgcgcttgaacaaacagcgggaggtcaaagcatcgccgttctgttaagcgatctcaataaagagtgacggcctcagcagaggccgtcagggttacagagctttcaggattgcatccacgctggctttggcgtcaccaaacagcatgtgggtgttttccttgaagaacagcgggttttgcacaccagcatagccagtgttcatcgaacgtttaaagacaatcacgttctgcgctttccacacttccagcacaggcataccagcaatcggactcttcggatcatcctgcgccgccgggttaaccgtatcgttagcaccaatcaccagtacggtatcggtatcagcaaagtcatcattgatctcgtccatttccagcacgatgtcatacggtacttttgcttcagccagcaatacgttcatatgtccaggcaaacgccccgcgaccgggtggataccgaaacgcacattaataccacgagcgcgcaatttctcagtaatttcagcgacaggatattgcgcctgcgcgactgccatgccgtaccccggagtaatgatcactgaatgggagtttttcagcagttccgctgtctcttctgcggtgatttcgcggtgctcacccacttcctgatcatcgccagtagaagagccgtcggtgccgaaaccacccgcaataacgctgataaaggaacggttcatcgccttacacataatgtaagaaaggatagcccccgaagaaccgaccagcgcaccggtcacaatcagcaggtcgttgctgagcataaagcccgcagccgcagccgcccagccggagtacgagttcagcatcgacaccaccactggcatatctgcaccaccgatggaggcgactaaatgccagccgaataccagcgcaattgcggtcattatcagcaatgccagcacttgcaggccgacgctgtccgtgcgaacaaatacaatcagcagcaggaaggaaacgaccagagccgccaggttcattttgtgacggtttggcagcatcaatggtttagacgaaatcttgccacacagtttgccgaacgccaccaccgaacccgtgaacgttaccgccccgatgaagataccgaggaacacttccgtcaggtgaatattgaccagaatcggtgccattcccgcgtcatgatgcagatagctgttaaagccaaccagcactgccgccagacccacgaagctatgcaggatcgccaccagttctggcatttcggtcatttcaactttcttcgccagacggataccaattgccccaccaatgaccatcgccagcaagatccagccaacattacccgtatccggtccaaaaatggttgcgattaacgcaatcgccatcccggcgataccgaagttgttaccctggcgagacgtttcatgtttcgaaagaccggccagactgaagataaacaggatcgcggcaacaatgtatgcagctgtaactaatcctccagacatatgttaccccttaatttttgcggaacattttcagcatgcgctgagtcacggtgaagccaccgaaaatattaatgctggctataagcaccgcgataaaactaaggaagctaacccagccgccctggccaatctgcaacagtgctccgacaacaataatccctgaaatcgcgttggtgaccgacatcaacggtgtatgcagcgcgtgcgatacattccacaccacgtaataaccgacaacgcaggccagcgcgaaaacggtgaagtgcccaaggaattctttcggcgcaacgcttgccatccagccaaaaagaatgattgccagcgccatcaacgcgtatttacgccacggtgagcaggtacatttttcctcagttttcacttccggtgccgctttttgtgccgcctgcggctgagctgatacctgaatcggcggtgccggccaggtaatttcgcccgcacggatcacggtcacgccgcgaatcaccacatcatcaaaatcaacagtgatattgccgtctttctctttgcacaacagtttcagcagattaacgaggtttgtgccgtaaagctgtgaggattgcgtcggcagacggcccggaagatcggtataaccaatcactttgacaccattttccgtagtgaagatttcacccggcacggtgtattcacagttgccgccgttttgggctgccaggtcgacaatcacactgcccgccttcatggagtcaaccatttcacgggtaattagcttcggcgctggtttgcctggaataagcgcggtggtgacaatgatatcgacctcttttgcctgggcggcaaagagttccatttccgctttgatgaacgcgtccgacatcactttggcatagccatcgccgctgccagcttcctctttaaaatccagctcgaggaattccgcgcccatactttgaacttgttctttcacttccgggcgggtgtcgaatgcacgcacaatcgcgccgagactgtttgctgcgccaatggcggccagacctgcaacacccgcaccaatcaccatcacttttgccggtggcactttcccggccgcagtaatttgcccggtaaagaagcgcccaaattcatgtgccgcttcaacaatggcgcgataaccggcgatgttcgccatcgagcttagtgcgtccagcgattgtgcgcgtgagatacgcggcacagagtccatcgccatcacggtcacgttacgttccgcaagtttttgcattaattccggattctgcgcaggccagataaaactcaccagcgttgtcccaggattcagtaacgcaatttcatcatctaacggcgcattgaccttcagaatgatctctgactgccagacgctattcccttctacaatttcagcgcccgcttgcacaaacgctttatcgtcaaaacttgccagttgacccgcgccgctctctaccgcgacggtaaaacccagtttcagcagctgttccactgtttttggcgttgctgcaacacgggtttcattggttaaccgttctcttggtatgccaattcgcatgatattcccttccatcggttttattgatgatggtttgcctgtgtcaggagccacacaagctgctcatgtacgagctaaatgttactccgttaaaataaattagtaacaaacgccctataacgtactgaaaattatgcctgtgatctagcgccaaaaatcagtatttcggcgtgaactcgcaaaatattaacgattcagccgtgatagtgggataaacaccttagaacgccggataaagactgataattgtcttcgacggtcgggtaaaacgagacatcgccccggcacgaatcactacttaacattaaattaacttatacaattcagttgcttcagtagtaatgatgctgatacggctgttttttaagcatagacggtcatttgagcaggattaaaattggcttaaggaatgtgatatgaaaaatgacgcagacagttacaccgtttaaatgcaataatcagccacgtttctcgttaataacaataccagtacctggtttgcgcaaggcgaaggattatttttatgaagcttaagaacaccctcctggcgtcggcactgctttctgctatggcattctccgttaacgcagcaacagaactgacaccggagcaagcggcagcggttaaaccttttgaccgtgtagtggttaccggtcgttttaatgctattggcgaagcggtgaaagccgtttctcgtcgcgcagataaagaaggtgccgcctctttttatgttgtcgacacttctgattttggtaacagcggtaactggcgtgtggtcgctgacctctataaagccgatgctgaaaaagcagaagaaacaagtaatcgcgtaattaacggtgttgtcgaactgccgaaagatcaggctgttctgattgaaccgtttgacacggtcaccgtccagggcttctatcgtagccagccagaagtcaatgatgccatcaccaaagcggcaaaagcgaaaggtgcctactctttctacatcgttcgtcaaatcgatgccaaccagggcggcaaccagcgtattactgcattcatctataaaaaagatgctaagaaacgtatcgtccagagcccggatgtgatcccggcagattccgaagcaggacgtgcagctctggctgccggtggcgaagccgcgaagaaagttgagatcccgggtgttgcgactaccgcatcaccaagttctgaagtcggtcgcttctttgaaacccagtcatcaaaaggcgggcgttacaccgtcacgctcccggatggcactaaagtcgaagaactgaacaaagcgaccgcagcgatgatggtcccgttcgacagcatcaaattctctggcaactacggcaacatgaccgaagtctcctatcaggttgcgaaacgtgccgcgaagaaaggtgctaagtattaccacatcacccgccagtggcaggaacgtggtaataacctgaccgtcagcgcagatctgtataaataactattcagttactcctataaggcggcttgatgccgcctttcgcatttttagtcacaaatttccccgcgaccattgcatgcagacacatctcttcgtaaaatcccgcgcttcagtggcaaactccatttttatgcgttttgccctaatatttattcttcttatcacgttttaatcactggatatcgatggaaaagaaactgggactgagcgcactcaccgcgctggtattaagctcaatgctgggcgcgggtgttttcagtctgccgcaaaatatggcggcagttgccagcccggcagcactgctcatcggctggggtattactggcgctggcattttattgctggcctttgccatgctgatcctcacgcgcattcgtcccgaacttgacggcggtatctttacctatgcccgcgaagggtttggcgagctaatcggcttttgttccgcatggggatactggctgtgcgcagtcatcgccaacgtctcctatctggtgatcgttttttccgcgttaagcttttttacggacacgccggaattgcgcctgtttggcgatggtaatacctggcaatcgatagtcggtgcatcggctttattgtggattgttcactttttgatcctgcgcggggtgcaaaccgctgccagcattaacctggtggcgacactggcaaaattgttgccgctgggtctgtttgttgtgctggcgatgatgatgttcaaactggataccttcaagctcgacttcaccggacttgcacttggcgtacccgtttgggaacaggtgaaaaacaccatgctgatcaccctgtgggttttcattggtgtggaaggtgccgtggttgtttctgcgcgtgcgcgtaataaacgtgatgttggcaaagcgacactgctggcggttctctccgctctgggcgtttacttgctggtaacgctgctttcgctgggtgtggtggcacgtcctgaactggctgaaattcgtaacccgtcaatggccggtctgatggtggaaatgatgggaccatggggcgaaatcatcatcgctgccggtttgatcgtttccgtttgcggcgcgtacttaagctggaccatcatggcagcagaagtaccgttcctggccgccactcataaagcattcccgcgcatttttgcgcgccagaacgcacaagctgcgccatccgcctcactgtggttgaccaacatctgcgtgcaaatttgtctggtactcatctggctgaccggttccgattacaacacgttgctgaccatcgcctcagaaatgattctggtgccctatttcctggtcggcgcgttcttgctgaaaatcgcaacccgtccactgcataaagcggtaggtgtcggtgcctgcatttatggcttatggttattgtacgcctctggtccaatgcacttgctgttatccgttgttctgtatgcaccggggctgctggttttcctgtacgcgcgcaaaacgcatacccatgataatgtactgaaccgtcaggaaatggtgctgattggcatgctgttaattgcctcagttccggcgacctggatgctggtgggataacgttcatcccatcgttggatagcaaaggagataacgatgggtaaaacccagcccttgccaatattaattactggcggaggtcgtcgcatcggcctcgccctcgcatggcatttcattaatcaaaagcaaccggtgattgtcagctatcggacacactatccagccattgatggactgattaatgcaggtgcgcagtgtattcaggctgatttttcgaccaacgacggtgtgatggcgtttgccgatgaagtactaaaaagcacccatggtctgcgtgctattttgcataacgccagtgcgtggatggcggaaaaaccgggtgcgccactggccgacgtactggcttgcatgatgcagatccacgttaataccccatacctgctcaaccatgcgctggaaagattactgcgtgggcacggacacgccgccagcgatatcattcactttaccgattatgtggtggagcgcggtagcgacaaacatattgcgtatgctgcaagcaaagcggcactggataatatgacccgctcgtttgcccgcaagctggcaccggaagtgaaagtgaattctattgcgccatcgctgatcctgtttaatgaacatgatgatgccgaatatcgacaacaggcgctgaataaatcactgatgaaaaccgcgcctggcgagaaagaagtgatcgacctggtcgattacttacttaccagttgctttgtcaccggacgcagtttcccacttgatggcggtcgtcatctgcgttaatgcagctttatccagcatataatcaacacccatgcgcttatcccccaacacgcaacagaaccaacaaaagcggcgggcaagcgcatcattccggtgaaataccacagcgacaccaggtaaacaaaatagggaataatcgaccacatactaaaaatgatggttgcgcgtaaggcttcaatgccgcgttcgctggcaacaatataatgcgcgataagcgcaaaggtcgggaaaagtggaatcagcccggcgatataataatttttcgtttttgctaaaacaccaatcaacagcactaccagcgcaccgagcgcggctttgattaccagccccatctttttaccttaacacttccataacaagtcatcagtagaatacctgatgaaaacttgtttagaaacgattgatagtaagtaaaaacagcgcggtgtattgtgacgtttttatatctaccgtgaatgttatgaacactatcgtatttgtggaagatgatgcggaagtcggttcactgattgccgcgtacctggcaaaacatgatatgcaggttaccgtagagccgcgcggcgaccaggccgaagaaaccattttgcgagaaaatccggatttggtgttactcgacatcatgctaccaggcaaggacggcatgaccatttgtcgtgatttacgcgcaaagtggtctggaccgattgttcttctaacctctctcgatagcgatatgaaccacatcctggcactggaaatgggtgcctgcgactatattctcaaaacgacgccccctgctgttttgctagcgcgtttacgtttgcatttgcgtcagaatgagcaagccacactgaccaaaggtcttcaggaaacgtctctgactccctacaaagccctgcatttcggcacgttgaccatcgatcccatcaaccgcgtagtcaccctggctaacactgaaatctcgctctcgacagctgatttcgaattattgtgggaattagctacccatgccgggcaaatcatggaccgcgatgcattgctgaaaaatttacgcggcgtcagttatgacggactggatcgtagcgtggacgtggctatttcgcggttaagaaaaaaactgctcgataacgccgcagaaccttatcgcattaaaactgtgcgtaacaaaggctatctttttgcgcctcatgcatgggaataagcgatgaaaaaactgtttatccagttttacctgttattgtttgtctgcttccttgtgatgtctctgctggttgggctggtgtacaaatttaccgccgaacgcgcgggcaaacagtcgctggatgatttgatgaacagttcgctgtatctgatgcgcagcgaattgcgtgagatccccccacacgactggggtaaaactctgaaagagatggatttaaatctctctttcgatctgcgtgtcgagccactgagtaaataccatcttgatgatatttccatgcaccgactgcgtggcggcgaaattgtcgccctggacgatcagtacacgtttttgcagcgtatcccgcgcagccactacgtgctggcagttggtcctgttccttatctttattatctccatcagatgcgattgctggatatcgccctgatcgcttttattgctatttccctcgcctttccggtgtttatctggatgcgtccgcactggcaggatatgttaaaactggaagcagcggcgcaacgatttggcgatgggcatctcaatgaacgtatccactttgatgagggttcgagctttgaacgacttggcgtcgcatttaaccagatggcggacaatatcaacgccttaattgccagcaaaaaacagcttattgacggtatcgctcacgaactgcgaacaccgttagtgcgcctgcgttatcgactggagatgagcgataacctgagcgccgccgaatcccaggcgttgaatcgtgatatcagtcaacttgaagctttaattgaagagctgctgacttatgcccgactcgatcgcccacaaaacgagcttcatcttagcgaaccagacctgccgttgtggctgtcaacgcatctggcagatattcaggcagtaacgcccgataaaacggtacggataaaaacgctcgtgcaaggccattatgcggcgttggatatgcgcttaatggagcgcgtgctggataatttgctcaataacgccctgcggtactgccattcaacggttgaaaccagcctgctactgtcggggaatagagcgacattaattgttgaggatgatggcccagggattgccccagaaaaccgcgaacatatctttgaaccttttgttcgcctcgatcccagccgggatcgctcaaccggcggctgcgggctggggctggcaattgtccactctatagcactggcaatgggcggtacggttaattgtgacaccagcgaactgggtggtgcccgcttctcgtttagctggccgttatggcataacatcccgcaatttacctctgcctgacactacgcgcacgatggtcaagtcaccacgactgtgctataaaataagtatgttgtaactaaagtggttaatattatggcgcgttacgatctcgtagaccgactcaacactacctttcgccagatggaacaagagctggctatatttgccgctcatcttgagcaacacaagctattggttgcccgcgtgttctctttgccggaggtaaaaaaagaggatgagcataatccgcttaatcgtattgaggtaaaacaacatctcggcaacgacgcgcagtcgctggcgttgcgtcatttccgccatttatttattcaacaacagtccgaaaatcgcagcagcaaggccgctgtccgtctgcctggcgtgttgtgttaccaggtcgataacctttcgcaagcagcgttggtcagtcatattcagcacatcaataaactcaagaccacgttcgagcatatcgtcacggttgaatcagaactccccaccgcggcacgttttgaatgggtgcatcgtcatttgccggggctgatcacccttaatgcttaccgcacgctcaccgttctgcacgaccccgccactttacgctttggttgggctaataaacatatcattaagaatttacatcgtgatgaagtcctggcacagctggaaaaaagcctgaaatcaccacgcagtgtcgcaccgtggacgcgcgaggagtggcaaagaaaactggagcgagagtatcaggatatcgctgccctgccacagaacgcgaagttaaaaatcaaacgtccggtgaaggtgcagccgattgcccgcgtctggtacaaaggagatcaaaaacaagtccaacacgcctgccctacaccactgattgcactgattaatcgggataatggcgcgggcgtgccggacgttggtgagttgttaaattacgatgccgacaatgtgcagcaccgttataaacctcaggcgcagccgcttcgtttgatcattccacggctgcacctgtatgttgcagattaacgcccggctttcatactgccgaccatctgttctggccgtacccagctgtcaaactcggcttcgctaagataccccagcgcaagggccgcagcttttaaggtcagcccttctttatgcgcttttttggcgatctcggcggctttgtcataaccaatgtgggtgttaagcgcagtcaccagcatcagcgattcattgagtaattgattgattcgctcacgattcggttcaatacccactgcgcagtgtttgttaaaactttccatgccatctgccagcaagcgcaccgattgcaggaaattgtggatcaccattggacggaagacgttcagttcaaagttaccggaagcgccccccatgttgatcgccacgtcgttccccatcacctgacagcagagcatggttaatgcctcacactgtgttgggttcactttccccggcatgattgagctgcccggctcattttccgggattgagatttcaccaattccgcagcgcgggccagaggccagccagcggacatcattggcgattttcatcagtgacgcagccaaccctttcaacgcgccgtgcgcctgaaccagggcatcacaggtcgccagcgcttcaaatttgttcggcgcggtaacaaacggtgcacaggtaatgactgccagttcatctgctacgcgacgcgcatactccggatgggtatttagtccagtacccaccgctgtaccgccaagagccagttccgctacgtgaggcaggctgtattcgatatgtttgagattatgctcgagcatcgctacccagccggaaatctcctgccccagcgttaacggcgtggcatcctgcaagtgagtacgaccaattttgacgatatcggcaaaagcacgggatttctcattcagtgtctgtgtcagggttttaagctgaggaatgagttgcttgcgcagcgccagcagcgccgcaacgtgcatcgccgtcggaaagacatcgttggaactttggcttttgttcacgtcgtcgttagggtgaactttacgttccatcccgcgcacaccgccgagtaattcactggcccggttagccagcacttcgttcatgttcatgttactttgcgtgccggagccggtctgccagatagccagcgggaattcgtcgtcatgctgtcctgccagtacttcatccgccgcctgacgaatggcgctcgctttctcttcagacaacaagcctaaatcttcattaacttttgccgctgcacgcttggttagcgccagcgcatgaatcagtgaggtgggcattttctccgtcgaaatgcggaaatgctccagcgagcgttgagtttgtgcgccccacagcttatctgccgggacatcaatcgcccccatcgaatctttttcgctgcgtactgtattcatgacctgctcctcacctgattaattttttctttctgttttgctttcgttaagcaacttttagctcacttattatttaccatttgataacaaatgtttggtctttcgtgccatgtaaaaaaaccgccccgaagggcggctctgtttatttcacacagcgggtgcattgtgtgagttgtatctgctggaagaagtcatttcctttatcatccacaaggataaacgccgggaaatcttccacttcaattttccagatggcttccattcccagttccggatattcaacacattccaggctcttaatacttccctgcgccaatacagcggccggaccaccgatactgccaaggtagaagccgccgtgttttttacaggcatccgtcacctgctggctgcggttgcctttcgccagcatgatcatacttccgccctgcgcttgcagttgatcgacataagaatccatccgtccggcggtcgttgggccaagagaaccggaggcataaccttccggcgttttggccggacccgcgtagtaaatcggatgatctttgatgtactgcggcagcccttcaccgttatccatccgctctttcagtttggcgtgagcaatatcacgaccgacgataatcgtgccgttaagcgataagcgtgtagaaacgggatactgcgacaactgtgcgaggatctctttcatcggacggttaaggtcaacgcgcaccgcttcgccttctcccgctttgcgcagctcttccgggatatatttgcctggattatgttccagtttttcgatccagatcccctgacggttgatcttcgctttgatattacggtcagcagagcaggagacgcccataccgaccgggcaggatgcgccgtgacgtggcaggcgaatcacgcggatgtcgtgagcgaagtatttaccaccaaactgcgcacccagaccaagattttgcgcttcgatcagcaattctttttccagttccacatcgcggaacgcctgaccgtgctcattcccttccgttggcagttcatcatagtatttcgcggaagccagtttcaccgttttaaggttcgtttctgcagaagttccaccaataacgaacgcaatatgatacggaggacaggccgccgtacccagcgtgcgcatcttctcaaccaggtaatttttcagtttccccggcgtcagtaacgctttggtttcctgatagagatacgtcttgtttgccgaaccaccacctttggcgatacagaggaatttgtattcgtcgccatcaacggcataaagatcgatctgcgctggcagattggtgccggtattcacttctttatacatatccagcggcgcgttttgcgagtagcgcagattatcttcgatataagtgttatagacaccgcgcgccagcgccgcttcatcaccaccaccggtccatacacgctgcccttttttaccaacaataatcgcggtgccggtatcctgacaggttggcagaacgcctttcgccgcgatgtcggagttacgcaggaattgcagcgccacatatttatcattttcgctggcctccgggtcacgcagaatgtcggccacctgttgttggtgcgccggacgcagcatgaacgacgcatcatgaaacgcctggcgcgccaacagagttaacgcttcgggtgcgactttcaaaatctcctgcccttcaaattcagatacgctaacgtgttcgctggttagcaggtaatactcagtatcatcttttttgagtggaaaaggagcctgataatgaaagggtttgtttgacattgttctctcacttactgcctggtttggttatgctctgggcgggtgttccgttgccctgttaaaagcgagtaacaatatcctacacacttttttaacaaaaactgagactagtacgactttttgcggctccaggttacttcccgtaggattcttgctttaatagtgggattaatttccacattaaaacagggattgatcatgcaaaaactcattaactcagtgcaaaactatgcctggggcagcaaaacggcgttgactgaactttatggtatggaaaatccgtccagccagccgatggccgagctgtggatgggcgcacatccgaaaagcagttcacgagtgcagaatgccgccggagatatcgtttcactgcgtgatgtgattgagagtgataaatcgactctgctcggagaggccgttgccaaacgctttggcgaactgcctttcctgttcaaagtattatgcgcagcacagccactctccattcaggttcatccaaacaaacacaattctgaaatcggttttgccaaagaaaatgccgcaggtatcccgatggatgccgccgagcgtaactataaagatcctaaccacaagccggagctggtttttgcgctgacgcctttccttgcgatgaacgcgtttcgtgaattttccgagattgtctccctactccagccggtcgcaggtgcacatccggcgattgctcactttttacaacagcctgatgccgaacgtttaagcgaactgttcgccagcctgttgaatatgcagggtgaagaaaaatcccgcgcgctggcgattttaaaatcggccctcgatagccagcagggtgaaccgtggcaaacgattcgtttaatttctgaattttacccggaagacagcggtctgttctccccgctattgctgaatgtggtgaaattgaaccctggcgaagcgatgttcctgttcgctgaaacaccgcacgcttacctgcaaggcgtggcgctggaagtgatggcaaactccgataacgtgctgcgtgcgggtctgacgcctaaatacattgatattccggaactggttgccaatgtgaaattcgaagccaaaccggctaaccagttgttgacccagccggtgaaacaaggtgcagaactggacttcccgattccagtggatgattttgccttctcgctgcatgaccttagtgataaagaaaccaccattagccagcagagtgccgccattttgttctgcgtcgaaggcgatgcaacgttgtggaaaggttctcagcagttacagcttaaaccgggtgaatcagcgtttattgccgccaacgaatcaccggtgactgtcaaaggccacggccgtttagcgcgtgtttacaacaagctgtaagagcttactgaaaaaattaacatctcttgctaagcttattaaaggcttataacaccttcaggcggccagtccgcctgatttcattttatggataatcattatgaataaatcgctggtagcggtaggcgtcattgttgcgctaggcgtagtctggacaggcggcgcatggtatacaggcaagaagattgaaacccatctcgaagacatggtcgcgcaggcgaacgcgcaactcaaactgacagctcctgaatccaacctggaagtgagttatcaaaactatcatcgcggcgtattcagcagccagttgcaactgttggtgaaacccattgccgggaaagaaaatccgtggattaaaagcggtcagagcgtcatcttcaacgaatcggttgatcatggtcccttcccgcttgcccagcttaaaaaactgaacctgatcccgtcgatggcatcaattcaaaccacgctggttaataacgaagtaagcaaaccactgtttgatatggcaaaaggtgaaacgccttttgagattaactcgcgcattggttacagcggtgattccagttccgatatttcgctcaagccactgaattacgagcaaaaggatgaaaaagtcgcctttagcggcggcgagttccagttaaatgctgacagagacggcaaagccatctccctttccggggaggcgcaaagtggtcggatagacgcagttaacgaatacaaccagaaagtgcagttgacctttaataatctgaaaaccgacggttccagcacgctggcaagttttggtgagcgtgtaggaaatcaaaaactgtcactggaaaaaatgaccatttcagtggaaggcaaagaactggcactgctggaaggcatggagatcagcggtaaatcggatctggtcaatgacggtaaaacgatcaatagccaactggattactcgctaaacagcctgaaggtacagaatcaggatctgggcagcggcaagctgactttaaaagtcggccagattgatggtgaagcctggcatcagtttagccagcaatataacgcgcaaactcaggcgctgctggcacagccagaaattgccaacaaccccgaactttatcaggagaaagtgacggaagccttctttagcgccctgccgctgatgctgaaaggcgatccggtgattactatcgcgccgctaagctggaaaaacagtcagggtgaaagtgccctgaatctgtcgctgttcctgaaagatccggcaacgactaaagaagcgccgcaaacgctggcgcaggaagtagatcgttcggttaaatctctggatgcgaaactgaccattccggtggatatggcaactgagtttatgactcaggtagcgaagctggaaggttatcaggaagatcaagcgaaaaaactggcgaaacagcaagttgaaggtgcatcagcaatggggcagatgttccgtctgaccaccttgcaggacaataccatcaccaccagcctgcaatatgctaacggtcagataacgttaaatgggcagaaaatgtcgttagaagattttgttggcatgtttgcgatgccagctcttaacgttccggctgtaccggcaattccgcagcagtaattcacggccaaaacgccggagaattttcactccggcgttttcatctgaaaacaaaccagagattgcctgatgcgctacgcttatcaggcctaccttttcctgcaacactttgaatttatgagtttttgtaggctggataaggcgtttacgccgcatccggcataaaaaacgcgcactttgtcaacaatctgaaacgccggagatttttctctccggcgttattttttacttcagcataaagtcatactgaatactcattttcacatcccagtaattcaggcgatcgcccagcgtactgccatcgcgcttttcccgccctttatcggcagcaagaaagaaattcatcccttgtaacggcccttcgctgacccgatagttcataccacctaagatacccgtgccttcaatccgcacatctcgtttactggattcatagccgcgagtcacaatcggtgcaaatgtcagcgtaaattgcggcgttaaacgatagttgacgcccaattgccaggactgcattccttcacggttacgatcaagacttaatgaaaagggatagccaatgtcggtatccaccacggcaccattcattgcatggcgcaaataaccaccactgccaaatacacttccccacggcgcattccaggtcaattgtccactaaccaacgccgtttcattgggctggctggtattacgacttaaaccttcgagctgcgcgtaaaagccgagcaactcccctttcaacgtataattcgggtcgagcggtatgcttttctcgagaatactttgtatctgattggaaacatctttctgtaccgatgcccccagagaatagcgactggtatcatcatgccaactggcggctaaaaaagaacgtgcgcgatgtttatcgtattttcccgtctggctgttatacaccccttcatcacgaataccggttgttgaatcagtccataaaaatactcgtgaacgccacattccccacagatcaatatttggtgttaaagcccaataacctaatgctccttcagaaactgtcggtaatgtacgttgcgaactgccagccattaacggaatacgataaggtaagctaccataactataatccgtcccgaagcgacctaatttaagcaggctattttcactgggttttatttttactgcccccagggcaaagccaaaacttttatcaccatcaagataccaccgggtactcatatcagcacgagcacctaatttataaacataatacgccccgccttcaacgccaataatattggaataataaccactattgaaatcgagcaatcctccctgtacccatgcgtaaatatctcttcccgcgccagcactgggcttatccgccctgcgcaattcgtttttcagtctgatgcgtagtcccgcttcatcgtcagccagttgcgccgcataagcagaggtaaggccagaggcagccgtcaggcaaataacggccatggccactatttttctcatagttgcacctttgatgttctgattatttttattgaatattaattagtgatatcgctgattaattgctgctgcacttttttacgattatcaatttcaaccacgatttctttgaattttttatccgtgagcggataaaaccagataataacgaatgccagtagcataaatccgcaaggtactaaggcaattgatgtgcggatgcccataataacttccggcgtttgcacctgattggcgatatatccgcttaaccccaaaataaaggcaggaattgaacctccgattgcctgaccgcatttacgggtaaatgagaatagtgaataggtgagcccttcaattcgcacgccggtcaggtattcaccgtattctacggtatcagcttccagcgcccacatcacggtcatggtaacgccctgaccaattgaagcgatggccaacgcaaccaacgccaccggcagtgaccagacggaaacccagaagaacagcagataaccgcaggttcccagcaaagcgccaatcaggaaggtattctttttaccgatcctcgcgaccatccccggcaccagcggtgccgatgccacagtaccaaccaggttttgcaccagtaccagcacagtgaacagcccggtatcatttaacacatagcgcacgtagaacaacgacgaggcgctgaccgcaaaggtcgaaatcagcacacacagcgcaccgatgcacaacataaacagcgggcgattccgtttcagggtttgcagactgatattcaatgacggctgcgcaacgatacgtaccacattctcacgcgtcgatttgaagcagatgaagtaaagcaccattccggcaatcgccagcacaattgtccagaaatggtataccgacaccatctcttccgggctggagttcttaatgctcggtcctatcagaaatgccaggcagacaaaggtcaatgaagcggcaatcccacgagccgcgcccagacgggcgcgggattgtggttgttgggtcatcgcggtagcaagtgaaccataaggaatattcaccaggctgtagcaaagcccgaggcccatgtaggtcaaatatgcatacaccactttgctaccatggctccagtcggtcagcacccagaataccagcacgctgaagatcattaacggcgcagtaccgaagagtaaaaacgggcggaattttccccagcgggtattcacactgtccaccactcgtccggcaaagacgtcggcgaaggcatcgaatacccgcaccagtaacagcatggtgcccgccgcagcggcaccgacgccagcgacgtcggtgtagtaactcaacaggaagagcgcccccattgcgaaggcgaagttattggcgacgtcaccgaggctgtagccgacgatggtgcgccaggagagttgttgattcattgtttgcctccctgctgcggtttttcaccgaagttcatgccagtccagcgtttttgcagcagaaaagccgccgacttcggtttgcggtcgcgagtgaagatccctttcttgttaccgccaacgcgcaatatgccttgcgaggtcgcaaaatcggcgaaattccatacctgttcaccgacgacggcgctgacgcgatcaaagacgcggtgatacatatccagccatgcacactgatactcttcactccacatgtcggtgtacattgagtgcagcccggctaacgtatccacgccgtattcggtgatgataatcggctgatgcagtttctcctgccaggccagaagttctttttccagtaccttctctgccgtttccaaatcgccgctttggacataccatccgtaataacggttcaggcacagcacatcaaagagatcgctgatggtatcggtgtgagcgtcgcagaacattacattgacgcaggtgatcggacgcgtcgggtcgagtttacgcgttgcttccgccagtggcgcgaaatattcccgtgcaccttgcggacgggtatccggttcgttggcaatactccacatcaccacgcttgggtggtttttgtcacgcgctatcagctctttaatcgcctgtaagtgcgcttgctgagtttccccgttgactgcctcttcgctgtacagttctttcggcttgttgcccgcttcgaaaccaatgcctaaagagaggttaaagccgacagcagcagtttcatcaatcaccacgatgccatgttcatctgcccagtcgagcatctcttcagcgtaagggtaatgcgaggtacggtaggagttggccccaatccagtccattaatgcgtggtcgtgcaccatcagcacgttatcgaatcctttgccacgcaagtccgcatcttcatgacgaccaaagccagtaaagtagaacggtttgtggttaatcaggaactgttcgcccttcactgccactgaccggatgccgacgcgaagcgggtagatatcacactctgtctggcttttggctgtgacgcacagttcatagagataaccttcacccggttgccagaggtgcggattcaccacttgcaaagtcccgctagtgccttgtccagttgcaaccacctgttgatccgcatcacgcagttcaacgctgacatcaccattggccaccacctgccagtcaacagacgcgtggttacagtcttgcgcgacatgcgtcaccacggtgatatcgtccacccaggtgttcggcgtggtgtagagcattacgctgcgatggatcccggcatagttaaagaaatcatggaagtaagactgctttttcttgccgttttcgtcggtaatcaccattcccggcgggatagtctgccagttcagttcgttgttcacacaaacggtgatacgtacacttttcccggcaataacatacggcgtgacatcggcttcaaatggcgtatagccgccctgatgctccatcacttcctgattattgacccacactttgccgtaatgagtgaccgcatcgaaacgcagcacgatacgctggcctgcccaacctttcggtataaagacttcgcgctgataccagacgttgcccgcataattacgaatatctgcatcggcgaactgatcgttaaaactgcctggcacagcaattgcccggctttcttgtaacgcgctttcccaccaacgctgatcaattccacagttttcgcgatccagactgaatgcccacaggccgtcgagttttttgatttcacgggttggggtttctacaggacgtaacataagggactcctcattaagataataatactggtcaacctttaatctgattagttaaccaattctgtgttgcacacagttatctgtgagaaacccatggaagagaaatggaaataaaaagaactgacaccgcgatcaaaaaaccaaaaactgcaatacccacagcgtgatatagatcgcattaatctttaaaacagcgttgacagaagccataaaataagcaaccgaacgttcgttcgagcgtattgggaacgataaactctcatgacatatggctacagtgaatattttggggggaattctccgaagccgggaaggataatttttgcacagagaaattacgatatgaaacgcgggcacagttatcaccagcccgccgaaaaagagagagaatcaggatgcggttaagataccgccaatcatcgcgcgtaatccctgagcaaacgacgcttcacgcgccaggtcttccgcttcgatatcggccagtacaccgtaggtcagatccagcagtaaacgtgaagtcattgccgtgttgatgtctgggcttatctcgcctttttgctgggcatcacgcatccgctgggcaacaaattccgtgatcgtcatatgcttatttttaagcatggcggcgacctgtgggttacgcatcccttccgccataatttcaaccaccagcgcccgttgtccaaaggcttcatgggtgagagagacaatggactcgaccatatagtcaacgaaatgaatcccttcaatcggttcccggaaacgggccagcgccctctcctggtcctgtaagataatcgcctgaatcaaggcttctttggagatgaaatggtgatagagcgtcccgggactaatggcgcaagatttacagatggctttcatcgaggcactgtgaaatccattttctgaaaaaatctctctggcagcattgaggatccgggtccgtgtcggttgtgcttcagtctgcatgttatccatcattaaaccattatagttagcgtgaataactagtttaccgcgttgtcaggtgagcgcctatcattgctgttgaatagtgcgaaggcacactctattcgtatacttttcactctgaaattggttaaccaatagccgtgatttggctgccagttatttagcagagacgttgatgagtttatcccggtaaacaacacgcacggttgtttaccggtccgttagtgtattaattgagctcctgtaccccaccaccggagacggtgagaatttgtccgcttacccagctcgcagcaggcgagcaaaggaacagcgctgcgttagcaatatcttgcggttggcccagacgtctgatcggcgtgtgctgtaacattttttgttcaatttctggtgtaataacggatttcagggcatcggttaatattgcccccggcgcaatgccatttacccgaatatttttttcacccaggtcaaacgccatatttctgaccagatgactggccgcagctttagatgatgcataggaagtcatgtttatatttttattttctgccgccatagaagtgatggtcagaataacgccaccgccatttttttccatttctggcgcaacaagttgtgacagatggaaaaaagaaaacacattcagttcataagcacggcgaaaatccgccattggcatatcaaacggtttaggtccaccgccaccggcgttgttaaccagaatatcaactttacccagcttactgatagcaaagtctgccagtgcagagagttcctgttcggaagtaatatcacaacggcaggcaaatgcctgaccacccagttgttgaatttcgtctacaacatggttagctgcgtcggcgttaatatcactgaccaccacagatgcgccagctgtcgcgaatgtaatggcgatttctttaccaatacctgcacccgcacctgtgatgatggcgcattttccgtcgagtctcaggttgtcagaattaaacacataaacctcctgtgaacttcagtaaaaataaaaggcaccgcctgtgtgccacattttttatcattaaccttgaggaaaggacactaccaggtatagcagataaagagaggattatttcgctgcaatgagccgggcgggaataataagattgcgtgaatgcgtctcttcatgggtgattttttgcatcatgcgatccgcaagtgtgataccaagttcccgcgctggcgtgctggcccaggtaacaggtatatcatcaagtgtggttggtgtcgcatcggtaaatgccgccagcgaaacctgttgctcaaagtaacgatcgactccgctttccccgctttgccgccctgctttgagcaaaccaaaccatgcccccatcgcaatagtttcgttatagcaaaccacggcactgatggtcgggttatgacgtaaaagcgccgtgatagcttccgcggcttgcttctggctggaagtgcactccaacacccaatcgctatgaaacggcaggccaaattttagtagagttgcacaatagcccccaacccgttctgcacgggttaatgaggaactttgccctcccagccaggcgatccgctgatgcccattgcgaatgagatgctccgtcaacaactgtgcagcctgcatgttgtccgggcgaaccgtatcaacatcatcaagataactggcacgggaagcgaaaatcaccgggatagctttttcttctgccatccgtcgcaggtcatcgctacttcctgcagctccggcaattaccacaccatcgacaccctgattcagtaacagtgaaaaccgctgtgccagctgctcaccgtctttaccgccgtgaagcaaaaaaaccatccgtccctgcgcttccagagcttccgtcaatccggccgtcaattcggcgtaaaacggcgcagataaatcacggacgatcaaaccaatgacgccgctttgcccgccgcgcagcgccgacgcctggcgattgcgcacaaatcccagctcttcaatggcggcgttaacgcgttctcctgtggcggtagagattcgccctttgccactaagcaccagcgaaacggtacttaccgacacgcccgcagccagcgcaacatcatgaatggttatttttttggcggtagccatgcagatgacctactccctgattatgtgacagataaaacgttttaccttttatttatcttatacccgctattatcgttgcgtaatgtgatttatgcctcactaaaatttgataaaacgttttatcttctcgcgcaatttactgaatccagattgttctctacgaggagtcgttttatgacggcgaaaacagcaccgaaagtcacgctgtgggagttcttccagcagttaggcaaaaccttcatgttacccgtggcattattgtcgttctgcggcattatgctcggcattggtagttctcttagcagccatgatgtcataaccctgatcccggtcctgggcaaccccgtgttgcaggctatctttacctggatgagtaagattggctcgtttgcttttagtttcctgcctgtcatgttctgtatcgccatcccgctgggcctggcacgcgaaaataaaggcgtagcggcattcgctggcttcatcggttatgcggtaatgaacctcgcggtaaacttctggttgaccaataaaggcattctgccaaccacggatgccgcggttctgaaagccaataacatccagagcattcttgggatccagtcgatcgataccgggatcctcggtgcggtgatcgccggtattatcgtctggatgctgcatgagcgtttccataatatccgcctgccggatgcgctggcattcttcggcggtacgcgcttcgtaccaattatctcctcgctggtgatgggccttgtcggcctggtgattccattagtctggccgattttcgccatgggtattagcggcttgggccatatgataaacagcgcgggtgatttcggaccgatgctgtttggtaccggtgaacgtctgctgttgccgtttggtctgcatcacattctggtggcattaattcgctttaccgacgcaggcggcacgcaggaagtctgcggtcaaaccgtcagcggcgcactgaccatcttccaggcgcaattgagttgcccgaccactcacggtttttctgaaagcgccacgcgtttcctttcgcaaggtaaaatgcctgcgtttctcggcggtctgccaggtgcagcgttagctatgtatcactgcgcgcgcccggaaaatcgccataaaattaaaggtctgctgatttctggcctgatcgcctgcgtcgttggcggcactaccgaaccgctggaattcctgttcctgttcgtagcgccagttctgtatgtcatccacgcgctgttaaccggcctcggcttcaccgtcatgtctgtgctcggcgtcaccatcggtaataccgacggcaatatcatcgacttcgtggtgttcggtattttgcatggtctgtcaaccaagtggtacatggtgccagtggtggcggcaatctggtttgtcgtttactacgtcatcttccgtttcgctatcacccgcttcaatctgaaaaccccggggcgcgatagcgaagttgccagctcaatcgaaaaagccgttgccggtgcgccgggtaaatcaggttacaacgttcctgcaatcctcgaagcattaggcggtgccgacaatattgtcagcctcgataactgcattacccgtctgcgtttgtctgtgaaagatatgtcgcttgttaatgtgcaggcactgaaggacaatcgggcaattggcgtagtacaacttaatcaacataacctgcaggttgttatcgggccacaagttcagtcagtaaaagatgaaatggccggtctgatgcatactgtccaggcataaggataagatatgttcgatttttcaaaggtcgtggatcgtcatggcacatggtgtacacagtgggattatgtcgctgaccgtttcggcactgctgacctgttaccgttcacgatttcagacatggattttgccactgccccctgcattatcgaggcgctgaatcagcgcctgatgcacggcgtatttggctacagccgctggaaaaacgatgagtttctcgcggctattgcccactggttttccacccagcattacaccgccatcgattctcagacggtggtgtatggcccttctgtcatctatatggtttcagaactgattcgtcagtggtctgaaacaggtgaaggcgtggtgatccacacacccgcctatgacgcattttacaaggccattgaaggtaaccagcgcacagtaatgcccgttgctttagagaagcaggctgatggttggttttgcgatatgggcaagttggaagccgtgttggcgaaaccagaatgtaaaattatgctcctgtgtagcccacagaatcctaccgggaaagtgtggacgtgcgatgagctggagatcatggctgacctgtgcgagcgtcatggtgtgcgggttatttccgatgaaatccatatggatatggtttggggcgagcagccgcatattccctggagtaatgtggctcgcggagactgggcgttgctaacgtcgggctcgaaaagtttcaatattcccgccctgaccggtgcttacgggattatagaaaatagcagtagccgcgatgcctatttatcggcactgaaaggccgtgatgggctttcttccccttcggtactggcgttaactgcccatatcgccgcctatcagcaaggcgcgccgtggctggatgccttacgcatctatctgaaagataacctgacgtatatcgcagataaaatgaacgccgcgtttcctgaactcaactggcagatcccacaatccacttatctggcatggcttgatttacgtccgttgaatattgacgacaacgcgttgcaaaaagcacttatcgaacaagaaaaagtcgcgatcatgccggggtatacctacggtgaagaaggtcgtggttttgtccgtctcaatgccggctgcccacgttcgaaactggaaaaaggtgtggctggattaattaacgccatccgcgctgttcgttaaccccaattgcgcaacgtaaaaaatcgttgcgcaatcgtggatttttaccctgctttgtttttataatggtgcgcacttttatatccagaaaaagagtgcgaccatgattgataccaccctgccattaactgatatccatcgccaccttgatggcaacattcgtccccagaccattcttgaacttggccgccagtataatatctcgcttcctgcacaatccctggaaacactgattccccacgttcaggtcattgccaacgaacccgatctggtgagctttctgaccaaacttgactggggcgttaaagttctcgcctctcttgatgcctgtcgccgcgtggcatttgaaaacattgaagatgcagcccgtcacggcctgcactatgtcgagctgcgtttttcaccaggctacatggcaatggcacatcagctgcctgtagcgggtgttgtcgaagcggtgatcgatggcgtacgtgaaggttgccgcacctttggtgtgcaggcgaagcttatcggcattatgagccggaccttcggcgaagccgcctgtcagcaagagctggaggcctttttagcccaccgtgaccagattaccgcacttgatttagccggtgatgaacttggtttcccgggaagtctgttcctttctcacttcaaccgcgcgcgtgatgcgggctggcatattaccgtccatgcaggcgaagctgccgggccggaaagcatctggcaggcgattcgtgaactgggtgcggagcgtattggacatggcgtaaaagccattgaagatcgggcgctgatggattttctcgccgagcaacaaattggtattgaatcctgtctgacctccaatattcagaccagcaccgtagcagagctggctgcacatccgctgaaaacgttccttgagcatggcattcgtgccagcattaacactgacgatcccggcgtacagggagtggatatcattcacgaatataccgttgccgcgccagctgctgggttatcccgcgagcaaatccgccaggcacagattaatggtctggaaatggctttcctcagcgctgaggaaaaacgcgcactgcgagaaaaagtcgccgcgaagtaacaaaatggatggtgcaaatgcaccatccatttttcatgcaaggcacaaagtcgcgcgatgtttggcggattcgatgcccagctcaatcaactccattacctggattgcctggcttgccggaaccggattttcaccatcgccatttaacgcatcacgaatagccgcatagtaagccggataattcccaggcaccgtcaacagcgtttcttcgacacgttcctcaccttccacgcgggtaagtacgccatcacgcatatcgtagccccagtcttcctgcggtagacgctcgccatttttcagacgttcttcctgtggatcgaggccatatttcacataactgcctcgggatccatgcacgatataccgtgctgactcagcggctgccagcatggtaccgtgtaaaatgactcgccgctgtggataggacaagatggcgtggaaataatcggtcgactgcgctccgggccgtaactgtgccaaatctaccgtcatgctgaccggtaaaccaaaaagcgtaatggcctgatcaagaagatgtggtgctaaatcgtaccagataccgctgcctgggccgccctgttcacgccaacgatcgcgcacctgcggacggaagcggtcaaaatgagactcaaagtaagcaacttcacccagcacgccttccgcgagtaaaccttttagcgtcaagaaatcgctatcccagcgacggttatggaatacagacagcacacgccccaggctttttgccagcgcatccagctctcgcgcttgtgacagtgtcacggtaaagggtttatcaacgaccacatgtttacccgcctcaagcgccgctttggctaacgggaaatgggtatcgttgggtgtaggaatgacaatcaggtctatgttgggatcgttaaacagatgcttcggctcagagacaaccgtaaccgttggccagtcggcttttacttttgtttcatcactgctggagattaccgccagttcctgcccgggcgtgcccgcaatcaggggcgcatggaaggttttgctcgcataaccatacccaatcaacccaacacggatgttgtcgctcatgtcattgcctctcattgaagtatgatggctatttgacactatcctttacccacgctcaacagtttaataacctgccagcaataagggatgttgtttaacttaagtcaaaaaaatagcgaattttccaacgacaaaagctaaatatcgcaaaaacctcagtaaaaatcttgctggagctattattgctaagtaacatttaccccctgaagttaatggatcaatcaagagagatgtgggctgtaatgaatcgtcttattgaattaacaggttggatcgttcttgtcgtttcagtcattcttcttggcgtggcgagtcacattgacaactatcagccacctgaacagagtgcttcggtacaacacaagtaagctctgcacttgtggagcgacatgctgcccgtccgggtgcatgttttcacttgtcggatattaaaccaggaatttattatcttgttcgatgttgttggtgattgtcagggatagtaaagcgcgttactcttttcagagcagtttttcatccctgaatatttgccatcagcgcattcttattattgtaataacacaagcgttcacttttggtgaaattttatcatcactaataatacctacccctttggtattaattattttatggaccttttatgactgttcaggactacttattaaaatttcgcaaaatcagttcactcgaaagtctggaaaaactctacgaccatcttaattacaccctgacggacgatcaggaactgatcaatatgtatcgtgctgccgatcaccgtcgcgcagagctggtttctggcgggcgtttgtttgacctcggccaggtaccgaagtccgtctggcactatgtccaataaagaaagtagcgatcggttataaaagccttataataacgcccctaaaattagatttgcctgtttgcgtcgctattctggagaacctatgaccaccacaacgccacaacgtattggaggctggttgcttggcccgttggcctggcttttagtcgctctgttgagtacgacgctggcgttgttgctgtataccgctgcgttatcttctccgcaaacatttcaaacgctcggcggacaagcactgacgacacaaatcttatggggcgtttcttttattaccgctatcgccttgtggtattacacactgtggttgaccatcgctttctttaaacgtcggcgttgtgttcctaaacactatattatctggctgcttatttccgtattgctggcagtaaaagcattcgctttttcacccgtggaagatggcatagccgttcgccagttgctgtttactttgttggcaaccgcattgatcgtcccctatttcaaacgctcgtcgcgggtaaaagcgacgtttgtgaatccgtaataaccttacagttaacctgttgtcgcctgctctggattaacggataataggcggcttttttatttcaggccgaaaaatgactgactacctgttactgtttgtcggaactgtactggtcaataactttgtactggtcaagtttctcggtctctgtccgtttatgggggtttccaaaaaactggaaaccgcgatgggcatggggctggcaacaacgtttgtgatgacgctggcgtctatttgcgcctggcttatcgatacgtggattttgatcccacttaatctgatttacctgcgcaccctggcatttattctggtgattgctgtggtcgtgcagttcaccgagatggtggtgcgcaaaaccagcccggtgctttaccgtctgctggggatttttttgccgcttatcaccaccaactgtgcagtgctcggcgtggcgttgctgaatatcaatctcgggcacaatttcttgcagtcggcgctgtacggtttttccgccgctgtcggtttctcgctggtgatggtgctcttcgccgccatccgcgaacgccttgctgtggctgatgtcccggcaccttttcgcggtaatgccattgcgttaattaccgcaggtcttatgtctctggcctttatgggctttagtggtttggtgaagttgtaatgaatgctatctggattgccgttgccgccgtgagcctgctgggcctggcgtttggcgccattctgggttatgcctcccgccgttttgcggtggaagacgatccggtcgttgagaaaattgacgaaatcttaccgcagagccagtgtggtcagtgcggttatcccggctgtcgcccctacgcggaagccatcagctgtaacggtgaaaaaatcaaccgttgcgccccaggtggcgaagctgtgatgctaaaaattgccgagttgcttaatgtcgagccgcagccgctggatggcgaagcgcaagagataacgcctgcgcggatggtggcggttattgatgaaaataactgtattggctgcactaaatgtattcaggcgtgtccggtagacgccatcgttggcgctacccgtgccatgcatacggtaatgagtgatctctgtacgggctgcaatttatgtgttgatccgtgcccgacgcactgcatctcgttgcaaccggtcgcagaaacacctgactcctggaaatgggatctgaacaccattcccgtgcgtatcattcccgtggaacaccatgcttaagttattctctgcattcagaaaaaataaaatctgggatttcaacggcggcatccatccaccggagatgaaaacccagtccaacggtacacccctgcgccaggtacccctggcgcagcgttttgttattccactgaaacagcatattggcgctgaaggtgagttgtgcgttagcgtcggcgataaagtattgcgcggccagccgcttacccgtggtcgcggcaaaatgctgcctgttcacgcgcccacctcgggtaccgttacggctattgcgccccactctacggctcatccttcagctttagctgaattaagcgtgattattgatgccgatggtgaagactgctggatcccgcgcgacggctgggccgattatcgcactcgcagtcgcgaagagttaatcgagcgcatacatcagtttggtgttgccgggctgggcggtgcaggattcccgacaggcgttaaattgcagggtggcggagataagattgaaacgttgattatcaacgcggctgagtgcgagccgtacattaccgccgatgaccgtttgatgcaggattgcgcggctcaggtcgtagagggtattcgcattcttgcgcatattctgcagccacgcgaaattcttatcggcattgaagataacaaaccgcaggcgatttccatgctgcgcgcggtgctggcggactctaacgatatttctctgcgggtgattccaaccaaatatccttctggcggtgctaaacaattaacctacattctgaccgggaagcaggttccacatggcgggcgttcatccgatatcggcgtattaatgcaaaacgtcggcactgcttatgcagtgaaacgtgccgttattgatggcgagccgattaccgagcgtgttgtaaccctgactggcgaagcaatcgctcgcccgggcaacgtctgggcacggctggggacgccagtgcgtcatttattgaatgatgccggattctgcccctctgccgatcaaatggtgattatgggtggcccgctaatgggctttaccttgccatggctggatgtcccggtcgtaaagattaccaactgtctgttggctccctctgccaatgaacttggcgaaccacaggaagaacaaagctgcatccggtgtagcgcctgtgctgacgcctgccctgcggatcttttgccgcaacagttgtactggttcagcaaaggtcagcaacacgataaagctaccacgcataacattgctgattgcattgaatgtggggcttgcgcgtgggtttgcccgagcaatattcccctggtgcaatatttccgtcaggaaaaagctgaaattgcggctattcgtcaggaagaaaagcgcgccgcagaagccaaagcgcgtttcgaagcgcgccaggctcgtctggagcgcgaaaaagcggctcgccttgaacgacataagagcgcagccgttcaacctgcagccaaagataaagatgcgattgctgccgctctggcgcgggtgaaagagaaacaggcccaggctacacagcctattgtgattaaagcgggcgaacgcccggataacagtgcaattattgcagcacgggaagcccgtaaagcgcaagccagagcgaaacaggcagaactgcagcaaactaacgacgcagcaaccgttgctgatccacgtaaaactgccgttgaagcagctatcgcccgcgccaaagcgcgcaagctggaacagcaacaggctaatgcggaaccagaacaacaggtcgatccgcgcaaagccgccgtcgaagccgctattgcccgtgccaaagcgcgcaagctggaacagcaacaggctaatgcggaaccagaagaacaggtcgatccgcgcaaagccgccgtcgaagccgctattgcccgtgccaaagcacgcaagctggaacagcaacaggctaatgccgagccagaacaacaggtcgatccgcgcaaagccgccgtcgaagccgctattgcccgagccaaagcgcgcaaacgggaacagcaaccggctaatgcggagccagaagaacaggttgatccgcgcaaagctgccgtcgaagcggctattgcacgcgccaaagcacgcaagctggaacagcaacaggctaatgcggtaccagaagaacaggttgatccgcgcaaagcggcagttgccgcggctattgcccgcgctcaggccaaaaaagccgcccagcagaaggttgtaaacgaggactaaatggtattcagaatagctagctccccttatacccataaccagcgccagacatcgcgcattatgctgttggtgttgctcgcagccgtgccaggaatcgcagcgcaactgtggttttttggttggggtactctcgttcagatcctgttggcatcggttagtgctctgttagccgaagctctcgtactcaaactacgcaagcagtcggtagccgcaacgttgaaagataactcagcattgctgacaggcttattgctggcggtaagtattccccccctcgcgccatggtggatggtcgtgctgggtacggtgtttgcggtgatcatcgctaaacagttgtatggcggtctgggacaaaacccgtttaatccggcaatgattggttatgtggtcttactgatctccttccccgtgcagatgaccagctggttaccgccacatgaaattgcggtcaacatccctggttttatcgacgccatccaggttatttttagcggtcataccgccagtggtggtgatatgaacacactacgcttaggtattgatggcattagtcaggcgacaccgctggatacatttaaaacctctgtccgtgccggtcattcggttgaacagattatgcaatatccgatctacagcggtattctggcgggcgctggttggcaatgggtaaatctcgcctggctggctggcggcgtatggttgctatggcagaaagcgattcgctggcatattcccctcagcttcttagtaacgctggcgttatgcgcaatgttgggctggttgttctcaccagaaacactggcagcaccgcaaattcatctgctgtctggagcgaccatgctcggcgcattctttattttgactgacccggttaccgcttctacgaccaatcgtggtcgtcttattttcggcgcgcttgcgggcttattagtctggttgatccgcagtttcggcggctatcctgacggcgtggcttttgccgtcctgctggcgaacatcacggttcctctgatcgattactacacgcgtccgcgcgtctacggccatcgcaaagggtaaaccatgctgaaaactatccgaaaacacggcattacgttggcgctatttgcagcgggttcaacagggttaactgcggccatcaaccagatgaccaaaacgacgattgctgaacaggccagtctgcaacaaaaggcgttatttgatcaggtgctgccagccgaacgctataacaatgcgctggcacagagttgctatctggtaactgcgccagagttaggtaaaggtgagcatcgggtttacatcgccaaacaggatgacaaaccggtagccgccgttctggaagcaaccgcgccagatggctattccggtgcgattcagctgctggtgggagccgattttaacggcacggtacttggcacgcgcgtgacagagcaccacgaaacgccagggcttggcgataaaatcgaactgcgcctttctgactggatcacccattttgcgggtaaaaaaatcagtggtgcagatgatgcgcactgggcggtgaagaaagatggtggtgatttcgaccagttcaccggcgcgacgattactccccgcgcggtggttaatgcggtaaaacgcgccggattgtacgctcagacgttaccggcacaactttctcaacttcctgcctgtggagaataaagcgtgagcgaaattaaagacgttattgttcaggggttgtggaaaaacaactctgcgctggtccagttgctcggcctttgtcctctgttggcggtcacgtccactgccactaacgctctgggtttaggacttgcgactacgctggtactgacgctgaccaacctgaccatttcgacgctgcgtcactggacgccagccgagatccgcattcccatttacgtgatgatcatcgcctcggtggtcagcgctgtacagatgctgatcaacgcctacgcctttggcctgtatcaatcattagggatttttattccgctgattgtcactaactgtatcgttgtgggccgcgctgaagccttcgccgccaaaaaaggtccggcgctttcggcactggacggcttttcaattggtatgggcgcaacctgcgccatgttcgtgctgggttcactacgcgaaattatcggcaatggcacattgtttgacggtgcagatgcgctgttaggtagctgggcaaaagtattacgcgtggagattttccacaccgactcccctttcctgctggcgatgctgccaccaggtgcatttattggcctgggactgatgctggcaggaaaatacctgattgatgaaagaatgaaaaagcgccgtgctgaagcagctgcagaacgtgcattgccaaacggtgaaacagggaatgtctgatgaataaagcaaaacgcctggagatcctcactcgcctgcgtgagaacaatcctcatcccaccaccgagcttaatttcagttcgccttttgaattgctgattgccgtactgctttccgctcaggcgaccgatgtcagtgttaataaggcgacggcgaaactctacccggtggcgaatacgcctgcagcgatgcttgaactgggcgttgaaggggtgaaaacctatatcaaaacgattgggctttataacagcaaagcagaaaatatcatcaaaacctgccgtatcttgctggagcagcataatggcgaggttccggaagatcgtgctgcgcttgaagccctgcccggcgtaggtcgtaaaacagccaacgtcgtattaaacactgcattcggctggccgactattgctgtcgacacgcacattttccgcgtttgtaatcgtactcaatttgcgccggggaaaaacgtcgaacaggtagaagaaaagctactgaaagtggttccagcagagtttaaagtcgactgccaccattggttgatcctgcacgggcgttatacctgcattgcccgcaagccccgctgtggctcttgtattattgaagatctttgtgaatacaaagagaaagttgacatctgaagaaaaggggtaacaccgattaccccattgataacctttctttatcctcttttaaaacatctttttaacgtcaatgatgccattgcttagcgttatcatcaggtaatccgtttgcggataaccaaaaatgcaggttaattgtttttttaatagcgaaattttctattcattcgtgatcaagatcacgatgctgtcgcaatgtaaaaacattgcaagaatcaggttaaaatcatttaaatttacacacgcaacaaatattgacctacaaaacattacactggctatttttcagaaactggactatctcactagtaaaaacgctaaatagcagaacatatcgccgttaagccatcacccccctctcagtgcagtgaaaaaatctgccgttacgttttttgaaaaatttaacgctggataacatttcccggaatggttgaattccccgcctcagttatatgtaacagattattacaaaggacttgtctgaaagtgcaagatagtgaacattacctgccgtttcccctcccactataacaattgcgcgtatgttttttatacataacgcgagaaagcacccccgttaatatgggatgtaaaaaaagaggtaaaagtgtccactgcaaaccaaaaaccaactgaaagcgtcagtttgaacgctttcaaacaaccgaaggcgttctatctcatcttctcgattgagttatgggaacgttttggttattacggcctacaaggaattatggctgtttacctggttaaacaactgggtatgtctgaagcggattcaatcacccttttctcttcctttagtgccctggtttatggtctggtcgctatcggcggctggttaggtgacaaggtactgggtactaaacgcgtaattatgctcggcgctattgtgctggcgattggttatgctctggttgcctggtctggtcacgacgccggtatcgtttatatgggtatggcggctattgcggtcggtaacggcctgtttaaagctaacccgtcttctctgctttctacatgctatgagaaaaacgacccgcgtctggacggtgcattcaccatgtactacatgtccgtcaacatcggctctttcttctctatgattgctacgccgtggctggccgcgaaatacggctggagtgttgcgtttgcgttgagcgttgtaggcctgctgatcactatcgttaacttcgccttctgccaacgctgggttaaacagtacggttcaaaaccagacttcgagcctatcaactaccgtaacctgctgctgaccattattggtgttgtggcactgatcgctatcgccacctggctgctgcacaatcaggaagttgcgcgtatggcgctgggcgttgttgccttcggtatcgtggttatcttcggtaaagaagccttcgcgatgaaaggtgctgcgcgtcgtaaaatgatcgttgccttcatcctgatgctcgaagccattatcttcttcgtgctgtacagccagatgccaacgtcactgaacttctttgcgattcgtaacgttgagcactccattctgggtctggccgtagaacctgagcagtatcaggcactgaacccgttctggatcatcatcggtagtccgattctggccgctatctataacaagatgggcgataccctgccgatgccaaccaagtttgcaatcggcatggtgatgtgttctggtgcgttcctgattctgccgctgggtgcgaaattcgcgtctgacgctggtatcgtgtctgtaagctggctggtcgcaagctatggcctgcagagcatcggggaactgatgatctctggtctgggtctggcaatggttgctcaactcgttccgcagcgtctgatgggcttcattatgggtagctggttcctgaccactgccggtgcaaacctgattggtggttatgttgcgggtatgatggctgtgccggataacgttaccgatccgctgatgtcactggaagtctatggtcgcgtattcttgcagattggtgtcgctactgccgttattgcagtactgatgctgctgaccgcgccgaaactgcaccgcatgacgcaggatgacgctgcagacaaagcggcgaaagcagccgtagcgtaaaattcagggaaactcttttacaagccgctaacttttcgttagcggctttttttttgttcagcaacgcactaccatactttaaaccacagacaaaaggagttaccgatgaaattgttctacaaaccgggtgcctgctctctcgcttcccatatcaccctgcgtgagagcggaaaggattttaccctcgtcagtgtggatttaatgaaaaaacgtctcgaaaacggtgacgattactttgccgttaaccctaaggggcaggtgcctgcattgctgctggatgacggtactttgctgacggaaggcgtagcgattatgcagtatcttgccgacagcgtccccgaccgccagttgctggcaccggtaaacagtatttcccgctataaaaccatcgaatggctgaattacatcgccaccgagctgcataaaggtttcacacctctgtttcgccctgatacaccggaagagtacaaaccgacagttcgcgcgcagctggagaagaagctgcaatatgtgaacgaggcactgaaggatgagcactggatctgcgggcaaagatttacaattgctgatgcctatctgtttacggttctgcgctgggcatacgcggtgaaactgaatctggaagggttagagcacattgcagcatttatgcaacgtatggctgaacgtccggaagtacaagacgcgctgtcagcggaaggcttaaagtaatagccatcggcccacaggtcgttgtgggccgaaatgagatatttcagagctttgttgcgctgaagtaatgttctggtttggcaatacgatcctgagcagccaccacttgcagctcatattcctgcattgctttggtggtcaccatgatttcgtagactgcagcggtcacatgttccagcgcctcctgcagcgttgccccctgaagcagtttcaccagcagtaaaccgctcgtcacatcaccaacacctaccggctggcgcataccaaaatccaccagcggacggctgatatgccaggcttcatcggcggtgaccagcagcatttcaaaacggtcacggctgtagccagctcgcgccaggtgtttaaccaacacaatttgtggcccttgcgcaatgagttcgcgcgctgccagaaccgcttcttcgacgttatttaccgcatgctcacagagtatttccagctcaaccagatttggcgcaatgatatcgctggcaggcaaaccgtgccgcacatgaaactctgcgacacccggtgcaacgatacagcctttttccggatgacccattaccggatcgcaaaaatatttcgcctgcggattcgcggctttcacctgacggacgataccgaggatatgttcaccctgctccgccgatcccagatagccacttaatacggcatcacaggtgtgtaatttatcaatggcggcaatgccttgcacaatttcggttaaatggctgggcggcatcacgcagccagtccatttgccgtattgggtgtgattagaaaattgaacggtgttcagcggccagacgttcgcgcccaggcggcgcatcggaaactctgccgcactgttacccgcatgaccataaacaacgtgagactggatagcgagaatatttttcatcatgttccctgtataaaaaccagggggagtgatttctcactccccctttccacttaatgcattatttccagcaaatcagacagtaattctttttaccgcgacgcagtaaggtaaaacgaccaaacagacgatcttcttctttaaagaagtattcaggatcggactgtttttcaccgttaatggtgatggcattggaggcgatagttttacgtgcctgaccacgggaaggttgcagttcagaatcgaccagtgcctgcatcaggtctgcgcccttttccatctcaaccatcggtacgccgtcctgcgccagctgttcgaagtccgcttcactcagcgcactcaaagaaccgctgaacaggcattcggtaatacgttttgccgcctgtaaaccttcttcaccgtgaaccagacgagtcacctgctccgccagtacatactgggcgcgcggtgctttaccgctgtttttatcttcttcttccagggcgttgatctcttcaatgctcataaaggtgaagaacttcaggaagcggtaaacgtcggcatccgcagtgttgatccagaactggtagaatttgtacgggctggttttcttcggatccaaccagactgcgccgccttcagttttaccaaatttggtgccatctgctttagtgatcagcggaacggtcaggccaaacacctgattctgatgcagacgacgggtcaggtcgataccagaagtgatgttaccccactggtcagaaccaccaatttgcagcaccacaccgtactgtttgttcagacaggcgaagtcataaccctgcaacaggttgtaggaaaactcagtgaacgaaatcccctgatcttcacggttgagacgctgcttaaccgcttctttgttgatcatctggttaacggagaagtgtttgccaatatcgcgcaggaaggtcagcacattcatattgccgaaccagtcatagttgttcgccgcgatagcagagttttctccacagtcgaaatcgaggaacggggcaacctgcttacggattttgtccacccactcctgaacagtttcttcggtgttcagcttacgctcggcagctttgaagctcgggtcgccaatcagacccgtcgcgccgcctaccagcgcaaccggcttgtggcccgcctgctggaagcgtttcaggcataacaatggaacaagatgccccaaatgcaagctgtcagcggtaggatcgaagccgcaatagagcgcgatcgggccttgcgccagtcgctctgctaacgcttcctcgtccgtcacctgggctaccagcccccgctcttgcaattgtttaatcaagttactgcttgccatcaaaatctccatgtatataacgactgcacctttgccggtacacgacttttcgccagatgcgaaagagacatagaataaagtgccagaatcaggagtaccagcgattaaagcaagatttttgcatcttttcagggtgcaagacgatcaatcttccacgcatcattttcacgctggtacaaaaagcggtcatgcaggcgatgctcaccaccctgccagaactcaatctgttcaaggctgacgcgaaaaccgccccaaaagctcggcaatggcacttcgccctgttgaaacttctgcttcagctccaggaatttactttcaaggataccgcgggcagaaatgcgactggactgcttcgaaacccatgcaccaatctggctatcacgcgggcggctatgaaaatatttcatcacttcgagagtcgaaagtcgttctgctttaccgatcaccatcacctggcgctcaagggtatgccacgggaacagcaggctaacgcgcggattattttcgatttgatgtgctttacggctgccgaggttggtgtaaaacaccatgcctttttcgtcgtaatgtttgagtaaaacgatgcgctgataaggctgaccatgttcatccacggtagcgaccaccatcgcggtagggtccgccagtttggcttcacaagcctgagagagccaacgttcaaaaagggttaatggatcggcgggaagatcgcggcggcgtaacccgcctttggtgtattcacggcgcagatgcgcgatttgctgcaattcgtcgttatcagacatggttttctttacggattgtcagtgggtgacgctattgtgcgccgcccctggaaaaatctcaacgctgtggattttgtaactgacagttattcaagacgatgcggtcgcgtttatagacagtcgcttcatcgcctttcgaccagaaaacatagattccgtcagtgtaacgcgcgccagaggctgaaatgccctgtttgagatgcagtagttgattatcgtaaacaaaactgacctcctggcgcggattattcagtttgaccgtcaacggtttttcatcacactggtattccagcgtatcggtttgcatgcgctcaaccagctgattaaaggcgctacagccggagagaaggaccggcaaaatgataattaacagttttttcatagtcatatcccgaagactttcctggtctggagggcaatacgccctccctaacgttccaagtgtaacggcagacgcggtaagaaaaattcagttaactctgatatcacgggttagcggggaaaatagcccccagtaccgtctcctggcttgcgccagtgacggaaggcagatttcctggtaatcccgccagcgtccgccaggcaagccaggcgaaagccaatgcttccatgtcatcgccactaatgccaacggcatcggtggtggtgacttctgtgcctggcagtaatgccgccagacgcgccatgagtagcggattacgactacctccaccacataccatcaatcgttcgcagccaccgctcaacaaaacttgttcagaaatggtcacggcggtgagttctgccagtgtcgcctgcacatctcggggatcaacacccggaaaatggcgcaaatggcgctccagccaaccatagttaaagtattcgcgtccggtgcttttcggtgcaggttgcgagaaatacgggtcgctgagcatattttgcagcagtgggagaataactttacccgcccgtgcccactcggcatctttatcgtaaggtttaccggcctgacgccagatccaggcatccatcagcatgttaccaggaccggtatcgtagcccccaaccggctgcccaggaatgagcagtgacagattggcgatgccgccaatattgagcaccattcgtcgctcggttgggtgagccagcagcgcatgatggaacgcaggtaccagcggtgcgccttgtcctcccaaggcaatatcgcgacggcgaaaatcaccgacaaccgtaattccggtgcgtgccacaatttgattgttatcgccaatctgtaaagtgtgtggtgccacgcccgtcggttcatgccagacggtttgaccgtgacaaccgatcgcaactatatctcttgcctgcagattttgttccttaagcaaggcattgaccgcatcagcaaaaagttgcccgagttgagtatcaagctgtccaaactgcgaaagtgtaagctgctggccctggcaaatatccagtacagcctgtttcagagataccgggatcggccaactcaaacttgccagctgtgcgacccggtgttcatcaattgtcgccaacacaacatcaacaccatcaaggctggtgcctgacataacgccaataaagcggcccgatttcatagttcatcctttttcaatctgacgtttgcgcaccactcaaacataaacttttcgtgaataccatgcggaatgaccgatttttaccgttggtagtaaaacattatcttcaaatcaataatcatcatgaatgttttgtttataattggttgatcctactttcattatgatttgctcatatttggtagaacatgtaaccatggattcacatatgccatatactttgaccatgagggatgcttgcgtggcgtttcatggtgaacaggagatttttcaatgattaaacgcgtattggttgtttcaatggtaggtctgtctcttgtcggttgtgttaataacgacaccctgtcaggggatgtttataccgcttctgaagcgaaacaagtacagaatgtcagctatggcaccatcgttaacgtacgtccggtacagattcagggcggtgatgattccaacgttatcggtgcaattggcggtgctgttcttggtggtttcctggggaatactgttggtggcggaaccgggcgttctctggctactgcagcaggcgctgttgcaggtggcgtagctggtcagggcgtacagagtgcaatgaacaaaacgcagggtgtcgagctggaaattcgtaaagacgatggtaataccatcatggtggtacagaaacaaggcaacactcgtttctctccgggccaacgtgtcgtactggccagcaatggcagtcaggtgaccgtttctccgcgctaaataagtttgcgtgtggtcaggttactgaccacacgcccccttcatttcaccctttggcctgtaactcaatgatattatgctcaagttttgcgatgagcgtaatcagttgctccagttcctctgcggagatgccatgtaatatttccgcgcgggttttgttaataacagcttccatttcgctgatcagcggctctgccttttccgtcagtttaatacgtttagcccgacgatcgctggcacaagtttgacgcgaaattaaccctttttcttccagttggtccagagtacggaccagtgatggctgctcgatgccaatcgcttttgccagttgaatttgcgactggtctggaggtaactgatggatattgtgtaacgtaacccaatgggtttgtgttaactccagcggtttcaggcgatggtctatcagagcacgccatatgcgcaccaaccgtgccagatcagaacctagtggcgattccaatttcatctccttataattagcttgctaagatattatgcggcttttagaatagtgtgcagcaattgtattgctaaaacaaatgtattgctgcatttggttaccgtcagacatatttttcagaaattgcgcgtaaatttttcgcacttaaagaatatttattaatctaacgcaatatattcggtcgtaaaggaatctactttgtgaagtttatgctcaatgcaacaggattgcccttacaagatctggtgttcggtgcgtccgtctactttcctccgtttttcaaagcattcgcgtttggattcgtcatctggcttgtcgtacaccgcctgcttcgtggctggatctacgccggtgacatctggcatcccttgttaatggatttatcgctgtttgcgatttgcgtttgccttgctctggcaatactgattgcgtggtaactatgtcaattaaaacaattaagtatttctcaacaatcattgtagcggtagttgcggttcttgccggatggtggctgtggaattattacatgcaatctccgtggacacgcgacgggaaaatacgcgcagaacaggtttctatcaccccacaggtgtcgggacgtattgttgagctgaatataaaagacaaccagctggttaacgcgggggatcttctgctcacgatcgataaaacgccctttcagatcgccgagctgaacgcacaggctcagctggcgaaagcgcaatctgacctcgcaaaagccaataacgaagcgaatcgtcgtcgtcatctctcacaaaattttatttctgccgaagaactcgataccgctaacctcaatgttaaagcgatgcaggccagtgttgatgccgcacaggcgacgctgaaacaggcacaatggcaactggcgcaaacggaaattcgcgccccggtgagtggatgggtgactaaccttactacccgcatcggcgattacgctgataccgggaaaccgctgtttgcccttgtcgacagccactcgttttacgtcattggttattttgaagaaaccaagttgcgccatatccgcgaaggtgcaccagcacaaattaccctctatagtgataacaaaacgttacagggtcacgtttccagtatcggtcgggcgatttatgatcagagcgttgaaagtgactcaagccttattccggatgttaaacctaacgtcccctgggttcgactcgcccaacgcgttcccgtccgctttgcgctggataaagtcccaggcgatgtcacgttggtgtcgggcaccacctgtagcattgccgtaggtcaataatgaacgcatcgtcatggtccttgcgcaatttgccctggttcagggccacgctggcgcaatggcgttatgcgttacgcaataccattgccatgtgtctggcgctgacggttgcctattatttaaatctggatgaaccctattgggcgatgacctcggctgcagtggttagctttcccaccgttggcggtgttatcagcaaaagcctcggacgcatcgctggcagtttgctcggagccattgcggcactgcttcttgccgggcatacgctcaatgagccgtggttttttctattgagcatgtcggcgtggcttggcttttgtacctgggcctgtgcgcacttcacgaataacgtcgcgtatgcatttcaactggcgggctacacggctgccatcatcgcctttccgatggttaatattactgaggccagccagctgtgggatatcgctcaggcgcgcgtttgcgaggtaatagtcggtattttgtgcggcggcatgatgatgatgatcctgccgagcagttccgatgctactgcccttttaaccgcattgaaaaacatgcacgcccgattactggaacatgccagtttactctggcagcctgaaacaaccgatgccattcgtgcagcacatgaaggggtgattgggcagatactgaccatgaatttgctgcgtatccaggctttctggagccactatcgttttcgccagcaaaacgcgcgccttaatgcgctgctccaccagcaattacgtatgaccagtgtcatctccagcctgcgacgtatgttgctcaactggccctcaccgccaggtgccacacgagaaattctcgaacagttgctgacggcgctcgccagttcgcaaacagatgtttacaccgtcgcacgtattatcgccccgctacgcccgaccaacgtcgccgactatcggcacgtcgccttctggcagcgactacgttatttttgccgcctttatctgcaaagtagtcaggaattacatcgtctgcaaagcggtgtagatgatcataccagactcccacggacatccggcctggctcgtcataccgataacgccgaagctatgtggagcgggctgcgtacattttgtacgttgatgatgattggcgcatggagtattgcttcgcaatgggatgccggtgccaatgcattaacgctggcagcaattagctgcgtactctactccgccgtcgcagcaccgtttaagtcgttgtcacttctgatgcgcacgctggtgttactttcgctattcagctttgtggtcaaatttggtctgatggtccagattagcgatctgtggcaatttttactgtttctctttccactgctggcgacaatgcagcttcttaaattgcagatgccaaaatttgccgcattgtgggggcaactgattgtttttatgggttcttttatcgctgtcactaatcccccggtgtatgattttgctgattttcttaacgataatctggcaaaaatcgttggcgtcgcgttggcgtggttagcgttcgccattctgcgtccaggatcggatgctcgtaaaagccgccgccatattcgcgcgctgcgccgggattttgtcgatcagctaagccgccatccaacactgagtgaaagcgaatttgaatcgctcacttatcatcacgtcagtcagttgagtaacagccaggatgcgctggctcgccgttggttattacgctggggtgtagtgctgctgaactgttctcatgttgtctggcaattgcgcgactgggaatcgcgttccgatccgttatcgcgagtacgggataactgtatttcactgttgcggggagtgatgagtgagcgtggcgttcagcaaaaatcactggcggccacacttgaagaattacagcggatttgcgacagccttgcccgtcatcatcaacctgccgcccgtgagctggcggcaattgtctggcggctgtactgctcgctttcgcaacttgagcaagcaccaccgcaaggtacgctggcctcttaattacttaattacaccacaggcatagcgttcaccgccaccgcccagcggtttaggttgatcggacatattatcgccgccaacgtggaccatcagcgctttgtctttgatttcatccagtgatttcagacgaggcgcgatgacggcatcggtagctttgccgtcattattgacgaccagtgcaggcagatcgcctaaatgcccggcaccttctggcccttcatgtttaccggtattttgtggatcaagatgcccgcctgcggattccgcggcgctggctttgccatctttggtggctggctggcagcttcctttggcatgaatatggaagccatgttcaccggggggtaatgctttcagatcgggcgaaaactccagacctttatcggtttcagtaatggtgacgctaccaattgactgccctaccccttgcgacgtgacgaggttcatctcgactttttcactggcagcttgtgcgccggttgcaacaaccagcgccagaatagccagactaaaacgtttcataggacctccgttcattgtgcattcctgaataagtgtaaaccagtgacacatttttgaacggcggctattcctaaaagtgcttacggtacgtcgtaccccagtgccgctttacggatacgaaaccattgttgacgggtcattttcagtgtttctgcttcgacagctgcccgtacgcgctcaattttacctgaaccgataattggcagcggctgcgatggtaaacgtaatacccaggcgtaaaccacctgttcaatcgagcccgcgtttaactcctctgccaccacagccagttcatcacgcagcggctggaaataatcatcattaaacagacgaccaccaccaaggcaggaccacgccatcggacgaacacgcagttgttgtagttggtcgagcgtgccatccagcagtaacggctgatgcaccggggatatttccacctgattagtggcaagggtaaacggcagacgtgattgcaacagggcaaattgcgcaggcgtaaagttcgatacgccaaaatgacgcactttgccgctctgatgcagatgtttgaacgcgtccgccacttcatcggcatccattaacgggtctggtcggtggattaacagcaaatccagatgatcggtcgcgagattaattagcgactgttcggcgctcttaatgatgtgatcgcggtcagtgatgtaatgaccaatgacgttttcttcacgcgcggtcgtcgcgataccgcatttactgacgatttccatccgttcacgcaggtgaggtgccagtttcagtgcctcgccaaacgccgcttcgcactgatagccaccataaatatcagcatggtccacggtggtcacgccgagatccagatgctcttcaataaaactgaccagctggcgggcggacatattccagtccatcaatcgccagtagcccatcacaaaacgggaaaactccgggccttgcggcgcaatagtaatacgctgaaccataatcgcttcctcttatcagatatgagaggagtatacgcaagattaggttcaaaagagtgatggttgctccggttcgtctgatgacgctggcttatttgcgcgtaatttgcgcattaatcgctgccgacaaaggcgcagcacctcttgtttttcgccatcgctcattttattccagttaaaacgctcatcacgactacgaaaacagccgcgacaaaacccgcgttcgtcagactggcaaattccccggcacgggctctggacgggaaagaactctaattgctccgccacttcgccctcctcagataagattattaccattattgaagctgttaatgtccaaagtagcaactttgcttgcactagaccgactggtctactacactccaacgcatgaacaaacacaccgaacatgatactcgcgaacatctcctggcgacgggcgagcaactttgcctgcaacgtggattcaccgggatggggctaagcgaattactaaaaaccgctgaagtgccgaaagggtccttctatcactactttcgctctaaagaagcgtttggcgttgccatgcttgagcgtcattacgccgcatatcaccagcgactgactgagttgctgcaatccggcgaaggtaactaccgcgaccgcatactggcttattaccagcaaacactgaaccagttttgccaacatggaaccatcagtggttgcctgacagtaaaactctctgccgaagtgtgcgatctgtcagaagatatgcgcagcgcgatggataaaggtgctcgcggcgtgatcgccctgctctctcaggcgctggaaaatggccgtgagaaccattgtttaaccttttgtggcgaaccgctgcaacaggcacaagtgctttacgcactgtggcttggcgcgaatctgcaggccaaaatttcgcgcagtttcgagccactggaaaacgcgctggcccatgtaaaaaacattattgcgacgcctgccgtttagcaggcattttttatcaccagacgaccgggagcctttatgtcatctgaaaaactgtattccccactgaaagtgggcgcgatcacggcggcaaaccgtatttttatggcaccgctgacgcgtctgcgcagtattgaaccgggtgacattcctaccccgttgatggcggaatactatcgccaacgtgccagtgccggtttgattattagtgaagccacgcaaatttctgcccaggcaaaaggatatgcaggtgcgcctggcatccatagtccggagcaaattgccgcatggaaaaaaatcaccgctggcgttcatgctgaaaatggtcatatggccgtgcagctgtggcacaccggacgcatttctcacgccagcctgcaacctggcggtcaggcaccggtagcgccttcagcacttagcgcgggaacacgtacttctctgcgcgatgaaaatggtcaggcgatccgtgttgaaacatccatgccgcgtgcgcttgaactggaagagattccaggtatcgtcaatgatttccgtcaggccattgctaacgcgcgtgaagccggttttgatctggtagagctccactctgctcacggttatttgctgcatcagttcctttctccttcttcaaaccatcgtaccgatcagtacggcggcagcgtggaaaatcgcgcacgtttggtactggaagtggtcgatgccgggattgaagaatggggtgccgatcgcattggcattcgcgtttcaccaatcggtactttccagaacacagataacggcccgaatgaagaagccgatgcactgtatctgattgaacaactgggtaaacgcggcattgcttatctgcatatgtcagaaccagattgggcggggggtgaaccgtatactgatgcgttccgcgaaaaagtacgcgcccgtttccacggtccgattatcggcgcaggtgcatacacagtagaaaaagctgaaacgctgatcggcaaagggttaattgatgcggtggcatttggtcgtgactggattgcgaacccggatctggtcgcccgcttgcagcgcaaagctgagcttaacccacagcgtgccgaaagtttctacggtggcggcgcggaaggctataccgattacccgacgttgtaatccaacattgcgagcggcgtaaagccgccgctatactaaaacaacattttgaatctgttagccattttgaggataaaaagatgcgtcttcttcataccatgctgcgcgttggcgatttgcaacgctccatcgatttttataccaaagtgctgggcatgaaactgctgcgtaccagcgaaaacccggaatacaaatactcactggcgtttgttggctacggcccggaaaccgaagaagcggtgattgaactgacctacaactggggcgtggataaatacgaactcggcactgcttatggtcacatcgcgcttagcgtagataacgccgctgaagcgtgcgaaaaaatccgtcaaaacgggggtaacgtgacccgtgaagcgggtccggtaaaaggcggtactacggttatcgcgtttgtggaagatccggacggttacaaaattgagttaatcgaagagaaagacgccggtcgcggtctgggcaactaatctcctgccgggcgtgaactcatcgcgcccgcatctttactgcatcgacaagtaatatttgtcataatgcgcgctgcaatttatccgtattaagagaatcagatgtccgataacgctcaacttaccggtctgtgcgaccgttttcgtggtttttatcctgttgtgatcgatgttgaaacagccggatttaacgccaaaaccgatgcgctgcttgagattgccgccatcaccctgaaaatggatgaacaaggctggctgatgccggacaccacattacatttccacgtcgaaccatttgtcggcgcaaatttgcaaccagaagccctcgccttcaacggcattgacccgaacgatcccgatcgcggcgcggtcagcgaatacgaggcgctgcacgaaatttttaaagttgtacgtaaaggtattaaagcgagcggctgtaaccgcgccattatggtggcgcacaatgccaattttgatcacagctttatgatggccgccgcagaacgcgcctcactgaaacgtaacccgttccaccctttcgccacttttgacactgctgcactggccgggctggcactcggacaaaccgtattgtcaaaggcttgccagaccgctggcatggacttcgacagcacccaggcgcactccgcgctgtacgacaccgaacgcactgctgtgctgttttgtgaaatcgtcaaccgctggaaacgtctgggaggctggccgctatctgccgccgaagaggtgtaatcgagtcgatgcctgatgacatgcaatgattcaggcatctatagtgaggctattccacgcatcctgcatgatattcacggggaatagcgttaatggcagataatccagacccttcatcgctcctgccggacgtgttttcaccggcgacccgcgactggtttcttcgcgcctttaaacagccgaccgctgtccagccgcaaacctggcatgtggcggcgcgaagcgaacatgcgctggtgattgcaccgaccggctccgggaaaacgctggcagcatttctctacgccctcgatcggctcttccgcgaaggcggcgaagatacccgcgaggcgcataagcgtaaaacctcacgcatcctctatatttcaccgataaaagccctgggcaccgacgttcagcgcaacttgcagatcccgttgaagggtattgccgatgaacggcggcggcgcggcgaaacggaagtcaatcttcgcgtagggatccgtactggcgatacgcctgcacaggaacgcagcaaactcacccgtaatccgccggatattctgatcaccacacccgaatcactctatctgatgctgacctcccgcgcgcgcgaaacgctacgcggcgtcgaaacggtaattattgatgaagtccacgcggtagcgggcagtaaacgtggtgcgcatctggcgttaagtctggagcggctcgatgcgctgctccacacctcagcacagcgaattggcctttctgccactgtgcgctcagccagcgatgtggcagcatttcttggtggcgatcgcccggttacggtagtcaacccgcccgcaatgcgccatccgcagatacgaattgtcgtaccggtcgccaatatggatgatgtctcatcggtcgccagcggcaccggcgaagacagccatgccggccgggaaggctccatctggccatatattgaaacgggtatccttgatgaagtgttgcgccatcgctcgaccattgtctttactaattcgcgggggctggcggaaaaactgacggcacgattaaatgagctttacgccgcacgcttacagcgttccccgtctatcgccgttgatgcggcccatttcgagtcgacctccggcgcaacctctaaccgtgtacaaagtagcgacgtttttattgcccgctcacaccacggctccgtctctaaagaacaacgagcaatcaccgaacaggcgctgaaatcgggtgaattacgctgcgtggtcgcaacctccagtcttgaactggggattgatatgggcgcggtggatctggtgattcaggtggcaacgccgctttctgttgccagtgggttacaacgcattggtcgcgccggacatcaggttggcggtgtatctaaagggctgtttttcccccgtacccggcgtgatttagtcgattccgcagtcattgtagagtgtatgttcgcaggcaggctggaaaacctgacaccaccgcataatcctctcgacgtccttgcgcagcaaaccgttgccgccgcggcgatggatgcattacaggtagacgaatggtactcccgcgtacgccgtgccgcaccgtggaaagatctgccaagacgtgtttttgacgccacgctggatatgctttccgggcgctatccctctggcgatttttctgcttttcgccccaaactggtctggaacagggagaccgggatattgaccgcccgacctggcgctcaattgttggcggttaccagcggcggcaccattccggatcgtggcatgtatagcgtgttattacccgaaggtgaagaaaaggccggttcgcggcgggtgggtgaactggatgaggagatggtatatgagtcgcgggtgaacgacattatcactctcggcgctacctcatggcggatccagcaaatcacccgcgatcaggtgattgtgactcctgctccgggtcgttctgcccggctccccttctggcgtggtgaaggtaacggacgtccggctgaattaggcgagatgatcggcgattttcttcatttgctggcggatggcgcgttcttttccgggactattcccccgtggctggcagaagaaaatacgatcgccaatattcaggggttgattgaggagcagcgcaacgcgacgggcatcgttccggggagtcgccatctggtcctcgaacggtgccgtgatgaaattggtgactggcgtattattttgcactctccctatggaagacgggtgcatgaaccctgggcggtggcgattgccgggcgaatacatgcgctatggggcgctgacgcgtcggtggtcgccagtgatgacggcattgttgcacgtattcctgacaccgatggtaaattgcccgatgccgcgatttttttgtttgaaccagaaaagttgctgcaaattgtccgcgaggcggtaggcagctcggcacttttcgccgcccgttttcgcgaatgcgccgcgcgggcattattaatgccggggcgcactccgggccatcgcaccccgctttggcaacaacggctgcgcgccagtcagttgctggaaatcgctcagggatatccggattttccggtcattctcgaaaccctacgcgaatgtctgcaagatgtttatgatcttcccgcactggaacgtttgatgcgtcgcctgaacggtggcgaaattcaaatatccgatgtaacgaccactacgccctcgcctttcgccacaagtttattgttcggctatgtcgcggaatttatgtaccagagcgacgccccgctggcagagcgccgggcatccgtactgtcgctggacagcgagttactgcgcaatctactcggacaggtcgatccgggggaattactcgacccgcaggtcattcgccaggtggaagaagagttgcaacgactggctcctggcagaagagcgaaaggtgaagaaggattgttcgacctgctgcgcgaactggggccaatgaccgttgaagacctggcgcaacggcatacaggcagcagtgaagaggttgcgtcgtatctggaaaatcttcttgcagtaaaacgaatcttcccagcgatgattagcggacaggagcgtcttgcctgtatggatgatgccgccaggctgcgtgatgccctcggcgtacgactaccagagtcattgccagagatttatttacatagagtcagttacccgcttcgcgacctctttctgcgctatctccgggctcatgctctggtcacggctgaacaactggctcatgagtttagtctcggtattgccattgtcgaagagcagcttcagcaactgcgtgaacagggtctggtgatgaatctgcaacaagacatctgggtgagcgatgaagtatttcgtcgtctgcgtttgcgctcgctgcaagccgccagagaagcgacgcgtcccgttgcagccacgacctatgcgcgattgctgctggaacgtcagggcgtattacccgccaccgatggtagcccggcgctctttgcctcaacatcgccaggcgtttatgagggcgtagatggcgtgatgcgggtgatcgaacagcttgccggagtcggtttacccgcctcactctgggaaagccagatcctgcctgcccgcgtacgcgactattcgtcagaaatgctcgatgaattactggcaaccggtgcggttatctggtcggggcaaaaaaaactgggtgaagatgacggcctggtggcactgcatctacaggaatatgctgcagaatcgttcactcccgccgaagcggatcaggcgaatcgttcggcgctgcaacaagcgatagtcgctgttctggctgacggaggagcctggtttgcacaacaaatcagccaacggatacgcgacaaaatcggcgaatcggttgatctctctgccctgcaagaggcgttatgggcgctggtctggcaaggcgtcatcaccagcgacatttgggcaccgttacgcgccctcacccgcagcagttccaacgcacgcacctcaactcgccgcagtcaccgggctcgtcgtggacgtcctgtctatgcgcaacccgtctcgccgcgggtatcttacaacacaccaaatctggctggacgctggtcgttattgcaggtggagccactaaacgataccgaaaggatgctggcgctggcggaaaatatgctcgaccgctacggcatcatcagtcgtcaggcggtgatagccgaaaatatccctggcgggtttccatcgatgcaaacgctttgtcgaagtatggaagactccgggcgaattatgcgaggtcgttttgtagaaggtctgggtggcgcgcaattcgctgaacgtctgactattgaccgattgcgcgatctggcgacacaagccacgcaaacgcgccactatacaccagtggcgctctctgccaacgatccggctaatgtgtggggaaatcttctgccctggcctgcacatccggcaacgctggttccaacgcgtcgggcgggtgcgctggtggtcgtttctggcggcaaattgttactctatctggcgcaaggtggcaaaaaaatgctggtctggcaggaaaaagaggaattactcgccccagaggttttccacgcgctgactaccgcactgcgtcgcgaaccacggctgcgctttacgctaacagaagtgaatgatctaccggtccggcaaacgccgatgtttacgctgctgcgtgaggcgggattttcaagttcgccacaagggctggattggggatagagaaaggactgacggatgcccgttcgcatccgtcagtattgcaggacggattattccgcgtccggctcttcagacttgtatttagcggcagtttctttgatcagctgctgcagttcgccacgctgatacatttcgatcacgatatcacaaccgccgaccagctcgccgtcaacccacagttgcgggaaggtcggccagttagcatatttcggcagttccgcacgaatgtccggattctgcagaatatcaacataggcaaaacgttcgccacatgcggcaagcgcctggactgcctgggcagagaaaccgcagctcggcagtttcggtgaacctttcatgtacagcaggatcgggttttcagcaatctggcgttggattttttcgatagtggtgctcattgtcttgcttcctcaaacttctttacggcagtaatctgacattgtagcgggtcagtgcggcatcggaaaataacattttcatcacgcttttgctattttatccctttgctctatttgttgcatttcaaatattcgtttcttctctgatgccggcaaactggcgtatttataaccatttttagctttcactgctgcatttttttgcgctcgccaacgaaacgtattttttaacaataaaagctattaactttctcttcttctatgcattagaatcatcaagttttgtaaatcagacgcaggcatgatagacctgcctttacagagggacgctcagtggcgcggataaaccgtatttcgatcacgctctgtgctttactttttaccaccctgcctttaacgcctatggcccatgcttcaaagcaagccagggagagttctgctaccactcatatcaccaaaaaagcagataaaaagaaaagcacggcaaccaccaaaaagacccagaaaacagcgaaaaaagccgccagtaaaagtacgaccaaaagcaaaaccgcttcttccgttaaaaaatcttccattaccgcttctaaaaacgccaaaactcgcagcaaacacgccgtcaataaaacggcctcagccagctttaccgaaaagtgtaccaaacgtaagggctataaatcgcattgtgtgaaagtcaaaaatgccgcgtcaggaactcttgccgacgcgcacaaagcgaaggtgcaaaaagctacgaaagtggcaatgaataaactgatgcagcaaattggtaagccatatcgttggggtggcagctcaccgcgtaccggttttgattgcagcggcctggtttattacgcttataaagatttggtgaaaattcgtattccgcgtacggcgaatgaaatgtatcacctgcgtgatgcagcgccaatcgaacgtagtgaactgaaaaacggcgacctggtctttttccgtactcagggacgcggcacagccgatcatgtcggcgtgtatgtcggcaacggcaaatttattcagtcaccgcgcacaggtcaggaaattcaaatcacttctctcagtgaagactactggcagcgccactatgttggcgctcgtcgggtaatgaccccaaaaacacttcgctaaaactttaccctgttgttacggcaacagggtaagttcatcttttgtctcaccttttaatttgctaccctatccatacgcacaataaggctattgtacgtatgcaaattaataataaaggagagtagcaatgtcattcgaattacctgcactaccatatgctaaagatgctctggcaccgcacatttctgcggaaaccatcgagtatcactacggcaagcaccatcagacttatgtcactaacctgaacaacctgattaaaggtaccgcgtttgaaggtaaatcactggaagagattattcgcagctctgaaggtggcgtattcaacaacgcagctcaggtctggaaccatactttctactggaactgcctggcaccgaacgccggtggcgaaccgactggaaaagtcgctgaagctatcgccgcatcttttggcagctttgccgatttcaaagcgcagtttactgatgcagcgatcaaaaactttggttctggctggacctggctggtgaaaaacagcgatggcaaactggctatcgtttcaacctctaacgcgggtactccgctgaccaccgatgcgactccgctgctgaccgttgatgtctgggaacacgcttattacatcgactatcgcaatgcacgtcctggctatctggagcacttctgggcgctggtgaactgggaattcgtagcgaaaaatctcgctgcataataactgatggcaaatgcagcattgcctgaagcgctacgcttatcaggcctacgcggatcatcgatgtaggtcggataaggcactcgccgcatccggcaagataaatcgcacgttgtcagcaactgtaacgcagaaggttatccttctgcgtttttgtttaattagctgttagcaacgcaaactgtttcaggttgttttctggctgacataaacaccagcaataatgccagtcccgcgacaatcgctcccatcaccggcacaaagctgtatcccagcccagcggaaattaccgcaccaccagcagctgctcccagcgcatttccaagattaaaggcaccaatattgactgatgaagacagacctggcgcttcactggcgacacgcatcacgcgcatctgtaacggcggtacgaccgcaaaggttgctgcgccccacaccaccatgctaatagctgcgccgaactcattgcgggccaggaacgggattgccagcataatcaccatcaacaacaacaaaaagcctttcaacgtgccgttaactgaacgatctgccagtttgccgccgagatagttaccgatagagaatccgacaccaatcagcaccagcattgccgtgacgaacaccggtgttgcgtgggtaatactttgcagtaccggagagatataggtgtagagagtaaacattgcaccagctcccagtaccgtcgtcagcaatgcagacagcacctgcggacgcattaataccgccagctcttttttcacttcaggtcgtgcccctgcaccacctttaggtaatgagaagaacagacttaccattgaaatcactcccagccccgccgttgccagaaatgacatccgccagccgatggtttcacccaaccaggtcgccgccggcacgccaccgatatttgccagggttaaccccataaacatagtggcaactgcgctggcctgtttatgttttggcaccacgcttgcggccacgactgaacccaaaccaaaaaatgctccgtgattcaggctggtcaaaatgcgtgaaagcatcagggtcatataatccggcgcgatggcggaaagtacgttgccgagcgtgaaaattgccatcaggaaaatcaacgcactgcggcgggcacgatgagaaagtagaagcgtcatcagcggcgcgccaaccattacgccaactgcataggcactgattaacattccggcagcgggaatcgagacatccacaccgcgcgcaatgacgggcaacaagcccattggcgagaactccgttgtcccgataccaaacgcgccaatcgccagcgccagcaacggatagttaattttcatgccttatctccacctcttcgcgtcattacgcgatattcattaaagtggcgaaagcatgacagcaatcacaaaaaaatgaaaataacaaaaagagaaaacacttttgccattttgctaacaaacaggaaggagatgcgagggagaacgcgctccctcgagaggaaatcagtgcagcgcggcagtcaaacccacggctacgatcaaaccgaggacgataatcgttgttaccagtgaaaatttaaggtcggtgctcatcaagttttctccttttttattaccacacaaaaagtgatattacgcatttttacacactgtgatgaaaaaatctcccgtcatttataatgataagtgtttttaccacttccccttttcgtcaagatcggccaaaattccacgcttacactatttgcgtactggccattgaccccttcctgacgctccgtgtcgtttttccggcgtaccgcaacacttttgttgtgcgtaaggtgtgtaaaggcaaacgtttaccttgcgattttgcaggagctgaagttagggtctggagtgaaatggaatggcaacaataaaagatgtagcgaaacgagcaaacgtttccactacaactgtgtcacacgtgatcaacaaaacacgtttcgtcgctgaagaaacgcgcaacgccgtgtgggcagcgattaaagaattacactactcccctagcgcggtggcgcgtagcctgaaggttaaccacaccaagtctatcggtttgctggcgaccagcagcgaagcggcctattttgccgagatcattgaagcagttgaaaaaaattgcttccagaaaggttacaccctgattctgggcaatgcgtggaacaatcttgagaaacagcgggcttatctgtcgatgatggcgcaaaaacgcgtcgatggtctgctggtgatgtgttctgagtacccagagccgttgctggcgatgctggaagagtatcgccatatcccaatggtggtcatggactggggtgaagcaaaagctgacttcaccgatgcggtcattgataacgcgttcgaaggcggctacatggccgggcgttatctgattgaacgcggtcaccgcgaaatcggcgtcatccccggcccgctggaacgtaacaccggcgcaggccgccttgccggttttatgaaggcgatggaagaagcgatgatcaaggtgccggaaagctggattgtgcagggtgactttgaacctgaatccggttatcgcgccatgcagcaaatcctgtcgcagccgcatcgccctactgccgtcttctgtggtggcgatatcatggcaatgggcgcactttgtgctgctgatgaaatgggcctgcgcgtcccgcaggatgtttcgctgatcggttatgataacgtgcgcaacgcgcgctattttacgccggcgctgaccacgatccatcagccaaaagattcgctgggtgaaacagcgttcaacatgctgttggatcgtatcgtcaacaaacgtgaagaaccgcagtctattgaagtgcatccgcgcttgattgaacgccgctccgtggctgacggcccgttccgcgactatcgtcgttaatcacccgttgcgggagtctcttccggctcccgcagccactccttattcagcgtctcactatcgccgagatactcaagcaaccaggttaacgcaggcgacatatcattttgctgccatgtcagacaacatgccgaatccggaaaggggttttccagttctaatgctacccacttcccctcattaagccacggtttggcgaaatgtgttggcaccatccctatgcataatcctgccgagatacaggttgccgatgattcccagtcaggcacgacaactcttttttggttatccagcaaccaggtaatacgtttaggtagcgttcgcgaggtgtcttcgcgcaccaacgacggccagttgcgcaacgtatcatcgctgaacgggccatccatcaacgccagcgggtggtgactggcaacaacgcaactccagcttagcatccccatatcccggaaggcataacgaccgcctaccggaatcgcgcgtgttgcgccaatcgccagttccacgcgcccgtcggaaagcgcatcccagacaccgttgaacacttcctgaaagacaagaagttcgacatcatcaaaatggcgataaaaatcaacgatcatctgccgtgtacgttctggcctgacaatattatccactgcgatagctaactgaccgcgccagccgttcgctatctgctgacattgctggcgggtgatctgcatttttttgacaacagagcgcccttctttgagaaaccacgctccagcagcggtcagctccacatcacggtgccgtcgttcaaagagcggcaccgccagccactcttccagctgacgcacggtatagctgaccgcagaaggaacgcgatgcagctcctgtgccgcagcgctaaaactaccattacgcgctaccgcatcaacaacttcgagtgaatattctgaccacatagtctgcctgcaaaatttttgaaaccagtcatcaaatattaccgtttcacaacactaatttcactccctacactttgcggcggtgtttaattgagagatttagagaatatacatgcaacctgggaaaagatttttagtctggctggcgggtttgagcgtactcggttttctggcaaccgatatgtatctgcctgctttcgccgccatacaggccgacctgcaaacgcctgcgtctgctgtcagtgccagccttagtctgttccttgccggttttgccgcagcccagcttctgtgggggccgctctccgaccgttatggtcgtaaaccggtattattaatcggcctgacaatttttgcgttaggtagtctggggatgctgtgggtagaaaacgccgctacgctgctggtattgcgttttgtacaggctgtgggtgtctgcgccgcggcggttatctggcaagcattagtgacagattattatccttcacagaaagttaaccgtatttttgcggccatcatgccgctggtgggtctatctccggcactggctcctctgttaggaagctggctgctggtccatttttcctggcaggcgattttcgccaccctgtttgccattaccgtggtgctgattctgcctattttctggctcaaacccacgacgaaggcccgtaacaatagtcaggatggtctgacctttaccgacctgctacgttctaaaacctatcgcggcaacgtgctgatatacgcagcctgttcagccagtttttttgcatggctgaccggttcaccgttcatccttagtgaaatgggctacagcccggcagttattggtttaagttatgtcccgcaaactatcgcgtttctgattggtggttatggctgtcgcgccgcgctgcagaaatggcaaggcaagcagttattaccgtggttgctggtgctgtttgctgtcagcgtcattgcgacctgggctgcgggcttcattagccatgtgtcgctggtcgaaatcctgatcccattctgtgtgatggcgattgccaatggcgcgatctaccctattgttgtcgcccaggcgctgcgtcccttcccacacgcaactggtcgcgccgcagcgttgcagaacactcttcaactgggtctgtgcttcctcgcaagtctggtagtttcctggctgatcagtatcagcacgccattgctcaccaccaccagcgtgatgttatcaacagtagtgctggtcgcgctgggttacatgatgcaacgttgtgaagaagttggctgccagaatcatggcaatgccgaagtcgctcatagcgaatcacactgatctatatcgatatacttatacttaggctgctaacaaaattttgttgtatgattgaaattagcggcctatactaatttcgagttgttaaagctacgataaatattatgtttttacggggacaggatcgttcccgactcactatggatagtcatttcggcaagggttcctcctttccctctgttctacgtcggattatagactcgcggttttttctgcgagatttctcacaaagcccaaaaagcgtctacgctgttttaaggttctgatcaccgaccagtgatggagaaactatgagttcatcgtgtatagaagaagtcagtgtaccggatgacaactggtaccgtatcgccaacgaattacttagccgtgccggtatagccattaacggttctgccccggcggatattcgtgtgaaaaaccccgatttttttaaacgcgttctgcaagaaggctctttggggttaggcgaaagttatatggatggctggtgggaatgtgaccgactggatatgttttttagcaaagtcttacgcgcaggtctcgagaaccaactcccccatcatttcaaagacacgctgcgtattgccggcgctcgtctcttcaatctgcagagtaaaaaacgtgcctggatagtcggcaaagagcattacgatttgggtaatgacttgttcagccgcatgcttgatcccttcatgcaatattcctgcgcttactggaaagatgccgataatctggaatctgcccagcaggcgaagctcaaaatgatttgtgaaaaattgcagttaaaaccagggatgcgcgtactggatattggctgcggctggggcggactggcacactacatggcatctaattatgacgtaagcgtggtgggcgtcaccatttctgccgaacagcaaaaaatggctcaggaacgctgtgaaggcctggatgtcaccattttgctgcaagattatcgtgacctgaacgaccagtttgatcgtattgtttctgtggggatgttcgagcacgtcggaccgaaaaattacgatacctattttgcggtggtggatcgtaatttgaaaccggaaggcatattcctgctccatactatcggttcgaaaaaaaccgatctgaatgttgatccctggattaataaatatatttttccgaacggttgcctgccctctgtacgccagattgctcagtccagcgaaccccactttgtgatggaagactggcataacttcggtgctgattacgatactacgttgatggcgtggtatgaacgattcctcgccgcatggccagaaattgcggataactatagtgaacgctttaaacgaatgtttacctattatctgaatgcctgtgcaggtgctttccgcgcccgtgatattcagctctggcaggtcgtgttctcacgcggtgttgaaaacggccttcgagtggctcgctaaaggctattctatcgccccctctccgggggcgatttcagatcaggcttctgtgcctggttgattcatggcattttctcgtgccgccagcacacgttctaccgtatctaccactgcctgagtttgtggatcgatttcaatgttgacgcgtgcgccaagttttttcttcccaagagtcgtgcgttccagtgtttccggaattaaatggacgcaaaaacgcgttggcgtgacttcgccgacggtcaggctaataccgtcgatgccaataaatcctttgtacagaatatatttcatcaactgactatcctggactttaaaccagatctggcgattattttctgaggttaatattttcgccacttcagcagtggtcataatatgacctgacattaagtgtccgccaatttcatcactgaatttcgccgcacgctcaacgtttacccaatcccccacttttaaatcgccaagattggtaatgcgtaacgtttctttcatcaggtcaaaactgacatggttgccgttaatttccgtcacggtcaggcagcaaccgttatgcgccacggaagcaccggtttccaggccgtccagcatgtggtcgggtaactccaccacatgcgtacgaaaatttggtttctcgtcaatcgacaccagttttgcggtgccctgtacaatccccgtaaacatacttacaactcctgaaatcagttaagacattctgttcagcacaatagcaggtggaaaacgcccttaccagtgaaggggtaagaatggctattttttcactggagaattaataaatcctcgctacaatagactgaatttcccctgcttcttctttttgctgcccattcaggcggctttttagtctctcatataactacaaataaaaggtgttcacgtgcagaagtatatcagtgaagcgcgtctgttattagcattagcaatcccggtgattctcgcgcaaatcgcccaaactgcgatgggttttgtcgataccgtgatggcgggcggctatagtgccaccgacatggcggcggtcgctatcggtacttctatctggcttccggcgatcctctttggtcacggactgctgctggcattaacgccggttatcgcgcaattaaatggttccggtcgacgtgagcgcattgcgcatcaggtgcgacaaggtttctggctggcaggttttgtttccgttctcattatgctggtgctgtggaatgcaggttacattatccgctccatggaaaacatcgatccggctctggcggacaaagccgtgggttatctgcgtgcgttgttgtggggcgcgccgggatatctgttcttccaggttgcccgtaaccagtgtgaaggtctggcaaaaaccaagccgggtatggtaatgggctttatcggcctgctggtgaacatcccggtgaactatatctttatttatggtcatttcggtatgcctgagctcggtggcgttggttgtggcgtggctactgcggcggtgtattgggtcatgttccttgccatggtttcttacattaaacgcgcccgctccatgcgcgatattcgtaacgaaaaaggcaccgcaaaacccgatcctgcggttatgaaacgactgattcaactcggtttgccgattgcgctggcactgttctttgaagtgacactgtttgccgtcgtggctctgttagtgtctccgctcggtattgttgatgtcgcaggacaccagattgccctgaactttagttcactaatgttcgtgcttccaatgtcgctggcggcagcggtaactatccgcgtaggttatcgtctgggtcagggctcaacgctggatgcgcaaaccgctgcgcggaccgggcttatggtgggtgtctgtatggcaaccctgacggccattttcacggtttcactgcgggagcaaatcgccctgttgtacaacgacaatcccgaggttgtaacgctggctgcgcatttgatgttgctggcggcggtatatcagatttctgactcaatccaggtgattggcagtgggattttgcgtggttataaagatacgcgttccattttctatattacctttacggcttactgggtgctgggcttgccaagcggctatattctggcactgaccgatctggtcgttgaacctatggggccagcaggcttctggataggctttattattggcctgacgtcggcagccattatgatgatgttgcgtatgcggttcctgcaacgtctgccgtcagccatcattctgcaacgagcatcccgctaataaagacaaggcgcaaccttcacgggttgcgcctgtatttttacgcaggctggagcgttgcgccaatcccgtcttcgtctggctgtaatttcagagcgttacacagagtttgccgactggcatctgttatctcaacgtgtatatccccggtaacttcccctttcacattgatgaagtcaggtgaaatttcttttgcactggtttgcaggcaaatcgctccctctccgcgcaggcgtttcactttcagttgcacatgcgttgccgcatcagtgatcagccacagttttccaccattcagattgatgttaccaacaatgaaagtgacactgtcaccttttaccgtactgccgtctagaatcaacacaccgccctgctgtacagtaatcgttgattgttgcagctctgcgccataaccaataatcattgaagcgccgtccagtaatgcaacactcccggtcagttcaaccggtgcgcgatcttcctctacgacaaaattttcgtccgcgctggtgggtgacaacaggatcactgtcccaccttgtattaccgcgttttccagcgtaccggcatgcacttcagcccgaccacccacattcacggacaggttttgcgtcttaccggaactgtagagctgaaggccatccgtccccagacgataaatggatccattctcaacaatagtgtcagagtcttcaccaccgagattattcatggtgccaccagcaagcaacgtatcactggctttcccggccagcataaaaacgccgccctgattaatctcacaattgctggcttccccacctggatacaccaacaattcaccaccttcatctaccacgaccgctgaggttgtcccattaaccaacaggccgccctcttgatcgagaatgattttttccgcgcgatgtccttccagtacacgcaggttaccgccattttccagcaacaaaccgcaggcataacctttatcaacgctgaattcaccttcgggatggcggccattaaccgtagcgagcgtagagagactaattgcgcctccctcggactgaacaatatctgtggcaatggcaccatcgctgaccgatagcgtgccattgttaccgtactgtgtgcatttggcgatcccaccggttgccactttcaaccagccagcccccgtgaccacggtattttcggctcttccgccagcttcaacaatcaactcgccttcagtaagttgcgtcgcgccaatgacctcgccggtcttaacaatttgcacgttcccgtcgctcatcaagtttttcgcatcagatcccatgatttattcctttgctgcatctgtgtgcctttattgctacctaagtgtaaaggctacggaggatttatccacgacagatttgagatggtggcaaacaactctgtttaaactctgatacacgaattattgggttgtatcagatgtaaatgcgatcctgaataaaaatcacccttgcaaatcaacaaaatatagccaatttgcttaaaagctctgcaaacggtcgaaatagcgcagaaaattacgttttgcctcttgccaccttcccactctgccgctaatattcgtccccgttgtcacctacaacgttgcgttcatagctcagttggttagagcaccaccttgacatggtgggggtcgttggttcgagtccaattgaacgcaccatcctgcgtccgtagctcagttggttagagcaccaccttgacatggtgggggtcggtggttcgagtccactcggacgcaccagattttcttaatctggtcttctcctttttccctctgtttcttctctgtatccaatacgttaaaagatttacactgtcttcgtatgcgttatcagaaggagaatcgctatggcaactttgttacaacttcattttgcttttaatggcccatttggcgacgcaatggctgagcagcttaaaccacttgctgagtcgattaatcaggaacctggttttctgtggaaggtatggacagaaagtgaaaagaaccacgaagccggtgggatctaccttttcactgatgaaaaaagcgcccttgcctatctggaaaaacatactgcccgactgaaaaatctcggcgttgaggaagttgtcgccaaagttttcgatgtcaatgagccacttagtcaaatcaatcaggcaaaactcgcctgacagaatttaatcaagggcggttagcgcccttttcatccctgtctgaaatttctcaaattctaaaaatctcaaccaaacttatctgataacactaaattcgaaagaatgcgtacaggtaagtaacaatgaaaaaaattgctattgtgggtgccgggcctacggggatctacaccttattctcgcttctacagcaacaaactccactttctatttctatcttcgagcaggctgacgaggccggtgtcgggatgccatacagtgatgaggaaaactcaaaaatgatgctggcaaatattgccagtattgaaataccgccgatttattgtacgtatctcgaatggctacaaaagcaagaagacagccatctccagcgttatggcgttaaaaaagaaaccttgcacgatcgtcagtttttaccgcgaattctgctgggcgaatatttccgcgatcaatttttacgactagtagaccaggcacgacagcaaaaatttgcagtggctgtttatgaatcatgccaggttaccgatctgcaaattacaaatgctggcgtcatgctcgctacaaatcaggatttacccagcgagacgtttgatttagcggtgatcgccacgggtcacgtctggcctgatgaagaagaagcaacccgaacgtattttcccagcccgtggtcaggcctgatggaagcaaaggtcgatgcgtgtaacgtgggtattatgggaacatccttgagcggactggatgcggcaatggcagtggctattcagcatggttcgttcattgaagatgataaacaacacgtcgtttttcaccgcgataacgcaagtgaaaagctaaatatcacgttgttgtcgcgcacgggtattttacccgaagccgatttctattgccctattccctacgagcccttacacatcgtcaccgatcaggcattaaatgctgagattcaaaaaggcgaagagggccttttggatcgggtatttagattgatagtagaggaaatcaagtttgctgatccagactggagtcaacgcatagccttagagagcctgaatgtcgattcctttgctcaagcctggtttgccgagcgcaaacaacgcgacccatttgactgggcagaaaaaaatctccaggaagtcgaacgcaataaacgagaaaaacatactgttccctggcgttatgtcattctgcgcctgcatgaagccgtacaggaaattgttccacatctgaatgaacacgaccataaacggttcagtaaaggccttgcccgggttttcatcgataattatgcggcaatcccttcagagtctattcgtcgcctacttgccttacgtgaagcgggaatcattcatattctcgccctcggtgaagactacaaaatggaaattaatgagtcgcgcaccgtcctgaaaacggaagacaacagctactcgtttgacgtttttattgatgcccgcggacaacgtccgcttaaagtgaaagatatccctttccctgggctacgcgagcaattacagaaaacaggggatgaaatccctgatgttggcgaagattatacgttacagcaacccgaagatattcgtgggcgcgtagcgttcggcgcgttgccctggttgatgcacgaccagcctttcgttcagggacttacggcatgtgcagaaattggtgaggcgatggctcgggcggtcgtaaagcctgcatcccgtgctcgtcggcgtctttcgtttgattaaaggtaaagctatcagcactcaacaaactgatgctgttcattaagacgatagcggactccggctcgaatattgttttcaccttcaatggcgacggcgaagcgaactctttcgccgtcatgatatgccagtgcggcgcttcctcctggcccgagaataattgagtcgaccacgcccgtgctcactaccgttgaattttcaccgctggcaatgatgtgtacattgtcgccgctgttggcaattctggcgtttgcgccaaagctggcgatttgcaccaggtcaccattactggcgacatgacaccgttcacccaatgtacaaacgcgtactcgcattccggtattcgcaatccgactgctatctccagcgctgcttatccgcgaagaattaccggttacagcaacccgtgcgcgttcaccggagctgccaatgtgactgttaaagccgacacttccaatccgcacgctataacccatactggcaatttgcgcggcatacccagcggttgcgattctggcgttatcctcacaacagccgatgcgagcatgatcgtcgctgcgggcaaactgactgcaaaatggtctctctccggggtctgtggccagtttttgcatagaggaaacttcctgatgcgcgaagttttcatccgccagccattttttccacgcatactcaaccagactctccgcccagtccgtatatccttcctcaatcagtgcatgatgaatatcggcataactaccgccgcgtgggaaatggcgcaggaaccagcgatacatcaccgctccgatacgccattctcgcaggtctgcttgtgtaatgatcattcgttagtgccggtgatagccatcgaccatgcttttaaaggtttcgtgtggcgtacgccccgtggtgcaaagataaagatgaccgaagataaaaaagaggcttataaatgccagagcaaaatgtgtctgcaataaccagtatcttacgccaggaaacacatctcccacggcttgcggatagagacacagcagccccgtcaatagtaacaacggcagcaatccatacatgacaccaacataggcgacctgctgtaagggattaaatttagactgggttgttgccgggaaaggatgttcttccccctgcataatgccaaacaaataaaatcgcgtttgttttgccgctcgttccagccacccctgacgacgaatgcgatagtggtgaccattatccccaacggcattgatcagcacaaagccgagccagcatgccagtaacaaaaatccgcaaacttcatgcaccgcaaccagacttttaaccgcagttgcgcccaccatcgcaaagtgatttatcagcccactggccagcaacaatacaaagagtaacgcattcgaccagtgccataatctgaccgctttgctgtaaagataaatcttctcaccatgatcggtggctgatttcttcacgccacgagcacgaagcaaggcatgcagccccagcaccaaccacatcccaaccagcaatactccggcaatgatcaaccacaccggccaaaattcgggagtgaactgtggcacatagttcgctaactggctctgaaactgttcagcatgttgcgacgggttcatacattttcctttttaatcaaatgttgaccgaaccggcgatacagatgcggtttcccggcaccaggtagctgatattgatagtatttattttgctgcaaccacgcctgaatttctgggctatcttcgcgaccaaagatcaatgcgtgttccgggcaggcgctgacgcaaatgggcggaaagccttttgccagtcgggactcagcgcagaaatcacatttatctgccactttagtgacagggttaaggtagcgaacctggtacggacaagcgccaatgcaataactgcagccgatgcactgcgatttttctacccgcacgatcccctgctcatcacgccacgacgcccccgtcgggcaaacgtcgatgcacggagcatcttcgcagtgctgacatgactggcgaaaaaagtgatactgcgtttcgttgtcgttatcggtgactggaatgtgtgctatcgataaacggcttccctgagcggggacgtggttagttttacggcatgcgcgggcgcaaatattacagccattgcaccgtgactcgtcatgaatcatggcataccgaacttccttttcttgcctcgtgttcgctaacagagaagacgcagaaccagtaaaaaagattactgttcccatccccagaacaaatttgcgtcgagtgaaggacatctgattatcccctaatgcagtggctgcaactgtccaccctatccatgacatctccctgaaatttcaggggttctgaaactgctctacctcgaaccattcgcataagccataagccttgccataggtcataaatcgctcgctaaacaagtacaacaccgccgtcgatgactccacctgccgtatatcggcatattcaggtgcaacatccatcgcggcgatcgcggcttcaatctgcgcttcctggaagtaatatggcgcttgcatcagcatggcgactttgtaaggacgaggatacgtctggcactcaaaacgaacggcgtgtgcaatggcgcgacaaatgtcctgctccacaacttgcaaagacatcgccgcgtagttttcactcatggcctgcgttgagtaatagtaatcatccttgcttcccgtcaaacaagcgatatccgcgtagtctccgttctgcttaatgctttccagcaaaactgacagttcctcttctgcaaccaaatagggtggcgagagaaacacggcgcgcgccaccagctgcccagccgcagaatgctggcgaatgaactcagccaggatttcagcaggttctggttcggttaccgtatcaacggggtgacgcatcccctgcaaccattgccgcttcgcctcgtcaacttcgctgactttcgctaacggcaattcatcctgatggttcatcttacccattccttacgcaggcagtagattgtgtgctgccagatcggcggcaatatcttccagccccagacgctgcaatgtttcgcgggttggacaaccaagctgtgggtcccagcccatttctttgtagaacatcgtgagcgaagcatgcatatcgtcacgatccattttgtcagtaccttcagtaaagaccgggatctgcggatccttgtcgaatacccaggaacagataagatcgtgttcattacgcatatctttggtttgcatcagttttaccgtgtaggcacgatgcaacgtaaaaatacgctctgcagctaaatctaatttttcctgagtcatctcttcgccggtgatcgctttgaagaatttggcttcaagcgccagatcgccccggtaattacggcttttcagcggcgaaacggtcattggccagacccagttgcacagggtgacggcgttatgcaaacagacccgcaacagcgaccactttgcatatttaatttttgcgtcattgattggcgtgtagtttttggtttcatcgtaagcatcttcagaaccaaaaagttctttcgccacttcacgttgcagtttcaatggcaagccggaaccaataaagttgatatgggtatgcgtcatgcagtcacggttgaacatacagttaacaatggaaccgacctgcgctgacgcttcattggcatggtgaaccggatagccaaacggcgaccagagtttatttttcgcgtagccccagtactcttcacccaaattccagcgttctgcgatggcatatgaaccatcagccaggtgactcagctcacccacacgatgcgccagacggtagtaaaaatctttaatgaagttaacgtcacccgcttccagttgatcccagcgaatttctgcatactcttcagctggcagaacacgcttgaacacacctttgctgtaacaataagtaaagtcgcgatgcaactgcccgtagttacaccataggccgtagtcatcgaacaaattcagacccaccaggttaccaatcacacgaccatcgtctttatcttcaaaatctttcggcccgttcgggaagatggtggtatggacaaagtttgctacacaagtgttaccacctgtgctgggcacgccaaactctttcacccgaggaatattcatttgggtcatacaacggatcgggcaagagtggcagccgctcatttttactgtgtatttctctgccgccggtcctaagtcaaaaacggatttataggtacgaaagccgaccgtattctgattgcctggcggaatttcacccgtttcaatcggaccaccttcagccgcgccccaaaacagccctttacgtgctgtccagcgtgacttgggatctgaatactctgcccacgattgtggcgtacttggcacgacatggttgttattcgcaccaataagttcagtcatcatgtaatcattgagacgcttcatctcctgacgatcggcaatgttgacccctttcgtcccttcaaccgcaatcgctttcaggtttttcgaacccattattgcgccagttcccgcaccgccgctgtggttacggctattcaacatgccagagagaggaacaaggttttccccagcctgaccaatagccgccacacaggtttccggactggtcaatcgacaaatttcttccgtcgttgcgcgcgtcccttttccccataagaaatcggctttttccaggctaactttgtcatctttaatcttcagccataccggtgatttcgccttcccttcgataataatgacgtcgtatccagcgaatttcatttgcgctgcaaaaaagccacccatatgggcatcgacgactaaatttcctttggtaaaagtagaaagtgaggtgatatttacgcgagaactacagggggcaccagatccagttaatgggccggtagcaaagactaatttattcgcttcatcgaaaggtttcgtgcctggcggtacttcgtcatacataattttgtagccgaagcccatgccaccgacaaaacttttaaacttactggaatcttcgagggtaatatttcctgtcgtgagattgactcttaatatattacctgtccaaccgttagccatgattttttcctttgcaagattcacacagtaatatctttccactcgataatttttaacgcccctgttgggcaggcgtttgcgcattcaccgcataacacacatttcgaggattttttactttcggtatttacggtggccatcatccacgggcatgccgtagtacaggcgctacagccaatacagcgtttatgatcgacggtaatacagccttctttctgctgccaggtaatcgcaccaatcgggcagacgttcatgcattgcggctctttgcattgacggcaggtgtccgcggtatagttgagatcgccatacaggccgccgccagagccaaccccgttgtcgccaaagaaataattgcgatggattttgatacgggagaagaatgtccctactgagccatcgttgaagttggtacaagagatttcacagcggtggcaacccgtgcatcgcgctcgctgggtcaccagcacccctttgggggtatttatcaaccctactgtgccgctatcaatatcttcctgtttgcaacccaaaagtgacagtaacgcaggggcaattgttagaccagcaaggccttttcctgatatacgcaagaattctaatcgcgttaagccaatatctaatagtggacgatcaaccgggttcatttatttcgcatcctcttcgcaaacacagtgctgacaattcagcagcctgatattaagcattcaactaatacgctgctgactctgtccccaacaccagatattttccctaacccgatagtgtatgagaaaagattaacgccgataaactaatcctttatggttaggagaaaaaataatgtgattattctgagcccttaacattgatcgttatcaattaaaattacaaagcaagaaattataagtgaactgatatttattatcatttgaaataaatttaacttaagcgacaattatttgtgactttcattgcagaaaataaaaataacattatcgctataaattaaaatacataccgaaattcgtataatttcagcagttgttatttagaatgattaactggaccgcaactgaagcaagaatatcaggatgaagcttaccgcctcatcctgaatggtcattttaccagtgcgttaatgacggtttccatcgcctgcttttccagctcactgcgctgaatgcgtttattggctaatgctgtacgtaatacgcctgcgataacaatatgctttggttcctgccccagatcgcgcatttccagcacaactttaccgacaactctgcacatttctcggtacagttcatcctcttttgtccgatttcccattctttatacctatttatcatgccaactatcagcatatatcaatctaaccaattaaacaaaaatcaaacaaaatcagacaaataacgcgataaattattttaactgtagcaattgagcgatgatatatttatacaccggatgaactttcacttatcctcacactgacaacttcggcaccagacgttgcgcaaacagtgaagtttttgcgtaaccttttccctggaacgttaaatctttgataacaatttattgtctaacaagttgtatattttttgaaacgctgtttttgttttccttttggattaatttcagcgtataatgcgcgccaattgactcttgaatggtttcagcactttggactgtagaactcaacgactcaaaaacaggcactcacgttgggctgagacacaagcacacattcctctgcacgctttttcgatgtcacctatccttagagcgaggcaccaccactttcgtaataccggattcgctttccggcagtgcgcccagaaagcaagtttctcccatccttctcaacttaaagactaagactgtcatgaaaaagaccaaaattgtttgcaccatcggaccgaaaaccgaatctgaagagatgttagctaaaatgctggacgctggcatgaacgttatgcgtctgaacttctctcatggtgactatgcagaacacggtcagcgcattcagaatctgcgcaacgtgatgagcaaaactggtaaaaccgccgctatcctgcttgataccaaaggtccggaaatccgcaccatgaaactggaaggcggtaacgacgtttctctgaaagctggtcagacctttactttcaccactgataaatctgttatcggcaacagcgaaatggttgcggtaacgtatgaaggtttcactactgacctgtctgttggcaacaccgtactggttgacgatggtctgatcggtatggaagttaccgccattgaaggtaacaaagttatctgtaaagtgctgaacaacggtgacctgggcgaaaacaaaggtgtgaacctgcctggcgtttccattgctctgccagcactggctgaaaaagacaaacaggacctgatctttggttgcgaacaaggcgtagactttgttgctgcttcctttattcgtaagcgttctgacgttatcgaaatccgtgagcacctgaaagcgcacggcggcgaaaacatccacatcatctccaaaatcgaaaaccaggaaggcctcaacaacttcgacgaaatcctcgaagcctctgacggcatcatggttgcgcgtggcgacctgggtgtagaaatcccggtagaagaagttatcttcgcccagaagatgatgatcgaaaaatgtatccgtgcacgtaaagtcgttatcactgcgacccagatgctggattccatgatcaaaaacccacgcccgactcgcgcagaagccggtgacgttgcaaacgccatcctcgacggtactgacgcagtgatgctgtctggtgaatccgcaaaaggtaaatacccgctggaagcggtttctatcatggcgaccatctgcgaacgtaccgaccgcgtgatgaacagccgtctcgagttcaacaatgacaaccgtaaactgcgcattaccgaagcggtatgccgtggtgccgttgaaactgctgaaaaactggatgctccgctgatcgtggttgctactcagggcggtaaatctgctcgcgcagtacgtaaatacttcccggatgccaccatcctggcactgaccaccaacgaaaaaacggctcatcagttggtactgagcaaaggcgttgtgccgcagcttgttaaagagatcacttctactgatgatttctaccgtctgggtaaagaactggctctgcagagcggtctggcacacaaaggtgacgttgtagttatggtttctggtgcactggtaccgagcggcactactaacaccgcatctgttcacgtcctgtaatattgcttttgtgaattaatttgtatatcgaagcgccctgatgggcgctttttttatttaatcgataaccagaagcaataaaaaatcaaatcggatttcactatataatctcactttatctaagatgaatccgatggaagcatcctgttttctctcaatttttttatctaaaacccagcgttcgatgcttctttgagcgaacgatcaaaaataagtgccttcccatcaaaaaaatattctcaacataaaaaactttgtgtaatacttgtaacgctacatggagattaactcaatctagagggtattaataatgaaagctactaaactggtactgggcgcggtaatcctgggttctactctgctggcaggttgctccagcaacgctaaaatcgatcagctgtcttctgacgttcagactctgaacgctaaagttgaccagctgagcaacgacgtgaacgcaatgcgttccgacgttcaggctgctaaagatgacgcagctcgtgctaaccagcgtctggacaacatggctactaaataccgcaagtaatagtacctgtgaagtgaaaaatggcgcacattgtgcgccattttttttgtctgccgtttaccgctactgcgtcacgcgtaacatattcccttgctctggttcaccattctgcgctgactctactgaaggcgcattgctggctgcgggagttgctccactgctcaccgaaaccggataccctgcccgacgatacaacgctttatcgactaacttctgatctacagccttattgtctttaaattgcgtaaagcctgctggcagtgtgtatggcattgtctgaacgttctgctgttcttctgccgatagtggtcgatgtacttcaacataacgcatcccgttaggctccacggaatatttcaccggttcgttgatcactttcaccggcgttcccgtccgcacgctggagaacaaggctttaatatccggtgcattcatgcgaatacaccctgaactgacgcgcaaaccgacgctgtccggcgcactggtaccatgaatgaggtattcgccattaccatgcgcgaggcgcagtgcgtaacgtcctagcgggttatttggtccggcaggaacgactggcggtaatttaatgccacgctccagcgaacgctgacgaatgcctgccgtaggcgtccaggttgggttagggattttctgcccaacacgcgtttccatcaccggcgtttccagcccctgcaatccaatacctattggataaacctgcacaatattttctcccggcggataataataaaggcgcagctctgcaaggttaacgataatcccctgacgcggtgcatcaggtaataacagttgtgaaggaatagttatcgtcgtaccaggttttggcaccggggcgatagtgttattggcttcaaggatcaacattgccgcagtatcaaaacgtcgggcaatagcctgaaggtttttatccccttcttgcaccgtatacgtttgattttgcccaaccagtcggcttccggttggtggtagcggataatcaaccgcccaggcagcctggatggcgctaaaagcgccgataagcgtgagtgtaagcaaagacgcgcgtttcattgtaaacctcctgtatttgccggagactcacgctgaaacgtcggatggcgcttatgttcacctgaaaccaaaacactcctgtgcaggtcagtgtaaacattgaccatccggcaatgtgagccaaccggatgaaagctgtccttttagtttagctaagtgcagcggctttggcgcgaattgcgcgaatcatcgcttccagaccttgtgaacgagatggggtgagatgttgggtgagcgccattttttcaaaccacggacgcacatcgaaattgacaatatcctgcggcgtcatctgatcgtagagaataaagacgaccgcaataagccctttcacaatcgccgcatcgctgtcgccctgtaattcaataattccctgggcattctggcgcatgacaatccacacctgactctgacagccctgaatgctattttgtggacttctgtcttcgtcgcgtaattctggcagacgctggcccagctcaataatgtagagatatttctcttcccagttggcgcagcgtaaaaaattacgcagcaacttttctttatccggcaataaagccatagtgcctccctgttatcccagcaaacggtgaatacgttgcaggccggtcaccagacgatccacttcttcatgggtgttatacatggccagcgacgcccgacacatcgcagggacgttgtaataggccatcaatggcattgcgcagtgatgtccggtacgcacagcaatgccgtaattatcgagaaaactgccaacatcataggcgtggtgtttaccgagattaaaagcaataacgccaagcctgttttgtgggccatagagagtgagatccggtacagattccagctgtgatagcgcataatgcatcagattctgttcatactcggctatgttattaagccccagcgccgaaacatactccagcgccgcgccaagaccaatgatgcccccggtattgggtgtaccggcttcaaaccgccatggtgctttggtccaggtagtgccttcactcaggctgacggtggcgatcatagaaccgcccccttcccacggcggcatctcctgcaacaaggcttctttcacataaagaatgccaattccggtggggccatacagtttatgcccggagaacacgtaaaagtcgcaatccagcgcctgaacatccaccggatgatgcatcaccgcctgagcgccatccaccagcacttttgcgccatgctggtgcgcaagcgtgatcatttccgccagtggattttctgtgccaagcacgttggagacatgagtaattgccagcaggcgagttttctcatcaaacagcgtaggcagcgtctccagttgcaacgtaccatcgggattgagcgggatcacacgcagctctgcgccaacgcgtgcgcaaagcatctgccagggaacaatgttagcgtggtgctccatctgactgatgatgatgttatcgcccgcccgcacgttgctgttgccccagctattggcgaccagattgatcccttccgtcgtgccgcggacgaacaccagctcttccgccgaacgggcattaataaacagcgatgcccgcttgcgcacgttctccattttctcggtcgcctgggcgcttaaggtatgaataccacgatgcaccgccgcgtagccatgacgataaaactcggcctcggcgtcaatcacctggctcggtttctgcgcactggcggcgctgtcgagataagccagcggcaaaccgtttacctcacgcgaaagcaccggaaagtcggcccgcactttgtcgacggaaaaaatcatcttgcacctcctggcagccgttgaccgattcgggccagcacctgctgtttaagcccctcatcacgcagtgcttccgtcagttcggcagcgaaggcgtaaatgatcatctgctgggcatcctgctgattgatcccgcgcgagcgcagatagaatatctgttcatcatcaatacgccccaccgtcgcgccgtggctgcatttcacatcatctgcatagatttccagctgcggtttcgtatccacttccgccagtttgcccatcagcagattgttgttggtcatctgaccatccgttttgatggcgtgctgcgcgacgttgatcaaaccgttaaataccgcgcggcctttgtcgctgacgatagttttgtgcaactgtcggctgttacaaaaacctttattgtgttccagccaggtacgggtatcacacacctcgtttttcaccggcatcgccaggctattgatccgcagcgtgctgttttcgccattgagttgcgtactggtgttgtgtcgtaacactgcgccacccagcaggaaactgtggctaaatgcggtggcatcctcagccagcaacaaatcgttatgagcaaagtggtgactgagcgggttttcaaacgccagcttgatatgctgcaagtgggcattcgctgcgacgttgatagtgaaccgtgccccggtaaaatgacgagcatcattcaggctgacaaaatgttcgatcaccgttgcttcggcaccttccgccagatccagatgatgtcggtaatgggcagtgttcacctcttcacctgccacgccctgggtgatatgcattaacagcaatggctttgccggccgttgaccgcgcttcacggcgatatgcgtcacgctttgtgccaggctttccgtcaaatgcagaaacacttccgcctgaatagcgtcgggtaaaccctgacggtcgtcgttaatgctcacttcatatccgctgccttcagttgcatcgctcagtgcgggcacgtaacgcccatcgacaaacaccagccgcacggagtctaacgttaacgctaaggcatcacgctgctgtggggatatctctcccgcaatgctgacaaactggctattgatcagcccttccagcggcgtatatttccagttttcatgtttacgtgtcggcagtccggtacgcagcaattgttgtaaatgctgctgtgcttgcggggagcgttttgtcccttcagcttcaaacaagtgatgccactgttgcagcgcgttactgctgttcggtaagccagccataaccctgctcctccagttgtttgaccaacgtgaaatcgccggatttcacaattcgtccctgatatagcacatgaacgtaatcaggcttgatgtagtcgagaatgcgttggtagtgcgtaacaatgatgaatgagcgcttgccatcacgcagcgagttcacgccatcggcgaccacttttaatgcgtcaatatccagcccggagtccgactcatcaagaatgcataactccggttccagcaccgccatttgcaaaatatcgttgcgctttttctcgccgccggaaaaaccaacgtttaccgaacgggttaataaatcttccggcatcttcaggagagcgattttctcttccatcaaatcctgaaaatcaaagcggtcgagcgtttcctggccgcgatagctgcgcaccgcattaagtgccgtttgcaggaaaaactggttactgacacctggaatctccaccggatactggaaggccataaagatgccttcgcccgcgcgatcttccggcgacagcgcaagcaaatctttgcctttgaactcaaccgtgccgcccgtcacttcataatcttctcgcccggcaagcgttgccgataaggtacttttgcccgaaccgtttggccccataatggcgtgaacttcgccgggatgaacgtcgaggcttaatccgcgcaggatagctttatcttccacgctgacgtgtaaatctttaatacttaacatgtttattccttatccgacgctgtgttcaagactgatggcgaggagtttttgtgcttcaacggcaaattccaacggcagctccgagaacacgtctttgcagaaaccgttaacaatcatcgagatggcgtcttcttcgctgatcccgcgttgcaggcagtaaaacagttgatcttcaccaatacgtgatgtcgttgcctcgtgttccagttgcgcactattgttacgacactcaacatacgggaaggtatgcgccccacaattagcgccaatcagcattgagtcgcactgagtgaaattgcgcgcattggttgccgtcggcatgattttcactaagccgcgataactgttctgactatgtccggcagagatccctttcgagataatggtcgatttggtgtttttaccgatgtggatcatcttggtgccggtatccgcttgctgatgaccgctggtcagcgccactgagtaaaactcaccaatggagttatcgccgcgcaaaatgcagctgggatatttccacgtaatcgctgacccggtttctgattgcgtccatgacattttgctgttttcgccttcgcacaaagcacgcttggtgacgaagttgagaataccgccggtgttgttatcgccaggaaaccagttttgtaccgtggaatatttcacctcggcgtttttatggatgatgacttccaccactgccgcgtgtaactgatagctgtcacgcaccggagcggaacagccttcaatgtagctgacgtagctgtcttcgtcggccaccagaatggtgcgctcaaactgcccggttttttctgcgttaatgcgaaaataggtggaaagttccatcgggcagcgcacgcctttaggcacataaataaacgtaccatcagaggctaccgccgcattaagcgcggcaaagaagttgtcattccccggcaccacggtgccgagatatttacgcaccagttccgggtgatcgtggatcgcctcaccaaaggaacagaaaataattccctgctccgccagtttttcgcgataagtagtggcaaccgaaactgagtcgaaaatggcatccaccgccacctctttgccttcccgcacgggaacgcccaactgctcaaacgccgcctccacctctttacttaaaaaggcgttcgcgccagtttgctgcaccgcgccaggttcagacgcgcaagtgtcgtcacaattaccgcacgatggtgctgagtagtagctgtaatcctgataattcagcttgtcgtagtgcgctttcaaccagtgcggttcttccatctccagccatgcgcgataggcgtttagacgaaactccagcatccactccggctcattacgcttcgccgaaattgcgcgcaccacctcttcgtttatcccctttgccagctcatcggtggctaactgggtgaagaatccttctttataattcagcgggccgccggtccaggttttgacatcgtcagttgcttcagtattacgagacatagtaccgcctataccccaaagctttcgccacagccacattcattctgggctttagggttgtgaaatttgaatatctgattaagtccttcacgaacgaaatcgacttccgtgccatcaataaacggcatcgcttgcagcgggacaaacagcttcgcgccgtcgtgttcaaacagcagatcgtctttgtccggctcgctaacactgtcgagcacatagccaaagcccgcgcagcccgtttgcttcacgcctaagcgcacgccgaccatacccggctgctttgccaccagctcacggatgtgtatcgccgctgcgggtgtcagcgttaagccttgccaggcgaaatcttgtgggttaaaggttcctgaatgcatgtccatcgatttacctcacttcatcgctttcagcgtataacagcatgttagtgataatgattatcagttcaacccagcaaacgcaggggctttaccgtaaaacatgctttttgcctgcttttaataagcatagaccctgatgtgtgggttaacaggcacgctaagaattaggtatctcattgttagataatggttattatctaaggagcattaaggctgtgatgaaaaagaaaaagttgtattgaaaatgactatttaagagataggtaaaaaagtgcagcgttcagaaataagaaaacccttaagtctgtgcgacacaggcttaagggtttctaccccatccggcgcttatctccggcactctcagtggcttagctcttgaaggggcgataagaataatctcataaagctaacccgccgttttaacacaaactgcgattagtattatttttgaacaatatcaggcggtagataagcagtattaagaaggtcatcgaacctggacggaggttaatccaggtcgatttggcgaacttgcggcattaagtcaggatcaatgcacgcccagacgccaggcaaagtagatttcttcttttaattcagcagaagagagagtaagcaggtcagcaaattcaagttctagttgtttcagacgtttgagatattgggcaggtgaaagattgctctggtcacggcgtaaaaattcaatggccagctgggtgggatcaagttgagtagacatagcatcctcgcttttagacaagacctgcacagtataccaccgtttactgtgcagataatgaccaaaagcaatatgcgtcacacttttctggtgacaacgtcacaaaatggcggtcgtcaatcgtgacgaacagcacaaacgccctttctcatcgaagatttcaatctgccagacctggtgacgcgaaccgagatgcaacggtttgcatacgccgcgcacccgcccttctcgtgccgagcggacgtggttagcattgatttccagaccaaccactttttgctcaccttcggtacataaataaccggcaacggaaccgatactttcggccagtaccacggatgctcctccatgcagcaacccgaaaggctgctttgtccgcgagtctactggcattgtcgcttcaagggtgtcatcaccaatatgttcaaagcgaatatccaggaaccccaccatgtttccttcacccatagcattcagtgcttccagggtgattttccgtttccatatcatttaataatctccagtaaagcctgcacaggatggcgtacccccgtgccttcaacccgttttacctggctacggcaggaatatccggtcgccagacagcggttacgcggcagtcgctgcatagcctgatgccaggataactcatagatcccgagcgaattttcatggtttttcgcttcatgtccgtaagtccctgccatgccgcagcaacccacgctgacattttccagtttcgcgccaaaacgggcaaatatcgcggcccattgtgctggcgcacccggcaaggcggtaacttcggtacagtgaccaaagaaataccatgattcaccgctgactgtagccactggctgtgactcaagtgcgcttgccagccattcattcgccagtaagacgttaaactcgccacgctcctcgcccagcgccagtttatattcatcgcgataacaaagtaccagcgccggatcgacgcccaccattggcatacccagcttcgccatacggttgaggaaatccgccgtctttttcgccgtcttcgcaaaacgattaagaaaacctttaatatgctgggctttgccatttggcgaaaatggcagtaacacaggctggaaacctaatttttcgaccagacggacaaaatccgccaccacttgcgcatcgtaatagctggtaaaggggtcctgcaccaccaacactgtgcgcgctttctgctctgcattgagagattcaagctgttccagcgtcatgtttgccgagcgatgccccaccatttgttgttgtagcgaggggaccgacagcagcggcaaatcaaccatgccgatatgtttttccgagagtttgcgcaccagcggctggttaatgaagaagttaaaggttttcggcgcgcgtgccatcagcggcgcgtagctctcgaccgtagcgacgaggtggtcgcgcagcgggcgtaaataacgggtgtgatagagctgcagaaaacgagagcgaaactccggcacatcaattttgatggggcactgggtcgaacacgctttacaggccagacagcccgacatcgcctctttgacttcgtgtgagaagtcatattcgcctttattcgcatgccagctattgcgcgtgcgggcaattaacgtccgcaaactgacgccggattcaggcagttcttgttccagtttgagtggatcaacgccgcgatccgccaacaaacgcagccattcacgcaccagcgttgcgcgccctttcggtgaatgaatccggttctgggtgatcttcatcgacggacacatcggactacgggcatcaaagttgaagcataaaccgttgccgttacactccatcgcaccgcgccactgctggcgtaccgcaatggggatctgccgatcgaatgtaccgcgcttcaccgcgtccactttcatcatcggcgcatcgagaccttctggcgggcaaatcttccctgggttgagtcggttatgcgggtcaaatgccgctttcactttgcgcagttctgcaaaaagttcctcaccgaaaaacgccgggctgtattcagcgcgaaaacctttgccgtgctcgccccacaacaaaccaccgtatttcgcagtcagcgccaccacgtcatcagagatttgcttcatcaaaatctcttgttgaggatcgcacatatccagcgctggacggacgtgcaagacacctgcgtcgacgtgaccgaacataccgtagcttaagccgtggctgtcgagcagcgcgcgaaattcagcaatataatccgccaggtgttccggcggtacgcaggtatcctcagcaaacggaattggcttagcggcacctttggcattgccaagcagaccaacggcttttttgcgcattgcatagatacgttcaacccccgccagctcacggcacacctgccagccgatgacacctgcttgatgactggcgatcagctcatccaaccgcgcacagagtgcatttacccgctcatcaatcagcgcctcatcatcaccagcaaattccacaatgttcagcccgagcatctcttggtcaggcacatcggtaatcaactcgctgacggaatgccagacaatatcttcccgcgccagattcagcacttttgagtccaccgtctctaccgaaagcgcccgcgcctcaaccataaacggcgcgttacgcagcgcagagtcaaaagagtcatatttgacgttcaccagacggcgcactttaggcaagcgtgtaatatccagccgcgcttcggtaataaaggccagcgtcccttctgaacccgtcagaatgcgcgtcaggtcgaactcggtcatctcatcgttaaagacatgacgcagatcgtaaccggtaagaaagcggttaagtttggggaagttgtcgataattaactggcgttgctgacggcaacgttgataaaccgtgttataaattcgcccgattgtggtattggatttacccagcgtttccgccaattcgacgggtaaaggttgcgtatcgagaatatcgccccccaacaacaccgcgcgtacgccaagtacgtgatctgacgttttgccatagaccagcgatccctgaccggatgcatcggtattgatcatcccaccgagcgttgcccggttgctggtcgaaagttccggcgcaaaaaagtagccgaacggtttcaggtactgattgagttgatcttttatcaccccggcctcaacgcgcacccagccctcttcagggttaatttcgatgatgcggttcatatggcgggacatatcaacaataatcccctggttgagcgcctgaccgttagtgccggtgccgccgccgcggggggtaaagatcagcgatgaatagcgttcctgcgcggcaagacgggcgatcagcgccacatctgcggttgaacgcggaaataccaccgcatcggggagaagttggtaaatactgttgtcggtcgacattgtcagacgatcggcataacttgtcgccgtatcgccggtaaaaccttgttgctccagctcttgcaaaaaattaagcaccagttgaacgacgccgggtgcctgggaaatctgtggaatcattatattgaccctttcctgcggtctgtgatgtaggtcgatacactattctttcaggctgctgcaatagcgcactgaaaggtgatgtttgtttactctatggatttcgtgttgcaggaaggcggcaagcgagtgaactccaggagcttacaatagtaagtgactggggtgaacgaacgtagccgcagcacatgcaacttgaaatacgacgagtaaatcgtttgcgtgttgcctgagttgttgtaccacatttttttctaacacgcccatcagaattaagggcagaatcggcctgttaaaaaccgctgaaattgctcatcattatgcaggtgagtttcgcgtgttcacgtcgcgtcgacgatttgacgcacaaaaaaggtgaaaagtagttatggtaaatgttcgtcagcccagggatgtcgcacaaattctgctttcggtgctgtttttagccatcatgattgtggcatgtctgtggattgttcaaccctttattctcggctttgcatgggccggtacggtggttatcgccacctggccggtattgttacgtttgcaaaagatcatgtttggccgccgctctctcgccgttctggtgatgacgctgttattagtgatggtgtttatcatccctattgctttgctggttaacagtatcgtcgacggcagcggcccgctaattaaagccatttccagcggtgacatgacgttacccgatctggcgtggcttaataccattccggtgattggcgcgaagctgtatgcaggctggcacaacttgctggatatgggggggacggcgatcatggcgaaagtccgcccttatattggcaccaccaccacctggttcgttgggcaggcggcgcatatcgggcgctttatggtgcattgtgcgctgatgcttctcttcagtgccctgctgtactggcgcggtgaacaggtggcacaaggcattcgccattttgcaacccgtctggcaggcgttcgcggagatgccgccgtgctgctggcggcacaggctatccgcgcggtggcgctgggtgtggtggtgacggcgttagtacaggcagtgcttggcggtatcggcctcgccgtatccggcgtaccttatgcaacgttgctaacggtgttaatgatcctctcctgccttgtccagcttggcccgttgccggtactgattccggcgattatctggctctactggactggcgataccacctggggaacggtattgttagtgtggagcggtgtggttggcacgctggataacgtcatccgcccaatgttaattcgcatgggtgccgatttaccgctgatcctgattctctctggcgttattggtggtttgattgctttcgggatgatcggtctgtttattggtccggttctgttagccgtttcctggcgtctgtttgccgcgtgggtggaagaagtcccgccgccgacggaccaaccggaagaaattctcgaagaacttggcgaaatcgagaaaccgaataagtaatttctcatcaggcggctctgccgcctgattgttaaccaccgctaattgatatttgcttgctcttccccatattttcctgcttaccgccattcagctggtagtacctgtcgcaaattctttacagtttttaaactaatgagacgaatctgatcgacgcaaaaagtccgtatgcctactattagctcacggttataaatcaacatattgatttataagcatggaaatcccctgagtgaaacaacgaattgctgtgtgtagtctttgcccatctcccacgatgggcttttttttaacatttttccgcttcgctacctcgcccctcactctttccaataatgttgcacaagatactgtgactctcttcaagccgtcagcaggctgataatgttatttatattttattgtttatttcatgcagccattacacgatgaacgcttatgaactccaggcactccgccatatttttgccatgactattgatgaatgcgcgacctggattgcccagaccggtgacagtgaaagctggcgtcagtgggaaaatggcaagtgtgccattcctgatcgtgtagtcgagcaactgttggctatgcgtcagcaaagaaaaaaacatcttcatgccatcatagagaaaataaataaccgcatcggcaacaacaccatgcgttttttccccgacttaaccgcatttcaacgagtctaccctgatggcaattttattgactggaagatctatcaatcggtagctgctgaattatatgcacacgatctggagcggctttgttaatttttccacagaaaggaattgtcgttgttacaacaataatgaacggatgctgacacaacatcgcttcactttttaaagcacctttgctaagtagaacctatgaaaaatccctatttccctaccgcacttgggttgtattttaattacctggtgcatggtatgggcgtccttttgatgagcctgaatatggcctcgctggagacactttggcagactaatgccgcgggtgtctcgatagttatctcatcgctgggcattggtcgattaagtgtcttgctttttgcaggattattatccgatcgctttggtcgccgcccttttatcatgctcgggatgtgctgctatatggccttcttttttggcatcctgcagaccaataacatcattatcgcttatgtttttggctttctggcgggaatggcaaacagttttctcgatgcaggcacttatcccagtttgatggaagcttttccacgctcacctgggacagccaatattttaattaaagcatttgtttccagcggacaatttttattaccgctaatcattagcctgttagtgtgggctgaactgtggttcggttggtcctttatgattgctgcaggcattatgtttattaacgctctgtttttataccgttgtacgttcccaccccatccgggtcgtcgcttacctgtcataaagaaaaccaccagctctacggaacatcgctgttcaattatcgatttagccagttataccttatatggctatatctcaatggcaacgttttatctggttagccagtggctggcacagtacggacaatttgttgcaggcatgtcatacactatgtcgatcaaactactcagtatctacaccgtgggttcgctgctttgtgtatttattaccgctccactcattcgtaataccgttcgcccaacaacattactgatgctgtacacctttatctcatttattgctctgtttaccgtctgcctgcatcccacattttatgtggtgataatatttgcttttgtcattggttttacctctgctggaggtgttgtgcaaattggcctgacgttaatggctgaacgtttcccttacgctaaaggtaaagctacagggatctattacagtgcgggcagtattgcgacctttactattccgttgattacggctcatctgtcccaaagaagtattgccgatattatgtggttcgataccgccatcgctgccatcggttttttactggcactgtttatcggcttacgcagccgcaaaaaaacgcggcatcactcgctaaaggaaaatgtcgctccgggtgggtaatgcaatattcttttcaggtcatgcaagatcttacggataaataactctttctgcgctaactaaggaaaatcgcgatcaaaaacaaactatgacatgcaatattcctggaaacataaactttatgccatgtacccagggaaaatcatcttcagtatagtaattatgtaaaccgtcggagaacaatacgtacggtaacgaaattatctttcagcaaggagctgtgaaaatgtctcaaaataaggctttcagcacgccatttatcctggctgttctttgtatttacttcagctacttcctgcacggcattagtgttattacgcttgcccaaaatatgtcatctctggcggaaaagttttccactgacaacgcgggcattgcctacttaatttccggtatcggtttggggcgattgatcagtattttattcttcggtgtgatctccgataagtttggtcgtcgggcggtgatattaatggcagtaataatgtatctgctattcttctttggtattcccgcttgcccgaatttaactctcgcctacggtctggcagtgtgcgtaggtatcgctaactcagcgctggatacgggtggctaccccgcgctcatggaatgctttccgaaagcctctggttcggcggtcatactggttaaagcgatggtgtcatttgggcaaatgttctacccaatgctggtgagctatatgttgctcaataatatctggtacggctatgggctgattattccgggtattctatttgtactgatcacgctgatgctgttgaaaagcaaattccccagccagttggtggacgccagcgtaactaatgaattaccgcaaatgaacagcaaaccgttagtctggctggaaggtgtttcatcggtactgttcggtgtagccgcattctcgaccttttatgtgattgtggtgtggatgcccaaatatgcgatggcttttgctggtatgtcagaagctgaggcattaaaaaccatctcttattacagtatgggctcgttggtctgtgtctttatttttgccgcactactgaaaaaaatggtccggcccatctgggctaatgtatttaactctgcactggcaacaataacagcagccattatctacctgtacccttctccactggtgtgcaatgccggagcctttgttatcggtttctcagcagctggcggcattttacagctcggcgtttcggtcatgtcagagttttttcccaaaagcaaagccaaagtcaccagtatttatatgatgatgggtggactggctaactttgttattccactgattaccggttatctgtcgaacatcggcctgcaatatatcattgttctcgattttactttcgcgctgctggccctgattaccgcaattattgtttttatccgctattaccgcgttttcattattcctgaaaatgatgtgcggtttggcgagcgtaaattttgcacccggttaaacacaattaagcatagaggttaaaggagttaattatggatgttaccgcaaaatacgaattgattgggttgatggcctatcctatccgccacagtttatcgcccgaaatgcagaataaagccttagaaaaagcgggattgccatttacctatatggccttcgaagtggataacgatagctttcctggagcaattgaaggattaaaagccctcaaaatgcgcggaactggtgtatcgatgccgaacaaacaactggcgtgtgaatatgttgatgaattaacaccagctgccaaactggtgggggccatcaacaccatcgttaatgatgatggctatctgcgtggctataacaccgacggcacgggccatattcgcgccattaaagagagcggttttgatatcaaaggcaaaacgatggtgctgttaggggccggtggtgcctcaacggcaattggcgcgcagggggcaattgaaggtttaaaagaaattaaactctttaaccgtcgggatgagttcttcgataaagccctcgccttcgcgcagcgggttaatgaaaacaccgattgtgtcgtcacggtcaccgatctcgccgatcagcaagcctttgctgaagccctggcttccgccgacattttaaccaatggcacaaaagtgggtatgaaaccccttgagaatgaatcattggttaatgatatcagtctgttacatccgggacttctggtcactgaatgcgtgtataacccgcatatgacgaagttattgcagcaggcgcaacaagctggttgcaaaacgattgatggatacggcatgttgttgtggcaaggggctgaacagttcacattatggactggcaaagatttccctctggaatatgttaaacaggtcatggggttcggtgcctgacaggctgaccgcgtgcagaaagggtaaaaaatgaaaaccgtaactgtaaaagatctcgtcattggtacgggcgcacctaaaatcatcgtctcgctgatggcgaaagatatcgccagcgtgaaatccgaagctctcgcctatcgtgaagcggactttgatattctggaatggcgtgtggaccactatgccgacctctccaatgtggagtctgtcatggcggcagcaaaaattctccgtgagaccatgccagaaaaaccgctgctgtttaccttccgcagtgccaaagaaggcggcgagcaggcgatttccaccgaggcttatattgcactcaatcgtgcagccatcgacagcggcctggttgatatgatcgatctggagttatttaccggtgatgatcaggttaaagaaaccgtcgcctacgcccacgcgcatgatgtgaaagtagtcatgtccaaccatgacttccataaaacgccggaagccgaagaaatcattgcccgtctgcgcaaaatgcaatccttcgacgccgatattcctaagattgcgctgatgccgcaaagtaccagcgatgtgctgacgttgcttgccgcgaccctggagatgcaggagcagtatgccgatcgtccaattatcacgatgtcgatggcaaaaactggcgtaatttctcgtctggctggtgaagtatttggctcggcggcaacttttggtgcggtaaaaaaagcgtctgcgccagggcaaatctcggtaaatgatttgcgcacggtattaactattttacaccaggcataagcaataatatttcggcgggaacaccctccccgccgaactaaaaaatatattcaatcgtatttaataaaaatatttcgtgagtctctgtgcgctaattctccatttggcgtagggaaaatcacatctgaatcaggaattaacaatgaaacctgtaaaaccacctcgtattaatggacgagtgccggtcctgtcggcacaggaagcggtgaattatattcccgacgaagcaacactttgtgtgttaggcgctggcggcggtattctggaagccaccacgttaattactgctcttgctgataaatataaacagactcaaacaccacgtaatttatcgattattagtccaacagggcttggcgatcgcgccgaccgtggtattagtcctctggcgcaagaaggtctggtgaaatgggcattatgtggtcactggggacaatcgccgcgtatttctgaactcgcagaacaaaataaaattattgcttataactacccacaaggtgtacttacacaaaccttacgcgccgccgcagcccaccagcctggtattattagtgatattggcatcgggacatttgtcgatccacgccagcaaggcggcaaactgaatgaagtcactaaagaagacctgattaaactggtcgagtttgataacaaagaatatctctattacaaagcgattgcgccagatattgccttcattcgcgctaccacctgcgacagtgaaggctacgccacttttgaagatgaggtgatgtatctcgacgcattggttattgcccaggcggtgcacaataacggcggtattgtgatgatgcaggtgcagaaaatggttaagaaagccacgctgcatcctaaatctgtccgtattccgggttatctggtggatattgtggtggtcgatccggatcaaacccaactgtatggcggtgcaccggttaaccgctttatttctggtgacttcacccttgatgacagtaccaaacttagcctgcccctaaaccaacgtaaattagttgcgcggcgcgcattattcgaaatgcgtaaaggcgcggtggggaatgtcggcgtcggtattgctgacggcattggcctggtcgcccgagaagaaggttgtgctgatgactttattctgacggtagaaacaggtccgattggcggaattacttcacaggggatcgcctttggcgcgaacgtgaatacccgtgccattctggatatgacgtcccagtttgatttttatcacggtggcggtctggatgtttgttatttgagttttgctgaagtcgaccagcacggtaacgtcggcgtgcataaattcaatggtaaaatcatgggcaccggtggatttattgatatcagtgccacttcgaagaaaatcattttctgcggcacattaactgcgggcagtttaaaaacagaaattaccgacggcaaattaaatatcgtccaggaaggacgggtgaagaaatttattcgggaactaccggaaattactttcagcggaaaaatcgctctcgagcgagggctggatgttcgttatatcactgagcgcgcagtattcacgctgaaagaagacggcctgcatttaatcgaaatcgcccctggcgtcgatttacaaaaagatattctcgacaaaatggatttcaccccagtgatttcgccagaactcaaactgatggacgaaagattatttatcgatgcggcgatgggttttgtcctgcctgaagcggctcattaacaggagtataatgatggatttttctttaactgaagaacaagaactgctgctggccagtattcgcgaactgattacgactaactttccggaagagtatttccgcacctgcgatcaaaacgggacatatccgcgtgagtttatgcgggcgctggcggataacggtatttccatgcttggcgtgccggaagaatttggtggtatccctgcggattacgtcacccaaatgctggcgctgatggaagtgtcaaaatgcggtgctccggcatttttaattaccaacggtcaatgtattcacagtatgcgccgtttcggttctgcagagcagctacgtaaaacggcagagagcaccctggaaacgggtgatcccgcctatgccctggcgttgacggaaccaggtgctggctcagataacaacagtgccactaccacttacacgcgtaaaaacggcaaggtctacatcaacggacaaaaaacctttattaccggtgcgaaagagtacccgtatatgctggtgctggcgcgcgatccgcaaccgaaagatcccaaaaaagccttcaccctgtggtgggtcgactccagtaagcccggcattaagattaacccgctgcataaaatcggctggcatatgctcagcacctgcgaagtctatctcgacaacgtggaggttgaagagagcgacatggtgggcgaagaaggaatgggtttcctcaatgtgatgtacaactttgagatggagcgcctgatcaacgccgcgcgcagcaccggctttgccgaatgcgcctttgaagatgccgcccgctatgccaaccaacgtatcgcttttggtaagcccattggtcataaccagatgatccaggaaaaactggcgctgatggcgattaagatcgacaacatgcgcaacatggtgctgaaagtggcatggcaagccgatcagcatcagtcactgcgcaccagcgcggcgctggcaaaactgtactgtgcacgtaccgcaatggaagtcattgatgatgcgattcaaatcatgggcggtctgggctataccgatgaggcgcgcgtctcccgcttctggcgtgatgtccgttgtgaacgtatcggcggcggtacagacgaaattatgatttacgtagcaggtcggcagatcctgaaagactatcagaacaaataatctgcaggcggcgcagcttcttaacaaactgcgccgccagatttatccaacaagacttaccggttgaggaaattcagataggatttcttgttccgcaaaacagtttttaaattgtctacggtaatcgctgggcgaacaaccgacatggcgcaaaaacagtttggcaaagtgatcgacattttcataacccacacgccaggagatctctgcctgtgataattcagtattagtgagtgaccattttgcttccgtcatacgccgttgaataacatagttaataggggaaatacgatactctttggtaaattcatggcaaatataactgacgctggcacgaaattttttcgataactgttctaaagtgattttttcgcgataattattattcagatagaaaagaatatcttttatcagaacatcttttttaatatacccctgctccgaacgataagcatttttaaaattttcgtagtaaagaatggctaacgtataggcaaatgcatcccataacgaagatgtttggctatttttactttgcggcaaaatcacacttagctcattaaataaggtttttatgacttcttttccctgccccgcggcaattaccggacaagaatgcggttgcagtagctgattttcctcagccccctgaaactgaaagccgtacagcgcacaggtacacgtcgttgccggatcgttaacgtcagaggccaccgcatgcagcctgccgcgttctatcaccacaatgtcatccgcatgtgcgacatataacgaagaatcgatggtaaaccttgcaacccctttcttgacgtaaatcaactcggtttcattgtcatgaacgtgatgtccggactcccattttggatcatcgctaaatgcaaaacgtgaaagccgtggcgttttaccggcgacaaacagcgtttcactggcgttatcaaaacagcgttgatacatgacaacctccctattccatgagcaagcaaaaacaatatatgccggataaaatacggcgtgtattgcggttatacaaccgcgtttagcgagagctaaacaagattatttacactgaatgcaagattgtacggtcatggaataactatattgccgcaaattgcacttttgttttagcgatcgcattttttttgcaagattgttggcaaggaaaacagcttgctccgtcgaaaaccccgcaccgctatcgcacactattttcaggccatttttaccttccatcggagatggttccgtatgcgactcacaggagaaatcatgaaaataataacctgctttaagctggtgcctgaagaacaggacattgttgtcactccagaatacaccctgaatttcgacaatgccgacgccaaaatcagccagttcgatctcaatgccattgaagctgcaagccagctcgcaacagatgacgatgagatagccgcgctgaccgttggcggctcattgttgcagaactcgaaagtgcgcaaagacgtgctatcccgcgggccgcacagcctgtatttggtgcaggatgcgcaacttgaacatgcactgcctctcgataccgcaaaagcgctggcggcagcaattgaaaagatcggcttcgatttactgatctttggtgaaggttccggcgacctttatgcccagcaggttggcttgctggtcggagaaattctgcaacttccggtgattaatgcagtgagtgctattcagcgtcagggcaatacactggtgattgaacgcacgcttgaagatgatgttgaagttattgaactctctgttccagccgtgctctgcgtcacctccgatattaacgtgccacgcattccttcgatgaaagccattctcggcgcgggtaaaaaaccggtaaatcagtggcaggcaagtgatattgactggagccagagcgcgccacttgctgaactggtcggcattcgcgtaccgccgcaaacagaacgtaagcacatcattatcgataacgattcgccggaggccattgccgagctggcggaacatctgaagaaagccctgaactgaagcctacggagaagaaacgatgagtcaattaaacagcgtctgggtctttagcgataatcctgaacgttatgctgaactgtttggcggcgctcagcaatggggccaacaggtgtatgccattgtacaaaataccgaccaggcgcaggcagttatgccttatggtccaaaatgtctttatgttcttgcgcaaaacgacgcgctgcaacgcactgaaaattacgccgaaagcattgctgccctgctgaaagataaacaccccgctatgttgctgttggccgcgacgaaacgtggtaaagcgctggcagcacggttaagtgtgcaactgaatgcggcgctggtgaacgatgccacggcggtggatattgtcgatggtcacatttgcgccgaacaccggatgtatggcgggttagcgttcgctcaggaaaagatcaacagcccgctggcgatcattacccttgcacccggtgttcaggaaccgtgcaccagtgatacctctcatcagtgcccgacagaaacggtaccttatgttgctccgcgtcatgaaattctctgtcgcgaacgccgtgcgaaagccgcaagcagcgtggacctgagcaaagcaaaacgtgtggttggcgtcggtcgtggactggcggcgcaggatgacctaaaaatggtccacgaactggcggcggtgctgaatgctgaagtcggctgttcacgtccaattgccgaaggcgagaactggatggagcgtgaacgttatatcggtgtctccggcgtgttgctgaaatccgatctctacctgacgctggggatctccgggcagatccagcatatggttggcggcaacggcgcaaaagtgattgtcgccatcaataaagataaaaatgcgccaatcttcaactatgccgactacggtctggtgggcgatatctacaaagtcgtccctgccctgattagccagttgagccgctaattcccctttcaaccacatctcccgctgtaaacgcagcgggaagggagcataacgcatgtcggatgacaaatttgatgccattgtggtcggtgcgggcgttgctggtagcgttgccgcactggtcatggcacgagccgggctggatgtcctggtgatagaacgcggcgacagtgccggatgtaaaaacatgaccggcgggcgtctttatgcccacacacttgaagcaatcattccaggctttgcagtatcagcgccggtagaacgcaaggtcacacgcgagaaaatctccttcttaaccgaagaaagcgccgttaccctcgattttcaccgcgagcagccagatgttccgcaacacgcatcttataccgtattgcgtaatcgtctggacccgtggttgatggaacaagccgagcaggcgggcgcgcagtttatcccaggcgttcgcgtcgacgcgctggttcgtgaaggaaacaaggtcactggcgtgcaggctggggatgatattctcgaagcgaatgtggtgattctggctgatggcgttaactcgatgcttggccgctcgctgggaatggttcccgcttccgatccgcatcattacgctgttggtgttaaagaggttattggcctcacaccagaacagatcaacgatcgctttaatattacgggcgaggaaggtgccgcctggctgtttgccggttccccttctgacggcctgatgggcgggggatttctctataccaacaaggattccatatccttggggctggtttgtggattgggtgatatcgcccatgcgcaaaaaagcgtgccgcaaatgctggaagattttaaacaacaccccgccattcgcccgctgattagcggcggcaaactgcttgaatattccgcgcatatggtgccggaaggcggtctggcaatggtgccgcaactggttaacgagggcgtgatgatcgttggtgacgccgcaggcttctgcctgaatttgggttttacggtccgcggcatggatttagccattgcatcggctcaggctgccgccacaacggtgatcgccgccaaagaacgcgcggatttctccgccagcagtctggcgcaatacaaacgtgagctggaacaaagctgcgtcatgcgtgatatgcagcattttcgcaagatcccggcgctgatggaaaacccgcgcctgtttagccaatacccacgaatggtagccgacatcatgaacgagatgttcaccatcgacggcaaaccaaaccagccggtacgaaaaatgatcatgggacatgcgaagaaaattgggctgatcaacttgctgaaagatggcattaagggagcaaccgcgctatgagccagaacgctacggttaacgtcgacatcaaattaggcgtcaataaattccatgttgatgagggccacccgcatatcattctggcggaaaatcccgatatcaatgaattccataaattaatgaaagcctgccctgccggactttataagcaggatgacgcaggaaacattcattttgattccgccggttgtctggagtgcggcacctgtcgggtgctgtgcggtaacactattctcgaacagtggcaatatcccgcaggcaccttcggtattgattttcgctacggctaatcatgcatcccacaggcccgcatctcgggcctgatgttctgtttcgagagtccaacatgaaagtgacattaacgtttaacgaacaacgtcgtgcggcgtatcgtcagcaagggttatggggcgatgcttcgctggccgattactggcagcagaccgctcgtgcgatgccagacaaaattgccgtggtcgataatcatggtgcatcgtacacctatagcgcgctcgatcacgccgcgagctgtctggcaaactggatgttagcgaagggtattgaatcaggcgatcgcatcgcatttcaactgcctggctggtgtgaatttaccgttatctatcttgcctgcctgaaaatcggtgcagtttccgtgccgctgttgccttcctggcgggaagcagaactggtgtgggtgctcaataagtgtcaggcaaaaatgttctttgcaccgacgttgtttaaacaaacgcgtccggtagatttaatcctgccgctgcaaaatcagcttccacaactacaacaaattgtcggcgtggacaaactggctcccgccacctcttccctctcattaagtcagattatcgccgacaatacctcactgaccacggcgataacgacccacggcgatgaattagctgcggtgctgtttacctccggaaccgagggtctgccaaagggcgtgatgctaacgcataacaatattctcgccagtgagcgggcttattgcgcgcgactgaatctgacctggcaggatgtctttatgatgcctgcgccacttggtcacgcaacgggctttctgcatggcgtaacggcaccattcttaattggcgctcgcagcgtgttgttagatattttcactcctgatgcgtgtctcgcgctgcttgagcagcagcgttgcacctgtatgctcggcgcaacgccgtttgtctatgatcttttgaatgtactagagaaacaacccgcggacctttcagcgctgcgtttctttctttgcggcggaaccacaatccccaaaaaagtggcgcgtgaatgccagcagcgcggcattaaattattaagtgtttatggttccacagaaagttcgccgcatgcggtggtgaatctcgatgatcctttgtcgcgctttatgcacaccgatggttacgctgccgcaggtgtagagattaaagtggtcgatgacgcacgcaagaccttaccgccaggttgcgaaggtgaagaagcctcgcgtggccccaatgtgtttatggggtattttgatgaacctgaattaaccgcccgtgccctggatgaagaaggctggtattacagcggcgatctctgccgtatggatgaggctggcggtaatgactccaacttattgatagtgttttatgttcagataatgcccgatgactttgtcatgcagctccaccgattttgagaacgacagcgacttccgtcccagccgtgccaggtgctgcctcagattcaggttatgccgctcaattcgctgcgtatatcgcttgctgattacgtgcagctttcccttcaggcgggattcatacagcggccagccatccgtcatccatatcaccacgtcaaagggtgacagcaggctcataagacgccccagcgtcgccatagtgcgttcaccgaatacgtgcgcaacaaccgtcttccggagactgtcatacgcgtaaaacagccagcgctggcgcgatttagccccgacatagccccactgttcgtccatttccgcgcagacgatgacgtcactgcccggctgtatgcgcgaggttaccgactgcggcctgagttttttaagtgacgtaaaatcgtgttgaggccaacgcccataatgcgggctgttgcccggcatccaacgccattcatggccatatcaatgattttctggtgcgtaccgggttgagaagcggtgtaagtgaactgcagttgccatgttttacggcagtgagagcagagatagcgctgatgtccggcggtgcttttgccgttacgcaccaccccgtcagtagctgaacaggagggacagctgatagaaacagaagccactggagcacctcaaaaacaccatcatacactaaatcagtaagttggcagcatcaccgaggctggctatataaaaattaccggacgcaaaaaagatattattgtccgcggcggcgaaaatattagcagccgtgaagtggaagatattttattgcagcatcctaaaattcacgatgcctgtgtggttgcaatgtccgatgaacgtttaggtgaacgatcatgcgcttatgtcgtgctgaaagcgccgcatcattcattatcgctggaagaggtagtggctttttttagccgtaaacgggtcgcaaaatataaatatcctgaacatatcgtggtaatcgaaaaactaccgcgaactacctcaggtaaaatacaaaagtttttgttaagaaaagatattatgcggcgtttaacgcaggatgtctgtgaagagattgaataagtttcatcttcggggatcacataaccccggcgactaaacgccgccggggatttattttatttcttcagttcagccaggcttaaccaggtttgcaccacggtgtccgggttcagagacaggctatcgatcccctcttccatcaaccatgcggcaaagtcttcgtggtcggacggaccctgaccgcaaatcccgacatatttgccctgtttcttcgcggcacggatagccatcgacagcagtgctttcaccgcatcgttgcgctcatcgaacaattcagacaccacgccggagtcacggtccagaccgagcgccagctgcgtcatatcgtttgagccaattgagaagccgtcgaaatattcgaggaactgctcggccagcaaggcgttggacgggatttcacacatcatgatgattttcagcccgttctcgccacgtttcagcccctgacgcgccagttcttcaaccaccgctttcgcctgatctacggtacgcacgaacgggatcatgatctcaacgttggtcagtcccatgtcgttgcgcacacgtttcactgcttcacactccagcgcgaaacagtcgcggaagctgtcggaaacatagcggcccgcgccacggaagccgagcatcgggttctcttcatctggctcgtaacgctcaccaccgaccaggttggcatattcgttcgatttaaaatcagagagacggacaatgacgcgcttcggataaaacgcggcacccagcgtcgcgatcccttcagtcagacgaccaacgtaaaattcacgcggagaatcaaaacctttcatcatctcgcggatttcgttttgcaactgcggttcctgatcgtcaaactcaagcagtgcgcgtgggtggacgccaatcatacggttgatgataaattccagacgcgcaaggcccacgccttcgttcggtaggcaggcgaagtcgaaagcacggtccgggttaccgacgttcatcatcactttcaacggcagatccggcatcgtttctacgctggagcttttcacgctaaattccagcaactccgcatagacgtaaccggtatcaccttcggcacaagaaacagtgacgttctcaccgtctttcatccgttctgttgcatctccacagcccactaccgccggaatgcccagttcacgagcgatgatcgccgcgtgacaggtacgaccgccacggttggtgacgatggcagatgctttcttcatgatcggttcccagtccgggtcggtcatgtcagtaaccagcacgtcgccaggttcgatgcggttcatttcgctgatgtcatggatgactttcaccggacccgcaccgatgcgatgaccgatagcacggccttcggcgataatcttaccctgtgaatgcagcgtataacgctccatgacctgaccgcgtgagcgcacggtttccggacgcgcctgcacaatgaacagtttaccggtgtggccatctttcgcccactcaatatccatcgggcgaccgtagtgtttctcaatttgtacggcctgttttgccagttcctgcacttcttcgttggtcagcgagaagatgtcacgctgttcctgcggtacgtcttcgattttaacctgcttgccgtgctcctgggtcggcgcgtaaaccatgcggatttttttcgaccccatggtgcggcgcacgatagccgggcgattcgccgccagtgtcggtttatgcacgtaaaactcatccgggttaaccgcaccctgcacgaccatctcaccaaggccccatgcggaagtgataaacaccacctggtcaaagccggattcggtatcaatggagaacatcacgccagatgatgcgaggtcagagcgcaccatccgttgaacaccggcggagagcgccacaccacggtgatcgtaaccctggtgcacacgataagagatggcgcgatcgttaaacagagaagcaaatacatgtttcactgccacgagaacggcgtcaaaaccctgaacgttgaggaaggtttcctgctgaccggcaaaagaagcgtccggcatatcttctgcggtggcggaggagcgcaccgcaaaagaggcgttttcgtcatcggcggaaagctgtgcataggcttcgcggatggcgttttccagctcaggctggaagggagtgtcgataatccactggcggatttgcgcgcccgctttcgcaagctgagtaacatcgtcaatatccgttttatccagcagttcataaatgcgctggtttacgccgctttggtccagaaactggttaaacgcgtcggcggttgtggcgaaaccattcggaacggaaacacccattccggaaagattagtaatcatttcacccagggaggcatttttgcccccaaccctgtctacatcattcatgccgagttggttataccaaagcaccagcggtgacgagccattgttggacatcgaacaatccttttgtgataaatgaacggtttgagaaacacatttctgcgcatttatctttgcatatttaaccggatgaaaaaaacggtgaatcgttcaagcaaatatatttttttactttttaagactgatcccagcgttgcgcaaatctgctctcttcgacaatttccacataaaccatcggtataaacgaaaccataaaaatgaaatgctgttttcataaaaaataaaattgaaggttcattttataaaccagacataacgttctacgcttctgtgcgtttttaatttatgctttcatagaattatgtctgcatcacgggaagaacaaaatggataatgctgttgatcgccacgttttttatatttctgatggtacggcaataactgcggaggtattaggacacgcagtaatgtcacaatttcccgtcactatcagcagcatcacgctgccgtttgtcgaaaatgagagccgtgcacgggcagtgaaggatcagattgacgcaatttatcaccagacaggcgtgcgcccgctggtcttctactccatcgtgttgccggagattcgcgccatcatcttgcaaagtgaaggcttttgccaggatatcgttcaggcgctggttgccccgctacaacaagagatgaaactggatccaacgccgattgctcatcgtacccatggccttaaccctaataatctcaataaatatgatgcgcgcattgcggcgattgattacaccctcgcccacgatgacggcatttcgttgcgcaatctggaccaggctcaggtgatcctgctcggtgtttctcgctgtggtaaaacccccaccagtctgtatctggcaatgcagtttggtatccgcgcggcaaactacccctttattgccgacgatatggataatctggtgctacccgcgtcgctcaaaccgcttcagcataaattgttcggcctgactatcgacccggaacgtctggcggcgattcgcgaggaacgtcgggagaacagtcgctatgcctcgcttcgtcagtgcaggatggaagtcgcggaagtggaagccttgtaccgtaaaaatcagatcccgtggattaacagtaccaattattcggtagaagagattgccaccaagatcctcgatatcatgggccttagtcgccgaatgtactagagaactagtgcattagcttatttttttgttatcatgctaaccacccggcgaggtgtgacacacctcgcacttgaaatcagcagcgattggtttatcgtgatgcgcatcacttcccggcagtcctgccgtagaagcaacaaatttctgagacttgtaatgaacagaactgacgaactccgtactgcgcgtattgagagcctggtaacgcccgccgaactcgcgctacggtatcccgtaacgcctggcgtcgccacccatgtcaccgactcccgccgcagaattgaaaaaatactgaatggtgaagataagcgactgttggtcattattggcccctgctcgatccacgatctcaccgctgcaatggagtacgccacccgtctgcagtcgctgcgcaaccagtaccagtcacggctggaaatcgtaatgcgcacctattttgaaaaaccacgaactgttgtcggctggaaaggactaatctccgatccagatttaaacggcagctatcgggtaaatcacggtctggagctggcgcgcaaattacttttacaggtaaatgagctgggcgtcccaaccgcgaccgagttcctcgatatggtgaccggtcagtttattgctgatttaatcagttggggcgcgattggcgcacgtactaccgaaagtcagatccaccgcgaaatggcttcggcactctcctgtccggtaggttttaaaaatggtaccgatggcaatacgcggattgctgtggatgctatccgcgcagcccgcgccagccatatgttcctctcgccagacaaaaatggtcagatgaccatctatcagaccagcggcaacccgtatggccacattattatgcgtggcggcaaaaaaccgaattatcatgccgatgatatcgccgcagcctgcgatacgctgcacgagtttgatttacctgaacatctggtggtggatttcagccacggtaactgccagaagcagcaccgtcgccagttagaagtttgtgaggatatttgtcagcaaatccgcaatggctctacggcgattgctggaattatggcggaaagtttcctgcgcgaaggaacgcaaaaaatcgtcggcagtcagccgctcacttacggtcaatccattaccgacccgtgtctgggctgggaggataccgaacgcctggtcgaaaaactcgcctctgcggtagatacccgcttctgaatgcgtgcccattcctgacggaatgggcatttctgcgcaacttgttgtcttctcaacaaattactgcttgctctggtcagccataatattgataataagaatcattgttatatcaattattattaatttttatgcgttatacggatagcagaaaactcacgcctgaaacggatgccaatcacaagaccgcttccccgcagcctattcggcgaatttccagccagacactgttaggtccggatggcaaactgattatcgatcatgacgggcaagaatatctgctccgtaaaactcaggctggcaagctgctgttgaccaagtagcctttaactcgagcagctgacttccagccgtttaccccagtcaggtggacgactgacatagtcatcatctctgtcgctgaaaggatttcgcaacgcctcatgcaggcggtgcaattccgtcatatcacccttttctgccgcttcaatcgcccgttgcgccaaccagttgcgcaataccagagcggggttaacgctttgcatcagttgctgacgctcactatcgctaacctcgtcttgttgcaaacgcccccgataacgggcaaaccagtcatcaaatgccgcacgatcaataaactcatcacgtagcggtgacgccgcgctgtgctgctcggtcagactcagcatgcggaatgtgcgggtataatcgctgcgctctcgcgccatcagactgaataattcattcagtagcgcgttatcctctttttgctccgtcatgaagcccagtttctgccgcatccgttctccataatgcgtcaacaaaacctgctgatagctgtccagggcctcattcagggcatctacggcaacaaatggcgacaatgtctgcgccagacgctgtaaattccacaacgcgacggcaggttgattatcaaagctgtaacgcccttgatgatccgagtgattacaaataaaaccgggttcgtaatcatcaagaaaaccaaacggcccgtaatcaagcgtcagccccagcagcgacatgttgtcggtattcatcaccccatgagcaaagccgaccgtctgccattgggcaattaacgacgcggtacgtgcgacaacatcgctaaaccagagacggtatttgtcctcatcatctgcaagatgtgaccagtaatgacgaatagcaaagtcagctaactgacgaaccttttccgactcgcggcggtagtaaaaatgttcgaaatgaccaaagcgcagatgacttggtgccacacgcatcagcatcgcgcctggctccgccgtttcccgatacactggcgaatcgctggtgacgatacttaacgcgcgggtcgtcggaatgcccagataatgcatcgcctcactggcgagactttctcgtatcgtcgaacgtaaaaccgcccgtccatcacccattcgcgaataaggcgtcaggccagcacctttcagatgccagtccattgtagtgccatcagcaagcagttgttcgccgagtaaaatgccgcgcccatcacccagttggcccgcccagacgccgaactgatgaccactgtaaacctgcgccagtggtgacataccaggcagtagggcttcgccgccccagacacctgcgccatttttaaacagcgacgatggaatactcagcgtgttagccagttcggtattatgccaaatcagccgggcattatttaaaggcgtaggggaaagtgctgtataggtttctggcaattcatcgcgccagcgggtaacaaaagacagggtcatagatcctcctgtttgatagtgtagacggttactctcgtcttaaacaccagcaaacagaagggttatcgctgaaccaacgtcgttatctgatttatgggaacggcaggccacaggcatccctggagagcatggaaatcgaagggggtaatctgtgccaatatttctgccgtatcaatgcctcccgcaatgatgcaattgcaacaaggggaaatttgcgcctggatcgcacgaataaacggttcgaaggagcggtgcgtgatttgttgctgaataaaacttttatccagcatgacgcgggtgaaaagaccatcaaaaaccgctttcattgtgctattgcctgctcccaaattacctaacacaaggggatacacttgcgataaggataaaagaccgcgattatcttttccttcattgagatgcgggtaattctcattaatcaacagttcaataaacggatattttaatagttcgcctgcgtaattatccctctctaataataatgtagccacttgtggcgttaaattaagccaggcaaagagtttatgttgaataaaaaaatgttggcatgattttagtaattccaactgctctgaaaataattgccaatgttgctcctcggtaagttgcgctataacccgactcgtcgggatacgaaccgtaccatcttcactggagaaatgggtaattaactcaacgccgacaaggacttgctggttgtctcttatcggcaggaaatagcaatcagaatgataaagattctccaaaaaaatcttcatggtaaccgtccctctcgaaggatgtttttcagtatccggctaaaagggatgaggccataagacataacaattacagaaggagtaactttcatttgttccatgttaaccactttttcaggggtcctttttttagattatcctgattataaacgaataatccatttacggaatttttgtctgcaaaatactactgtattcaggagtaaatggacggcgatgtatcatcgccgtccatttttcgacatactagattcgtctcgcctgccagaaatttttctgccaatagacattatcaagtgaggaacgcatcactcccttgctggtagaggcgtggataaattggttgttggtatcgtaaatacctacatgcaaaccattttgtccggaccccgttttgaaaaagaccaggtcacctggcagcaactcgtctttatcaatttgcgtgccaatagaggcttgttgtttggtttcacggggcagctgcaaatcgaaacgatcgcgcatcgtcacaaccacaaatcccgaacagtccacaccgcgccgcgtcatgccaccataacgatacggcgtgccatgccagctttgtagctggtcgttcaaaccggcaataacggtaatcgaatcagaaagtctggcatttggcggcggtgctttatggtggctacacccggccagaagcagtgctgtgatcaaaataaggcagaaacgcattccgtacggttcctctgttttttattcttgcattaatttagcgtcgtaattacccgattttcaagatactaatgaaatcagatggtcgaaatcagcattctgtgaccttcgatatccagacggcgaaaattcatcccataggcctgcgccagatttggcggcgtgagcacctcttccctgcgtccactggccagcatttttccaccttttagcaaccacgcccgatgcgcatgacgcaatgtgtggttgagatcgtgactgctcatcacaatcgccagtccttgctgacacagcgcgctcagaattttgtctaacgcactttgttgcgcaacatcaagactgttcatcggctcatcaagaagcagcaattggcctgcgggattggcttgtggtgtgatttgcaacaccaccgcagcaagacgtacgcgttgccattcaccgccggaaagttgattggtgctacgtccgagtttgtcatcaagagccagcgcccctgcgacatcattcagtagttcggtacgcgttttatcgtgctgatgcagtgtcaggtagtgccagaccggcgttgcaaacggcggcgtctgctgttgtgaaagataggcgcgatgcagcgcgagttttgttgcggaccatgcttccagtggttgccccgcgaactgaatgcttcccttaccgctggtcattccggccattcgcgccagtaaggtactcttacccgcgccattcggccccaccaggtgcaggatctccccagcccgaacctcgccagaaagcggccccaggcgggtagattccgcaacatcttgtaactgcatcacaatagacattattttgccaacgccagtttaatgctttccatcacaatgggatcttccggcgtcatatccggggaaaaacgctggatgacttttccgtccctgccaaccaggaatttttcaaaattccataaaatatcatccgggtacagcggtgcacggcctttgctgaccatacgggcatagaatccgctctcttccggcgcgactgcggtcggcgctgcggcaatcaatttttgatacagcggatggcgtccttcgccattaacttcaatcttactgaacatcgggaacgtcaccccccatgtggtggtacagtaagttttaatctcttcatcgctgcccggttcttgttccagaaactggttgcacgggaatcccagcaccataaaacctcgatcgacccaggctttctgaatattctccaactgctcatattgcggcgttaagccacactttgaggcgacattgacaatcaacagcacattaccggcgaacttctccagcgtggtcacttcaccgtcgatatctttcactacggtcgtcagaatggaatcttgcatcgtttctcctgggtgtggtcagtaaaaatcttagcttttaatcatagaccgtctttttgcggctaacgtcctgcttttaacaataaccagataaacaccggcgcacctaacgttgcggtgaccacgccaataggcagctctgcggcagctaatgccaggcgcgctacaatatcggccagcagcaatgcgctcgcccctgccagcgcgcagccgggaagtaatacgcgatgatcggttaaaccacacaaccggagaatatgggggatcaccagaccaataaagccgatagcacccgccagcgccacactgacgccaaccatccagccggtcgctgccaccagcacattgcgccagaaccacaggggtaaacccagttgccgcgccgagatctcgccaagtgctaacatattcatcggcctggactgacaacagatccacaacaacacggggatcaatgccagcatcagccagctttgccgccagtctacgccgccaaaaccgcccatcatccagtacatcagctgacgcaaatcaactgaggtggaaaagtagatagcccacgtcattagtgcgctacagataatccctaatgcaacgccagccagcaataaccgactggtcgaaagatgacgacgggcgaaacgtaagagtattaaagtgatgataagcgcgccagcaatcgcacacagccctagcgcccagttggggagttgcccttgcccaagcaataccgcggcgataagccccacgcctgcgccgttagagacgccaagtagtccaggttctgccagaggattttcaaacaacgcctgcattacagcgccggatatagccagcgccgcaccaaccagcaatacagccagcgtacgtggcaggcgaatttgccagacgaacagttcgccacgaggagtaaaccagtcacctggcgagatccattgttcaccggcgcaaaggcttaagagaagcgccagcagcatcaaaactgacaggcataataaccagcgaatattttgtcgctgttgttggcgggcaagtgtcagcatggtatccgttctgctgaagtgtcatggcgttgattttacggtgactcttcgacagtgaaaagaaaaaaggccgcagagcggcctttttagttagatcagattactcgtctttgggcgaagcgttttcgacccggctttttaacttctgcccgggtctgaaggtcaccacgcgccgtgctgtaatgggaatatcctcgcccgttttcgggttacgtcccgggcgttgattcttatcacgcagatcgaagttaccaaaaccagagagtttcacctgttcgccgttttccagagcgcgacggatctcttcgaaaaacagttcaaccagttctttggcatcccgcttgctaagcccaagcttatcaaacagatattctgacatttcagcttttgtaagcgccataggttcaatccctcaatgatgcctggaatcgctcttttaatgcctctacacatttggcgacggtagcggcaatctcctcttcttcgagtgtacggctggtatcttgcaggatcaggcttatggcgaggctcttatacccctccgcaacacccttaccgcggtacacgtcaaataagtttacgccaactacctgatttacgccaactttcttacattcggataaaatatccgctgcgggaacgttttctgcgaccaccaccgcgatgtcacgacggttcgccgggaagcgagaaatctcgcgcgcctgaggcaccacgcggtctgcgagcttgttccactccagttcgaacaccagagtgcgaccgttaagatccagtttacgttccagttcaggatgaacaaccccaacaaaaccaatacgttcacctttcagataaatcgctgcggattgccccggatgcagtgccggattcgcttctgcacggaactcaacctcattcagtttaccggtcaggtcgagaacggattcaagatcgcctttcaaatcatagaaatcaacggtctcttttgccaggttccagtgctcttcgtaacggttaccgcaaatcacaccggctaacatcagatcctgacgaatgcccaacggtgcctgagtatctggtacgaaacgcagaccgctttcgaaaatgcgcacacggttctgctgacggttctggttgtacaccacggttgccagcaggccagtccacagagaaagacgcattgctgacatttcaacagagatcgggcttggcagcagtaaggcttcaacgcctggatggatcatctgctgcactttcggatcaacgaagctgtaggtgatcacttcctgatagcctttgtcgttgagcagcgttttcacgcgcttgagcgacaggtcagcttcacggtgagtacccataatcaggcttgcctgtaccggctcatccgggatgttgttgtagccgtaaacacgcgcgacttcttcaaccagatcttcttcaatctccatatcgaaacgccagctcggcgcaactgcctgccattcgtctttgccttcggtcacttcgcagccgagacgacgcagaatgtcagttacctgctcatccgcaatatgatggccgatcaggcgatccagtttgctacgacgtagagtgatggttgcacgcttcggcagcgttgcttcgttggtgatatcaattaccgggccagcctcaccaccgcagatgtcgatcagcagacgggtcgcacgttccatcgctttgtgctgcagtgccggatcaacgccacgctcataacggtgagacgcatcggtatgcaggccatgacgacgagcacgaccggtgatagacagcgggctaaagaacgcgcattccagcagcacgttttgtgtttcgtcattcacgccagagtgttcgccaccgaagatgccgcccatcgccagcgccttgttgtggtcggcgatgaccagagtgtcagcattcagcttcgcttcagtaccgtcgagcagcaccagcgtttcgccctctttcgccatccgcaccacaatgccgccttcaatgcgatctttatcgaaagcgtgcatcggctggcccagttcgagcagcacatagttggtgacgtcaacaactgcatcgatagaacggatcccgcaacgacgcagtttttctttcatccacagcggagttggcgctttaacgttaatgccttttaccacacggccaagataacgcgggcaggcttccggcgcttcgactgtaatcggcagcgtgtcgtcgatggtcgcaccaaccggaacgatttccggttgaaccagcggcagctggttcagcacggcaacgtcacgcgcaacaccaatgatgcctaagcagtcggcacggtttggcgtcacgctgatttcgatggtgttgtcatcaagtttcaggtattcacggatatcggtgccaatcggcgcatccgcaggcagttcgataatgccgctgtgatcgtcagaaatgcccagttcagagaaggagcacagcatcccttcagacggttcgccacgcagtttcgccgctttaattttgaaatcacccggcagaacagcaccaatggtcgctaccgctacacgcaggccctgacggcagtttggcgcaccgcagacgatgtccagcaggcgatcgccgccgacattcacttttgtcacacgcagtttgtcagcgttcggatgctgcgcacactcaaccacttcaccaacgaccacgccgtggaagctgccggcaaccggttctacaccgtcaacttccaggcccgccatagtgatttgatttgccagcgcatcgctatcaatcgccgggttcacccattcgcgtaaccacagttcactgaatttcataatctattcctgccttatttaaactgtttgaggaaacgcagatcgttttcgaagaatgaacgcaggtcggtgacgccgtaacgcaacatagtcagacgctccatccccatcccgaaggcgaaaccagagtaaacttccgggtcgatgccaacgttacgcaacacgttcggatgcaccatcccgcagcccagcacttccagccatttaccgtttttacccatgacgtccacttctgcagaaggttcggtaaacgggaagtaggaaggacggaagcgaatctgcaaatcttcctcaaagaagttacgcaggaagtcgtgcagcgtgcctttcaggttggtaaagctgatgttggtatcaacaatcagaccttccatctgatggaacatcggcgtgtgagtctggtcgtagtcgttacgataaacacggccaggcgcgatgatacgaatcggtggctgctgggctttcatggtgcggatctgtacgccagaggtctgggtacgcagcaggcgggtagtgtcaaaccagaaagtgtcgtggtcagcgcgcgccgggtggtgaccaggaatgttcagagcatcgaagttatgataatcgtcttcgatttccggcccggttgccacggtaaagccaagctcaccgaagaaactttcgatacggtcgatggtacgggtaaccggatgcagaccgccgttttcaatgcgacgacctggcagagagacatcaatcgtttccgccgccagacgcgcattcagtgcagcgctttccagttccgctttacgcgcattcagcgcctgctgaacctgctctttcgcttcgttgataaccgcaccagctgccggacgctcttctggcggcagctcacgcagggtcgtcatctgaagggttaagtgcccttttttacccaaatattcgacgcgcacattatctaacgcggcaacatctgacgcctggctaatggccgccttcgcactggcaaccagttctgcgagatgtgacatggttttcctcattgtgtcagtggtgacactggttcgttggacttagagcctatcccatcaggctattttacttgccattttggtcccgggctgtgctcgaaattctcacgtacttaaatacgctccggtttctccgcgctggccgtgtccagtctggctgcgacaattacacctgatgagacaggctttttatttttcaaaacgcgcatacaaaaaaagcctccactgggaggctttcaggcgctgttttccgtttctcttctcacgcgctagcctcctggattcaggtgctaaagtaaaaaaagaagcggaaaatagcagcattcattgcttgcgttaccttttggtactcttcaaaagacctttattgaaaaggctacggcgataaaagtcaatgttttgatggcgttgaaacgaaaagagggagactagctccctctttcaactggcttatgccagagctgctttcgctttttcaaccagagcggtgaacgctactttgtcgaatactgcgatatcagccaggatcttacggtcgatttcaacagaggcttttttcaggccattgatgaatttgctgtaagaaataccgttctgacgtgctgctgcgttgatacgcgcaatccacagttgacggaactgacgcttacgttgacgacggtcacggtaagcatactgaccagctttgataacagcctggaaggcaacgcggtatacgcgagaacgcgcaccgtagtagcctttagcttgtttcaaaattttcttgtgacgtgcacgtgcaataacaccacgttttacgcgagccatatgtgctctcctgtatctatattctaattaaaaagttaaaaacgttaacggcttatgcgtacggcaggcacgcgattaccaggcccagatcgcctttggaaaccatggctttcggacgcaggtgacgtttacgtttggtcgcttttttggtcagaatgtgacgcaggttagcgtgcttgtgcttaaaaccacctttaccggtttttttgaagcgcttagcagcaccgcgtacggtcttaatttttggcattttaataacttccacttcgcattgttaataaacgaaacaaaggcgaacaaagcctgtgaagcccgaaggctccacagacagtgctacttgaaggccttactgtttcttcttaggagcgagcaccatgatcatctggcggccttcgatcttcgttgggaaggattcgaccactgccagttcttgcaaatcgtctttcacgcgattaagcacttccataccgatttgctggtgcgccatctcacgaccgcggaaacgcagcgtgattttggctttatcaccctcttcgagaaagcgaatcaggctgcggagttttacctgatagtcgccttcatctgtaccaggacggaatttaatttccttaacctggataactttttgctttttcttctgttccttagaagacttgctcttttcatagaggaatttgccgtaatccattatacgacaaaccggcggctcggcgttagggctgatctcgactaagtctactccggcttcttctgctttctccagagcttctctcagactcacaataccaagctgctcgccttccagacctgttaagcgaacttcctgggcgcgaatttcgccattgatacggttagggcgcgccgtttgaactcgttttccgcctttaataccttattcctccaattgtttaagactgcggctgcgaatctcttgttgcagcttctcgatcacttcatttacgtccatgcttcccaggtctttaccacggcgggtgcgaacggcaactttgcctgattccacctctttatcaccacagaccagcatatatgggacgcgacgcaaagtgtgctcgcggattttaaagccaatcttctcatttctcaagtctgctttaacacgaatgcccgcatttgatagtttttgcgtcaattcgttaacgtattcagactgtgaatcggtaatattcatgataacaacctgaaccggcgcaagccaggtcgggaagaaaccagcgaactcttcggtcaggataccgatgaaacgttccatcgaccccagaattgcgcggtgaatcattaccggtactttacgttcattgtcttcgcctacataagaagcgctcagacgagacggcaaagagaagtccagctgtactgtaccgcactgccatgcacgatcgaggcagtcatacagggtaaattcaattttcggaccgtagaaagcgccttcacccagttgatattcaaacgggatgttgttttcttccagcgcaaccgccaggtccgcctcagcacgatcccacatttcgtcgctgccaatacgtttttcaggacgagtggagagtttgacgacgatcttctcgaagccaaaagtgctgtacatatcatagactaaacggatacatccgttaacttcatcgcgaatttgttcttcagtacagaagatatgcgcgtcatcctgggtaaatccacgcacgcgcatcaggccatgcagcgaacctgacggctcgttacggtggcagctaccaaactcggccatacgcagcggcagatcgcgataagacttcagcccctggttgaaaatttgtacgtgacccgggcagttcatcggcttaatgcagtattcacggttctcagaagatgtggtgaacattgcatctttgtagttgtcccagtgaccggttttttcccacaggacacggtccatcatgaacggacctttaacttcctgatactggtactctttcagtttagaacgaacaaacacttccagttcacggaagatggtccagccgtcgttgtgccagaataccatacccggcgcttcttcctgcatatggtacaggtcgagctgtttaccgattttacggtggtcgcgtttcgcggcttcttccaggcgctgcaggtaagcgttaagtgcttttttgtctgcccacgccgtaccgtaaatacgttgcaacattttgttgttgctgtcgccacgccagtaagcccctgccgttttcattagtttgaaatgatggcagaaacgcatgttcggtacgtgcggaccgcggcacatatcgacatattcttcatggaagtacagacctggcttgtcatcatgggcgatgttttcgtcaagaatggagactttgtagctctccccacggttggcgaaagtttcacgcgcttcgtgccagctgactttcttcttaatgacgtcgtagtttttctcagcaagctcatgcatccgcttctcgagtgcttcgacatcttcctgggttaacgtgcggtcaagatcaacgtcgtaataaaaaccgttgtcaataaccgggccgattgccattttggtatgcggccaaagttgtttaatcgcgtgccctaacaggtgcgcacaggagtgacgaatgatctccagaccttcttcgtctttggcggtaatgatcgacagttgtgcgtcgttttcaatcagatcgcaagcatcaaccagttcgccattaacgcgccctgcgatacaggctttcgccagacctggaccaatgtccagcgcaacatccatggggcttacagcgtgatcgtaatggcgttggctgccatcaggaagagttataacaggcattttatatccttatttgcagtggtgacccacacgaaagatcacatacaaagaaaaatttgtttattaacagttcattgcgaaaccatctagccaacaaatgctaaattggttcgcaatcaggtacacaaatgaaagacattaacctctcaccttccacccggttgagcgatgttaacactaaaaaaagggagattgtacctttccgtttcacattgattcgattcgcaattcgtttgtagtgagtacaccagcaaaacgcttaaagaacaactgataacatcacggtgcgtctgaaaggtttactgcgagcggatttacagcagcataaactgaatccagcaaagttcgttgcgtgatttggcggtagtattttaaacgctcatgagattaatgacgaagtggtcatatcacaatgataaaagtgacacaattcttataacaatttttcgtgcacatttcgttctggcgataataattaatcatcatcctcaaaacctccagatatatataaggcgaacagattatgagtcaaaacgatatcattatcagaactcattataagtctcctcatagattgcacatcgatagcgacataccaacaccttcatcagagcctattaatcaatttgcgcgccagctcatcaccctacttgatacctctgacttaagttcgatgctgtcatactgtgttactcaggaatttaccgcaaactgtcgaaaaatatcacaaaattgttattccactgccctttttaccattaactttgccacttcacccatccatacagaaaatatactcattacattacactataaaaaagaaatcatttccttattactggaaaccacgcctattaaagctaaccatttgcgaagcatactggattatattgaacaggaacagttaactgctgaagatcgtaaccattgtatgaaactgtctaaaaaaatccatagagaaaaaaactatacacccaacagtaaatctcaatggtagtgcatgttttttgcaatctccttctgacgctattttttgtcgccatctgtcattgcaatacgcccttgattcattgagaaatggaaaaggcaaagtcaacctgattaaacattactcctccgttgaatccatacagcagcatgtccccttagtccgggacgcggagttcagagcattacttcgccatcctcctgcagggagtcgcgttatcgcgagtaaggattttggcttcgctttagatattttcttttgtcgaatgatggcaaacaatgtcagtcatatgtccgcgattttatatatagacaatcatactttgtcagtaaggctacgaataaagcagtcagtgtatggacaattaaattatgttgtgtccgtttacgacccgaacgataccaacgttgccgtcagagacacccacaggacagcacggggctttctttcgcttgataagttcatcagttcaggtcccgatgctcagacctgggctgatagatatgttcgcaactgtgcaattgctattctgcccctattacctgtgggagttccaggggctattttcgcgggtattgcatcacgaatgccatttgcccctatacatccatcggcaatgttgttaataatggctacaggccagtctcaacagcttattacattattcaaacagttgcccatactccctgaaaaagaaatcattgaaataataactgcgcagaatagcgttggtacacctgctttatttttggctatgatgaacggacatactgacaacgtgaaaatatttatgcaagaaattcagtcactggtagataatcacatcattcatgaagataatctggttaaattactgcaaactaaaagtgctaacgaaacacctggactttatatctccatgttgtatggattcgatgaaataatcgatatctttctgaatgcattaaccactccaatagcacaagagcttttaaacaaaaaactggtgatgagtattttagccatgaaaatacatgatggtgagccaggattatacgccgcaatggaaaataatcaccctttgtgtgtcacacggttcctctctaaaattaatggcatcgcctttaaatacaagttgagcaaagctaacatcatggatttattaaaaggagctacagcacagggaacccctgcattatacatcgccatgagcaagggtaatgaagacgtcgtgttatcttatatatcgacgctgggtgcttttgcaaaaaaacattcttttagtcaacatcagttatttacactattggccgctaaaaatcatgacaacatgtcagctgttcatatagccattcatcataagcattataaaactgtagaaacatattatgctgctattaatgcaatcagccaaagcctgagttttagtgctgatgaaataaagacgtatttataaccagctatttacgatatatatcgatacataattttatttttttcataaaacgcagaaacagtgaccatgtgcacaacgccacccgacggctgtaataacaaaaaatcccttgatgcctgtcccttttgttacactccgttatcacgcacaagagatatgcaggacactggtatgccgactaaacgctttgataaaaaacactggaagatggtggtggtgctactggcaatctgtggcgctatgttgttgctacgttgggcagcaatgatttggggctgagcagtgacaaacgaagacagccagaccgcataacacggtccggcagataattttacatgctgtagcccagcgataaggttgtccgacggtcggtatgttccggtgcagactctggaggttcagagttccatgtgacgttgtaagccaccttcagtccaaaatgttcattaatagcaacatttaatgcgctttcggagttcagcgttgtgtcttccgcgccaaagaccgaaacaccctgcgtaaatttagcgttgtcagtcaactgccatgcataagccccggaggcatagcccagcggctgggtttcactggcattgtcggtatatttgtcgtaacgcacacctggaccgaattcaaagcggaaactgtgtaccgggccattcaaaaactgacgaccataacccgcggtcaacacatcgcgctctcgatagccgttataacggtctgtcagccagcttgcctgaccaaataaatagtcataatcagttaaattaaaacggctacgcccgcccgccgcatatttttctgaagaacgctcatcattagaagaagtattactggcgttcccccacagcgaccaggcagtggtgtgtccataccaggtcatggtggtgtcagccgtaagtgaggagcttttcgtattgcctgattgtgcaagatatcctgcgttcagattaccttcgaaaggttttttagcgctggcaggatcatccatgacagtaaaaacggaatcatcggcagctgcattcagtgacgcaaacatgccccccgccaacataacgatggcaggaactgtcttcaaaagcttcatttatcaagagtccgtacaacaaaaaaagagaccatcgcggtcccggaaactttcttaaggatcaaagattagcgtccctggaaaggtaacgaattataaaaaggcgcgaataacttagcaatgtattcttatttcattttttgaataagcatgtggcgaaaacagatttttatttatatatatttatctgcaaaattttaaataaagctccaataaatcatattgttaatttcttcactttccgctgattcggtgccagactgaaatcagcctataggaggaaatgatggtacgtatctatacgttgacacttgcgccctctctcgatagcgcaacaattaccccgcaaatttatcccgaaggaaaactgcgctgtaccgcaccggtgttcgaacccgggggcggcggcatcaacgtcgcccgcgccattgcccatcttggaggcagtgccacagcgatcttcccggcgggtggcgcgaccggcgaacacctggtttcactgttggcggatgaaaatgtccccgtcgctactgtagaagccaaagactggacccggcagaatttacacgtacatgtggaagcaagcggtgagcagtatcgttttgttatgccaggcgcggcattaaatgaagatgagtttcgccagcttgaagagcaagttctggaaattgaatccggggccatcctggtcataagcggaagcctgccgccaggtgtgaagctggaaaaattaacccaactgatttccgctgcgcaaaaacaagggatccgctgcatcgtcgacagttctggcgaagcgttaagtgcagcactggcaattggtaacatcgagttggttaagcctaaccaaaaagaactcagtgcgctggtgaatcgcgaactcacccagccggacgatgtccgcaaagccgcgcaggaaatcgttaatagcggcaaggccaaacgggttgtcgtttccctgggtccacaaggagcgctgggtgttgatagtgaaaactgtattcaggtggtgccaccaccggtgaaaagccagagtaccgttggcgctggtgacagcatggtcggcgcgatgacactgaaactggcagaaaatgcctctcttgaagagatggttcgttttggcgtagctgcggggagtgcagccacactcaatcagggaacacgtctgtgctcccatgacgatacgcaaaaaatttacgcttacctttcccgctaacaaaaacattcccccagcattgggggaatcatcaccaacctgtcggcaacgcgtttctccgactatgctcaaaagtcatgtgataacaaaggggtgaactatggccagtggcgatcttgtccgttatgtcataaccgtcatgttgcatgaggatacattgactgaaattaacgagttgaataattacctgactcgcgacggttttttgctcactatgacggatgatgagggaaatatccatgagctgggaactaacacttttggacttatcagtacccaaagtgaagaagaaattagagaactggtttcggggcttacccaaagtgcaaccggcaaagatcctgaaatcaccatcacgacctgggaggaatggaatagcaacagaaaataaatggtttttgggcaataatcagtctgtggtgtgcgttagctcgtgtttttacaccgcattcttgcgctaaccttatgatctggcagacaacatgggagagacatcatgtggcaggcaatcagtcgtcttttgagcgagcagttaggtgaaggcgaaatcgaactgcgtaatgaactgcctggcggagaagtccatgccgcatggcatttgcgctatgcaggacatgattttttcgtcaaatgtgatgaaagggaactgcttcccggttttaccgccgaagccgaccaactggagttactgtcgcgtagtaaaaccgtcaccgtgcctaaggtttgggcagttggcgctgaccgtgactacagttttctggtgatggattatctcccacctcgtccgctggatgcgcatagcgcatttattcttggtcagcaaattgcgcgtttacatcaatggagcgaccaaccacaatttggccttgatttcgataacgcgctctccacaactccacagcccaacacctggcaacgtcgctggtcaacgttttttgctgaacaacggattggctggcagttggaactggctgcagaaaaagggatcgctttcggcaatatcgacgccatcgtcgagcatattcagcagcgtctggcctcacatcaaccgcagccttctctgttgcacggcgatttatggtccggcaactgtgcactgggtccggatggcccgtacattttcgacccggcctgctactggggtgaccgagagtgcgacctggcgatgttaccgctgcatactgaacagccgccacaaatctatgacggctatcagtcagtatccccgctacctgccgatttccttgaacgtcaaccggtttaccaactctacacgctgttaaatcgtgcaaggttatttggcggtcagcatttggttattgctcagcagtcattggatagattattagcagcatgatatgggttgaggataatggccgctccgtgcggccttttgattaaataaacccaagcagagaaaagaacacataacctgcagcaatacaaataaccggcaggatatacagtgagaaaaactgcaggaaaatagtatggtgcggaacaacaatacgggactcaatttgttcacgcgttagcccctcttcccctttggctttttccagaatgagttgatcttcaacaccttcccgcaagaagcgcgcctggcgactcatccgggcaccggaatcctgcaacgccagtccgacaaaaatcaggatgaaaatcacccagaacataacgttcacgccaccattaaaattgggcgtcggggagttataccagaatagattcaaaaaaggcgtattcgcctgcatcatatcgatcatgacatgagtaaagtcgagcatgaccgcattaatgccttccttgttttcctgccgggtattcataaatttcagcaaagaaatcaatgtagagatcaatgcaggtataaaaatcacccaacccaaaatccttttcaaaacagcaatgcgtccagcttgttgatacgtcatgagttctccttgattaagacgcgtcgtttcacttagtttacctgtagatatctgttttcgcccattctttaaaggcgatatgataggcgcttaatcataagcacggcttaataccttacacataatgctctaaaggagaggttgtaatgtcaaccccgcgtcagattcttgctgcaatttttgatatggatggattacttatcgactcagaacctttatgggatcgagccgaactggatgtgatggcaagcctgggggtggatatctcccgtcgtaacgagctgccggacaccttaggtttacgcatcgatatggtggtcgatctttggtacgcccggcaaccgtggaatgggccaagccgtcaggaagtagtagaacgggttattgcccgtgccatttcactggttgaagagacacgtccattattaccaggcgtgcgcgaagccgttgcgttatgcaaagaacaaggtttattggtgggactggcctccgcgtcaccactacatatgctggaaaaagtgttgaccatgtttgacttacgcgacagtttcgatgccctcgcctcggccgaaaaactgccttacagcaagccgcatccgcaagtatatctcgactgcgcagcaaaactgggcgttgaccctctgacctgcgtagcgctggaagattcggtaaatggcatgatcgcctctaaagcagcccgcatgcgttccatcgtcgttcctgcgccagaagcgcaaaatgatccacgttttgtattagcagacgtcaaactttcatcgctgacagaactcaccgcaaaagaccttctcggttaatgaccaggggcagtgatctcgctgcccctggttctttatctgaaattgcattcaactgacggattaatcgtcaatttaagagaaagagttacaccgtcaccacttccgtgcactgtataaaaatcctatactgtacgtatcgacagtttagtgagttttatcatgacggcggaaggtcaccttctcttttctattgcttgtgcggtatttgccaaaaatgccgagctgacgcccgtgctggcacagggtgactggtggcatattgtcccttccgcaatcctgacgtgtttgttaccggacatcgatcacccaaagtcgtttcttgggcagcgattaaaatggatatcaaaaccgatcgcccgcgcttttgggcatcgtggttttacccacagtctgctggcggtatttgcgctgctggcaaccttttaccttaaggttccggaaggctggttcattccggctgatgcgctacaaggaatggtgctgggttatttgagccacatacttgccgatatgctgacacccgccggtgttcccctgctctggccatgccgctggcgtttccgcttgcctatcctggttccccaaaagggcaaccaactggaacgttttatctgcatggcattatttgtctggtcggtatggatgccccattcattacccgagaacagcgctgttcgttggtcatcgcaaatgatcaataccttgcagatccagtttcatcggcttattaagcatcaggttgaatactaaaaaggcaaaaatcacctttctggaataagcaattccatttgaatataagagccagctcacagttctgttaatcttgcgccaacactatgactgctacgcagtgatagaaataataagatcaggagaacggggatgaactttccattaattgcgaacatcgtggtgttcgttgtactgctgtttgcgctggctcagacccgccataaacagtggagtctggcgaaaaaagtgctggtgggtctggtgatgggtgtggtttttggccttgccctgcataccatttatggttctgacagccaggtacttaaagattctgtacagtggtttaacatcgttggtaacggctatgttcaactgctgcaaatgatcgttatgccgttagtcttcgcctctattctgagcgcggttgcccgtctgcataacgcatctcagttaggcaaaatcagttttctgaccatcggtacgcttttgtttaccacgctgattgcggcgctggtcggtgtgctggtcaccaacctgtttggtttgacggctgaaggtctggttcagggtggtgcagaaactgcacgtctgaacgccattgaaagtaactatgttggtaaagtctctgatctgagcgttccgcagctggtcttgtcctttatcccgaaaaacccgtttgccgatcttaccggagccaatccgacgtcaattatcagcgtggtaatttttgccgcattcctcggcgtagctgcattgaaactgctgaaggatgatgcgccgaaaggtgaacgcgtcttagccgctatcgataccctacaaagctgggtgatgaaactggttcgcctggtcatgcagttgaccccttacggcgttctggctctaatgaccaaagtggttgcaggttctaacttgcaagacatcatcaaactgggaagtttcgttgtcgcgtcctacctcggtctgctgattatgtttgcagtgcatggcattctgctgggcattaatggcgtgagtccgctgaagtacttccgtaaggtatggcctgtgctgacgtttgcctttaccagccgttccagtgctgcgtctatcccactgaatgtggaagcacaaacgcgtcgtctgggcgttcctgaatccatcgccagtttcgccgcctctttcggtgcaaccattggtcagaacggctgcgccggtttgtatccggcaatgctggcggtgatggttgcgcctacggttggcattaacccgctggacccgatgtggattgcgacgctggtcggtattgttaccgttagttccgcaggcgttgccggtgtcggtggtggtgcaactttcgccgcactgattgtactgcctgcgatgggcctgccagtaaccctggtggcgctgttaatctccgttgaaccgcttatcgacatgggccgtacggcgttaaacgttagtggctcgatgacagctggcacgctgaccagccagtggctgaagcaaaccgataaagccattctggatagcgaagacgacgccgaactggcacaccattaattcttatgctggcaacggtccgttttgtataggggccgttgccttactttttaaatgttccatcgcggcgatgcatactgactcatatttaaacagatcgtcagcgaaaaaaatgtccaacttatcaatacattcctggctcaatgaatgtgcctgtagcgagaagcttaaaacctcatacccgagacgttttctaagtgaactatctggaatactcataatatcttcaagcacaccacttcccattcccggaagatttagtggattaaaaagaagattgatattaagcattgatattatcgaaggaaactttaggagactctcatttttttgaatcgcagcaaaaatgctcccgacaggatgtatataattttgttcatagtatatagtccttaaatagtgaataaccaacctgttttttatactgatcaaattggtcattttttctgggcgaaatacagaagtgacatccattccaataaaatctttatttatacctcttatccgaatttcactaccataaagattattaattattactctatatttaacattgtcctgcagatatgtatcaaaactaagtgctggcgctcctggctttgaggcatcatagttaatgttagacatataggcaatcatataattaaagtttgattctgctatttcatcgcagtcacattgacccgttgatataaagaaagtgagtgctgtcatagtagactgcagcctttctttaaaagagtcgaaagccaggcttttaatatttaaatcaccataattactctgtattaagtttgtagaaaacatctcccgcctcatattgttaacaaaattattatctcatttaaatctaagtcatttacaatataagtttaagagcgacgccacaggatgaactatcaaaaatagctcatcatgattagcaaaacttaaccattttaaaataaataaacaattaaagaaaaaagatcacttatttatagcaatagatcgtcaaaggcagctttttgttacaggtggtttgaatgaatgtagcaacgaaatacagaatttcaggtcatgtaactcccggcaaaaccgggaggtatgtaatccttactcagtcacttccccttcctggcggatctgatttgcccaacgttgggcagattcaggcacagtaaacgccggtgagcgcagaaatgactctcccatcagtacaaacgcaacatatttgccacgcagcatccagacatcacgaaacgaatccatctttatcgcatgttctggcggcgcgggttccgtgcgtgggacatagctaataatctggcggttttgctggcggagcggtttcttcattactggcttcactaaacgcatattaaaaatcagaaaaactgtagtttagccgatttagcccctgtacgtcccgctttgcgtgtatttcataacaccgtttccagaatagtctccgaagcgggatctggctggtggtctatagttagagagttttttgaccaaaacagcggccctttcagtaataaattaaggagacgagttcaatgtcgcaacataacgaaaagaacccacatcagcaccagtcaccactacacgattccagcgaagcgaaaccggggatggactcactggcacctgaggacggctctcatcgtccagcggctgaaccaacaccgccaggtgcacaacctaccgccccagggagcctgaaagcccctgatacgcgtaacgaaaaacttaattctctggaagacgtacgcaaaggcagtgaaaattatgcgctgaccactaatcagggcgtgcgcatcgccgacgatcaaaactcactgcgtgccggtagccgtggtccaacgctgctggaagattttattctgcgcgagaaaatcacccactttgaccatgagcgcattccggaacgtattgttcatgcacgcggatcagccgctcacggttatttccagccatataaaagcttaagcgatattaccaaagcggatttcctctcagatccgaacaaaatcaccccagtatttgtacgtttctctaccgttcagggtggtgctggctctgctgataccgtgcgtgatatccgtggctttgccaccaagttctataccgaagagggtatttttgacctcgttggcaataacacgccaatcttctttatccaggatgcgcataaattccccgattttgttcatgcggtaaaaccagaaccgcactgggcaattccacaagggcaaagtgcccacgatactttctgggattatgtttctctgcaacctgaaactctgcacaacgtgatgtgggcgatgtcggatcgcggcatcccccgcagttaccgcaccatggaaggcttcggtattcacaccttccgcctgattaatgccgaagggaaggcaacgtttgtacgtttccactggaaaccactggcaggtaaagcctcactcgtttgggatgaagcacaaaaactcaccggacgtgacccggacttccaccgccgcgagttgtgggaagccattgaagcaggcgattttccggaatacgaactgggcttccagttgattcctgaagaagatgaattcaagttcgacttcgatcttctcgatccaaccaaacttatcccggaagaactggtgcccgttcagcgtgtcggcaaaatggtgctcaatcgcaacccggataacttctttgctgaaaacgaacaggcggctttccatcctgggcatatcgtgccgggactggacttcaccaacgatccgctgttgcagggacgtttgttctcctataccgatacacaaatcagtcgtcttggtgggccgaatttccatgagattccgattaaccgtccgacctgcccttaccataatttccagcgtgacggcatgcatcgcatggggatcgacactaacccggcgaattacgaaccgaactcgattaacgataactggccgcgcgaaacaccgccggggccgaaacgcggcggttttgaatcataccaggagcgcgtggaaggcaataaagttcgcgagcgcagcccatcgtttggcgaatattattcccatccgcgtctgttctggctaagtcagacgccatttgagcagcgccatattgtcgatggtttcagttttgagttaagcaaagtcgttcgtccgtatattcgtgagcgcgttgttgaccagctggcgcatattgatctcactctggcccaggcggtggcgaaaaatctcggtatcgaactgactgacgaccagctgaatatcaccccacctccggacgtcaacggtctgaaaaaggatccatccttaagtttgtacgccattcctgacggtgatgtgaaaggtcgcgtggtagcgattttacttaatgatgaagtgagatcggcagaccttctggccattctcaaggcgctgaaggccaaaggcgttcatgccaaactgctctactcccgaatgggtgaagtgactgcggatgacggtacggtgttgcctatagccgctacctttgccggtgcaccttcgctgacggtcgatgcggtcattgtcccttgcggcaatatcgcggatatcgctgacaacggcgatgccaactactacctgatggaagcctacaaacaccttaaaccgattgcgctggcgggtgacgcgcgcaagtttaaagcaacaatcaagatcgctgaccagggtgaagaagggattgtggaagctgacagcgctgacggtagttttatggatgaactgctaacgctgatggcagcacaccgcgtgtggtcacgcattcctaagattgacaaaattcctgcctgatgggaggcggcgcaattgcgccgcctcaaatgatttacatagtgcgctttgtttatgccggatgcggcgtgaacgccttatccggcctacaaaactgtgcaaattcaatatattgcaggaaacacgtaggcctgataagcgaagcgcatcaggcagttttgcgtttgtcagcagtctcaagcggcgcagttacgccgcctttgtaggaattaatcgccggatgcaaggttcacgccgcatctggcaaacatcctcacttacacatcccgataactccccaaccgataaccacgctgagcgatagcacctttcaacgacgctgatgtcaacacatccagctccgttaagcgtgggaaacagtaagcactctgacggatagtattatcgataaacgccggatgacacatcacctccagcgaacgatcaccccgatggcctgcgtcatccagcacttgcaggaacagcgactcactgatctcttcaccgtagaatgcactgctgaatccctgggtagtgcgcaggttgaccggcaaatcaaacgccatctgacgatccgcccgcaacgcaatgccctgctctgccgcaaacctggcaacaatcgggaaaatctgcgggaacatatgcacatgatgatggctatcaagatgcgtaggtttgcgtccaaatagctcaatgaaacgcaaatactgactgacaagctcctgagtaatttcttccagcggtaaagcatcttcttctgccaactgccagatccattttcccagcacaccatcgcgggttaaccccggcatagctgtcagtggcttacccatagtaaggacaaagtgcatccctatggccagactcggttcatcacgactcaactgcaccgcatggtcaatagcctgcccattcaccagcgccgtcgtcgacgtgacaatcccattgcgacaggcctcgataatgccgtagttctgacctttgcttaagccaaaatcatcggcattaacaatcagtaagcgttccataatcagcctcggttaatgtgcttttttaagctctgcgatgcagtcggcaaagtttggcagccatttctcgtgcgccagaatcatctcgcgtgccagcagctcagcatcgcgatcggaatgcaccaacggactaaggtttagcgccagtaacacatcgttaaattctccgctaagtgcggcgttactggcagcaatctcgaagcctttaatggtgtgaatcagccccattactttatcatcgaaatgcgtaatgcgcggatgtggcgtcgcgccatcgcgccccagcttacaggtcatttctactgcccagtctgccggaatattatcaatctgcccatgatgcgggatattaacgtaatgttctgcttgcttgtcgttgtagatagcgttgatcacttcgcatgctgcatcagagtaataagccccaccgcgctgttccagttctttcggcttaactttcagctcaggatttttatacagctcaaaaagttgtttctcgactttctgtactacctgcgctcgtgcgccgcctttgtagtattcgcccatttcaatagccagcatctctttctgcttgaagtaatacagcagataagaacatggcagcagattcaacgaacgaattaagccctcactaaatggcagatcgaaaatattttttacagaggacgcttttaactgccctgacgccacaccatcaagcaattcggcaaagcgcgacttgccatttatcagcacatccttaatgaacaccatatggttgaggccgaacaaatcgatagataaatcatcgctgtctttcagcatcagaacatcgcgaataaacatcttcatgccgatcggaatattacacacgccgataaagcgtttaaatccggtatgacgataaacggcttcagtgaccattcccgccgggttagtgaagttaatcacccatgcattcggacaaagttcttcgacatcttttacgatgtcaaaaatcaccggaatggtacgcagacctttaaacaaaccgcccgcgccgttggtttcctgaccaagataaccatgacttaatggaatacgttcatccagttcacgcgccggtaattggccaacgcgcagttgggtagtaacgaaatcagcatctttcaatgcttcgcggcgatccagcgttttataaagcttcatcgggacgccagcgttatcaatcatccgttggcagagatcgaaaataatatccagtttcggtttaccaccttcgacatccaccagccataattcgctgaccggcaattcgtgataacgcttaataaatccttccagtaactccggggtatagctgctcccgccaccaatagtgacgacttttaatttctggctcataatttctcccttcagtacagaatactgatatctggcatatctgcccccccggacataaataatccagcaacaggacagatatgtgaattgtcaggtataacgacttactgattaaattcagtcaatttcttacgatagctcttaggcgtaaaggacgttaatttcttaaacgttttaataaacaaactcgggctactataaccggcctcaaacgcaatatccgtcactgaatagttggtcatttccagttgttttttggcaaaattaatacggatttcattaataatctgcattggcgttttgccataatatcgttgagtcgctcgcgtcaaatattcctgtgatttggctgacaacgccaccatattctccagcgccgattcactaaactgctctttatcatgcatcttttctaccgtacttttcagccactgcggtacatcatcaatcacctgttcttcgcggtaatgacgtaaacggttaatgacataaaaagtaaccatctcaacaaactcttccagccctgtttcgcggaaattcaatgaagaaatcactgtttccacataggtgagaaaagcgttattggtccggtatacctgcgaagcgacaaagcaataaggcaacaatggcaggtaatgctgctcaaaaaagcgtttactgatcccaacgttcaatatgcgcgtggcaccaaactcataaaaactttgatggtgcgaacctaacggaataaaaacaaaatcgccccgttccagtaacacgcgcttaccgttaatctcctggaaataacgcccggttaataccagagtaaattcataatagtcgtgctgatgcagtccgctgatactctcagttttgttatagataaacacatggaagtttttgccattaaacaactgctgttctcgggcagtggcaatttccggcgcgttaatcactggctgcatcatcgactccttatgccttcagtttttcatgaagctcaattaattcagtaatcagttcacgcgcaagcatggacgtcattaaatgatcctgagcgtggaccagcaccagactcactttcatcttaccttcgcccgcatcgccttcaatcagtttcgtctgtaccagatgcgcttcattcaatgccatccgtgactgatccatcatggcttttgctgcggcaaaatcgccctgcttcgcctgtttcagtgccgcatacgccaggctgcgcgcttgtccggagttgatgatcagccccatcaccacttcttccagctcttcagcttccgtttgcgtatcgggaatgttatcgagatccatcatacatcgttcctctcttttcttaccggcacgattacccgtaccggcatcgattaaaatttcagggcgttagcgatatcttcttcgctctcttctttatcaatcgcattttgtgctttgttagccaccacaacaaagggcagataaattaacgttgcgatgccaaggttgaagagtgcgaccagcaatgcggcgacgctaccgttggtgttaaagaaggctcccagaccggttggcatggtccacggtgcaatattggtcaccggaggaataatgcccatgtagtacgctgcgagggtgattgccgccagaatcggttgtaccagtacaaacgggataaacatcaccgggttcatgataattggcagaccaaacagaatcggttcgttaatctggaagatgccggacggcagcgccagttttgccacctgacgataatcagcacggcgagaggcgataaagatagccaggatcaggcctaaagtcgcaccactgcccccaaggaaaataaaggagtccagcatcggcttggcccagatatggaaggtcttaccggctgccagcgccgcttcgacggaaccatattgctgataggtcgcgatattttccagtgcccacggcgtcataatgccgttgtccagtgcggtcagcgccagcgcgccatgaataccgaagaaccagagcagtggaacaaagatcacataggcccagcccaccacgctacccaacgatgccagtggggttgagatggtatccataatgatctgatggaagttggtgccccaggtattcaacgcccaggcaataatccccatcacggaaagaataataaagccgggaattaatgccgagaaggaacgcgatactgaagcaggtacgctgtcgggcagtttaatgacccaattgcggcggacaataaaggtaaacatttctgccaccaccaggccaataataatcccggagatgatattcgccccacctaaccagtttgcaccaaccgcataggcctcaccgacactatatggggtgacggtcataaatgctgcaacggataacaacccagccgccagcgcatcgactttacgctcttctgccagcgccatgccaataaagaacggtgccattaaagacattattcctaatgttccgttatatacgttgccgccaatacctttcagaccattaagtgtttcaatggttgaggcgtcgaggcgaatacctaaggaataaaaaaacgacccctccccaaagcttagaaaaacgttgttaattaatacaaacatggcccccgcaagggttaacggcattaagcgaataaagccatttttgattgcattaacgtgtggctgctttcctattttaactgcaaaagggaggagtaccttttcaagcgatgcaataacattactcatagaaaaatacccttaaaaaccgcaatttaaatattgcggtattgatttatgaaataactctttgacgggaaaatttaaaataaattaatttgctgcggcttttttaatcgctgcaaccgcagccttaagcacgcctaaaccatcgactttgccataaagcagcgagtcaattacttcaaccggtttgttgggtaacaaacgctggatttcgggcaacatataagcaatctgcggccctaataacacgacatcggcattctgacctttttcaccagccagtgtttccggaaatgcttcaataatgaccggaacttcatatttttctgcctgtgcgcgcatttttgataccagtaaagaggtagacatgcccgcagaacaaaacagataaatgtgtttcttttccataaaactgccctcatcgacgattatctgtcagccagacactccgcaagccttaacctgcttccatgctctgggtaacttgcgaaaccaacatgactttttttgtggctgaaaggagtatacggtatagacctgagcaatagtatttctttgaccttataaattgtttctccttgacctgtggttatgaccctcttcacatttcgggcaaataattcgcgaagataattaagaactcaggccaaaaaaaaccggcgcaatggccggtttccgttgttactcaagctttcagacgaattgattacttcgcagcctgtggatcagtgtcgtattcagcacaggtctgataaccggagttgatgacatgtccggtatcatctaacgcgacaaagtaggtttctgctttaccatcacgttgacccaggatgtaggtctggcaagtaccgcgagcatggatcatgctcacttcagacgaaggtttacccgcaatttgtgcaacctgcgcccggctcatgccttttttgacgtctttcaccacaggctgtacaaactggtctttggtacgatcataagccgtacaacccgccagcatggttaataccgccgctgcactcagaattcctgccatattcttgttcatattccgtcctcttgtttatcagcgtgttagataagcctggaatacattgggcgctttttcaagcccgtgaacgaaacggctccgctttcagaggattcctgtatgacgttttaaccaccattcagcccgctgtcgcttgtcgtttcagtagcaacgggttagctttaaggaagttttgtcttttctgtctggaggggttcaatgacattgcaacaacaaataataaaggcgctgggcgcaaaaccgcagattaatgctgaagaggaaattcgtcgtagtgtcgattttctgaaaagctacctgcaaacttatccgttcattaaatcactggtgctcgggatcagcggcggtcaggactccacgcttgccggaaagctgtgccagatggcgattaatgagctgcgcctggaaaccggcaacgaatcactgcaatttattgccgtacgcctgccctatggtgttcaggccgacgaacaagattgccaggatgccattgcctttattcaaccggatcgcgtattaaccgttaatatcaagggcgcggtattggccagcgaacaggcattgcgggaagcaggcattgaactgagcgattttgtccgtggcaatgaaaaagcgcgtgagcggatgaaagcacaatatagcattgcgggtatgaccagcggtgtcgtggtgggcaccgatcatgcagcagaagccattaccggattcttcactaaatatggtgacggcggtacggacattaatccgctgtatcgtctcaacaaacgtcagggtaaacagttactggcggcattagcttgcccggaacacctttataagaaagcgccaacggccgatctggaagatgatcgcccttctctgccagatgaagtggcactcggcgtgacctatgacaatatcgacgactatctggaagggaaaaacgtacctcaacaggtcgccagaacaatagagaactggtatctgaaaaccgaacataaacgccgtccgccaattaccgttttcgatgatttctggaaaaagtaataatttgcacatattggattgtgcgaaaaagagtaatttgttcacgccggatgcggcgtgaacgccttattcgacctataaaactatgcaaattcaatacattgcaggagtcgaataggcctgacaggcgtagcacgtcagacggtgtaacctttgtcatcgacccgcctcttttttaatcgcttcccgcctgttacactggatagataaccagcattcggagtcaacagtggtacggcgtttaacttctccgcggctcgaatttgaagctgcggcaatttatgaatatcccgaacatttacgttcattccttaatgacttacccacccgaccaggggtgtatctgtttcatggtgaaagtgacaccatgccgctctatatcggcaaaagcgttaacatccgcagccgcgtcctttctcatttacgtaccccggatgaagccgccatgctacggcaatcccgacggatcagctggatatgtaccgccggtgaaatcggcgctctgctccttgaagcgcgattaatcaaagaacaacagccgctgtttaataaacggttgcgccgcaatcgccagctctgtgccctgcaattaaatgaaaagcgcgtcgatgtggtgtatgccaaagaggtggatttttcacgagcccccaacctgtttggcctgtttgccaataggcgcgcagctttgcaagcattgcagaccatcgctgatgaacaaaaactttgttatggcctgctgggactggaaccgttaagtcgcggtcgtgcatgttttcgttcagcgctaaaacgttgcgccggagcatgctgcggtaaagagagccatgaggaacatgcgctacgcttgcgccagtctctggagcgtttgcgggtggtgtgttggccttggcaaggggcggtggcgctgaaagaacagcacccggaaatgactcaatatcatattattcaaaactggctgtggctgggggcggttaattcgctggaagaagcgacaacgttaattcggacacccgccgggtttgatcacgacggttataaaattctttgtaagccgctgctttccggtaactatgaaattactgaacttgatccggcgaatgaccagcgagccagttgatttcactgaacaacagtttaccttgcggttgtaaaagccgcagggtgtgcctgccatcgaaccagcacgcgccctggtcggtagtgagcaatttatcgcccagttgccacgccccgttaatcacaaacaccaccccgccgcgtgagccaaaggtagtaaacgtacgttcggcaattctgactttcgccttacagacatccaggcgtgtcatgatgttgaaatccatcgacatctgccctgccgtcagtttcgcttttaccacctggtccgctgcaaaggcaaaaggctggaacggttttaaggtatggttaaagcggtctgcgctttcaaggagcatctcgccgccttccagcaacgtcactatcctttccatgccgggaaacaaagaaaactccccattcgccgcgatggatgcaatgctggcacgccagtaaaaatcacgttttgccggtgggaacgtgcaaatttcgcgcgtttcaccggcagcatttcgccacagattcaccgacattttacgcatatcaaagtattccatactcgctcccggcccgttcttttcattgttatcgttcaggtaaccgtggatggttatcggcaactcgggtgatttacgttagtggtgatcaggctttttttacaactgtttgagaagagaaaagaaaaccgccgatcctgtccaccgcattactgcaaggtagtggacaagaccggcggtcttaagttttttggctgaaagattattcagcagttgcaggcattttaccttttgccgctggacgttctgtcagacgcttctcaaaattagcattaaattgctttttctgttccggcgtcaggatgttgtaaattttgttctgggtttccatgtgcgccagcatgttagctttgcgctgttcttccatttttgcgatctgcgcttcagcttttactttatcgaaggtatcgctggcaatgatgtcatgcattgcgcggcgttcttccagcggcggacgtttcatctggtcacgctggcctttcatgatttcgcggatctgctgtttctgcgcgtcggtcaggttcaggtctttgaacatcatgtcctgatgcggaccgaacttgcctttgtggtgcatcatcggcttcgcgtcagccggtgctgcggtagtggtgtctgcggcatgggccaggttagccgcgccaagagccagggtagaggcaacaaacagtgcagttaatttacgcatattctatatccttcctttcagttatttattacggctttcttaagtagcgtgccgtgttgacgagattaactttactgactttagcgtcaattaatcagagcaacggtaaaacaatgaaagtgtaaaaaacacttttgcgccaattatggagaaaaaaagaaaatttgatggagagtgatgagagaatattacaacacgatgattttgcagagattatgaagaactataccggatgactggtgataaataaagcaaataaccaggattaatctgtattaatttataagaaagcaacttaatacccgcagaatgatttctgcgggtaagtattagcttattttttcgagcattaatcccgcgcgtaatcccaacgctaccaacggattagggaataacacatactctacatcatgggttacggtaaaacgttcctctccgtcctgcgccagcaatgttcctttctcaaacggcataaaattcagcgtgtcacttgccatatgcatttcgaaggacggcgagtggcgagtaatttgcgaaaccacccgataacggagcggcggtgttctcacgataccgacactctcaccagatagcagcgcagcaattgcgctggcagttactgcaaactggcgaagatcgttttgcccaaagggcaacgctttgccaagttccagcgtacaggccagcgcgccaaaatgtctggcgctgaaatgggtaaacgtaccaccaggttcctgatggaacaccagcgcctccagccccgccgcacccagccacgtcagaaatttctcgtcccagggaatgtcgcgttgcggtaatacaccgaactgcggatgcaaggagccacgaattgcggtatgtagatcaaggtgccagcgcacagattctttgccctggtcataaaaatcttccaggcactgttccagttcgcgcgcccgacaggtttctccgctttcagcaaatagctgccaacgaccgccaaacattcgattcatatcgctatggcaataacgtttcccttgcttcagcgcaggaggattcccgaggatcaccagcaaccgccaacgtaacgggatctcgccgtgagatatcgcgccaagcaacgcgtccagcatctccacaggtgccgtctcattaccgtgtattcccgctgaaatcaccagtgcgccttgcggtggcgttaatggcgtcagttccagcacaccatcgcccagccagcgccagcgaacgccgttgatttctcgctcggtgataaccggttttttacccgttaaggtcagagcaagaaaattatccattgccccctccctcgcgctggaacggataaaccgaaccgagattcagtaattggctcaatacatccagtgcttcccgcccttcgcgcagcaattgcgggtcggccagatcggcagcagtaaggcgatcgcggtagtaacgatccacccagtcattgagcgcattaaacagcgtatcgttcatcatcaccgccggattcaccgcccggcgttcttcttctgtcaataccacccgcaaccgcaggcacgccgggccgccgccattcgccatgctttcacgtaaatcaaagacttttagttcgctaatcgggttgtcagcggcaaggagttcattgagataaccccatactccggcgtgttcccgacactcctgaggcagcaccaacatcatggaaccatcatcgcggctcagcagttggctgttaaacagataggtagacaccgtatcagacacggaaacctgagttgccggaacttctatcgccataaaaccattgacccgcgcacgcaggtttgccagtaactgtgactggcgagcgaacgcctgttggtggcaaaacagcacctggcggttactcacggcaatcacgtcattatgaaaaacgccctggtcgataacgtccgggttttgctgggcgaaaatcacctgttggggattcacctgattcagccttgccaccgcctcgctggcttcgcgagtctgtcgcgccggataacgggaaggccgggtatcattgccttcttctcgcccgtagacaaaaagttgcatacccggttcaccgtaatgaccgccgagacgattgtggtttgccgccccctcatcaccgagcaacgctacctgtggcaacgccgaatggacgctaaatttctcttcgtcgttaaaaatcgcttttaacagcgattcagtgacgggcgcttccagcgaacggtgaaatttattgttcaggttggcaacggtgagatgcactttgccatccagcgtatcggcagatggcgcgatcgttgccgcattggctacccacattggcgaagcggaactgacgctggaaagccagtgcggtgcctggcgtgcaactttttccagtacctgctcatcgctaccactgaatcccaactgacgcagcaccggaataaacggacgctcgtgcggcgggatcacggcctgggggaatcccgcatcggcaagggctttcattttcagtaagccctgcttcgccgccagtcgcgggttagacacctgaaaacggtgacgggtagaggcttcattaccaaacgacaggcccgcgtaatgatgcgtcagccctaccagcccgtcgaaattgacttcccaggcgttcatcgcaccacctcatcggaaaaatccagcccggggttaagcgtggcgggcaatgttaacgagtccgactccaggctcgccatcggccatgcgcagtaatctgcggcataccaggcgctggggcgatggttaccggaagcaccaatgccgccgaatggcgcggtactggcagcaccggtaagcggtttgttccagttaacaatccccgcccgcgcctccagcaacagttgatcgaacttttcccgctcgggggaaaccagaccgcaagagagtccgaagcgagtgttattcgccattcgaatcgcttcatcgaaagtatcataacgccagacgcgcaataacggtccgaacacctcttcatctggtacgccagcaacgcctgtcatttcaatgatccccggcgtcagcaacgatgtccctgcttgtaataagcgcggcgcaagcaggggtcgtccgcccatcgcttccagttgctgccatgcagtaaccacctgctgtgcggcctgttcagaaatcagcccgccaataaacggctgcggttcgtcatcccagttgcccggcgttaatcgctggctgacggcaaccagacgagcaagaaacgcatcgccctgcgccccgcttttcagcaataaacggcgggcgcaggtgcagcgttgaccggctgtgacaaacgccgactgaatggtcagatggacagccgcgtcgatatccgccacctcatcgataattagcggattattaccgcccatctcaagggcgagaattttctccggctgaccggagagctggcgatgcaactggtagcctgtattggcgctaccggtaaacagcaaaccgtcgagatcctccagcgcactcagcgcctgacccgtttcacgcccgccctgcaccaggttcagcacgcctggcggcaagccagcctgctgccataaacgcattaccgcttcgccactccacggtgtcagttcgctgggtttaaagataatggtgttacctgccagcaatgccggaacgatatgtccgttcggcaaatgaccagggaaattatacggcccaaacaccgccagcacgccgtgcgggcgatgtcgcaggctcgccgcgccgtccggcatttcactacgctgctcgccggtacgaacgtgatacgccttaattgatatcgcgattttattgatcatcgccgtcacttcggttgccgcttcccagcgcggcttacccgtttctctggcaataatcgcggttaattcggctttattgctttccagcagtgcggcaaagcgttcgacaacggcatgacgttcagcaaatgaaagccgcgcccagcgcggaaacgccgcacgggctgcccgacaagcctgctcgacctgagcggcatcggcatcattgccttgccataacacctcgcccgataccggattacgcttcacacgcgatgcgccctggcccgttatccagtcaccgttaatccataaagtcatgctgttttctcctctgcgcacaggcgcaccagacgaacgcgatccccggcgtggcatttgagggcatccagttgtgcggcggttaaaatcaaacgctcggttgccggatcggtacgcaccagcaccacgcggaaatggtgataattttcattggcgaccaggcaggctgggaaatcgccctgcgcaggctgcccttctgccacttccaccagccgacttttacggatggcgcgcacgcggtcgatgtcacactcaagcgtcggcccaccgtcaaagatgtcgatatagttacggtagcgaaaaccttctttctccagcaccgcgcgggcaggcgcggtttgcggatgtacctgaccgatgacgtcctgggcttcctgggataaaaagtgggtatagatcggatgtttcggcatcagttctgcaataaatgccttttgcccggtgccgcagagaaaatcggcgcggctaaaatccatcgaaaagaagcgtttaccgaggctttgccagaacggtgaatagccgtgttcgtcaatcaccccgcgcatttcagcaaccactttgtcattaaacttgtcgcgaaaagccgccataaacataaagcgcgatttcgacagcaaatagccgttgccctctttgcgccagtccgggtcgagaaacagcgtgcacagctcgctgctgccggtgtgatcgttactgagaaacagcgtcggcaatgcgttatagacattcagctcttttgaggcgtgaaccaacgtgccgacgcgatagttgtaccagggatcgttcagcccaaccgccacctcaatggcacaaatccccgccacggtgcctgtctcgctatcttccagcacgaacacatagccctgctcacttttgggcagttcgccttgccaggttttgattgccctttcgatacgcgccgaaagcgtggcttcattggcgggaagcgacgtcaggccgccgcccgttttgctggcaagctgcatcagcgccgagacatctgatcgctcaacgggacggatgaccatcatgatgaacctcggctaacaaagtgttcgcaagcagctgcaaagcgatccagtccggtcgtcacctcttcttcgctgacattgagcgcaggcgcaaaacgcaccacgttgccacccgcaatcagtaccatcacgcctgctttcgccgcttcctgagagatctgtttcgcttgcccggcgtaatcggcattcagtacacagccaatcagcaaacctaagccgcgaacttcactgaacaaaccatagcggtgattaatagtattaagacgctcaacaaaccagtcgtgacgctgtttaacgccattaagcatctctggtgtgttgatgagctccagcactttgcctgccaccgccgaggccagcggattaccgccataggtggtgccatgagtgccaacggtcatcacgcgggcgcactcttcggttgccaacaacgcaccgaccgggaaaccgccgcccagcgctttggcggtagttaacagatcaggcgtcacgccgtagtgcatataggcatacagttccccggtgcgcccgacgccggtttgtacttcatcaaaaatcaacagcgcattgtggcggttacacaattcacgcagaccttgtaaaaacgcgttgctggctggcaccacaccgccttccccctggatgggttcgacaatcaccgcacaggtagagtcgtcaatcagcgcgctggcagagttaatatcgttatatgcagcatgacgaatatccgccggcagtggcgcaaaatcctgtgaataggctggctgcccacccgcactgacagtaaacagcgtgcgaccatgaaacgcatttttgaacgccacgatgccgctcttatggctgccgtagcggtcgtgagcgaatttacgcgccagttttagcgccgcttcgttggcttccgcaccggagttacaaaagaagacgcgatcggcaaacgtggcgtcgatcaattttttcgccagtcgcagtaccggctcgttggtgtaaccgttgccggtatgccagaacttactcgcctgttcgttcagcgcttcacgcagttccggatgcgcatggcccagcgcgttcaccgcaatgccacccgcgaagtcgatatactctttcccctgctgatcccacaagcgcgaaccttcgccacgtaccggtataaagggtgccggagcgtaaacaggtatcatccattcatcaaagttttcacgcgtaattggctgagacatagcgacctctacagtaaataattcgttatttatatgttaataataagtaatgtttgcgctgtaaatgtagattgcagggttcgtgccagccagtgataaaagtgcataaacggcggaggctaactggaaatcaaggagttataaccaaaccatatgcatttaaagtgcatataaagtgaatacgtttgcgatgtgggtgaataaaaagaataaaaaacgcaatgttatgcagaagtaaaatataattctggaattgtgatcattgacgaaatttactggaaattactgcgccattctgacgcagcgcgcaccaaaagcgggcattttttgcgccatcgttgacatcattaacaaccatcgatcaaatcacttaacaacaggcggtaagcaacgcgaaattctgctaccatccacgcactctttatctgaataaatggcagcgactatgaaatttgtctcttttaatatcaacggcctgcgcgccagacctcaccagcttgaagccatcgtcgaaaagcaccaaccggatgtgattggcctgcaggagacaaaagttcatgacgatatgtttccgctcgaagaggtggcgaagctcggctacaacgtgttttatcacgggcagaaaggccattatggcgtggcgctgctgaccaaagagacgccgattgccgtgcgtcgcggctttcccggtgacgacgaagaggcgcagcggcggattattatggcggaaatcccctcactgctgggtaatgtcaccgtgatcaacggttacttcccgcagggtgaaagccgcgaccatccgataaaattcccggcaaaagcgcagttttatcagaatctgcaaaactacctggaaaccgaactcaaacgtgataatccggtactgattatgggcgatatgaatatcagccctacagatctggatatcggcattggcgaagaaaaccgtaagcgctggctgcgtaccggtaaatgctctttcctgccggaagagcgcgaatggatggacaggctgatgagctgggggttggtcgataccttccgccatgcgaatccgcaaacagcagatcgtttctcatggtttgattaccgctcaaaaggttttgacgataaccgtggtctgcgcatcgacctgctgctcgccagccaaccgctggcagaatgttgcgtagaaaccggcatcgactatgaaatccgcagcatggaaaaaccgtccgatcacgcccccgtctgggcgaccttccgccgctaatttagcagctctcctggctcaaactgggtcaggagaattaaccttgagaaaaatcaacaaactgtcagtaatgatttgttgcctgccgtcctttgttataccgtctctgcgtttttagttgtctgaccacttctctattatcaagtttgatataggaaactccacgatgaacgctgagcgtaaatttctttttgcctgtcttatttttgcgctggtcatttacgctatccacgctttcggtttattcgatctgctcaccgatttaccccacttacagacactcatccgccagagcggatttttcggctatagcctctatattctgttattcatcattgccaccctcttgctgttaccaggaagcatactggtgatcgcgggaggaatagtttttggcccgctcttagggacactactctcattaattgccgccacgctggcctcctcgtgctcattcctgctggcgcgctggctgggacgtgatttactgctgaaatacgttggccatagcaataccttccaggccattgaaaaaggcattgcgcgtaacggtattgattttcttattctgacccgcttaatcccgttgtttccttacaatattcaaaattacgcttacggattaaccacaatcgccttctggccttatacccttatttcggcactcacgaccctacccggtattgttatttataccgtgatggcaagcgatctcgccaatgaaggcattacgctgcgctttattttacaactctgtctggcgggcctggcgctgtttattctcgtccagctcgcaaaactctacgcccgacacaaacatgtggatctgtctgcttcgcgccgcagcccacttactcacccaaaaaatgaaggatagaacgatgttgcaacattattcagtgtcatggaaaaaaggactggctgcactctgtttactggctgttgctgggcttagcggctgcgatcaacaagagaatgcggcggcaaaagtggaatacgacggactttcgaacagccaaccgctgcgtgtcgatgccaataaccatacggtaaccatgctggtgcaaattaatggtcgtttcctcaccgacgacactcgtcacggtattgtgtttaaagatggctccaacggacataaatcgctgtttatgggttatgcgaccccgaaagcattttatgaagccctgaaagaggcaggtggtacgccgggcgaaaacatgacgatggataataaagaaacgactcatgtcacaggcagcaaactggatatttcggtcaactggcaaggggcggcaaaagcgtattccttcgatgaagtgattgttgacagtaatggcaagaaactggacatgcgctttggcggtaatttaacggcagcagaagagaagaaaacgggttgcctggtgtgtctggatagctgcccggtcggcatcgtcagcaatgcaacatacacttatggtgcggttgaaaaacgtggtgaagttaaattcaaaggcaatgcctcagttctcccggcggataacacgctggcaacggttacctttaaaatcgccgaataaagccaggataaaggatgatgatgatgcaatcgcgaaaaatctggtactaccgtataaccctcatcatcctgttgttcgctatgctgctggcatgggcgctgcttcccggcgtccatgagtttatcaatcgcagcgttgcggcgtttgccgccgtggaccaacagggtatagaacgctttattcagtcttacggcgcactggcggcagttgtctcgttcttgttgatgattttgcaggccattgctgcaccgctacctgcgtttttgatcacctttgccaatgcgtcgctgtttggcgcgttctggggcggcttgctgtcgtggaccagttcgatggccggcgcggcgctgtgcttttttatcgccagagtgatgggccgcgaagtggtggaaaaattaaccggcaaaaccgtgcttgacagtatggacggctttttcactcgctacggcaaacacaccattctggtctgtcggttattgccttttgtccctttcgatccaatcagctatgctgccggtttgacttcaatacgttttcgctcgttttttatcgccaccgggcttggtcagttaccggcaactattgtttattcctgggcgggcagcatgttaacaggcggtactttctggtttgtcaccggactgtttattctgtttgccctgaccgtggtgatttttatggcgaagaaaatatggcttgaacgccagaagaggaatgcctgatgggtttaccgccgcttagcaaaattcctttaattttacgtccacaggcgtggctgcatcgtcgccattacggcgaggtgctaagccccattcgctggtgggggcggatcccgtttatcttttatctggtgtcgatgtttgttggctggctggagcgcaaacgctcaccgctcgatccggtagtacgatcgcttgtcagcgcgcgcattgcgcaaatgtgcctgtgtgagttttgtgtggatatcaccagtatgaaagtcgccgagcgcaccggcagcagcgataaactgctggcagtggctgactggcggcaaagcccgctctttagcgatgaagaacggctggcgctggagtacgccgaagccgcaagcgtaacgccgccaacggtcgatgatgccctgcgtacccgactggctgcgcattttgacgctcaggcgctcaccgaactgacggcattgatcggcctgcaaaatctgtcagcccgttttaattctgccatggacattcccgctcaggggctgtgccgtattcctgaaaaacgttcttaaggagagatgatgcgccattgtgggtggttgctgggattgttatcgctgttttctctggcaacacatgccagtgactggcaagaaattaaaaatgaggccaaagggcaaaccgtctggtttaacgcctggggcggcgataccgcaattaaccgctatctcgactgggtgagcggcgagatgaaaacccattacgctataaacctgaagattgtccgtctggcggatgccgcagacgcggtgaagcgcattcagaccgaagccgcagccggacgtaaaacgggcggctcggtggatctgctctgggtgaacggcgaaaacttccgcaccttaaaagaggccaatttattacaaacgggctgggcggagactctgcccaactggcgctatgtcgacacacagctgccggtgcgggaagatttttctgtgccgacacaaggtgcggaatcgccctggggcggcgcacaactgacgtttatcgcccgccgcgatgttacgccacagccaccacaaacgccgcaagccttactggagtttgctaaagccaatcccggcacggttacctatccgcgcccaccggactttaccggcacggcgtttcttgaacagttgctgattatgctgacgcccgatcccgccgcattaaaagaagcgccggacgatgcgactttcgcccgtgtcactgctcccttgtggcaatatcttgatgtgctgcatccgtatttgtggcgcgaaggaaaggatttcccgccttcacccgcgcggatggatgctctgctgaaagccggcacattgcgcctgtcgctgacctttaaccccgcgcatgcgcagcaaaaaatcgccagcggcgatttgcctgcaagcagttacagttttggctttcgcgaggggatgattggcaacgtgcatttcgtcaccattcctgccaacgcgaatgccagtgctgcggcgaaggtagttgccaatttcctgctctcacccgatgcgcaactgcgtaaagcagatcccgctgtctggggcgatccttctgttctcgatccgcaaaaactgcctgacgggcagcgcgaatcattgcaatcaagaatgccgcaggatctgccgccggtactggctgaaccgcacgcaggttgggtaaatgcgctggaacaagaatggctacaccgttacggtacgcattaatctttttgctgtgggcgatggtggcggtgatttatgcaccgctgatcccggcagctctcacgctgatatcgcctgctttgtcgttgacacactggcaggcgttatttgccgatccacagttaccgcaggcattactggcaacgctggtgtcgacaaccatcgcggcggtcggggcattgttgattgccctgctggtgattgtggcgctgtggcctgggccgaaatggcagcgtatgtgcgcccgtctgccgtggctgctcgccattccccatgtggcttttgccaccagcgcccttctgctctttgctgacggagggctgctttatgactatttcccgtatttcactccgccaatggaccgatttggcatcggtctgggcctcacccttgcagtgaaagaaagcgcatttctgctgtggatcttagcagcagtattgagcgaaaaatggctgttgcagcaggtcattgtgctggattcgctgggctacagccgctggcaatgcctgaactggctgctgttgccctccgtcgcgcctgcgctggcaatggcgatgctggcgattgttgcctggtcgctgtcggtcgtggatgtggcaattattctcgggccaggtaatcccccgacgctggcggtaattagctggcagtggttaacccagggcgacattgaccaacaaacaaaaggcgcgcttgccagcctgctgttgatgctgttactcgccgcctacgttttgctgagctatctgctatggcgcagctggcggcgcactattccccgcgtagatggcgttcgcaagcctgccacgcctttattgccgggcaatacgctggcgatttttttacccttaaccggtgtgctgtgtgtggttctgctggcgatcctcgcggatcagtcgacgatcaatagtgaagcgctcatcaacagcctgacaatggggctggtggcgacattcatcgctttgctcctgttactgctgtggctggaatgggggccacagcgtcgccagttgtggctatggttgcccattttattacctgctctgccactggtggcgggccagtacacgctggcgctatggctgaaactggatggaagctggacggcggtggtctgggggcatctgctgtgggtgatgccgtggatgctgtttatcctgcaacccgcctggcagcgcattgattcacggttaattttgattgcgcaaacactgggctggtcgcgggccaaaatcttcttttacgtgaaatgcccactcatgttgcgccctgtgctgattgccttcgcggtgggatttgcagtcggtattgcgcagtatatgccaacgctgtggctgggcgcggggcgttttccgacgctcaccactgaggcggtggcattaagcagcggcggcagcaacggtattctcgccgcccaggctttatggcaactgctattaccgcttattatttttgccctgaccgcgttagtcgcaaaatgggtaggttatgtcagacaaggactccgctaatgctctgcgtgaaaaatgtttcgctacgtttaccagaaagccgcttgctgacaaacgttaactttacggtggataaaggtgacattgtcacgttaatggggccgtctggctgtggaaaatccactctgttttcatggatgattggtgcactggccgaacagttttcttgtacaggtgagctatggctcaatgagcaacggattgacatcctacccaccgcacagcgtcagattggcattctttttcaggatgcactgttatttgaccagttcagtgtcgggcaaaatttactgctggcgctaccggcgacacttaaagggaatgcccgacgtaatgccgtgaatgatgcacttgagcgttcaggccttgagggagctttccatcaggatcctgccactttgtctggcggtcagcgagcgcgcgttgctctactacgcgcccttctcgcccaaccaaaagcgttactcctggatgagccattcagccgtcttgatgtggctctgcgcgataattttcgccagtgggtgttcagcgaagttcgcgccctggcgatccccgtcgttcaggtaacgcacgatctccaggatgttcctgctgatagttctgttctggatatggcgcagtggtcagaaaattacaacaaactgcgataacgcaaagtttttctcaatgcgtcagttcagaatggcgcactcaaaactacaatgtcgggattttcgatgaaacgtgtttctcaaatgaccgcgctggcaatggctttagggctggcttgcgcttcttcgtgggccgctgaactggcgaagcctcttacacttgaccagcttcaacaacaaaatggcaaagcgatagatactcgccccagcgcgttttataacggctggccacaaaccttaaatggcccttctggtcatgaacttgccgccttaaacctctctgccagctggcttgacaaaatgagcaccgaacagctcaacgcgtggatcaagcaacataacctgaaaaccgatgctccggtggcgctgtacggtaatgacaaagatgtcgacgccgtcaaaacgcgactgcaaaaagcaggtttaacgcatatctccatcctgagtgacgcgctaagcgaaccttcccgtctgcaaaaactgccgcattttgagcagctggtttatccgcaatggctgcacgacctgcaacaaggtaaagaggttacggcgaaacctgccggtgactggaaagtcattgaagcggcctggggcgctcctaagctttaccttatcagccatattcccggcgctgactacatcgataccaacgaagtggaaagtgaaccgctgtggaacaaagtttctgatgaacaactaaaagcgatgctggcaaaacacggcattcgccatgacaccacggtcattctgtatgggcgtgacgtatacgctgcagcgcgtgtggcgcagattatgctttatgctggcgtgaaagatgtgcgcctgctggatggcggctggcaaacctggtccgacgcgggactgcctgttgagcgcggaacgccaccgaaagtgaaagcggaaccggatttcggcgtgaagatcccggcacaaccgcagttgatgctcgatatggaacaggcccgtggactgctgcatcgccaggatgcatcgctggtgagcattcgttcgtggccagaatttatcggtacgaccagcggttacagctatattaaaccaaaaggtgaaatagccggcgcacgttggggacacgctggtagcgactcgacgcatatggaagattttcataacccggatggcaccatgcgcagcgccgatgatattaccgctatgtggaaagcgtggaatatcaaaccagagcagcaagtttcattctactgcggcaccggctggcgcgcgtccgaaacctttatgtacgcacgcgccatgggttggaagaatgtttccgtgtatgacggcggctggtacgaatggagcagcgatccaaaaaatccggtagcaaccggtgaacgcggcccggacagtagcaaataacattgcaattactgacgctggagcgacttcagcgtcagatacccactccacacccgcgtaaaggtcgtcatccagcacaacgcaccgaagatccacgcaaaccacgcaaaccatgcagggaataaacatcccagcacaaacagtaagatcgtttctgtgccttcggttaatccccccagatagtaaaacgacttatgtgcataaccggggttatcaatctgatgttttgctgccagtgcagcaaaggcgagaaaactgctgcccgtgccgataaacgcaaacaacaaccagccgcctgccagcgcattttgctccggtgcagcaagaataaagccaaacggcaccagcgcgtaaaagagaaaatcgagagaaatatcaagaaagccgcccgcgtcggtaagctctctgcgccgcgccagcgcaccgtccagaccatcaagcagcctgttcaacaaaatgacgactagcgccgccagataccagcccagcgccagaaacggcagagccagcacgccgatggcaaatcccactaatgttaaaccatctggcgtaatgcccggtttatcaagaacccgcacgcactgatgcaacaacggtttaatccggggatgaagatggcggtctagcacaggcactccttaaatataaagcctttctgattgagcaacagtgcggatattatggcatttttcgcttatctgcccgtgtgtaatttatgaaaatgattgaagttgttgccgccatcattgaacgtgatggcaaaattttactcgcgcaacgccccgcccagagcgatcaggcgggattatgggagtttgccggtggtaaagtcgagccggatgaaagtcagcggcaggcgctggtgcgtgagttacgcgaagaactgggcatcgaagcaactgtgggtgaatatgttgccagccatcagcgagaagtttcggggcggattatccatcttcatgcctggcacgtacccgacttccacgggacgttacaggcacatgaacatcaggcgctggtctggtgctcacctgaagaggcgctgcaatatccgctggcccctgctgacattccattattagaggcgtttatggctttacgcgccgccagaccagcggattagtgctaagggttttgtcatcacgctggcattgcagcagtattccttcggctttaattaccgccccttcagaataattttgatcctgataaacgcagcactgagtacagggctgcgctgactgcccgcctgaactgaacacttctggcggtacgtttacctccacgtccggacgataatgcgggttagccagtgcaattaatggaaatgctaatactacggcgaacaatgctcgactcacagggaactccttaacgttattgtctctgctactgataacggtagccgggtggcaaaactttagcgtctgagttatcgcatttggttatgagattactctcgttattaatttgctttcctgggtcatttttttcttgcttaccgtcacattcttgatggtatagtcgaaaactgcaaaagcacatgacataaacaacataagcacaatcgtattaatatataagggttttatatctatggatcagacatattctctggagtcattcctcaaccatgtccaaaagcgcgacccgaatcaaaccgagttcgcgcaagccgttcgtgaagtaatgaccacactctggccttttcttgaacaaaatccaaaatatcgccagatgtcattactggagcgtctggttgaaccggagcgcgtgatccagtttcgcgtggtatgggttgatgatcgcaaccagatacaggtcaaccgtgcatggcgtgtgcagttcagctctgccatcggcccgtacaaaggcggtatgcgcttccatccgtcagttaacctttccattctcaaattcctcggctttgaacaaaccttcaaaaatgccctgactactctgccgatgggcggtggtaaaggcggcagcgatttcgatccgaaaggaaaaagcgaaggtgaagtgatgcgtttttgccaggcgctgatgactgaactgtatcgccacctgggcgcggataccgacgttccggcaggtgatatcggggttggtggtcgtgaagtcggctttatggcggggatgatgaaaaagctctccaacaataccgcctgcgtcttcaccggtaagggcctttcatttggcggcagtcttattcgcccggaagctaccggctacggtctggtttatttcacagaagcaatgctaaaacgccacggtatgggttttgaagggatgcgcgtttccgtttctggctccggcaacgtcgcccagtacgctatcgaaaaagcgatggaatttggtgctcgtgtgatcactgcgtcagactccagcggcactgtagttgatgaaagcggattcacgaaagagaaactggcacgtcttatcgaaatcaaagccagccgcgatggtcgagtggcagattacgccaaagaatttggtctggtctatctcgaaggccaacagccgtggtctctaccggttgatatcgccctgccttgcgccacccagaatgaactggatgttgacgccgcgcatcagcttatcgctaatggcgttaaagccgtcgccgaaggggcaaatatgccgaccaccatcgaagcgactgaactgttccagcaggcaggcgtactatttgcaccgggtaaagcggctaatgctggtggcgtcgctacatcgggcctggaaatggcacaaaacgctgcgcgcctgggctggaaagccgagaaagttgacgcacgtttgcatcacatcatgctggatatccaccatgcctgtgttgagcatggtggtgaaggtgagcaaaccaactacgtgcagggcgcgaacattgccggttttgtgaaggttgccgatgcgatgctggcgcagggtgtgatttaagttgtaaatgcctgatggcgctacgcttatcaggcctacaaatgggcacaattcattgcagttacgctctaatgtaggccgggcaagcgcagcgcccccggcaaaatttcaggcgtttatgagtatttaacggatgatgctccccacggaacatttcttatgggccaacggcatttcttactgtagtgctcccaaaactgcttgtcgtaacgataacacgcttcaagttcagcatccgttaactttctgcgatagcagcagatatgccagtaaagaaatcccatttgactatttttttgataatcttcttcgctttcgaacaactcgtgcgcctttcgagaagcaagcattatataatgccaggccagttcttcttcaattgtcccgttttgaaaagctgtgcttgatatcgagatcatccatgataattccgccgcccatattagcttcgccgaggatttaccggagctatgattagcgcaatcagagatatagtctgagggaaaaacagcaaatttattcaacaaggcgataacctgctctggggcttcctccatgtttgctttaaaggtattggctccatggtcgccagaaagaaaatgctccattaaggcacaataactttcgctatcttcgataccccattgatcctctaaagactcgcgtcttttacttatgatatcgatcgagtcaaaaggaagcacatgatattggaaggtatctttgccaggttcaggctttcgcggccagaactccagcgtttcagaccattgcttatgatagaatcgataaggtgcgatcaattgtagcgcctgtaacttctcgatactgagcggctcaatacctttagcctgataataatgcagttgttctttttttgctttaaaaccggcccgaacaataagccccatcataattaatagataaagaaaagagcatcccgcggtaatcaggcctctttcattcaaaccgttggatgttatcgctgcgaacacaaacattacagcgacaacacatgttaaataaaacccccacttacaaagcagcatggccttattttctttaatcatccgttcaaaattactattaaatatttcccagccattaaaagaatacttctcgctcccaggatggttttgtaataaaacttttttcatcacattccctgttattacatactttagaggcgataattttatccatgcaaaaaaaatatccaacgaattttcttgatccgctggatatttcagaatatgactcgaatagcacgaaagattcactcgcttacgctatcgccccgcttccgacttcatctgctggcggactttttttcgcactacgtttacgcggtgcagcctttttcttatcagcactgccaccactgcccggagccacaatgccgcgaaactgccgcaccggcgtacgtttggcttgatcaataagctgatatagcgtccccaccagcggctgcataaagtcctgatagcgacactgcttttcgctgatttgcgtcagcaccgattcccagtgcgcggtcatgtccggtcgcgtcgccatctccggcagcgaatggaatagcgcttttccggcgtcggtggagtggatatagcgcccttttttggtcaggaaaccacgcttgaacaacagttcaataatcccggcacgcgttgcctctgtccccagaccatcggtcgcacggaggatctttttcagatctttatcctgcacaaagcgcgcgatcccggtcatcgccgaaagcagtgttgcatcggtaaaatggcgcggcggctgggtttgccgctctaccacttcacctttttcacacagcaactcatcgcctttcgccaccacaggcagtggcgtgccgtcgttttcttcatcgcgctctttgctgcctaacagcgtgcgccagcctgcttcagcaagaaaacgcgctttagcgacaaatttgcctttggcaatgtccagttcgataacacacttgcggaacaccgcatccgggcagaattgcatcagatactgacgggcaatcaggttatagaccttcgcttcgttctccgtcaggttgatcgcagaactccgtgcggtcggaatgatggcgtggtgcgcatcgacctttttgtcatcccaacagcggttgcgtatatctggatctaccactggctgcggcaacagatccggtgcatgaacactgatggcattcatcaccgcgtggcgtccggcaaaatgttcttctggcaaatagcgacaatcagaacgcggataagtgattagcttgtgcgtttcgtacagtttctggcagatatcaagcacgttctgcgcactcagaccaaaacgttttgccgcttcaatctgcaacgctgaaagcgaaaaaggcagcggcgcggattctgattcccgtttatcgttatagctggtgacaatagccggttgaccactaatgcggttaaccacatgctccgccagtggacgatgtaacaagcgcccttcttcatcctggtacggttcacacgcttcgctcggttgccagatagcggtaaaccgctcatcggcaggtgtcacgatatgtgctttgacttcaaagaagtctttcgccacgaagttttcaatctcttcatcgcggcgcaccaccagcccaagcacgggcgtctgcacgcgtcccacggaaagtacgccctgataaccggcattgcgaccgagaatggtatacgcacgggtcatattgatgccgtacagccagtcggcacgcgctcgcgccagcgcagaaacgcacagcggtacaaactcactgttggaacgaagacggtcgatcgcccgctcaaccgcctgcgggttcaggtcgtttatcaagcaacgctgtacctgctggcgcttttccggtgccagttgcagatagtccagcacttcatccaccagcaattgcccttcacgatccgggtccccggcgtgaacgatttcgctggcttcatgcaggaaccgtttgatgacgttaagttgtttggtcacggagggtcggggctgtaattgccacttttccgggacaatcggcaaatccgcaagattccagcgcgcatagcggctgtcgtaggcgtctggctgcgcctgctcaagcaggtgaccgatacaccaggtcaccacctgaccattaccgcactcgataaagccatcgcctttccggtgcggtttgggcaggacatcagcaatggcgcgcgccagactcggtttttcggcaataaacaaccgcattgaattaacgaatctcaaccatggcacgaccgccgcgcgctggcaccagttcgccaattgccgtcagttcaatgccaaactcggcggctgtagctttgacctcattttctgcttccggcatgaccgccagcagcaaaccgccagaagtttgcggatcacacagcagatcgcgcacttcacgcggcatttcacccatcagatgaccgtagctggcaaagttacgttcagtgccgccaggtactgcgcccaacttaatgtactcttcaacaccggggagtttcgggatcgcttcatagtcgacgcgtgcctgcacaccagccccctgacacatttcgctcaagtggcccagcagaccaaagcccgtaacgtcggtcatcgcttttacgccttcgatgttggcaaaggacgcgcctgcgatgttcatccggcacatcacttccgtcgccagtccctgatgttctggtttcaacagtgattttttctcagccgtggtaagaacgccgatccccagcggtttcgtcaggaacagtttgcatccggcttgtgcggtactgtttttcttcacccgctcggtcggtacgatccccgttaccgccagaccaaaaatcggctccggcgcatcgatggagtgaccgccagccagcgcaatacccgcctgacgacatgcatagcgtccaccttcggtcacttcgcgggcaatttctggggaaagtttgttaatcggccagccgaggatcgcaatcgccataatcggtttgccccccatcgcgaagatatcgctgatggcgttagtcgccgcaatgcggccaaaatcgaaaggattatcaacgatcggcataaagaagtcggtggtactgataacgctggtgccattgcccagatcgtacaccgccgcatcgtcgcgggtttcattacccacaagcaaattcggatcaacaaacttcgcctgctcactatgcaggatggtttccaacacttttggggaaattttacagccgcaaccagctccgtggctgtattgggtcaaacgaatcgagttctcgctcatggacatctcctgtcaatgcaatccgggtatggtaaccctcattccgtgaagtgataagtgagagtgtctgaattcctgcgcctttgctcacaatccagacagtttcgcgacaattatcagaaataagttacaaacggcgtcgggtccgggacgttaatcgacgtagatgctttcagctgcggcgtaccgaggtagagaaaaccgacaattttatcctgctcacggcaaccgaatgcttcacgcactaccggactttcagttaatgcgccactgcgccagatgccgccaaacccctgggcaactgctgccatttgcatcgccatgaccgcgcatccggcagacatttcctgttcccagcgcgggactttatgattctcttcgcatttcgccaccaccgtgatgatgagcggtgcgcggaacggcgcattacgggctttgtcgatagctttgtcatcactaccggcagcaatcgccccctgttccagtacggcgctgaaacgctcgcgcccttccccttcaatcacaaaaaaatgccacggttgcatggacttatggtccggcgcacgcatacccgcacgcaggatgttttgcagttgttcacccgttggcgcgggttcagccaagcgggaggcgctacggcgattgatcaatagttcgagtgcatccatttgattaactcctgtcgtgatatttattcacaaaattaacacgagagtggattttgttacagcacagtccgcaattcctgctgacaagtaccggttgggtcattacgataaccacatctattgcgcctgtgacaggtgtgaccttaagttgggagaatacatgcgaaccctttggcgatttattgccggattttttaaatggacgtggcgtctgctgaatttcgtccgtgaaatggtacttaacctgttctttattttcctcgtactggttggtgtggggatttggatgcaggtcagtggtggtgattcgaaagaaacggccagtcgtggcgcactgctgctggacatttctggtgtgatcgtcgataaacccgacagttctcagcggtttagtaaattaagccgccagctgcttggtgccagttccgatcgtctgcaggaaaactcactgtttgatatcgtcaacactattcgccaggcgaaggacgaccgcaatatcaccggtattgtgatggatctgaaaaacttcgcaggcggcgaccaaccgtctatgcagtacatcggcaaagctctgaaagagtttcgtgacagcgggaaaccggtttatgccgttggcgagaactacagccaggggcaatattatctcgccagtttcgccaataaaatttggctgtctccgcaaggcgtggttgatctgcacggctttgccaccaacggtctgtactacaaatcgttgctggataagctgaaagtttccacccatgtgttccgcgtgggtacgtataaatctgccgttgaaccgtttattcgtgatgatatgtcaccggcagcccgcgaagctgacagccgctggattggtgagctgtggcaaaactatctgaatactgttgccgctaaccggcagatccctgctgagcaggtattccctggcgcgcaagggttgcttgagggtttaaccaaaaccggtggcgataccgcgaaatatgcactggaaaacaagctggtcgatgcactggcatcgagtgcggaaatcgaaaaagcactgaccaaagaattcggctggagtaagactgataaaaattatcgcgccatcagttattacgattacgcattgaaaacgccggcagataccggtgacagcatcggtgtcgtctttgctaatggcgcaattatggatggcgaggaaactcaggggaatgttggcggtgataccactgcggcacaaatccgcgacgctcgccttgacccgaaagtgaaagcgattgtcctgcgtgttaatagcccaggcggcagcgttaccgcgtctgaagtgattcgcgctgaactggcagcagcccgggcagcgggtaagcctgtggttgtatcgatgggcggcatggcggcatctggtggttactggatttccacgccagctaattacattgtggctaaccccagcaccctgaccggttctatcggtatcttcggcgtgatcaccaccgtagaaaatagtctggattcgattggtgttcatactgatggtgtctcaacttcaccgctggcggatgtttctatcaccagggcactgccgccggaagcgcagctgatgatgcagttaagcattgagaatggctataaacgctttatcacgctggttgctgatgcgcgtcattcgacgccggagcagattgataaaattgcccagggccacgtctggaccggtcaggatgcaaaagctaacgggctggtcgatagtctcggggatttcgatgatgcggtcgccaaagcagcagagctggcaaaagtgaaacagtggcatctggaatattacgttgatgaaccgaccttcttcgacaaagtgatggacaacatgtctggttctgtccgggcaatgttgccagatgcgttccaggccatgttacctgcaccgctggcctcggtagcctctaccgttaaaagtgaaagtgacaagctggccgcgtttaatgacccacaaaaccgttatgcgttttgcctgacctgcgccaacatgcgttaagtcttgtactgagtggccgacagatcgtcggccacattattttttacgtcgacgaatcctcttcccgctgtttcgccccatatttccttatccgcatagtatcaggtgcgctccccctgcctcacgtatatacttttgctctttcgatatcattcatatcaatatcatgcaaaagaaatcaatttacgttgcctacacgggcgggaccatcgggatgcagcgttccgagcagggttatataccggtgtcaggtcatctacaacgccaactggcgctgatgccggaattccatcgcccggagatgccagatttcaccattcatgaatatacgccgctgatggattcttcagatatgacgccggaagactggcagcatattgctgaagatattaaagcgcactatgacgactatgatggttttgtcattctgcacggcaccgacacgatggcgtataccgcctctgcgctgtcgttcatgctcgagaatctcggtaaaccggtcattgtgacagggtcacaaatcccgctggctgagttacgctctgacggacaaattaatctgctgaatgcgttgtacgttgcggcgaattatccgatcaacgaagtaacgctctttttcaataaccgattgtatcgcggcaaccgcactaccaaagcccatgccgatggttttgatgcgtttgcctctccaaaccttcctccgttactggaagcaggtatccatattcgtcgtttgaatacgccacccgccccgcacggtgaaggggaattaatcgttcatccaatcaccccacaaccaattggcgtagtgacgatttatccagggatttctgctgacgtcgtgcgcaattttctgcgccaaccggtgaaagcattgattctgcgctcctatggcgtgggtaatgcgccacaaaacaaagccttcctgcaggaattacaagaagccagcgatcgcggtattgtggtggtcaacctgacacaatgtatgtccggtaaagtgaacatgggtggttatgccaccggtaacgccctcgcccatgccggcgtaattggcggtgcagatatgactgtagaagccacgctaaccaaactgcattacctgcttagccaggaactggatactgaaaccattcgcaaggccatgagccaaaacctgcgcggcgaactgacgccggatgattaaggagactgtaatgccccctcgcgccctgttactggtcgatttacaaaatgatttctgtgctggtggcgcgctcgccgtgccggaaggtgacagtacggtggatgtcgctaaccgcctgattgactggtgccagtcgcgcggtgaagcggttatcgccagtcaggactggcacccggcgaatcacggcagttttgccagtcagcacggtgtagagccttatacgccaggccaactcgacggtttgccacaaaccttctggccagatcactgtgtgcagaacagtgaaggcgcacaattacatccgttactgcaccaaaaagcgatcgcagcggtgttccataaaggcgaaaatcctttagttgacagttacagtgccttttttgataacggccgtcggcagaaaacctctctcgatgactggttacgcgatcatgaaatcgatgaattgatcgttatgggcctggctactgactattgcgtgaagtttaccgtgctggacgcgttacagttaggttataaggtaaacgtgattaccgatggttgtcgtggcgtgaatatccagccccaggacagtgcgcacgcgtttatggagatgtcagcagctggggcaacgctatatacgctggcagactgggaagagacacaggggtaattttacgctggcctacaattctgtactggcattgtaggccaaataaaacacgtcagtggcacatctggcaattgatgccatcaacgaaagatttaattcacctcagaaatctcttccaacgacaccttccgcgtttcgatgccaaaaatggagagaaccagcgcacagagcaataacataacaccaagtaccataaacaccgtgatcgacccataatgtgttaataatgccgcaacgccatagggcgtgaagactgcgacgatccgtccgacggcattaacgaaacccgaaccgcgcaggcgtaaatgcgttggccaaagctccgggatataaaccgccgacgcgaagcaaacatacatgtataaaaagaagatcatcaccagtccatagattaaaatcgcccactctgtagtctgaattgaatagatatagcctaacacggcaataataataagtaaggtggagccaaataaccgacgaggaaaatgatcaataattaatgccgcaataaatattcctaccggagcgccaatcataataacagcggtcattaatattgatttatcgacatcaatgccggagttaacaaatatggtcggtatccatacggtgatggtataaagcgaaatgttcattgcaattaaaacagtaatcgcgactaatgtacgtcgtaacatttcacctttaaacaggagccagaaagtacccttgattactttaaccttgctgttgctctgatacgaagtaagcgggggtaaacgaatactcttctctctttcaatttgctgctctacttcacgaagttggcattctgcacctgcgatttgccctttccctgccagccatcgtggcgactcgataaagtatttacctgagagaaaccaggctaacagtatgccaataccacccagcagaaacattattcgccaactaaaaaaagcgataaccaccacgcctatcgccgcagacagcatgggcgaccagttaccaacaaatgagagccgcgcggaccattttccacgcaccgtcgcggggataaactccgtaaatgaggcatagccaaccataatcagcgcccccattcctgttcccatcaggaagcgaaagaagatgagccagtacatatcagggacaaaagcggcccctgttgcagcaataccgacgatgagaagatttatgcgaaacgccctgcgccgcccaaagtagtcaccaataaacccaccagtaagtgagccgatgaaataaccaaacattaatgccgaggtaaaggcggcattgaggaaattatttgaccatccattgcttaccagctttgctaagacgacattaccggagtaactcaaaaaccctgttaataacagactaaagcttataataccaaatatacgataatgaaaccgggccaaaggcaagcggtccagtcttgcgccaatttgatcatattgttccattaggtgcctcggatttgctaaaaaggtagcaattgcggcaaattcacttgccgcatctttatcatcattttatttcaaggcgcaggaacaaataatattgacaacgtgtgcttaaattaccacaccagctggatattattgtctttgcaaaatgctatccactctgcacccggtgatttatcagttattatgtaattaatatgactaaaatcagctaactggacaaaagctttgcgatcaaacttagagtgatcaaccaataacgcaacttctgtcgcctgacggatcattgtctttttgatttcagcttccgcttcattagagtccagcgcgccgctgttaatatcaagacctttacaactcattaccatgatatcgacatgatagcgcctgatgatctctttagtaattcttccttgcagtgaaagtgtatttttgtttagttccccacccgttgaaacgactttaatttctgactgagccagaacatgaatcgcttccgccgagttggttagcaacgtcaggccactacggtcctgtaacaatttgagcaattccattacggtactactggaatcggctgccatggtggttttattgtcgataaagggtagtgccttgcgtgcaataagctgcttctcttcataaaacgatgaagcgcgcttataaaaatggatattctccgtcaacatcgctgtatttaaaacagcaccaccataggttctggtcaaaaagccttcatcttccagcttctcaagatcgcggcgaatggtttcttcggttacctgaaaaatcccactcaaatttgagactgtcacctttttatcgttggcaaccatttgcttaattgcctgaatcctgtcttttgccgccacgattacacccctgtatctttttacatcacattagcgcgattatcgcataaccgatgtttactttcaaaataacctgtttgaatcacagattttcatcacagttttcacagaaacagaggtgaatcgtgttgagtatttaacgctccagggcctctgccatttccctcatcaatgttgcgtctgcatccgataagttgatattcagtgccgcgacattttcgcgtacctgttccggtgcagtagccccactaagaatggagattaaatcactctgttttaatatccacgccagtgccagagtgggaattgtgcactgataacgagcacaaagtggctgccactgttcaagcatatcaatcactttcagcatgttttcacgctggaaccagactttatttgcccgagcgccgcccggaacgtaatcacgagtgatggtgccggtcaacaatccctgctctagcggggaataaacctgaaccacaatgccattatcacgacatagtggcagcagttcgttttccattgcccggtcgaggatactgtatttcgcctgaataatatccagttcaccatattgcagatactcgcggatatggtcagcatcgacgttagcagcgcctatagcgcgaattttcccttcagactttaactcattaagcactgcgacagtttcagcgatcggcgtaaaaaatggcggcaccgactgccagtgcgtcatgtagatatcgatgtaatcaatacccagacgttgcaagctcgctgctacctcttcgcggatagattccggggaaaggtttttatacaactgccgatcgccaactttgttgaataaacttccttttcgttcccagacaatgccgcatttggtttctactacaacctgttcacggggcagtttttttaacgcctgaccgacgataacttcactattgccaaagttatatcctggcgcagtatcaatcagattaatgccacaacgatgggcttcaagaatcgtatcaatacatatttgccgatcgagatcgccattccatgcaggaccgccgccaatggcccatgtccccaaccccattcgcgaaagcgtaatatccgttgtgcctaaaggtatctttttcatttgccttcattatccttcgtattcttccagcaattgttcgaccagctttctgttttttacgccggtggtggcaccgacgcttagaaccgagatagccgccgttgcattggcaaagcgtgcgcattcacgcagatttttgccttctaacagtgccgcaataaaacctgaagcaaagttatcgcccgcgccaatggtgtcgatggcggttattcctgcgaccgccggcaccttcatcgtcatgtcaccacgcttgataaagcagccgtctttacccgttttaatcaccaccgtttttacgccgcacgcaagaaagcagtcagcaatttcatccagtgtctctttcccggtgagtaattttgcctcggcaaaattaggaaacagataatcgacataactcaatgcttcgcaaatatcatccagcgtttcattcaaccgcggtttgatcatatcggcacagataatcatctgccgggctttagcttgcgtaaaaatttctgttagcgctttaccatccaatagtggactgttgaaaatactggccagtgataataatttcgcctgagaaaaccgcgcaaaatcaacatcgtcaatattcaatttccacagactgccattacggtttgtgacaaacgtccgctcgccatcctccgtcaccagtccaacgttaatagaggtatctatgctgacgtcctgcttcaggctttgaatatcaatattctctttgcggcaatggtcgagaataaattgccctgcggcatctttaccaatacgactcattaatgctgtgcgatggcccagacgagaaataattgttgcttcatttattgcatcacccccggtggtcattgcgattctttcaagaggataagaatccacatcaaagatatttttactgaccggttgcaatggaatatcaacaatagcggcacctatacaaataacgtcgagattatccatatcattattccgctttgccatcagaaccgaacagtttaattttttccaatgcccgttcttttacagctttacgtacttcacgttctaaatgcaggaaaggctgatcctggttttctttcactgcaaccattgcggcctgacagagctccgtatgaatgttgattttcgcgatacccaacgaaattgcagttttaatgtcggcatcactgatccccgatgcaccgtgcaaaaccagcggaacagaaacggcatcgcgtacgcgtttgacgacctcaaagttcaattgtggctctgacgtataaaccccatgctggttgccgatggcgacagccaatgaatcacagcccgtacgttcaacaaattcagccgcctggtcaggatcggtatagtgatagcccgccagcgcttcctcataaacggtttcattaccgacatgccctaattccgcctctaccggaatacccagcggatggaagaaatcgacagcctctttggttaaacgaatattttcttcgaaatcaaacgcggaagcatcacgcattaatgaattcataccatgagtccaggcgttatgaataatctccatactccgaccatgatcccaatgagttattaccggcaccgttgctttttgtgccattgataccatcatgtgagagaaatcttcaaatgaggtgttaccgacaaaacctgtaccaaaagaaataataaccggggatttcgcttcttcggctgcgtcgataacgcccatcaacatttctgcattccatacgttaaaatgggcaattgcataatgtttatttgtggcatcgttttcccaatatctgatatctgcgagcatgttctgttctcccgtattaattaatcgctaattttaataacgcctttaataatgtcgcgtttgttgttaactgactcttcaaatgcctgttgtacatcccgataatcgtaaatatgcgtcaccatcgatttcacatcgaatcgccctgaagaaatagcttcaatcgtgaccggataacgattggcatagcggaataccgtctggatagtgacttcgcgattgattttgaggaaattgattgccgaatcgccgggtacagtaccaacaatcataattttaccgccgcgcattaccagataaggtgcctgtttaacggtgaccgcagaacccgctgtttcgaaaacaatatctgcgcccatgtcttcggtaaattgctgacagcgtgcaatagtgtcttcttttgcgccgttaataaccactgtcgcaccaagctgttccgccattgccagacgtttttccagcacatcaacgacggcaatttccgttgctcccaggcatttgcacgcttgcaacgtcatcaaaccaatacaacctgctcccagaataattatcttcttacccggtttaacatctgccagcatcgcggcatgcatcccgactgcggcaggctccaccagcgccccttccatcgtgtccatattgtcgggcagtttgtaagtaaagctctccggatgacacagatagtgcgttaatgcgccgcggtagttgggttgtgtcgccataaaatcaacgtccgggcagatgttatatttgccttccagacagtaacgacagtgaccgcaaggaacgccaggttcgatatttacccgatcccccggtttaaatttgcgcacgcggcttcccacagccacaaccgtcccggcgcattcatgacccaggccaatttcttgatttgggtctttaggcggaataaacgggcctgattcaaaaccatgtacatctgaaccacaaataccgacatattctactttaatcaaaacttcatcttctttaggcactggtatttctgctgaaataattttcattgtgcccggcacctgcaatattgcttttgaatttttcattttgaatccacccgtattatttattggctactgcatcaatacttaaactttcaacggagacacctttggtttcgattccaatggtggcgatagcaattgcgacaataattgaaaccgcccccagaagaataaagactcccgtaacgccataactactgagcagcactgcaacggcataaggtgcggcaataccactgattcgccctaccgcattcgccagaccggagccacggagtttggcctctgtcggccagatttcagggacatacactgccgaggcatagcaaacgtacatatagacgaaagtaatcaggaagaaaccaatcaacgttatgagcaacatactggtttgcagtgaatagatatatccgagcaccgcaatcaggattaatagccccacacccattgttttacgcggaattttatccatcaccagcatggcaataaaaataccaaatggcgcgccaaacatactcatggtatttaaaacaatcgagtcttttaaattaatcccctgggtcatgaatattgttggcaaccagttaattagtgtgtactgcacaacgttcatggcaatcagcacacaagagcctaatatcacgcgtttcagtaatactcctgtcagtaaggctgaatacggcaccgcttgtggcgctttaccgtcatcagcaataaccacaggcggcaaaggtttacccgtctggcgtatgacgccttcttctatactccgcatgactttctcggcttcctgataccgtccgcgcgattccagccagcgcggggattcaggaaagtagcgccaggccagcgccgtagcgataagcgacaatattgcagggataagcagttgtacccgccagttccactctgcactaatcagcggcgtgagtcccatcgctatcaatgaacagagcggatatgaccagttgccaataaaggaaacccgacttgaccacgttccacgatttctaccgggcatatattcggtgaaaccagcaaacagcgtaaccagtaaagctcccagcccaactcccatcacaaaacggcaggcaataaggaaatccatattcggtgagaaagcaccgacaaccatcgaggcaatatgaatggcctcatagaggatgaacgcatttctgcgaccggttttgtcgccaatgatgccgcccaccagcgcaccgagaaacattccggcggtcgtgattgctgagaatgtggctgtggtggaattatctgtccagcccaacgctttcagctgcgcgaggatcaagccaccaacggcattactccagcagacaagcaagccaaacgcgacgatggcaaacattgatgaatgccagcggcaatccggtaagcgatccagccgtgcaccacaatgcggttttgttatctgttccatgcgataacgttccttcaggagagtggttattcatcaaagtcgtaagtcatgatcactttgattgcggttttatcgaccatcgcatcaaacccttcgcgccattgcgacaggccgatacgatgcgtgatcatcggtttgactttgatagcgccgctggctaatagcctgatagcgttacgccatgaggtggagtcataggccatatgcccaatgatgcttttgttccaggcggtaatgtcattaatcgagaaatcaagaggtttgaagcccattccaacgcgtaccacttccccgttcgggcggagcatttcgatggcttgtttcagtgcgatattggcaccggagcattcaatcaccagtcccagattgtctttgccacaaatttgctggcagcgcgccaccacatcttcggtagaaccatttactactgccgtcgcacccagttcttttgcaaccgggaagcggaccgccacatcttcttgcagaccaacgacgacgatatttaccgcccccataattcgcgccatttgtacggagaacagcccgagtgggccagtgccgatgacgaccacatcctgaccaggaaggaatttcgattgctgcgcgatggatttgtaggcattacagatagggtcaagtacggctgcgtcctcataatcaacaccatcagggatttcccacaacgcatgacgatgaattttgagaatttcaccaggaaccagacaatatttggaaaaaccaccgccccaggtattattatccagaccaaggtttactttttctgtacaacacagaaaatcaccttgttcacaggccggacaaacaccgcaaacgtgaccgctgttatccgatacgacgcgttgccccactttccagtctttgactttttcaccaacctgcgcaatacaacctgcgaactcatggccgcggatagagttaaactcatcagaaccgctatcgacattgtagtgcttcatgtctgcgccgcagattgccgcggctttaatttcaatcactacatcttccgggccacacatgggttgtgggacatcaatcatcttgtagccgccaaaggccttgccaaaccgagccagtgctttcattgcgtcatcctctgtgtttagttttgcttagatggccatcatacttacccacatgatttttgaggtcaacattaaatctgtaaaacacagataatgatctgcgttttacaactcagatcacaattacgcagaaaatggctgggtctgttacaggttgatggaaggcggggcgcaaaaagagcaaattcgagagggattaccggccaaataggtctgagacttaagttcaggagaagtcattcaggtgtgaacgggacggcaagagatcggactgggacttagccaggtcatggcgagataattgagatgagtcgtggggtcattgttggctatccccttcatagccgaggcaaaaaggggatgaaccacttacttaaacatggcaataggctttgctgagataccaaaatcttcttttaactgctgtttgctcttcatgaccatctgaccatttgtgtcaattgtcatatgctgtgcttcgatattatggcgggcttgccacagcatcaccagttgcaggcagttctctttttgttcctcggtcaacgcaacgccatcaggccatttccccagttcaacggcggtcgacaaacgctggtatacctcaggcatcatgctgttgataatgtcatcaagattcataatttttccgctcctgtggaataagttgctgaatcgttttttcaaccgttgatttcttcgccgttttcgccatcggtaaagcgtaaagaggcagagttaacacaataacgttcgcccgttggctgcggcccgtcggggaagacatgccccagatgggcatcacagttaccgcaacgaatttctatgcgctgcattccatgtgacaagtctttgatataacgaatggattcttcacttaccggttcgtagaaactgggccagccacagccggaatcatacttggtttgggaatgaaacagcggggcatcgcagatcaaacagtgatatacgccgtcacgcttgttatgcagtaaacgacccgtaaatggcggctctgtcccatgattctgcgtcacgtaaaactgcatctcggacaaattttttttcagttcttctgccgaaggtttattagccatttgctcacatctcactttaatcgtgctcacattacgtgactgattctaacaaaacattaacaccaactggcaaaattttgtcctaaacttgatctcgacgaaatggctgcacctaaatcgtgatgaaaatcacatttttatcgtaattgccctttaaaattcggggcgccgaccccatgtggtctcaagcccaaaggaagagtgaggcgagtcagtcgcgtaatgcttaggcacaggattgatttgtcgcaatgattgacacgattccgcttgacgctgcgtaaggtttttgtaattttacaggcaaccttttattcactaacaaatagctggtggaatatatgactatcaaagtaggtatcaacggttttggccgtatcggtcgcattgttttccgtgctgctcagaaacgttctgacatcgagatcgttgcaatcaacgacctgttagacgctgattacatggcatacatgctgaaatatgactccactcacggccgtttcgacggtaccgttgaagtgaaagacggtcatctgatcgttaacggtaaaaaaatccgtgttaccgctgaacgtgatccggctaacctgaaatgggacgaagttggtgttgacgttgtcgctgaagcaactggtctgttcctgactgacgaaactgctcgtaaacacatcaccgctggtgcgaagaaagtggttatgactggtccgtctaaagacaacactccgatgttcgttaaaggcgctaacttcgacaaatatgctggccaggacatcgtttccaacgcttcctgcaccaccaactgcctggctccgctggctaaagttatcaacgataacttcggcatcatcgaaggtctgatgaccaccgttcacgctactaccgctactcagaaaaccgttgatggcccgtctcacaaagactggcgcggcggccgcggcgcttcccagaacatcatcccgtcctctaccggtgctgctaaagctgtaggtaaagtactgccagaactgaatggcaaactgactggtatggcgttccgcgttccgaccccgaacgtatctgtagttgacctgaccgttcgtctggaaaaagctgcaacttacgagcagatcaaagctgccgttaaagctgctgctgaaggcgaaatgaaaggcgttctgggctacaccgaagatgacgtagtatctaccgatttcaacggcgaagtttgcacttccgtgttcgatgctaaagctggtatcgctctgaacgacaacttcgtgaaactggtatcctggtacgacaacgaaaccggttactccaacaaagttctggacctgatcgctcacatctccaaataagttgagatgacactgtgatctaaaaagagcgacttcggtcgctcttttttttacctgataaaatgaagttaaaggactgcgtcatgattaagaaaatttttgcccttccggtcatcgaacaaatctcccctgtcctctcccgtcgtaaactggatgaactggacctcattgtggtcgatcatccccaggtaaaagcctcttttgcattacagggcgcacaccttctctcgtggaaacctgcgggtgaagaagaagttctgtggttgagcaacaacacaccgttcaaaaatggcgtcgctattcgcggtggcgtaccggtttgctggccgtggtttggtccggcggcacaacaaggtctgcctgcgcacggttttgcccgcaacctgccgtggacgctgaaatcacatcatgaagatgctgatggcgtagcgctgacttttgaattgacgcaaagcgaagagacgaaaaaattctggccgcacgactttacgctgttagcgcatttccgcgtgggtaaaacttgtgaaatcgatcttgaatcacatggcgaatttgaaaccacctctgccctgcatacctactttaacgtgggtgatatcgctaaggtaagcgtcagtgggctgggcgatcgcttcattgataaagtgaatgacgcgaaagaaaatgtactgaccgatggtattcagaccttccctgaccgtaccgatcgcgtgtatctgaatccacaagattgcagcgtgattaatgatgaagcgctgaatcgtattatcgccgtaggccaccagcatcatctgaacgttgtcggctggaacccgggaccggcgctttcaattagcatgggcgatatgccggatgatggctacaaaacatttgtttgtgtagaaacggcttacgcttcagaaacgcaaaaagtgaccaaagagaaacctgcacatctggcgcaatccattcgcgttgcgaaacgttaatttacgttaatgttgtgtgccgggtgcaatgcatccggcacacaacatcacaccatatccagcgcagtttttccttttggtgccggatatgccttatccagcatagctaattccgctgaagaaagttcgacctcaagcacagccgcattttgttggacatgggcaatcgtggccgcttttggaatcgccatcacaccctgatgactgatcacccacgccaacaatacttgtgccgcgctgatattgtgagcatgtgcaatttcgttgactaccgcgttttttaacagtccattgcgcaaccgcccggcctgggctaacggactgtaagccatcaccggcatctgctgttgctggcaccaggggagtagatcgtactcaattcctcgtgaaccgagatggtaaagcacctgattagtggcacactgatttccccccggcagctgccagagttcctgcatatcagcataatcaaggttagaaacgccccagcggcggatttttccctgggcgatcaatttttccatcgctgcgacagtctcttcaaaagcgaaactgccagaccagtgtaataagtaaagatcgagataatcagtattgagacggcgtaaactggcttcgcatgcatttatcgctttttgcccgccagcattccacggatagactttagagacgagaaagaccttctctcgcagaccggttaatgcttccccaaccaccttttcggcaccgccatcggcatacatttcggcggtatcaatgagggttaaaccgagttcaatgcccgcgcgtagtgcagcaacttctgttttgcgctgactggcatcttcgcccatataccatgttccctgccctacggctggcagtgagacatcgccactaaattgaatcattttttgttgcattgtttcctcccaggtattgcaccaccgtaatgcaaaacagggcgtgacgccctgtttttatgcacaaaatgccctggaaagatgcattatcagaatttgtaggtgatcccggtagaaatcaggccagtccaggatttatccaccatcgggctgtcagtaacttcatcagacagacgggtgtagcgtgcggtaccgtaaacactccagtcgccgaggaagttgtagctggcgctcagctccaggtaagggctccagctgtcgttcgggttatagccacgcagaccgctgcgagcggactctttgcgcgatacgccataatagtattcgttctggttttcgctgttccactgcacaccaatacccggagtcacggtcaggccaccgttggtgtaacgatacaaccaggccatatcccagacgatgccgttgctgttatccagggtatcgccagccagggtggtacgcaggtaaccgtactgggtaaagtgagcataagacagaccagccatcatggtgctcttacggtcatccaggtgacgcatttggtgatcgccactgtctttcgctttgaagtaaagcggcgaccagtaagcggtaattgaaagtttatccgttgcgtcattccacaggtagtaaccaccacctaagccacggaaccagaagttatcgccttcatagttgattaccggtactgggtaaacatcggtatcgtaatctttatatgggtgttcaacgacacctacgcctgcgcccagggaaaatttaccttcagcgtgcgctacgcctgcagacgttgcgataagcactccaagtgccagaagtttgagtttggtcacaattaatcattccttaaacaaatgtttagcgggcgacaaagtttacccgtcaatacatcgaaacccaacctttttacgttttcattttttaaagtaactgtttaattttcctgacgcggatgacaccgcgcttacagccaaatgaatttagcgttactggcgagcctggtctttacattaattatgcaaaatttatggatgagttgttgatatgccattgaaattaagaaagccgtgcaggcaagttttccatttgccatctacgcttaattttgaaggtgtatcaccgggcacgttgttctcatcgtcgataaaatggcatgagagttgctgtgttttagcaagagacgtcgttcagtttacctcttccgggagcctctactattcatatgaacggctcttaacctgtgctaaaaaacgaaaggacggcataccatgaatatattcgatcactatcgccagcgatatgaagctgccaaggacgaagagttcacactgcaggagtttcttaccacttgtcggcaagatcgcagtgcttatgccaacgcggctgagcggctattgatggctatcggtgagcctgtcatggtcgatacagcccaggaacccagactttctcgactcttttctaaccgggtcattgcacgttatccggcgtttgaagagttttacggcatggaagacgcgattgaacagattgtctcttatctgaaacacgcggctcaggggctggaagagaagaaacaaatcctgtatctgctggggcctgtgggtgggggtaaatcatcgcttgctgagcgactgaaatcattaatgcagctcgtaccgatttatgtattgagcgcgaacggtgagcgtagcccggtcaacgatcatccgttctgtcttttcaatccgcaggaagatgcgcagattctggaaaaagagtatggcattcctcgccgttatctcggcaccatcatgtcgccgtgggcggcaaaacgcctgcatgaatttggtggcgatatcactaagttccgggtagtgaaggtctggccgtcaattctgcaacaaattgctatcgccaaaacggaacccggcgatgagaacaaccaggacatctccgcgctggttgggaaagtcgatattcgtaaactcgaacactacgcgcagaatgacccggacgcctacggctattccggtgcgctgtgccgcgccaatcaggggatcatggaattcgttgagatgtttaaagcaccgattaaagtgctgcatcccttgttaaccgccactcaggaaggtaactacaacgggacggaaggtatctccgccctgccgttcaacgggattattctcgcacactcgaacgagtccgaatgggtcactttccgtaataacaaaaacaacgaagccttcctcgatcgtgtttacatcgtgaaggtgccgtattgcttgcgcatttccgaagagatcaaaatctacgagaaattgcttaatcacagtgaattgactcacgccccatgcgcccctggcacgctcgaaacactgtcacgtttttccattctttcgcgcctgaaagagccagaaaactccagcatttattcaaagatgcgggtttatgatggcgaaagtctgaaagacaccgatcccaaagccaagtcgtatcaggaatatcgtgactacgccggtgtcgatgaagggatgaacggtctgtcgacgcgttttgcgtttaagatcctctcccgcgtgttcaacttcgatcatgtagaagtggcagcaaacccggtccatctgttctacgtcctggaacagcagattgagcgcgagcagttcccacaagagcaggcagaacgctatctggagttcctgaaaggttatctgatcccgaaatatgccgagtttatcggcaaagagatccagacggcctaccttgaatcctattccgaatatgggcaaaacattttcgaccgttatgttacctacgcggatttctggattcaggatcaggagtatcgcgatccggataccgggcagctgtttgaccgcgagtctcttaacgccgagctggagaaaatcgagaaaccggcggggatcagtaatccaaaagatttccgcaacgagattgttaacttcgtactgcgcgccagagcgaataacagcggacgcaatccgaactggaccagctatgaaaaactgcgcacggtcatcgagaagaaaatgttctccaataccgaggagctgttgccggttatctcgtttaacgccaaaacgtcaaccgacgagcagaagaaacacgacgactttgtcgaccgtatgatggaaaaaggctacacccgtaaacaggtgcgtttactgtgcgaatggtatttgcgcgtacgtaaatcgtcttaacaaccctggcccggtacacatgttaccgggcctacaacgacagcgaaccgtgggcctgagaagcggcaacacaggcgtagcatacagttggcaaatgtagtacggggggcatatgacctggtttattgaccggcgtctgaacggcaaaaacaaaagcatggtgaatcgccagcgttttttacgccgttataaagcgcaaattaaacagtcgatctccgaggccattaataagcgttcggtgactgacgtcgacagcggcgaatccgtatccattcccacggaagatattagcgaaccgatgtttcatcaggggcgtggcggtctgcgccaccgcgtgcatccgggcaatgaccatttcgtccagaacgaccgaattgaacgtccccagggtggcggcggaggttccggcagtggtcagggccaggccagccaggatggtgaaggtcaggatgaatttgtctttcagatttcgaaagatgagtatcttgatctgctctttgaagatttggccttaccgaatctgaaacaaaaccaacaacgccagctgaccgaatataaaacgcatcgggcgggttataccgctaacggcgttccggccaatatcagcgttgtgcgttcattgcagaactcactggcgcgacgcacagccatgacggcaggcaagcggcgggaacttcatgcactggaagagaatttggccatcatcagcaacagtgaacctgcgcaactgctggaagaggaacgtctgcgcaaagaaattgcagaattacgtgccaaaattgaacgcgtcccttttattgacaccttcgatttacgttacaagaactacgagaagcggcccgatccctccagccaggcagtgatgttttgcctgatggacgtttccggttcaatggatcaatccactaaagatatggctaagcgtttttatattctgctgtatctgttcctcagcagaacgtataagaacgtggaagtcgtatacatccgccatcatacccaggcgaaagaagtcgatgaacatgagtttttctactcgcaggaaacaggcggcaccattgtttccagcgccctgaaactgatggatgaggtagtgaaagagcgttataacccggcacagtggaatatttacgctgcacaagcatcggacggcgataactgggccgatgactctccgctttgccatgaaatcctggcgaaaaaattattacctgttgttcgttattacagctatatcgaaattacccgtcgtgcacatcagacattgtggcgagaatatgagcatctgcaatctactttcgacaactttgcgatgcagcacatccgcgaccaggatgatatttatccggtgttccgtgaactgtttcataaacaaaatgcaacagctaaaggctaaaactatcagccaggtcattatcgcctggctgatttttagcttactgtaaattatctcatttattacatacattagcttacaatcgctttaaatatgacagcataacctttacataatttagttccagaaaacaatcattcggaaaaatgattcagtcaacacgtatttccatggggttattctttaaatattttttatcgttaacgaaaattgatcctggtcaaaactatatatctctgccatcaataaaatccagcactcacattgctctcctttttatggtttctatgggtacacaaaaattaaaagctcaaagcttttttattttcagtttattgctgacgttaattttattttgcattactaccttatataacgaaaacacaaatgtaaaactcatcccacagatgaattacctgatggttgttgtggctttgtttttccttaacgccgtcatttttcttttcatgttaatgaaatatttcactaacaaacaaattttaccaacactcattttaagccttgcatttttaagtggccttatctatttagttgaaaccattgtaattatccataaaccaattaacggcagtacactgatccagacaaagtcgaatgatgtttctattttctatattttccgccaactcagttttatttgtttaacctcgctggcgctcttttgttatggaaaagacaacatccttgacaacaataagaaaaaaacgggaatcctgttgctggcgctgatcccttttttagtttttccccttctggcacacaatctgagcagttataacgctgactattctttgtatgtcgtcgattactgtccggacaaccatactgcgacctggggaatcaactatacaaaaatattggtttgtctgtgggcatttttactgttctttattatcatgcgcacacgattagccagcgaactatggccgttaatagcattattatgtctggcatcgctatgctgcaacttacttctactgactctggatgagtataattatactatctggtatatcagtcgcgggattgaagtttccagtaaactgtttgttgtgtcttttctgatttataacatttttcaggagctgcaactctccagcaaactggcagttcatgatgtgctgaccaatatttataatcggcgctactttttcaacagcgtagagtcattattgtcgcgacctgttgttaaggacttctgtgtcatgctggttgatattaatcagttcaaacgcatcaatgcccaatggggacatcgtgtgggtgataaagtgctggtttcaattgtcgatattatccagcaaagcatccgccccgatgatattttagcgcgactggagggtgaggtgtttggcttgctatttaccgaactcaatagtgcccaggcaaaaatcattgcggaacgtatgcgtaaaaatgtcgaactcctgaccggctttagtaacagatatgatgttcctgaacaaatgaccatcagtattggcacggttttttcaacgggtgacacgcgtaatatctcgcttgtcatgacggaagcagataaagccttacgcgaagcgaaaagcgaggggggcaacaaagtgattattcatcatatttaagtgcaaaaatattcagagccatgctttttgcgtggcttttgcatacaatttattactattacccctaaatttcccctccccagcggcgcagagatgagtataattagcgcccctgtgccaggccgcaatcgaactttatctggttttctcgtttcactaaccgaaggagtgccatttatcatgaaattgcaccatagaatgctccggcattttatcgccgcaagtgtcattgtgctgacatcttccttccttatttttgaacttgtcgccagcgacagagcaatgagtgcctatctgcgctatatcgtgcagaaagcagactcctcctttctttatgataagtatcagaatcagagtattgccgcgcatgtgatgcgcgctctcgctgctgagcagtcggaagtgtcgccagaacagcggcgcgccatctgcgaggcttttgagtctgccaataacacccatggcttaaacctgactgcccataaatacccgggcttacgcggcacactacaaaccgcatccactgactgcgacacaattgtggaagctgcagcactattacccgcttttgatcaggcagtggaaggcaaccgccaccaggatgattacggttcaggtcttgggatggccgaagagaaatttcactattatctcgatctcaatgaccgctatgtctatttttatgagccggttaatgttgaatactttgcgatgaataactggtccttcctgcagtcaggaagtattggcatcgatcgcaaagatattgaaaaggtatttaccgggcgtaccgtattgtcgagcatttaccaggatcagcgtactaaacagaacgtgatgagtttgctgacgccggtatatgtcgcagggcagctaaaagggattgtgctgctggatattaacaaaaacaatctgcggaatatcttttatactcatgaccgccctctcctctggcgttttctcaatgtcacgctaaccgataccgattcggggcgcgacattatcatcaaccagagcgaagataatctgttccagtatgtcagttacgtccatgacttaccgggcggcattcgtgtctcgttatccattgatattctttactttatcacgtcttcgtggaaaagcgttctgttctggattttgacggcgttaattttgctgaatatggtgcggatgcacttccgtttataccaaaatgtgtcgcgagaaaatattagtgatgcgatgactggactgtataatcgcaaaattttaacccctgaactggagcagcggttgcagaaactggtgcaatccggttcttcggtgatgtttattgctattgacatggacaagttaaagcaaataaatgacaccctcggtcatcaggagggggatttagcgattacgttattagctcaggcgattaaacagtcgattcgtaaaagtgattatgccatccgactcggtggcgatgaattctgcatcattcttgtcgattcgacgccgcaaattgcagcacaactgcctgaacgtatcgaaaaacgtctgcaacatatcgcgccgcagaaagagatcggcttctcttccggtatttacgcgatgaaagaaaacgatacgttacatgatgcgtataaagcttccgatgagcgtttatatgtcaataagcagaacaaaaacagccgttcatgataaccttctgtggttgtttgcttgtaatctcaggagcgtgaaatgactgaaatggctaaaggaagcgtgacgcatcagcggttaatcgctttattatcacaagaaggtgctgacttccgcgtcgttacccatgaagcggtaggtaaatgtgaagcggtgtcagaaattcgtggcaccgctctaggccagggtgctaaggcactggtatgtaaagtcaaaggcaatggcgtaaatcaacatgttctggcgatcctcgcagccgatcaacaggccgatctgagccaactcgccagccatataggcggattacgcgcttcgttggccagcccggcggaagtcgatgaactcacaggctgtgtcttcggcgcgatcccccctttcagcttccatccaaaactcaaactggttgccgaccctctactcttcgaacgatttgatgaaatcgccttcaatgcaggcatgctggataaatccgttattttgaaaaccgcggattatttgcgcattgcgcaaccagaactggtcaatttccgccgcactgcgtaactagccggtccgttcgataagaagaacggacaaaaccagtacaacagcaatggcaaaaaacgatgacgtgataatcagtgtctcgacaaacatttgatcgttcatagcatgcccccgggagatagctgttttcacgttattgttagcgtgcacaaatggcagtttgatgacagttcgcctgattttttatgcaaaaaacgtaaagattttctacttccttcctgcagcaagcgtaaagtaagcaggcttattattttttggcaaggaaaccacgatgtttgatgtcactttgctgatcctgctcgggttagctgcgctgggctttatcagtcataacaccactgtcgccgtttcaattctggtgttaatcattgtccgcgtcacaccgttaagcaccttttttccgtggattgaaaaacaggggctaagtatcgggataatcattctgacgattggcgttatggcccccatcgccagcgggacgctaccgccctcaaccttgattcactcgtttctgaactggaaatcactggtggcgattgcagtaggcgtgattgtctcctggctgggtgggcgcggcgtgacgttaatgggcagccagccgcaactggtcgccgggctgctggtaggcactgttttaggcgtagcgctgtttcgcggcgtaccggttgggccgcttattgccgcgggtctggtttcgctgattgtggggaaacagtagttaatctcgcaatatatcggcctggcgtttgccccaggcctttcttaaacatagtaataaaggccgttgttgaatcataccccagcgtatgagcaactttctgtacagtatcgcctttcactaatccctgaagcgccataatcagctgtaactgctgacgccactggcgaaaactcaaccccgtctcttttactatcagtcgggcaagattgcgttcactcatcgcaaaaaagccagcccattgccccaatgccccccactcgacaggccctttcgccatcatctccaccatcgtgcggattttaggatgagaagaaacgggcaggtgcagctgttgttgtggctgctgagggagttcatcaaacaggacctgaattaatctgcgggtcattggctcagcacgctgagtcgtcgtcctgtttgccagggttaaaattaattcccggcataagggcgatattttcaatgtgcaacatgttgtcggcattgtcactgcgctgggttcgataaacagaaaacagagttcagcattagctgttacttgattgctatgttccaccccgcccggtatccaaaccgcatattgtggcggcaccatccacaaagcattttccaccgtacaggtaattgcaccatgtagcgccagtatcagctgtcctttgcggtgctgatgtacaggactggttaactcatccgttccggcgtgaatacaaaatgcgaccgcggcttcatggtgtcggtcgggttcatagccattgagattcaacctgtgcatcattttgtccgaacttagcgataatttgtcattttagcttgattcaacataacaataaaaacggtaaggtacagcctcgtttgtaacaatgagaagcatatgacctgttcaacttcattaagcggcaaaaacaggattgtccttatcgctggcattctgatgattgccacaacattacgcgtcacctttaccggcgcagcaccgttactggatacgattcgttccgcttactcgctgacgacagcgcaaaccggcttattgaccaccctgccattattggcctttgcgctaatctcacctttggctgccccggtagcgcgacgttttggtatggaacgtagcctgtttgccgcgttacttttgatctgtgctggtatcgcaattcgctctctcccttcgccttacttattatttggcggtacagcggtcattggcggtgggattgcattaggcaatgtcttactgccaggattaattaaacgcgatttccctcattccgtcgccagacttaccggcgcatattccctgacaatgggagctgcagcggcactgggatcggctatggtcgtgccgctggctttgaacggttttggctggcaaggcgcgttgctcatgctgatgtgttttcctctgctggctctttttttatggctgccacagtggcgaagtcaacaacatgcaaatttgagtacctcgcgcgccttacatactcggggtatctggcgttcaccgcttgcctggcaggtcacattgtttcttgggatcaactcactggtctattacgtgattattggctggcttccggcgatcctcatcagtcacggctatagcgaagcacaggcgggttcactgcatggtttgctgcaactagccacagcagcacccggtttgctgatcccacttttcttacatcatgtgaaagatcagcgtggtattgcagcgttcgttgccttgatgtgcgcagtgggcgcggttgggctctgctttatgccagcgcacgcgatcacctggactctgcttttcggttttggttccggcgcaacaatgatactggggttgacgttcattggtctgcgggctagttctgcgcatcaggcggcggcactctcggggatggcacaatccgtcgggtatttgttggcagcctgtgggccgccgctgatgggtaaaatacacgatgctaacggtaactggtctgtaccacttatgggtgttgccatactttcactactgatggcgattttcggactttgcgccgggagagacaaagaaattcgctaatatccggtgctatagtgacgtaacaaatcatgcgtgaaagggagaacaaacacgatgaatattcagtgcaaacgcgtttatgatccggctgaacagagcgatggttatcgcatactggtcgaccgcctctggccgcgcggtatcaaaaaaaccgatttagcccttgatgagtgggataaagaaatcacgccgtcaacggaactgcgcaaagcctttcacggcgaagtcgtcgattatgcaacctttcgcgagcaatatcttgcagaactggcgcaacacgagcaagaaggaaagcggctggcggacatcgccaaaaaacagccgctgaccctgctctactcagcaaaaaacaccacgcagaaccatgcgctggtgctggccgactggctacgtagcttgtgattttagtacagcatccggcggttatttttcaccagccggatggtcacgccgccacaatgcccattcatcaatcgtttcaccgcccggtaatttgcaattgttgctgaccccttgcgctgtctgcactggaatgagcgtcccgcccttctgctggcaatagaccgacgccggatttgccataccaatctgcggcggtttaggtgcttctggctgagaaggggttgaacaaccagccaggaccagcaagcaaggcagaacaaaactgataattttcatttattgatctcacatatttatccaagattagagtatcgcggtatcgttttgttttgcagcactatttttattacattcactcaaaacatattacgtcttgtttcatctttgttgatgatgttttatcatgcctgcaaagattaaataatcagcatttacccgccgtatcctggagttgttccgtgtcagatcagattatcgcccgcgtctcgcaatcccttgccaaagaacagtcactggaaagtctggtccgacagcttctggagatgctggaaatggtcactgatatggaatcaacctacctgaccaaagtggatgtcgaagcgcgcctgcagcatattatgtttgcccgtaacagccagaaaatgtacatcccggagaattttaccgtctcgtgggattactcgttatgcaaacgcgccattgatgaaaactgctttttcagcgatgaagtccccgaccgttggggtgactgtattgcggcacgcaatcttggcatcaccacatttctgagcacgccaattcacttaccggatggatcattctatggcacgctttgcgccgccagcagtgagaagcgccagtggagtgaacgcgcggaacaggttttacagttattcgccggactgattgcacaatatattcaaaaagaggcactggttgaacagctgcgcgaagccaatgctgcgctgattgcgcaatcgtataccgactcgttaaccgggctaccgaatcggcgggcgatttttgaaaatctgacgacactgttttccctcgcccggcatcttaaccataagataatgatcgcgtttatcgatctggataacttcaaattaatcaatgatcgttttggtcataatagtggcgatctgtttctcattcaggttggcgagcgccttaatacgctccagcaaaatggcgaagttattggtcgtctcggcggtgatgagtttttagttgtttcactaaacaacgagaatgcggatatttcgtcgctgcgagaacgcattcagcagcaaatacgtggagaatatcacttaggtgatgttgatttgtattatcccggtgccagtcttggcatagtagaagtcgatcctgaaacaaccgatgcagacagtgccctgcatgctgccgatattgcgatgtatcaggagaaaaaacacaaacagaaaacaccttttgtcgcgcatccagcgctacattcctgaggcgtattcacatccttttgattggtgataacatgcgaatcggtattatttttccggttgtaatcttcattacagcggtcgtatttttagcatggttttttattggcggctatgctgccccgggagcataaagatgaaaaaaacaacgattattatgatgggtgtggcgattattgtcgtactcggcactgagctgggatggtggtaacgtcacctctaaaaaatagcaaaggctgcctgtgtgcagcctttgtgcaatttaagcgttaacttttaatcttcctgtagataaatagcacgacaatcgcaccaataacggcaaccacgaagctgccaaaattgaagccatcgactttaccaaagccaaacagcgtgctgatccatccgccgactacggcaccgactatccccagcaggatagtcataaagaatccacctccatctttacctggcatgatccacttcgccagaataccggcaataagcccaaaaataatccatgacagaatgcccattgtttcctcacttatctgttttgcattagcgggttagtcgctgataaaaagcatagcacaacatcgggagggcaagatttgtgacgagcatcacggaggttttttttgcgatggcgcagaaattgcgccatcaacgatcagtgataattaccaaccacaaacatcatgttcgttttccgtgtcataagaacgtacggtattcaccagatcttttatcacttcagccgccacttctggcaccagcaaagtcatcggcgtctctgtttcataatcgacagaaacgccattgctgttattggtgacggtcacggtatacgttgctttgcccatgattcatttcccgttatgaatgactttccgttgttgcgcaccttccatcaggacttcaggagccacgaagaagtcaatgttgaaataagtatcgtcagtcatggcttcaatgttgtgccacttttctggagggaacaccgcaaactgccccgcttcgataaggatcacctgatcaggctctgcactgtgttcatcagcgtagccgagatatttgaccgccccatgcataacggaaaggcgtgggtaaacccccgggcgcgttcctttatcaagatgacgttcgaatattccggcaggtgcagtttgtttattccagaaaggcgttgagcgcgtatgaatataattctgtgggatttgaagcatccttttccctccttcggtgaatgcgctgaaaacggtttattccagccgtttcagggtacgcctgataatttgcattttaaataccatttattggttactttttagcaccatatcagcgaagaatcagggaggattatagatgggaagcccgcgacaacgcgggctgaaagcatcaggattgcagcgtcgccagtcgggcagcgaaacccacgaacatcaaaccaatcagtgagttgccaactttagccagtttctttttggtacgtatgtactgcgtgacaaaagcaccagatataatcaggaagctcaaatagcagaaactcaccagttccagcgtcgccgccagaataaagaatgaaattcccgtatgtggggcattaacatcgataaactgtacgaaaaacgacacatagaacaaaatggctttcggattagtcaggctcaaaattaacgcgcgtttaaaaatagcaccgtattggggctcatcggatttggcctcgctatttttacccttcagggtcgcgtaaagaattttactccccagatagagcaaataaaacgcaccaagataacgtacaatgttgaataatatcggggtggtcttaattaatgtcgccactccagcccatgccagaaacatcaataccgcatcgccaataaatacaccgcaggccgcaagataaccgcctttcataccgctactgacgctatttttgagtacaaacagggtatttggccctggcaccaacacaataaaaatggccccaaccagataggtccagtaattcagaaccccgtattcagcgaacacattaacctctttaattatctttcgatcatgcgcgattaaaggtgaatatgctaaccaatctgtagcggcttagaaaggagaaaatcaggttttaacctgatatcaacccgataattgaatcattaatcaggcatgctccagtgaaaaattcgggtagtgctcggcaaaatactggcgtaaaaattctaccgttatccgcactttcgctgacgtcgccagccttgaaacataaacggcccagacgttcgctggctggtaatattccggtagcacttgcactaaatgaccactggcaatgttttcgctaacatcccaccaggaacgcagagcaatcccctgcccatcgagacaccactgatggacaatttctccatgattagacgacagtgggccggtgactttaatcgcatgggggccttctttattgcgtaattgccagacaccaaaaggatgatcgcgctctttaatgaccaggcacggcaatgcagaaagatcggttaaatgtttcggcgcgccatgttgcgcaataaattccggcgacgcgcagagaatacggtaattggtcgccagtttgcgggcgattaaattaggggcgatgtcatcgccaatgcgaatatcgagatcgacaccttcattgaccaaatcgaccagtcggtcttccacatcaaaacgtaattccagttgcggatacgccttcgccagcgctaataacgccggagccaccacctgtcgtccaaaaccaaagctgctgataatacgcagcatcccctgcggcacctgacgcacgtcagaaagttcgtccatcatctgaccgacatcctgcaaaatccgctgcgcccattcataaatccgctctccttcttcggtaatggtgacgcggcgggtggtgcggtgtaacaacaccacgtttagcgtttgctccagcaaggcgatgcgcttgctgacgaacgccggtgaaacgcccagttcttccgccacggcggcaaaaccagcccggcgagccaccagcataaagacgcgcaaatcattcagcagcggtaaattattcatgattcgtgttttatgtttcaccagttacggggattaattccttttcagtcaattataggatggtgatgttgtcaattttgatggtcaggaagtgagaacccaatgatgaaaacgatgcgtattgctgcgatcccgggagacgggattggcaaagaagtccttcctgaagggattcgcgtgttacaggctgccgctgagcgctggggcttcgccttgagttttgagcaaatggagtgggcgagctgcgagtattacagccatcacggtaaaatgatgccggacgactggcatgagcaacttagccgtttcgacgccatctattttggtgccgtcggctggccggataccgttccggaccatatttcgttgtggggttcgctgctgaaatttcgtcgtgaattcgaccagtacgtcaacctgcgcccggttcgtctctttcctggcgttccctgcccgctggcgggaaaacagcctggcgacatcgatttttacgtggtcagggaaaacaccgaaggcgaatattcctcgctcggcggtagagtgaatgaaggtacagagcatgaagtcgtcattcaggaatcggtatttacccgccgtggtgtcgatcgcattttgcgttatgccttcgaacttgcgcaaagccgtccacgtaagacactaacttctgccactaaatcgaacggtttagccatcagcatgccgtactgggatgagcgagtggaagcaatggccgagaattacccggagatccgctgggacaagcagcatattgatattctctgcgcgcgttttgtgatgcagccggaacgattcgatgtggtggtggcgtccaatttgtttggcgatatcctttccgatcttggcccggcctgcaccggcaccattggcattgccccatccgccaacctgaatccggaacgcactttcccgtcgctcttcgagcctgtccacggttccgcgccggatatctacgggaaaaatattgctaaccctatcgccacgatttgggccggggcaatgatgctcgattttctcggcaatggcgatgagcgtttccagcaagcgcataacggtattctggcagcaattgaagaagtgattgctcacgggccgaaaacacctgatatgaaaggcaatgccaccacgccacaggttgccgacgcgatttgcaaaattattttgcgttaaggtcaaaccagtttatttgaaccgcgtcactgacgcggtttttttattcgttctttgcagtaaataacctgcgtcatttcaccttttattgtttccgtttcgtgttttatggctttccgtattcttaattgtttaatttatgtaacatgcaaattttgttacgcgtacgttaggttccgccgtacaggtattggttttgctggcaatgggactggtgatttatttagccaccagtaaatacggcaatattcgtcttggcgaaggaaaaccggaatacagcacgctctcctggctgtttatgtttatttgtgccggtttaggttcttctacgctttattggggggttgctgaatgggcctattattatcaaacacctggattaaatatcgcaccgcgttcacaacaggcactcgaatttagcgttccctactctttcttccactggggcatcagcgcctgggcaacttatacgctggcctcattaatcatggcttatcactttcatgtgcggaaaaacaaaggtctgagcctttccggcattattgctgctattaccggcgttcgcccgcaaggcccatggggaaaactggtcgatttgatgttcctgatcgccactgtcggcgcactgaccatttcccttgttgttaccgcagcaacctttacccgtgggctttccgcgctgaccggtttacccgataacttcaccgtgcaggcatttgtgatcctgctttccggcggcattttttgcctaagctcgtggattggtatcaacaacggtttgcaacgtctgagcaaaatggttggctggggcgcgttcctgctgccattactggtgctgattgtcggcccaaccgaatttattaccaacagcatcatcaatgccatcggcctgaccacgcaaaacttcctgcaaatgagcttattcaccgatccgcttggcgatggttcatttacccgcaactggaccgttttctactggctgtggtggatctcatacacccctggcgtagcaatgtttgtcacccgcgtttcccgcggtcgtaagattaaagaagttatctggggactgatcctcggcagcaccgtcggttgctggttcttctttggcgtaatggaaagctatgccattcatcagtttatcaatggcgtaatcaacgtcccacaggtgctggaaacactgggcggcgaaacagctgtacagcaagttctgatgtcgttgccagccggtaaattgttcctcgccgcatacctgggcgtgatgattattttccttgcctcgcatatggatgcagtggcctacaccatggcggcgaccagtacgcgtaatctccaggaaggtgacgatcctgaccgtgggctgcgtcttttctggtgcgtggtgatcactctgatcccgctttccatcttgtttaccggtgcttcgctggaaacgatgaaaaccaccgtcgtgctcacagcccttcccttcctcgtcattttactggtgaaagtcggcgggtttattcgctggctgaaacaggattacgccgacattccggctcatcaagttgaacattatctcccgcagacaccggttgaagccctggaaaaaacgccagtgctccctgcgggaaccgtattcaaaggcgacaactgagcgccatcatcctaacgataaaggtatccctatgagcaatctgagccctgactttgtactacccgaaaatttttgcgctaacccgcaagaggcgtggaccattcctgcccgtttttataccgatcagaacgcgtttgaacacgaaaaagagaacgtcttcgccaaaagctggatttgcgtcgctcacagcagcgaactggcgaatgccaatgattatgtgacgcgtgagatcattggcgaaagcatcgtgctggtacgcggtcgtgataaggttttgcgcgcgttctataacgtgtgtccgcaccgtggtcatcagttgttgagcggtgaaggaaaagcaaaaaatgtgattacctgcccgtatcacgcatgggcattcaaactcgatggcaacctggcccatgcacgtaactgcgaaaacgtcgccaatttcgatagcgacaaagcgcaactggttccggtgcgtctggaagaatatgccggattcgtcttcatcaacatggaccccaacgccaccagcgtagaagatcaattacccggcctgggcgcgaaagtgctggaagcctgcccggaagtccacgatctgaaactggcggcccgctttaccacccgcacgcctgccaactggaagaacattgtcgataactatctcgagtgctatcactgtggtccggcgcatccaggtttctccgactccgtacaggttgatcgttactggcacaccatgcacggtaactggacgctgcaatacggtttcgccaaaccgtccgaacagtcgtttaaatttgaagagggtacggatgcggcattccacggtttctggctgtggccgtgcacgatgctgaacgtcaccccgatcaaagggatgatgacggtcatttatgaattcccggtggattctgaaactaccctgcaaaactacgatatttacttcaccaatgaagagttaaccgacgagcaaaaatcgctgattgagtggtatcgcgatgtgttccgtccggaagatttacgtctggttgaaagcgtacagaaagggctgaaatcgcgtggctatcgtggtcaggggcgcatcatggccgacagtagcggtagtggcatttccgaacatggtatcgcccatttccataatctgctggcgcaggtgtttaaggactaatgacatcggcggcggtattttccgccgctgggctgatttttgatggagtacagcaatgtcagactatcaaatgtttgaagtacaggtgagccaggttgaaccccttaccgaacaggtgaaacgcttcacgctggtggcaaccgatggcaaaccattacctgcgtttaccggaggaagtcacgtcattgtgcagatgagcgatggtgataaccagtacagcaatgcgtattcactactgagttcgccgcatgacacctcttgttatcagattgccgttcggctggaggaaaactcgcgcggcggttcccgctttttgcatcagcaggtaaaagtgggcgatcggttaacgatttcaacgcctaataacctgtttgcgctaattccctcagccagaaagcatctgtttatcgcgggcggtattggtatcacccctttcctgtcgcacatggcagagctgcaacacagcgacgtcgactggcagctacattactgctcgcgaaatccagaaagttgcgcatttcgtgatgagctagtccagcatccgcaggctgagaaagtccatttgcatcattcatcaaccggaacacgactggaattagcgcgattattggcggatatcgaacctggcacacacgtttatacctgtggccccgaggcgctaattgaagcggtaagaagtgaagctgcgcgtctggacatcgccgccgatacgctgcactttgagcaatttgctatcgaagacaaaaccggcgatgcatttaccctggtgcttgcccgttccggaaaagagtttgtggtgccggaagagatgactattttgcaggttattgaaaataataaagccgcgaaagtggaatgtttatgtcgtgaaggggtatgcggaacctgcgaaacagcaatactggaaggtgaagctgaccatcgggatcaatattttagcgatgaagagcgtgccagccagcaaagtatgttgatctgttgttcgcgtgcgaagggtaaacgcctggtgttggatttgtagtttgccgaagccggatgtggcgctgagcgcgcccagtccggcttcggaagattttactgcggatattcctgcaataaattgtgtaatgcttccgccatcagctcaccacgccagccggaaatcagctccggcaaattgttctgcggtttcagtttccagtgccagttcagcagttggttgatttgccgacgcgatgccagcaattcggcgctgatcttatgcgtttcgctcacgtcagtaatcagcgacttaatcgctttaaacgctttacgataacccggcatgtccatcaggttaagcatcggctgcggtaaggcatcttccggcaatgtctgcgctttttccaccagcgctagcagcgttttaccgtgaaagcggatttcgctaccggataaacccaggctgtccagttcgcctaaacttcccggcatataacgcgctaccgaccacaaatgctcttcacgcacgacaaagttcaccgccagatcgcgctctcgcgccttgcgcagtcgccagtcggctaacagttgcagacaggccagttggcgtgtgcgtaattgccaggcattggtgatatcacgccaggcatcttccggcgcaacgacttcctgacgacgcatttgcatcaggcggcattcatccagcgccgcaggtagccagccggaggcctccgtttctaccataagcttggcggtgatcggtaacagataccagacatccgccgctgcgtattcacactgacgttcggtcagcggtctggccagccagtcggtgcgcgattcactcttgtccagcgtaacgccggaatactcttccaccatggaagcgaaaccccatgacatcgggcgtccgcagaaggcagcaaggatttgcgtgtcaatcaagggttgtggtaattcgccaaagacattgaggaacacttccagatcttcactgcctgcatggagaaattttgtgatggacggatcgcgcaggatcgctttcagcggtgaccagtcggtgatcccgagtggatcgattagcgccagatgctcgccatcgaaaagttgaatcaaccccagctgcgggtaataagtgcgcgtacgaacaaattcagtatccagggctatcgccggaaaggcacggacggcttcacacaaagaagccagcgcatcgtccgtggtaatcatttggtaattcaaattgttttctctttagtgggcgtcaaaaaaaacgccggattaaccggcgtctgacgactgacttaacgctcaggctttattgtccactttgccgcgcgcttcgtcacgtaattctcgtcgcaaaatttttccgacgttagatttcggtaactcatcacgaaactccaccagcttcggtactttgtatcccgtgagctgacggcggcaaaaagtcaccagtgactcttcggtaagcgatggatcttttttcactacgaagattttcaccgcttcaccactggagccggaaggtacgccaacagccgcgacttcctgtacgccaggatgctgcatgacgacatcttcaatctcgttgggatagacgttaaaaccggaaaccagaatcatgtcttttttacgatcgacaatgcgcaggaatccttcttcatccattaccgcgatgtcgccggtgtgtaaccagccatttttgatgatttcatcggtagcatcgggacgctgccagtaacccagcatcacctgcggtcctttgacacaaagctcacccggttgacctggtggtacttcattatcatcatcatccaccagtttggcttccgtcgacggcaccggcaaaccgatgctaccactatgataatcaatatcatatgggttaacgctgaccagcggcgcacactcggtaaggccatagccttccagcagatactgtccggtcagtttcacccaacgctctgccaccacttgctgcactggcatcccaccgcctgcggaaagatgcagactggagaaatccagctgctggaactctttattgttcagcaacgcattgaacaaggtgttaacgcccgtgatagcggtaaacggatatttcgctaactcttttaccaaccctggaatatcgcgcgggttagtgataagcaggttctgcccacccagttcgataaacagcaggcagttaatggtcagggcaaaaatgtgatacagcggcagcgccgtcaccaccagctctttgcccggatgcaacagcggaccataggtcgcgttaacctgttccaggttcgccagcatattgcggtgagtcagcatcgcgcctttcgccacaccagtggtgccgccggtgtattgcagaaaagctaaatcttccggcaccagttcgggtttgacgtactgcatccggtagccgttatgcagtgcgctacgaaatgaaatggcatctggcagatggtatttcggcaccaaacgcttgatgtatttaacaacgaaattgactaccgtgccttttgccgtagatagctgatcgcccatacgggtcagaattacgtgctgaacggcggttttatcaaccactttttccagtgtgtgagcaaagttagacacgataacaatcgccgatgcgccgctatcgttaagctgatgctcaagctcacgcggggtatacaacgggttaacgtttacgacgatcatcccggcacgcaaaatgccaaacagcgccaccggatattgcaataaattaggcatcatcaacgcaacgcgatcgcctttcttcagccccaacccttgttgcaaataagcggcaaacgcgcgactgcgttcttccagcttgcggaaggtcattacctcccccatattcacaaacgcaggttgatcggcgtagcgcgcgaccgactgctcaaacatatctaccagagattgataacggtcagggttgatctccgtcggaacgtccgcgggataacggttaagccaaaccttcttcaattcttcacctctaaaatgcgtgttcgtcgtcatcgcaaccccaaatgatatacatgccgttaacataatattaactcatcataccagcttgataattacccaacgaaaaggttgcgaagcgcgtcactatttatttttatctttaccgtaagaatgcagaaacagcggaccagccgctgtttctttttctttaaaaacaagcaattattcagttacaactgtttgtactctcgcggggccgggattataccagccccatccgccgtagccatagggccagccacgaccgccataaaaccatggatcaatcggctgaggcggcataatcacctgctgggttaaatgccaacgtttgtaacccgttacttgcatcaccataaatttatagggcgtattgccgattttgccgtcaaccgcaccagtgattggcccgactaccgtaaccagttgtccacggaaatccaccgggtccagaaaaccgttcacatcggcataaatgcgaccgcgagaaggttctcccagcgtcggtctggctccgctgtccagcggtacggtagcaatttccaggcgagttttcccttgctggttttgtaccgcaaccactttgccaccaaagcgtgcctcctgaccaacgtacagctgcggcgcactcatcacccgaactaaatcttgttgcggcgtgggactgctgcctttaatggcgtccggcacagtgacacaaccgctcagcattagcgcaaacgtacctgccagtatgcctttgataacattcttttgaaccgccatggtgcgactcctttttttctcagggcatactcttaagattcattctttgcccggaagtttcttccatgcgacgttgttacgtaaataaaccggttcggcatgttccaccgccaccgttttaccctcagcaaacatctgacacgcaatcggcagcatatcttcagcagcaggcagtaacacttcgccatcgcgcaaaaccagcccgctctctttaccgagatccggccaagcttgccagcccgtccctaccgtcacccattcgccggaaagctgttgcattcgttcatggacgatttcgggtttgagtacggcttcggtttcttcaccgtgccagataccgttttcatcacgctgatattcggcccagtaaacttcgcccattcgcgcgtcaatggctgccagcacgcgggttgcgccgtttttgcgccacgccccttgcgccatcgtcattagcgtggagacgccaatcatcggtaattccgcgccaagcgccagcccttgcgcgatgccaataccaatgcgcacgccagtaaagctaccggggccgcgcccgtaagccagagcgttaatatcagtcagggaagttccgctggtggtcaggatatcctgcaccatcggtaagattcgttgagtatgttcacgagggcaaagctcaaaatgagcgttgacagtaccgtcgttccacagggcgacagagcaggcctctgtcgcggtatcgatagccagaattcgcatgggtcttcgtgcttagatcaataaaaaggcgcgcatcataccatactccgtaacaaattacctggaggatggtatcgcaaggaaacgaaccgcacgggcaatgtcacgggtgcgtggcgcgggcggcagactggcgagaaacgtcgcgccgtaaggacgcatcaccagccgattgtcacaaatcaccagcacgccacgatcgtcggcgtcgcgaatcagtcgccctaccccctgtttgagagtaatgacggcatctggtagttgcacttcatcgaacgggtcgccaccgcgcaaacgacaatcttccatgcgcgcttttaacagtggatcatccggcgaggtaaacggcaatttgtcgataattaccaatgacaatgtatcgccacgcacgtccaccccttcccagaaactgctggttgccacaagaagcgcattaccggcgctgacaaattgctgcaacagttgccctttgctggtttccccctgcaacaatacaggaagcgtcatggtagcgcggaactgctcggccagatcgcgcatcatggcgtgcgaggtacaaagcataaaacaacgaccgttgttagcttcgatgatcggtcgcagcattgccgctaactggcgagcagaacctggctggttggtttgcggcagattgcgcagcacacagagtaacgcctggcggctgtaatcaaatgggctgggcaacagcaacgactcggcctgttcgatgccaagccgcgaggtgaaatgatgcagatcgtcgttcaccgacagcgttgctgaggtgaagatccagctaccgggtttttgcgccattaactctttgaatttatccgccacgctgagcggcgtgagagccagagtaaaatggcgcgaagtgcattcgtaccagtagctgtagcccggctgattgatctcttttagccgcttcagccgtgtgcgatacaacgtggcgcgctcaaatgccgcatccagcaaggcggaacgccccagtgacagtttcgccacgtcataacaaagttccagggtgtcatcgagcagtaaaaatgcccgctgaatttgcggattagctaacagctcacgcaggttaccgcgataacctggctcaccgagttgcagacgaaaatcctgcgcactctgggcaagacgatcagcgcacttttgtaactgctgggtgtcttttaattcggtgcggtaggcgatggtgatgtcttttgccaggtcgagcagttgtcgactggagagtgactgaccaaaatactggctggcaatgtccggtagctggtgggcttcgtcgaagatcatgacgtccgcttccgggatcagttcgccaaatccactctctttaaccaccatatccgccagaaagagatgatggtttaccaccaccacatcggcgtccatcgcttttttacgtgctttgaccacaaagcaatctttatacatcgggcagtcgctgccaagacagttgtcgttggtgctggtgaccagcggccacgcctgtgaatcttccgccacgctgacgcaggtgctgatatcaccatcgactgtttgattagaccaggagcgcagcaggatcacatcgcttaagatttgtaccggcagatcgccccccgccagcgcctgctgttcgagacgttcgaggcagaggtagtttgagcgccctttcagcagcgccacgttgcccgtatatttcaatgcctttgagactgttggcaaatcgcggctgtagagctgatcctgcaacgcttttgagccggtcgagataatgactttctttttcgcccgcagcgcaggagccaggtaagcgtaggttttgcccgtaccggttcctgcttccaccaccagcggctggcctttttctatcgcctgggtgacggctaccgccatctgtcgctgtggttctcgcggcttaaagcctggtatcgctttcgccagctgaccgtctggtgcaaaatcgtccgtcacactaccccctgttgatttgaacagggattatgtcaggatgagggcgctttcgccagttgaagtggtgacggcgacctcacattgtggcagtctttgcagcacgaaaatggaagtataatgaggacaaaatgatgactatcgttcgtatcgatgctgaagcccgctggtctgatgtagtaatccacaacaacacgctctactacactggtgtaccggaaaacctcgacgccgatgcctttgagcaaaccgccaacacgctggcacagattgacgccgtgctggaaaaacagggcagcaataaatcgagcattctggatgccaccattttcctggccgataaaaacgacttcgcggcgatgaataaagcgtgggatgcttgggttgtcgcgggtcatgcgccggtgcgctgcacggtacaagcgggtttgatgaacccgaagtataaagttgaaattaagattgtggctgcggtgtaagctttatcgaagcaaaataagtcagacgataatttatcgataatactggtcggttttacataaatcgaccagagaataagatattactgttgatgcttctgctaattcattatttatatttataatttcaattttatctataaaactaactatataaataaacataaacatgccgttgtgttcgccctttgattagcaactctggttttctttcttagctgaacaatctggttatagcgtgcggactgaccgttaaatttctccatcttactggataacacaccatgagctgctacctttaaaacacctgaatgtcaacaggttaactcgtgccatatcgttataatccctttgatattagatgcaaattaaggtcatatatagccttatcgataacatggttaattttaaggataagaatatgcctgctgtaatagataaagccctggatttcattggtgccatggatgtatcagcgccaacaccaagttcgatgaatgaaagcacggcgaagggaatctttaaatatttaaaagaactgggagtacccgcgagtgccgctgatattacggcgcgagctgaccaggaaggctggaaccctgggttcacggaaaaaatggttggatgggcaaaaaaaatggagacaggtgaacgttctgtgattaaaaatcctgaatacttttcaacatatatgcaggaagaactaaaagcactggtctgagttaaatttatatcagcataaatgggtcaggacgcttttaatcacatataaaaagcgtcctttttctcacaatcaaatgatcatcggcttctataacgaaatcgatacggattagtgtgttactcgtcttcatcctcaaaacgcgccacgattcgctcgccggagtggttggcacgcagctcttctgccaccagcgcgattgcctggccgctgctcatcccttgtgccatcagttcctggatccgctcgacagctttttgctgctgttcatgggtgagtgaaggtaaacctgcaaacattgttaactcctgctaaattgttggcgctaattatttcatgctacccggcacatagccagtagagtcaggactgatgaagacgttatctcccgctgtgattactttactctggcgtcaggacgccgctgaattttatttctcccgcttaagccacctgccgtgggcgatgcttttacactccggctatgccgatcatccgtatagccgctttgatattgtggtcgccgagccgatttgcactttaaccactttcggtaaagaaaccgttgttagtgaaagcgaaaaacgcacaacgaccactgatgacccgctacaggtgctccagcaggtgctggatcgcgcagacattcgcccaacgcataacgaagatttgccatttcagggcggcgcactggggttgtttggctacgatctgggccgccgttttgagtcactgccagaaattgcggaacaagatatcgttctgccggatatggcagtgggtatctacgattgggcgctcattgtcgaccaccagcgtcatacagtttctttgctgagtcataatgatgtcaatgcccgtcgggcctggctggaaagccagcaattctcgccgcaggaagatttcacgctcacttccgactggcaatccaatatgacccgcgagcagtacggcgaaaaatttcgccaggtacaggaatatctgcacagcggtgattgctatcaggtgaatctcgcccaacgttttcatgcgacctattctggcgatgaatggcaggcattccttcagcttaatcaggccaaccgcgcgccatttagcgcttttttacgtcttgaacagggtgcaattttaagcctttcgccagagcggtttattctttgtgataatagtgaaatccagacccgcccgattaaaggcacgctaccacgcctgcccgatcctcaggaagatagcaaacaagcagtaaaactggcgaactcagcgaaagatcgtgccgaaaatctgatgattgtcgatttaatgcgtaatgatatcggtcgtgttgccgtagcaggttcggtaaaagtaccagagctgttcgtggtggaacccttccctgccgtgcatcatctggtcagcaccataacggcgcaactaccagaacagttacacgccagcgatctgctgcgcgcagcttttcctggtggctcaataaccggggctccgaaagtacgggctatggaaattatcgacgaactggaaccgcagcgacgcaatgcctggtgcggcagcattggctatttgagcttttgcggcaacatggataccagtattactatccgcacgctgactgccattaacggacaaattttctgctctgcgggcggtggaattgtcgccgatagccaggaagaagcggaatatcaggaaacttttgataaagttaatcgtatcctgaagcaactggagaagtaagacgtggaataccgtagcctgacgcttgatgattttttatcgcgctttcaacttttgcgcccgcaaattaaccgggaaaccctaaatcatcgtcaggctgctgtgttaatccccatcgtccgtcgaccgcaaccggggttgttgctgactcagcgttcgattcatctgcgtaaacacgctggacaagtggcattccctggaggtgcagtcgatgacacggacgcatcagctatcgccgccgcgctgcgcgaagctgaagaagaggtcgctataccgccttccgccgttgaagttatcggcgtgctgccgcccgtcgatagcgtcactggctaccaggtaaccccagtggtcggcattatcccgcccgatctgccgtatcgcgccagtgaagatgaagtctcggcggtgtttgaaatgccgctcgcccaggcattacatctgggtcgttatcaccctttagatatctaccgccgtggtgattcacatcgggtatggctgtcctggtacgaacagtattttgtatggggaatgaccgcaggcataattcgtgagctggcgctgcaaattggtgtgaaaccctgactatacttatctttacatctacaaaacactacttgagacaatcatcgcaatattagttaaatcgcggtttttgattagtttaattcatgtgaatagttaagccagtcgccgcgttccctcttacactatgcgctgttattagttcgttactggaagtccagtcaccttgtcaggagtattatcgtgattagtctattcgacatgtttaaggtggggattggtccctcatcttcccataccgtagggcctatgaaggcaggtaaacagttcgtcgatgatctggtcgaaaaaggcttactggatagcgttactcgcgttgccgtggacgtttatggttcactgtcgctgacgggtaaaggccaccacaccgatatcgccattattatgggtcttgcaggtaacgaacctgccaccgtggatatcgacagtattcccggttttattcgcgacgtagaagagcgcgaacgtctgctgctggcacagggacggcatgaagtggatttcccgcgcgacaacgggatgcgttttcataacggcaacctgccgctgcatgaaaacggtatgcaaatccacgcctataacggcgatgaagtcgtctacagcaaaacttattattccatcggcggcggttttatcgtcgatgaagaacactttggtcaggatgctgccaacgaagtaagcgtgccgtatccgttcaaatctgccaccgaactgctcgcgtactgtaatgaaaccggctattcgctgtctggtctcgctatgcagaacgaactggcgctgcacagcaagaaagagatcgacgagtatttcgcgcatgtctggcaaaccatgcaggcatgtatcgatcgcgggatgaacaccgaaggtgtactgccaggcccgctgcgcgtgccacgtcgtgcgtctgccctgcgccggatgctggtttccagcgataaactgtctaacgatccgatgaatgtcattgactgggtaaacatgtttgcgctggcagttaacgaagaaaacgccgccggtggtcgtgtggtaactgcgccaaccaacggtgcctgcggtatcgttccggcagtgctggcttactatgaccactttattgaatcggtcagcccggacatctatacccgttactttatggcagcgggcgcgattggtgcattgtataaaatgaacgcctctatttccggtgcggaagttggttgccagggcgaagtgggtgttgcctgttcaatggctgctgcgggtcttgcagaactgctgggcggtagcccggaacaggtttgcgtggcggcggaaattggcatggaacacaaccttggtttaacctgcgacccggttgcagggcaggttcaggtgccgtgcattgagcgtaatgccattgcctctgtgaaggcgattaacgccgcgcggatggctctgcgccgcaccagtgcaccgcgcgtctcgctggataaggtcatcgaaacgatgtacgaaaccggtaaggacatgaacgccaaataccgcgaaacctcacgcggtggtctggcaatcaaagtccagtgtgactaatacttcttactcgcccatctgcaacggatgggcgaatttatacccgctttctcgtctgctgtaatattccccactacacttccactgttgcgtcaggcgtttgtcgccatacgcttacagggtggcccgcatgcaaaaagcacaacggatcattaaaacctatcgtcgtaatcgaatgattgtttgtacgatttgcgcactcgttacgctcgcttcgaccctgagcgtgcgatttatttcacagcgtaacttaaatcaacaacgggtagtacaattcgccaatcacgctgtagaggaattagataaagtactgcttcccctacaggcaggtagcgaagtcttgcttccgctgattggtctgccctgctctgtcgcccatttgccattacgtaaacaggcggcaaaactccaaactgtgcgatccattggcctggtgcaagacggcacactttattgctccagcatttttggttatcgcaatgtgcccgtcgtggacattctggctgaacttcctgcaccgcaaccacttttacgcctgacgatcgaccgtgccctgattaaaggcagtccggttttgattcaatggacgcctgcagcgggcagtagcaatgctggggtcatggagatgattaacatcgacttactgacggcaatgctgcttgagccacaactgccgcaaatcagtagcgccagcctgacggtggacaaacggcatttgctctatggtaatgggctggtagattcccttccgcaacctgaagacaatgaaaactatcaggtttcttcgcaacgctttccttttaccattaacgttaatggtccgggggctacggcgctggcatggcactatcttccaacacaattaccgctggcggtgctgctaagtttactggtgggctacatcgcctggctggcgaccgcttaccgaatgagcttttcccgcgaaatcaatctgggcctggcgcaacatgagttcgaattgttctgtcagcctttgcttaatgcgcgcagccagcaatgtattggtgtagagattttgctgcgctggaacaatccgcgtcagggctggatttcaccggatgtgtttattcctatcgcggaagaacatcatttaattgtgccactgacccgctatgtgatggcagaaaccattcgtcagcgccatgttttcccgatgagtagtcagtttcatgttggcattaacgtcgcacccagccattttcgccgtggtgtgctgataaaagatctcaatcagtactggtttagcgctcacccgattcagcaactgatcctcgaaatcaccgaacgcgatgccttactggatgttgattatcggattgcccgcgagctgcatcgtaaaaacgtcaaactggcgattgatgacttcggcaccggcaacagctcgttttcctggcttgaaacattacgtcctgacgtgctgaaaattgataagtcatttaccgcagctataggttctgacgcggttaactcgacggtgaccgatatcatcatcgcgctggggcaaagactgaatattgaactggtggcggagggcgtggaaacgcaagaacaggcgaagtatttgcgccgtcatggcgtgcatattttgcaagggtatttgtacgcacagccgatgccgctacgtgattttcccaaatggctggcgggcagccaaccgccgcccgcccggcataatggacatatcacgcccattatgccgttacgttaacgcttactcatcttcatcgtgcgccggttgctctttaacaatgcgaaccagatcaacacgataatcattggcttcaatgatggtgatatgcagtggccctacatcaatcacatcgcccacacggggaatgtgaccatttgccgagatcacgaggcccgcgaccgtcgcgatatcatcgtcatcggcaaggtgctcaacatcaagcgcctgctgcaaggcatgcaaatctgtaccgccttttaccagccagccgtcaccatcagtaatgatttccggcgtttcgtcagcgtccgggaattcacccgcaatggcttccagcacatccagcggcgtgaccagaccttgtaccacaccaaactcgttggtcacgataacaaagctcccgcgagcacgacgcagcacgcccaacaggttgatcggatcgagggtttccgggacgataatcgccggagacgccgaagcaatcgccgccacatcaacgccctcttccagcgccaccagcagttctttagcacgtacaataccgatgatttcatccagttcaccgcgacataccgggaacagactgtgcggtgaagagagcagttgctcgcggatttcatcgaccccgagattagcgtcaacccagcttatttcaccgcgcggcgtcatgatcccgcgcagagaacgcgacgccagcgtcagtacgccgttaatcatgtaacgttcttcttcggcaaatgcaccttccgggatcggcatcggcatcgggttatcggcatcgtgctgaacattggcctgacgtttcccgcccatcaaacgcaggatggcatcggcagtacgcgctcgcagcggcaaagtcgactggtggcgaataaagttgcgacgcgcaatctggttaaacacttcgatgatgatcgagaagccaatcgcggcatacaggtaacctttcggaatgtggaaaccgaaaccttctgccaccagactcagaccaatcattaacaggaagctcagacagagcaccaccaccgtggggtgctggttaacgaatcgcgtcagcggtttggatgccagcaacataaccgccatcgcaatcactaccgccgccatcatcaccggcagatggttaaccatccctactgcagtaattaccgcatccaacgagaagacggcgtcaaggatgacaatctgtgtgacgaccacccagaaactggcgtagcctttaccgtggccggaatcatgatcgcggttttccagccgttcatgcagttcggttgttgctttgaacagcaagaatatccccccgaacaacataatcaggtcgcgtccggagaaggagaaatccatgacggtaaatagcggtttggtcagcgtgaccatccatgaaatcagcgacagcagccccagacgcataatcagcgccagtgataaccccagcaaacgcgctttatcgcgttgttttggcggcagtttgtcagcaagaatggcgatgaagaccaggttatcgatacccagcacaatttcgagaacaacaagcgtgagtagccccgcccaaattgaggggtccattaagaattccatgacaagctcctgcttaaggaatagctattcgacgccagaaataatgcaggcgtaacgacaaaatgcaaacgaaaggtgcggcatagagtgccagaaaggcaggcgttaaaaggcctgatgctgaaatgacgtcggtgacgatccatactgcgggctactgccctatactccatggttgttaaacgggagttaaacatatcagagacgcctctgatttggcaaagatttaccttcctttgcaaacgaatgtgacaaggatattttacctttcgaaatttctgctaatcgaaagttaaattacggatcttcatcacataaaataattttttcgatatctaaaataaatcgcgaaacgcaggggtttttggttgtagcccttatctgaatcgattcgattgtggacgacgattcaaaaatacatctggcacgttgaggtgttaacgataataaaggaggtagcaagtgaccattgctattgttataggcacacatggttgggctgcagagcagttgcttaaaacggcagaaatgctgttaggcgagcaggaaaacgtcggctggatcgatttcgttccaggtgaaaatgccgaaacgctgattgaaaagtacaacgctcagttggcaaaactcgacaccactaaaggcgtgctgtttctcgttgatacatggggaggcagcccgttcaatgctgccagccgcattgtcgtcgacaaagagcattatgaagtcattgcaggcgttaacattccaatgctcgtggaaacgttaatggcccgtgatgatgacccaagctttgatgaactggtggcactggcagtagaaacaggccgtgaaggcgtgaaagcactgaaagccaaaccggttgaaaaagccgcgccagcacccgctgccgcagcaccaaaagcggctccaactccggcaaaaccaatggggccaaacgactacatggttattggccttgcgcgtatcgacgaccgtctgattcacggtcaggtcgccacccgctggaccaaagaaaccaatgtctcccgtattattgttgttagtgatgaagtggctgcggataccgttcgtaagacactgctcacccaggttgcacctccgggcgtaacagcacacgtagttgatgttgccaaaatgattcgcgtctacaacaacccgaaatatgctggcgaacgcgtaatgctgttatttaccaacccaacagatgtagagcgtctcgttgaaggcggcgtgaaaatcacctctgttaacgtcggtggtatggcattccgtcagggtaaaacccaggtgaataacgcggtttcggttgatgaaaaagatatcgaggcgttcaagaaactgaatgcgcgcggtattgagctggaagtccgtaaggtttccaccgatccgaaactgaaaatgatggatctgatcagcaaaatcgataagtaacgtattgtgttgattatcactcagttttcacacttaagtcttacgtaaacaggagaagtacaatggagattaccactcttcaaattgtgctggtatttatcgtagcctgtatcgcaggtatgggatcaatcctcgatgaatttcagtttcaccgtccgctaatcgcgtgtaccctggtgggtatcgttcttggggatatgaaaaccggtattattatcggtggtacgctggaaatgatcgcgctgggctggatgaacatcggtgctgcagttgcgcctgacgccgctctggcttctatcatttctaccattctggttatcgcaggtcatcagagcattggtgcaggtatcgcactggcaatccctctggccgctgcgggccaggtactgaccatcatcgttcgtactattaccgttgctttccagcacgctgcggataaggctgctgataacggcaacctgacagcgatttcctggatccacgtttcttctctgttcctgcaagcaatgcgtgtggctattccggccgtcatcgttgcgctgtctgttggtaccagcgaagtacagaacatgctgaatgcgattccggaagtggtgaccaatggtctgaatatcgccggtggcatgatcgtggtggttggttatgcgatggttatcaacatgatgcgtgctggctacctgatgccgttcttctacctcggcttcgtaaccgcagcattcaccaactttaacctggttgctctgggtgtgattggtactgttatggcagtgctctacatccaacttagcccgaaatacaaccgcgtagccggtgcgcctgctcaggcagctggtaacaacgatctcgataacgaactggactaacaggtgagcgaaatggttgatacaactcaaactaccaccgagaaaaaactcactcaaagtgatattcgtggcgtcttcctgcgttctaacctcttccagggttcatggaacttcgaacgtatgcaggcactgggtttctgcttctctatggtaccggcaattcgtcgcctctaccctgagaacaacgaagctcgtaaacaagctattcgccgtcacctggagttctttaacacccagccgttcgtggctgcgccgattctcggcgtaaccctggcgctggaagaacagcgtgctaatggcgcagagatcgacgacggtgctatcaacggtatcaaagtcggtttgatggggccactggctggtgtaggcgacccgatcttctggggaaccgtacgtccggtatttgcagcactgggtgccggtatcgcgatgagcggcagcctgttaggtccgctgctgttcttcatcctgtttaacctggtgcgtctggcaacccgttactacggcgtagcgtatggttactccaaaggtatcgatatcgttaaagatatgggtggtggcttcctgcaaaaactgacggaaggggcgtctatcctcggcctgtttgtcatgggggcattggttaacaagtggacacatgtcaacatcccgctggttgtctctcgcattactgaccagacgggcaaagaacacgttactactgtccagactattctggaccagttaatgccaggcctggtaccactgctgctgacctttgcttgtatgtggctactgcgcaaaaaagttaacccgctgtggatcatcgttggcttcttcgtcatcggtatcgctggttacgcttgcggcctgctgggactgtaagactgttgtacactaccggggccttttggccccgtttttttatctggaggattaatgacaatcacggacctggtactgattcttttcatcgccgcactcctggccttcgcgatctacgatcagttcatcatgccccgccgtaacggccccaccctgctggcaattcctttgctccggcgtggtcgcatcgatagcgttatcttcgtcggattgattgtcattcttatctataacaacgtcacgaatcatggtgcgttaataacgacatggttattaagcgcactggctctgatgggtttttatatattctggatccgcgttccgaagatcatctttaaacaaaaaggttttttcttcgccaatgtctggattgaatatagccgaatcaaagcgatgaacttgtcggaagatggcgtgttggtgatgcaattagaacagcgtcggctgttaatccgcgttcgaaatatcgacgatctggaaaaaatttataagcttctcgtttcaactcaataagttatgaatttagccaaagctatgtttagtgtatttttaataatcagacatagcttaggctatattacctcttcccttatttgttatttattttaacgtttcattgatatataaatccaaatgaaaatcgttatcaataaagcaatgaaataatatattccaacagttgttttatattctcaaaatatgttaaggttgcgccctcatttggggagtagccgatttccagattccggaaatgtacgtgtcaacatactcgttgcaaaacgtggcacgtacggactgaatactttcagtcaggcgagaccatatgcacatcaatcgctatgcctgcatgaacgcgaaaaccatcacggcttgttgttcatgtatgcatgtttgctgggggcgatgatgtgttttatggataccccggtcaggacattgtcatgaatatcactgctactgttcttcttgcgtttggtatgtcgatggatgcatttgctgcatcaatcggtaaaggtgccaccctccataaaccgaaattttctgaagcattgcgaaccggccttatttttggtgccgtcgaaaccctgacgccgctgatcggctggggaatgggcatgttagccagccggtttgtccttgaatggaaccactggattgcgtttgtgctgctgatattcctcggcgggcgaatgattattgagggttttcgtggcgcagatgatgaagatgaagagccgcgccgtcgacacggtttctggctactggtaaccaccgcgattgccaccagcctggatgccatggctgtgggtgttggtcttgctttcctgcaggtcaacattatcgcgaccgcattggccattggttgtgcaaccttgattatgtcaacattagggatgatggttggtcgctttatcggctcaattattgggaaaaaagcggaaattctcggcgggctggtgctgatcggcatcggcgtccagatcctctggacgcacttccacggttaataagaacgctgccagaggtgaatattaaagtccgtctggcagtcgaacacttcttttgctgccagtgtttgccagacttctggcttcgcacgccaggcaaacggcgtcatctgcaataatgcgacggcttcatcaccgcgaagacgcatcggataacacaactccgcactctgctgtaatgtaaaaccttccagttgttctgcatgaggtgcatgaagatgtacttcattgtaaatcagccccttcagctccatcaaatgtcgcggtcccggcgtggcagtaatgacccagccgccgggcttcactactcgtgctaattcttctgctttacacggcgcgtaaatacgtattatggcgtccatactggtatcggaaaacggcaaacggtggctggaagcgacacaaaaagtgacctgcggatagcgtttcgccgccgcttttatcgctaccttcgaaacatccagaccaaacgtggtgatttcgggcaacgcatcggcaaatgcgtgtgtgtaatacccttcaccacagccaatatccagcaccgccgtggccttatcatcaagccgttccctcagttgggcgacaattgcatcacgcagcggctgataatgtccggcatctaagaatgcgcggcgtgcttgcatcatttccgcgctgtcgcccggatcacgagaccgtttatgctgaacgggcagcagattgacatacccttctttcgccatatcaaactgatgtcgctggggacagatatagctgtttttttcacgcgaaagaggctgatggcaaagtggacaggaaaaagacatgacaactccggcaggatactaaaggccgcaagtgtaacgcgaatcacgcggcgggcaaatatccgaacgccaggagcgaagataaagcatagtaaaaagcctcgcattcgacgaggctttatagcgagattgaagcgtattcacacttcagatcagtggattcgatcagatagctgttacgttaacagctgccggacctttctggccgtcctgaatttcgaactcaacgttctgaccttcagccagagttttgaagccattaccctggatagcggagaagtgtacgaacacatctttgctgccatcagccggagtaatgaagccaaaacctttagactcgttgaaccacttaacctgacctttaatctttgccatttgaaaaattccttagattgttttcttcgcccgcaggcataacatagataaaactgacacattactgcatgaggcaccaatataaggctcggcagagaagcggtattcaacgtcaacgtgtttactcaggacttctttactgaaaatgccacacataaacagaactgtacctcgtttaacccgaaatctgttatcacatacaacgttaattatggcaagccatttttaaacatgtctcgatcagacgcacaaatctcgatacgtcttccactttttttgcacacttatgcaacggaatacgcgccgatatatcattgtgcttaaccttgccagttcaggcagatacttaaactggcgtattttctaacatagttcaataagttcagttgttccaggccagtgggagaagttattacatagtgcgtgcaatatcacattttttgctatgcaatgaataaaaagttatatcactttttctcataaaacagtcagttaacggctattaattaccctaaagagaagtcaatccccaaagggattgtaaatttaaaataagaaaaattgatgaatgagcaaaaaaatcaagagagaaacgtttcgctaataaataataccacgcttaatcacaaatccgatgtaaacatcctaataaattaatggggtaaatatctttttctgatatcccgttacgcaaataaataatatgataattatttgaagtcagaccagagttttaatttgaagcagttgcaccatgacagtgcgtataatcaggatgaattgagtaacccttcaacgacggggttactcaagattgaggaaggattatcgttcggcgaccagacgaataatatcttcgtcttcaaccgatttttgactctcaacggtctttttatctgctttctctggttcgtttgcttcgcacaaacgacgtaacagtgcattttgacgtttttgctgatccagcaacgcctcaagcagttcaatctgttcgttagtccgtgaactggcacgattgataaaaaaccacaagatgagcccgataagaagaaccaccaccgatacaaccaaagacgcaatgttcatcacgcctgaatttacaacttcgttcatttcaccacctctgagtagaggcgctattctaccactgctggagaggaagaaaatctagtgctgaaaaaatgatatcaccacgggataaactggttaatggcacaaattccgctgaaaaattgtacatcctgatcgcacatcatgttgaatacctgcgcccaaagcagcaagcaagccaacaccacgacaaccagaacgacccatcgaaactttttcactccaatctccgtttcacctaccttatgtcattaaactagcatgcgttagttaaacagcgcctaactatgtcgatattcgtgctttttcggaatgagtcgcttgcttcagcgcatattgccgctacgattaagcgaacataaaaagagaagaggttgtaatgcgattcatcattcgcacagttatgctgatagcactggtatggataggattattactcagcggatatggcgttttgattggaagcaaagagaatgccgcaggattaggtttgcaatgtacctatctgactgccagaggcaccagcacggtacaatacttgcacactaaaagtggttttttggggataacagattgcccgctgttacgcaaaagcaatatcgtggtcgataatggttaagggcaataaataaccagattctcactcctgagtaaaatactcttatagcaagcgcgtttaatataacgccaccttcaactttatttttctcatgctaaataaagaacctgtctgtttgatattccgacaggttcttactctcatcagaacggatagtcgtgataacccatttgggcagaaattttgcgcgctgcggtatgcaacattgcgacatattcctgtaaacgctcttcagagaaacgcaacgtcgggaaggagatgctcaaaccggcaatgaccacgccaaagcgatcaaataccggtaccgcaatgcatcgcagcccttcttcctgctcttcattatcttcgccatacccctgctcgcgcacctggtccagaacgggtaataacgcttctgtactggtgatggtccgctcggtactgcgtttatactccacgccctcaagaatttgcttcacttcatcgcgatcgcgccatgccagcagtaccttaccaatcgcggtgctgtacagcggattacgacgcccaatccgtgaatacatgcgcaaattgtacatagagtcaattttgtgaatgtaaacaatactgtcttcgtccagtgcgccgaggtggatagtttctttggtcaggcgggagagctcacgcatctggatatctgcgctacgaattaaatcgacgttttgtaacgcgcgagcgcccagttcaaacaatttcagggtcagggaatatttctccgactccccttcctgcgccacataacctaaggttttcatggtctgtaaaaagcgataaacggtgctttttgacatcatgacgcgctgcgacagctcggttatccctatttcgcgctcttcacccagcgcctgcaaaatgccaaaaacttttagcacggaagatacagaatcaggctgtttatccagatctgcgttagccatttatcacctcattgcgagtgttttataaaaatcagaactgttttttattataatttcgcaccagggtggtcgcaatccatcttttgccggttagttacaattctgcgacatccaccgtgaatatcagtgctagaatcatacccctgttgattattcaccaaagatataaaattcctatgccaaaagttcaggccgacggcctgccattgccccagcgatacggtgcgatattaaccattgtgattggtatttcgatggccgtccttgacggcgcaatcgccaacgtcgccctgccaacaatcgccacggaccttcatgccacgccagccagttccatctgggtagtgaacgcctatcaaatcgccattgtcatctccctgctctcgttttcgtttctgggcgatatgtttggctatcgacgtatttataaatgcggtctggtcgtttttctgttgtcttcactgttctgcgccctttctgattcgctgcaaatgctcacccttgcgcgtgtcatacaaggtttcggcggtgcagcgttgatgagcgttaataccgcacttatccgcctgatctatccacaacgttttctgggtagagggatgggcataaactcgtttattgttgccgtctcttctgctgccgggccgacaattgctgcagcaatcctctccatcgcatcctggaaatggttatttttaatcaacgtaccgttaggtattatcgccctgcttctggcgatgcgttttctgccacccaatggttctcgcgccagtaaaccccgtttcgacctgcccagcgccgtgatgaacgcgttaaccttcggcctgcttatcactgcgttgagtggtttcgctcaggggcaatcgctgacgttaattgctgcggaactggtggtaatggttgttgttggtattttctttattcgccgccagctttctcttcccgtaccgctgctaccggtggatttactgcgtatcccgctgttttcactttctatttgcacatctgtttgctctttctgcgcacaaatgctggcaatggtttccctgcccttttacctgcaaaccgtgctcgggcgtagtgaagtcgaaacaggtttacttctgacaccgtggccgttagcaacgatggtgatggctccgctggcaggctatttgattgaacgcgtacatgcaggattgctgggggctttagggttgttcatcatggctgcggggcttttttccctggttctgctgcccgcgtcacctgcggatatcaatattatctggccgatgatcttatgtggtgctggatttggcttattccagtcacccaataaccacaccattattacctccgcgcctcgcgaacgtagcggtggagccagtggcatgttaggaacggctcgtctactgggtcagagtagcggcgcggcgctggtggcgctgatgctaaatcagtttggagataatggtacacacgtctcgctgatggctgcggctattctggcagtgattgctgcctgtgtcagtggtttacgtatcactcagccacgatccagggcataaaaaaagcgcgtcgatcaggacgcgctttttagtatttacttcatattacttcaggtattcacccgtacgcagagcttcaattcgtttatccagcggcgggtgggtcatgaacaactcactgagcgatttcgacttaccgttaatgcagagagccatcatgctggttgcttcttgcggttcatagctggttttcaggcgctgcagcgcggcaatcattttctcgcgaccaaccagttttgccgaaccggcatcagcatggaattcacgatgacgcgagaaccacatggtgataatgctcgccagaataccaaacaccagttccagaaccgttgcaaccgcaaagtagatcagcgggttgccgttgctctcttcaccttcatcacgatttccgcccataaaacccgcggcaagctgcgccagaatacgggaaataaagataacgaaggtgttcaccacgccctgaatcagcgtcatggtgaccatatcaccattggcgatgtggctgatttcgtgagcaattaccgcctcggcttcatccgggctcatgttctgcagcaaaccggtgctgacagcaaccagagaggcatcacggcgcgcaccggttgcaaaagcgttgatgtccggcgcatggtagatagccacttgcggcatagcgatccccgcctgacgagcctgggttgctacagtattgaccagccaacgttccctttcgttacgcggttgctcgatcacttccccgccaacagatcgtaatgccatccatttggacatcagaagcgaaacgaaggaaccaccaaaaccgaacagcaaggccatgatcatcagcccctgaacgctgctcgactgtatccctgtcaggctcagtaccagcccgaaaacgaccattacggccaggttcgttagcaggaagagcgcgattcgcatcataattttctttttacctcagtttaacaaaacgcaatatgcgatacccacatcgtatgggttacgcgactattttcaagtctggatagtgcgtaagtcaccagaaagacacaactttacattttgtagcatctgatttacggcatcttgtcgctgttaaaaaatcaggcacaatttcttgtgcctgattgatattacttgacgggagcgggttgttccgcgggtctggctttttcaagcttcgccagatcgagtgcgatattcaccgtctcatccagataaggatccggctcctggtaatctttcggtagatcatccagtttcttcaactccggtttaccttcgcgtttaaagcgttcgttcaaacgcgccagacgcgtcgcatcatcttcattattctctttctcacgcacagcgtaattcagagaaacgatattgcgcttgtccttcatagcgttgaagcgcgcgatatccttcatgatgttctggaactcaggatctttcgcgatacgcgcattatgttccttcagcagctccggttcaaaggccgttaaatctcctgatttcacataagtcgcggcatcaatgctatcccacggcagcgcgttatcttcgaatttctcacccgtttccgtttcttcattacccgtcggcatgatgatgtctggcgttacgcctttacgttgcgtactgccgccgttaacgcgatagaatttctggatcgtgtactgcacagaacccagcgctggccattcaggacgtaacatctgatcgtaaatacggttcaatgaacggtattgctgaacggtgcctttaccaaacgtcggttcacccacaaccagcgcacgaccgtaatcctgcattgccgcggcaaagatttctgaagccgaagcactgaagcggtcaaccagcaccaccagcgggcctttatagaaaacctgtccgtcggtatcgctatcttcacgaaccttgccgttgttatcgcggacctgaacaatgggacccgcaggaataaacagaccggagagcgatacggcttcagttaacgccccaccgccattgctacgcaggtcgatgatgacgctgctgacattctgtttttccagtttctgcagttgcactttgacatcgtctgtcaaacccacatagaagcccggaatatccagcacgccgactttctctttaccgacggtcttcaccgacattttaaccgcgcggtcttcgagacgaatacgttcacgggtcaacgttacagtacgggtcttggtccctttaccagcaggtaaaatttccagacgaactttactgcccttcggccctttaattaaggcaaccacatcatcaagacgccagccaatcacgtcaaccatcggcttgcctgtttgaccaacaccgacaattttgtcaccaacgctgatagctttactcttcgctgccggaccacctgccaccatcgaattgataacggtgtagtcatcatccatttgcagcactgcgccaataccttccagcgacaaactcatttcagtgttgaactgttcggtattacgcggggaaagatagttggtatgcgggtcgatttcacgcgcaaacgccgtcattgccagcgagaaaacatcttcgctgttggtttgcgccagacgacgaatggcaaatttgtagcggcgagtcagggtttcacgaatttctttatccgtttttcctgtcagcttcaggcttaactcgtcgaatttgactttactgtcccacagcgcgttcaactcagcctcgtttttcggccagggcgctttgctgcggtcaaggttataagtgtcgttgccggtgaaatccatcggcttttccagtaccgacaaagcgtactggtaacgctcaaaacggcgcttttgcgccagattgtagagatcgtagaaaacgtcgagtttgcctgaacgcagttcatcgcctaactcggttttctttttcgcgaactgttcaacatcgcttgccagcagcacgttgtggctgtaatcgagcagattcaggtagcggtcaaagattttggccgaaaatgcctgatcgaggtcgaactggcgataatgagaacgggtgaagcgcgacgttacgcgctcacttaccgtcgcatgctgcgtctcttcctttaataccggaatttgatcagcacgcgtgatatcttctacagcgaaggtctggcctgctattgcaagcaggccagctaacgcggtaagcctaaaaaacatgttcatgcctggcccggcctccgtttcagaacaccaggtgttctgcgcgcacaatcaaagacatacccgaattcagctggacgcggacgccgtctttggtgatttctaatacggtggcatccatcgcgttttgacccgctttcaccttcagggcttgtccgacagtcagagctgaaatgtcagaaaccggggtgtgctgttcttcgcgaggtgcttttactgtttttggcgctttctctaccggcttttgcgcacgaggtttacgttcagcgccttctttgcggcgtggcgtagtcggacgtggcttgcgttcgcggcgcggtgcgtcttctttctcaccagcagttgcggcagcttcgcgttttttcgcttgctgttcagcacgctgtgcctgaacacgcgctttcgcttcttcaagctgcttgcgagcatgctctacatgttgctcgtccagctcaccgcatgggttgccgtcaagatcgacacgcgttgcgccgggtttaacaccgtaaagataacgccagctcgaagtgtagagacgtaaagcggatcgcaattgcgttttgctcaggttcatttccccagcaacacgatcgaccaaatcctgaaaaataccgattttcagcggacgcgcttcaccttccgcactgaaacagtggggaaaacgttcggccagaaacgcgattacttctttactgctattcaacttaggttgattttccatgaaatttcctgattacaacggacgtagccaacaagcgcaggcatgaacaggcgtcattataatgacgctatcagtaaatgctacgttatccgttgattatcctgcgacgctcgcaaagaattttttgtaatccgtcgttgcaagcactttttcaagctgtgccacaagctgacgtaagccttgctcgtcctcgtctgtaaagcgaccgaagacggtactatcgatgtcgagaacaccaataatctgatttttcaccaccagcggcagaacaatttcagaattactcgccgcatcacaggcaatatgcccgtcaaacacatgaacatcctcgatacgctgcacttgattgcgggcaaccgcagtgccgcacacgccgcgcccgacgggtatccggacacaggcaattttgccctgaaatggtccgagtaccagtgtatcgtcctcaagcaaataaaaacctgcccagtttatgtcagtgagacgctcatataacaacgcactggtgttcgcaagcgttgccagaaaactggtttctcccgccatcagcgcgttaaagtcgcgatttaaatccgcgtaaaattctgttttgttcattatataatcacttggttgtcttacctggatctgccagcctattaaaataagcattaaatgcgttaatgctcaagatcattcccatcatgggttaagattaatgttaattcttattacatttggcacgtcatggctcttaacacaccacaaattacgccgacaaaaaagataacagtgagggcaatcggcgaggaactgccgcgtggtgattaccaacgttgcccgcaatgtgacatgctgtttagcctgcccgagataaattctcatcaaagtgcctattgtccgcgctgtcaggcaaaaattcgtgacgggcgcgactggtcgctaacgcgcctggcggcaatggccttcaccatgctgttgcttatgccgtttgcctggggcgaaccgctgttgcatatctggctgttaggcattcgtattgacgccaacgttatgcaaggcatctggcaaatgaccaaacagggcgatgcgataacggggtcgatggtctttttctgcgttattggtgccccgctcattctggtgacctccatagcttatttatggtttggtaaccgactgggaatgaatttacgtccggtactgctgatgcttgagcgacttaaagagtgggtaatgctcgatatctacctggtcggcattggcgttgcttctataaaggtacaggattatgcccatatccaggctggtgtcggcttgttctcttttgtggcgttggtgattttaacgacggtgacgttgtcacatcttaatgtcgaagaactgtgggagcgattttatccgcagcgccccgctacgcgtagggacgagaaacttcgtgtctgtcttgggtgccattttaccggctatccagatcagcgtggtcgctgcccgcgttgccatatcccgctacgcctgcgtcgccgtcatagtctgcaaaaatgctgggcggcgctgttagcgtcaatcgttttattgttacctgccaacctgttgcctatttctatcatttatctgaacggaggacggcaggaagatacaattctttccggaattatgtcgctggcaagtagcaacattgcggttgcaggaatcgtgtttatcgccagtattctggtaccgtttactaaagtgatcgtcatgttcactttactgttgagcattcattttaaatgccagcaaggtttacgcacacgcattctgttactgcggatggtgacctggattggtcgctggtcgatgctcgacctgtttgtcatatctttaaccatgtcgctgattaatcgcgatcagatcctcgcttttactatgggaccggctgcgttttatttcggcgcagcggtaattttgactattcttgctgtggaatggctggacagccgcttactttgggatgcacatgagtcaggaaacgcccgcttcgacgactgaagcgcagattaaaaataaacgccgtatctcacctttctggctgctgccgttcatcgcgctaatgattgccagttggctgatttgggacagttatcaggaccggggtaataccgtcaccatcgactttatgtcggcggatggtattgttccaggccgtacgcctgttcgttatcagggcgttgaagtcggaacagtgcaggatatcagcctcagcgacgatcttcgtaagattgaagtcaaggtcagcatcaagtccgatatgaaagatgcgctgcgcgaagagactcagttctggctggtgacgccaaaagcatcgttggcaggtgtctccgggctggacgccctcgtcggtgggaactatatcggcatgatgccgggtaaaggtaaagagcaggatcactttgtcgcactcgatacccaaccgaaatatcggctggacaatggcgatctgatgatccacctgcaagcccccgatctcggttcgctgaacagcggttcattggtctatttccgcaagatcccggtgggaaaagtctacgactatgccatcaatcccaacaagcaaggcgtggtgattgatgtcctgatcgagcggcgttttaccgatctggtgaaaaaaggtagccgtttctggaacgtttccggcgttgatgccaacgtcagtatcagtggcgcgaaggtgaaactggaaagcctggcggcactggttaacggtgcgattgccttcgattcaccagaagagtcgaaacctgccgaggcggaagatacctttggtctgtatgaagatctggcccacagccagcgtggcgtaataataaaactggaactgccgagtggggccggattaaccgccgactcgacgccgttaatgtatcaggggctggaagtcggacagctgactaaactggatttaaatcctggtggtaaagtcacaggggaaatgaccgttgatcccagcgtcgttaccctgcttcgtgaaaatacccgcatcgaattacgcaacccgaaattatcccttagcgatgctaatctcagcgccctgctgaccggcaaaaccttcgagctggtgcccggcgatggcgagccacgcaaagagttcgttgttgtgccaggcgaaaaagcactgctgcatgaacctgatgttctgacgctgaccctgaccgcgccggaaagttacggtattgatgcgggtcagccgctcattcttcacggcgtgcaggtaggccaggttatcgatcgtaaactcaccagcaaaggcgtcacctttaccgtcgccatcgagcctcagcatcgcgaactggtaaaaggcgatagcaaatttgtcgtcaacagccgtgtcgatgtgaaggtggggctggatggcgttgagtttctcggtgccagcgcctcagaatggatcaatggcgggatacgtattctgccgggcgataaaggtgagatgaaagccagctatccactgtatgccaatttggaaaaagcgctggagaacagccttagcgatttacccaccacaaccgtgagtttgagtgcagagacgctgccggatgtgcaggcaggatcggtagtgctgtaccgtaaatttgaagttggtgaagtgattaccgtgcgtccgcgagctaacgcgtttgatatcgatctgcatattaagccggagtatcgcaaccttctgaccagcaatagcgtgttctgggcagaaggcggggcgaaagttcagctgaatggtagtggtctgaccgtacaggcatccccgctctccagagcattaaagggagccattagcttcgacaacctcagcggtgccagcgccagtcagcgtaaaggcgataagcgtattctgtatgcttccgaaacagcggcccgtgcggttggcgggcagattacgcttcacgctttcgatgccggaaaactggcggtcgggatgccaattcgctatctcggtattgatatcgggcaaatccagacgctggatctgattaccgcacgcaatgaagtacaggcaaaggcggtactttacccggaatatgtccagacctttgctcgcggtggtacgcgcttctcagtggtcacaccgcaaatttcggcagctggcgttgagcatcttgatactatcctccagccgtatatcaacgtcgaaccaggccggggcaatcctcgccgcgactttgaattacaagaggccaccattactgattcgcgttacctggatggcttaagcattattgttgaagcgccggaagccggttcgttaggcatcggtacgcctgtgctgttccgtggtctggaagtcggtacggttacaggaatgacgctggggacattgtcagatcgcgtgatgattgcgatgcgcatcagtaaacgctatcaacacctggtgcgtaacaattccgtcttctggttggcatcgggttacagtctggactttggtctgacgggcggcgtagtgaaaaccggcacctttaaccagtttatccgtggcggcatcgccttcgccacgcctccgggtacgccactggcaccgaaagcccaggaaggcaaacacttcctgttgcaggaaagtgaaccgaaagagtggcgtgaatggggaactgcgcttcccaaataatgcccactgctccggcgtgcctgcgccggagcgtttatgctaaactgcgcgcctgtttttttgccagtggtacatgctcgtggcccaacacaccgtttatttcccggacgcctttctgacacaaatgcgcgaagcgatgccttcgacgctctcatttgatgattttcttgccgcctgtcagcgcccgttgcgccgcagcattcgcgttaatacgctgaaaatctccgttgctgatttcctgcaattaaccgctccttatggctggacgcttacgccaattccgtggtgtgaagaaggtttctggattgaacgcgacaatgaagatgcattgccattgggtagtaccgccgagcatttaagtggcctgttttatattcaggaagccagttcaatgttgcctgttgccgccttgtttgctgacggtaatgcaccacagcgggtgatggatgtcgctgccgcgcctggctccaaaacgacgcaaatttccgcgcggatgaataacgaaggggcaatccttgccaatgagttttccgccagtcgggtaaaagtgttacatgccaatatcagccgctgtggtatcagtaatgttgcgctcacacattttgatggccgcgtgtttggtgcggcagtgccagaaatgttcgatgccattttgctggacgctccctgctctggcgaaggcgtggtgcgtaaagatcccgatgcgctaaaaaactggtcaccagaaagcaatcaggaaatcgcagctacacaacgggagcttatcgacagcgcctttcatgcattacgtcctggtggtacgctggtttactcgacctgtaccttaaaccaggaagaaaacgaagccgtttgcctgtggctgaaagagacttaccccgacgcagtagagtttttaccacttggcgatctcttccctggtgcaaacaaagcgctgaccgaagaaggctttttgcatgttttcccacaaatttacgactgcgaaggcttcttcgttgctcgtctgcgtaaaactcaggcgattcccgccttacccgcccccaaatacaaagtcggtaattttccgttcagcccggtgaaagatcgcgaagctggacaaattcgtcaggcggctacaggtgttggcttaaactgggatgaaaacctgcgcctctggcagcgtgacaaagaactgtggttgttcccggtgggcattgaagccctgatcggtaaagtccgattttctcggttggggattaaacttgccgagacgcacaacaaaggttatcgctggcagcatgaagcggttattgctcttgcctcacccgataatatgaatgcattcgagctgacaccgcaggaagcggaggagtggtatcgcgggcgcgatgtttacccgcaagccgcgccagtggcggatgatgtattggttactttccagcatcaaccgattggtttagccaaacggattggttcgcgattgaaaaacagctatccgcgtgaactggtgcgcgatgggaaactttttaccggtaacgcctgacagcgcacaaaaaaagcgcactttttgactggcacattcggctgcctcaactaggctgaaaaatggtgcgatcggactggtcgtaccacaatcggcagctaaatggagagcacgaagatgaaaaccagtgtgcgcataggcgcttttgaaatcgacgacggcgaattacacggtgaatcgccaggtgatcgaacgttaaccattccttgtaaatctgaccccgatttatgtatgcaactggatgcctgggatgctgaaaccagtatccctgccctgctaaatggcgaacactctgtcctttaccgtacccgttacgatcaacaatctgatgcctggattatgcgtcttgcctgatccaaaaagaacccgtcggcatggcgggttatttgtcctggttattcccccgttgtaaaatctctcctaaacttaacggtacggcaccacacttcggggatgaaatgttcgcgctggtactttttgtttgctacctggatggcggttgtgaagatattgttgtggatgtctacaacacggaacagcagtgtctttattctatgagcgatcaacggatccgccagggcggttgttttccgattgaggattttatagatggtttctggcgacctgcacaggagtacggtgatttttaattattgcaattgcacaagagtcagttcgcccccaaagacagcaccggtatcaatataatgcaggttgccaatatccacgcgatgtcgcaacggtgtatgaccaaaccagaaatgatcagcacctgtaattccctgccctttttggcgttcacctaatcgcgagcggctccacaagacctgatgcaaatcaacgtccttttgccattcataaacatcatctggataatcggcatgagcaataacatgcttgccggtgcgactgtgtacttcaagaataaagggcaaatgctgacatttttccagcgccgttttcgcttgtttctgttgattatctgccagcgcaataaaccagtcgccgccattcatcaaccacaaagacatctgctgggatgccagcgcatccatcgccatctgttcatgattgcctcttaccgcacaaacccaatgttgttccagtaactgcagacaacgtaaactttgcggcccacgatcgataacgtctcccactgagataagtaaatctcgccacggatcaaaacgacaatgccataatttgcggcgcaactgctcaagacaaccgtgtatatcgccagaaagccagatatgtcgccattgatgacccgcaattctctgataaacgggcgcaggctgtttcatcaatattttcctcccgcgctaaagatcacataatcttaacaagaatgttaaaaaacgctggactcagacagtagagtgtgtgttatggttgactataaagtcagcgaaggaaatgcttctggcttttaacagataaaaagagaccgaacacgattcctgtattcggtccagggaaatggctcttgggagagagccgtgcgctaaaagttggcattaatgcaggcttagttgccttgccctttaagaatagatgacgacgccaggttttccagtttgcgtgcaaaatggtcaataaaaagcgtggtggtcatcagctgaaatgttaaaaaccgcccgttctggtgaaagaactgaggcggtttttttattggaaatcaaaaggctattttaggtaattaacagagtttttcagctcgttctataaacggtgccagactcattttttcgccgggattgttaggatcatcaatctgaatcaccgaaatgggttgggcattggtcttcccactggcaacttccttttgtgcgatatcgtttaaaggatactgcacgagggtactcggattaataacatacaaagcattacccggtcggcaagtcagcatcacctcttcgcgattaaacgcccatttgtctttacccacttcaaaacgactgacggtaatcacctgcggtgcagccagcgccgctgcagaactggtgagtaacagaaacgccagaatactttttttcatcattttcgtaatccatcaaaaaggttcgagagtcgcaagcaggctgatgatcaccagcactaccgcacctatcgcccattcgagtttagtcatccacacaaaccagggtgccgcacgatcttcatcctgcctcatgcgcggtacaagaacataacgattagccagcgcaatgaccaccataatcatcaccaggatggctttgagcaataagagttggccccagtaagtcgtaagcgtggggggaaatccggtaatcaacaatgcattaagcacgccgcttgccagtacgccgatcaccgcaaaatgcccgcaccaggaaaaacgcatcagcgcctgaatagcctggtgtcgccaacggcctttgatgagttgcatacaccagagcaccggcagtaatcccccaaaccacgccgccgcacaaatcaggtgaatcgcgtgattagtctgatggattttcgctgttaccccttcattcagcgtcgcatgccccactcccgccagcagaataaattgcgcggtagtgagcataaacagcaaacgtggcatattccgcggttgcataagggcgacgatcaacgttacgagggcgagaacaatttgccataaccagatgccaccaaactgcgtttgcaaaacagcctgccaaatgtttggcgaaaatacatctgtccatcccgttcccatcaacccgccctgaacggcgagcattgcagtggcactgatcaaactccagacggcagcgtgctgttgtaaacgcagaaaacgcttcgccagcaagcgacgaatcgtcaagggggccagccaggcaccgtacattgcgaagccaaaaaccagcatcagcgaggtgaaatggataaatcgcagcgcgatccaggtaaacgccagcatgatttatttcacgctaaaggtgtagtgtcctttcgttttatgcccgtccaccgaaacaacatgccagtcaacggtgtaggttccgggtttcagcgaatcggccagtggaacaatcagttgcttttggtcctgctcatttcgcttcgccggtaatgttttaatattttcgttttttggccccgtgatttttgcaccactgaatcctgtttcaacaccttccgagaagtttaaagtgattgcctgcggtgcagctgtcacttgcgcgtttgccgcaggatactgatgcgttaaatgcgcatgtgcccagacggaaggtgtcaccaacgaagtggtcaggattgccagcgcgtagcgaagggagcgtgcagttgaagccatattatctattcctttttgtaataacttttttacagagcataaccttgtctaatgtctgagtcgaggatcatcaattccggcttgccatcctggctcactcttagtaacttttgcccgcgaatgatgaggagattaagaatgctgaagaatctggctaaactggatcaaacagaaatggataaagtgaatgtcgatttggcggcggccggggtggcatttaaagaacgctacaatatgccggtgatcgctgaagcggttgaacgtgaacagcctgaacatttgcgcagctggtttcgcgagcggcttattgcccaccgtttggcttcggtcaatctgtcacgtttaccttacgagcccaaacttaaataaaacttatacagagttacactttcttacataacgcctgctaaattatgagtattttctaaaccgcactcataatttgcagtcattttgaaaaggaagtcattatgtcgttctggaaagttgcagcagcgcaatatgagcctcgtaaaacctcactcaccgaacaggtagctcatcatctggagtttgtgagggccgccgccaggcaacaatgtcagctgttagtttttccatcgctttctttactggggtgtgattattcgcgacgtgcccttcctgccccacccgatctctcactgttagacccgctttgttatgccgcaacgacctggcgaatgaccatcattgccggccttcccgttgaatataacgatcgctttattcgtggaattgcggtgttcgcaccgtggcgaaaaacgcctgggatctaccatcagagtcatggtgcatgtctgggccgtcgttccagaaccatcacggtggtcgatgaacaaccgcaaggtatggatatggacccgacctgttcactgtttactacagggcaatgtctgggagaacccgacctgctggcgtcggcccgtcgcttacaatttttttcacatcagtactcgattgccgtgctgatggcaaatgcccgtggtaacagtgcactatgggatgaatatggtcgtctcatcgttcgcgccgatcgtggttcattattgttagtcggtcagcgttcatcacagggttggcaaggcgatatcattccattacgctaggctttttcggcctggagcatgccatgttgcgcattatcgatacagaaacctgcggtttgcagggagggatcgttgagattgcctctgttgatgtcattgacggaaaaatcgtcaaccccatgagccacctggtgcgccccgatcgtcctattagtccacaagcgatggcgattcatcgcatcaccgaagccatggtcgccgataaaccgtggattgaagatgtgatcccacactattacggtagtgaatggtatgtcgcgcataacgccagctttgaccgccgcgtactgcctgagatgcccggtgagtggatttgcactatgaaactggcccgtcgtttgtggcctgggatcaagtacagcaatatggcgttatataaaacacgcaagctcaatgtacagacgccgccgggcctgcatcatcaccgcgcgttgtatgactgttatatcaccgccgcgttgcttatcgatattatgaacacctccggctggacggcagaacagatggccgatatcaccggacgtccgtcgttgatgacgaccttcacctttggcaaataccgtggcaaagcggtttccgacgttgccgaacgcgatccgggctatctgcgctggttatttaataacctggacagcatgagcccggagctgcgtttaacactgaaacattatctggaaaatacttagtccgcaggcgtagcgggtaatgttccctgcgccagcgcgaccagaaaagcatattccatcgctacgccttcgtacgatttaaagcgaccagatttaccgccatggcctgagtccatgtcggtacagagcaataaaagatggtcatcggttttcagctcgcgcaatttagcgacccattttgccggttcccaatattgcacctgagaatcgtgcaaaccggtcgttaccagtaaatgcggataagcctgtgcggtgacgttgtcatacgggctgtagcttttcatgtactcgtaatattgcggatcctgcgggttaccccactcttcaaactcaccagtggtaagaggaattgattcatcaagcatcgttgttacaacatcaacaaacggtacctgggcgataacgccgtggaataattccgggcgttgattaattgcaacgcccatcaacatgccccccgcactcccgcccatcgcataacaaagcgaaggagagccatagcccagttttaacaatgcatcgcaggcatcaagataatcattaaacgtatttttcttcttcagaaattttccgtcttcgtaccattgttgccccagctcaccaccgccgcgaacatggacaatggcgtagacaaagccacgatctaacaaactcaagcggctaaaactgaaatcggcatcaatacttgcgccgtaagaaccatagccatacaccagcaacgggttgtgtcctttgcgaaaatgtttgcgatggtagaccaacgaaaccggaacttcgacgccatcacgggcgactatccacaggtgttcactgcggtaattcgccgcataaaaaccaggaacttccgtttgttttaatacacgacgctcaccggtatccatatccagttcaaacaaagtgtctggtgtagtcatggaagaataaccataacgcaatcgcgcggtttcaggttctggattgtaggcaatccaggtcacataggccggatcatcaaaggcaataccaatgacttcccgggtcttgcggttaatttggcgcaaactggttaacccgcgctgacgctcttcaaccaccagccagtcggtaaacagcgtaaacccttccagcatgatgttttcgcgtggcggaattaactcttcccactgttgctcatcacgcatacgggtacggtataagccaaagtttttgccgtggcggttggaacgcagataaaaacgatgctggtagtgatcaaggctgtattcgtgatctttgcggcgcggcagaaaaacaaacggctcggcatcggccatttccgcgtccagcaggcgaacttcactggtggtggcgctggccaaatgaatgactacatagtgcttcgaggtcgttttatgcaggctgacgtaataggtatcgtctttttcttcgtagatcagtttatcttgcgatgctggcgtaccgatggcgtgacgccagacctgataaggcagcagcgtcaccggatgcttgcgaacatagtagaaaatccaggagtcatttgcccagacaaagctgggttcaacgttatccagcagttccgggtaccagttaccagtttccagattacgaaaacgaatgccgtactggcgtcgggaaagaaaatcttctgccagcgccataatggtgttatcgggcgtaatcgccattccgcccatcgaataaaactcactatgagctgcgcgcttattggcatcgagcaatgtttcccactcatcccactcttcactgaatgccgattgacgctggtagatagcatattcacagcctggttcataaatatgccgatagcggtagccatttttgatgtagggcgcagaaacttctcgttgcggaatgcggtcgatgatttcctttaagatgcgatcctgcaaggcttgttgtgaggccatcacccgatgaccgtaactattttcttgttgcaggtagtccaggacttctggctgagaacgcgtatcgtcccgcagccagtagtaattatcgatgcgcgtatcgccatgaagcgtcatggcgtggggaatgcgggcggcttttggtagcatgttattgttctttctggttgaaacatcttataagggtggcaaaactcaccggggatgcaagcgaaacaggggagtcattgcttagatgatgacaggtaatggcgcggatatcgaatgttatgcagacagagaaaatcagcctgttcaaatggctgtgcgattctggatagcccgaaatagtcaacttcaggctatccagagagcggaattattccgccaaagtgcgtttttgctgttcgagatcgcgttcaatgccgtcacgaacatcctgggggattttcagcgcgtcacccagtgcattcaggtaactgcgttccataaaatggtcaatatcaatagccgcgcaactcaggaaatagatttccagcgcctcttcttcattgcggaccccggtagccaggcgttgtggatccagcggttgttcgattgcctgctcaatgagtacacgcccctgctcttccacgccggctccacgcaattgctggtcgattgccgcacgttctttggcatcaatatgaccatcacttttagcggcaaagaccagcgcaaggatcaaacgtgctgtacgctcatccagcggcgtactttgcgcgccaaactgcggttcgtcctgatgcgccgcgcgaattttatctttgtatttattccacagcaccgtacccgctaccgctccgccgccaaccagtaacgcgttggtgccatatttcgtaagaagtttacgtgctgatttatttgcgaccagcagcccagccagtccgcctaatgcgcctggcactaacagtttgaccaatccctgatccgcagacgaggaggtagaagaactgctttgcccaagcagggattgcagttgatttaaccagttagccatatttgctcctcaataaccatttttagtgcctgtagcatagcggatgaggatgtcagaaaatgtatatcgagacaaaagatgcgcaaataagcggggcggtaggccgttattcaaagaaattcgcgccaggtaaggtatttactgtatatcaggtgataagggtattttaggtgaaagtagtttgtcgttttgagtggcattgtttgatgctgattgcccgatgcgacgctgttgcgtcttctcaggcctacgattgtggtgcgttctggggcggacaaggcactcgcgccgcatccgccaacagtcaatcgaattatcagaagccattaacgccgctgatattccgccattcccgctttgcagtccacgctgacctggtaatgaatatcggcacttttaccacgcacggttagcggtactgaccatttatcatctttaccctgaatgtcctgcaaactgacccaagccacgggatcggcctgaccgacaattttttgatcatctgcccaacgcgccacgcgattttgttgataatcacgttttacgctcgcggcaattccggcagcatccagatcttcacactttgggaaagtgaccgacttgctggtttcattattggcagcgaaaactgatgcgcaggcagaaaccaacaacagccctaaaaacgcccctctttttttcatgtttttctccatagcacaatgattcaggagaaagcatggtacaaattgtcaggagcgcaagttgcttcaggccgcgtgtgaggcatcttcctcttcggattcagcaccgacgacctgtggggacggtaatttgccggttttcagaatggtgctcagcacatctttttgttctgccagccatagcgaaagggcttcacgttgctcgtcttccatttgcactggagaatttgtcagccaggtgtcaagcagatccgccgtatcaagcattttgtcataagcatcggcttcctttttgctggtaaacgacattttctcttcgccctcacgaatgactacgtatttaacttcaaccgccatttgcagcctctcataataactgtgattttatacagtatatttcttttcggttgagaaatcaacatcagcaataaagacacacgcaaacgttttcgtttatactgcgcgcggaattaatcaggggatattcgttatgacgttattaggcactgcgctgcgtccggcagcaactcgcgtgatgttattaggctccggtgaactgggtaaagaagtggcaatcgagtgtcagcgtctcggcgtagaggtgattgccgtcgatcgctatgccgacgcaccagccatgcatgtcgcgcatcgctcccatgtcattaatatgcttgatggtgatgcattacgccgtgtggttgaactggaaaaaccacattatatcgtgccggagatcgaagctattgccaccgatatgctgatccaacttgaagaggaaggactgaatgttgtcccctgcgctcgcgcaacgaaattaacgatgaatcgcgagggtatccgtcgcctggcggcagaagagctgcagctgcccacttccacttatcgttttgccgatagcgaaagccttttccgcgaggcggttgctgacattggctatccctgcattgtaaaaccggtgatgagctcttccggcaaggggcagacgtttattcgttctgcagagcaacttgctcaggcatggaagtacgctcagcaaggcggtcgcgccggagcgggccgcgtaattgttgaaggcgtcgttaagtttgacttcgaaattaccctgctaaccgtcagcgcggtggatggcgtccatttctgtgcaccagtaggtcatcgccaggaagatggcgactaccgtgaatcctggcaaccacagcaaatgagcccgcttgcccttgaacgtgcgcaggagattgcccgtaaagtggtgctggcactgggcggttatgggttgtttggtgtcgagctatttgtctgtggtgatgaggtgattttcagtgaggtctcccctcgtccacatgataccgggatggtgacgttaatttctcaagatctctcagagtttgccctgcatgtacgtgccttcctcggacttccggttggcgggatccgtcagtatggtcctgcagcttctgccgttattctgccacaactgaccagtcagaatgtcacgtttgataatgtgcagaatgccgtaggcgcagatttgcagattcgtttatttggtaagccggaaattgatggcagccgtcgtctgggggtggcactggctactgcagagagtgttgttgacgccattgaacgcgcgaagcacgccgccggacaggtaaaagtacagggttaaacccggcaaaaaaacgctacaaaaatgcccgatcctcgatcgggcattttgacttttacagcttagcgccttctacagcttcacgcgccagcttagtaatgcggtcgtaatcgcccgcttccagcgcatctgccggaaccagccaggaaccaccgatgcacagcacgcttttcagcgccaggtagtcacggtagttagccggagaaataccacccgtcgggcagaaacggacctgggagaacggacccgcgatcgcctgcagggctttcacgccgccgttagcttcagccgggaagaatttgaactctttcaaaccgtagtccatacccagcatcagttcggaaacagtgctgatccccggaatcagaggaatagtcccttcggtagcagctttcagcagcggctcggtcagacccgggctaattgcgaactgtgcacccgcttcagtgacttctgccagctgctgtggattcagcaccgtaccggcacccacaatcgcttcaggcacttctttggcgatagcacggatagcgtcaactgcacactcggtacgcagagtcacttccagaacgcgcaccccaccagcaaccaacgcttttgccatcggcaccgcgtgttccagtttttttaccacgataaccggtacaaccgggccggtggtcaggattgattctgcacttgttttccagtttttcatcagagttttctctcgcctgattacaaatttgtcgtcttaaaaagtgatacaggttgcgccctgttcggcaccggacagtttttcacgcaaggcgctgaataattcacgtcctgttcccacgcgtgacgcgctcaggtcaggaatgtgcggttcgcgagcagccagttccgcttcgtctaccagcagcgtcagttcgcctgtctgtccattcacacgaatgatgtccccgtcgcgcacttttgccagcagcccgccatcgtaggcttctggtgttacgtggatagctgacggcactttacctgaagcgccggagagtcgtccatcggtaactaacgcaattttgaaacaccggtccaataatacaccaagtggcggcatgagtttatgtaattctggcattccgttcgcttttggcccctgatgacggacaacaacgacacaatcgcggtccagcaaacccgcttcaaaggccggcataacgtcatgctggctttcaaaaacaaccgctggcgcttcaatcacctggttctcaaccggcacggcagaggttttcataaccgcacggcccaggttaccgcttaacacttttgtcccaccatgatgagagaaaggttgttcgaaggaagcgatcacattgctgtcgagtgatttttccgccccttcccgccagtccagttcaccattattcagccatggttcaagggtataacgagacagaccaaaacctgccaccgtattgacatcttcatgcagcaggcctgctttgagcagttcacgcaccagaaccggtacgccacctgccgcctggaagtggttaatatcggccggaccgttcgggtagagacgtgccatcagcggtacaacatcagaaaggtcagagaagtcatcccagttaatctgaataccggccgcgcgcgccatcgccaccaggtgcatggtgtggttagtggaaccaccggtcgccagcagtgcaacgataccgttcaccaccactttctcatcgatcatcttaccgatcggcatccattcattaccattaccggtcatgcgtgtaacctgacgcgcagctgcggcggtcaaagcatcgcgcagcggagaatccggatgaacaaaagaagagcctggcaactgcatccccataaactccaccaccatctggttggtgttggcagtaccgtagaaagtacatgttcccggcgcatggtaagacgcggcttctgactccagtaaggccatgcggtccactttaccttcggcataaagctggcgaatacgcactttttctttatttggcaaaccgcttgccatcggtccagacggcacaaacaccgcaggcaaatgaccaaacgacagggctgccatcgtcagacccgggacaatcttgtcgcacacaccgaggaacagagcaccatcaaacatgttatgggacagccccaccgccgcagacatcgctatcacttcgcggcttagcagcgacaattccattccatcctgcccctgggtgacaccatcacacatcgccggaacaccgcccgcaacctgaccaaccgcattcgcttcatgcagggctttacgaatgatttctggatagtgttcataaggctggtgcgcggagagcatgtcgttataggaggtgatgatggcgatattgttacgcaacatgcttttcaaagaggctttgtcttctggctggcaggcagcgaaaccgtgtgccaggttaccgcatgccaactgcgaacgatgaacggtcgaagttttcgcttgttctatccgggcgagataagcagagcgagtctcgcgcgaacgttcaatgattcgatttgttacgcgtaacaattgtggattcataaaggctcctgaaattgagttgtcagagcaggatgattcacaacgcgtttcattcagaggatttatgactgaaacgcctgtaaccggagctcatagggcaaaaacgtttcagtcagtgtaataaaaaaagcctcgtgggtgaatccgcacgaggcctgaaagtgtaaaaattgttctacaatctgcgcaagatcatgttaccggtaaaataaccataaaggataagcgcagatattactcaaactcattccaggaacgaccatcacgggtaatcatcgccaccgaggcaacgggtccccaggttccggcctgatacggtttcggcgcatcattgtccatcgcccacgcctcagtaatggagtctacccatttccaggcttcttccacttcgtcgcgacgtacaaacagtgcctgaataccacgcatggtttccagcagcaaacgttcataggcatccgccagatgcgtctgattaaaggtttctgaatagctcagatccagcttggtgatttgcaggttatgtttgtggtcaaggccaggaactttattcagtacctggatatccacgccttcatcaggttgcagacggatagtcagtttattctgcggcagatcctgccacgattctttaaacagattcagttcaggtgttttgaaatagaccacgacttcagaacatttggtcggcagacgtttaccagtacgcaggtagaatggcacaccggcccagcgccagttatcaatgtcgacgcggatcgccacgaaagtttctgtattgctgctcttgttcgcgccctcttcttccagatatcccggcacttttttgccctgggcgaagcccgcagtatattgcccgcgtacggttttttcgcgtacgttggagcggtcgatgcggcgcagagacttcagtactttcactttttcatcgcggatgctgtctgcgctcaggtcagacggcggagacatcgcaatcatgcaaagaatttgcagcaggtggttctggatcatgtcgcgcatctgaccggctttatcaaaatagccccagcgcccttcgatccccacttcttctgccacggtaatctcaacatgatcaatggtgcgattgtcccagttattcacaaacagggagttagcaaaacgcagcgccaacaggttcagcaccgtttctttaccaagatagtggtcgatacggtaaacctggcactcctcgaagtattcgccaacctgatcattgatttcctgcgaggtcgccagcgacgtccccagcggtttctccatgactacgcgtgccggtttagcattcagttttgcctcgccaagccctttgcaaattgcgccaaaagtgctgggcggcatggcaaagtagttaatggtgatacgatttttttgatccagcatcgcgccgagacggctgaatgcagcagtgtcattgacatcgagattacaaaaatccagacgtgcactcagggtgtcccataaaccttcatcaatggtttctttcatgaaagtttcgagcgcctcgcggacaactttggtatatgccgctttatcccagtcagcacgccctacgccgataatccgggtgtccgggttgagctgaccggctttttccagttgatacagggaaggcagcaatttacgacgcgcaaggtcgcctttcgcgccgaaaatgaccaggtcacaggcctgggctgtttgcgttaccgccatgtcattctccttaagttaactaacccggtacttaagccagggtatacttgtaattttcttacggtgcactgtactgcttttacgagcttgcgaaaactgtaaacgcttatccacccgtgcgattacgggaaaagcgcgcaaagtgcggcaaaactgataaaaaaatcatcgttttccattgggtaaaaatctgacactgatcatgttatgaaaaaaaataacaacttttttatctgcttttgtcattaacacggcacacaggcgtaatatctgacaaaactgcatttcgatttctttcagtgcggaaatcgtcattacccgtgagtctctttacatcatgaatatgctggaaaaaatccagtctcagctggaacatttgagcaaatcagagcgcaaagttgccgaggtcattctggcttcgcccgataacgcgatccattcgagtattgctgctatggcactggaagccaatgttagcgaaccgacggtgaatcgtttctgtcgcagcatggacacgcgcggttttcctgattttaaacttcatctggcacagagtctggcgaatggcactccctatgttaatcgcaatgtcaatgaagatgacagcgttgaatcatacacagggaaaatatttgagtccgcaatggcaacgcttgatcatgtccgtcattcactggataaatctgccatcaaccgcgccgtcgacttgctcactcaggcaaaaaaaatcgcctttttcggattaggctcttcagccgccgttgcccacgatgcgatgaataagttctttcgttttaatgttccggtggtgtactccgatgatatcgtgctgcaacgcatgagttgtatgaattgtagcgacggagacgtggtggtgctgatttctcacactggaagaacaaaaaatctggtcgagctggcgcagctggcacgcgaaaacgacgccatggtgattgccctcacctctgcgggtaccccgctcgcccgggaagcaacgctggcaattaccctcgacgtaccggaagatactgacatttatatgcccatggtttctcgacttgcacagctgaccgtgatagatgtgctggcgacaggatttactttgcgacgcggtgcaaaattcagagataacttgaagcgggtcaaagaagcgctgaaggaatcgcgttttgataagcagttacttaatttaagtgacgatcgctaaaaacgactgtcactgtcctaatcttatacgacatccgaatgagattaatttatcgccatcgcggcgttatttcattcggatttcatgttcaagcaacacctggttgtttcagtcaacggagtattacatgtccagaaggcttcgcagaacaaaaatcgttaccacgttaggcccagcaacagatcgcgataataatcttgaaaaagttatcgcggcgggtgccaacgttgtacgtatgaacttttctcacggctcgcctgaagatcacaaaatgcgcgcggataaagttcgtgagattgccgcaaaactggggcgtcatgtggctattctgggtgacctccaggggcccaaaatccgtgtatccacctttaaagaaggcaaagttttcctcaatattggggataaattcctgctcgacgccaacctgggtaaaggtgaaggcgacaaagaaaaagtcggtatcgactacaaaggcctgcctgctgacgtcgtgcctggtgacatcctgctgctggacgatggtcgcgtccagttaaaagtactggaagttcagggcatgaaagtgttcaccgaagtcaccgtcggtggtcccctctccaacaataaaggtatcaacaaacttggcggcggtttgtcggctgaagcgctgaccgaaaaagacaaagcagacattaagactgcggcgttgattggcgtagattacctggctgtctccttcccacgctgtggcgaagatctgaactatgcccgtcgcctggcacgcgatgcaggatgtgatgcgaaaattgttgccaaggttgaacgtgcggaagccgtttgcagccaggatgcaatggatgacatcatcctcgcctctgacgtggtaatggttgcacgtggcgacctcggtgtggaaattggcgacccggaactggtcggcattcagaaagcgttgatccgtcgtgcgcgtcagctaaaccgagcggtaatcacggcgacccagatgatggagtcaatgattactaacccgatgccgacgcgtgcagaagtcatggacgtagcaaacgccgttctggatggtactgacgctgtgatgctgtctgcagaaactgccgctgggcagtatccgtcagaaaccgttgcagccatggcgcgcgtttgcctgggtgcggaaaaaatcccgagcatcaacgtttctaaacaccgtctggacgttcagttcgacaatgtggaagaagctattgccatgtcagcaatgtacgcagctaaccacctgaaaggcgttacggcgatcatcaccatgaccgaatcgggtcgtaccgcgctgatgacctcccgtatcagctctggtctgccaattttcgccatgtcgcgccatgaacgtacgctgaacctgactgctctctatcgtggcgttacgccggtgcactttgatagcgctaatgacggcgtagcagctgccagcgaagcggttaatctgctgcgcgataaaggttacttgatgtctggtgacctggtgattgtcacccagggcgacgtgatgagtaccgtgggttctactaataccacgcgtattttaacggtagagtaagtacgttgccggatgcggcgaaaacgccacatccggcctacagttcaatgatagttcaacagatttcgaatattctgaagcaaacttgaacttatcatcaggcgaaggcctctcctcgcgagaggcttttttatttgatgggataaagatctttgcgcttatacggctggatttcgcccggtttgcgagttttcagcaattttagtatccaggtgtattgttctggtcgcggaccaacaaaaatctcgacttcttcattcatccgccgcgcaatcgtatgatcatccgcctctaacagatcatccatcggtgggcgcacctgaatcgtcagacgatgcgtcttgccatcataaatcggaaacagcggtacaacgcgcgcacggcacactttcatcaaacgaccaatcgcgggcaacgtcgctttataggtggcaaagaaatccacaaattcgctgtgctctgggccatgatcctgatcgggtaaataatatccccagtacccctgacgtaccgactggatgaatggtttaataccgtcatttctcgcatgcagacgaccgccaaagcgacgacgcaccgtgttccagacataatcaaaaaccgggttgccctgattatggaacatcgctgccattttctgcccttgcgaggccatcagcatggcaggaatatcgacggcccaaccgtgcggcaccagaaagataactttctcgttattacgccgcatctcttcgatgatctccagcccttgccagtcaacgcgcggctgaattttctccggcccgcgtattgccaactcagccatcattgccatcgcttgcggcgcggtggcaaacatctcatcaacaatcgcttcgcgttcagcttcactacgttctggaaagcagagcgacagattgattaacgcacgacggcgtgagctttttcccagtcgtccggcaaaacgtcccagccgtgccagaatgggatcacggaactttggcggcgttaaagcgatacccgccatcgctgctacgcccagccatgctccccagtagcgcgggtggcgaaaggatttatcaaactcaggaatgtattcgctattattttttttcgtttccatgcttttccagtttcggataaggcaaaaatcaatctggtgatagtgtagcggcgcaacttgccccgcaccaaataaaaaaagccggtactgactgcgtaccggctgcgaatggatgttaattaatcaaaccgtagctgcggcacaatctctttggcctgcgccaggaattcgcgacgatcggagccggtcagcccttcggtacgcggcagttttgccgtcagcgggtttacggcctgctggtttatccatacttcatagtgcagatgcggcccggttgaacgtccggtattaccggaaagcgcgatacggtcgccacgtttcaccttctgtcccggtttcaccagaatcttgcgcaagtgcatataacgcgtggtgtagctgcgaccatgacgaatagccacataataacctgctgcgccactgcgtttggcaaccaccacttcaccgtcacccactgaaagcactggcgtaccctgcggcatggcgaaatcaacacctctgtgtggtgcaacgcgaccggtcaccggattagtacgacgcgggttaaaattagacgagatacggaactgtttcgccgtcgggaatcgcaagaatcctttcgccagaccagtaccgttacgatcgtagaatttgccatcttcagcgcggatagcgtaataatctttaccttctgaacgcaaacgtacgcccagcagctggctttgctcacgtttaccatcaagcatttctcgagacattaacaccgcaaattcatcgccttttttcagtttgcggaaatccatttgccactgcatggctttaatcactgcgctcacttcggcgctggttaaaccggcgtttctggcgctggcaacaaagcttcccccgacggtacctttcagcagattgttaacccactctccttgctgcatttcgctggtcattttaaaaccgttagcggcagtacggtcataggttcgggtttcacgacgagacacttcccaggtgaggcgctgcagttcgccgtccgcggttaatgtccaggagagttgttgaccgattttcaggttacgcaattctttgtcggccgcagccagttgggtgatatcacccatatcaataccatactgattgagaatgctgcttagcgtatcgccagtggaaacaacatattcatgcacgcccgcttcaccggcgattttgtcatccagttcgtcctggggaatggcttcatcttcttgtgcagcttgatcaatcggctcactggcttcaggtaagagcgaacgaatttcgttctgttccagctcaatggttttgacaattggcgtggcatcacggtgataaacataaggccgccagacagcgacggccagagtaagaacggtgagcgaccccaacataacgcggtgtggtcgcggtaaattattaaacgccagggcgacagagcgggctatctgttgcacgtaatcacttcctcattaatctcctttcaggcagctcgcatactggttggctaattgactcaggaattctgaatagcttgttttacccagtttgatattcgtccccaggggatccaacgttcccatacgaacggatgtccctcgtgcgacgctctcaacgaccgctggcctgaactgtggctcagcaaaaacgcaggttgctttttgctcaaccaactgtgttcttatttcatgtaaacgctgcgcgccaggttgaatctcagggttaacggtaaaatgaccaagcggtgtcagtccaaactgtttttcgaaatagccgtaagcatcgtgaaaaacgaaataacctttccccttgagcggcgcgagctcgttaccaacctgcgtttcggttgaggctaattgtgcctcaaaatccttcaggttggcgtcaagtttggctcgactttgcggcataagttccactaattttccatggattgcaaccgctgtagcccgcgctatctctggggaaagccaaagatgcatgttgaaatcgccgtgatggtgatcttcgtcacttttttccgcgtggtcgtgatcatcatcatcgccgtgaatacttttcatcagtagcggtttcacatcttcaagctgcgcaatcgttacctgcttcgctcctggtaatttgcttaccggtttttgcataaacgcttccatctccgggccaacccaaacgactaagtccgcgttctgtaagcgttttacatccgatgggcgcagtgaataatcatgttctgaagcgccgtcaggaagtaaaacctctgtttctgttaccccatcagcaatggcagaagcgatgaacccaacgggtttaagcgaagcgacaacggcggcatctgcggcctgtgttgcacctccccagagagcggcggataatgctgcgaaaagaagcgtttttttatgtaacataatgcgaccaataatcgtaatgaatatgagaagtgtgatattataacatttcatgactactgcaagactaaaattaacatgacaagtctggtttccctggaaaatgtctcggtttcttttggccaacgccgcgtcctctctgatgtgtcgctggaacttaaacctggaaaaattttgactttacttgggccaaatggcgcaggtaagtcgacactggtacgggtagtgctcgggctggtaacacccgatgaaggggttatcaagcgcaacggaaaactgcgcatcggctatgtaccgcagaagctgtatctcgacaccacgttgccactgaccgtaaaccgttttttacgcttacgccctggtacacataaagaagatattttgcctgcactgaaacgtgtccaggccgggcacctgattaacgcaccgatgcaaaagctctctggtggcgaaacgcagcgtgtactattagcgcgagcattgttaaatcgcccgcaattattagtgctggatgaacccactcaaggcgtggatgtaaatggccaggtggcgttatatgaccttattgaccaactgcgtcgtgaactggattgtggcgttttaatggtttctcacgatctgcatctggtgatggcaaaaaccgatgaagtgctgtgcctgaatcaccacatttgttgttccggcacaccggaagttgtttccctgcatccggagtttatttcaatgtttggtcctcgtggtgctgaacaactgggtatctatcgccatcatcataaccatcgtcacgatttacagggacgaattgttttgcgtcggggaaatgatcgctcatgattgaattattatttcccggttggttagccgggatcatgctcgcctgtgccgcgggtccgctgggttcgtttgtagtctggcgtcgtatgtcttatttcggtgatacgctggctcatgcctcattacttggcgtcgcgtttggtttgttgctggacgtgaatccattctatgcggtgattgccgttacgctgctgctggcgggcggtctggtatggctggagaagcgtccacagctggcgatcgacacgttattagggattatggcgcacagtgccctgtcgctgggcctggtggtcgtgagtctgatgtctaatattcgtgttgatttgatggcttacctgttcggtgatttgctggcagtgacgccagaagatctcatctctattgcgattggcgtggtcatcgtggtggctattttgttctggcaatggcgcaatttgctgtcaatgacgataagcccggatctggcgtttgttgatggtgtgaaattacagcgagtgaaattgttgttgatgctggtgacggcattgacgattggtgtagcgatgaaatttgtcggtgcgttgattattacttcgttgctgattattcctgctgctactgcgcgtcgctttgcccgcacgccggaacagatggctggtgtcgctgttttggtggggatggtggcagtgactggcggtttaaccttttccgcggtttacgatacgccggcgggtccgtcggtggtgctatgtgcggcactgttatttattctcagtatgatgaaaaagcaggccagctaatctatcgctgaacacatttgtcggatgcggcgcgagcgccttatccgacctacggttcggtatctctggtagtcctggtaagacgcgaacagcgtcgcatcaggcatattgccagtgccggatgcggcgcgagcgaccaatccgacttacggcatttctggcggcgttatgccaaagtgattccacgcccgcgtcgtcgccatacgcccacgcggtgtacgctgcaaaaagccttgctgaatcaaataaggttccagcacatcctcaatggtttcacgttcttcgccaatggctgccgccaggttatccagacctacaggtccaccaaagaacttatcgattaccgccagcaacaatttgcggtccatataatcgaaaccttcagcatcgacattcaacatatccagcgcctgagcagcgatatctgccgagatggtgccatcgtgcttcacttcggcgaaatcacgcactcgacgcagcagacggttggcaatgcgcggcgtaccgcgagcgcgacgagcaacttccagcgcgccgtcatcactcatctcaagccccataaagcgtgcgctgcgactgacgatatattgcagatccggcacctgataaaactccagacgttgcacaataccaaaacggtcgcgcaacggtgatgtcagcgaacctgcgcgcgtggttgcaccaatcagggtaaacggcggcaaatcaattttaatggagcgtgccgccggaccttcaccaatcatgatatccagttggtagtcttccattgccgggtacagcacttcttcaacaactggcgatagacggtggatctcatcaataaacagcacgtcatgcggttcaaggttagtgagcatcgcagccaaatcgcccgccttttccagcaccggaccagaagtcgtgcgtaaattaacgcccatttcattggcgacaatgttggcaagcgtagttttacccaaccccggaggaccaaaaatcaacaaatgatcgagggcatcgccgcgcagtttcgctgctttgatgaaaatctccatctgtgaacgaacctgcggctgaccaacatactcttccagtaatttggggcgaatggcgcgatctgctacatcttccggcaaagtggtaccggcagaaatcagacggtctgcttcaatcatcctttacctcataacgcggcgcgtagggcttcgcgaattaaagtttcactgctggcgtcagggcgagcgattttgctcaccatgcggcttgcttcttgtggtttatagcccagcgccaccagcgcggcaaccgcttcttgttcagcatcgtcggtcgccgggctggcaggagacgtgagtaccaggtcggcggctggcgtaaagagatcgccatgcaaacctttaaatcggtctttcatttcaacaatcaagcgttcggcggtttttttgccaatacccggcagtttcaccagtgcccccacttcttcacgctcaacggcattaacgaactgctgcgctgacattccggagaggatcgccagcgccaacttcgggccgacgccgttggttttgatcaactctttgaacaatgtgcgctcttgtttattgttaaaaccgtacagcagttgcgcgtcttcacgcaccacaaagtgggtgaaaacgatcgcttcctgacccgcttcagggagttcataaaaacaggtcatcggcatatgcacttcatagcctacgccgcccacttcaattaacaccagcgggggttgtttttcaatgatgatgcctctgagtctgcctatcacatgacgctcctgcgtaatgaatcaaagataatgctgtatgataaaaaaatgctggatagatatccagcgaaggatgaagaaaacttgcgaggtgtctcgatgaactgaaaaatggcacagtataatttattctacaggttatattggaagcaaatattttaatattacatattcagtgaagaaatgcgtaataaaaatatacattgcgcctcctgaaaaaataaattttttatgctattacgtatatttgtatctatttcaatggaatgacaacgtgaatattaattaccctgctgaatatgaaattggagatatcgtctttacatgtataggtgctgccttatttggtcaaatatcagctgcatcaaattgctggagtaatcacgtcgggatcattatcggtcataacggtgaagacttcctggttgcagaaagccgggttcccctttcaaccatcaccacgctatctcgttttattaaacgttcgtctaatcaacgctatgctataaagcgattagacgctgggctgacagaacgacaaaaacaacgaattgttgaacaggttccctcccggctacgcaaactttaccacaccggttttaaatacgaatcttcgcgccagttctgttcaaaatttgtttttgatatttataaagaagcgctatgtattccggtgggtgaaatagagacgtttggagaattgttaaatagcaatccgaatgcaaaactcactttctggaaattctggttcctgggttctattccgtgggagcgtaaaaccgtcacgccagccagtttgtggcatcatccgggtttggtgttgattcatgcggagggagtggaaacgcctcagccggaactgaccgaggcggtataacttaacgcagtcgccctctcgccaggttcagccgcgattcgctcatctgcatcgcattctgactaacgtggcagtgggtgatagcaatcgccagcgcatcggcggcatccgcctgtggattagcgggcagtttcagcaaggtgcggaccatatgctgcacctggcttttttcggcactgccaatacctaccaccgtttgctttacctgacgtgccgcgtattcaaatactggcaactcctgattcaccgccgccacaatcgccacgccgcgcgcctggcccagtttcagggctgagtcagcgttctttgccataaagacttgttcaatggcgaaataatcaggctggaactgggtgatgatttccgtcacgcccgcatagatgagtttcagacgagacggtaaatcatccactttggtgcggatgcatccgctacccaggtaggacagttgcctacctacctggcggatgacgccgtagccggtcacgcgcgaacccggatcaatgccgagaataatagccatcacgcgtctccgttttgctgtttagcaggcctcatcagagagtcgctgcgacctcatcagagatttcaccgttatggtaaacttcctgcacgtcgtcgcaatcttccagcatatcgatcagacgcatcagtttcggtgcggtttctgcatccatatcagctttggtagacgggatcatggaaacttccgcgctgtctgctttcagacctgccgcttccagagcgtcgcgcactttacccatttcttcccatgcagtgtagacatcaatcgcgccgtcatcataggtcacaacgtcttcagcacctgcttccagtgctgcttccatgatggtgtcttcatcgcctttctcgaaggagatcacgccttttttgctgaacagataggcaacggaaccatcagtaccgaggttaccgccacatttgctaaatgcatgacgcacttcagcaacggtacggttgcggttgtcagacagacattcaatcatgattgccgtgccgccaggaccgtaaccttcgtagatgatggtttccatgtttgcatcatcatcaccgcccacaccacgtgcaattgcgcggttcagtgtgtcacgggtcatgttgttagacagtgctttatccaccgccgcacgcagacgcgggttagcgtccggatcgccaccgcccagcttagccgcggttaccagctcacgaatgattttagtgaagattttaccgcgcttagcatcctgcgcagctttacgatgtctggtgttggcccatttactatgacctgccataaaaatatctccagatagccctgcctgttcaggcagcgttaattacaaactgttcaatcgcctgccggttgctccaggacttagtgagcgccgccgcagcaggcgcatcaagccacttgtaagccagatgttcagtgaaaacgatctgccgctcgtgcggaagcgcaagacagaaccatgattccgtattacgcgtcacgcccggcgcatagcgatgacgtaaatgtgaaaaaatttcaaactctaccgtgcgctgacagtcaattaaggtcagttgttcagcgacaacatcaatggtgacctcttcctttacttcgcgcatggcagcttgcggcgcggtttcaccctcttccacgctgccggttaccgactgccagaaatcgggatcgtcacgccgctgcaacatcagcacccgtttcgtatcttgtgcgtagatgaccactaagatcgaaacgggacgcttatacactttatccttcacgctgcctcttcgttgactgccttcgctcatcccattcacatagttatctatgctcatgggagttcactcagttgccgcctcgatgcaacgcgaatgatttcgtgtatttgagtcatatcagttattctcagccttcttcacaacctgaatgctcagctcagccagtgcagtcgggttagcaaagctcggtgcttcagtcatcagacacgctgccgccgtggttttcgggaaggcgataacgtcacggatattgtcggtgccggtcagcagcatggtcagacggtcaagaccgaatgccagacctgcgtgcggcggagtaccgtatttcagagcgtcgagcaggaagccgaatttctcgcgctgttcctcttcgttgatacccagaataccaaacaccgtctgctgcatatcaccattatggatacgtactgaaccaccgcccacttcgtaaccattgatgaccatatcgtaagcgttcgccaccgcattttccggtgcagctttcagttctgcagccgtcatatctttcggtgaggtgaacggatggtgcattgccgtcaggccgccttcaccgtcgtcttcaaacatcgggaagtcgataacccacagcggtgcccatttgctttcgtcggtcagaccaaggtctttacccactttcaggcgcagtgcacccatcgcgtcggcaacaattttcttgttgtcggcaccgaagaaaatcatatcgccatcttgcgcggcagtacgatccaggatgtcttcgatgatttctgcattaaggaacttcgctaccgggctgttgataccttccagacctttcgcgcgttcgttaactttgatgtaagccagacctttcgcgccgtagattttaacgaagttaccgtattcgtcgatctgcttacgggtcagcgatgcgccgcccggaacgcgcagagccgctacgcgacctttcggatcgttcgccggacctgcaaatacagcaaactcaacagatttcagcagatcagcaacgtcagtcagttccatcgggttacgcagatccggtttatcagaaccataacggcgttctgcttccgcaaaggtcattaccgggaaatcgcccagatccacacccttcacttccagccacagatgacgcaccagcgcttccatcacttcacgcacttgcggcgcggtcatgaaagaagtttccacatcgatctgagtaaattcaggctgacggtcagcacgcaggtcttcgtcacggaagcatttaacgatctgatagtaacggtcaaaaccggacatcatcagcagctgtttgaacaactgcggggattgcggcagtgcgtagaatttacctttgtgcacacgagaaggcaccaggtagtcacgcgcgccttccggcgtggctttggtcagcatcggagtttcgatgtcgaggaagccgtggtcatccataaaacggcgcaccaggctggtgattttagcgcgggttttcaggcgctgagccatttccggacgacgcaggtcgaggtagcggtatttcagacgcgcttcttcggtgttgacgtggttagagtcaagcggcagaacatctgcgcggttgatgatagtcagcgaggacgccagcacttcgatttcgccggtcgccatatcgcggttaatatttttttcgtcacgcgcacgtacggtgcccgtgacctgaatgcagaactcattacgcagttcagaggccagctttaacgcgtccgcacgatccggatcgaaaaatacctgcacgataccttcgcggtcgcgcatatcgatgaagatcaggctaccaagatcacgacgacggttgacccaaccacacagagtcacctgctgccccacgtgggacaaacggagctgtccacaatattctgtacgcatgagatatcccttaacttagctgccggcggatgccccctgctgcgcaggtgaccaagtcgcagcgttagctgtatgtcacaactgaatgaaaaaaggcggctattatactggaaattctgccgcaccgtaagagcctggcccgcgctggaacgcctcgttaccactttatatcgggcctgaaatcagactctacgccagtttgctataaaggtgttgcccgaactcataaaaattaacaaaatttgtcgttccgccatcggctaatcgcattaaggtgtgaggcacgattttgttttttcaggagtcattatgcttgaacttaatgctaaaaccactgcgctggtggtgatcgatttacaagaaggcatcttaccttttgccggtggtccacatactgccgatgaggtagttaatcgcgccgggaagctggcggcgaaatttcgcgccagcggtcagcccgtgtttctggtgcgcgttggctggtctgccgattacgctgaagcattaaaacagccggtcgatgcgccctcaccggctaaagtgttgcccgaaaattggtggcaacatcctgctgcattaggtgcaaccgacagcgatatcgaaatcatcaaacgtcaatggggtgcgttttacggtacggatctggagttgcaattacgccgccgaggtatcgatacaatagtgttatgtgggatctcgaccaatatcggtgttgaatccaccgcccgcaatgcctgggaacttggctttaatctggtgattgccgaagacgcctgtagtgccgccagcgccgagcagcacaataacagtatcaaccatatctacccgcgcatcgcccgtgtgcgtagcgtggaagagatcctcaacgcgttatgatttacatcggtctaccgcaatggtcgcatcctaaatgggtgcggttggggatcaccagccttgaagagtatgcccgccactttaactgcgtggagggcaacaccacgctttacgccctgccgaaacccgaggttgtcctgcgctggcgtgagcagaccacagatgacttccgcttctgttttaagtttccggcgaccatttcgcatcaggcagcattacggcattgcgatgatttagtgactgaatttttgacccgcatgtcaccgttggctccgcgcattgggcaatactggctgcaactgcctgccacattcggcccacgggagctgcctgcgctttggcattttctcgattctcttcctggcgaatttaattatggcgtggaagtccgccatccacagtttttcgccaaaggagaagaggaacaaacgcttaatcgcggtttacatcagcgcggcgttaatcgggtgattttagacagccgcccggttcatgcagcacgtccacacagtgaagctattcgcgacgctcaacgaaaaaaacctaaagttccggtacatgctgtactgacggcgacaaatccgctgatccgttttatcggtagtgatgatatgacgcaaaaccgggaattatttcaggtctggttacaaaaattagcgcagtggcatcagaccactacgccttatctttttttacatacgccagacattgcccaggcaccggaactggtacataccctgtgggaagacttacgtaaaacgcttccagagatcggagcagttccggctattccacagcaatcttctcttttctgaatttgccacctatcatagacaggtgccatcggccattttaaagggagtttgtatggtaagcgcgctgtacgccgttttaagtgcgttgttattaatgaagttctcttttgatgtcgttcgcctgcgaatgcagtaccgcgttgcctatggcgacggcggttttagcgaactgcaaagcgctattcgcattcatggtaacgcggtggaatatattcccatcgcgattgtgctgatgctgtttatggaaatgaatggcgcagaaacctggatggtgcatatttgcggcatcgttttgcttgctggtcgtctgatgcattattacggttttcatcaccgtctgttccgctggcgacgttccggcatgagcgccacctggtgtgcgctgttgctgatggtgctggcgaatctttggtatatgccctgggagttggttttctccctgcgttagcgcacaatacgccactttctttttcccggatttttacgttatgtctcaccgcgacacgctattttctgcccctatcgccagactgggcgactggacctttgatgaacgggtagctgaagtcttcccggatatgatccagcgttccgtacccggctattccaatattatttccatgattggtatgttagccgagcgcttcgttcaacctggtacgcaggtttacgatctgggttgttctctgggcgcggcgacgctctcggtgcgtcgcaacattcatcatgataattgcaaaattattgccatcgacaactccccggcgatgattgaacgctgccgtcgtcatattgacgcctataaagcccctacgccagtagacgtcattgaaggtgatattcgcgatatcgccattgaaaacgcatcgatggtggtgctgaattttaccctgcaattcctggaaccttccgagcgccaggcgttactggataaaatttatcaagggctgaaccccggcggcgcgctggtgctttcggaaaaattcagtttcgaagatgccaaagttggtgaactgttgttcaacatgcaccacgactttaaacgtgccaacggttacagcgaactggagatcagccagaagcgcagcatgctggaaaacgtgatgctgaccgattccgtggaaacccataaagcacgcctgcataacgccggttttgagcatagtgagctgtggttccagtgctttaactttggttcactggtggcattaaaagcagaggacgctgcatgatcgactttggtaacttttattctctgattgccaaaaatcatctttcacactggctcgaaacgctgcccgcgcagattgctaactggcagcgcgagcagcagcacgggttgtttaagcagtggtcaaatgcggtggagtttctacctgaaattaaaccgtatcgtcttgatttattgcatagcgttacggcagaaagcgaagagccactgagcgcagggcaaattaaacgcattgaaacgctgatgcgcaacctgatgccgtggcgcaaagggccgttctcactgtatggcgtcaacatcgataccgaatggcgttccgactggaaatgggatcgtgttctgccccatctttctgatttaaccggacgcaccattctggatgtcggctgcggcagcggttatcacatgtggcgcatgattggcgcaggcgcgcacctcgcggtggggatcgaccctacgcaactgtttctgtgccagtttgaagcggtgcgtaaactactgggtaatgatcagcgcgcgcatttgttaccgttaggtattgaacaacttccggcactgaaagcctttgataccgtcttttcgatgggcgtgctttaccatcgccgttcaccgctggagcatctatggcagttgaaagatcaactggtcaatgaaggtgaactggtgctggaaacgctggttattgatggtgatgagaacacggtgctggtaccaggcgatcgttacgcgcaaatgcgtaatgtctatttcatcccttccgcgctggcgctgaaaaactggctgaagaagtgtggttttgtagatatccgcattgcggatgtgagcgttaccaccacagaagagcagcgacgcaccgaatggatggttaccgaatcgctggccgatttcctcgacccacatgatccgggtaaaacggtggaaggttatccggcacctaaacgcgcggtgctgattgcgcgcaagccgtaaaggtctggtattactgccggatgcggcgtgaacgccttatccggcctacaaaaccttgctaattcaatatattgcagggactatgtaggcctgataagcatagcgcatcaggcagctttacgtttgcataacctcagcgcccgtttccgggcgctattcacgtcttacgcctgaacagctggctgatcaaacgccgttaacttcggtgcattgcccgtatatttttcgatatacaccaacgctgagttaccggcacaggcatttgccagctgcgagctggggatatccgccgttaacacgttcgcactgccgtttttacacaagccattttccagatctggccatgcaccttcatgcacgcataccacgccttttttgatcccgtcagtcaccaccgcgcctgtcaaaatctgaccacgtttgttccagacacgcaccagatcgccattcgcaataccaaagcgtgcagcatcttcggtgtgaatagtgattggttcacgatcggcgatcgcatattttttacgcagttccgcatagttaagctgactgtgtaaacggtgtgccggatgtgcggtcagaagctgtaactgcttctcgtcggcggtacctttccattcatcaggagccagccaggttgggtgtgccgggcaatccttatagccaaatttttccaacgtttttgaatagatttcaattttgccgcttggcgtacccagcgcatttttcaccggatcggcgcggaaatcaccataacgaacgtactgttcgttcttctcgctgtggcgcatttcgatcagtttattttgctgccagaaggcattaaacattggcatagtgacgcgttgcgcacgggcacctttctgagcggcatcatagaaaaatttcagccacgccatttcatctttaccttcggtatagatctcttttccgccaggtttgagtaattccgcaagatcggcaaacacgtcaaaatcgttacgcgcttcaaattgcggagcaacagcctgcttcatcggcacaatatgctggttgctgtaatcaccggtcatcgtcaagtcattgcgctcaaacgatgtggtgatcggtaatacgatatctgcgtgtttggctgctgcggtccagtagcattcagaaacgacgatcatctccggtttctgccatgctttaatcagacgattagtatcctggtgatgggtaaagttaccgccacccgcccaccagatcattttgatattcggatacgtttgttctttaccgttatgctgatatttgccgccaggattttccagcgcatcgacgatacgggcaacaggaatcgccgtcattccgccatcatcagcggcctcgctggcatgtccggcaatcgccgcagacatttccggcagcacgccgccaacacgcgtcgggttgccaccgttggagtaatgataagagaaaccaaaaccgccgcccggtgtaccaatctgccctaacatcgccgccagcgtcaccagcatccagtgtttctgttcaccatattgctggcgctgaattccccagcctgccatcagcattgtgcgattcgccgccatcagttcagcgagtttgactatctgcgcttccggtacgccagtaatttccgccgcccagaccgcgctcttcggcgtattatcgctcttacctgtcagatactcttcaaactgcggatacccggtagtgtatttttcaaggaacactttatcgtgtttgccttgtgtcatcagggtatgcgcaatccctaacatcagtgccacgtcggtgcccatattcggcgcgatccaggtggcattatcgtcaaagaattcgatggtttcggagcggataggatcaatggcaatcactggtttgccagattttttcagctgatggaagtattccagcccttgctcatcggtactgctccaggcaatttttaaggtattcagcgggttcattccccacagcaccacaacctggctgttttccagaatcagcggccaggaggtctgctgttcatacacctctacagaaccgaccacatgcggcatgatcacctgtgctgccccggttgaataatcgccgctatgcccggaataaccgcccgccaggttcatataacgttgcagtaaggtttgcgctttatgcaacacgccagaagagcgccagccgtaagatccggcaaaaatggccgatggtccgttagctttacgaatacgatcatgttgctcatgaatcagttttaatgcctgttcccagctcacctgtacataggtatcttcgccacgacctttcgccggttgcagtggattatcgagatagctttttctcaccatcggatgctgaatacgcgccgtggtgtgtacctgatccgccgccgtagactgtaaggaattcggtatggttttcgccagcgcgcctgttgaagaaacaatcttgccgtccttcacttctacgttcatcgctccccaacgtcccgcggtgaggattttaccgcccttctcttctgcccatgcggggagcggtgctgccgatgtcaccaccagcgctccagcggcaataccgctgtgtttaataaattcacgtcttgttaatgtcataacttcctccctgatcaacgaggatcactgtttctcggtaatatctttggcgttgtactggaaataccgcgttaaaatgtccagttcgttttcgctcatgctggttcgtgcccccattcctttggcaatggacggccacgcattgacggtgtaatggtcggcggcaataggggcatgacaaccagcgcaataggtatcgtcaagtttttcagcgtattgccatagcggtttacggtccgctaatgcgggatcggtaagcgcaccctgtaaagacgcctgacgccattgattgccgtattcgtcagcctgccattccccgtttacagtgagcgccttgataccttcttcacttaatgtggctagcgccagccgttgacctgccgccaggtagagcgtgttttcactgccctgcatttgataaccctgcaacagaacgatcggctgtttgccactggcatcaacgacggtgagatcggttccaggattcacggtagccagctcgcctatgtgagaagttttgaaaggataaatatgtgcgccattagtaactgaagtagcggcctgactttccagctcatgcgccgcgttgtcatccatttttatttctggcggaaaatgggcaatgcctttatgacaatcgatacaggtttcgctgtccttttgtgctttgttatgcattttctgcgcagattcactttgcgaggcaatatccatggcatcaaaagaatggcaactacggcacgttgcagagtcagtggcttttaattctttccatactgtttcggccatttcctggcgatgagcttcgaacttatcgtcactgtctattttgccgctaacaaattcatgataaatatctttagatgcctttaatttagcaaataaataatccatccctgactttggaatatggcaatcggcacattccgcacgtatccctttctggttcgaaaagtggacagttccctgatattcctcaaaaggtttactcatcgagtggcaggaaaggcaaaatgctgtatccgacgttttatgtaagactttttgcgccagcaataacccgccgccaccaaccacaaccgctatcagcaaaaacaataacccaatgcgttttttccctcgcatagattcctctaattaaattactggacaccgaaatcattgtataattaaatatacaacgaattaaccgcttgcataattaggcacaacactgcctgaaacaatcgataaagaatatgatttattacaatgtaatcattaattgctaaggaataacccagttgctatttagaatatatatttatcagttttagtaatttaaatcccataattaatgtgaatatatacaatatttttagcacaacgctatgcgcactgtcacccgctcaacagatcacggttatcgttcgttttttatactgttcagggataaaaaaaggcccctgttgaaattgcaggggcctggtacgagcaagcatcatattgggcgacatgatgcaacggtaaaaatcatttggcctgatggcgttcaatgattcctttcatttcagcaaccgccgccccgtctacgatataacgcgaatactcgtccgcgtgttcatctgatgacatggacaatccttgattacgataacgcatcggtgaggcttgccacgctcccgcggagctatggacttccagcactccggcatcgaggaagtggtgcaggttttctgcacggactcctgctccggccataatgattggagcatcacgatgggcaataagttccataatttttgataaaccttgcagtgcgtctgatttttgccctgatgtcagtacccgggcaatgcccaattccgcaagattattgagtgtatataaagggttagcgcacatatcgaaggcgcgatgaaaagtcactgccagcggaccggcagcagccattattttttccattcgtggcatatcgacattcccgtcaacatcgagaacgcccgtcaccagtccaggaaaacctaattcgcggaccgtgcgcacatcctcaagaatggcggcaaactcaccgtcgctgtagcaaaaatcaccaccgcgtgggcgaattatcggatgcacagggatcgtcacccgctggcgcacggatttcagtacacccaacgacggcgttaagcccccctcttttggggctgcgcataattcaactctgtctgcgccgttttgctgcgccgttagtgcacattccatgctgtaacagcaaatttccagtaatgccatttttactccttaattacgccgactgctcgctggcaacgatctcttcaatggaccacggatgaaacttaatagttgttttgccatcggtgaccgccagcgtcggattcggtaatcgctcatgctcaccttttggcgaactggttttcactgagatccccggtaggctgagtccttcatcagaaagcaatgccagcgcacgggcattcagcgtttctggatcacccggcagaacgatttcaatatgttcccaaccttcgtgtgggtaacgtttttccccgggccacggtagctccacaatagaaaactgccagtgcgcaacctgtaccggttcatgcaatttaaacagacaaatcggtctgccattgatcatattttctgacaaaagctcgccacactgttcaaacccgcgacgccagcgttcagcagtggcgttttgatggcaacgcaaagaaatgtgatcggcagtcagcggagtgatattcaaccccagacggcgggaaagttcatctaatgcgtggataaatcgcggtaaatccgatgcaatatcctgcagctcgtcgatagattgccagttcgccataatcactcttcgtctttcagtaaaagcgttaatttaccctgttgccctgtgccaaccaaccgctgatttcacgccgcttctgatgcaatagtgaaaacggcaatacgccacgcgcacgttgctgacgaaaacagccatttgcagtatactcccgccctaatttctttaactggtgcgggcaatttttgctcgcttcatcaatgtaaggtattccggtgaatattcaggctcttctctcagaaaaagtccgtcaggccatgattgcggcaggcgcgcctgcggattgcgaaccgcaggttcgtcagtcagcaaaagttcagttcggcgactatcaggctaacggcatgatggcagttgctaaaaaactgggtatggcaccgcgacaattagcagagcaggtgctgactcatctggatcttaacggtatcgccagcaaagttgagatcgccggtccaggctttatcaacattttccttgatccggcattcctggctgaacatgttcagcaggcgctggcgtccgatcgtctcggtgttgctacgccagaaaaacagaccattgtggttgactactctgcgccaaacgtggcgaaagagatgcatgtcggtcacctgcgctctaccattattggtgacgcagcagtgcgtactctggagttcctcggtcacaaagtgattcgcgcaaaccacgtcggcgactggggcactcagttcggtatgctgattgcatggctggaaaagcagcagcaggaaaacgccggtgaaatggagctggctgaccttgaaggtttctaccgcgatgcgaaaaagcattacgatgaagatgaagagttcgccgagcgcgcacgtaactacgtggtaaaactgcaaagcggtgacgaatatttccgcgagatgtggcgcaaactggtcgacatcaccatgacgcagaaccagatcacctacgatcgtctcaacgtgacgctgacccgtgatgacgtgatgggcgaaagcctctacaacccgatgctgccaggaattgtggcggatctcaaagccaaaggtctggcagtagaaagcgaaggggcgaccgtcgtattccttgatgagtttaaaaacaaggaaggcgaaccgatgggcgtgatcattcagaagaaagatggcggctatctctacaccaccactgatatcgcctgtgcgaaatatcgttatgaaacactgcatgccgatcgcgtgctgtattacatcgactcccgtcagcatcaacacctgatgcaggcatgggcgatcgtccgtaaagcaggctatgtaccggaatccgtaccgctggaacaccacatgttcggcatgatgctgggtaaagacggcaaaccgttcaaaacccgcgcgggtggtacagtgaaactggccgatctgctggatgaagccctggaacgtgcacgccgtctggtggcagaaaagaacccggatatgccagccgacgagctggaaaaactggctaacgcggttggtattggtgcggtgaaatatgcggatctctccaaaaaccgcaccacggactacatcttcgactgggacaacatgctggcgtttgagggtaataccgcgccatacatgcagtatgcatacacgcgtgtattgtccgtgttccgtaaagcagaaattgacgaagagcaactggctgcagctccggttatcatccgtgaagatcgtgaagcgcaactggcagctcgcctgctgcagtttgaagaaaccctcaccgtggttgcccgtgaaggcacgccgcatgtaatgtgtgcttacctgtacgatctggccggtctgttctctggcttctacgagcactgcccgatcctcagcgcagaaaacgaagaagtgcgtaacagccgtctaaaactggcacaactgacggcgaagacgctgaagctgggtctggatacgctgggtattgagactgtagagcgtatgtaatcgatttttcgtgagagtgaagcctgatcagggttagccgatcaggcttttttattgccatctaaatgtattctgaaaatggacatgccattgttttctcactgttggataagaggccagaagcgtaatatccggccccagggaaacgataacggttgaatttaaggaataccgcagtgtttaaatttcttgtattaacattaggcattatctcttgccaggcttacgcagaagatacggttatagtaaacgaccatgacatttcagccatcaaagattgttggcaaaaaaattcagatgatgatactgacgttaacgtgatcaaatcatgcctgcgacaagaatacaatctcgtcgatgcgcaattaaataaagcctatggtgaagcttatcgttatatagaacaagtgccacgcacaggtgtaaaaaaacctgataccgaacaacttaacttgcttaaaaaatcacagcgagcctggctggattttagggacaaagaatgtgaattaatcctttcaaatgaggacgttcaggatttaagtgacccttattctgaatcagaatggctctcatgtatgatcatacagaccaatacgcgaactcgccagttgcagctataccgtaactctgaagatttttatccaagccctttgacaagaggataattcacatctttttggcatgttttgttgcaagctattcctgataaataattgcaacaagacatcgagcctttttcactgagttattaaacatactcgcgagcgcgtaatttttttgtccttcagcgataattcacaatcacttcattacgttgtacctttagcggtggaattaaccgcccaccgcctggcacttcccagataaatcgcaacggttctgctgccgctataccggaaaaggccacggtggttccgctctgcccctctaattcgacacaacgagattgcgaacacaagcgaacccgcagtcctgaaggtgtcgggccgataagctgataacgccacgctaccagcgtcatcaatcctgaagcaggttgtcgcgtagaaagaggcgcagacgacatcgactcaccgcgatgatttagcgtaattcctacactacttgcctgccacatcccctccccggcggcttgcaccagcagcggaaacaataatattgctaataaggttctcattatttgccgccaattgtcgccgtcatgcggatatgtcggttatcagacagttccagattcgacaggaccactaactgcggcaagctgcggcgcaggaagcgagacaataatggtcgcagcgcgtggttcaccaacaatactggcggcgcacccagcatctcctgacgggatagcgcttcctgagtttgcgccagtaaacgatccgccagccctggctccagtcctcccccgccctgcagcgcctgtagtaacaaacgttccagcggtgtatcgaggccaataacatggacttcatctttgccaggaaaccactgctgggtaatcgcccgtcccaacgccacgcgcacgacggcggttaattcatgtggatcgctttggatgggcgcatgttccgccagcgtttcgagaatggtgcgcatatcgcgaatcggtactttttcatcgaggagattttgcagcactttatgcagtgtggtgagcgtgacgacgccaggaacgagatcttccgtcagctttggcatctcctgggcgacgcgatccaacagctgttgcgcctcctgacgaccaaacagctctgcggcatgctggctaatgaggtggttaagatgcgttgctaccaccgtgctggcctcaaccactgtgtacccctgaatctgcgcctgttcttttagcgcactttcaatccagatagcattcaggccaaatgccggatcgacggtcgcctcaccaggtaacgtcccggcagcggttccagggttaatcgccagccagcgccccggataagcatcaccactgccaatctccacgcctttcatcaaaatgcgatagcgggcaggttgcagatccatattgtcgcgaatgtgcaccactggcggcagaaatcccatctcctgggcaaatttcttgcggatactgcgtatacggcccaacaactcaccatcctgctggaaatcgaccatcgggatcagtcgataacccacttccattcccagagaatcttccagttgtacatcgttccacgtcgcttcgacaacggtattattctctgccatttttaccggtttgggttcggcaggcgctttttgttcgcgtccgcgtatccaccaggccagcccgagcaatccggcagtgaacagcaaaaataccaggttcggcattccaggcaccaggccgagtaaaccgagcacggcggcgcttaacaacataacgcttgggttactgaaaagctgattcaccatctgctcgccaacatcctgatcggtgctgacacgcgtaacgatgacccccgcggcggtagaaatcaccagcgccggaatttgtgccaccagaccgtcgccaatggtcaatagcgtataactttccgccgcgtgtcccatgctcatgccatgttgcagcacgccgaccagcaacccgccgacaatgttaatgaccatgatgaggatcccggcgatggcatcgccgcgaacaaacttacttgccccgtccattgagccgtaaaaatcggcttcctgagtcacttcggagcggcgttttttcgcctcatcttcaccaatcaatccggcgttaaggtcggcgtcaatcgccatctgcttacccggcataccatcgagaacaaagcgcgcacccacttctgcgatacgcccggcacctttggtaatgaccataaagttgatgatcacgagaatgacaaacaccacgataccgatagcgaaattgccaccaacgaggaagtgaccgaacgcttcgaccaccttccctgccgccgccgcgccggtatgcccttccattaaaatgatacgggttgaagccacgttaagtgccagacgcaacagcgtggtaaacaacagaatggtcggaaacgcagcaaactcaagcgtgcgctgggtaaacatcgccaccagcaacaccatgatcgacaaggcaatattgaaggtaaacaacaggtcgagtatgaatgcgggcagtggcagcaccatcatcgacaagatcaacaggatcaaaatcggtccggcaaggatctgccattgtgtcgatttcaggtttgcgggcaggcgcagcatcgcggccagattactcatgggtcggtttctcgttaataaaatccagggcttccggcaccggaagatgagtaggttgtacagggcgctgtccaccagccagacgccagcgtttcagttgccagacccaggccagcacttccgccaccgcggcgtacagttgacccgggatttgttgaccaatctccgcatgtcgatacagcgctcgcgccagcggcggcgcttcaagcgtcgggacgttattttcagcgccaatttcacgaatgcgcagcgcgaccagccctgcacctttagcgaccactttcggtgcgctcattttgttttcgtcatactgcaacgctaccgaatagtgggtcgggttattgacaatgacatccgctttcggcacatcggccatcatccgacgccgtgcagcagctcgctgcatctgacggatccgccctttaacatgagggtcaccttcgctttgtttgaactcatcacgaatatcctgccgtgacatacgcagctttttcaggtggctgaatatttggaaaaagacgtcaaatcccaccattggaatgacaccaagcaccaccagcagtgcgcatagccctaccaaatccatcgcattacccatggcggtaatcggagactcggccatcaagcgcatcatctgcggccagtgatgccagagaaaaaaccccgtcacgctgccaaccaggatggttttcaaaattgctttaagcaactccgcgccagtctgagccgagaacatccgtttaatgcccggtagcgggttgagtttggaaaacttcggctgcaaggatttgccgctaaataccagccctcccagcatgaccggagaaatgagcgccaccagcaccacgccgctaatcagcggcagcagcgccagcatggcttctctgatcagcagaataatctgcccgaggatcagattcgggtcattgataatactgtgatcaaaatgcagcccagcggagagcatgcccgacaatcgacgggccagcgacacaccgccaaaccagataacactaacgcccaccagcaaaatcagcagtgaggtcagttcacgggaacgcgggatttgcccctcttcccgcgctttttctagtcggtgaggtgtgggggcttctgttttgtcgtcgctctcgtcagacacgtcgccaatcctggaaagagtattaagcgtgaatgatgccagagcgcaaagcgttcaatggtttgagtaaggggcaaaacaggcgggatttagggcttttgctgccacacatcaagcatagtgtgcgtttgtcggatgcggcgtcatcgccttatcagaccgcctgatatgacgtggtcacgccacatcaggcaatacaaatcaaaatccaagactatccaacaaatcgtccacctgatcctgactggctaccacaccggctttgctggtatcgacctgaggtccattaagcaaactctggttttcacgttttggacgcgactcctgttccgggatgttttccaacagcaccatcagcaactggcgttcgatctcctgaatgacatccatcatccgcttaatgacctgcccggtgagatcctgaaaatcctgcgccatcatgatttccagcagttgcgcgttagtaaagctggtatgcgcgggtacatctgccagaaattgtcgtgtatctgttaccagttcacgggcgtcggcaaggtcaatcggatcggcaaaccagtcatcccaacgttgggttaacgcttttgctgatttctccatttgatcctgatgcggttgtgacgcctcaacactgttcagcgcccgctccgcagcctgggcggtcatctgcacaacatagtacaaacgatcgcgcgcatcggggatggcttccgccgcttcggcaatggcctgatccagccccagttcccgcaaactgtcgcgcagcatacgcgtcaggctgccgatgcgcgcaatgatatcgccagctgaatgctcgtcagcaggtttgattgatggttgcatcatagtcgcatcctcacatgcccagtttctcaaagattttgttgagtttttcctccagcgtcgcggcggtaaatggcttcaccacatagccactggcccccgcttgcgccgcagcaatgatgttctctttcttcgcttctgcagtcaccattaacactggcaatgccgacatcgcgccatccgcacgaattgttttcagcaattccaggccatccatattgggcatgttccagtcggagataacaaatccataaccgcctgcctgcaacttattgagagcgtcgacgccatcttccgcttcctcaacattattgaatcccagctctttcagcaggttacgcactatgcgtcgcatggtggaaaagtcatccacaaccaaaaatttaagttctttatccgccatttcacactcctgatttaaatacgtatcgcctgtccggcactaatttttgccaacatttgctggcttacctggctaagatcgaccacttcgcagacaccacccatattgatggcctcgcgcggcatgccgaacaccacgcaacttgcttcgttttgcgcaagggtccatgcccccgcctgacgcatcgccaacattcccgccgcgccgtcgttgcccataccggtcaggatcaccccaaccgcattacgccccgcctgtttggcgacagaatggaacaacacatctaccgaaggccgatgacggttaaccgccgggccatcgtgaattttgatttggtaatttgcgccactacgcgacagctccatatgccgatcgcccggcgcaatataggcatgccccggcaagacacgttctccgtcttcggcttctttaaccccgatctggcaaagcttattaagtctgtcggcaaaagagcgggtgaaaccgggcggcatatgctgggtaattaacagtgccgggctggaaagcggcaacggttgcagtacgtgacgaattgcctcagttccacccgttgaagcaccaatcgcaatcagtttttcagaactcaacaacggccccgccttcagcgttgtcggtgccgacaatggcttatgtgctgcaaggctcgcctttgctgccgtacgcaccttttcagcaatcatttcgttatacgccagcataccttcgcgaatacccagttgcggtttggtgacaaaatctatcgcccccagctccagcgcgcgcagcgtgacttctgaccctttgccggtcagggaagaaaccatcacaacgggcattggacgcaaacgcattaatttttcgaggaaatccagtccgtccatccgcggcatttcaacatccagcgtcagcacatcgggattgaatttcttaatcaagtcacgcgcgaccagcggatcaggcgcggtcgccaccatttccatgtcgctatggctgttgatgatttctgtcatgatctggcgcatcagtgccgaatcatcgacagataacaccctgattttgctcatcgttaatccttacttagcgcatacaccgtctgaccacgcagcgtgaagcggcgctcaaggtggctaaagttttcagagtgacccgcaaacagcaatccgtcgggtttaaggagcggaacaaagcggcgcaaaatctcctgctgggtagtttgatcgaagtagatcatgacgttacgacagaagatcgcatcaaacggccccggcacggtgtactgtttcgccagtagattcagcggggcaaaatcaacatagttcgccagctcctgacgcacgcgtaccagcccttcatgcggccccgtccctcgcatgaaataccgttgcagttgctgcggcgtcaggtttttcaactcttcatggcgatagataccgcttctggctttttccagcacttcggtgtcgatatcactggcaaacactttccagcgtccgggcgcggtgcccaatgtgtcagccagcgtcatcgcaatgctgtacggctcttcgccggtcgaagccgccgcgctccatacgcgatactcgccagaacggcgacgtgcgtgatccgcgagcagagggaaatgatgtgcctcacggaaaaatgccgtcagattcgtggtcagcgaattgataaacgcctgccactcaccgctgtgctgattagattccagcaagttcagataatgaccgaaatccgtcagtcccagcgaacgcaaacgacgaaccagtcggttgtaaaccatgtcgcgtttatggtcagccagaacgatcccggctcgttgatagatcaattgacttatccgccgaaaatgcgcgtcggaaagcgccaggcgctcggtcatctgtaacaataaagacgtttgcccacagggcagagatgaagtcatagcgccttctcaatcacttcaggataccactggcgcaatttgtaactgcaccgactcatgtcgtgctacttcatgttcttcaagggtaaataccgccacacgcgacgaaagatggtcggcctgattcgccagttgttccgttgccaccgccgcttcttctaccagcgaggcgttctgctgagtcacctgatccatctggctgacagcctgtgcaacctgctcaatcccccgctgttgttcttccgacgcagaggcaatttctcccataatgtcgttcacgcgggtcaccgaactgacaatatcgatcatggtcgcggcggcgttattcaccagtttcgaaccctgctggacacgattgactgactcttcgatcagccctttgatctcttttgctgcctgcgcgctacggctggcaagattgcgcacttcacctgccactaccgcaaaaccacgcccctgctctccggcgcgagccgcttccactgccgcattcagggccagaatattggtctggaaagcaattccgtcgataacgctgataatgtcgccaattttttgcgagctggtggcgatctcctgcatggtgtgagtcatggtactgacctgaacaccgcccgcctgcgccgttgtcgcggcattttttgccagttccgacgcctgtcgtgcgttatcggcgttttgccctaccgtggcggttaattgctccatactggcggccgtttgtgccagcgatgccgcctgctgttcggtacgacttgagagatcgttattgcctgcgacaatctccgcgataccaatgtgcatctcctggcttcccttacgcacatcacttaccgtcccacgcaaagcctgctgcatggtcttcagactggcaaaaatggcggtgatctcattacgaccatataccgcaatcggacgcgccagattacccgcagcaatgctgtcaaaatggctaccgataatggccagtggttgaacaatcatcttgcgcgtccaccacagcgcactgctgatgtagatcgccgcaacaataatcatgctgataaacaccagtgccgaaatctgatagttacgctggctttgcgcactggcggcttccagcacatggttgatctccagctgccaggcctcaaagttaacgtcaaacgcattctgtgatccctgcaccggcgcagtgaggaaatccgaaagttgattactttcaagccaggtcgcctgatgttcgagatcgttgtgccagcgggcaaaacttttctccgtctctttttgcaatcccctgacgtgctcgttgcccgcagtcatcgccataaaacttttaaacagcgtggtggattgcgtcagactggcgcgcgccgtcgtcatcaacgttttaatgtcatccgccggatagctaagtgccgtcagagtgcccgctttgttcagcgcggtactggcctgtaacattaccgcccgagtttgcgctaatgccgcacgttgctgattgctctgctcgacctgattcagtcgttgcaaatcgtcgcgaaatgcccaaaaagacatgccgttactgccaatctgcaagatcccgcagagaatcaaaattaaaaacagcgtggtcgaaattcgaatacgattaaacatcaacgctccccatcaggcggcaatgaccgcgttagtaaatactcgtcaaaatgtttcccagtttggatcttgttcagcaattcgcagtcgtggctgagccggtggttgctcactggcaggacgggatggtgtttgcggtttattggtgagtgggctggctgccagacggaacgcggaaactgcttgcgttaaacgactcgcctgttcttccagcgcagcggcggcggcagctgattcctgcaccagcgatgcgttctgttgcgtgacgcgatccatttccgaaaccgccaatgcgacttgatcgatgccacggctctgttcatccgatgccgatgcaatctcgcccataatgtcagtcacgcgagtgacagcattgacgatattgttcattgtttccccggcgctttcgaccagcaccgaaccggtatcaacgcgtgagacggagtcttcaatgagggctttgatctcttttgccgcctgggcgctgcgactggcaagattacgcacttcacccgccaccacggcaaaaccacggccctgttcacccgcacgcgcggcttcaaccgcggcattcagcgcgaggatattagtctggaaggcaataccgtcgataacgctgataatgtcggcaattttcttcgaactatcggcgatctcatgcatcgttttcactacgccatccaccactttgccgccgtgctgggcggtgtcggaggcactttgcgccagttgcgaggcctggcgggcgttatcggcgttttgcttcactgtcgcggtgagctgctccatgctggcggcagtttcttccagcgcggatgcctgctgttcagtacgggaggaaagatcggtgttgcccgccgcaatttcacgggtaccggcatagatggcatctgaaccttcgcggacatgagtgacggtgtcagtcaaagagcgttgcatatgtgaaacgctctgcgccaggtcgcccatttcactgcgcccgtcaatggtcagggtattcgccaggttaccaccggcgatttcgcgaatgtgagcaataatttttgccagcggagtaagcaacatacggcgaatgccgtaccacgccaccagcagaatcaataccaccaccagcgcgataaccgccagttgccactgggcaaatcggtaatcatctgcgttgtcagtgacgatatcgcgatacagtttttcactgctgagggcgtactgagcaaacgcttcgcccattgcattttgcattccctgggttggctgagcgaaataagctccagtattgccataatctagataatcaatcagttcagttaacgctgtgtaatagtttttatatttttcatcaatattacgactggtagcgaccatttcaggtaacggtgccatgcttttgaattttttataatgcgtcgctgcctgcgccaatgttttcctggcgctatcgagcaattcaactttggcgttactttgttgattggaggaatccatcatcatccgtaccgctgaacgactcaggttaatgcgcgtttgcagcattaaatcccaggttgacgtcagctcgccctgctgttcccgtaattgattggaaaccacaaagctcttctggctatggtgaagggaagaaaaaaacagactgccggaaataagctgtaacagtgcgaatacccccagcaccattaccaacagcgtgactacgcggatacggttaatcataaggcaccttcctgaaaacaagttgatctcgttatcggcaaggaggggggaaactttattgctgatgccacccgccgcgaaattgaaataaaaaacccgatgcgcagatcatcgggttcatttcaattgaggaaatcgggagaattacgccacttctgacgccgcgctatctaacagcgccatctcttcgctgttcagcagtttttcgatgttcaccagaatcaacatccggtcgcccagtgcgcccagtccagtgagatattctgttgaaagcgtcacggcaaattccggtgccggacgaatttgctccgccgtcaatgaaagcacgtctgagacgccgtcaaccacgatgccgaccacccgctgtccgagattcaggacgataactaccgtgttgtcgttatagtccacatccacctggctgaacttaattcgtaagtcaacaatcggcacaataacgccgcgcagattcgtgacgcctttgataaacgctggcgtgttcgcaatccgtgttacctgatcgtagccacggatctcctgcactttcaggatatcaataccgtactcttcatcaccaagggtaaataccagaaattcctggcctgacggctcgctggccagctttgttacattcgtcataccggtcatattgttacctttttactcattcaggcggcggtgttcgccatacgttgttcgcggtttatcgcctgcaaggcggagacatcaacaatcagtgccacgctgccgtcgccaagaatggtcgcagcagaaatgccggggactttgcgatagttactttcaaggtttttaaccacaacctggtgttgaccaattaattgatccaccagcaaggcgtagcggcgaccgccactttgtaagatcaccacaattccctgggtggcttcggttttcgcgcccgcgacgttgaacactttccacagttcgacgatgggcagatattcaccccgcacttccagcacccgctcgccgccggccagtggatggagatcggcttcacggggttgcagtgattccataacagcattcagcggcagaatgaaaacttcatccgcaacgcgtacggacatgccgtcgaggatggccagcgtcagcggcagtaaaatgcggatcgtagtgccagtaccctgcttcgactggatttcgacatgaccgcccatcttctggatattacgtttaacgacgtccatgccgacgccgcgcccggagacgtcggtgacctgctctgccgtggagaagccaggtgcaaatatcagcatcgcgacttcgtcgtcgctcatgttttcgctgacagtcaaaccttgcgaggccgcttttgccagaattcgctcacggtttagccccgccccatcgtcggtcacttcaatgcaaatgttgccgccctgatgttcggcagacagaattaaatttccgacgctgtttttacctgcggcgagccgtttttctggcagttcaataccgtgatcgaggctattgcgtaccaggtgggtcagcgggtcgataatgcgttctatcaggcttttgtcgagttcagtagaactgcccaccagcgtcagttctacctgcttgccgagttttcccgccagatcacgcaccagccggggatagcgactaaaaacatattccatcggcatcatgcgaatcgacatcactgattcctgcaaatcacgggcgttacgttgtaactgccccatgctggttatcaaatcaccatgattaaccgggtccagttcgctggaacgctgggcaagcatggactgggtgataaccagctcgccgacgaggttaattaattgatcaaccttttctaccgctacacggatgctggtggattcattgctgcgcgtcgttttttcccgctccacgcggccggttggcgcttgttcggctgccagtttaagcactggtggggtggatatttttggcgagacttctactgtttcaaaggtaatctgatcggcttcaatcacaaaacagagtaccgctgtgatgtcatcttcggcgatgtcgcccggtaatattgccgagagcgaatccgcccctttcaccacgtcagttaacgttgtcagatgtcccagttcttcttccagcaggtcgacttccccggccttcaggcgcgaaaggataattcgtcgcggcgactgactgcgactctgctcatcttgcggttcacttttggcaaccacacttaatcgggtcactgcggatggcgtttcgcctttcgcttctaatgccagttgacgcaaggcctggcagatataatcgaagctggcggcatccggctcttgcgactgtttataagcgtcgagctgttcttgcatgatgtccttcgtttccaaaaacagattgataatgtcggtgttgagttgcatctcacctcgtctggcttcatcgagcaggttttccatcagatgcgtggtttcctgcaaaacgctgaagccaaaagttcctgcccctcctttgatcgagtgggcagcccgaaagatggcattcaattgttcggcatctggcgcttccggctgcaaaaccagcaaatgctgctccatgtcagccaacagttcgtccgcttcatcaaaaaatgtctgataaaaatcgcttatatccatgctcacgctgtcacctcggttcggctgatggcattgtgggaacactgacctgtggtgcaacctcaggtttttccagggcgcttactggctcattctggctttcggcgttttcatgcaaaatggcctgttcggcttgtttgttcagtaccagcaggctgatgcgacggttgacggcatcatcaggtccgcgatcgcttaagcgcatcgttgccgccatgccgacgacacgtaacactttgccgctatccaaccctccgaccatcagttcgcggcgggatgcattggcccgatcggcagaaagctcccagttgctatatcctttctcaccgctggcgtaggggaaatcatcggtatgacctgaaaggctaatacggttgggaataccgttcagtacaggcgcaatggcgcgcagaatgtcgcgcatatagggttcgacatcggcactgccggttctaaacatcgggcgattctggctatcgatgatctgaatacgtagaccttcctggaccagatcgattttgagatggggacgtaacgcccgcagtttcggatcggactctatcaactggtcgagatcaccccgcaatttccgcaatcgactttgctccatgcgttttttcagctcttcgatgttcggctgcttattcacttccccctggctttgggtgtaatcatcaccaccgccgggaattgggctttcactattagaaatgcgatcgccgcccgtaaccgcagtcgccagtggagtccggaagtactccgcaatctgaatcagctcttttgggctggagatggagatcagccacatcaccagaaaaaaggccatcatcgcagtcataaagtcggcataagcaatcttccacgatccatgtgctgccccgtggcttttggctttgcgtcgtttgacgacaataatcggatgcgcttgattcttcatgcttcctcggttgtcgtctgttgttgcggatttttcaccgcacgcacatgctcttccagttcaataaacgacggacgttcgctggaatagagcgttttgcgaccaaactcaacggcgataggcggtgcgtaaccgttcagattagaaagcagagtgactttgacgcactgcatcattttgctggtttcggcgcttttctgacgtaaaacagtcgctaatggggaaataaatccgtaagccaataaaatgccgaggaaagtccccaccatcgcatgtgcgataagcgcacccagctcggcggcaggacgatcggctgaacctaacgcgtgaacgacccccattacagccgcaacaataccaaacgccggaagtgagtccccgaccagcgccagactgttcgccgggacttctgcctcgctttcgtgcgtctcaatctcttcatccatcagagcttcgatttcgaaggtgttcatgtgaccgctgataatcaggcgcagataatcgacgataaaatcaagcatgacgctatccgcgaggatgcgtgggtagctggcgaagatctcgctctcacggggattttcaatatcacgttccagcgaaaacatccccatctgccgcgatttcgccatcaaccgataaagcagagccagcagatccatatacattgctttggtgtatttggagcgacgaaacagcaacggcagcgccttcagcgtgcctttaatcgctttgccattattgccgacgataaacgacccaatccctgcaccggcaataatcaccagttcagcgggttgatagagtgctccaaggcttccaccggtcatcaaataaccgccgaaaactgtaccgagaacaaccaggtaacctaataagataagcacgacatcatccttccactgttgaccatgacaggatgttcagtcgtcaggcgttaacgcgcgattggggcaaaaaaaagcagcggtacgtcgttaccgctgctggaatgttgcgcctcaccgtatcagttaaacagcctgtactctctgttcatccagcagttgtgggataatatcggcaggattctgggaaagtttacgtctttttactgcccgggatggcggttgacataagctgcaggcaaagctgccaacaggctggtgagcgtgggtaataaaattgccgccgcagcagttgcagctggaaagttgcagtaatccactttcaacaaaccgcaccaatgtccaggcacgggttaatgccagcagtggtccttcttctgcttgtgggcactgttcaaggtataaacggtaggctttgatcaccgcatcgacgccattacacaaaccggttttcagtaaaaactgccatgcattacagaacatcgaagcatgaacgttttgttcccaggtcataaaccagtcggttgagaatggcagcatgcctttcggcggtgggcttccgcgcagttctttataaagttttatcaggcgtccgcgacttaactgtgtttcgctttccagcatctgcaaacgagcgcccagggtgatcaattccattgccagctgaatatcccgcgcttcctgaacaatgcttttttcactcatgatcaggcccttttcttgcgcagcgcttcttcaggctgattaacatcattcagcaagcgtgttgagagcatgatgccggtatgaatttgctggagatcgtcaacgcgggaatcttgcgtcaactgagtaatcgtctggtggctgtcaaaacggaagtgacaaaccagttgattggtttctgccagcttaaccatttgcggaagagtcagtgccgctaacgttgtcgccatttcttcatttatgccgagacgaaacatagcggacgctttgtcctgaacaatcaaacgctgtgcaagtagtaaatatgacaagttgatgtcataaatgtgtttcagcaactcggaggtatgcattattcccacccagaataaccaactttatttttatgcggtttcaccgcaccccgtgatgtcgccgggaagccccggtaaaaaataattagcattagaatagttgcgataagctgcaataagcagaaccacctttttggtttaatatgtccttacaaatagaaatgggtctttacacttatctaagatttttcctaaatcgacgcaactgtactcgtcactacacgcacatacaacggaggggggctgcgattttcaataatgcgtgatgcagatcacacaaaacactcaattacttaacataaatgtataagtcatacttttgttttgggtgtatttcaatctgttaaaaagtttttcgctacgctagcaagcaaaaatgaaacaggaataatcgaaatgggatgttgcgcacagtcaaaataactcaccgtaaataatcatctgctataaataatcactttcatgcaataccagataagctatttttaaacagacacttaccgcacaacaaactaattaaatacaaagaaaggcaacaatcaacttaatgttaatgaaatgttttacatatattaaccacttgtttaatgcggagaatcagtacactattttcttataattacatttgaaattatatgatcaccgggagtgattgattaattatctttactaataatcagactaatatttacctgtttgaccgagttgggattgcgtcgtttctccattaggagtaaagctttaatgtcacctgaagttcacagaataaggaacaggttatgagctatagcaatattcttgtcgctgttgcggttacaccggaaagtcagcaactgctggcaaaagcggtatctatcgccaggccagtaaagggacacatcagtttaattactctcgcttccgacccggaaatgtacaatcaattagctgcgccgatgcttgaagatttacgcagcgtgatgcatgaagaaacgcaaagctttcttgataagttaattcaggatgcggggtatcccgttgacaagacgtttattgcctacggtgagttaagcgaacatattctggaagtatgtcacaagcatcatttcgatttggtgatttgcggtaatcacaatcacagtttcttttcgcgagcatcctgctcggcgaaaagagttattgcctcaagtgaggtcgatgtgctgttagttccacttacgggagattaaccgctcctacgcaagctttggaaaggtagcaactttatcgcgctgctggctttccgcgcttcgcggaactatctgctttaggtcgctaatgaagcactcctgccagtggttaatatcgtttttcacgataacgtccagcatttctgcatgacgggaaatacgttccgccagcgacatagtcaatgcacgatccagcgcagctgcaacttcgtcacgatcgtaggggttaacaattaacgccgacgttaactcgtttgccgctcccgcaaattgcgaaagaacaagaacgcccggattggctgggtcctgagcagcaacatactcttttgctaccaggttcatcccgtcacgcagtggcgtcactaagcccacgtcagagtagcggaatattttcatcagtaatttacggtcaaaatgctgattcaaataataaagcggcgtccagcctaattgcccgtatttaccattaattcgtccagcttcattttcgagctgatgacgaatatcctgataggcttgcacatcaccacgcgacgttggtgcaatctgggtataacgaattttaccatgatgctgcggatatttttccagcaacgcttcataggcgagaaaacgctctggcaaacctttggaataatccagccgttcgacagaaaagatattttgtacgtttttcagttccgctttaagttgcgccagttttggcggcagtggcccggcagcctgtttggctatttctttcggttcaatgccgatcgggtagacttctgttcgaaatgctttgccccaggctgtatggctttttgcgctacgtgtcgtgacgcgggtcaggttagaaagacaatccaggaacgccagacgatcgttttctgtctggaaacccagcaaatcataatcacaaagctgttcaagcaaggtgtcatatgtcggcagcgcgttgaagatttccggtgtcgggaaaggaatatgcagaaagaaaccaatgcgattattcactccccgtttgcgtaattcatgcgcaaatggcaacaggtgataatcgtggatccagataatgtcatcgtcttgcaacagcggcagtaatttatctgccagcaacgcatttacgcgtagatagccgtcccaggcaggacgctgaaattgcaccagatcgagccgataatgaaaagcgggccagagaacggcattggagaattggttgtagtattcgtcaaggtcctgttcgctgaggttaaaagaggcccacgtaatgttaccttttttcaccttttttagcggctgatcctcattccctgtttcaccactccagccaaaccacagtccgcctgcggctttcagtgcccccagtatgccaacggcaaggccaccggcactggcggcgtgctcgtctggtggtgcaatccggttagatactacgactaaacgactcatagtcatcactcctgttattttctcttttttgttgtaatgcggtggttatcatttcaagccagctccagacatccggcacacccgccagtcgccatgatgcctgagttgcacctgtgccaatttttactgacattccgcccagtcggttaacgactgcgaagccagattcatcggttaaatcatcgcccagaaatacgggcgttcgcccgataaagggagcttcctgcataaaagctgcaattgcctcacctttactggtacctctcggtttgatctcgacaacacactttccctgctgtaacgccatttgtggccagatctgagtaatacgttgcgctaatgtcattaatgcgtcttcatgctgcggagcctgacgataatgcagcgcaaaagccatccctttcgcctccagctccgcgccgggatactgagcgatgactgtatgcagttgcacgctaatatcacgcgcaatcgcatccggcagatgaacgatatgtgttttaccattgatgtcacggcgctccgccccatgcacgcccgctaacgggaagcgataaggttttgccagtgcgtcaagctccaccattgagcgccctgatatcaatgccaatgcaccatcacttgcggttgccagtagctgtagtccttgcagaatattgtcaggcacgacgacctgatcgggatgcggtttgatttccgccagcgttccatcaagatcaaaaaaccaggcatatttcgcggatagttcaggggtttcggttaacggttctgtcacccggttctcctccttctcttttcttattgtgttgcgcagaacgcgctttacagacatgtaagtatagacagtgtgacgggggtcgccatttgcaacgaagaacagccaaccgttatggcggttggctatggtgggaaaaaacgctaaattgttgcagaaaaaagcatcagacagtgcgtttcgctttttgcttgtaacggtcgaagatcaccgctgccagcaggattaagccgcgaaccacgtactgcgcgaaaggagaaatattaagcaggttcatggcgttttccacggtgcctaaaattaagatacccgccaccacatatgagatttttccgatgccacctttcagagaaacgccacctaaaacgcaggcggagataacaatcagctcataaccaatcgacgtcattggctgcccactggtcatacgtgaagccagaataattccggctatcgctgataccaggcctgagagaacaaagataataattttggtgcgaacaaccggtacacccgccagacgcgcggcctcttcgttcccgccaatcgccagggtgttacgaccaaaggtggttttattcagcagcaaaccaaagataatcagacacgcgacggtgagccagattggcgcaggcagaccgaaccagttggcgtaaccaagggcaaagaagctttcatcttcgataccgaccgctttaccgtctgaaatgatgtacgccagacctcgaacaatctgcatcgttgccaatgtcgtgatcagagcatttattttcagtttggcgataacaaagccattgaccaggccacagagaacgcccagcaacaaccccgctgccacgccaatccacaggctttcagtcaggttaataaccaccgccgtggtgacacccgcacaggcaattacggaggcgacagaaaggtcaaagtcaccggaagcgaggcagaacaacatgccacaagccaccatccccgacatggaaattgccaggcccaaccctttcatattaatgaaggtggcaaaatttgggacaaaaatggcacaggcgataaagagcaccgcaaacaccaccagcatgccgtactgatcccagatacgcccgaagctgaatgacgacttaggtgcgccagaccccgatgtagaaacagaagacatcatactctccttactcaggcaacagcctggctgactttaggcatcgcaaggctcagtgcctgacgctcatctgcctgctcgtgtaacaattcaccggcgatttcaccttcccgcatcaccacaatccggtcggcaacgccgaggacttcaggtaagtcgctggaggcaaacagcaccgccacgccctgcgccgccagcgcataaattacgttatatatttcgtgcttagcgccaacatcaatgccgcgcgtaggttcatccagcaaaatgaccttcatctcttccgataaccagcggcccagaatggctttttgctgatttccgcctgagagattcatgatcagttgctccgcgcccggcgttttgatgttgagcgaacgaatgtggtgatcggcattgttttcttcccaaccgttgttgattacacaaccgccgagcacatgtttacgtctggcactgatgttgatattgtcgcgaacggagtgcacgggaataatgccttccgctttgcgatcttccgggcagagcatcatgcctgcggcaatggcgtggctcggtttacgaatatcgatcggctgttggtcgatataaacctgaccggcggtgatttgcgtcccgccaaacatgcctttcattaattcgctacgccccgcccctaccagaccaaacagcccaacaatttcaccactgcgaaccgccagacttattggcgtacgcacgcctggtgctttcacagcatcaagacgtaggcgctcctcgccataactacgcggttgccagccgtagatatcgccaatgtcgcgcccgaccatcgcctgcaccagcgcgtcgtggtcaacctgctgcatatcggtaaaggttttgacataacgtccatctttaaagacagtaatggcatcgctgagggcaaatatttcttccatacggtgagaaacgtataagattacccgcccctcttttcgcagttcacgaataacgcggaaaagattgtcgatttcacgggcagagagggagctggttggctcatcaaaggcgataattttggcgttacgcgccagcgctttggcgatttcaaccatctgccactgaccaatggagagatatttcagcggcgtgtccgggtcaatatccataccaagatgtttaagttgtaaacccgcctcataattcagcaatgagcgattcacaatgccgcctttatgcggcagctggccgagatagatgttttccgcgacggtcatttccggcacgagatgcagttcctggtaaataatcgccacgcccgcgttaagtgctgcggtcgtgtcggaaaaggacatttcctgcccattaatcactacagaacccgtggttggcgcatagttgccgctgaggatttttaagagagttgattttcctgcgccattttcacccatcaacgcatgaacctgaccggcatagcagtcaaaactaatatccgtcagcgccttaacgccgggaaacgttttaccgatgccgcgaaatgagagatacggggtagactgttgcataacgtctccgtgaatcactggtcgttcacaccccctctgcatcatgcagaggggaatttttccggcaaattacttaccgcctaaaccttttttctccagttcttctttaaagttgtcacgcgtgatcagtaccacgtcggtaacttcggtaaattttggcggttcaacgtcttttgctacccagttgtaaagcatttcgctggatttatagccatgtacgtccgggcttggcagcagggaaccgtagaagccggttgcctgtgctttagacagttcgctcaccgcatccacaccgttaatgccaatgccgatgatatcggccgctttaaagccctgaccttccgtcgcgcgtacgccgcccagcacggtgctgtcgttcataccgacgatcagccaatgtttaacttccggatgttgaaccagcattgagttggcagcgtcaaatgcccccgggatgtcgttagatttggtaggtacctgataaatttgtttttccgggaatccggccgctttcagcgcatccatagatcccgtagtacggcggcgggcggtatccagttcgttggcggtaatcgccatcaccgcgctttctttgacatcccagccacgtttctgcatctctttatacagttcctggccctgacgttcgccaattttagtcgccgccatcatcaccagcggaacggtatccattggcttacctttggcgttaacaaactggtcatccacggcaatgactttcatatcgtagccacgcgctttcgcgacgatggcagagccgagtttggggtccggagtacaaataacgaaaccttttgcgccactggcagccaggctgtcgatcgcgttcaatgttttttcgccatccggcacggcaatcttaataacctcaaaccctaaatccttcccggctttatcggcaaacttccattcggtctggaaccacggctcttccggttgcttcaccagaaaaccgagcttcaggttctccgccatagcggattgtgacataacggctgccagaccaatggctgccagggctttagtaaatttgtgcatggttctctccagctttagtgtcgttttgtgtagggcaaaaacgaatgacattcgttaaattaatcggaaaacaaagcattaccttttaactaaaagataagtgactgtgttgacatagttttagcgagaaattaattctccataggagagcaatatcacatcgcagaattacagtgagaacgtgcataaatttagcgggaaaagacataagggaaagccaatttgtcagacaaattgtcgaatgcacagcagattaatccataagattagcctggaaatccttgttgtctttggtacccatgcgggatgtcttctttttaaccagtcaataggccgcattacctggcgttgagtttttgaaatggtgtaataaccgcaactcaaagatgtggaaaatgcacgtcattcatttcgtcattaattatcactgtgctcattaattaacagaacacgtataatgagagccatctcgcaaaaatgaaaaaacgttttataaaatcatcacttcatcatgaattcaaattcattgattaatatcaacaagatacaaaaagcactatcattaaaattcattgcagttacattgatttcatcaatgaaatgtaaaaatatataaacttgatgatttaagcattttcttatacccgttcagacgttattcttatttcagatcatcgtcagaattgactccacgatcacatttcggaccggcagaaaggaattattctgcaaacagtaattatggtgttttgatttatcttgcacctctccacttctggatataaggatattaggtatggcaaccgctggaatgcttctcaaactcaactctcaaatgaaccgcgagttttacgcatccaatctctaccttcacctgagtaactggtgttctgaacagagtctgaacggcaccgccactttccttcgcgcccaggcacagagtaatgtgacccaaatgatgcgcatgtttaactttatgaagagtgtcggcgctacccccatcgttaaagccattgatgttcccggtgaaaaactgaactctctggaagaactgttccaaaaaacgatggaagaatacgagcaacgttctagtacgttggcacagttagccgatgaagcgaaagaactgaatgatgattcaaccgtcaatttcctgcgcgatctggaaaaagaacagcagcatgatggtctgttgctgcaaaccattcttgatgaagtgcgcagtgcgaaacttgcgggtatgtgccctgtgcagaccgaccaacatgttctgaatgtcgtgtcacaccagctgcattgatcatcatcggcgctaatgcattgcgccgatgaaggttttgagaaaccgctgcctcatctgtttgaagcagcggtttttttaatgggattcaccctgtggggtaaacttgagttcaataagcgcgatggctttttggattgcccgcatggtgaccgggtctgcggcggcgggatggttagtaaagtcgatattcttcagctgactggacattttttcacgaacttcaacgggcgcgattacatcgagaacatccagaatttgtttgataaccaactggcaagcaaccacatcagaaaccaattcctgatcggcattcagcggctgggacatcgtaaactcctgatagcattttgaaagccgttatagtagcgacttcacatcttcagcgatagtcacatccaccgtcatcaggacacaaaaaaacctgccggagcaggttttttgttatcggaacatattgcctggcggtacgtctttgaacgtcttgcaatagttattgaacatacttttcaggattttgcgcagtttcatcgcggcactccgaccatttgttatacaggtgttattgtctttgcgcttataatatgacaaccatcacaaaaatcaatctttatgtgatacaaatcacataaatacccctttaatgttataaaaatgataatcaaaaaacagcccccctatttctgacacctacagatggcaagaaatagcgcctgccaggcgtcttttccggccattgtcgcagcactgtaacgcgtaaaatagtgctttctcttactcttctggctggaccatgagacttctgattctgactctttcattaataacgctggcggggtgtacggttactcgccaagcccatgtgagcgaagttgacgcggcaacaggtattgtacggttagtttatgaccaggcttttttgcagcatgcccataccgatcgttatgtcagtcgcgggatcgccgatcgcgcatgccagcaggaaggctatacccacgcggtcccctttggtcagccagtaggcaactgtagcctttttgcgggttccttatgtttgaatacggaattcactttgtcatatcagtgccatcattccgccttccctgtctttctctaaatattttaatcagcgaggggatcttcgctgattaaagaaatagcggtaatgcgttttattcccattcgtatttttaataattgaagtttatattttaccttttgcaaataataaaataacaaattatagtgacgccacagcaacaaatataacctttgtggagcactatcatgctgaaaccagaaatgattgaaaaacttaatgagcagatgaacctggaactgtactcttcactgctttatcagcaaatgagcgcctggtgcagctatcataccttcgaaggtgctgccgcgttcctgcgccgtcacgcccaggaagagatgacgcatatgcagcgtctgtttgattacctgactgataccggcaatttaccgcgtattaataccgttgaatctccgtttgctgaatattcctcacttgatgaattattccaggaaacctataaacacgaacaattaatcacccagaaaattaacgaactggctcatgctgcaatgaccaatcaggactacccaacatttaatttcctgcaatggtatgtttctgagcagcatgaagaagagaaactgttcaaatcgattattgataaattaagcctggcaggcaaaagcggcgaaggtctgtattttatcgacaaagaactctctaccctcgacacacaaaactaatgctctccggcggcaggtttactgccgccgtttcaaatcagtgacggcaaatcttactctgatcggtcgaaaaaccgtctttcgaaggtataaatttgccttttgctgccagaaacgctaccagctctcccgctgtcatcccttctgccgagcaggtgtgaaaacgtgcctgttcaccaaaacgcgctttaatcgcagcttccagactggcatgcgtatattgctcgcctgattcaatcatcatatttaacacttcatgaccgtgaatagagtccatcgtccctcctcaaaaaaagcctagcgtagcgattgccgcttatgaagactttgcgccagcgcaggactgaatgctttttattgtacatttatatttacaccatatgtaacgtcggtttgacgaagcagccgttatgccttaacctgcgccgcagatatcactcataaagatcgtcaggacagaagaaagcgtgaaaaacagaaccctgggaagtgtttttatcgtggcgggaaccacaattggcgcaggcatgctggcaatgccgctggctgcggccggtgttggttttagcgttacgttaatcttgttgattgggctttgggcgttgatgtgctacacggcgctattactgctggaggtgtaccagcatgttccggcagataccggtctgggcacgctggcaaaacgctatctgggacgctacggtcaatggctgacgggcttcagtatgatgttcttaatgtatgctctgactgcggcatacatcagcggtgccggtgaattgttggcctccagcatcagcgactggacaggtatttctatgtcggcaaccgctggcgtgctgttgttcacttttgttgccggtggcgtggtttgtgtcggaacttcactggtcgatttatttaaccgttttctgttcagcgccaagattatttttctggtggtaatgctggtactactgctgccgcatattcacaaagtgaatcttttaaccctgccgttgcaacaggggctggctctgtctgcaatcccggtgatttttacgtcgtttggttttcacggtagcgtgccgagtattgtcagctatatggatggcaacattcgtaagctacgctgggtgtttataatcggtagtgcgatccccctggtggcatatattttctggcaggtggcgacgcttggcagcattgattcaacaacctttatgggattgctggctaatcatgctggattaaacgggctgttacaggcgttacgcgaaatggtggcctctccgcatgttgagctggcagtgcatttatttgctgatttagccctcgccacgtcatttctcggcgttgcgttaggcttatttgattatctggctgatttatttcagcgttcaaataccgttggtggacggttgcaaactggtgcaattacgtttctgccgccgttggcgtttgcactgttttatccacgaggatttgtgatggcgctgggttacgccggtgtggcgctggcggtactggcattgattatcccttcgctgttgacctggcaaagcagaaagcacaatcctcaggcgggttaccgggtcaaaggtggtcgtccggcgctggtggtggtgtttctctgtggtattgctgtgattggcgtgcaatttttgattgcggcagggttgttaccagaagtggggtgatcagatagcctcaaattccttattgggtgccagaattaacgctgacacccaatttggcctcttaatgcaggcagcactgcttaaatttcttaccactaccgcacgggcaaggatcgttacgccccggtttctcttctgctttgatcggttgctgaacagctttttcctgcggatgcgccatccagtacgcatgtagatcaagcgccgccagtcgaatggcatctacgctctcttcaaacgcttctggcgacatcttttctacccgctcgaagttttcctcagtaccgtgcagcgcaatcgcctccagcgctggttttaacgaatcgggcaacgttgaccagtcagaaagtgccacgccccgcatatagccaaagcaccactcctcaacaatcgtcagctcgctgccatcaacttctcgcaagccgaataacggctcaaactgctccgggaattcgttcagacgctctgcggtatcggccatatgttgaaaagccagattcataaagcgcgtcatctctttctctgacgcccagcgcggcacatagtcagccccaccccacacggcaaccagccactgttccggttcaatctcttgcggagaactcaacaccgccgtcaataaaccgtccagctccgccacatcaaggatggcgtggtcagtgttgtatttggtcagaatatcgtccagccattccaactcactttcgtttaacggtcccgttttcatacgcttttccttgtggatctcaactcgccagcacctatcttacatgccggtccgtatcagagatactttttgagtggctttgctggtgattaaaaattaaggagggtgtaacgacaagttgcaggcacaaaaaaaccacccgaaggtggtttcacgacactgcttattgctttgattttattcttatctttcccatggtacccggagcgggacttgaacccgcacagcgcgaacgccgagggattttaaatcccttgtgtctaccgattccaccatccgggctcgggaagaaagtggaggcgcgttccggagtcgaaccggactagacggatttgcaatccgctacataaccgctttgttaacgcgccaaattcttcaggcctttcagccagacatccgcttgacgccgatgtcttttaaactggagcgggaaacgagactcgaactcgcgaccccgaccttggcaaggtcgtgctctaccaactgagctattcccgcattcatcaagcaatcagttaatcacttgattttattatcgtctggcaatcagtgccgccgttcgatgcgttgcattctacttacctggcgcgatgagtcaacgatatttttcaccacttttgatcgtttgctgaaaattacgccgaaacgatcactgatcaagcaaatctgcacgcgcagcgctcaaatattgcaacattgaccacagagtcagtaccgcagccacaaagaaaagtgcaataccggcgtactcaacccaaatgttcggacgccacagcagccatgccaacgccaccatctgggcagtggttttcactttcccaatccaggagacggccacgctactgcgtttacccaactccgccatccattcgcgtagcgcagaaataataatttcacgggcgatcatcgttgccgccggtaatgtcacccaccagctgtgataatgctcggttaccagcaccatggcgatagccacgagaactttatctgccacagggtcaaggaaagcaccaaaccgggtactctggttccagcggcgtgccagaaaaccatcgaaccagtcagtcaccgccgcgacgcagaaaatgagcgcggcggcaaacggcgaccaggtgacaggcagataaaagaccaatacaaagaatgggataaggatgacacggaacagtgtaagcaacgtagggatattaaattgcataatgacgggtaactatctgttgtcagtaagattacccctatgttgctacagagacatcaatgtttcaacgaccagaagatcttttctgccagaccttgcgaaatacccggcacttttgcaatttcctcgacgctggcgttacgtaaaccttgcaaaccgcccatatatttcaacaacatttgccgacgttttggcccgacgccttcaatggtttccagggaactggtatttttgaccttcgcccgttttttacggtgcccgccaatcgcgtgatcatgtgattcatcgcgaatatgctggataacatgcagcgcgggtgaatctggcggcaaactaaatccctcaccttccggctcaaagaacagcgtttccagtccagccttacgatctgctcctttggcaacgccaagtagcagcggatgatttttatcccatgagacatccagttcggcgaagacatttttcgcctgcgcaagctggcctttgccgccgtcgataaggatcacatccgggatcttactgtcgtcaatggctttaccataacgccgacgcagcacctgattcatcgccgcataatcatcgcccggcgtgatgcctgtaatgttatagcgccgatactccgcacgcagcgggccgttagcatcaaacaccacacaggaagcgacggtttgttcgcccatggtatggctgatgtcaaagcactccatccgcttcacttccggcaatttcaacacgctggcaagcgcggtcagtcgctggtgaacggtagattgctgcgaaagtttgctggttaaggccgtcgccgcattggtgcgcgcgagtttcagataacgcgccctatcgccgcgaggtttggtttgaacattaatcttgcgtcccgccagttctgaaagggaatcggcgagcagcgttttatcgctaagattaaaatcgagcaggatctcacccggtaaggtgcgcatctggctgccttgtaaatagaactggcctacgaaggtttctaccacctcgctcagttccgtaccgccaggcactttcgggaaatagctgcggctgccgagcactttgccctgacgaatgaacaatacgtggacacaagccatgcccgcatcgaacgccacaccaataacgtcgaggtcgtcgccggtattggaaacgaattgtttttcggtgacgcgtcgcaccgcctgaatttggtcgcgaatacgtgcagcttcttcaaactccagattctggctggcagtttccatacgactaatgagttgcgtaagcacctgatcatctttgccagacaaaaacaggcgcacatactcgacctgctgagcgtattcttcttcactcaccagtccttcaacgcacggtcccagacagcgccctatctggtattgcagacacggacgcgagcgattgcgataaacactattttcgcactggcgaatggggaaaatcttttgcagtagcgccagtgtttcacgtacggcatagccattcgggaacgggccgaaatattcacctttggcatgcttcgcaccacgatgcatcgccagacgcgggtgggtatcaccactcaggaagataaaaggatatgatttatcatcgcgtagcaaaacgttgtaacgcggctgatagagtttgatgtagttgtgttccagcaacagcgcttcggtttctgtgtgagtaaccgttacatcaatttgctggatctgggcgaccagcgcttcggttttgcgcgaagcgaggttgctacggaaatagctggaaagccgttttttcaggtctttcgctttgccgacatagataaccgtaccaccagcatcgtacatgcgataaacgcctggctggctggttacggtttttaaaaacgcttttgcgtcaaactgatcactcactgacttgataatgtctccgcattacacagaccatggcgaattgccaggtgagtcagctcaacatcgccatgaatgtttagtttactgaacatacgatagcggtagctgttcaccgttttcggactgagattgagctgttctgagatctcattgaccttctggcccttggtgatcatcagcataatctgcaattcacgttcagacaaactggcaaatgggctttctgttttttctggttcgatctggcttaacgccatttgttgagcgatgtcagaagcaatgtaacgctgccctgaatagacagaacgaatcgcactcacgacttcctgcggagccgcgcctttgctgaggtagcccgcagcaccggcctgcatgactttcgctggtaaagggttttctgtatggacggtaagcatgatgattttgacatcagctgtggaacgcgcgattttacgcgtcgcctcaagaccgccaatgcccggcatactcatgtccattagcaccacgtcaacggcatttgtccggcaccacttaacggcgtcttcaccgcacgatgcctcaccgacgacttttataccctttatatcttccagaatgcgtcgtatccctgcgcgcaccagttcgtggtcatcaacaagtagaacgttgatcaaaggaatatctccagaaatagggataacgctactgatagttagtcattcgtatattagcggtttttattgcaactttgaaacgttaaaaatggtgggtattcgatttttctctcgtttttgtcaattcgattgtccacagttatggtcacgcccgtcaccaacggcttaccggatcgtttcacagtaagccctacgatgaaatgtgacaaaaattgactttattcagcaaaaatgaaaatcagcccgctgaatatgtaacattaattaacccgaacaatacgggcaaaaaacattcatgataaaaatatttattggtcattatattaacgtattttatagcactgccgatatcacgctcaaaaaacaaccactgctatttttagcaaagcttatggtatactccgccgccttaacatttttcaccgcaaattttcattgcaacatgacgaggaaaataaatgagtacgcctgatttttctactgccgagaataatcaagaactggcaaatgaagtctcctgcctgaaagcgatgctgacgctgatgctgcaggcgatgggacaagctgacgcgggccgcgtgatgttaaagatggaaaaacagcttgcgctgatcgaagacgaaacccaggctgcagtattttccaaaacggttaagcaaattaaacaagcctaccgtcagtaatataaaaccggctgatagcgtgcctttcagccggtttttgcatctggcacgcaggacagaaaagagatcaaattaagccagtagcggccgcgtaacaggcaacctgggtcttatttggtgcattaatttttttctgcatgtttttctggtggaaattgaccgtattctcagagattgacaaaatcatcgctatctctgctgatgttttcccttccgccgtccacctcagaatttctttttcgcgcttgctgaaattcatctctggcgtcatcactatttcatcatttaaacgcatcagagccatcagactttcgcgcaccagtaactgcatttttaattgcagttcatcactaagaatgggtatttcgcgcgcgctgcaacgggaaaaggacaaaaagcccagcgcccggtttggcagcattaaatactgagtgacaccgcggcgtaaaccatgtgcgcgcgcggcttcccataacggctgtgcttcgctgaataagtcatcattccacattaaatggccctgactaaagttttcagggttcagcaccggatcaattgcgagaaagttttttgcctgataataactaacccacgcctcagggtaattggtgtaaaaagccactttaggtcgagtgaatggtaccgggtggcggacacataacgaatagtaatcgtactccagctgctgagcctgaagctcaatttcatggtagacctcttctgcggtctccatcctctgaaaacgcaacagcatcgtgcgacgccagctgaaaaaatccttatcctgcatagtaaaccgcaacgcccctgagagtgagtatcatttataatgataattcaaactatcacataaataagatttatatataatttatattattcaggcaatgaattacttttgcaagccatcgcattctcttatgttattaatgagttatgctgatttgttaagcagttttatcaggcttgaaatggcgtccagccccgacaggtgaatcgtcggggctgattttttcttattattgcagcagaaacttctcgaggaactggcgggtgcgaggctgctcggggtcggcaaataacgcttttgcggccccctgctcgactatccgcccctggtccataaagatcgcccggtccgcaacatcccgggcaaagctcatttcgtgcgtcacaatcaccatcgtgcgcttttcctgcgccagctgacggatggtgttcaggacttcacccaccagctctggatccagcgctgacgttggctcgtcaaacaaaatcacctcaggacgcattgccagcgcacgcgcaatcgcaacacgctgctgttgaccgccagacaaacgacgtggatagctggtttctttacctgccagcccaacttttgccagcagctcgcgagcgcgcgccgtggcctcttctttcggttcacctttgacgatcaccggcccttcaataatgttctccagcaccgtacgatgcggaaacaaattaaagttctggaagacaaacccgacgtgctgacgcaactggcgaatcagagatttttgctgacttaatgaacgtgcagtatcaatagtgatatcgccaacggtgatcgttcccgcttcgggttgttccagcagatttatgctgcgtagcaacgtggttttgccggaaccactcggaccgataattgccaccacttcgccaggctttacctcaaggtcgataccgtgcagcaccgtctgaccgtggaattttttcaccaggttcttaacttcaatggcactcattttggttctctctcctggcgattaagttgattctcaaaatggttctgcaacgtcgataacacagtcgccatgatccagtagatgagcgaagccgccagatacatggtgaacacctccagcgtacgcgaggtaatcaactgcgcctgacggaacagctccggcacctggattgtcgcggccagcgacgtatcttttaccaggctaataaagctgttcgacagcggcggcaacgccacacgcgccgcctgtggcaaaatcgcgcgacgcatggtctgccacggcgtcataccaatactggctgccgcttcccactgacctttatcaatagaagaaatggcggcgcgcagcgtttcggcagcataggcggcagtgttcaacgacagaccaatcattgctgacggaatgggatctaattcgataccaaactgcggcaggccgtaatagatcataaacagttgtgcgatgagcggcgtaccacgaaaaatagagatataaaaacgcgccagccagcgcacgggccagattggcgacagacgcatcagcgcgagaataaacccgagcagtaagccaaaaaacatgccgccgatactgagttgcagcgtatacccagcccctttcagcaggaacggcaaggaatcaataaccagttgtatactttcttgcatgagcgtttccggagctaaacgtggggatgataggcgaacagcgcaggcgcaccgccggtatgaataaacagaatcggcccttcatctttgaagcgtttctgactgataccgtcaatcagccccgccatcgcttttccggtatacacaggatcaagcagaatgccttccagccgcgccagcaatttcactgcttccatgccttcgtcgttcggcacgccgtagccaggtgcaaaatagtcatcccagagtaaaatttccgctgatgcggtcagctccagttctttcgcaatcgcctgttgtaggttaaccactttcggcaattgatcggcaacggaacgcgacacggtcacgccaatcagttcgctttcaggcatcaggtgttccagcccaacagccagtccggcgtgagttccggcactgcccgatgcgactaccaccgatgaaatattaaccgccccttcacactgttgcgcgatttccagcgcactctccacataacctagcgcgccaagagcattagaaccgccaaccggaatgacatacgggcgaaagccttgtgcttcgactcgcgtcgccagctcttccagttgggcattgggatcggtcagtgcgtcgcacatttcaatctgggtattgaacagatccagcaacaagcgattgccgttggttaaatagttttctgcggttgtgccaataggattttccagcagcgccacgcagtgcagaccgagtttggcagcgactgcggcagtctgccgcacatggttagactggatcgccccggcagtaatcagcgtatcggcaccttcacgcagagcatctgccgcgagaaattccagcttacgtaatttattgccgcccattgccatgggggtgacgtcatcccgtttgatgaaaatttcccgtcctagataatcagaaaagcgcggcagatattcgagcggcgttggcgcgccgataaactccagccgtggaaaacgggttaaattatgcagtggcataacagcctccgatgtgtgttgttgtgattttcttattatgcacgctgaaaacgcgtaaataaaaaaggcgctagtgaaagcgcccttttttgtcattatgctgattatttggtcacatcagcaccaaaccatttttcggaaagggcttgcagagtgccatctttttgcatttccgcaattgcatcattcactgctttcagcaggtcctcatttcctttacgcagcgccacgccagactcctgacgggagaatgcttcaccggttactgccagcgtatcgttggttttcttcaccagatccagcgccgccagacgatcaacgaggatcgcatcgatacgccctacgcgcagatcctgatatttggtcgggtcatcatcataggtacgcacatcgacgccctgaacattctgccgcagccactcttcatagttggtgcccagaccgacccccacttttttgcctttcagatcatcggctgttttaatggtgccttcgttaccttttttcaccagcgcctgaataccagaaatggtgtacggggttgagaaatcgtattttttcttgcgctcatcagaaatggtgacctgattaatcaccacatcaatacgtttagagtccagcgacgccagcataccgtcccatttggtcggttttagtgacgcctcaacgccaagatgttttgccagctgttgggcaaattccacttcaaaaccggttaatttgccgtcatctccctgaaaactgaacggcggataagttccttccagccctaccagcagcgtgccgcgctctttaactttattaagcagaccttcatctgcaaaacttttaacgctcatgcccgcaaccagcgccacggccatcacacccatcaatgcctgacgtcccagatgtgctaatttcatattcaccccgaatgttgttatgtctgtttgcagtgtagagccattgtttgtaaacacaaaaacaactccgctacatcttattcttatttaatatatatcagaagaaggcaggctggaggatttctgcacaagtctggtacaggtttggcgctgatagtgttgatacttccgtaacgcgatgcggtaattgttggtgctggtggtgggcagccacggggcgaggatttcatcaaggaaaccgtcctgcagctgatcgagggaaatattttgctcgtgtagatgattccccaaacggcgcaaacgaacgacatattcacgcaccgtacctgggctcatttcagtttgctcaaaaagaaattgcttaaagccgataatatcgaaaaaatcactctgcgttttgcaatgtaaatcaccgcaaaatcggcacaatgccgcccatgatttttgttccgtttgccagccattttcatcaagcagcgtgtccaggcgggaaatctcgattttattcactattttgccgtcgcgaactaaggtaatgcgatcgagtaatttacggcaatgcgcgcaatgggtctggctgtgtttaaagtctttaagatagcggcttaatggccgtcttttcaggtgctgcaccatcattaagaactcctggtagtcaaagttaaagtgcggcatttactgacgttataacttacccagtttagtgcgtaaccgtttaatagcctggctgtgtaactgactgacccgcgattccccgacctccagcaccgcgccaatctctttgagattcagctcttcctggtaatagagggttaataccagtttttcgcgctccggcaacgtttcgatggcttccatcacccgctggcgcagattactgtccagtagttgttgtagcgggttttctcgctgatgatcatcagtaaccagttcgatgctatcgccgtgctcttcgcgccactcatcgtaggagaagagctggctgttattggtgtcgagcaacatttggcgataatcggcaatatcgatccctaaacgttccgctacctcagtttccgtggcgttgcggccaagttcctgctccagttgccctattgcctgtgccacttcacgcgcgttgcgtcgcacgctgcgcggcacccagtcacggctgcgaagttcatccagcatagcgccacggatacgctgcactgcgtaagttgtaaatgccgttccttgtagggcgtcatagcgttcgacggcattaagtaacccaatgccgcccgcctgtagcagatcgtcaagttccacgctcgcgggcagtcgaacctgcaggcgcaatgcttcgtgacgcaccagcgggacataacgctgccacagcgagtgtttatccattacaccttcagcggtatagagtgaattcacgataaacagccctgcgttatatgagttatcggcatgattatccgtttctgcagggtttttaatcggacgattagtgggtgaaatgaggggttatttgggggttacaggtaaattccaggcagaaaaaaaccccgccggtggcggggaagcacgttgctgacaaattgcgctttatgttgccggatgcggcgtaaacgccttatccggcctacaaaaatgtgcaaattcaataaattgcaattcaacttgtaggcctgataagcgcagcgcatcaggcaatttggcgttgccgtcagtctcagttaatcaggttacaacgattaaccctgcagcagagacagaacctgctgcggtacctggttagcttttgccaacacggagttaccggcctgctggatgatctgcgctttcgacatattggacacttcggtcgcatagtcggcgtcctgaatacgggactgcgcttcagacaggttggtagtggtgttgttcaggttggtaaccgcggaatccagacggttttgcaccgcaccgagggaagaacggaatttgtctacagatgcgatagcatcgtccagcgctttcagcggatccgtggttttaccatttgcaacagcagtcagagcctcaccaccagcagtcaaacctgtttgcagattaccgccatttaaatcggcagaatcgtatgttttaccatcaatatcgaccacttctgttttgccatcatctccgcccagtttgaccgcggttggagaactggcggcaccggaagagtcagtataggtaatagttttaacagaaacagcaccagtagtttcattcacatccgcagcgtaaagattgccatttgtatctttaagcgcatatgtatcggtatcattacccttggaatcctgcagttttactaagctaacagcaccaaggttggcagttgcggaacctgcagtattatcaatctgaacaggtgtaccgcctgaagtgatagttgtagctttagtagtatttgcatcagttacagttgcatttgccgttgctccagtcgccattgtcactgtaccatcattagcaactgttactgcgtaatacttcccatcgttatcaccaccggtgattttcgcatagtaatcattaccattatcagtataaacaccctcaattgaagctgggttagttccgccagtatcagtggctgcttccgtagaaagggtaattccagtaagtttaatattgtttgtggtggtagcaccaaaagcagttactggagcactagtggtaactgtatcgttatttttaacgctaaaaccatcaaggccaagagttttagcatcaatctgcttcagatcgatagtgatagtctggttatcatttgcgccaacctggattttcatggagccattttttgccagcacgttcacgccgttgaactgggtctgaccagatacgcggtcaatttcatccagacgggatttaatttcgtcctggatagaagacagatcagactcagagttagtaccggtagtggcctgtaccgtcagttcacgcacacgctgtaagttgttgttgatttcggacagcgcgccttcggtggtctgcgcaacggagataccgtcgttggcgttacgggccgcctgagtcaggcctttaatgttagaggtgaaacggttagcaatcgcctgacccgctgcgtcatccttcgcgctgttaatacgcaagccagaagacagacgctcgatagaactcgacagcgcagactggttcttgttgatattattttgagtgatcagcgagaggctgttggtattaatgacttgtgccatgattcgttatcctatattgcaagtcgttgattacgtattgggtttccacccgtcggctcaatcgccgtcaaccctgttatcgtctgtcgtaaaacaacctttagaatttttttcaaaaacagccattttttgttagtcgccgaaatactcttttctctgccccttattcccgctattaaaaaaaacaattaaacgtaaactttgcgcaattcagaccgataaccccggtattcgttttacgtgtcgaaagataaaaggaaatcgcatggcaagtatttcatcgctgggagtcgggtcaggtctggatttaagttccatccttgatagcctcaccgccgcgcaaaaagcgacgctaacccccatttcaaatcagcaatcgtcgtttaccgctaaacttagcgcctacggtacgctgaaaagcgcgctgacgactttccagaccgccaatactgcattgtctaaagccgatcttttttccgccaccagcaccaccagcagcaccaccgcgttcagtgccaccactgcgggtaacgccatcgccgggaaatacaccatcagcgtcacccatctggcgcaggcgcaaaccctgaccacgcgcaccaccagagacgatacgaaaacggcgatcgccaccagcgacagtaaactcaccattcaacaaggcggcgacaaagatccgattaccattgatatcagcgcggctaactcatcgttaagcgggatccgtgatgccatcaacaacgcaaaagcaggcgtaagcgcaagcatcattaacgtgggtaacggtgaatatcgtctgtcagtcacatcaaatgacaccggccttgataatgcgatgacactctcggtcagcggtgatgatgcgctacaaagttttatgggctatgacgccagtgccagcagcaacggtatggaggtctcggttgccgcccagaatgcgcagctgacagtcaacaacgtcgccatcgagaacagcagcaacaccatcagcgacgcgctggaaaacatcaccctgaacctgaacgatgtcaccacgggcaaccagacgctaaccatcactcaggacacctccaaagcgcaaacggcgattaaagactgggtgaatgcctacaactcgctaatagataccttcagcagcctgaccaaatacaccgccgtagatgcgggagctgatagccagagttctagcaatggtgcactgctcggcgactccacgctgcggacgattcagacgcagttgaaatcgatgctgagtaataccgtcagttcttccagctataaaacgttggcgcagattggtatcacgaccgatcccagcgatggcaaactggaactggatgccgacaaactcaccgctgcactgaaaaaagatgccagcggcgtaggtgcattgattgttggcgatggtaaaaaaaccggcatcacgaccaccatcggcagcaacctgaccagttggctttcgacaacgggcattattaaagccgctaccgatggcgttagtaagaccctgaataaattaactaaagactacaacgccgccagcgatcgcattgatgcgcaggtcgctcgctacaaagaacaatttacccaactggacgttttaatgacctcgttaaacagcaccagcagctacttaacgcagcagttcgaaaacaacagtaattccaagtaagcaatattcatcgggagacaggtcatgtacgcggcaaaaggcacccaggcctatgcacaaattggcgtcgaaagcgccgtaatgagcgccagccagcagcagctggtcaccatgctatttgatggagtgctgagcgcactggttagagcgagcctgtttatgcaggacaacaatcagcaaggcaaaggcgtctctttgtcaaaagcgatcaacatcattgagaacggactgcgggtgagtcttgatgaagagagcaaagacgaactaacccaaaacttgattgctctttatagctatatggtcaggcgcttgctgcaagccaatttacgcaacgatgtctccgcagtcgaagaagtggaagcattaatgcgcaatattgccgatgcctggaaagagtcgttactctccccttctttgattcaggacccagtctgatgaaccatgcaccgcatttatatttcgcctggcaacaactcgtcgaaaaaagccagctcatgttacgcctggcaacggaagaacaatgggacgaactcatcgccagcgaaatggcgtatgtgaatgcggtgcaggagattgcacatttgactgaagaggttgacccgtccaccacgatgcaggagcagctccgcccgatgctgcgcctgattctcgacaacgaaagcaaggtaaagcagttattacagattcggatggatgaactggcgaaactggtcggtcagtcatcggtgcaaaaatcggtgttaagtgcctatggcgatcagggcggctttgtgctggctccgcaggataacctcttttgaatctgaatgagtcgatggctcgcgaataatccgattacggctacgcttctaatgttccccttgaatggagtcgaagaatgcgtaatcccacgctgttacaatgttttcactggtattacccggaaggcggtaagctctggcctgaactggccgagcgcgccgacggttttaatgatattggtatcaatatggtctggttgccgcccgcctataaaggcgcatcgggcgggtattcggtcggctacgactcctatgatttatttgatttaggcgagtttgatcagaaaggcagcatccctactaaatatggcgataaagcacaactgctggccgccattgatgctctgaaacgtaatgacattgcggtgctgttggatgtggtagtcaaccacaaaatgggcgcggatgaaaaagaagctattcgcgtgcagcgtgtaaatgctgatgaccgtacgcaaattgacgaagaaatcattgagtgtgaaggctggacgcgttacaccttccccgcccgtgccgggcaatactcgcagtttatctgggatttcaaatgttttagcggtatcgaccatatcgaaaaccctgacgaagatggcatttttaaaattgttaacgactacaccggcgaaggctggaacgatcaggttgatgatgaattaggtaatttcgattatctgatgggcgagaatatcgattttcgcaatcatgccgtgacggaagagattaaatactgggcgcgctgggtgatggaacaaacgcaatgcgacggttttcgtcttgatgcggtcaaacatattccagcctggttttataaagagtggatcgaacacgtacaggaagttgcgccaaagccgctgtttattgtggcggagtactggtcgcatgaagttgataagctgcaaacgtatattgatcaggtggaaggcaaaaccatgctgtttgatgcgccgctgcagatgaaattccatgaagcatcgcgcatggggcgcgactacgacatgacgcagattttcacgggtacattagtggaagccgatcctttccacgccgtgacgctcgttgccaatcacgacacccaaccgttgcaagccctcgaagcgccggtcgaaccgtggtttaaaccgctggcgtatgccttaattttgttgcgggaaaatggcgttccttcggtattctatccggacctctacggtgcgcattacgaagatgtcggtggtgacgggcaaacctatccgatagatatgccaataatcgaacagcttgatgagttaattctcgcccgtcagcgtttcgcccacggtgtacagacgttatttttcgaccatccgaactgcattgcctttagccgcagtggcaccgacgaatttcccggctgcgtggtggtcatgtcgaacggggatgatggcgaaaaaaccattcatctgggagagaattacggcaataaaacctggcgtgattttctggggaaccggcaagagagagtagtgaccgacgaaaacggcgaagcaaccttcttttgcaacggcggcagcgtcagcgtgtgggttatcgaagaggtgatttaaattcatccccggcggcaagccggggagatttcattacggcagtggcgtcggtaacggcgctttatccagcgcggcggcacactctgctgtcgggcgatccacacgctccatcgtcataccatcgtactcaatggtgttaccgtcacgctcaacctcgtacagctcacgttttacggtaacgttagtgagatcatcagacatcaatgtcaacttacccggcacggcaatcacccgctgccactgacggcaatccagggtatcgccctctttagtgacaatcaggctgcctatcgcttccgggctgaccagcgcacgttgcggccctttggtctgccagtagcccgccagccagtccggcgcgggggttttcacgacattgttatagttttcgacttcggcacagcccgccagcaacaagagcgcgcctgcaattgcgagttttttcatcattcgtcctgcatgagaagaaaagaggattgtggcattaaagccctgatgtcgccagcctttcaaggttcagagagaaatttgatctaactattatttttgtgaattattaccccgaaaataaatttgcatggtgtatgattcgcgactcttgtttcaaaccttctgagttcagaggctacattcatgtcatggcagcaattcaaacacgcctggttgattaaattctgggcccccatccctgcggtcatcgcggcgggtattctctctacttactattttggcattactggcaccttttgggctgtcacgggtgaatttacccgttggggcggccagctcctgcaactgttcggcgtccatgctgaagagtggggttactttaaaattatccatctggaaggatcgccattaacccgcatcgacgggatgatgatcctcggtatgtttggcggctgctttgccgcagcgctgtgggccaacaatgtcaaactgcgaatgccgcgcagccgtatccgcattatgcaggccatcattggcggcattatcgccggttttggcgcgcgtctggcaatgggctgtaacctggcggcgttctttaccggtattcctcagttctcgctgcatgcctggttctttgccatcgccactgccattggttcatggtttggcgcgcgctttaccctgctgcccatcttccgtattcccgtgaaaatgcagaaagtttctgccgcctcaccgctgacgcaaaaaccggatcaggcgcggcgtcgttttcgtctcgggatgctggtctttttcggcatgctgggctgggcgctgctcacagcgatgaaccaacccaaactggggctggcaatgctgtttggcgtcggctttggtttactgattgaacgtgcgcaaatctgctttacttcagcgttccgcgatatgtggatcaccggacgtacccatatggcgaaagcaatcattatcggtatggcggtgagtgccatcgggatcttcagttacgtacagttaggcgttgaacccaaaatcatgtgggcgggaccaaacgcggtaattggtggtttactgtttggttttggcatcgtgctggctggcggctgcgaaaccggctggatgtaccgcgcggtagaaggccaggtgcactactggtgggtcggtctgggcaatgtgatcggctcaacgattctggcgtattactgggatgatttcgctccggcgctggccaccgactgggacaaaatcaacctgctgaaaacctttggtccgatgggtggcctgctggtgacatatttgctgttgtttgctgcgctgatgttgattatcggctgggaaaaacgcttcttccgccgtgcggcaccgcagactgctaaggagatcgcatgaaaaatatcgttcctgattaccgccttgatatggtgggtgaaccctgcccttatccggcagtcgcaacccttgaggcgatgccgcagttaaaaaaaggggaaatcctggaagtggtgagcgactgtccgcagtcgatcaataatattccactggatgcgcgtaatcacggctatacggtgctggatattcagcaagacgggccgaccattcgttatttaattcagaagtaatccctcattcccgctgtgacccacagcgggaacatcgttacctttgtatcacatagattttacccgcccccactcctattcttttcagtatgatctcaggaggtttctatgtgtggacgctttgcccaatcccaaacgcgtgaagattaccttgcgcttctcgcggaagatattgaacgcgatattccctatgatcccgaacccattggcagatacaacgtcgcgccgggaaccaaagtcctactgctcagtgaacgtgatgaacaccttcatctggatccggttttctggggatatgctcccggatggtgggataaaccgccgctgattaacgcccgcgtagaaactgcggcaaccagtcgtatgtttaaaccgctctggcaacatggtcgggcaatctgttttgccgatggctggtttgagtggaaaaaagaaggcgacaaaaaacagcctttttttatctatcgtgctgatggacaacctatttttatggccgcgataggtagcacaccatttgagcgtggtgacgaagccgaaggatttttgatcgtcactgctgcggcagatcaaggtctggtagatattcatgaccgccgcccactggtactgtcgccagaagctgcgcgggaatggatgcggcaagagattagcggtaaagaagcctcagaaatcgcggccagtggctgtgttccagcaaaccagttctcctggcacccggtatcgcgcgcggtgggtaatgttaaaaaccagggcgcggagttaattcaacctgtttgataagcctggagattattgatcaacaatactgcgtcataagaaatctctattagacaaagatttcattacctgttggcatattgcaaaaataacaccaatacggaatcgtcatgttcacgattaaaacagatgatctcacccatccagcagtgcaagcattagtggcttaccatatttccggcatgctgcagcagtctccccccgaaagcagtcatgctttagatgtgcaaaaattacgtaacccgacagtgacattctggtcagtatgggaaggcgaacaactcgcaggaattggtgcgctgaagttgctggatgataaacacggcgagctgaaatcaatgcgtaccgcgccaaattatttacgtcgtggtgtcgccagtctgattttacgccacattttgcaggtcgcccaggacagatgccttcatcgcctgagcttagaaacgggtacacaggctggatttacggcctgccatcaactttatttgaagcatggtttcgctgattgcgaaccgtttgctgattatcgacttgatccacacagtcgatttttatcattgacgctatgcgaaaataatgaattgccatgagccagacgcagcacattcttgcattcgacgtgctgcgcctttatttatcaccagcaggaaacgccttgtccatagacgccccttccacatgcgccacaagaaacctctattccagtgacacaattgcgcctaattaattacatttaatatttaattatgagttcctcaccatctattacatactttttaaccatatcggaatatttatcataatcagcgggattcgtaacaatatattttcgctgcgatctttcatagcaaatccctgtcaaagtccatgatataaaaatgtctcttcaaaagaattacattctttaaaaagtaattctttattgctatatatcgcagagacaacctcaatatcacactccatacgtgctttctccagatgatttgggaagtattgaatttcttttatcttattatcgccacaattaaacagcttagtagtctcaggcattgctggtatttaccatattttattgcgataaatagaaattgtcatagcctttgacggagatgagtcaacacgcgatatcagattattatctacggagacctgggtaattccatcggatacttttggaaataccatataattattgaaatcgagctctaattctttgcagaatttgggaatttgtattgtggcaaggccattatgacgaagataaagcacctcaatccaggatggaagaggtggcaaagaccccaagtgaagatctgttaagtcaagtttactattgtggagttcaacacatttaaacaatctcaccaatgctatatccacattttttttgaagtcattcgatgcgccttcttttactgaattagcccagtcgctgaaacctttgcaaagtctggaatctgtaattttcgtaaagttgtctagaaactctgcaatattagtcgatataaactctaatttatgccgaatgggtgggttaccagttccctgattttttctatcatgataaaacctatcttattataaatcgagaaatcttgaaaccagagactataatcaccccattcgaaatattctgagtgcaataacttaaattctgacagcatattaaataatttgctgtcttcactaattggtgtaaacttaccatttccaagacaactgactaactcacttgataattcatttatgattgcatcatcagatactaactcatgttgttttatcgtagattcagtattagatgtgactttatttaattgaaccggctgagtttttaacgaaagatcatttaatggaaacatttacactcctgtttaataaattatattgcccagggcgcattctaaaacacaataaaattaccactatcaaaaatcgctcatatccatcgcccggaatatgaataaaaacatcaacaaagattaaattatccagaggttactgttgcgtctgtggtcgtaacaacatccgacgtggtgatgtgtcaaatgagacgctctgatgttcaggggggttatcgcgtatacggatcgtggatggcagaaaacgttcaggatcaggtatccattttaaaccagaaattgagtgagtttgccccatccatgccccacgcggtgagatcggatgtaattaacaacaggttacaaaacctacacctgcatgctcatcacttcctgatacgccgccaccagcttattacgcacctgaatccccatttgcatagaaactgaggctttttgcatatcggtcatcacatcgtttaacgccacgccgggttcaccgagagtgaatttttctgcctgcgtgcgggcagctgtttgtgtatcactaatgcgatcgagcgcggcgtgcagctgcccggcaaaactaatggtcggttgcggcagtgattcctgcgcacgcgcactcatcgccgtagcctgtaactggctgataaccccttcaatcccctgtatcgctgacattctcgtctcccggataatttctggtagcaaagcctaccagtaagtcaataagacaaaggcgctaaatagcaacaaaaaaacgggtttattggcggatagaaaaaaacgaaagcacaaataatgggagcgtcaatttttcgagtttgctgacccgggagtgagtcttgttccactttgccaataacgccgtccataatcagccacgaggtgcgcgatgaatgcgactgcagcccagacaaaatctcttgagtggcttaatcgcctgcgtgcgaatccgaaaattccattgattgttgccggttccgcggcagtggcggtcatggtcgcactgatcctgtgggcgaaagcccccgactaccgcacattattcagcaatctttccgatcaggatggtggcgcaattgtcagccaactgacgcaaatgaatattccttaccgcttcagcgaagccagcggcgctattgaagttccggcagataaagttcacgaactgcgtctgcgcctggcacaacaaggtttgccaaaaggcggcgcggtcggtttcgaactgcttgatcaggaaaagtttggtatcagccagttcagcgaacaggtgaattatcagcgggcgctggaaggcgagctttctcgtaccatcgaaactatcggcccggtaaaaggggcgcgcgtacatctggcaatgccgaaaccgtctttattcgtccgtgaacaaaaatccccttctgcatcggtgacggtaaatctgttacccggccgcgcactcgatgaagggcaaattagcgccattgtgcatctggtttccagcgccgttgctggtctgccgccgggaaacgtcacgctggtggatcagggcggacatctgttaacccagtccaataccagcgggcgcgatcttaatgacgctcagttgaaatatgccagcgatgtcgaaggccgtattcagcggcgtattgaagcgatcctgtcgcctattgttggtaacggtaatattcacgcccaggttacggcgcagctggacttcgccagtaaagaacaaacggaagaacagtatcgccctaacggtgatgaatctcatgcggcgcttcgttcacgccagcttaatgagagcgagcaaagcggttccggttatccgggcggcgtaccgggggcgttgtcgaatcaaccggcacctgcgaataacgcgccaatcagcacgcctccggcaaatcaaaataaccgccagcagcaggcgagcaccaccagcaatagtgggccgcgtagcacacagcggaatgaaaccagtaactacgaagtcgatcgcaccattcgtcataccaaaatgaacgtgggcgatgtgcaacgtctgtcagtcgcggtcgtggtgaattacaaaaccttgccagatggcaaaccgttgcctctcagcaacgaacagatgaagcaaattgaagatctgacccgcgaggcgatgggcttttctgaaaaacgcggtgactcgctcaatgtcgttaactcgccgttcaatagcagtgacgaaagcggcggagaactgccattctggcaacagcaagcgtttatcgatcagttacttgctgccggtcgctggttgctggtactgctggtggcgtggctgctgtggcggaaagcggtacgtccgcagctaacacgtcgcgctgaggcgatgaaagctgtacagcaacaggcgcaggcccgcgaggaagtggaagatgcggtggaagtccgcctgagcaaagacgaacaactacaacaacggcgcgctaaccaacgtctgggggcagaagtcatgagccagcgtatccgtgaaatgtctgataacgatccgcgcgtggtggcgctggtcattcgccagtggataaataacgatcatgagtaacctgacaggcaccgataaaagcgtcatcctgctgatgaccattggcgaagaccgggcggcagaggtgttcaagcacctctcccagcgtgaagtacaaaccctgagcgctgcaatggcgaacgtcacgcagatctccaacaagcagctaaccgatgtgctggcggagtttgagcaagaagctgaacagtttgccgcactgaatatcaacgccaacgattatctgcgctcggtattggtcaaagctctgggtgaagaacgtgccgccagcctgctggaagatattctcgaaactcgcgataccgccagcggtattgaaacgctcaactttatggagccacagagcgccgccgatctgattcgcgatgagcatccgcaaattatcgccaccattctggtgcatctgaagcgcgcccaagccgccgatattctggcgttgttcgatgaacgtctgcgccacgacgtgatgttgcgtatcgccacctttggcggcgtgcagccagccgcgctggcggagctgaccgaagtactgaatggcttgctcgacggtcagaatctcaagcgcagcaaaatgggcggcgtgagaacggcagccgaaattatcaacctgatgaaaactcagcaggaagaagccgttattaccgccgtgcgtgaattcgacggcgagctggcgcagaaaatcatcgacgagatgttcctgttcgagaatctggtggatgtcgacgatcgcagcattcagcgtctgttgcaggaagtggattccgaatcgctgttgatcgcgctgaaaggagccgagcagccactgcgcgagaaattcttgcgcaatatgtcgcagcgtgccgccgatattctgcgcgacgatctcgccaaccgtggtccggtgcgtctgtcgcaggtggaaaacgaacagaaagcgattctgctgattgtgcgccgccttgccgaaactggcgagatggtaattggcagcggcgaggatacctatgtctgataatctgccgtggaaaacctggacgccggacgatctcgcgccaccacaggcagagtttgtgcccatagtcgagccggaagaaaccatcattgaagaggctgaacccagccttgagcagcaactggcgcaactgcaaatgcaggcccatgagcaaggttatcaggcgggtattgccgaaggtcgccagcaaggtcataagcagggctatcaggaaggactggcccaggggctggagcaaggtctggcagaggcgaagtctcaacaagcgccaattcatgcccggatgcagcaactggtcagcgaatttcaaactacccttgatgcacttgatagtgtgatagcgtcgcgcctgatgcagatggcgctggaggcggcacgtcaggtcatcggtcagacgccaacggtggataactcggcactgatcaaacagatccaacagttgttgcagcaagaaccgttattcagcggtaaaccacagctgcgcgtgcacccggatgatctgcaacgtgtggatgatatgctcggcgctaccttaagtttgcatggctggcgcttgcggggcgatcccaccctccatcctggcggctgtaaagtctccgccgatgaaggcgatctcgacgccagtgtcgccactcgctggcaagaactctgccgtctggcagcaccaggagtggtgtaatgaccacgcgcctgactcgctggctaaccacgctggataactttgaagccaaaatggcgcagttgcctgcggtacgtcgctacgggcgattaacccgcgctaccgggctggtgctggaagccaccggattacaattgccgctcggcgcaacctgtgtcattgagcgccagaacggcagcgaaacgcacgaagtagaaagcgaagtcgttggctttaacggtcaacggctgtttttaatgccgctggaggaagtcgaaggtgtcctgcccggcgcgcgtgtttatgccaaaaacatttcggcagaagggctgcaaagcggcaagcagttgccgctcggtccggcgttattaggtcgcgttctggacggcagcggtaaaccgctcgatggcctgccctcccccgatacgacggaaaccggtgcgctgattaccccgccatttaacccgttgcaacgtacaccgattgaacatgtgctggacaccggcgtgcgcccaatcaatgccctgcttaccgttgggcgtgggcagcgtatggggctgtttgccgggtccggcgttggtaaaagtgtgctgctggggatgatggcacgttacacccgcgccgatgtcattgtcgtgggtttgattggtgaacgtgggcgcgaagtaaaagattttattgagaacatcctcggtgccgaagggcgtgcacgctcagtggtgattgccgctccggcggatgtttctccgctcctgcgaatgcagggtgccgcctatgccacgcgcattgccgaagattttcgcgatcgtggtcagcatgtgttgctgattatggactccctcacccgctacgcgatggcccagcgtgaaattgcgctggcgattggcgaaccccccgccaccaaaggttatccaccgtcggtgtttgccaaattaccggcactggtcgagcgtgccggaaatggcattagcggcggcggctcgattaccgcgttttataccgtgctcactgaaggcgatgaccagcaggatccgattgccgactccgcgcgggcgatcctcgacggtcacattgtgctgtctcgccgactggcggaagccgggcactatccggctatcgatattgaagcgtcgatcagccgcgcaatgacggcgttgatcagtgagcaacattacgcgcgagtgcgcaccttcaaacagctgttgtcgagttttcagcgtaaccgcgatctggttagcgtcggcgcgtatgccaaaggcagcgatccgatgctcgataaagccatcgccctgtggccgcagctggagggctatttgcaacaaggcatttttgaacgcgcggactgggaagcgtctctccaggggctggagcgtattttcccgacagtgtcataacccaggagataacggcagatggcagaacatggtgcgctggcgaccctgaaagatctggcagaaaaagaggtagaggatgccgcgcgcctgctgggtgaaatgcgtcgcggatgtcagcaggcggaagaacagctcaaaatgctgattgattatcagaatgaatatcgcaataacctcaacagcgatatgagtgccgggataaccagcaaccgctggatcaactatcagcagtttatccagacgctggaaaaagccattactcagcatcgccagcaacttaatcagtggacgcagaaagttgacattgccctgaacagttggcgagaaaaaaaacaacgtttgcaggcctggcagacactgcaggaacggcaatccacggcggcactgcttgcagaaaaccgcctcgatcagaaaaagatggatgagttcgcccagcgcgccgccatgaggaaacctgaatgattcgcttagcgcccttgattaccgccgacgttgacaccaccacattgcctggcggcaaagccagcgatgctgcacaagattttctcgcgttgttgagcgaagcattagcaggcgagacaactaccgacaaagcggccccccagttgctggtggcaacagataagcccacgacaaaaggcgagccgctgatcagcgatattgtttccgacgcgcaacaagctaatttactgatccctgtggatgaaacaccgcctgtcatcaacgacgaacaatccacatcaacaccgttaaccaccgctcagacgatggcgttggctgcggtggctgacaaaaatacgacaaaagacgaaaaagcggatgatctgaatgaagacgtcaccgcaagcctgagcgccctttttgcgatgttgccgggttttgacaatacgcccaaagtgactgatgcgccgtcaaccgtgttaccgacagagaaaccaacgctcttcacaaaactgacttctgagcaactcacaacagcacagcctgatgacgcccccggcacaccagctcagccattaacaccgctggtagcagaagcccagagtaaagcggaagtcatcagcacaccttcaccggtgaccgctgccgccagcccgctaatcactccacaccagacacagccactgcccaccgtcgccgcacctgttttgagtgcaccgctgggttctcacgaatggcaacaatcattaagccagcatatttcgctgttcacccgccaggggcaacaaagtgcagagttgcgtctgcacccgcaggatttaggtgaagtgcaaatctccctcaaagtggatgataaccaggcgcaaatccagatggtttcaccgcatcagcatgtacgcgccgccctggaagcagcgctgccggtactgcgcacgcagctggccgaaagtggcattcagttagggcaaagcaacatcagtggcgaaagctttagtggtcagcagcaggccgcttcccagcaacagcaaagccaacgcacagcaaaccatgaacctctggcgggggaagacgacgatacgcttccggttcccgtctctttacaagggcgtgtaacaggcaacagcggcgttgatattttcgcctaacgtcagaggtagcaccgtaatccgcgtcttttccccgctttgttgcgctcaagacgcaggataattagccgataagcagtagcgacacaggaagaccgcaacacatgactgattacgcgataagcaagaaaagcaagcgatcgctttggatcccgattctggtattcattaccctcgcggcctgtgccagcgcaggttacagctactggcattcgcatcaggttgccgctgacgacaaagcgcagcaacgcgtcgtgccctcaccggtcttctacgcgctggataccttcacggtcaatttgggcgatgcggatcgcgtactttatatcggcataaccctgcgcctgaaagatgaagctacccgctcgcggctgagtgagtatttgccggaagtccgtagtcgcttgctgttactgttttcgcgtcaggatgctgccgtactggcgacagaagaaggcaagaaaaacctgattgccgagattaaaaccacactttccaccccgcttgttgccgggcaaccgaaacaggatgtcaccgacgtgctgtataccgcttttattctgcgataacgacatgggcgatagtattctttctcaagctgaaattgatgcgctgttgaatggtgacagcgaagtcaaagacgaaccgacagccagtgttagcggcgaaagtgacattcgtccgtacgatccgaatacccaacgacgggttgtgcgcgaacgtttgcaggcgctggaaatcattaatgagcgctttgcccgccattttcgtatggggctgttcaacctgctgcgtcgtagcccggatataaccgtcggggccatccgcattcagccgtaccatgaatttgcccgcaacctgccggtgccgaccaacctgaaccttatccatctgaaaccgctgcgcggcactgggctggtggtgttctcaccgagtctggtgtttatcgccgtggataacctgtttggcggcgatggacgcttcccgaccaaagtggaaggtcgcgagtttacccataccgaacagcgcgtcatcaaccgcatgttgaaactggcgcttgaaggctatagcgacgcctggaaggcgattaatccgctggaagttgagtacgtgcgttcggaaatgcaggtgaaatttaccaatatcaccacctcgccgaacgacattgtggttaacacgccgttccatgtggagattggcaacctgaccggcgaatttaatatctgcctgccattcagcatgatcgagccgctacgggaattgttggttaacccgccgctggaaaactcgcgtaatgaagatcagaactggcgcgataacctggtgcgccaggtgcagcattcacagctggagctggtcgccaactttgccgatatctcgctacgcctgtcgcagattttaaaactgaaccccggcgacgtcctgccgatagaaaaacccgatcgcatcatcgcccatgttgacggcgtcccggtgctgaccagtcagtatggcaccctcaacggtcagtatgcgttacggatagaacatttgattaacccgattttaaattctctgaacgaggaacagcccaaatgagtgacatgaataatccggccgatgacaacaacggcgcaatggacgatctgtgggctgaagcgttgagcgaacaaaaatcaaccagcagcaaaagcgctgccgagacggtgttccagcaatttggcggtggtgatgtcagcggaacgttgcaggatatcgacctgattatggatattccggtcaagctgaccgtcgagctgggccgtacgcggatgaccatcaaagagctgttgcgtctgacgcaagggtccgtcgtggcgctggacggtctggcgggcgaaccactggatattctgatcaacggttatttaatcgcccagggcgaagtggtggtcgttgccgataaatatggcgtgcggatcaccgatatcattactccgtctgagcgaatgcgccgcctgagccgttagtgatgaataaccacgctactgtgcaatcttccgcgccggtttctgctgcgccactgctgcaggtgagcggcgcactcatcgccattattgccctgatcctcgctgctgcctggctggtaaaacggttgggatttgcccctaaacgcactggcgttaacggtctgaaaattagcgccagtgcttcactgggcgcgcgtgaaagggttgtggtggtcgatgtggaagatgcacggctggtgctcggcgttaccgcaggtcaaatcaatctgctgcataaacttcccccttctgcaccaacggaagagataccgcagaccgattttcagtcggtcatgaaaaatttgcttaagcgtagcgggagatcctgatgcgtcgtttattgtctgtcgcacctgtccttctctggctgattacgcccctcgccttcgcgcaactgccgggtatcaccagccagccgctgcctggcggtggacaaagctggtcgctcccggtgcagacgctggtgttcatcacctcgttgacgtttattccggcaattttactgatgatgaccagtttcacccgcatcatcattgtttttggtttattgcgtaacgcgctgggaacaccctccgcgccacctaaccaggtattgctggggctggcactgtttttgaccttttttattatgtcaccggtgatcgacaaaatttatgtagatgcgtaccagccattcagcgaagagaaaatatcaatgcaggaggcgctggaaaaaggggcgcagccgctgcgtgagtttatgctgcgtcagacccgtgaggcagatttagggttgtttgccagactggcgaataccggcccgttgcagggacctgaagccgtgccgatgcgcattttgctcccggcctacgtgaccagcgagttgaaaaccgcatttcagataggcttcacgattttcatcccttttttgattatcgacctggtgatagccagcgtgttgatggcattggggatgatgatggttcccccagccaccattgctctgccctttaaactgatgctgtttgtactggtggatggctggcaattgctggtcggttcgctggcgcagagcttttacagctagagaggcaaaatgacacctgaatcggtcatgatgatggggactgaagcgatgaaagtcgcgctggcactggctgccccgctattgttggtagcgttggtcacgggccttatcatcagtattttgcaggccgccacgcagattaacgaaatgacgctgtcgtttattccgaaaatcatcgccgtatttatcgccattattattgccggaccgtggatgctcaatctgttgctggattacgtccgcaccttgttcactaacctgccgtatatcatcgggtagccgtactatgttgcaggtgacaagcgaacaatggctatcctggttaaacctgtacttctggccgttactgcgcgtgctggcgctgatctccaccgcgccgattctgagcgaacgcagcgtaccgaaacgggtaaaactgggtctggcaatgatgatcacgttcgccattgccccatcattacctgccaacgatgttcctgttttttcgttctttgctctgtggctggccgtgcagcagatcctgatcggcattgcgcttggttttaccatgcaatttgcctttgccgctgtgcgaaccgctggcgaaattatcggtctgcaaatggggctgtcatttgcgacgtttgtcgatccggccagccatcttaatatgcccgttttagcgcgtatcatggatatgctggcgttactgctgttcctgacatttaacggtcatttatggttgatttcactgctggtcgatacctttcacaccctgccgattggtggcgaaccgttgaacagcaatgcgtttctggcactcaccaaagcagggagtttgattttccttaacgggctgatgctggcgttaccgctcattactctgctgctgacactgaatctggcattaggtttacttaatcgtatggccccgcaattatccatttttgttattggatttccattaactctgactgtcggcatctctttaatggcggcattaatgccgttaattgcacctttttgcgaacatttattcagtgaaatttttaatttgctggctgatattattagtgaattgccattaatataattccgtaacgtttatcatgttatcctaaggattatccgaaaaataatacctacgaacatcttccaggatactcctgcagcgaaatatttgttttaagctcactcacatatcgcaacatttactttactttaagacaattccaggcaaattatacaacactttacgggatagtaagtccgcctgaaaaatcgcgagagtggcgcattaggtgacccatgttgttccgtttagtcatgatgaaatattcaggtaaggggaattatcgttacgcattgagtgagggtatgccatgtcaacgattattatggatttatgtagttacacccgactaggtttaaccgggtatctgttgagtagaggggttaaaaaaagagaaatcaacgacattgaaaccgttgatgaccttgccatagcttgtgattcacagcgcccttcagtggtgtttattaatgaggactgtttcatccacgatgcttctaacagtcagcgtatcaagctcatcattaatcaacatcccaatacgttatttatcgtttttatggcaattgccaatgttcattttgatgaatatctattggtcagaaaaaatttattgatcagttctaaatcgattaaaccggaatctctcgacgatatccttggcgatattctgaaaaaagagacaacgataacctcgtttttaaatatgccgacgttatcattgagccgaaccgaatcgagtatgttgcgaatgtggatggcaggtcagggaaccattcaaatctctgaccaaatgaatatcaaagccaagaccgtttcatcgcataaaggtaatattaaacgtaagatcaaaacgcataataaacaggttatctaccatgtcgtccgactgacggataatgtgactaatggtatttttgtcaacatgcgctaacacattctgactggtggtttcccaccagtcaggctgaataagattactctgctttctccacaaagataccgtcctgatgccctgcttcattaaagaaccagatgccgagcgggtagtcttccagcgaaaccaggtacattgtgccttcactaaactcctcaactgccagtaccacgccaggacgacgcggaccgccatccgttttgactgttacccgatcattcaccttcatcgttttcctcctgtggctttgtgccagtgtagaacaatttcgtttttctggcagcgccaggcgcgcgcgagtgctgattttctcgacggtctatacttaagagatgccaggcggacttaacgactggcggcaacaacagagtaacggttgcgaggaaagatgatgaaaaccgcaaaagagtacagcgataccgcaaaacgtgaggtcagcgtcgatgtcgatgccctgctggcggcgatcaatgaaattagcgaaagcgaagttcatcgcagccagaacgattctgaacacgttagcgtcgatggacgtgaatatcatacatggcgtgaattggcggatgccttcgaactggatattcatgacttcagcgtctctgaagtgaatcgttgaatgcacaataaaaaaatcccgaccctgagggggtcgggatgaaacttgcttaagcaagaagcacttaaaaaattcgttacaccaggaaatctgatgtgttcatcaccttatccgcaatttttttcgctgacaagaaaatattcgccatatgaatgattaacgctacttatgaatagaaatgtgacgcacgtcaccccttggtggctctggcgtcagcgggatcgctcccgaaaaaatcatctttgataatttgtgcggttttgagaatcatcctggtaagaggagtactgcgcgactatgttttcaattcaacaaccactactggtttttagcgatcttgatggcaccctgctggacagtcatagttatgactggcaaccggcagccccctggctcacccgtttacgcgaagcaaatgttcccgtcattctctgtagcagtaaaacatcagcggaaatgctgtacttgcaaaaaacgttggggctacaaggtttaccgctgattgccgaaaatggcgcagtgatccagcttgctgagcaatggcaggagatagacggttttccacgcatcatctcaggtattagccatggcgaaatcagcctggttttaaatacgctacgcgagaaagaacattttaaattcacgacttttgatgatgtcgacgatgcaaccatcgccgaatggacgggattaagccgtagccaggcggcgctgacgcagcttcatgaggcgtcggtaacgctaatctggcgcgacagtgacgagcgtatggcacaatttaccgctcgtctgaacgaactgggcttacagtttatgcagggtgcgcgcttctggcacgtactggatgcttctgccggaaaagatcaggctgccaactggattatcgcgacctatcaacaattgtcaggcaaacgcccaaccacacttggcctgggcgatgggccaaacgatgcgcccttactggaggtaatggattacgcggtgattgtgaaagggctaaatcgtgaaggggtgcatctgcatgatgaggatccggcccgcgtctggcgaacgcagcgtgaaggaccggaaggatggcgtgaagggctggaccattttttctccgcccgttaagcgttatcgctcgcgaatacccgattacgcccagcctgtttagcgagataaagccgacggtcggccagtgactggagttgttcaaaatcataatcaccggtttcctcgctgctgcttacccccagcgaggcactgatgcgtatcgtcgtactcttggcgatcaacatctctttttcatttaatttcagtcgaatacgttctgcgacctccgcagcctccgtcagactcgcgcctggcagaatcacacaaaactcctcaccaccgacccgcccggcaacgtcctgcgcacgcaaggaactgctaattaatccggcagcatgagaaagaacacggtcgcccgcctgatgaccaaagcggtcattaatcgctttaaaatggtcaagatcgacctgaatgacagaaaaaggatgttggtgcgtctgacacaatttagcgagcggacgggctttttcgaacagtgcgccacggttatataaacgcgttaaggtgtcgtgccacgcctgccactgcaacgagctttgcagaacatacatgttgctaaccatccggcgaatcacataccaggagatgagtaacatggtggtaaagagcgcccacagcagggttaatgcaatgctgatactgccgaaatcgccgcgcacgccttcgcttaacgtatggacacgcaccagcacaccgtcgaaatggtccagacgttcccagctaacatagcgactgtccatacgaatgccgccccgcgtgtcatgttccattgcctgcgccagcaaggccagttcacgaggatcaaaaatattccctgttggatggtcaggattggaagaggtcaaaaatctcagcttactgtcatagagctgatactcaccatcgaggtttttatcgatggcgtttcttaaaaattgctgcatagtacgcacgggaatactcatccccagcacgccataccagtagttattactgtctaccggaacactgacggtaacctgcggttcagtattgctggcgtgttccggttgcgaagtgaaccagcgtaccgcgcggtgacgattttctcgttgtgaatggccaataaaccagggttgggtgacatagccgtaataacgcgttggaacattgcgcgtaaacaaggtcggctgcgtcgaaacgtaaaatccggcacgcgagacatacatcgcctgttcaaccatcgacgaggagttgtgcgctagtcgcagcaagtaaccaacttccagtgcagcggtaatttcattgtcgaggctttcattttcgcgagacaggagattcccctcgctgactaatgcatccgacacaccattaactggcagagtgcgtcgtcggttgagttcgattttccaggcgtgctcgtcgcgatgctgttcgaactcggttacagcatcacgcagagaggtgaaatccagtggcgctacgagagcttcgcgcatgccattacgtaaaaagatcagtttgtcgacgttatactgcaaatgcttatcgagcgcgttggcaacgttttccagatgattacgctggctggagatataggcatcttccagcaccaccacttcacgccaggtgagcaaggtggaaaaaagcaataccacgataaagcagagattaacgacatgaccaggccccaggcggcgtgcgagttttttcaaccagctctggttttccatttttgtctcgtgctgcaccctgacgactcccaacctgcttttttatgattctggcataacctggcgatagcgtaccgcaaaacagcgataattttataatggtggcatgataagacgcgactatcattcattgcaggcattagcacaccaggccggatgtgatccggcctgatgttaatgataccctttcacacttcttccgcagaacgactcccctcccccggaacaagctcggtttcatgaaaagcttcccgcttgaccccgtaaccgtcataccaacgacactcaaccataccgctggagtatccagtgacaatcatccgcgggccgccctctttaaccgtaacttcctcactaaccataaagctcatactcgcctccttttttcgagtgaaacttgttcaccttagttgaagatggcgaattttgcataatagccagtgcgagtattaatgtgcctgaccgcgcattttctctacggctttcactcccagcaccacgatgccgccgatgataaatccaagaatcagatttaaaacagtcggtaatatcatcgccactactgcactttgctgcccggcgaaatgttcaatggcgtgatgcagcggcgcaattccatgtaccacaatcccaccgccgacgaggaacatcgccagcgtgccgacaatcgataacgctttcatcagccagggcgcgataatcaataaccctttacctaatgcctgcatcagcgcgctggatttttccgccagccaataccccaggtcatcaatcttaacgataacccctaccagaccgtagacgcccacggtcactaccagcgcgatgcctgaaagcaccagcacctgattaagcaacggcgcttcggccacaatccccagcgtgatggcgacgatttccgcagacaatataaaatcggtacgaatcgccccttttattttgtccttttcaaacttcagcggatcctgcgccgccagcttctccagacgctgctggctctgcgccggatcttctttatgtttacgcgcctccagcatatgcagcactttctctactccttcaaagcagagaaacgcgccaccaatcatcaacagaggcgtaatcgcccacgggataaacgcactgatgatcagcgccagcggcaccagaatcactttattaatcagcgatcctttcgccacgccccagaccacgggaagttcccggttggcccgcacgcctgaaacttgttgcgcattgagcgataagtcatcccctaatacaccggcggttttcttcgccgccagtttgcccatcacggagatatcgtccagtagtgtggcgatatcatcgagcaacgtcagtaaactactcccggccaaaagcattccctctcatttttattgttgaagggtgtaagtatgaagcaaaaacggcagctctgatacttgcttcacaggtcaacatttttttaacaatcaagtgcaattatatctctcgccagcagaatgattttcacgtttactatgaaccacctttttatttccaccgtgagggattatgcgtttccgccagttgttaccgctttttggcgcgctgtttgcgttgtatatcatttggggctcaacctattttgtcattcggattggcgtggaaagctggcctccgttaatgatggcgggcgttcgattcctggcagccggtattttattgctggcatttttgctactgcgcggacacaaactccccccgctacgtccgctgctcaatgccgcgctgattggcctgttattgctggctgtcggtaatggcatggtgacggttgccgaacatcaaaatgttccttccggcatcgccgccgtagtggttgcaaccgtgcccctctttaccctgtgcttcagccgcctgtttggcattaaaacgcgcaaactggaatgggtgggtattgccattgggcttgccggaatcatcatgctcaatagcggtggaaatttaagcggcaatccgtggggcgcgattctgattttaatcggctcgattagctgggcgtttggctcagtttatggctcgcgcattaccttacctgtagggatgatggcgggtgcgattgagatgctggcggcaggcgtggtgttaatgatcgcgtcgatgattgcgggtgaaaaactgacggcgctcccttccctttcaggcttccttgcggtcggctatctggcgctgtttggttcgattatcgccatcaacgcttatatgtatttaatccgtaatgtcagtccggctctcgccaccagctacgcttacgttaacccggtggtcgcggtcttgctgggtacgggactgggtggagaaacactgtcgaagattgaatggctggcgctcggcgtaattgtcttcgcggtggtactggtcacgttgggaaaatatctcttcccggcaaaacccgtagttgcgccagttattcaggacgcatcaagcgagtaaatgaatcccctgcgtgtcgatctgcgcgctggcaccttcgccgcagatccactcttccagacgctcggtaagcgcttcatccgtcagcttctcgcgcccacgtaacgcgcactcccagacaatcaatacgcgccagccgagttcctgcaagcgactgatatcgcggcgatcgcgctcaacatttttacctatcttctccagccagaactcggttcgagtcgcaggcactttaaacagatagcagtgatgatgatgccagaagcagccatgggtaaatatcacgcagcgatattcatcaacgacaaaatccggacgtccgggcagactggcgtcctgaacgcgaaatgccaggccctgcccggttaacagactggcgaggcgcttctctatcgccgtatcacgcgtggcaatcgcgcgcatatttttgctgcgagtggccttatcgtgaacgtcggccatgttgtgcctcttgctgacgcaacgccaccgcctgtttgatttttggctcaagcagttttgccaccgcggcaaagaccggcacgaccaccgagttaccgaactggcgataggcctgagtgtccgaaaccggaatacggaatttcgcttctcccggcgcttcaaaacccattaagcgcgcgcattcccgaggcgttaaccgacgtggacgatgttgctgattcagcggatcgtcaaagtctttctcacccgtggccatatcccagccgcgatcgattaaaatttccgcgccatctttgtaataacgcgcagacagcgtacgcgtgacgctttgcggattgttcggataaaccattccataaccgaagccgttaccgcgcgcctgatgttttttcgcatatcgatagaggtacttccacagcaccggcgtcaggatatatttcgcctcgaccatcgggtccaacagctgcgccagcgtcactcgctgcgcagggaaacattcgctgatatcacgcagggtaaaatcggctttcagattcagatcgcgacgaaaacccaccagcacgatgcgttcacggtgctgcggcagaaaatgtttgccgtcgatgattttcggatcgtctggcccattatcttctgcatcagccacgtcatagcccagttcgtccagcgtctgcatgatgatgcggaacgttttaccctggtcgtgacttttcaggtttttgacgttttcgagcacaaacatcgccggacgacgcgcgtcgataatgcgtaccacatcaaaaaacagcgtgccctgggtatcgcaggcaaaaccgtgcgcccgcccgagcgagttctttttcgatacgccagccagcgaaaatggctgacaagggaaaccggccagtaaaacatcgtgttcaggaatgtgttgacgaatatgttccgccgccgcctcatcactcacgccttctttatggctgagggtgatgtcgcggatatcttcattaaaatgatgcgtcgccggatcgcaataatggttggctttataagtgcgtaccgcatgtttgttccattcgctggtaaacacgcactgtccgccaatcgattcaaaaccgcgacggatgccgccaattccggcgaatagatcgataaagcgaaacgcataatgcggatgatgtgccggtggtttgggtaataacgtttgcagatgggcgaactctttctcacttaaacggtgccatgccgagtcattcgccagcgcacgttttaaaattgccgcgctccagtgattctcacctacaccattaagctgcgccaccaacgttttaacatcataaatttgcagcagtttctccagcattgcctgtgcggcattcccggtgctgtatgaatcggttactgatatattttcctgcatagatttcaccggccatctgagatggccgacaggttaacataattacagccatttagggccacgcgctcagccagcggatgaaaacgcatctatcaccttgtgatcgacaccttcattctcccccgccagttcggcactgagcttcgccataaactcgactaaaaaatgcgcgttgtgctgcgccagctgcttgcctcttgcggtttgcatggtttgcggtagcttcagcaacttagtctggaaatgatccagcgcgtagcgtttatcatcaagcgggcgatgctgtgcgaacggatcttcaccatcaaacagcgccacgcccaatgcccctgaaacggcaaacacgcgcgccaggccaatcgcccccagggcttccagccgatccgcatcctggacaattttagcttccgttgttaagggggcgatttgcgcgctgaaactgtgagcggcaatggcatgacaaacggcctcgattttctccgccggaaattgctcgaactcttcacggagcaggcgacgcgtctcttctgccgccaggattgaagaacgctgcctttgcggatgatttttcgccaggctcacaatatcgtgaaaataacaggcggttaaaatcaccagcatatcgacatcgtcatctgccgccagcttctgtgccgtagcccagacgcggcgaaaatgacacacgtcatgggccgcgtcctggtgctgatgatggtttttcaaccagttttcgaactgtgcctgccagtgttgtaagtccatacgcgctccgttgccaaagagtcgccaccttagcagtttttattcatagcgtctgctacgtgcgggacgaggtcgggtgtaccaggcaatgctgcctaacaatgccccgaccagagccataaataaaaatccgaccagtgcccctaaccactttcccgcggtagagcctaaatcgctttcaaatcccgacacgggggcatcgggaatccggctcatcacccagatgtaacgcgccattgcccagacgaaatagccacaccatgtatagaaagcccacaaagccagtttgccgccagggctgcgagagagtctctcttccatctttgtcgaaccgtattccattttgagataacccggaaaattcagacttagtactattatgtgataaaagtcacatttttccacattggatgagccagtcaagactcaatcattttttgaacaaatagataaattttgcgcaacggcagtgaatacaggaaaaatcgttttgagcgattttatttatctttgatatcggctttattaattcatttaatcaatatattagcactgattacaattatacctttttattattctgtgtcatgatgcttccgttattagccttttatcgtcttgtttatattttttgggccggcatgatgccggcttttttttatgccttcattaatgtgcgcctgatcacaccagccgtttggcgcaacaatcattgataccccctatgtttccgctcaactcataacatattgatatacatttataattttcatgaatatttatatttagaattcataattatgaattatattaaatagattagaaacattttgatatcttttaaatacatttgttacatgtaatccttaaaataaaatgaacttcatagaatagtatccaaatgtgcttttttttggataacggcacttattgatatattcatgaagattataatcacaagggaatacataatgaaaagaaaagttctggcaatgctggtcccggcgttattagttgctggcgcagcaaatgcggctgaagtctataataaagatggtaataaactggatttgtacggaaaagtagtgggtctgcactacttctctgatgattctggcagcgatggcgacatgtcatatgcccgtatcggtttcaaaggtgaaactcagatcgctgatcaattcactggttatggtcagtgggaatttaacattggcgcaaacggtcctgaaagcgacaagggtaataccgcaacgcgtctggcatttgcaggtttaggctttggtcagaatggtactttcgactatggtcgtaactacggtgtcgtatatgacgtagaagcatggaccgatatgctgccagaatttggtggcgatacctatgctggcgctgacaacttcatgaacggtcgtgctaatggtgttgcaacctaccgtaacaatggcttctttggttaggtcgatggcttgaactttgctttgcaatatcagggtaataatgaaagtggtggaccattcgggcaggaaggttccggtagtggtgatggccgtagcctttccaaagaaaatggtgatggtttcggtatgtcaacatcctacgacttcgacttcggtttaagtctgggtgctgcatatcaaactctgatcgttcagatcgtcaggttggagttggtttaaatgatcgtaaccatagcaacagaaatgctggtggtgaaaccgctgaagcatggactgttggtgcaaaatatgatgctaataatgtgtatttagcagctatgtacgctgaaactcgcaatatgaccccatatggtggtggcgagtttgataatggtgaatcaagatcagccatcgctaacaaaacccaaaactttgaagttgttgctcagtatcagttcgactttggcctgcgcccgtccatcgcttacctgcaatctaaaggtaaggatttaggcggttgggctcatgacggcaacggcgacccacgttacaccaataaagatctggttaaatacgttgatattggtgcgacctactacttcaacaaaaacatgtccacctatgttgattacaaaatcaacctgctggacaacgacgatgacttctacgaagcaaacggcatcgctaccgatgatatcgttgctgtgggcttagtctaccagttctaatcagtcaactcgctgcggcgtgttactgtaaaactgaacactagcctgagttcgtccctcatcgaactcaggcttttttattggcatttcatctccatctgcggcacacgcaattgccgaagcatatcgatacagcaccttaccctgcccctcctggcacaataacatcaaccagctactcttcaagctaacacccaaatgcatttctttatgaattaatccgtaacaaacacgcttcccatatagaaatatttgcaaaaatagtgcatgaaataagctttttctctaccaatccgggatataaatattcatcagcaccacaatattccacagcactaaatctctccccgccaccccgtacctctgataatggtctaaaatcattgaagccacttgcgacgacgttgctcaataaggaaaatttggcgtgaataatattcaacaccagtgcagcatcatcattacatacttacagccgccgactaccgctttcgatatattgactcaattttccagcctggttaaaaatagcgaccagctcagtcgcaaatatagtgactaccctaactaagcaacaataaggaatacactatgactgttcaaacaagtaaaaatccgcaggtcgatattgctgaagataatgcattcttcccttcagaatattcgcttagccaatataccagtcctgtctctgatcttgatggcgtggactatccaaaaccttatcgcggtaaacataaaattctggtgatcgccgcggacgaacgttatttgccgaccgataacggaaaactgttctcgaccggtaaccatccgattgaaacgttgctgccgttgtatcatctccatgctgcaggtttcgaattcgaagtggcgaccatttccggtctgatgaccaagtttgaatactgggctatgccgcacaaagatgaaaaagtaatgccattctttgagcagcataaatcgttgttccgcaatccgaagaaactcgcggatgttgttgccagcctcaacgctgatagcgaatatgcagcaatctttgttcctggtggtcatggcgcacttattggtttacctgaaagccaggacgtggctgccgctttacagtgggcaatcaaaaatgaccgttttgttatctccctttgccacggcccggcggcttttctggcgcttcgccacggcgataacccactgaatggttattccatttgcgcattcccagacgccgcagacaaacaaacgccagagattggctatatgccgggtcatctcacctggtacttcggcgaagaactgaagaaaatgggcatgaatatcattaatgacgacatcaccgggcgagtacataaggaccgtaaacttctcaccggcgacagtccttttgcagcgaatgcgttgggtaaactggcggcgcaggaaatgctggcagcttacgcgggttaatccctgttacgtttgaatgtaagcgcataatcaatcgcggccgcgttagtactcacgacgtggctgcgttttttcacggttaatttatggcgtactgaagccctatgttaatttctttgcggtaacgtaatccggaacacattatgcttattgagatagtgatacgtagcacttcccccatgcaattcggcaatcgctttgactaaagaaaggcctagtccctgacctacggaatgacgcgaattatctccccgccaaaatctacggaagagtttttcaggctcattaattttcgttccagggctggcgatatcaatattaagatagctgttggtatcaagaaaactggttatatgaatacgcgatttttctggcgaatatctaatggcattaacaataagattcgataacattcgttgtagtaaaattttatccgcaaagatttgctgattgcactcgaccttaaagcaaatctctttctcgtctgaaaggtattcaagatagtccaacaaattttcgacttccttattgagagaaagcgagtccagtttcaccaaaacattgtttttatctgccctggcaagaaacagtatgttctctgttaaccgcgaaatattttccagctcttcaatgtttccggcaattgttttttgatattcagcgatacttctggtttgactgagcgtaacctgattctgacccagtaatgcattaattggcgttctaagttcatgagcgagatcgtcagcaaactgacttagacgctcaaaatctttgactaaagcatgatgcattttattcaacgcctgcccaagaggttttagttctctcggtaatgcgctaacctcaacaggctctcggctatcgttataattcagcgcttccgttacaccactcaactttttgatctctcgtaatcccgttctgattaacagcggacttaatactgagcaaagtacaatggcgacaatgcaaattataatgctattaattttatactgttcaagcatgttatgtctggctgaagccaatttagccacagtaaccgttaatgatggcgaaacttcatcaatattaattcgtaaagcatctatctctgtatcattaataatgcttctgtaaatgccagctgcgctgattgtctcactagcaggtatgttatttaacatgccatcactgacatttgtccggttaacaattttattgatgctatcaccatgaataatcaagatatcctgactaacatccatcatccggttaaagtacacaggtaacgtatctggatttaccccatcaattaacaactgcttgatctgcgctgtccggttaatgagtgttgtatcatcgcgccatttcaactcacttgccaggccattatagagagtccagacaattccggcgccagcaacagacagtagcaatataaaaagcaaggttaaacggacggttatagatagtcttttcattatttttttaccgctacgaatgaatagcccatcccccggattgtggcaattagcttttcaggaaaaggatcatcaacttttgcgcggagcctgcgaatggcgacgtccaccgtattggtatcactatcaaagttgattccccaaatttcactcgcaataaccgttctgggtataatttcgccagctctggaggccagtagccaaagtaactgaaactccttgcgcgtcagtgtaatactgatattgtccctgctcacactatgactaacagagtccattcttaagccgctgatttctaatgttgaattcaaagcgtgatgttgccttaattgtgcccgaacccttgccagcaactcagaaaatgaaaaaggttttaccagataatcatttgccccactgtccagccctctgactctgtcatcgacagaatcccttgcagtaaggcaaataacaggggtttgctttgctgttcttaacgtttgtaagatctgccagccatccatacccggaagcataatatccagaatgatcaatgcataatcatccttcagcgcaagataaagcccatctctgccatcagaaacggcatcgatgacataacccgcttcggaaagcccctgcgttacccattcctgggtcctttgattatcttcaataagtagaatcttcatgaaaataatatgccataaatcatatgttatagaaacagcctggttcattacaaaattgtaatgctgctgtaaggttaccctggacgctttttcgctatcctcaaaactcattcacatgacaaggatataaacatgttaaagcgttatttagtactctcggtagcaacggcagcattttcattaccttctttggttaatgccgcacaacaaaacattcttagcgtgcacattttgaaccagcaaacaggaaaacccgctgctgacgtgacagtcactcttgaaaagaaggcggataacggctggttacaacttaataccgccaaaacagataaggatggacgaattaaggcactgtggcccgagcaaactgcaactacgggcgattaccgtgtcgtatttaaaaccggggactatttcaagaaacaaaatcttgaaagtttcttccctgagatccccgttgaatttcatattaataaagtgaacgagcattatcatgtgcctttattacttagccaatatgggtattcaacctatcgtggcagttaatgcataaatatgtaaaagcagatctctgctactgttagggaggacactccctgacagattaacagtaaacggctcttgctggctaacgacaaaaaagtgtgatggcttatgaaaaagaatcaatttttaaaagaatcagatgttacggccgagtcggtattctttatgaagcgtcggcaggtgttaaaagcactgggcatcagtgcaactgcactttctttgcctcacgctgcgcatgccgatctgcttagctggtttaaagggaacgatcgcccgcccgcccccgccggaaaagcgctggagttcagcaagcctgccgcctggcaaaataacctgccactgacgccagcagataaagtttccggttataataacttctatgaattcgggctggataaagccgatcccgccgctaatgctggtagcctgaaaaccgatccatggacactgaaaatcagcggcgaagtggcaaaaccattgaccctcgatcatgatgacttaacccgtcgcttcccgctggaagagcgtatttatcgtatgcgctgcgtggaagcgtggtcgatggtggtgccgtggattggttttccgctgcacaaattgctggcgcttgccgaacctaccagcaatgcgaagtatgtcgctttcgaaacaatttatgcaccggaacagatgccaggccagcaggaccgctttatcggcggtgggctgaaatatccttatgtcgaaggattgcgtctcgacgaagcaatgcatccgctcacactgatgaccgtaggtgtttatggcaaggcgttaccgccacaaaatggcgcgccggtgcgactgattgtgccgtggaaatatggctttaaagggattaaatcgatagtcagtattaagctgacccgcgagcgtccgccaaccacctggaatctggcagcgcctgacgaatacggtttttacgccaacgttaatccgtatgttgatcacccgcgctggtcacaggctaccgaacgatttattggttcaggcggcatcctcgatgtacagcgccagccaacgctactgtttaatggttacgccgcccaggtggcatcgctgtatcgtggcctggatttgcgggagaatttctaaatgcgtctgacagcaaaacaggtgacatggctgaaagtttgcctgcatcttgccggattgttgccgtttctctggctggtctgggcgatcaatcacggtggactgggtgccgatccggtgaaagatattcagcattttactggtcgcactgcactgaaatttttgctggcgaccttgttaatcacccctctggcacgctacgcaaaacagccgttattgatacgcactcgccgcctgttaggattatggtgctttgcctgggcgacactgcatttaacaagttacgcattgctggagctgggcgtgaataatctggcgttattaggtaaggagttaattacccggccttatttaacgttaggtattatcagctgggtaattttgcttgctttagcgttcacttcaacccaggcgatgcagcgaaaactcggcaagcactggcaacagttgcataatttcgtctatcttgtcgcgattctggccccaatacattatctgtggtccgtgaagattatttcaccgcagccgctcatctacgctgggctggctgtactgcttttagccttacggtataagaagttgcgttccctttttaaccggttacgcaagcaggttcacaacaaattatctgtataacttcatattgccgacaaagtacgcgttatccctgccggatgtggcgcgagcgccctatccggcatacacagatcgcatcaggttatgtttcgtttgtcatcaacctcaaatcaccaaaataatttattttatttcaataagatagataagtagaactgagaaagccatgctctcgtttcctaagagttgttgcattttgctatatgttacaatataacattacacatcatatacattaactctggaggaaactgttttggcgattcgtctttacaaactggctgttgctttaggtgtctttattgttagcgctcctgccttttcgcatggtcatcactcacacggcaaacccttaacagaggtcgaacaaaaagctgctaatggtgtttttgatgatgccaatgtacaaaaccgaacgctcagtgactgggatggagtctggcaatccgtttatcctttactgcaaagtggcaaacttgaccccgtctttcagaagaaagcggatgcagataaaactaaaacatttgctgaaattaaagattattatcacaaaggttatgcaacagatatcgagatgattggcattgaggacggcattgttgaattccatagaaataatgaaacaacatcgtgtaaatatgattacgatggatacaaaatactcacctataaatcaggcaagaaaggcgttcgttacttattcgaatgtaaagatcctgaaagcaaagcccctaaatatatacaatttagcgatcatataattgcaccacgaaaatcatctcattttcacatttttatgggtaatgattcacagcaatctttattaaatgaaatggaaaactggccaacgtattatccatatcagttgagtagcgaagaagtggtcgaggaaatgatgtctcattgagtattctcatgataacgcctcgatgccgctttagtaagttatcataactgccactggtccatccacaaacgccactgaacgcaagctagctacagacacgctcatcactatgacgtgtctgtatattaataagctaacccgcattgagttaaccaataacggattccatacacaatacggccaacagagaaagatacctgtgctcacgccattgcttatattggctggttacaatatgcactatcaattttttaaataacaaattattaaaaccacatctgtataaggaatttttaaggttcgtgggatagcttgactgtgaaaatcacaggagctacaaaaatgaaccgattctcaaaaactcaaatttatttacattggataacgctgcttttcgttgcaataacctatgccgcgatggaactccgtggctggtttcctaaaggtagtagtacttatctgctgatgcgagaaacacattacaatgcgggtatattcgtttgggtgttaatgttttcacgcctgattataaaacaccgttatagtgatccttctattgtgccaccgccacctgcctggcaaatgaaagcggcttcgctaatgcacatcatgctttatataaccttccttgcacttcctctgctggggattgctttgatggcttacagtggaaaatcgtggagtttccttggtttcaatgtgtctccctttgttaccccaaacagcgaaattaaagcactgataaaaaatattcacgaaacctgggcaaatataggctactttttaatcgcagctcacgctggcgcagcactctttcatcactacattcagaaagataatactctgttacgaatgatgcctcgccgcaaataagtcgatccccttacaaggaaatgtgaaccatggacatcaacgcgtcataaatgtttacgcaagtgcacaatgcaccctttccactatcaacaaggaggagcagaaactgtgtaaatcgtacaatggtaagacttatcaaaaatacaggttaattttggtatttaaaccttttttacttgttagtatgatacaaaggctttcaaaaaagctgcgaaattcaacaactcttggaaattatggactttgtcccgcggctttaatctgacggccgcgttccttttttgactcaattattgaacccttctctacgcaacttcagttcccaccaccaactttgcggcagtttcataggatgaatgtctaaaagaataatggtgagcgataagaaaacgactgaataactgcacattttcgctcgaaagcttcctgtcagatccatagcgaatcaagtgctgaatgtcacagtatcgaacagaaaacagtgacgatctaacccttcaagaatattctacgattgttctgtttaggaaaagcaaggcgggaagtcgggagataagtcattgataaagtggcggagagagggggatttgaacccccggtagagttgcccctactccggttttcgagaccggtccgttcagccgctccggcatctctccgttcagatggttgccatgatgccaggaaatttggcattttaacagtccctgtccgtgcaattttgttcaagtgacgagtttgcgagcaaaacgatgattaagtggccctggaaagtacaagaatcagcacatcaaactgcccttccctggcaggaagcactatcgatcccccttttaacgtgtctgacggaacaggaacaaagcaaattagtcactcttgccgaacgttttttacagcaaaagcggcttgttcctttacagggctttgaactggattcattaagaagctgccggatagcacttctattttgcctacccgttctggagttaggactggaatggctggatggttttcatgaagtcttaatttatcctgcgccatttgtggtcgatgatgaatgggaagacgatatcggtctggtgcataaccaacgtattgttcagtcaggtcagagctggcagcaagggcctatcgttttgaactggttggatatacaagattcttttgatgcttctggttttaacctgattattcatgaagtcgctcataagctggacacccgtaacggcgatcgcgccagcggagttccctttattccgttgcgtgaggttgctggctgggaacacgatcttcatgctgcaatgaacaacattcaggaagaaatcgaattggttggcgagaatgcggcgagcattgatgcttatgcagccagcgatcctgctgaatgttttgccgtactttctgaatatttctttagcgccccagaactttttgctcctcgtttcccttcattgtggcaacgtttctgccaattttatcaacaagatcctttgcagagactgcatcacgctaatgatacagactcgttttcggcgacgaatgttcattaattaacaactttgcagattaattaaccaattgaaatgacttatgaaatttagtgttgacagacaaggtaccgctaagtaatattcgccccgttcacacgattcctctgtagttcagtcggtagaacggcggactgttaatccgtatgtcactggttcgagtccagtcagaggagccaaattctaaaaattcgcttttttagcgcaatgtcactgaccttagttgaacattgttttttaacggatagcgggtttttaacatcttaagcgccctcgacctttatggttgagggcgttttgctatgaacgccatcaccattttcccctcgattataaaacttgagttattcagtagtctcccctcttgcaactcacacccaaaactgcctaacgaaaagttattaattttcaatcatattgctatcagtatttacattttttcgctgtgctagaaagggcgcatttatgttagctcgttcagggaaggtaagcatggctacgaagaagagaagtggagaagaaataaatgaccgacaaatattatgcgggatgggaattaaactacgccgcttaactgcgggtatctgtctgataactcaacttgcgttccctatggctgcggcagcacaaggtgtggtaaacgccgcaacccaacaaccagttcctgcacaaattgccattgcaaatgccaatacggtgccctacacccttggagcgttggaatcggcccaaagcgttgccgaacgtttcggtatttcggtggctgagttacgcaaactcaaccagtttcgtacgtttgctcgaggttttgataatgtccgccagggtgatgaactggatgtcccggcacaagttagtgaaaaaaaattaaccccgccgccgggtaatagcagtgacaacctcgagcaacagatagccagtacttcacagcaaatcgggtctctgctcgccgaagatatgaacagcgagcaagcggcaaatatggcgcgtggatgggcctcttctcaggcttcaggcgcaatgacagactggttaagccgcttcggtaccgcaagaatcacgctgggcgtggatgaagattttagcctgaagaactcccagttcgattttctccatccgtggtatgaaacgcctgataatctctttttcagtcagcatactctccatcgtactgacgagcgtacgcagattaacaacggcttaggttggcgtcatttcactcccacatggatgtcgggcatcaacttctttttcgaccacgatcttagccgttaccactcccgcgccggcattggcgcggagtactggcgcgactatctaaaattaagcagtaacggctatttgcgactgaccaactggcgcagcgcacctgaactggacaacgattatgaagcacgcccggccaatggctgggatgtacgcgcagaaagctggctacccgcctggccgcaccttggcggtaaactggtctatgaacagtattatggcgatgaagtggccctgttcgataaagacgatcggcaaagtaatcctcatgccataaccgctggacttaactatacccccttcccgctgatgaccttcagcgcggagcaacgccagggtaaacagggcgaaaatgacacccgttttgccgtcgattttacctggcaacctggcagcgcaatgcagaaacagcttgacccgaatgaagtcgctgcacggcgtagccttgcaggcagccgttatgatctggtggatcgcaacaacaatatcgttctggaatatcgcaaaaaagaactggttcgcctgaccctgacagaccccgtgacagggaagtcaggagaagtgaaatcactggtttcgtcgctacaaaccaaatatgccctgaaaggctataacgtcgaagccaccgcactggaagctgccggtggcaaagtggtcacaacgggtaaagatattctggttaccctgccggcttaccggttcaccagtacgccagaaaccgataacacctggccgattgaagtcaccgccgaagatgtcaaaggcaatttgtcgaatcgtgaacagagcatggtggtcgttcaggcacctacgctaagccagaaagattcctcggtatcgttaagtacccaaacattgaacgcggattcccattcaaccgccacactgacttttattgcgcatgatgcagcaggtaatcctgttgtcgggctggtgctctcgacgcgtcacgaaggtgttcaggacatcaccctttctgactggaaagataatggtgacggaagctatacccagatcctgaccacaggagcgatgtctggcacgctgacgctgatgccacagctgaatggtgtggatgcggctaaagcccccgccgtggtgaatatcatttctgtttcgtcatcccgaactcactcgtcaattaagattgataaggaccgttatctctccggcaatcctatcgaggtgacggtagaactgagagatgaaaatgacaaacctgttaaggaacaaaaacagcaactgaataacgcagtcagcatcgacaacgtgaaaccaggagtcactacagactggaaagaaaccgcagatggcgtctataaggcgacctataccgcctataccaaaggcagtggacttactgcgaagctattaatgcaaaactggaatgaagatttgcataccgctggatttatcatcgacgccaacccgcagtcagcgaaaattgcgacattatctgccagcaataatggtgtgctcgccaatgagaatgcagcaaacaccgtctcggtcaatgtcgctgatgaaggaagcaacccaatcaatgatcataccgtcacgtttgcggtattaagcggatcggcaacttccttcaacaatcaaaacaccgcaaaaacggatgttaatggtctggcgacttttgatctgaaaagtagtaagcaggaagacaacacggttgaagtcacccttgaaaatggcgtgaaacaaacgttaatcgtcagttttgtcggcgactcgagtactgcgcaggttgatctgcagaagtcgaaaaatgaagtggttgctgacggcaatgacagcgtcacaatgaccgcgaccgtccgggatgcaaaaggcaacctgctcaatgacgtcatggtcactttcaatgttaattcagcagaggcgaaactgagccaaaccgaagtgaatagccacgacgggatcgccacagctacgctgaccagtttgaaaaatggtgattatagggttacggcctctgtgagctctggttcccaggctaatcaacaggtgaattttatcggtgatcaaagtactgctgccctgaccctcagtgtgccttcaggtgatatcaccgtcaccaacacagctccgcaatatatgactgcaaccttgcaggataaaaatggcaacccactaaaagataaagaaatcaccttctctgtgccaaacgacgtcgcaagtaagttctcgattagcaacggaggaaaaggcatgacggatagtaacggggttgcaatcgcctccctgaccggcacgttagcgggcacgcatatgatcatggctcgtctggctaacagcaatgtcagcgatgcacagccaatgacgtttgtggcggataaagacagagcggttgtcgttttgcaaacatcgaaagcggaaatcattgggaatggcgtggatgagacaactctgacagcaacagtgaaagatccgtcgaatcatccggtggcggggataacggtaaacttcaccatgccacaggacgttgcggcaaactttacccttgaaaataacggtattgccatcactcaggccaatggggaagcgcatgtcacgctgaaaggtaaaaaagcgggcacgcatacggttaccgcaacgctgggtaataacaataccagtgattcgcagccggtaacatttgtggcggacaaagcctcggctcaggttgtcctgcagatatcaaaagatgagatcacaggtaatggcgtcgatagcgcaacgctaactgcaacggttaaagatcagttcgacaatgaggtgaataatcttccggtaacattcagctcagcctcttcaggactcaccctgaccccgggagtaagtaataccaacgagtctggcatcgcgcaggccactctcgcaggcgttgcctttggtgagaagacggttactgcatcactggctaataatggtgccagcgacaacaaaactgtgcattttattggcgacacagcggcggcaaaaattatcgagttggcgcctgtcccagacagcataatcgccggtaccccgcagaacagctccggcagcgtcatcaccgccacagtcgttgataataatggctttccggtgaaaggtgtgactgtgaacttcaccagcaacgcagcgacagccgaaatgacgaacggcggtcaagccgtgacgaacgaacagggtaaggctaccgtcacttataccaatacccgctcctcgatagaatcaggagcgagaccggataccgttgaggccagtctggaaaatggtagctccacgcttagcacatcaattaatgtcaacgctgatgcgtctacggcacatctcaccttgctacaggcactttttgatacagtctccgcaggcgagacaaccagtctgtatattgaggtgaaggataattacggcaacggtgtcccccagcaggaggtaaccctcagcgtttcaccaagtgaaggcgtgacccccagtaataacgctatatatactaccaaccacgacggcaatttttacgcaagctttaccgctacaaaagccggggtttatcaattgacggcaaccctcgaaaatggcgattcgatgcaacaaacagtgacctatgtgccgaacgtcgcgaatgctgaaatcacgctggcagcctcgaaggatccggtgattgccgacaataacgatctcacgacactaacagcaacagtcgctgatacagagggcaatgcgatagccaacactgaggtaacatttactctgccggaagatgtgaaggcgaacttcacgctgagcgatggcggtaaagtgattactgatgctgaaggcaaagcgaaagtcacgctgaaaggtacaaaagcaggcgctcatactgttacagcatcgatgactggcggtaagagtgagcagttggtggtgaactttattgcggatacgctcactgcgcaggttaatcttaacgttaccgaggacaattttatcgctaataacgtcgggatgaccaggctgcaggcaacagtgactgatggaaacggcaacccgttagccaatgaggcggtgacattcacgctaccggcagatgtgagcgcaagctttactctcggacaaggcggttccgccattactgatatcaacggcaaggctgaagttacactgagcggtacaaaatccggcacctaccccgtgacagttagcgtgaacaattatggtgtcagtgatacgaaacaggtgactttgattgccgatgctggtaccgcaaaactagcctccttaacctctgtatactcattcgtcgtcagcacgaccgagggcgcaaccatgacggcaagcgtcactgacgctaacggcaacccggtagaaggcataaaagttaatttccgcggaacctccgtcacgctaagcagcaccagcgttgaaacggatgatcggggtttcgctgaaattcttgtgacaagcaccgaggtcggactgaaaacagtttcagcctctctggcagataaacctactgaagtcatctcgcgattactgaatgccagtgcagatgttaattctgcgacgattaccagtctggagataccggaaggtcaggtaatggtcgcacaagacgtagcagttaaagctcacgttaacgaccagtttggcaacccggttgcgcatcaacccgtgacattcagtgcagagccatcctcgcaaatgatcatcagccagaatacggtctctactaatacgcagggtgtagccgaggtcaccatgacgcccgaaagaaacggttcgtatatggtgaaagcatccctgccgaatggagcctcacttgagaaacaactggaggctattgatgaaaaactgacactcacggcgtccagtccgcttatcggtgtctatgcccctacaggcgctactctgacggcaacgctaacctctgcaaatggcactccagtggagggtcaggtcatcaactttagcgtaacgccagaaggggcgacgttaagtggcggaaaagtgagaactaactcttcaggtcaggctccagtcgttttgaccagcaataaagtcggtacatatacggtgactgcatctttccataacggcgtaacaatacagacacagacaaccgtgaaagtcactggcaactcaagcaccgcccatgttgctagctttatcgctgatccatcgactatcgccgccaccaacactgatttaagtaccttaaaggcaacggttgaggatggcagtggtaacctgatcgaaggtctcactgtgtacttcgccttaaaaagcggctctgccacattaacgtcattaacagcggtgaccgatcaaaacggaatcgcgacaacaagcgtgaaaggagcgatgacaggtagcgtcacggtaagcgcagtcacgaccgctggtggaatgcaaacagtagatataacgctggtggctggcccggcagacacctcgcagtccgtccttaagagcaatcggtcatcactgaaaggggactataccgatagtgctgaattacgtcttgttctgcacgatatatcaggcaatccgatcaaagtttctgaagggatggaatttgtgcaatcaggtactaacgtgccctatataaaaattagcgcaattgattacagtctaaatatcaacggtgattacaaagccactgttacaggaggcggagagggtatcgcaacgctgatccctgtattgaatggtgttcatcaagctggtctgagtaccacaatacaattcactcgcgcagaagacaaaataatgagcggtacagtatcagtcaatggtactgacctaccgacaactacattcccttcgcaggggttcaccggggcgtattatcagttgaataatgacaactttgccccaggaaaaacggcggctgattatgagttttcaagctctgcctcctgggtcgatgttgatgctaccggtaaagtgacatttaaaaatgtcggcagcaattcggaaaggattacggcgacgccaaaatcaggaggccctagctatgtatacgaaatccgtgtgaagagttggtgggtgaacgccggcgaggctttcatgatatacagccttgctgaaaatttttgcagcagcaatggctacacgctccccagagcaaactatttaaaccactgtagttcccgaggcatcgggtcactgtacagtgaatggggagatatggggcattacacgactgacgctggttttcaatcaaatatgtattggtcatctagtcccgcaaactcaagcgaacaatacgtagtttccctggcaacaggtgatcaaagcgtatttgaaaagcttgggtttgcttatgcgacatgttataaaaacctgtgattttccgttataatttcttaaagagtgttccattcggggcactcttttttacattccctctacagaactagcccttctctcacagaaaatgaataaataaaaatgcggcaccgccagaatcgcgttcgatgtgactatgatcattttcggtgagtactgctttgatctaaaggctggttttctgtgatgattgaccagcctcagagtattgatgacaccaccgttcataacagatcggcattactatgcataagtactgtctcatattctcgccaaaacactttttaatgcctttgcgaattcatccagacttatattgtcaattttttgcccaacgacgactgactccgagacatcggccattgcgggccatcgcgttttgtaatcagcataaattgcaacaacaggggtattataggcacttgccatatgtaatattgaggtgtcaggagttattgcgatataagcatcttttatgattgctgctgaacgtttaatcgagggtggtaaggataaacggtagacattattataacaatccactaatgccctggctttatcttcacctttgggtccatgaacgatcactattggtatatctgtttcactttaaatttttgctattagattttctgcaatcgataatgaaaatgtacgttcctgcgagctaccttctaaattgaacgcaatgtaagatcctaacgatcgcatttcctcgcgcacctcatcgagtacatcctcacttagtggcaattcatatattggcctgactgctggaaaacccgcctcacgcatcataaatgcccatgtcataggtacgggagcccggagtttctgatccatactggacgcgttcttgcacaaaggggagaagcaattcatggttataccaacaacctgaaaattcgtttttgctttcaactgactgataaataacatcgttttcaggttctttttacgcatcccctcaatgcaaagatccggcgtaccgtattgctgtgttatgttctttgctaaatcttttatttcttttaatgttgcgtgatcctgcatagtcattgtgactaatgttaatttagtctgttcaagtttaagcgcattaaagacttctaaattaattgtcgacgttacaattaaaagatgcttaattttatgcaattcaagcgcccgaataacaggaaagatggccatagcatcgccaatctgatcgggaatatggatgacaacaaagtctgttttttcaatattgaaattataagctttataatcgtagtaactaaatgcaatacgtctcaacaatgatgctaaaaacatacctaacctcgcctccctactggttataatgcaatgcagtctatcagactcatcagggtgccattttgtgcatatgcggacttttatgtttcatatctctaacctgtgggtcctctgcttaatccttaaacaacaccagcaactcctgcgctttcatcttccatcgaatttttcatgttgccgctaatcagccataaaatcatttgcagatgcgctctgtcgaggtagtctcataaggttcgtttatagatcgacggcaatgtgagttaccttttccatactaattataaaaagacagtacaaacaggatcattatggactccacgctcatctccactcgtcccgatgaagggacgctttcgttaagtcgcgcccgacgagctgcgttaggcagcttcgctggtgccgtcgtcgactggtatgattttttactctatggcatcaccgccgcactggtgtttaatcgcgagtttttcccgcaagtaagcccggcgatgggaacgctcgccgcatttgctacctttggcgtcggatttcttttccgtccgctcggcggtgtcattttcggtcactttggcgaccgactgggacgtaagcgcatgttaatgctgaccgtctggatgatgggcatcgcgacagccttgattggtattcttccttcattctcgaccattgggtggtgggcacctattttgctggtgacactgcgtgccattcagggatttgcagtcggcggcgaatggggaggcgcggcgttgctttccgttgaaagtgcaccgaaaaataaaaaagccttttacagtagcggtgtacaagttggctacggtgtaggtttactgctttcaaccggactggtttcattgatcagtatgatgacgactgacgaacagtttttaagctggggctggcgcattcctttcctgtttagcatcgtactggtactgggagcattgtgggtgcgcaatggcatggaggagtccgcggaatttgaacaacagcaacattatcaagctgccgcgaaaaaacgcatcccggttatcgaagcgctgttacgacatcccggtgctttcctgaagattattgcgctacgactgtgcgaattgctgacgatgtacatcgttactgcctttgcacttaattattcaacccagaatatggggctaccgcgcgaacttttccttaatattggtttgctggtaggtggattaagctgcctgacaattccctgttttgcctggcttgccgatcgttttggtcgccgtagggtttatatcacaggtacgttaatcggaacgttgagcgcatttcctttctttatggcgcttgaagcacaatctattttctggatagttttcttctccataatgctggcaaacattgcgcatgacatggtggtgtgtgtgcaacaaccgatgtttaccgaaatgtttggtgccagttatcgctatagtggcgctggagtcggttatcaggttgccagtgtggttggcggtggatttacaccttttattgccgctgcactcatcacttactttgccgggaactggcatagcgtcgccatttatttgctggctggatgcctgatttccgcaatgaccgctttgttgatgaaagacagtcaacgcgcttgatagcctggcgaagatcatccgatcttcgccttacacttttgtttcacatttctgtgacatactatcggatgtgcggtaattgtatggaacaggagacacacatgaataataagggctccggtctgaccccagctcaggcactggataaactcgacgcgctgtatgagcaatctgtagtcgcattacgcaacgccattggcaactatattacaagtggcgaattacctgatgaaaacgcccgcaaacaaggtctttttgtctatccatcactgaccgtaacctgggacggtagcacaaccaatccccccaaaacgcgcgcatttggtcgctttacccacgcaggcagctacaccaccacgattactcgccctactctctttcgttcgtatcttaatgaacaacttacgttgctgtatcaggattatggtgcgcatatctcagtgcaaccctcgcagcatgaaatcccttatccttatgtcatcgatggctctgaattgacacttgatcgctcaatgagcgctgggttaactcgctacttcccgacaacagaactggcgcaaattggcgatgaaactgcagacggcatttatcatccaactgaattctccccgctatcgcattttgatgcgcgccgcgtcgatttttccctcgcacggttgcgccattataccggtacgccagttgaacattttcagccgttcgtcttgtttaccaactacacacgttatgtggatgaattcgttcgttggggatgcagccagatcctcgatcctgatagtccctacattgccctttcttgtgctggcgggaactggatcaccgccgaaaccgaagcgccagaagaagccatttccgaccttgcatggaaaaaacatcagatgccagcatggcatttaattaccgccgatggtcagggtattactctggtgaatattggcgtgggaccgtcaaatgctaaaaccatctgcgatcatctggcagtgctacgcccggatgtctggttgatgattggtcactgtggcggattacgtgaaagtcaggccattggcgattatgtacttgcacacgcttatttacgcgatgaccacgttcttgatgcggttctgccgcccgatattcctattccgagcattgctgaagtgcaacgtgcgctttatgacgccaccaagctggtgagcggcaggcccggtgaggaagtcaaacagcggctacgtactggtactgtggtaaccacagatgacaggaactgggaattacgttactcagcttctgcacttcgttttaacttaagccgggccgtagcaattgatatggaaagtgcaaccattgccgcgcaaggatatcgtttccgcgtgccatacgggacactactgtgtgtttcagataaaccgttgcatggcgagattaaacttcccggccaggctaaccgtttttatgaaggcgctatttccgaacatctgcaaattggcattcgggcgatcgatttgctgcgcgcagaaggcgaccgactgcattcgcgtaaattacgaacctttaatgagccgccgttccgataataagttctgaaccttcttatcagaaatagatgtgaaggagtaagtaagacacctggcaaatagcctgcaataatcgtgggctgtttgcttccttgggcggatacgagttttattatcgtcttaatgatttccacatattaaaagcaagtatgctttcaaaacacaattataaaaaatcccgccaacaatataagtttttataaaattaaatataagattatggctttagaatatttttatttctaatagacgagatttttcctgttatgatataatatgctgaattaacacatgttaacgatttaccagtaatgtaaataaattttcgaggagatcattccagtgggacgtaaatgggccaatattgttgctaaaaaaacggctaaagacggtgcaacgtctaaaatttatgcaaaattcggtgtagaaatctatgctgctgctaaacaaggtgaacccgatccagaattaaacacatctttaaaattcgttattgaacgtgcaaagcaggcacaagttccaaagcacgttattgataaagcaattgataaagccaaaggcggcggagatgaaacgttcgtgcagggacgttatgaaggctttggtcctaatggctcaatgattatcgccgagacattgacttcaaatgttaaccgtacgattgctaacgttcgcacaattttcaataaaaaaggcggcaatatcggagcggcaggttctgtcagctatatgtttgacaatacgggtgtgattgtatttaaagggacagaccctgaccatatttttgaaattttacttgaagctgaagttgatgttcgtgatgtgactgaagaagaaggtaacattgttatttatactgaacctactgaccttcataaaggaatcgcggctctaaaagcagctggaatcactgagttctcaacaacagaattagaaatgattgctcaatctgaagttgagctttccccagaagatttagaaatctttgaagggcttgttgatgcccttgaagatgacgacgatgtacaaaaagtttatcataacgtcgcaaatctctaattatcttttaaagaaatctgtctttacggcagatttctttaatctcatataattcttataaaaaatataatattcaactcgtcatattgattatacccccccgttcccagagaaataatatttattaaaattccagttcttctttttctgattacagaaggcaaagtggcaattacgcatagtttcccgataaagacgcgatagcgacatcccgcataaggcatttttctctttatctttgtacggtacttcatggaacagagtttttgaccttgcgaatcgtgatgtctgttggggagggacaatttgctcactgaagcgtgagactcgattaagcgcacgaaacacagaaatcaaaaaacccggtcacttttttacaaggtaaccgggtaaaaataatttttattttttaactgttttgagactcatagagatgtctcaaaactaaaatttggctcctctgactggactcgaaccagtgacatacggattaacagtccgccgttctaccgactgaactacagaggaatcgtgagaacgaggcgaatattagcgatgcccacccacaatgtcaaagcctgttttttaaatttgaaatcgtttgctgaaataatctgcattttgtcgtttattccgacacaactggctttttttcacacttttgcggctcgggtcgagggtatttccatagccaacgtccagtaaccattcgccagtaaaacagcacggcccgcacagcccagtcggcaaacattcccatccagacaccaaccacaccccagccaagcatgattcccagcacataaccgactacaacccgacaaccccacatgctcaacatcgaaacccacatggcgtaacgggcatcacgagcacctttaaatccagcgggtagcacccatgaggcggaccaaataggcataaataaagcatttagccaaatcagaatcacaacgacatgtttaacctgtggatcctgggtgtaaaacgatgccataaccccggcaaagggagccgttagccaggcgatggccgttaatccaagagtggaaagccagaacacatgccgcaactgaatctctgcttgcgctatctgccctacccccaaccttcggcctgtaatgatcgtagaagcagagccgagcgcacttccgggtaagttgataagagccgcaattgaaaacgcgataaaatttccggcaataacactggtccccatcccggcaacgaacatttgggttaataaccgaccactggtaaataacactgattcgacactcgcgggaataccaatccccatgacttcccagataatgctaaaattcagcggtttaaaatagctctttaacgaaatccttagcgcaggattaaaaccaatcgccagcacccacaaaattgcaactgcgccaatataacgagaaatggttaaacccagccctgccccgacaaatcccagtcccggccaggagaaaaggccgtaaatcaatatgccgctaataataatattaagaatattcaggctaccgttaatcaatagcggtattttcgtattccctgcaccacgaagtgccccgctaccaataagagtgatggcagctgctggataactgagtaccgtcagctccagataagtcaacgccagtgctttaacttctgtcgtggcatcacccgcgacgaaatcaataatttgttcgccaaaatgatgaataagcgttgccaacagtacggcaaacaacgtcatgatcaccaatgactgccgcgtcgccaccctcgctcgtcgtcgatcccgcttaccgagactaaatgccacaacgacagtagtaccaagatcgatagcagcaaaaaaagccataatgaccatattgaagctgtccgccaatcccacgccggccatcgcatcttttcccagccagctgaccagaaaagtgctcagaacccccatcaacaggacacaggcattctccatgaagataggaacagcaagcggggttatctcgcgccagaacaacactttgtagctcttgcgtttagcgtgccagcgagtgccgtgaacaacctggcgtaaagcagaggagatattcaaagccgaccttaattgcagaaagtgaaaccacatttcaaataatgagggagaatcagcaaagctgcaaagattttcgccaacaaattgtctgcaaatgcaacaaactgttgatagaaacggcaaacagttggggaatttaaaaatcgggtttgacaaaagatttttcgccgttaagatgtgcctcaacaacgattcctctgtagttcagtcggtagaacggcggactgttaatccgtatgtcactggttcgagtccagtcagaggagccaaattcctgaaaagcccgcttttatagcgggatttttgctatatctgataatcaatttcctcttcactgctttccatcacctgccgcttgatatcctcaactgacagtcctgcattacaaagttccagaaagcgccagacatagttacgctgaagttgtcctcgcttcagtcccaaccagacagtattagcatcaaaaagatgccgcgtatccaggcggattaaattctcttcctcttgttcgccactggattgctcggcaactaatccgatcccaagcccaagagcaacataggttttaatgacatcagaatcctgcgcacttaatacaatatctgccagcaaacctttgcgggcaaatgcgtcatcaatacgtgagcgccccgtaatcccctgtcggtaagtgattaacggccacttcgctattgattccagcgtcaatggtgaaatttgcgtcaagggatgatcgtgtggaacaagcaaactatggtgccaacgaaaccacgggaaggcgacgagctgcgggtcattactcaaacgctcgctggcgataccaatatcagcttcgccattttgcaacaatgtcgcaatttcctgtggcgtcccctggattagctcgagccgaacctccgggaaaagttcgcgaaaagctttaatgacctctggcaagctataacgtgcctgagtatgcgtcgttgcaatagtgagaacgccagacgtatcgttggtaaacaggtctgcaagccgacgaacattactggcttcattcagaatacgttctgcaatgaccagtaatgctttgcccggttcagtcatgcccagcagtcgcttacctcgtcgaacaaatatttcgatgccaagttcatcctccagttcccgaatatgacggctgacgcctgactgtgaggtaaaaagcatattcgcaacctctgtcaggttgtaatcctgacgtgcagcctcgcggattatctttagttgttggaaattcacggtaaactccgggcagttcagatttcccgttattgttaaagtctaatgcccggcataacaaataataaaaacccgcatcttattccatcccgatataacacttagctcaccaattgccactgccttttttccatcactggagaactaatcactgacattaacaactctttcactgcctgtgcctgtggcgataagttcgctctggcgggtaaatttaatgacaaagagagactcatggaaggagtggtaatgcgtgacatccacccatttactgcgccacataacgaacgcgcggccgattcgggtaatactgcaacgcccatgccgctggcaatcgctgcggtaagcgtggcaatagactcaatttcaccaataacttttgccgtgagtcgccgtagggaaaaagcctcatcaacacgaagtctaatagcactgtaatcactggggagaaagaggttcatttgcgcaatagcattcacatcaacgctttgccccgggcaatcttgagttcctaccagaaaaagatcttctttcagcaaagcctgactggatacaccagccacaggggaatgctcataaatcaccgccatatcgagttggtgatttatcaatttttcgttaagcactgcaccactattttcatgaagatagataacgatctccggaaattcagcgcgaaccgcctgtaataagggcatggtgatggatgacgcagcggttcctggtgcaaagccaatcgagacttgccccgataatgcctgaccaacgttatgcaccgccagttgggcctgttcacactgacgtaaaatggcccgcgcatgggtatagagaatttttccggcgtctgttggtgtaacgccccgctttgtacggatcaaaagttgttgatttaactcaccttccagtgtggcaacctgctggctgagcgctggttgtgcgatatgcaatacttcagcagcctgggtcaggctaccaatatctacaatttttacgaagtatttcaggcgtctgaagttcatgttgcctccggtttttaagaatcggcccaagtgccgccattacttacaaccagattgcaagatgcttgccagttttattttggtgttgatgtacaagctaaccaactgtcaaataagagattatgatagattcgtcatttgctcctttaatcagctgtcgcgttcccctgccctataaaaggagggtatgcaccacgatggttcattacccaataagattgaaagctcaccactttgttgaaattgacagcaaacaaacaaaaaaatgcatttcaccctttgacatcaccatgcactgccattaatatgcgccccgttcacacgattcctctgtagttcagtcggtagaacggcggactgttaatccgtatgtcactggttcgagtccagtcagaggagccaaattcaaaaaagcctgctttctagcaggctttttgctttctaattaccaacgctcttaaaacatctgtcttgaaccagaactaatttgcacaggcattcccgatcgacgttgcaacgcagcatttgcgcgatttacatcaacttcttgcccgttgataaacgcccgcaaagatggggttaccggcaatggcacttttcggtcagactcatattctgcacgattgcgcgacaatggctcatgaacttccagccagttcgagccatctggttcagtggtgtattttactggctggtcgataatttgcacacgcgtcccaacaggaacattatcaaacagatatttgatatcgtcattgcgcagacgaatacagccctgacttacccggagcccaataccaaaattggcattggtaccatggatggcatacaacctgccaatataaatcgcgtacagccccatgggattatcggggcccgcaggaacaaatgcgggcaaactctcccctcgtttcgcatattcgcgccgagtgttcggcgttggcgtccaggttggagcttcttgtttacgttcaacggtagtcacccagttacgcggggtttctcgcccagcctggccgataccaataggaaagacttccacagtattactgtctggtgggtagtaataaagacgcatctcagcgacgttaacaacaatccctttacgaacagtgtcgggcaaaatcagttgctgcggaatggtgagttgcgagccagacttcggcaaaaaaacatcagcgcccgggttcgcttccagcatgttacttaacccttgcccgtattgtgcggcaaaagtctccagcggctgggtattgtgatcaggaacagttacagtaaacgactgccccactaaacggctaccctctggaggtaatggataagttaccgccaggctagtatggctggcaaaaagcagagcaaatgagcaaagaatatttacacgacgcatcatgtccctttcctatgtcgcgaaagctatccgttaagtatagcttttatcagacttttcgtttttaactgttcaaatcagaagtcgtattccccggtagaacaatattactggcagcaagttcgcccatgttgttgtatatcgcacaggcagcttcgatgatgggcatcgccagagctgcgccactcccctcacctaaacgcatctccatattgagataaggctccagccccaaatgcgagagcgctatacgcgcgcctttttctgccgacaggtgagaaggaatgagatacggtttgatcgcaggagacatctggcaggctgcgagcgcagcagcataagaaagaaatccatccagcaacacgggtaaaccgcaggaagcagcacctaacatcactccagctattccgaccaaatcaaatccacccacttttgccaggacatcaacaccatcctgaggatttggttgattcaacgtaatcgcccgacgcacaacatcaattttattagccagtttatctgtcggcaggtttgcgccaatcccaaccacttcttcaggatcccggccagtgattgtgctgactattgctgctgccggtgtcgtgtttgccatccccagttcacctacaccaaacagcgtgacaccgttttttgccagctcctgcgtataacatatgacgtccaaaagcaacttttcagcctgacggcgactcattgccggagctgaagcaatattgccgctacctcgtgcgacacgcatgttgataagcccggggataggctcagcagtatcaataccaacatcaattacgtggacgttagcgcccgcttgttctgccagcacacacacgccggttgttccacgggtcatattttcagcctgtatggctgtcacttcttttggagaaatagcgaccccttcctcccagacgccgtgatcggcacacataaccagtaccgcttttttgcccacatgcggtatgccattcaaccccggcattcctgccagttgtatggcaagcacctccagctttcccaggctaccaacaggtttgagtaacccgtcaatatgccgttgtgcacgcgacatagcggtagaatcgatggctgggatcgtattcagtaaatcggcaagtatttgcatctcacgtctctttatagcagtgccagcaggaagaccagttcaccaagctctatggctgctcccagcgtatcgcccgtttgcccgcccagcgtacgtttgagaagctgaccgaggatgaaaatcgccaccatcgtcaccaccatagcagccacaccatgcatacccggcaataatacggcagcaaaaatagcggctaagccgagtgtgacgcaggtttgtcgcccatcaattttgccaatgaacacattgccaagcccttcttcccgcgcataacgatgacgatacatcaataatgcggcagtcccgcggctgaccgcacatgctgccgccagcgatgcaaggatcgattcgccacgcagagccaactcgcttaacaccagaatctttgccagtaccacaaaaatcaatgccagaccgccgtgggtgcctaaacggctatcacgcatgatttccaacatgcgatcgcggctacgtgcagaaaatacgccatcacaggtatcagcgaggccgtccagatggaatcccccggtcatcagcaccagcacaagtacgctaaacagtgccgccagtggtgcgccacaccatgcctgcagcaccatgaagaccagcccgctaatcgcgccaagcaataatccaatcaaaggaaaagtaataataccgcgagaataatgctcgaaatccagtccctgggaccagcgacgcggtacaggcagacgcgtaataaatgagagcatcgcccaaaataatttactcatttgatttttactccaatacccgaaaccaccagccatacttcatttgccgcagcggccaactgctgatttacccgcccggcaatatcacgaaaatgtcgtgccagacgactctccggcacaatccccattcccacttcgttagtcactaatacaacctttgcggggcaacgttggcaggcagcaatcaacgactgaatctcagcattaatcgcctgttccatcgcctgataatcccattcatcagggtctttatcgccgccataatcaaacaacagattagtcaccattgtggtaacgcattcaagcaacacaacctcattcgggttaatgtctgcatgaattaattcatcaagatgttgccagcgctccactgtgcgccagtgctccgggcggccttgccgatgatgttctatccgtgcagccatctcatcatcaaggatttgcgaggtagcgatatacagaacctgtgaagagtccccaataagcgcctctgcgtggcgactcttcccgctccgtgcgccccccgtcaccaaaatcatcataccgactcctgattcaaatgtatgatggtattcattgaacagaacaatggatcccccaccgttgctgaccgcaaaacatttacgcgattaatactgcgcgtaatataattaaaaatccagcattctcaatccattacgaaataagatggcattacggaatagccagactttctcgtgttaacgtccgacaaaatgcgtcattgacagcggtttctgtggattgacacatttcattcagataatgaattaatgctactgccggaacaaccagcaaacgggcattgtgttctgaaatccaggctattgattcaacgtcagcgacagatctgcgctgtaaaagaacttgtaaaacaacgtaatagaattatccggaatggtggcgactatgcactagggaaggtgcgaataagtggggaaattcttctcggctgactcagtcatttcatttcttcatgtttgagccgattttttctcccgtaaatgccttgaatcagcctatttagaccgtttcttcgccatttaaggcgttatccccagtttttagtgagatctctcccactgacgtatcatttggtccgcccgaaacaggttggccagcgtgaataacatcgccagttggttatcgtttttcagcaaccccttgtatctggctttcacgaagccgaactgtcgcttgatgatgcgaaatgggtgctccaccttggcccggatgctggctttcatgtattcgatgttgatggccgttttgttcttgcgtggatgctgtttcaaggttcttaccttgccggggcgctcggcgatcagccagtccacatccacctcggccagctcctcgcgctgtggcgccccttggtagccggcatcggctgagacaaattgctcctctccatgcagcagattacccagctgattgaggtcatgctcgttggccgcggtggtgactaggctgtgggtcaggccgctcttggcatcgacaccaatgtgggccttcatgccaaagtgccactgattgcctttcttggtctgatgcatctccggatcgcgttgctgctctttgttcttggtcgagctgggtgcctcaatgatggtggcatcgaccaaggtgccttgagtcatcatgacgcctgcttcggccagccagcgattgatggtcttgaacaattggcgggccagttgatgctgctccagcaggtggcggaaattcatgatggtggtgcggtccggcaaggcgctatccagggataaccgggcaaacagacgcatggaggcgatttcgtacagagcatcttccatcgcgccatcgctcaggttgtaccaatgctgcatgcagtgaatgcgtagcatggtttccagcggataaggtcgccggccattaccagccttggggtaaaacggctcgatgacttccaccatgttttgccatggcagaatctgctccatgcgggacaagaaaatctcttttctggtctgacggcgcttactgctgaattcactgtcggcgaaggtaagttgatgactcatgatgaaccctgttccatggctccagatgacaaacatgatctcatatcagggacttgttcgcaccttccctagaacaccacaatttcgctctctcggtaaggcactgtcacagcattcaacagaatgtgacttgccagatttattagcgccaccagatgtttaaccgggtaaccacgacccagtcggggatatattccatcttctcgctgacatcatcaagaataaaaaggtttatcacactcagagcaacgttcttcagcaggcgggataattcttcaacatttagaagatgtgttattaaaggcatacaaactggacgtattgtattttcttttggtggttgacctaaggtagcagtttatcctgatgcgctgagatttctgtaatatctacgtcaacattctcctcgaatagaaaatgcagccccggcaagtgattcacattttttaacaaaacgttgttagcgtgccattttcagaagctctccaagaaagcgaattcttttctcaaattctgcattctcagacacagctttctactccatggtaatggcccaaatacgaagttgctcaggatcattagtggtgctgagaagttaaataaccatgcggagtaccactcgtcatcacgtatttatatatcatgaagctattgttgtgttttgtacatcagtagatatattctgatatactccttttgctagacataacctttcacctgcttgcaaagcttctgtgttctgacattgccaaattgttgcaattctgtatccagccttctttcagtcatagcttcgggccgcgataagactcactgatctgaccctgattcctcttgcagactttatagaccaattaaaatgcagtttctgcaggtcaacgtctgaccatcattgtcatcactctggccattagagtaaccttctgcattcatccttttgtaaaaagtttatattagtatcagcaattaaccggacctgatactgatatgagtcttaccgcatatacggtcaatttcagcaattaattacattatccacgccaaagtatttgtcatcacaatgatggtaccttctttcagacaccattttttcaactccgttttccacggaccgcactcttatgtcaagagtgcggtccgtggatacaaccagagaccgactgacacgagtcagaggaaacgacggatatgttcagtcgtaaaatatctatcaaaaaacatgattaaggtcaaaaatgtttgatatttacaatttatgaagatgacaataattatagatatatgagaacataaatgaaaataattatcattacagtaatcatttgtactttgtattaatgagggatgaaatgttatataatataccttgtcgaatttatatcctttccactctgtcattatgcatttctgggatagtttctactgcaaccgcaacttcttcagaaacaaaaatcagcaacgaagagacgctcgtcgtgaccacgaatcgttcggcaagcaacctttgggaaagcccggcgactatacaggttattgaccaacaaacattgcagaactccaccaatgcctccatagccgataatttgcaggacatccccggagtagagataacagacaactccttggcaggccgtaaacaaatccgcattcgtggctggatttgcccctatatttccagacatctgttatcacttaacccattacaagcccgctgccgcagatattcccgtggcgagcgataacccagcgcactatgcggatgccattcgttataatgctcgaacgcctctgcaaggttctttgctgccgttaacccgtctggtttgggcatgatactgatgtagtcacgctttatcgttttcacgaagctctctgctattccgttactctccggactccgcaccgccgtgttcttcggttcaagtcccaacatccgggcgaactggcgtgtttcattagcccggtagcatgaaccattatccgtcagccactccactggagacgacggaagatcgttgccgaagcggcgttccaccgctcccagcatgacgtcctgtactgtttcactgttgaagccgccggtagtgaccgcccagtgcagtgcctcacgatcacagcagtccagcgcgaacgtgacacgcagtctctctccgttatcacagcagaactcgaacccgtcagagcaccatcgctgattgctttctttcacggccactctgcctgtatgtgcccgtttcgatggcggtacagcaggttttcgctcaagcaacagcgcattctggcgcatgatccggtaaacacgtttggcattgatcgcaggcataccatcaagttctgcctgtctgcgaagcagcgcccatacccgacgataaccatacgttggcagctctccgataacatggtgtatacggagaagcacatccgtatcatcagtgtgacgactgcggcggccatccatccagtcatcggttcgtctgagaatgacgtgcaactgcgcacgcgacacccggagacaacggctgactaagcttactccccatccccgggcaataagggcgcgtgcgctatccacttttttgcccgtccatattcaacggcttctttgaggagttcattttccatcgttttcttgccgagcaggcgctggagttctttaatctgcttcatggcggcagcaagttcagaggcaggaacaacctgttctccggcggcgacagcagtaagacttccttcctggtattgcttacgccagagaaataactggctggctgctacaccatgttgccgggcaacgagggagaccgtcatccccggttcaaagctctgctgaacaattgcgatcttttcctgtgtggtacgccgtctgcgtttctccggccctaagacatcaatcatctgttctccaatgactagtctaaaaactagtattaagactatcacttatttaagtgatattggttgtctggagattcagggggccagtctagtggcgaagcatcctcccgtgttttaattctcattgatggtcaggaggtaacttatcagcgcgccggagataattatggtgtgggactgttgatagatgagtctgcgctggagcgtgttgaggtagtgaaaggtccatattccgtactgtacggttcacaggcaattggcggtattgttaacttcatcaccaaaaagggtgaatctccggactccctatatcacttaaattgatacaactttttagagtagtcattagtgaacagataattgataactcagaaccagtaaaatgcaaaagacgcaccacgctgggaaaatcgctgctattcagcagagttttgtatcgagaatggtggccagccacttattgctctcgcgtaagcgggtaccgtgacattctgcctgaacttgacctggtactgtggctgattaaagccgatgaccgtgccctgtctgtggatgagtatttctggcgacacatcctgcagtgcggacatcagcaggtgctgtttgtggtgacgcaggccgacaaaacggagccctgccatgaatgggatatggccggtattcagccttctcctgcacaggcacagaatattcgcgaaaaaacggaggcggtattccgtctgttccggcccgtacatccggttgtggccgtatcggcccgcaccggctgggaactggatacgctggtcagtgcgctcatgacagcgcttcccgaccatgccgccagtcccctgatgacccgactgcaggacgagctgcgcacggaatctgtccggtctcaggcccgtgaacagtttaccggtgcggtggaccggatatttgacacggcggagagcgtctgtattgcctctgttgcacgcacggttctgcgtgccgtccgtgacacggtggtctctgttgcccgtgcggtatggaactggattttcttctgaacctgtcgtgactgatgccctccctgactctgagtctgctcacaaaagcactgttttcgttactgtctctcttgtccgtgcaatagctcaataatagaataaaacgatcaatatctattttatcgatcgtttatatcgatcgataagctaataataacctttgtcagtaacatgcacagatacgtacagaaagacattcagggaacaacagaaccacaattcagaaactcccacagccggacctccggcactgtaaccctttacctgccggtatccacgtttgtgggtaccggcttttttattcaccctcaatctaaggaaaagctgatgaaacgacatctgaatacctgctacaggctggtatggaatcacatgacgggcgctttcgtggttgcctccgaactggcccgcgcacggggtaaacgtggcggtgtggcggttgcactgtctcttgccgcagtcacgtcactcccggtgctggctgctgacatcgttgtgcacccgggagaaaccgtgaacggcggaacactggcaaatcatgacaaccagattgtcttcggtacgaccaacggaatgaccatcagtaccgggctggagtatgggccggataacgaggccaataccggcgggcaatgggtacaggatggcggaacagccaacaaaacgactgtcaccagtggtggtcttcagagagtgaaccccggtggaagtgtctcagacacggttatcagtgccggaggcggacagagccttcagggacgggctgtgaacaccacgctgaatggtggcgaacagtggatgcatgagggggcgatagccacaggaaccgtcattaatgataagggctggcaggtcgtcaagcccggtacagtggcaacggataccgttgttaataccggggcggaagggggaccggatgcagaaaacggtgataccgggcagtttgttcgcggggatgccgtacgcacaaccatcaataaaaacggtcgccagattgtgagagctgaaggaacggcaaataccactgtggtttatgccggcggcgaccagactgtacatggtcacgcactggataccacgctgaatgggggataccagtatgtgcacaacggcggtacagcgtctgacactgttgtgaacagtgacggctggcagattgtcaaaaacgggggtgtggccgggaataccaccgttaatcagaagggcagactgcaggtggacgccggtggtacagccacgaatgtcaccctgaagcagggcggcgcactggttaccagtacggctgcaaccgttaccggcataaaccgcctgggagcattctctgttgtggagggtaaagctgataatgtcgtactggaaaatggcggacgcctggatgtgctgaccggacacacagccactaatacccgcgtggatgatggcggaacgctggatgtccgcaacggtggcaccgccaccaccgtatccatgggaaatggcggtgtactgctggccgattccggtgccgctgtcagtggtacccggagcgacggaaaggcattcagtatcggaggcggtcaggcggatgccctgatgctggaaaaaggcagttcattcacgctgaacgccggtgatacggccacggataccacggtaaatggcggactgttcaccgccaggggcggcacactggcgggcaccaccacgctgaataacggcgccatacttaccctttccgggaagacggtgaacaacgataccctgaccatccgtgaaggcgatgcactcctgcagggaggctctctcaccggtaacggcagcgtggaaaaatcaggaagtggcacactcactgtcagcaacaccacactcacccagaaagccgtcaacctgaatgaaggcacgctgacgctgaacgacagtaccgtcaccacggatgtcattgctcagcgcggtacagccctgaagctgaccggcagcactgtgctgaacggtgccattgaccccacgaatgtcactctcgcctccggtgccacctggaatatccccgataacgccacggtgcagtcggtggtggatgacctcagccatgccggacagattcatttcacctccacccgcacagggaagttcgtaccggcaaccctgaaagtgaaaaacctgaacggacagaatggcaccatcagcctgcgtgtacgcccggatatggcacagaacaatgctgacagactggtcattgacggcggcagggcaaccggaaaaaccatcctgaacctggtgaacgccggcaacagtgcgtcggggctggcgaccagcggtaagggtattcaggtggtggaagccattaacggtgccaccacggaggaaggggcctttgtccaggggaacaggctgcaggccggtgcctttaactactccctcaaccgggacagtgatgagagctggtatctgcgcagtgaaaatgcttatcgtgcagaagtccccctgtatgcctccatgctgacacaggcaatggactatgaccggattgtggcaggctcccgcagccatcagaccggtgtaaatggtgaaaacaacagcgtccgtctcagcattcagggcggtcatctcggtcacgataacaatggcggtattgcccgtggggccacgccggaaagcagcggcagctatggattcgtccgtctggagggtgacctgatgagaacagaggttgccggtatgtctgtgaccgcgggggtatatggtgctgctggccattcttccgttgatgttaaggatgatgacggctcccgtgccggcacggtccgggatgatgccggcagcctgggcggatacctgaatctggtacacacgtcctccggcctgtgggctgacattgtggcacagggaacccgccacagcatgaaagcgtcatcggacaataacgacttccgcgcccggggctggggctggctgggctcactggaaaccggtctgcccttcagtatcactgacaacctgatgctggagccacaactgcagtatacctggcagggactttccctggatgacggtaaggacaacgccggttatgtgaagttcgggcatggcagtgcacaacatgtgcgtgccggtttccgtctgggcagccacaacgatatgacctttggcgaaggcacctcatcccgtgcccccctgcgtgacagtgcaaaacacagtgtgagtgaattaccggtgaactggtgggtacagccttctgttatccgcaccttcagctcccggggagatatgcgtgtggggacttccactgcaggcagcgggatgacgttctctccctcacagaatggcacatcactggacctgcaggccggactggaagcccgtgtccgggaaaatatcaccctgggcgttcaggccggttatgcccacagcgtcagcggcagcagcgctgaagggtataacggtcaggccacactgaatgtgaccttctgacagaaccatcgcctctctgtggtcccggtcatcatgaccgggacccggaccggcgcaacggatcttcaacgccacattcgctggcattaacaataacatgatattcatcacggagtgactatgttacagatagtcggcgcgctgatcctgctgatcgcaggatttgccattcttcgccttttgttcagagcattaatcagcacggcttctgcgctggcagggctcatattgctgtgtctgttcggcccggccttactggctggctatatcaccgaacgcataacccggttgttccatattcgctggctggcaggcgtatttctgacgattgccggaatgatcatcagcttcatgtggggacttgatggtaaacatatcgcgctggaggctcacacctttgactctgtgaaatttattctgaccaccgctctcgccggtggtctgctggctgttcccctgcagatcaaaaacattcagcagaacgggatcacaccagaagatatcagcaaggaaattaacgggtattactgctgtttttatactgcctttttccttatggcgtgttctgcatgcgcaccattgatcgcgttacagtacgatatttcaccgtcactgatgtggtggggcgggttgttgtactggctggctgcattagtgacgctgctatgggcggccagccagatccaggcgctgaaaaaactgacctgtgccatcagccagacactggaagaacaaccggtgctcaacagtaaatcgtggctgaccagtttgcaaaacgattacagccttcctgactcactgacggagcgcatctggctgacgctcatttctcaacggatttcccggggagagctgagggaatttgaactggcagacggaaactggttactgaacaatgcctggtatgaaagaaacatggcagggtttaacgaacagttgaaagagaacctgtcattcacacctgatgaactgaaaacgctcttccggaaccgcctgaatttatcaccggaagcgaatgacgattttctcgatcgttgcctggacggcggtgactggtatcccttttcagaaggtcgccgttttgtatcattccatcacgtggatgagcttcgtatctgtgcctcctgcgggctgacagaagtacatcatgccccggaaaatcataagccggatccggaatggtactgctcctctctttgtcgcgaaacagaaacactgtgtcaggaaatttatgaacgcccttacaacagctttatttccgatgcaacggcgaatggtctgattctcatgaaactgccggaaacctggagtacaaatgagaaaatgtttgcttccggagggcagggacatgggtttgccgctgaacggggaaaccatattgtcgacagagtccgtctgaaaaacgcacggatcctcggtgataataatgccagaaatggagcagacagactggtcagcggaacagaaatccagacgaaatattgttcaactgcagcccgtagcgtcggtgcggcattcgacggacaaaacggacagtatcgttacatgggaaataatggccccatgcaactggaagtcccccgtgatcagtatgccggcgctgttgaaaccatgaggaataagatccgcgaaggtaaagtagaggagagatgacgcccggcgagcgcagcctcattcaacgggccctgaaaaccctggaccgccatcttcatgaacccggcgtggccttcacctccacccgtgcagcacgggaatggctgattctgaacatggcgggactggagcgtgaagaattccgggtgctgtatctgaacaaccagaatcagctgattgccggtgaaaccctcttcaccggcaccatcaaccgcacggaagtccatccccgggaagtgattaaacgcgccctgtaccacaatgccgctgccgtggtactggcacacaatcacccgtccggtgaagtcacacccagtaaggcagaccggcttatcaccgaacgtctggtacaggcactgggcctggtggatatccgggtgccggaccatctgatagtcggtggcaaccaggttttctcctttgccgaacatggtctgctttaacccttcacaaccacatcacacctgttttcacttttatcttctgtcttcagaggtatcccattatgaaaattatcacccgtggtgaagccatgcgtattcaccaacaacatccgacatcccgtctttttccgttctgtaccggtaaataccgctggcacggcagtgctgaagcgtataccggtcgtgaagtgcaggatattcccggtgtgctggccgtgtttgctgaacgccgtaaggacagttttggtccgtatgtccggctgatgagcgtcaccctgaactgagtgggaattctgatgagcagaattatcgccactaccggaccattcttagccgattttctgtaaggattttatcgtgtcagacacactccccgggacaacacttcccgacgacaatcacgaccgcccctggtgggggctgccctgcaccgtgacgccctgtttcggggcacgtctggtgcaggagggtaaccggttgcattaccttgccgaccgcgccggtatcagaggcctgttcagcgatgcagatgcgtaccacctggaccaggcctttccgctgctgatgaaacaactggaactcatgctcaccagcggtgaactgaatccccgccatcagcataccgtcacgctgtatgcaaaagggctgacctgcaaagccgataccctcagcagttgtgattacgtttatctggctgtttatccgacgcccgaaatgaaaaattaactctccagaatagccttctgctacggcctggtgttttcaccacgccacttttccatttttatatctgcatatcaggaaaatcttcagtatgaaaacattacctgtattacccgggcaggcggccagttctcgcccgtctcctgttgaaatctggcagatactgctgtcccgactgctggaccagcactatggcctcacactgaatgacacaccttttgccgatgaacgtgtgattgagcagcatattgaggcaggcatttcactgtgtgatgcggtgaactttctcgtggaaaaatacgcgctggtgcgtaccgaccagccgggattcagcgcctgtacccgctctcagttaataaacagcatcgatatcctccgggctcgcagggcgaccggcctgatgacccgcgacaattacagaacggtaaataacattaccctgggtaagtatccggaggcgaaatgatgacactggaagccgacagcgttaacgtacaggcgctggatatggggcacattgtcgttgacattgatggtgttaatatcactgaactgattaataaggccgctgaaaacggttattcactccgcgtggtggatgaccgtgactctaccgaaacaccggcaacttatgccagccctcaccagttgctgtaagacaatgcagtgatacagggtatagtgccattaaccacagaaacagcactgttgtcctgtattaagcaggcaagagaagatgtccttaccctgcgccatctgcagcttctgcaccagaaccggtgaatctcactcaacaggcttcatttctcctgacgccagcctgaatacagctggcgttttcatttataaacagaaaggaaaaccgataataatggaatggacgccccgaccatgaagcaacggtaggatattactgataaaccttccagtggaggtgcgttatggccgttttaacgattagcattgacctgacaaaaaatgaattccaaatccacggtctgggtaggaacagaaaaatctaagctcagaaaacggattaaagtaagcgtcaacggagcaccgtattgacgcttatttattggtgagaactacgttccatggcaggagttcgtcaacacggttggagggccattccggcagtatgctcagaatatggcgcagatacgcttccggatcgataccgttcagacggcaggtgcctgcttttctggcaacaagcaggaatctcagcgctgaagcaggaattagaggtaaaaacgccctaccgggccatgaatcacccggtcattggagtagtaaccaaagcagatttagccagcatggaacaaatatctttggtgaaaagttggttacgggaagctggagcgcacaacgtgttagtaaccagtgcagttaataacaatggagttacagaactttttgccttgctgcatacagaagaaggctgttgttaatttcgattggttctcggatgagaatgatgacggtgatacacagataagaatcaatgagcaatgagggttgccgggcaaccctcattgaataaaacgggaattacttcgcttcgccgtttttcatttcgcccatagctttcagctttttggagatatcgcggcgttctttggagagctcggcatttttgatgatgtaatcgtcaacgcgatcttcatagtcacctttcatgctggcgatgatgccctggattgcttcaacgctcatccccggcttgatgtaatcgctcaggttgtccagcagcaggacgcgcttctggttgtcacggatctttttctcaacgtcctgaatttcacgttgcagtttgttcttacgacggaacagacgaacaaattccagtacgtcctggaatgaaggcttggtagtttccatttttatacccctgataatgtgagagtcggattcgtttaagcaaccgctattcgttagggccaacattactcatagctgccgcagatgacaatgcttttatcccttttcactatcataccctttatccttgctgaatcgaagcagcagcaagatgattctgaagttcaggaattatttgcgcaaggcccggcaaatcagattcgatagcaactcaagctgatgcgccgtttccatgttcagccacacataaccatagattggtgtttccacaaccttcaggtcatggtggttattgagcaactgacgcagctcttccacagcatcgttcaatttttccgtattggcaaaaaccggctgcggattaccttcgtacagcgcatgaacaaggctcagcagtatttgctgcatcatgtgctgggtatcacgaagtttttgcgcgttcaataacacgaaatggctggggcgcgtggcccagtatgcattgatttgcaactccagcatacaaaccagattgcggttaatggtctggataccttcatatatcgattttggaatacgggtttctttgctggcgggcgcaatcagtccacgcattttcacggcatcggtcaggagtttttgtagatggctttccagacgtgggcgttcgagtaagttcggtgagaatgcagattgatagacccgattatactcggtcagacttttcgccagttgaatgcgccagtggatgaacgcccgttgtggccagataccggtaaacaacattgccagtaaagagccgaggatcacatcgccgcttcgccataacgccgtatcaatttcacctgtcggggaacccacaacaattgccagcgtcaccccaatcaataaaccttgatacggtttcttgcccagcgccagccaaccgcaaaggaacatggccgccgcgcaccagactaacatcagcggtaacgagattaactccagttgcagagcgataagacctaaaatcgaacccaacaccgtaccgccaatacgctcaaaggcgcgagggacaacgttaccccagaacgagattggccccataatcaccaccatggtgaccagcggccaggtgctttccgggatagtaaacaggcggataatgagaaaagtgagcaggaatgccagcgcgacccgagtaccatgcacaatgcggtaatggcggtatacccggatttcaaacgggcttaatgacttatcggcacgcacgcagaaactccgtaatgagattaaaagcgctcataactcatctgtcggccagaaggcgcgcctctgaattatccgacggacaaaccgggaacagtgtaatttcccggcaggagcgaaaaaattgaaaggcgcatcttactcttttcgctttcaaaaaaaagagtggtcatcgcgttaacacaccgccctgagatgaattagtgatgttttggctgcaccgcaacatacatttcgatatcccagtacccatcttccgcgccattgttcaaataaacctcgaagcagggctttggtaacatttcataagcactgtcctgcaagagactattaaagaactgataccagggtttagcaaaatcatcaccgactacacgagctaccgccaccgcatactgaccacctgtaatttctgtcagaatgacgccctcactgttttcgggaagcgtaaagtaacccggcaccgtcacgacggtgtcgcagcgtaatttttcggcgggtgtttcatctggattgtcgtaatagacagcaacccactccttcggcacaatatttttgctatctacccacatcatcaactgctcaaagcctttctttaccgtctgttcccacgggccaacgagatggaaacctgcaacggtacgtttctcttcctgcttaatctcgtagttcatgacgcctccattgatactgtttttatatacagtatagttgcaaaattaaaaccacaaggaatgagtgttgattatgcgagcagactcgcactcctgccagtctgctgcaaaagaaaggtcaggccttatggtggaaataatcactcaggcgagaaaacatgctgccttccccgacagattccagggtaaccagcggccagtgcgccacctgtttatcacggtcgtaaagttcaatttcccctacccgctgatgggcgctaattggcgcggtgagttctttaccatcaagggtatatttggctttgatatgtggaatttcggctttcggtagcaccatccagaactcttgttccgttcccaggtcgatattttctttatcgccataccagatgcgttccgttccgacctttttcccacggtgcaaaatttgcaccgtagtaaagttttgttgcccccaacgcagtaattttcttgcctcttcctcacgaccttttgcactgtcagcccccattaccactgcaatgagacgacgctgcccatctacagccgaagcaatgagattaaacccggcaccagaagtatgacccgttttcaggccgtcaacattcatggttttatcccacaacaacccgttacggttttgctgggtgataccgttccaggtgagacttttctcactgtacatatgataaaactcgggctcgccgtggatgatagcacgagaaagcacagctaaatcataagccgagctatgctggccaggtgcatccagaccatgcactgtttcaaaatgcgtatccttgagatgcagcttctcggcatagttgttcatcatttcaacaaactgccgttgcccaccggcaatatagtcagccagagcaacacaagcgtcatttccggaatccacaattaaaccacggcttaaatcacgtaccgatacgcgatcgccctctttcaaaaacatcagtgaagaaccgacaaacaccggattatctttcgcccacgcatcgcgccccacggtgacaatatcgtctggcgtaatgcgatgactatcgatagcgcgatccacgacataacccgtcatcagctttgtcaggctggcgggattgcgctgttgatgctcattacccgcggtgaggatctgaccggtggtgtaatccatcaatacccaggacccggcatgaatctctggaggctgaggtgaaaaaggaatgttttccgccgcaaaaccagacgataagttaaaaacgaacaaagaagcagcaataataagacggcgtttcaacagcaaaccctcaggagtttcaaatagctgttctttttacggaaatacttatgaactggctggaataaagtgcaagaaaatgtgactaccctctcatttttatctgacatgatctgttgccactcgctgccaaattgtggcgctaaagctgattagcacggtgatatttgatactctggcagacagcagaaataacggatttaacctaatgatgaatgacggtaagcaacaatctacctttttgtttcacgattacgaaacctttggcacgcaccccgcgttagatcgccctgcacagttcgcagccattcgcaccgatagcgaattcaatgtcatcggcgaacccgaagtcttttactgcaagcccgctgatgactatttaccccagccaggagccgtattaattaccggtattaccccgcaggaagcacgggcgaaaggagaaaacgaagccgcgtttgccgcccgtattcactcgctttttaccgtaccgaagacctgtattctgggctacaacaatgtgcgtttcgacgacgaagtcacacgcaacattttttatcgtaatttctacgatccttacgcctggagctggcagcatgataactcgcgctgggatttactggatgttatgcgtgcctgttatgccctgcgcccggaaggaataaactggcctgaaaatgatgacggtctaccgagctttcgccttgagcatttaaccaaagcgaatggtattgaacatagcaacgcccacgatgcgatggctgatgtgtacgccactattgcgatggcaaagctggtaaaaacgcgtcagccacgcctgtttgattatctctttacccatcgtaataaacacaaactgatggcgttgattgatgttccgcagatgaaacccctggtgcacgtttccggaatgtttggagcatggcgcggcaataccagctgggtggcaccgctggcgtggcatcctgaaaatcgcaatgccgtaattatggtggatttggcaggagacatttcgccattactggaactggatagcgacacattgcgcgagcgtttatataccgcaaaaaccgatcttggcgataacgccgccgttccggttaagctggtgcatatcaataaatgtccggtgctggcccaggcgaatacgctacgcccggaagatgccgaccgactgggaattaatcgtcagcattgcctcgataacctgaaaattctgcgtgaaaatccgcaagtgcgcgaaaaagtggtggcgatattcgcggaagccgaaccgtttacgccttcagataacgtggatgcacagctttataacggctttttcagtgacgcagatcgtgcagcaatgaaaattgtgctggaaaccgagccgcgtaatttaccggcactggatatcacttttgttgataaacggattgaaaagctgttgttcaattatcgggcacgcaacttcccggggacgctggattatgccgagcagcaacgctggctggagcaccgtcgccaggtcttcacgccagagtttttgcagggttatgctgatgaattgcagatgctggtacaacaatatgccgatgacaaagagaaagtggcgctgttaaaagcactttggcagtacgcggaagagattgtctaatttgaagcctccgccgctggtacggcggaggacaatgttgagtcaggctttttgaacggtgatgctccacgctgcatcgccaatctgctgataatcggtgatggcatgtccttcttctgccgcccactgtgggattgcttcagttgcctgggtgcaatcaaactcaatcactaactcatcgccgctgaccatttctgccagagctgcttttgcttctatgagtggaaacggacagacctgcgtcaccacatccagctttttaatcaccatctttacaccttacttaatttgccgcagcagttgccagtcgcgccttacgctgcggtcgaacatacacaagccaggacgcagtccagactccgagaatcataaatacaaggccaatccagccctgccaggtcatcattgcagtcataaccagtccattaccgatagagcaaccacctgcaatactggcaccgaagcccatcagtacaccacctaacccgctacgtaatgttgtttgtgcatcagctgcgcgaacgcggaactcacggctcgctttggctgcaataaatgaccccacgaagatccctaacaccaggaaaacgccccagttaatgtatttcatgtcacccgcgaccagaaattgcagaatattggccgttggggaagtgattcctaacccaaacatgcgtccggttgcttcactcaggggccaggctaaaagcgcaatcaaaccgatgagtacagctgtgacaaagggatgccagcgtttttcaaacagaatatgagcgatcccggttcggcgcggcggtaaggtcgcgactttgagttttggcttcttcaactctttcatcaccacccagagcgttatcaccagcaaaacggcaaccaacggccacacagacaaattaaaagtctcagcaatagagttatgttcagtactgtagtgctgcaaggtttgatttaaaccactggcatgtggagaacgcatcaccgcactcatcaccatataagtgaaaagcgcgatccaactgccgatcaatccctcacccgcgcgataccaggtcccggtggcacatccacccgccagaacaattcccagcccgaagatatacccacctataacagtaccaagccacgggaacgccccggcttcgtaagtcagtaggcccgcctgaattaacgcaaaaacccccacgctttgtaccgaaattgcaatcagcaaggcgtaaaacatgcgattatttttcacgatatacatatcgcgaaaaccacctgtcaggcaaaaacgcccacgctgcatgacaaatcccagcagagcaccacaaattagcccgcttaatatcattgaaaacataaattaattaaccagatgaatgttaatgaggaaattattcatgactggtggaatgcagaccaataaccaaattctctaaattagaacaaatggttattaatgaggagttcgatacaaaagaataaaaaaaccggagccaaatgttcattcgactccggtttattattagaaaagatgattatgctacgtcttcgtactgcggaaccggattacggaagctcttggtgacgcaagccaggtaaatcagaccgatagcagcccagatcagacccagaaccattgagctttcttccaggttaacccacagcgcaccaacggtcagcgcaccacacatcggcaggaacagatactggaagtgatctttcagcgtcttgttacgcttctcacggatccagaactgcgagatgaccgacaggttaacgaaagtgaacgccaccagcgcaccaaagttaatcagcgccgttgccattaccaggtcgaagttgattgccagcagggcaatcgcgccaaccaggatgatgttcatcgccggagtacgccatttcgggtgtacataaccgaagaagcttttcgggaatacgccgtcacgacccattacgtacatcagacgcgctacgcctgcatgcgccgccataccggacgccagtacggtaatggtggagaagatcagcgcgccaacctggaacgctttacccgcaacgtacagcatgatttcaggctgtgacgcatccggatctttaaagcgagagatatccgggaagtacagctgcaggaagtaagttgcaaagatgaagatcatgccgccgatcagcgcggtcaggaaaatcgcacgcgggatcacgcgctctgcatctttggtttcttccgacaggttgctgatgccgtcaaagccggtaaaggagaagcacaggattgtcgccccggtaatcatcgggataacatgcgcatcgccagaccagaatggacgagtgctcgccagcgtaccagcgccttcaccttcaaatacgccataaacaaccatgcccagaatcaccgcgatcagcactacctgcaacacgacgattacagtgttgaagttcgctacggatttcagactacgcaggttaaaggcggtcataaaggccaccagcgccaccacaaacatccacgatgggatggaaggcaccagagcttcaaaatagattttcgccagtagaatgttgatcatcggcgcgaacagatagtcgagcagagaagaccaacccaccataaagccgacagtcgggctaatggatttctgggcgtaagtgtatgcagagccagcagaaggatagcggcgaaccagcttcccgtagctcagagccgtaaacaggatcgcaatcaatgcgaacgcataggctgtcggcacatgaccatccgtgaggcctgaaacgataccaaaagtatcaaacagcgtcatcggctgcatataggcaagacccatcattacaaccggaactaacgtaagcgttttacgcaattccacgcgagaggtgtttggagtaacgttatgcgacatggtcattctcctttacggtgataaccgtcgcgtaagcaaaaaattgccccatttttttggattcctcagcgacaacaactgtcgatttttagtaaatatctatccggtacgaagcccggcctcttggtatgaatgattggtttgaagcaaaaaataaccgacgctgatgaaacgtcggtttttagtcattttttgacagcggcgcattgtgcctaaatgggggggaaatgacaagagaatgagaggcttgtcagaataatttttctttaaatggctgattttccgtcatcagattttgcataaacaccggcgatcgcactatttgctaaaatttcatcccgccaccagccactggcaagtcctgcggtctgttcgttccagccaatccagacgggttcaaagagagtttgggcgaccactttcttctcgattaacgcgccactatcgagaaaacgttgcgccagataacggggtaaatagccgcagccgaggccgctaatttgcagctccagtttggttttaaaatcgaaaacggtaatggcttcttgttcgtcgagaagttgtgatgccgtagaagcgcctgcctgcgcagtatcccccaccacaatcgcccgatatcgcttaataatacgacgatttaacggctcttcttccagggctaacggatgatgaggcgcgaccgcaaagacttgttccagatcgcccaaccgtgaaaaaccaaactcactggaagatggtggctcatgcatcgcgccaacaataatatccgctcgcccctgagtcagggcatcccatgaaccaccgagtacgccattgataaacttcaggcgcgtcacgctatgatgttgataaaaagcttcaatgagtggcgcaagcagagaaaaaggaaacgtgtcgtccacgccaatcaccagctcgttttcccagccttcatgcagtttgatcgcctgcttttccagttcccgcacggtatgcagaacttcccgccctttctctaataacatttttccggtgcgggtgaatttagcgcggtgtccgctacgatcaagcaattgaatattaaggtcgctttccagcttgtgaacggtgtaactcagagcggacggcgtcttgtagagtttggccgacgccgccgcaaaactgccttctttttctaaggcatcgaggatcatcaacacatccagcagtggtttcatacacgcccccttgcagtgcatgcggcgtcctgctggcgtgatcgtttactccagcggcattaccagcggatcgggatactggtattcaaatcccagttcattacaaatccgactgccatcaataatcttacctttgccgctgtccagactatttctgaactgcggaggttccagccccagtaaacgggccatctgcggatagaaaacattacgcgcagggtgagctggcgcacatatattatagatgtgtccgcctttaggtgcctgtaacaacagagtgatagcgccaataacatcttctaaatggactaaattaacaccatgttcaccatcaggcgcggtttttccggcaaagaagcgtccgggatgacgtcccggtccgaccaggcccgcaagacgcagaatatcgaccgaagtaccgggtaaattgtgcagccagtcttcgagttcttctaatactcgtccactgttggttactggattacgcggggtggtttctttcaccgtgccttgcgcgtcgccatagacagatgttgagctggtaaaaataatgcggggaatacgatgggccagcgcgctatccactaactcttgtaccgcttgtaaatagaactcatcgccggggccgctacgacgtgccggaagcgtaatgaccagcgcatcggcatccatcagggcatccagatcgtcagaatcgcaaactagctcaggctccatgcgaagcagatagctatcaatgccactcattcgggccgcttcgacaccatcttgtgtggttttactcccggtgacttgccagcctcgcgctgaaagtgacatcgccagcggcatgcctaaccaccctaacccgacaattgcgacctttttcatccgttatctcctgatacaccttagatctataaggctacgctagcgtatcaaaactgacaattcattctatgaatgaatctgttcaataatgataacgacatgctgcaatgagcagtgaatcgtcggtaaccgcgtataccagacggtgctcctctgtaatgcgtcgggaccagaaacctgacaaattatgtttcaggggttctggcttccccttaccttcaaatggcgttctgcgggtatctttgataagttcattgatctttttaacaattcgcttatctgtttcctgccagtacagataatcgtcccatgattcctcagaccagattagtttcactcaatgatgtccttttccgttcctttgcctgatttcaggctatcgattgagtccatcaatctccgggcgttagcgggggagcgcagtagataagccgtctcttccagcgagttgtattcttcgagtgacatcagaacacaagcctctccattctgacgagtaataaggatcggggcatgatcttcaacggctttcatcattgttgccgacaaattctgacgcgcttcgctgtagctaattgtacgcatgtcaatctcctcttttgtacagttcattgtacaatgatgagcgttaattaactatttattaattagtttgtagatcaaggtattgtcagtgagacgaaaatccaggcttcgctatttttggtgccatcagctaagaggacagtcctcttagccccctcctttccccgctcattcattaaacaaatccattgccataaaatatataaaaaagcccttgctttctaacgtgaaagtggtttaggttaaaagacatcagttgaataaacattcacagagacttttatgacacgcgttcaatttaaacaccaccatcatcaccatcatcctgactagtctttcaggcgatgtgtgctggaagacattcagatcttccagtggtgcatgaacgcatgagaaagcccccggaagatcaccttccgggggcttttttattgcgcggttgataacggttcagacaggtttaaagaggaataacaaaatgacagacaacactcgtttacgcatagctatgcagaaatccggccgtttaagtgatgactcacgcgaattgctggcgcgctgtggcattaaaattaatcttcacacccagcgcctgatcgcgatggcagaaaacatgccgattgatattctgcgcgtgcgtgacgacgacattcccggtctggtaatggatggcgtggtagaccttgggattatcggcgaaaacgtgctggaagaagagctgcttaaccgccgcgcccagggtgaagatccacgctactttaccctgcgtcgtctggatttcggcggctgtcgtctttcgctggcaacgccggttgatgaagcctgggacggtccgctctccttaaacggtaaacgtatcgccacctcttatcctcacctgctcaagcgttatctcgaccagaaaggcatctcttttaaatcctgcttactgaacggttctgttgaagtcgccccgcgtgccggactggcggatgcgatttgcgatctggtttccaccggtgccacgctggaagctaacggcctgcgcgaagtcgaagttatctatcgctcgaaagcctgcctgattcaacgcgatggcgaaatggaagaatccaaacagcaactgatcgacaaactgctgacccgtattcagggtgtgatccaggcgcgcgaatcaaaatacatcatgatgcacgcaccgaccgaacgtctggatgaagtcatcgccctgctgccaggtgccgaacgcccaactattctgccgctggcgggtgaccaacagcgcgtagcgatgcacatggtcagcagcgaaaccctgttctgggaaaccatggaaaaactgaaagcgctgggtgccagttcaattctggtcctgccgattgagaagatgatggagtgatcgccatgagctttaacacaatcattgactggaatagctgtactgcggagcaacaacgccagctgttaatgcgcccggcgatttccgcctctgaaagcattacccgcactgttaacgatattctcgataacgtgaaagcacgcggcgatgaggccctgcgggaatacagcgcgaagtttgataaaaccacggttaccgcgctgaaggtgtctgcagaggagatcgccgccgccagcgaacgcctgagcgacgagctaaaacaggcgatggcggtggcagtaaagaatattgaaaccttccacactgcgcaaaaactgccgccggtagatgtagaaacgcagccaggcgtgcgttgccagcaggtcacgcgtccggtagcttcagttgggttgtatattcctggcggctccgccccgctcttctcaacggtattaatgctggcgactccggcgagtattgcgggctgtaaaaaagtggtgctgtgctcaccgccgccgattgccgatgagatcctttatgcggcgcagctgtgcggtgtgcaggacgtgtttaacgtcggcggcgcacaggccattgccgcactggcgtttggtacggaatctgtgccaaaagtggacaaaatcttcgggccgggtaacgcctttgtcaccgaagcgaaacgtcaggtgagccagcgtctggacggtgcggcgatcgatatgcccgcaggcccgtcggaagtgctggtgattgctgacagcggcgctacgccggatttcgtggcttctgatttgctctctcaggctgaacacggcccggactcacaggtgattttactgacgcccgctgctgatatggcgcgtcgcgttgccgaggccgtcgaacgccaactggcagaactgccgcgtgccgaaaccgcccgccaggcactgaacgccagccgcctgatcgtgactaaagatttagcgcagtgcgtggagatctccaaccagtacggcccggagcacctgatcattcagacccgcaacgcccgtgaactggtcgatagcatcaccagcgccggttcggtatttcttggtgactggtcaccggaatcggcaggtgattacgcctccggcaccaaccacgttctaccgacttacggttacaccgccacctgttccagcctcgggctggcagatttccagaagcgcatgaccgtacaggaactgtcgaaagaggggttctccgcgctggcttcaaccatagaaacactggccgccgccgagcgcctgaccgcccacaaaaatgccgttactttgcgtgttaacgcccttaaggagcaagcatgagcaccgtgactattaccgatttagcgcgtgaaaacgtccgcaacctgacgccgtatcagtcggcgcgtcgtctgggcggtaacggcgatgtctggctgaacgccaacgaataccccactgccgtggagtttcagcttactcagcaaacgctcaaccgctacccggaatgccagccgaaagcggtgattgaaaattacgcgcaatatgcaggcgtaaaaccggagcaggtgctggtcagccgtggcgcggacgaaggtattgaactgctgattcgcgctttttgcgaaccgggtaaagacgccatcctctactgcccgccaacgtacggcatgtacagcgtcagcgccgaaacgattggcgtcgagtgccgcacagtgccgacgctggacaactggcaactggacttacagggcatttccgacaagctggacggcgtaaaagtggtttatgtttgcagccccaataacccgaccgggcaactgatcaatccgcaggattttcgcaccctgctggagttaacccgcggtaaggcgattgtggttgccgatgaagcctatatcgagttttgcccgcaggcatcgctggctggctggctggcggaatatccgcacctggctattttacgcacactgtcgaaagcttttgctctggcggggcttcgttgcggatttacgctggcaaacgaagaagtcatcaacctgctgatgaaagtgatcgccccctacccgctctcgacgccggttgccgacattgcggcccaggcgttaagcccacagggaatcgtcgccatgcgcgaacgggtagcgcaaattattgcagaacgcgaatacctgattgccgcactgaaagagatcccctgcgtagagcaggttttcgactctgaaaccaactacattctggcgcgctttaaagcctccagtgcggtgtttaaatctttgtgggatcagggcattatcttacgtgatcagaataaacaaccctctttaagcggctgcctgcgaattaccgtcggaacccgtgaagaaagccagcgcgtcattgacgccttacgtgcggagcaagtttgatgagtcagaagtatctttttatcgatcgcgatggaaccctgattagcgaaccgccgagtgattttcaggtggaccgttttgataaactcgcctttgaaccgggcgtgatcccggaactgctgaagctgcaaaaagcgggctacaagctggtgatgatcactaatcaggatggtcttggaacacaaagtttcccacaggcggatttcgatggcccgcacaacctgatgatgcagatcttcacctcgcaaggcgtacagtttgatgaagtgctgatttgtccgcacctgcccgccgatgagtgcgactgccgtaagccgaaagtaaaactggtggaacgttatctggctgagcaagcgatggatcgcgctaacagttatgtgattggcgatcgcgcgaccgacattcaactggcggaaaacatgggcattactggtttacgctacgaccgcgaaaccctgaactggccaatgattggcgagcaactcaccagacgtgaccgttacgctcacgtagtgcgtaataccaaagagacgcagattgacgttcaggtgtggctggatcgtgaaggtggcagcaagattaacaccggcgttggcttctttgatcatatgctggatcagatcgctacccacggcggtttccgcatggaaatcaacgtcaaaggcgacctctatatcgacgatcaccacaccgtcgaagataccggcctggcgctgggcgaagcgctaaaaatcgccctcggagacaaacgcggtatttgccgctttggttttgtgctaccgatggacgaatgccttgcccgctgcgcgctggatatctctggtcgcccgcacctggaatataaagccgagtttacctaccagcgcgtgggcgatctcagcaccgaaatgatcgagcacttcttccgttcgctctcatacaccatgggcgtgacgctacacctgaaaaccaaaggtaaaaacgatcatcaccgtgtagagagtctgttcaaagcctttggtcgcaccctgcgccaggccatccgcgtggaaggcgataccctgccctcgtcgaaaggagtgctgtaatgaacgtggtgatccttgataccggctgcgccaacctgaactcggtgaagtctgccattgcgcgtcacggttatgaacccaaagtcagccgtgacccggacgtcgtgttgctggccgataaactgtttttacccggcgttggcactgcgcaagcggcgatggatcaggtacgtgagcgcgagctgtttgatctcatcaaagcctgtacccaaccggtgctgggcatctgcttagggatgcaactgctggggcggcgcagcgaagagagcaacggcgtcgacttgctgggcatcatcgacgaagacgtgccgaaaatgaccgactttggtctgccactgccacatatgggctggaaccgcgtttacccgcaggcaggcaaccgcctgtttcaggggattgaagacggcgcgtacttttactttgttcacagctacgcaatgccggtcaatccgtggaccatcgcccagtgtaattacggcgaaccgttcaccgcggcggtacaaaaagataacttctacggcgtgcagttccacccggagcgttctggtgccgctggtgctaagttgctgaaaaacttcctggagatgtgatgattattccggcattagatttaatcgacggcactgtggtgcgtctccatcagggcgattacggcaaacagcgcgattacggtaacgacccgctgccgcgattgcaggattacgccgcgcagggtgccgaagtgctgcacctggtggatctgaccggggcaaaagatccggctaaacgtcaaatcccgctgattaaaaccctggtcgcgggcgttaacgttccggtgcaggttggcggcggcgtgcgtagcgaagaagatgtggcggcgttactggaagcgggcgttgcgcgcgtagtggtcggctccaccgcggtgaaatcacaagatatggtgaaaggctggtttgaacgcttcggtgccgatgccttagtgctggcgctggatgtccgtattgacgagcaaggcaacaagcaggtggcagtcagcggctggcaagagaactcgggcgtttcactggaacaactggtggaaacctatctgcccgtcggcctgaaacatgtgctgtgtaccgatatctcgcgcgacggcacgctggcaggctctaacgtctctttatatgaagaagtgtgcgccagatatccgcaggtggcatttcagtcctccggcggtattggcgacattgatgatgtggcggccctgcgtggcactggtgtgcgcggcgtaatagttggtcgggcattactggaaggtaaattcaccgtgaaggaggccatcgcatgctggcaaaacgcataatcccatgtctcgacgttcgtgatggtcaggtggtgaaaggcgtacagtttcgcaaccatgaaatcattggcgatatcgtgccgctggcaaaacgctacgctgaagaaggcgctgacgaactggtgttctacgatatcaccgcttccagcgatggccgtgtggtagataaaagctgggtatctcgcgtggcggaagtgatcgacattccgttttgtgtggcgggtgggattaagtctctggaagatgccgcgaaaattctttcctttggcgcggataaaatttccatcaactctcctgcgctggcagacccaacattaattactcgcctggccgatcgctttggcgtgcagtgtattgtggtcggtattgatacctggtacgacgccgaaaccggtaaatatcatgtgaatcaatataccggcgatgaaagccgcacccgcgtcactcaatgggaaacgctcgactgggtacaggaagtgcaaaaacgcggtgccggagaaatcgtcctcaatatgatgaatcaggacggcgtgcgtaacggttacgacctcgaacaactgaaaaaagtgcgtgaagtttgccacgtcccgctgattgcctccggtggcgcgggcaccatggaacacttcctcgaagccttccgcgatgccgacgttgacggcgcgctggcagcttccgtattccacaaacaaataatcaatattggtgaattaaaagcgtacctggcaacacagggcgtggagatcaggatatgttaacagaacaacaacgtcgcgaactggactgggaaaaaaccgacggacttatgccggtgattgtgcaacacgcggtatccggcgaagtgctaatgctgggctatatgaacccggaagccttagacaaaaccctcgaaagcggcaaagtcaccttcttctcgcgcactaaacagcgactgtggaccaaaggcgaaacgtcgggcaatttcctcaacgtagtgagtattgccccggactgcgacaacgacacgttactggtgctggcgaatcccatcggcccgacctgccacaaaggcaccagcagttgcttcggcgacaccgctcaccagtggctgttcctgtatcaactggaacaactgctcgccgagcgcaaatctgccgatccggaaacctcctacaccgccaaactgtatgccagcggcaccaaacgcattgcgcagaaagtgggtgaagaaggcgtggaaaccgcgctggcagcaacggtacatgaccgctttgagctgaccaacgaggcgtctgatttgatgtatcacctgctggtgttgttgcaggatcaggggctggatttaacgacggtaattgagaacctgcgtaaacggcatcagtgagttgcggggtaagcggatgcgatattgttgccgcatccggcaaaaaaacgggcaaggtgtcaccaccctgccctttttctttaaaaccgaaaagattacttcgcgttgtaattgcgtagagcattacgccccagcacaatccccgcgccaaccatgccacccagcagcaccgccagaatcaaggtaattgcctttttcgggctatcacgacgaataggtaacatcggtttcatcacataacggtaagcatgaatatcaagatcatcaacttttaagctttcgatatccagcaggttttgacgagtctgatagtagtttggcgagaacaccaacggacgggtcgcctcatgcttaatcatcgactccagcgcttcgctccccaaaaggaacaacgtatcttgtgtgatatcttcgccagtctgttgaatctgcggttttgtcacctgcgcctgattcgcatactgcaacgcttcctgaatctgacggatacgcagatctttctgctcctgcgcgactacttcctgcgttcttaaagagtcctgcaagtttttccgtcccagagcaatgttgtctttgagatccttttctagctcttgattcactttatcgtcaacttgctgaatgtattgggccaacttcatttgtgcgccctctgcagtttgcccaacataagaaacagtcaatggtaattgctggttcttaacagaaggttcgatggtaagtttttctcgttcttcctgattatccagcgtttctgctaatgcagagaaggcagaactgaagcgaccaattaacgtctcctgcaaatccgatactttcggtgcagcctgaccatagataacattcatggcattgttatagccagcaatttgccccacgtcgggctgagtgataattgctgttgacgtccatttctccttcgctactgccaaatatccaatagccagggcaatagccacaatgacggaaatgatgattgtcatcttgccacgccacaactgcactagtaaatcaatcaaatcaatctgttccgggtcatggttttgcccagaaacattattattttctactctcatcattaccctaactgacggaaatttccaagtccgcatagtttagcgataatcctcgtgaatgctataggataagtgataaaaataatgaattgttgtgtaagtaacaaaagacaatcagggcgtaaatagccctgataacaagatgttagtcgctgccaaagagatcgcgggtgtataccttatctgccacatccttaagctcttctgccattcggttagagataatgacgtcggcttgttgtttgaaggtggcgagatcacgttccaggcgagagttgaagaatgagtcttctttcatcactggctcgtagatgatcacttcaacacctttcgccttgatacgtttcataatcccctgaatagaagacgcacggaagttatctgaaccgctcttcataatcagacgataaatacccaccacttgcggcttgcgtgacaaaatggcatcggcaataaaatctttacgcgtgcggttagcatcgacaattgccgagatcaggttattcggcacagactggtagttcgccagtaactgcttggtatctttcggcagacaataaccaccataaccaaacgacggattgttgtaatggttgccaatacgtgggtcgagacaaacgccttcgattatttgacgggaattcagacctaaactttctgcatagctatccagttcgttaaagtacgccacgcgcatcgccaggtaggtgtttgcaaaaagtttaatcgcttctgcttcagtggagtcggtaaacagcatcgggatattttgcttaatcgcgccttcctgtaacagagcagcgaaacgttctgcgcgttctgaacgctcaccgatgacaatacgtgaaggatggagattatcgtaaagggctttaccctcacggagaaattccggggagaatataatattttcagtgcgatatttcttatgcatcgctgcggtaaaaccaacgggaaccgttgatttgatgaccataaccgcataaggatttatctcaactacgtctttaattactgattctacactggatgtattgaaataattagttttaggatcatagtcggttggagtggcgatgatgacataatcagcatcccggtaggcttcatttttatctaatgtggcattaaagtgtattttatctgattgcaaaaactgctgaatttccttatcaacaataggagatatccgatcattcagcatagcaacgcgtgacggtaaaatatctaatgccacaacctcatgattttgtgcgattagaagcccgtttgacaagcctacatagccagtaccggaaatggtgattttcatttcatgctctcagaattaacttaactgtgaatcatgatgtttttagcatcctgataagagctaaaagttttaacgctacgttgttcgatggtcaacgcaacgaaaaacaattcagattttctttataagaatagctgatatttattaagttaatattaagcagtgaaatttagtctataagatatttggcaaaaaaaagcccggtgcaatatacgccgggcctcaattttattgttggttaaatcagattaatccagccattcggtatggaacacaccttctttatcaatacgcttataagtatgcgcaccaaaatagtcacgctgtgcctggatcaggttcgcaggcagaacagcagcacggtagctgtcgtaataggcaaccgctgcggagaaggtcggaaccggaataccgttctgtactgcataagcaacgacatcacgcagcgcctgctggtagtcatcggcaatttgcttgaagtacggagccagcaacaggttagcgatctgtggattttcggcataagcatcggtgattttctgcaggaactgcgcacggatgatgcagccagcacggaaaatcttcgcgatttcgccgtagttcagatcccagttgtactcttcagacgcagcacgcagctgagagaagccctgggcgtaagaaacgattttgcccagatacagcgcacgacgaactttttcgatgaactcagccttgtcgcctgctggctgtgcttgcggaccagagagaactttagatgcggcaacacgctgatctttcagagaagagatataacgtgcaaacacagactcggtaatcagcgacagcggttcgccgagatccagcgcgctctggctggtccatttaccggtacctttgttagccgcttcatccaggatcacatcaaccaggtagttaccgtcttcatcttttttggtgaagatatctttggtgatgtcgatcaggtaactgctcagttcaccgttattccactcggtaaaggtctgcgccagttcttcgttggtgaggttcaggccacctttaagcagagaataggcttcagcaatcagctgcatatcgccgtattcaataccgttgtgaaccatcttcacatagtgacctgcgccatcggcaccaatataggtaacgcatggttcaccgtcttcagctacggcggcgattttggtcaggatcggtgctaccaattcataggcttctttctggccaccaggcataatagaaggacctttcagcgccccctcttcaccgccagaaacaccggtaccgatgaagttaaagccctctgctgaaagctcacgattacgacgaatagtgtcctggaagaaggtgttaccaccatcaatgatgatgtctcctttatcgagatatggtttgagggaatcaatagcagcatccgtgcctgcacctgctttcaccattaacaggatgcgacgaggcgtttccagagattcgacaaactctttcaccgtatagtaaggaaccagtttcttgcctggattttcggcaatcacttcttccgtcttctcacgggaacggttgaaaatagagacggtataaccacggctttcgatgttgagcgcaaggttgcgtcccatcactgccataccgactacgccgatctgttgcttggacattacatactcctgtcaggtgtgatcaccgcgctgaatgctcgcggcctggaatgttcgcaaataagtatacaaagtacttattaaagtataaatagcttatccatgcttatatgcttacggctttatattacgggtgaaaaactgatgaaattcgatcaaagttgcgatttgataaaatacgttttctggctaaatatctaaaagtactttttaagtgccatctgaaggcttttgaaaaaaaacttcgattgtcatgatgagcataatgtatcgcatgaaaagcgggaacataatgaagtctgacaccagccaggctaagcctcaagcacaggtcaatatcttcacagtacataaagtaaccttgatcgaagccatttacacgcacaaaatctgaaaaacgtaccagcataaatgatcctgcgcaccaatcaacaaccgtatcagaatagatactttctttaggaatttttgttttattaaggaaggtgcgaataagcggggaaattcttctcggctgactcagtcatttcatttcttcatgtttgagccgattttttctcccgtaaatgccttgaatcagcctatttagaccgtttcttcgccatttaaggcgttatccccagtttttagtgagatctctcccactgacgtatcatttggtccgcccgaaacaggttggccagcgtgaataacatcgccagttggttatcgtttttcagcaaccccttgtatctggctttcacgaagccgaactgtcgcttgatgatgcgaaatgggtgctccaccctggcccggatgctggctttcatgtattcgatgttgatggccgttttgttcttgcgtggatgctgtttcaaggttcttaccttgccggggcgctcggcgatcagccagtccacatccacctcggccagctcctcgcgctgtggcgccccttggtagccggcatcggctgagacaaattgctcctctccatgcagcagattacccagctgattgaggtcatgctcgttggccgcggtggtgaccaggctgtgggtcaggccactcttggcatcgacaccaatgtgggccttcatgccaaagtgccactgattgcctttcttggtctgatgcatctccggatcgcgttgctgctctttgttcttggtcgagctgggtgcctcaatgatggtggcatcgaccaaggtgccttgagtcatcatgacgcctgcttcggccagccagcgattgatggtcttgaacaattggcgggccagttgatgctgctccagcaggtggcggaaattcatgatggtggtgcggtccggcaaggcgctatccagggataaccgggcaaacagacgcatggaggcgatttcgtacagagcatcttccatcgcgccatcgctcaggttgtaccaatgctgcatgcagtgaatgcgtagcatggtttccagcggataaggtcgccggccattaccagccttggggtaaaacggctcgatgacttccaccatgttttgccatggcagaatctgctccatgcgggacaagaaaatctcttttctggtctgacggcgcttactgctgaattcactgtcggcgaaggtaagttgatgactcatgatgaaccctgttctatggctccagatgacaaacatgatctcatatcagggacttgttcgcaccttccttaatccctaacataaatgacacaataaaatcagaaagcacaggaaattttcttacggaataatcatgtaaagatttcgcttcatctcggaacaggcataatgtactaaaagcataacgcttactttcgacatatttaatatatgtcagcaaatcatcatgcttcatgatgatatcgggattcaaaaacaaaatgtaatcatcatctgcgggtctatatttttcctttacatacgccaccgcaatattattattatgaccaaagccgtatacacctccactaatatagtccaggcctgcataatgctggcatatttgtttcaataatagagagtctttgttgtcgcgtacgataatcttgtagtgctcatcgtcagcattaagattttcgagtaattttttgatgtagtcttcatgtccgtgggaaacgattattatatataccatttcaatgttcttcagtaataaaattaactagttcatcaaacccaactaatacattttcattacgataaatgaaatttgcatcagagatatcttttttgaggttaccttttttgaagtcaataataagtttaactaacatgtcatcgttattagaatcaaaaaaagctttcttttcataactaccaagagtttctctagtaaatgggaaatctgatgctaatacccacttacctcgctctttagcttcagacaacggcaatccccatgtttctaacctagagggaaaacaaactatatctgaaatattataacaatgatcgattttttctttatccaagtacccgaggaaatgaacattatccagtccttctgcaagactgataatatattttgcatacgcattttctgtaccactgatagtaagcagaaatttaatattggattgttctttcaatttccttgctgcactaataataagctcgtaatttttaaatactcgtggaacagcagggtaaaatattgtcaactcagaagggttattcttaaattgagaatcatcatcagtaagttggcttttatcagataatttaatttctggccgactgacaatgatgttatttatagaatatttcttgataaatttttctttcatccagaattgttgaacaaacactgcagtattttttttaatgtttattttatatatcagcccgtatagcattttaaataagaaaaagctaggctccataagaatttcacggaataaaattcctttataaaaaggtgcagggttatgacaatacacatatctttttttagtgacgacattggccgtaatatcatgcagacaaatccaatgcgtagcattcagctcttttgaaagttttttacaaactacatattcaaagtgcaaacgttttagccacgaccctttaacctcaggaaactcaatgaatttaacccatggataactttcttttaactctttagcagaatggactaatgcgataaaactgacattttctttattattagttgctgccaaaaattttttcaaaatggtaaatggaccgccagtggtaaaattgaccgcagaaacaacgactatgctttttcccataatttggtctcatgattgtatttctttatgatttttgctggtactcccgcaatgacagtattttcgggaatagaacctctaacaacagaattggcgccgactacgactccattaccaataattgttccaggcaaaaccgtcacattctcacccaaccaaaccctctggccaattacaacagctgaagattccaacgtgcgcatgtctggaggtatatttggcgaactcattggatcagagtgcttaaaggaaccgtgattatgatcggtaataaatactttacttgcaataagcgtatcccgacctatcgtaacgctctcaattgaggcgatatgaacatagtcgttaacttgcacattatcggaaaaaaaaatcacgccacgtccaaatgcatccagcctgagaccgactccacttgtgaaattttcaccaaaattaatgctaccatcattgcgaatatagcagggaaatcgaataattctacagttccggtaaaatacacgagtcaataagacatctctaacaagccgaataaaaccacagagaccatatcgtttagcgagttttaagatcatcgatcacctcttcaagaacatccctgaagtaacttcctgttcgaattttctgagaaataatttttgtattctcactaatttgcttataagtttctattgtcatggagtcaacaatctcttgcatttctttgattgatcccactgcatatcctattctattatctacaatgaaatccgcaagggcggctttatcccatataaatactggaagttccattgaaagataaagagatgtcttatgagggttattaaactttaaatagtcgccaaaggcaccactacaggtttcgacagaatctccatcccaaatgagtccaaattgcatgcctgggaggttaatcttttccggagattgagcatcaaaacttccaagatatttaggattatctttattttcatagttgacaccaaagagagtaaaatcgcatccttcagtatatatgaaagaacatttatgcctagaaaggttgccagcatatatgacccctcgttgcttatccgtaacatctcgatgctccacatcagatgagacgaggtaatcaaatatttttatgtctttgattttatcctgagacatatatttactaaggtactttgtcatttgtggattgtgacttatgaccatatcacaggtagcaagccgcacagaatcactaccccctcctcctcttaattcatcaatatcatgaatcagaggtactattctaaattttagaaggcggtgaaagaatgacaatatatgccaaaatggtttggccatcgggaaattgaaaattaaaacatctttattttcaagaccgcagagaaatgtactaagcttaacagaactaataattctctggactactccaccccatagaggaatgttaacaacagaaatgttttcataatctgaagcaatgtccagtgcatcttttcttgctttaaatccagcatcgcgtctagagaaatttaaatcattcaaaaaatacattttcactttattttctgggccttaagaaattgagagaatactatgatacaaagagttatttgtatccaactgctaatattagtcatgaagctttcatgataaaaaatgaaagaaaaggtataaataaaatatgaataaaatattttcacagatatgtaatttcgagacaatctccataaaacacctgaaatacagccatgaataaccatcatcaaatagcttagctccgcggaaatataaacataatccgaaaaagcagtataaacatttgttggcaaacccacccacacaaattctttatgcaacgacatagagactccacctgttaatagccccatcagcctttcaaaaaaccaaaagacatgagaactggcagagttagatacttgctgaaaataaaactcctgaaacgcgattatagggctgaccaaatacatggatagataatatgccatccccccaggcagtccacgtaaaaagagcatatacaaggagaatagaacacctacagctgtaataagataaacataatgttttactctattaacacctacgatgaatgcataagagatgataaccataaagacaatttgcttaccagtattcagtataattgcaaagatgaatacaataaaaacaagtaaagtaaatgttttacttacctttgtattagtaaattttttagaccaaataaataaagcaaaagtagttagaatgattggctgcatgtatgctgagaaatttcttgatgtgtcttcaacatcagcatctcttatcaaattcatatagctaagtaagctagtcccgaactggtagttacttaacctcatgcatatatatatcatcgaaaaagaaataactaacaagcctacattatgcactttcttcgatggtatgctataaatagcattattgacttttctgatatttagatctaatacactttccgtcaataaacatgacagggtaaatgtcaaaacattgcaaagtagaaaaatcaacgtagcgtcatttaactgaaaagcatatatatctgacgttatttcatatcccaataagaccagtgcgaagatgatattaacgcatacggctggataaaatatatccttcttaagatataaacagataaatgctgtaatgagaaagacactaattacaagatagatcattaatccgtactcattatatttttcacttgataaagagcggcagatatcacttgatgcatatcataatatttatactcggccaaacgcccgccaaatataaccttgtcttctctgctagctaactctctatatttcttaaaaagctccatgtttttattatcattaactggatagtagggttcgtcgccaactttccactctaatggatattcttttgtaacaaccgtatgctttgtctcaacatagtcaaaatgtttatgctcaattattctggtatatggtacattagcatcagtgaaatttattactgcattcccttggaagtttggaaattcatggcgttccgtctcaaattttaaagagcgatattctaacgctccaaacctatagtcgaagtactgatcaatgggtccagtgtagatgattctatgggctttactcgctagagaatctttgtctttcaaaaaatcaatgcctaattttacgtccacaccttcaagcattttttcaataagcttagtgtagcctcccaccggaataccttgatagcgatcggaaaaataattgttatcaaacgtaaatctcactgggattcgcttaataataaatgcaggcaattcttttgcacttcttccccactgcttctccgtataaccctttatcaatgcttggtataagtcctccccaactaatgaaatcgcctgctcctccaaattttcaggtaccttgtcaccatacttttttttctgagcattaatgatattttgagcttcttgaggatctttaactccccacatttggtggaaagtattcatattaaaaggaaggttgaataatttgtctttataaatcgccagtggagaattagtaaaacgattaaattctactaaatcattaacgtaatcccatatatatttatcattggtatgaaaaatatgtgcaccatatttatgaatctggataccctcacagtcctctgtgtacgcatttccaccgatatgatttcttttctcaatcactaaaacttttttgtttagcttttttaactcattcgcacaaacggcaccaaacaaaccagaaccaacaatgatataatcgtacataaaatcctcagcaaaccagtaatttattatttcttacgaacatcagcatgagtgacgtaactaagcactctgttgcaagcaatgttattgctgcaccaatctctttaaaaagagttgttagcggaaaaatcaacaacaaactcaacaaacccgcagcgattaaaatcttactgaattctttcttataattatgggtcagcataacttgaatgccatagacattacttaatgaaataagaaaaggcagaggcgatataatcattagcacaatcactgcattatcatatcccggccctatacttatttttactagtatagatgcacccaagagcagaattaatgaaaaagcaccaccaatcaaactcaagcaggtcaatgattttttaattaaaatcacacccttcacacgattaagaacaagcgtacttgatattcttgggtatattgcttgggtgataggatttaatagcccttgaagcgcgtttcttatagtattggccgcattaaaattccctacggacgttggtccagatataaatcccaggataataactattcccgtagaatataaactaatagcagatgtggaaataaaaacatgaaaaccgtctgctaaagatcgacgcacattatgtaatgatagcgtaactttaccaatccaaccttcatgaacaacgatagctagtgcaataattccagcaaccagatttgcacttgactgaataaaaccggcaattgctatatctgactttgtgttcacaaaaataaatgttagagggataatagccaagcgggataaaatactacttaaagtcagccatttcattttttcttttccctgaaacagccagatagggtagattaaattcccgactaatgcaggaacaaacgaccatataattacggcatgcttgttatattcaggaacaagcaaggtcatcgacgttaagaaaatcaatgtaatgacgataagaactatttttgaaaatatcaccgcccaaaaaatagacgttactttatctttactatctgctgctttggcaatactctgagttgctgtgagattgaaaccatattcaacaaacattatcatatatagcatagtcgcttggcaaaaaccgaatataccgaaattttcaggaccaagtgttcttacaagatatggaaatgtaagcaatggtaaaagataattgctaccttgaacgacagccagatatataacgtttcttcttaaagataatttattcgtattcatgcaattaattttaatctgataagctcatctaacgtaaagagcctttcatcttttggcgaaaggattaaccctgatgtttggggccaatcaattgcaatgcgttcatcattccaacatattccacaatcgctttcaggatgataatagtttgtagttttatattgaaattcagcgatatcagacagaaccaaaaagccatgagcaaacccttttggtatccacaactgctgcttattatcagctgaaagcagaacaccaacccatttaccaaaggataccgaattgggtcgaatatcaacagcaacatcaaaaactgctccatgagtgcagcgtacaagtttatcttgtgcgtactcgccgcgttgaaagtgaaggcctctgagtacattttttgatgaacgtgagtgattgtcttgaacaaagctgaccggatagcctagaatatgttcaaatgctgattgattaaagctctcataaaagaaacctctatcatcaccaaatactcttggctccagaattagcacatcttcaatttcagttctaatcacattcattaatttgaatccttcgtcattttataaagatactgcccataattattctttattagtggtacagctaattttcttacttgctcaacatcaataaaacctttacgaaatgcaatctcttcaggacaggaaaccttcaatccctggcgctcttcaattgtcgcaataaaattacttgcttctatcagactctgatgagtccccgtgtccagccacgcgtagccacgccccatcatcgcgacagacagacgtccctgctcaagataaatacggttaatatctgtaatttctaactcaccacgtgcagacggcttcaagtttttcgccatctgaaccacgtcgttatcataaaagtacagacctgtaacggcgtaattactctttggttctaacggtttttcttccagactgattgccgtaccgtttttatcaaactcaacgacaccatagcgttctggatcattaacgtgataggcaaataccgttgcaccactttctttgttaacagcggcctccattagcttcggcagatcgtgaccgtaaaagatattatcaccaagaaccaaagcacaatcatcaccaccaataaactcttcaccgatgataaatgcctgcgcgaggccatctgggctaggttgcactttgtactgaagattcaggccccactggctaccgtcacccagcaattgttgaaaacgaggagtatcctgaggtgtactgataatcaaaatatcgcgaatacccgccaacatcagtgtagagagcgggtaatagatcatcggtttatcataaataggtaatagctgtttactgacagccatagtcacaggataaagacgtgtaccagaaccacccgctaaaataatacctttacgcattttcatttcatcattccttttaattcatcttgctccaccatcacgaacaagatgcaaaaactattaaattgctgtagtcgtaaataattcattgagcattcgtttcacgccaacctgccagtcaggcaagacaagcgcaaagttctgctgaaatttttctgtattaaggcgagagttatgtggacgacgagctggtgtaggataggctgttgttggtactgcgttgagcttgttgagtgcaaggggaatgcctgctttgcgcgcctcttcaaaaaccagcgcagcataatcgtaccaggttgtggtaccactggctaccaaatggtacaagcctgcgacatccggtttattcagtgcgacacgaatggcatgtgctgtacaatcagccagcagttcagcacctgttggcgcaccaaactgatcgttaataaccgctaattcttcacgctcttttgccagacgtaacatcgttttggcgaagttatttccttttcctgcatagacccagctggtccggaaaataagatgcttcgcgcaatattcctgtaacgctttttctccggctaacttggtttcaccgtaaacatttagtggtgcggttgcatccgtctccagccatggcatatcgccatttccagggaagacgtaatcagtcgagtaatggataacccaggctccaacttcatttgctgctttcgcaatcgcttcgacacttgttgcgttaattaattgtgcaaactccggttctgattctgctttgtctactgcggtgtgagcggctgcattgacaataatatccggccgaatgcttcttacggtttcagctacaccttcaggattactaaaatcaccgcaataatcagtagagtgaacatcaaaagcaatcaaattacccaaaggtgccagagcacgctgtagttcccaacctacctgccctgttttgccaaaaaggaggatattcattactggcggccctcatagttctgttcaatccacgattgataggcaccacttttcacattatcaacccattttgtattggacaggtaccattccaccgttttacgaatcccgctctcaaacgtttcctgtggtttccatcccaatgcgcgaccaatcttctcagcatcaatagcatagcggcgatcgtgtcccggacgatcagcaacataagtgatttgctcacgataagatttctctttcggtacaatctcatccagcaaatcacaaatagtgagcactacatcgatgtttttcttttcgttgtgcccaccaatgttataagtttcacccgctttaccttcggttacgacggtatataacgcacgcgcatgatcttcaacatacaaccagtcgcggatctgatctcctttgccataaataggtaatgccttaccttccagtgcattaagaataaccagtggaataagcttttccgggaaatgataaggaccatagttgttcgagcaattagtcacaattgtcggtaaaccatatgtacgtttccacgcgcggactaaatgatcgctggatgctttggatgcggaataagggctgcttggcgcgtaagctgtcgtctcagtaaataagggtaattcttctgtattatttacttcatctggatgaggcaaatcaccatagacttcgtcagtagaaatatgatgaaaacggaagctatttttcttgtcgctatcaagagcagaccagtaattgcgagcggcttccaaaaggacataagtaccaacaatattggtttcaataaatgccgcagggcctgtaattgaacggtcaacatggctttcagcagccaggtgcatcactgcatccggctgatgctgagcaaaaatccgtgccattgcaggtgcatcgcaaatatccgcatgttcaaaaacatagcgttcagaatcagaaacatcagcaagtgattcccggtttccggcgtacgttaatttatcgacattaacaacactatcctgcgtattatttataatgtgacgaactacagctgaaccaataaatcctgcgccaccagtaacaagtattttcacttaatttattccatattacttcagagcatgctgtgaaataagcggctctcagtttgattaatagaggtattaatgcacgctaccgcccctggctttacagctaccagagcactgcatgcatgcctatgatgtgacgagcgttacccactcgcgctaaacccgaaaaattcaaacgctaattgtcttaccaatccgctctggaaacaaggaaaatcctggaaaactttgaataaaaccctactgctaactcgttgttattctgatggtttatataaaacaacggcaggaagattcgcaacaaattacttttgctgcgaattttcactgccgttataattttcttatcaaccgttacatccggtcagattttcattattcgcttaacagcttctcaatacctttacggaacttcgccccttctttcaggttgcgtaggccatacttcacaaacgcctgcatatagcccatttttttgccgcagtcgtaactgtcgccggtcatcagcattgcatcaacggattgttttttcgccagctcggcaatagcatcagtcagctgaatacgtccccatgcaccaggctgagtacgttccagttccggccaaatatcggcagaaagcacatagcgacctacggccatgatgtctgagtccagcgtctgcggctgatccggtttttcgataaattcaacaatgcggctgactttaccctcacggtccagcggctctttagtctggatgacggagtattcagagaggtcacccggcatacgttttgccagcacctggctgcggcccgtttcgttgaaacgtgcaatcatggcagcaaggttgtaacgtagcgggtcggcgctggcatcgtcgatcacaacgtctggcagtaccacgacaaatgggttgtcaccaatggcaggtcgcgcacacaaaatggagtggcctaaacctaaaggttcgccctgacgcacgttcataatggtcacgcccggcggacagatggactgtacttccgccagcagttgacgcttcacgcgctgctcaaggagtgattctaactcataagaggtgtcgaagtggttttcgaccgcgttcttggacgcgtgagttaccaggaggatttctttgatccctgcagccacaatctcgtcaacaatgtactgaatcattggcttgtcgacgattggtagcatctctttgggtatcgccttagtggcaggcaacatatgcatcccgagacccgctacaggaataactgcttttaaattcgtcattatttcatccacctgtaaaatggttgctgaattatagcttgttcgatttttttcgccagcatcaattaccctgaattgattactgaattacttgtgatgttacgccgcttcgttgtggattgcagtagcattgttcctaagtatgactccatttttccaggaatggtcgcaaatctactccctcagttccggcaatctaaagttaatcttctccacattaacaatatggtgattaatcctgtcgatatcgacggagctttgtcctttttcattcaccgcatgaacatttgcaagagacagcagtgtttcttttttcgccataaaaacaccacgaacgtctttgcgcatgtcaaagttcatgctcaatgcgggtccaactgaggattcctgcatcacattgatatttcgcataaaaaaatgttgcggtttgttgtgtaactccagcgacgcacgcttcatctcaatgttagttagcgccacaaaggaaacagcattcccggcggagatttgaatgccgcgcaatttataagcaagatgagtattatccagttgaatatcattcacccggaaattttgcggtatcgagagatatttgcctttaattaccccatagccgattaacatcccggcgctattaatcatttcaatattatcaatcacgaaattgtcacaaccgtaaatagcgactgtcgcgttatcaatgcccgctttcttactgaaatccggcgtgatattgcgggctttgatattacgaataacaaaatgtttaccattttcaacatgtatcaactgccgacaatccgatcccgtgatattcgccacgacaaagtttttcactgcctggtcttccgggtagttgttatcataagtgcttcccgcaaggcctatgccgatgccccagttgattttgccgttggtacagttgatgcgctcgatgacatggtcagatatcaaaatatcacggtcgttaattgccacgttccattcaatggcgtcgccttgtaagtcgctgaacttacaattggtgatgttggcaccgataatctggttatgaaatccctggcgtaagatggcgtaattagcgtggctaacggtcaggttatcgatgatcaggttgcgcatgacccgtttgtttttgccgccgatataaatctgcgtcaccgggccaaagccgctcatagtcagccctttgatggtgcagtcagaaccacgcacatccagggtgatgttatgcatactgccgccatcctcccctgtcacctggctgccgtcctgtaagacaaatcgccctctgccgttgccgcgcaagcttccaagaatgtgtaacgttttaccgggagggataaagatgccggtgttgatattgtcacaaaccaatccggcaggcacgacgactgtttgcccttcgctgaaggcttgtttaaatgaggcgatccagtcgtgtgggttgtagtcgttaatgttaacgctttgtcgggcgggaagcgcgcgggcgaaaggggtatggaggaaggcaagcgccgagcttgccgtcaggaacgtgcgtcgggagagttttttaaatggcatgcgttctcctctataaagcctgcagcaagctggcgagttctcgattgatcacctgctggttaaaatcgtgttcaactttttcgcgcgcgcgtttgacgaccggagccaattcgtcggtgtccagttggctaaacgccgccagtcgttgcgccagtgcgcgagcatcgttctcaggcaccagccagccggatttgtcagcctccaccagttccggtattccactatgcagagtagaaaccaccggaataccgaccgccatcgcttccattagcgccaccggaataccttccatatcaccatccgcacctgtaaccgatggcaacaggaagacatccgcgtcgtcgagcatcgctttcacttcatggctcggtttaaagcccggcatctccaccacatcttccagttgatattgttcgatgagggtgcgcaggcgtctttcccacgggccaatgccgaggatgcgatagcgaaatgccacgccctgctctttcaactgacggcaggcttcgatcgccacatgcaggccttttttctcggttaagcgtgcgacggaaataatctccagcggcgttgcgggcgctttcacgggacgcgggctaaagcgcgtcatatctacgcccatgcgcgatacggcgattttttccctcgggcagcccattttttgcagccttccggcccacagatcgcttatcggtaacatcaggtcgccacggcgaaacagttgctgatattcgggagtgtagtggttgagcacttcccgactggagatatcaataccgtggaagatagtggcaattttgccgcgaatgacacccagttcgcggagttttgctgcggttacccccgcgggaccaaaatgagcgatgaacacatcggcgcgaaacggtgttgcgacctggccgcaaatggcagacaaaatcaggttccgcgactcggcaccatagcgtttgaggttgagcgcctgccaggtatttttacgatgaatgccgcgcaaggtctggctggctcggtggcgcagtttcgccactttgcccgtaggttcgtcctgtaaccagcgggttctggcagcaaggttgtatttcgtccatgccgcgtgggtgttttgtgtgtcgcctttttgcagcgcgagaatctctacctcaaatcccatatcaataaacgcggtaatttggttaaggacgaaggtttctgacgacagcgggaatttcagtaaaaagaagccgaccttcatttcacctccccgatgcgctcaagcacagactgcaccatctgcattcctgtctgacgctcacgactgacggcttcactaagtcgcgcattcagcgccggaagctggcctaaggtatccgcaaccatcgcttgcaggctgccgtctaataaatgacggatatcaattgccatctccggtagtcccagctgctgcataatcccggcggatttatgttcgtagttgatggcaattgccggagtggcaaaattcatcgagataatggcagagtgcaggcgcgtaccgacggtgagttcacaggcccccagaattttgcccatttccagatcgttgagttcatccatcactacgtggtaacgggcaggatcgctgatgtgctggcgcaggttgagcgccaccatgcggtcgtctttgttatagctgtcaatgcccgtacaggtggagagcgcaatcacctgatacccttcatcgagaatgcgattgaccaccccggcaaaggctttttcatacgcttgttgagtggtgccgagacgtttgtcaaacggtgccagttcgcgcagggtaatggccaccgttttctgttgtgcggcaacgtccagccagtgttgaacggcatagctggcggtgaagtcttctgtgtggtgatcgaccagccacgcggtatcgacgccatgttccacttttgcggtggtgatattgctgcgtttcatcagatcaaagctgaccgattcgcgcaggatcagcgcgtcgcagtgaccaaaaacgtagttcgccagttggttaaattgctcatcctggaacgggccaacactgtgaccaatcataaacagcggctttttcgccataaacgtgcaaagtgcatgttcaaactgcggcacgccatagagatcgacaaaaaacgatccgccgacctggataatggcgtcgtaacctgacagcaggcgcacgaagtcggtgaatccctgggcgatggcgatattgcgcagcttgccagtgtcggtgacgcgtgagagcaatacctgatgctggtagcggcgacggaggacttttttaacgcgcccgacaacgcccgccgcgctgttgtgttgtttcatttgcaggaacagcggatcgcccattaccgggcggttgagcagccaggaagaactgaccggatagcggctcatcacatccacttcggcgtgtggattgagaatgttgatggcatcaagtaagccgcgcaggatggcgctgtcgccacgattgccgcaagtgtggttgcccagaataagtaatttcattttttcctcataaatttgatgccaggtgaggctgcgtttgttttgttcgttgccgctttttgcctgatgcgacgctgacgcgtcttatcaggcctacaagacccgagcacagaaccgtaggacggataaggcgttcacgccgcatccggcattcagtgcctgatgcgacgctgacgcgtcttatcaggcctacaggtcccgagcacagaaccgtaggacggataaggcgttttacgccgcatccggcaaccgttgtcggaaccgaaaacagcaactcaccccgcccgtaaaagcattttcattttttcgctgcgacaaaactgacgcttcacttccaccaccagcggatggcgcgacagcacaatcatcaccacaaacgccagcacccccgtggctatttgcaccgccagcagcatccccagcgccagttgccctttcagcacaatgcccagcgcataactgaccaccagcgtcggcagcgagagataaaacggcagccataaactcaggatgtactggcgataactggaaccaagaaccggtttaatcatcacgaagtaactcagaatggtgttgataatttgcaccagcaggaagccaagcgtgacgccgatcgcgcccgccatctgcccacctataacaatcgccggaataaacagaaatgttttgaatacgttgaatttaaagctgatatcgacccgcgctttcgccatcagcagcgaaccaatcgggttacctacggagcgcagcagacccaccacacacagcaattgcagcaccggaataatgctgttccacttctcaccaaagaccagcggtacaaagttattcgacaccaccattagcccgagcagcgccggaaagttgataatccccactaccgacagcagcttgtagaagttaacacgcagcttttcggtatcgtcctgaattttggcgaatgccggaaacaacacgcgggtgatgattgggttcagcttcatcggtggcacaacggccacgttgtacgccaggttgtatccccctgccacgcccgcgccgagaatacgcgccagcacgagcgttgaaaggttggtattgagatagttgatgatgctgtccgccgtcagccaggcaccaaagcgtaagttcggtgccaccgacgccagcgagaaatgcagaccggggcgataaattttgcggccaaagtagccaaacagcagcgttctcaccgcactattgaccagataaccgaggatcgcggtcatcgccagcggccagaaatgggcgctaaccaccgtacaagtgaagcccgccagcaccgcgctggtttcgatcatgccgattttgttgaactccagctctttttgcatcaacgcgcggaactgttgcccgtgggggattaccacaaacgccagcgataatgttttaatcaacggtgccaggtccgggttattcagcacgtcgccgatgagatcactcaacaaaaacaccgccacgcacaccacgatccccagcccgacgttcagccagtacaacgtggtgagttcaaggtgactgatttcttttcgctgaataatcgagttagcgataccgaagtcagaaagcgtatctgccagcgcgataatcaccagcgacacggtaagcaggccgaactggtggttgtcgataatccgcgccagcacggtcatctgcaccagcccgaggccgatgatgatcaccgtggcaatcgccgaccacttcgcgccgctgatggttttttcacgtaagctcatatcaatatgccgctttgttaacgaaacctttgaacaccgtcaggaaaacgattttgatatcgaaccagacgctccattcgcggatgtactcaaggtcgaactcgacgcgtttttccattttctccagcgtgtcggtttcgccgcgccagccgttaatctgcgcccagccggtaatgcccggtttcaccttatggcgcagcatgtagccttcaatgagctgtcgatactgttcgttatgcgctactgcgtgcggacgtggaccgacaatcgacatccccccggtcagcacattgataaactgcggcaattcatccagcgaggtacggcgcagaaagttccccactttggtgacgcgcggatcgttctgcgtcgcctgggtcaccactttgtcgttctccatcactttcatggaacggaacttccacactttgatcggcttgccatccatgccgtagcgagtctggcggaaaataaccggccctggtgaactgagtttcaccgccagcgcaatacagcacagcaccggggagatcagcagcagaataagcgtcgccagcacaatgtcttccgcacgtttgagcaggcggttaaccccggaaagcggcgtgtcgtaaagcggcaccaccggtacgccgttcatctcttcgaggcgtgaatggagaatgttgaaggtaaagacgtcggggatcagcagcaccgaacaggtggtgtccgccagttgatggaccagttttttcactcgcgcgccgtcgcacatttgcatcgcgatatagacgttatgaatcttgcccgctttcgcgtcctcgaccagctgttgcaggttacccgcccagtcgttagaaacgccgcccggtttcgggtcgtggtaaacgcccaccacttcaaaccctaaccacggctggttacggaagctctccatcagcatttgcccggcggctaaatcccccgccaccgcgaccatgcgcttgttatagccatgattacgcagccagcccgccccaatgcgaatacacgaacggcaaaccaccagtccgatgctggtcagcgcataccacgccagccagattttcagttgcgtgtcgaaatcattgttgaacgccaccagtccggcgctgaaaatcacgcttaaggtccagttttgtagcaacagggcaaattctgtcgctgcccgaacaccgcgccatgagcgataaaaatcggtgatgccgcccagcatctggaacaccaccagcgtaatcagcgccaccaacaggtgcatgtagaggaatgacagtccgctgacttcgcaaaccagccatagtccggcaaacatgatggtgatatctgaaaagcgttgcaccatagagattaacgatgcattggttttcgctcgctcgcgcttttttagatttgtcatcgttgttcctgttattagccccttacccgcagtggggtaagggaagatccgacattactcgttcagcaacgtcagcagagttcgcgttcgcgcttccatcagcggcacatcaccgcgcgattccacattcaggcgcaccaccggttcggtattggaggtgcgcaggttaaagcgccagtcggcaaaggtcatgctgatgccatcggtgcgatccaccgccagcgcctcacggctaaaatgctgttccacgcggttaatcgcctcaacgggttgcgccagtttgctgttgatctcaccgcttgccggaaacgccgccatccggtcgcgtaccagttcgcccagcgttttatctttcaggcacaccagttcggcgaccagcagccacgggatcatgccgctgtcgcagtaagcgaaatcacggaagtaatggtgggcgctcatttcgccaccatagatggcgtcttccttgcgcatacgttctttaataaaggcgtgtccggttttcgacattaccggcgtgccacctgcggcagtcaccacatcaacggtgttccaggagagacgtggatcgtggatgatcttcgcgccgggatttttttcgaggaatgcttctgccaacaggccgacaatgtagtagccctcaataaactgccctttttcgtcaaacaggaaacagcggtcaaaatcgccatcaaaagcaatgcccatatccgcgccgtgtttgatgaccgcattgcgggtgtcgtcgcggcattccggcagtagtgggttaggaataccgttggggaaattgccgtccggcgtgttgtgcactttgattaattccacgggcgcgccgagggctttaaagcgggcttcaatggcgtccaccaccggacccgctgcgccgttcccggagttgatcaccagcttgagcggcgtgaggtttttgacattgatataaccgaacaggtgatcaacgtaagcgtcacgcaggttgatttgctgatagcgaccgcgtttggtttcatcgacgggaggaaagtcgttggcttcagccagacgctggacgtcgcgcagtccggtatctccgctgatcgggcgagccccctcgcgaaccagcttcatgccgttataatccatcggattatggctggcggtaacttcaatgccgccatccacgccgagatggaacgtggcgaaatagatctcttcggtgccggacataccaatatccagcacgtcaacgcccgcatcctgtaaacctttcgccagcgccagttttaaggtttcgctggtgaggcggacatcaccgcctaacacaatggttttcggtttgagaaattcgccataggcgcgaccaatgcgccaggcgatatcttcattcagttcttcgcctaatttcccgcgaatatcataggctttaaagcaggttaattttttcatatcgttaccctttttcaggcaatagttggccctgaccgaagcggccaattttatttttgtcgttatttacaccgcggtttcgcattcattgcctgatgcgacgtttacacccgtccgtagcgatccgcgaaacgcaccacatcatcctcttcgagataagagccggagcgcacttcaattaaatcgagcggaattttccccgggttttccaggcaatgcgtcgcccccagcggaatataaatggactcgttttcaccaagcagtttgatatcaccatcaatggtgacttttgccgttcccgcgacaaccacccagtgttccgcgcggtgatggtgcatctgtaccgacaagccctcgcccggtttcacggtgatgcgtttcacctggtagcggtcgcccgcgtcgatagagtcatatttgccccacggacgatacacttcgcgatgcacccgatgctcatggcgaccatcggctttgatctgctcgaccacttttttcacatcctgtaccgcgttacggtcggcaatcagcaccgcatctttggtctgcaccactaccagatctttcaccccgacggtggtgaccaggccagattcagcatacacatagctgttttcagttttgtgattaatcacatcgccgtggcaaacgttgccctcggcggtgtgggcgctgatctcccataatgaagaccaggagccaacatcgctccagcccgcatccatcggcaccacaacagcatctgccgtacgttccatgaccgcgtaatccaccgactcttccgggcaggcgagaaacgcttcttcatccacgcgaataaaattgagatccggatcgacggcgctcatcgctttttcacaggcatcgaggatatccgggcgatattttttcagttcttcgagatagcgtccggcgcggaacaggaacataccgctgttccagtaatattcgccgcttgccacataggcctgagcggtttccagattcggtttttcgacaaactgcgccacttcaaaggccaccatatcctgctcacccgcagacacttcaccgcgacgaatatagccataaccggtttctggtagatccggcacaatgccgaaggtcaccagcttgcccgcttcggcatatggcatggcattacgcacggcggcacggaacgcgtcttcatcggcaatcacatgatccgccgccaataccagcattaacgggtcgctctccgggctatgacgttttgccgccagcgccgccagcgcaatggcaggtgccgtgtttcgccctgccggttcgagaataatgttctcggtaagtttgttcagttgacgcagctgttccgcgacaataaagcggtgctgctcattgcaaatcaccaccgggctttcgcactccacgccgttcaggcggcagatggtggtttgcagcatggtgagatcgcctttcaggcataaaaactgcttgggataaagtacgcgggaaagcggccataagcggctaccggagccacctgccatcacaactggatagagtttcgactgcgccataattatccccgaatatcatttataaattgacgtaacacgttctctttatcgagcgtgcgttcggcatattcacgtgccaccgtgttgtgtttgggcagcaggagcgcctgacggatccccgccaccagcgcctcgaccgattccggttcaacgcaaaccgcaatgcccggaaaggtttcgcaaagctgccccagttctgtgtaggcttcagcagtaatcaccgcgttaccgcctactgccagaatattggtcagtttcgacggcaatacggcatctgccgcgccgcgtttttgcaccaccagatggcaatcgcccatcttcagcagtgcgggtaaagcgtcatacgattgcagcgggaaaaattgcatgttgcgcagtccacgctgctgcgccattttttccagccgcgctttgccgccgccctgcccgacaatggcaaaaatcagcggttcatcgcgcagacgatcggcagcttcaataacgttttccagcccctgcttttcaccaatattgccggagtaaagaatgatttttttgttatccggcaggtcaagctggttacgaagggcatcaacatcggcatctgcaacatgctgaaaacgggcaatttccgaccagttggggaagaagatgacgttttccgccgccacgcctttttcgatggctttattcatcatcgaacgcgaaatcgtggagacgttatcgacgttatgcagtccgctacgttcgaacgccgttgccagctgtgccactttgccgcctttgccttttccggcaaggcccagccccagcatggcgtccacttcgtaatcctgaatatgcagcacggtacgcgcaccagagagtttcgccagcaggcgcattcccggcgcgcaaaacagcgttggcaccacgccaataatgcgatccggcttccagcgacgttgcgccatcagcggaaagaaactgctgacggcaaaactgcccagatgcaacaggcgtttcagggtgctcggctgttttggcacatacagcgggcagcgccacaccgtggcggccccctcttctcgtttgtagcgccaggcggaatagttctcgcccacctgccattgcgggtagtaaggcggtgcggtaatgacccgcacctcatgaccttgtgccgccagccattccaccatctcgccggtgtatttgccgatgccggttaactccggcgagtagttaatgccgtagaccagtattttcataatccgggtactccggtacgcttctcagcgagaaaataggcgcggctgttagcatgaacattatcactggcgagcagcgcgtccgacgtcagccagcggtaatcgtcatgctgctcatccggcagtaacagctcttcttccgatactctgaagcgaaaaccgagcaccacatagtgagtggtgaaatccgtgccagagaagttatcgtcataaaagtgctgccagacaccgtaaaactggcctgctgttatcggcaaacgcagccccagttccgccatcgtcagccgctcaaatgcggcttccagcgtttcgtctttctgcacgcgccctcccggcacaaaccagtaaccctgcgccgggcggttggttcttttgccaagcagaaactcgccgcgactgttctcgacaataaagtcgagagagacaagcggagtggagcgcactaccgtggcaaagtcttcctgacgtaaaaacatcattacccccgaaagcggtcttgattctcaaggaaccactggtaagtgctggcaagccccgcttccagtgagatttcgtgataccagccaagctgatgcaggcgcgtcacatccagcagtttgcgcggcgtgccatccggtttgctggcatcaaaaaccacccggcctttgtaacccaccactttggcgatggtttgcgccagctcgcggatagtgcagtcaacgcccgtgccgacgttaatgtgcgacaacatcggctgggtgttctccagccagacttcatgcgccagctccatgacatgaatgctcgccgccgccatatcatcgacgtgcagaaattcgcgcatcggtgtaccgctgccccataccaccacgtccggcgcattctgtgccgtcgcctcgtggaagcgacgcagcaatgctgggatcacatgcgaattactcgggtggaagttgtcgtgtggcccgtacaggttggtcggcatgactgagcggtaatcgcgtccgtactggcggttgtatgattcgcacagtttgatcccggcgattttggcaatagcataaggctcgttagtcggctccagcgtgccctgcaacaactcgctttctgccatcggctgttttgccagtttcgggtagatgcaggacgatccgagaaacagcagtttgttcacgtcgttctgatgcgcggcgtgaatgatgttgctctcaatcatcatgttctggtagatgaaatccgccggataggtgttgttggcaacaatgccgcccactttcgccgccgccagatagacctggtcaatacgttcgctggcaaagaaatcatgcacggcgcggctgtccagcaggttcagctcgtcgcgggtgcgtaataccagttccacatcaccgcgctgttcgagctgccgcctgatggcggaaccgaccatcccgcgatgaccagcaataaaaactcgttgtttactcatgcttatgactccagcgcgatcgccacgtcgtagccgtgagatttcagcagagagtgttttttcgccgcttcgaggtcattagccaccatttcagacaccatctctctgagggtgatttccggtttccagcccagtttttcgtgcgctttggtcgggtcgccgagcagcgtttcaacttcagccggacggaagtaacgcgggtcaacagcgataatcacatcacccggtttaacgcccggcgcgtcatgcccggtgacggaaaccacaatgcccttctcttcaacgcccgtgccttcaaagcgcagtttgatgcccagctgtgctgccgccatttccacgaactgacgcacggagtactgaacgccggtcgcgataacgaaatcttccggctgttcctgctgcagcatcatccactgcatttttacgtagtctttggcgtggccccagtcacgcagggaatccatattgccgaggtacaggcacgactccagcccctgggcgatgttggcgattgcgcgggtgattttgcgggtaacgaaggtttcgccgcggcgcggggattcatggttgaagagaattccgttacaggcgtacatgccgtaggattcacggtagttaacggtgatccagtaggcgtacagtttggcgaccgcatacggagatcgcgggtagaacggcgtggtctctttctgcggaatttcctgcaccagaccatacagttcagaggtggaagcctgatagaaacgagttttcttttccagaccgaggaagcggatcgcctccagcaggcgcagcgtacccatcgcgtcgacgtcagcggtatattctggtgactcaaaagagaccgcaacgtggctcattgcgcccaggttgtacacttcatccggctgtacttcacgcaaaatgcgcgtcaggttagaggtatcactcaggtcgccataatgcagatggaatttcgggttgcaggtgtgcggatcctgataaatgtgatccacgcgctcggtgttgaatgacgatgcgcgacgcttaataccatgcacctcgtaacctttttccagcagaaactctgccaggtaagaaccgtcttgtccggttacaccggtgatgagagcgacttttgacatgtattattcctctgtatttttgaatttattcagtttcaacgcgttcgcgtatcaccactgcgggattcccccggcaaaccacatttgccggaagcgatttaaaaacactgcttcgtgcacccacgacggtgccgtcgccgattgtgacgcctggggcaacaaagacatcggttgccagccagcatttctcgccaatcacaataggcgtggcgttaatggtgaaatgttgacttgcatggtcgtggctaccggtgcataaataacttttttgcgatatcaccgaatgtgcgccaatggttatttcaccgagggtatataaattgacgtcatcgccgacccacgcgtaatcacctaaggttaatttccacggataggtaatttttactgacggacgaataactacgttttttcctatttttgctccgaataaacgtaataaaaaagcccgccagcgatacaatacttgtggcgaccaggcaaatattgttgcctgtactgcccaccataattgcactttaatagcgttgccgccccggaaccctttcggcaccgagaaaccgcttaaatcttgcattggttttccttatattcagactttgttatataaggctttcgtctttgaggtagtacgttggcgtaaatgccaggataattcagcccaaaagccaggcacatgtaatatttgtcgttggacttttttcgcgtcagcacacaattccatattattggtggtagataccccacccatggaaaattcagacaccaggccattgagttttttaaatgcataaccggctttatacattttggctgccagcgcgtagtcggaagaaactttatattccaggtcataacgccattttttcaagccggatacagggaaaaatatcgcctgatgactggcgggcaggctgtgataaatataccagcccggtttggcgctacgtttaattttatgcccgtcgccaaaatccagcagcgcatcgccggtgatcatcacgttatctttttgcatttttaacttacggacaaaatttgcggcattctgatgaaaaatatcgcccgaattgagaaacaacgcgaacttgccttgtgccatcgcaatgcctttgttcatggcgtcgtagataccgttatctggctcgctgacaaagcgtaggttaaagataccattgagattttccagatactcacgggtgccgtcgttggaaccgccatcgacaacaatccattcgaagctgatatcttccacctgcgccagatgcgccagcgaggcatgtgttttgactatcccttcgaggttacgaaacgcgacagtgattatgctaagcaacatgttcttattcttacctcgtaatatttaacgcttttcgcaaaataaacggacagacgattaaaaatgcatattccgggctaaatatcgaaccggtaaaaaacagcgataccggagtaaaaagatataattgcacgcgaaaattgcggttatcaccaaaagcgttgatcatcatttttatcactttccccatgtaccacagtgataaaaacaccgcgaaccaggaaaaataaataatcagcagatacaaaccattgtctatggtttttccgacatccgcaccgttaaatattccgaatgatgcgacatattcataaagtgagccaaatctgactacaccgtcaatatgggtcaaagaataaccgaccatcaccagcggaccgacaatacgataatatgatgacgatccttccgtacctaaatcgcccagacgggtggaaatataaggaaacgcgattaccacaccaaccaggaatacagccagagaaatcaatgctaacggtaactttttcttaatcgcctctttattcagatattgaaatgcccactccagcaaataaaacaggataaaggtcataacccctgaaaacgatccggataatattatccctgcgagaatcatagcatctgttttaggcgttttgataccaaactgtttgatgctgagccaaattgagattaatgccagagcgaaaaatgccggttcgaaataaagtgctgtcgtgcgcttgccgccgaatttaatgaaattcagcacatagctgttgctgtaaatcagatatttcgaaatcgactccataatactgctgccaccggtgaggataatttgtgccatctccaccgccgccagcgccaccaccagcccgaccaccagataaaagaaacgtaatatcttgcgatggttgtgtggcgaaattgttttaaaacgaatactccacaccatgccaataatgatcacaatatagacaaacagcatagttgaagtgacgtatttactggcatccagcgactgaccaaacagatagttaaacgccgtgagtcccgcgccaatccctaaggcaatcatcaattttttaacgctgatgcgttctaaaaacagcagtaacaagacaggtaaaaaagtgacgatggtgatggggaaactttcgccaagctgggcgattttgacgttaaccagcagataaatcagcggcagcaacaggtagctacagattctgatagaagttgacatactcctccagcatctgttgtccactgtaggcggcgcggctgcgttggctgaactcagccagcgtggtaccaaatatcgcctgcgcgatttccggtttgcttaactgcaccagttgcagcacctcttcttcgctgacggttttaccgccggatttttgcaacacttcccgcgccgcatcgctatgggtggcaatcaccggcacgccaatcgatagcgcctcacacaaaatcagcgggtagttatcgacgcgagaactgaataccagcgcatccatctgattgagcgcgctcatcagcttacgtttgtcggtttcaaagccgtgattaaccacgttgccagcggtgaacggcgagaacttaccaaaggtatgcagttcaattttgtcgcccagcgccatcatctcgcgtaccagttgctggttagttttgccgtcgtaacgcagatcatgcgccaccaccgcgattttcggcttgccctgggtttcgcgcaccggaggcaagtccgccagaatcgcttcagttgccatatcaatgccattattgataatccggcaacgccctggaccgtacaggctattgaaagcgtcagccacatgctggctgggggaaataaactgacagcccagcgccagcatctcacggaataactggcgtttgcccgccaccagttggtgtgcgcgatcaatcttcaccggcggatagttatttaaggtcgggcatttctggcagcctgttttccagccttcgcaaccgtcggtaaaggcgcagcgtccggtaacactccagtggtcgtgcagcgtccagaccagagtgacgtccggtttatggtttttcactttttcgcaaaagcgcaccacgctcttaagatttagccagtagctgtgcagcacatgaaaatgcaggaccaccggacccgctgtgcgagtaatggtgcgatataactcattgaaattgccaaacagatcgcgattaaacagacgaaacagagcaatattcgccatcgcggtcatccgcggcgtatgtttgatgacctgcggatagttctgatggctgacgctctctttgccgcctttgccgtaaccgtagacaaaatgtgacgccagcccctgttgcagcgcacgctggtggagatctaacgccacacctgctgccccgccttccgccagtcgcacattaaattgcaaaatattcatttaattaccttcactcgcgctttttctcccaccaccagcgcgttgtccgggacagagtcgagcaccacgctgcccgcgcccacggtgacgttgttaccaagcgtgatatcaccaagaataatgacgttggcaccgagttcgacgccgttgccaatgtgtggacatgccatgttatcggcaccacgattgccgatagtgacgccgtggcgaatggtaaaatcatcccccgctaccacgtttttattgatcacgacggcgtaaccgtgatggatagtaaagcggcggccaatggtcgcggcagcctggatttcataaccgaaaaagcattcggtgataatgcgatacagcaccagcagcggggccgcccacagattgttgaggacgttctttttgcgccacaccgaacaaaaatgagcaacacgataggcaagaaccatgcagcacgggcgtaaactccagctgttggcgcgcagatcttccagcatctttagcgcccccgaataccatcagccagacgtttgccgttacgcaccgacagcagcgtcagcaaagtgcgccaggtcatacgtttattgcggatctggtagagggtaaacagctgatattttttgctggcgcggtcgaatttgtctttgtgcttgcggtaaaagtggaagtacccggagaattttttcggtgacgaggtgatctgcatttcaccgtgattgatatgcaggatctgcgtcgcctcttctactttccacggttcgccgtactccaccaccatccgcaggaagatgtcgtaatcctgtgccgctttcagttcggtatcgaacaaacactctttgaaacgccatgcccaggtaaagacctggttgccaatgatattgcgtttgtagaacaggcggcgtgaatacggcgatttgggatacagcggcaagcttgccggttgggaatagacttcgccctggcaaacgtagtcgttagcgtacaaaaaggcgtgtgtgaccagttgctgtttatgggcgaggaagacgctcagacggttgggtgtccattcgtcatcgtcatcaatcccggtgatatattccccttgcgccagcataatcgcctggttacgtaccgcgcacgccccgctgttaatgtcgttgtgaatgtaagtgatacgcggatcgttgagggcggtgacgtactgttgcagttgttcccaggaggtggagcaatcatccacgatgatcatctcccagttgctgtagtcctggcgcaaaaccgattttattgcccgaatcgccagttgttggcggttccaggtcggcatatagattgagatcagcggattgtttttcataggttgttctcccggcttatgagctggtttgcttgccggatgcggcgtgaacgccttatccggcctacggggcggtgcgaatgcaggcgtcgttatttcgcatccgacttatattcgtattcgtaatagccataatcctgatacgcgctggcgcggcggaagatggagttcagaatcacccctttcaccggaataccgttttgctcaaagcggctcagactggtttccacttctttcaatgtgttgaccgcataacgcgccaccattaacgtggttccgacatgacgaccaacaattgccgcatcggtcactgccagaatcggcggcgtatcaatcaacaccaggtcatagtttttactcgcccagttcaccagttcggcaaagcgttcgctcatcaacagttcagaaggatttggcggcacctgaccgcgcgggatcaggtcaaatttggcaatagaggtcggtttagcagcggtagtaatatcgccctgaccaatcagaatttccgacaggccattaacgttattagtgcccaacagctcgtgggtgtagcctttgcgcatatcgcagtcgatcaacaacacgcgtttattggtctggctgatcaccgccgccaggttggcgcagacaaaggttttaccaattgacgggctaaccccggtcatcatcaacacattgttctgtgcctgcatcatcgcgaagtgcaaactggtacgcagactacggatggcttcaatcgccagatcggttggattccccaccgccagtagctggctctgtttatagcgtttaatccctttgatggttttgacgctatcacgcgctttctgccattccgacagcgggatgctggcatagacgctaataccgtgttcttccagtacttgcgggctttcaatgccgcgattaaacaacgagcgcagcagcacacccacgatagaaagcatcaggccaaggataatcgcgccgaggataatcagccctttcttcggtttcagcacgccaggctgagtgattgccgggtcaacaatgcgcacatcgccgacggtgctggcctcggtgattttcagctcctgctctttattcagcagttgcatatagacctgctgaccagactcgacatcgcgggtcagacggacaatctcctgctgggttttcggcatcgccgttacgcgaccgttaagtttggctttttcgtcttccagcgcctgacgtttctccagcagcgtgcggtacgccgggtgaactttggtgtacagcttggagatttccgcctctttaaaggtcagttcgttcaactgcgcatcgatgttcaccatcgaatcgagcaccgcttttgcttccagcggcagatcaacagaatctttatcctgacggaaggcattcagtttgttttcggcaacatccaagcggctacgtacttccggtaactgttgcgcgaggaaggcgaggcttttcgacgcttccgccgatttgcgctcaatattttgttcctgatagttacgggcgatgctgttaagaatgtcgcggatctgttcacgatcttcaccggtataagtcaggctcaaaacgccagcgtctttgccgttctccgttaccgtcaggctgttttgcagttggttgatcatccccagcgtggagtatttggtgacggtaaactcactgcccgggctggcgtgaatggcttcaaccatcagcgtgacgccttcttttttcagcatctggcccgcttgcccccgggcgctaaagccgccgtcgctgctcagggtgtagtttttgttgtccagcacattaagcgtaaacacctgatccgccatctctttcgggcggttaaaggtggtcactttcaccgtctcgttctgacgtcccatcaggcgatcccagcccgcaccgaaaatcgggaacgtgtttttgctcactgcaatatcgaggtcgagatcgtccaccgttttaccaagcaccagacgcgaacgaatcaactggatctcggcgtccgatgcaggcggtttgttggctaatgccgaaccaatgtcctgcactaacgaattgccgctgttttgctcgatttgtaccagtgcgtcggcactataaatcggcgtggcgaagaaggtgtaaaccacggcacagagggcgaatacggtggtgatgccaatcacccaccagcgcgcttcaatgacggtgccgaccaggcgaccaatatcgatttcatcactgcccgttaccggagcggcatgttgttttactttttctgtcattcttatacctgctctgcgttcaatgcctgcgcccactggcgggcagaccgttcaagtaatgtgtacaccgctgcaaacgtttcccggcttttgcgatacggatcggggatttcacattcgttatcccagtgaccaaacagcatcactttgccgcgcatctccggtgccatctcgcataagcgttcgatatggcgcttttccatggtcaaaatcaggtcgtagttgcgacacagacggcggctgatttgacgggcacagtgaccttccagagacagttgatgttctgcggcgacgctgatagcggtaggatcagcgcccttaccgaccagcgcgccgagtccagcggactccactttcagctccgggtgataacgttgcagtaagcgttccgccgtcggggaacggcaaatattgccgacacagacaactaagatgttgttaaacatgacgattaccagttatgaatgtcgctggctgtatccgtcatgtaacggacaccgctaatagttggcagcaactgattgatcagacggttccagcgggaaaccggggcggtggtgacatacaccacgtcataaggttgcaggcggaattctgtcgccatcaccagcgacgtggcatcggacatatccagctggtagatattggcaatcttgccgttacgcccgccctcgcctttcagcggacgaatgacaaagatgccgctggcgttggaggtggtcatgtcgatgccttcagcattgcccagggcttcagtcagggtcatgccgctaaagtccattttcagggtgctctgtttcttcacttcacccatcacaaatactttcagatcatcattacgtggcacgtagagaatatcgccggggtaaagcaggcgattctggttgaggtcgccgttttgcatcagcgcctgcaaagaaatgcgctcttcacgaccattgtgtgttagcaccacgttgcgccagtcagcggtgtcggtcaggccacctgcggcgttgatggcgtcgagaatagtcagtggcacgttggtgatcgcctgttgaccggatttattcacctgaccggagatataggccttttgtgagcggaaggcggcgatattaacgtccacctgcgggtcagcgatgtacgtcgctaagcgcccggtaatatcactgcggatttcagcgagcgttttcccgactacgtggaccttgccgatatacgggtaaaacatagtgccgtcaggctgtacccagttgccggtgtcgctggagctgcggtactgaccggctggcgtggtgagttccgggtgatcccagacggtgacattaagaacgtcccccggcccgacgcgatactggtaattcgcgatctcactttccagcgtcatattggggcgcgctacattcgggcgtgggcgtaattggtcaatcaggcgcggggtcagcggataaacattcaccattttgtcgagatcgaaatcagcgtcctgctgtttgatgacgtctttgcccatcgtcgacatattgctgcccggaagtactgtgcaaccgcttatcaaggttactgacaccaataatggcatcaatttcattttggatttcatcattgtttatttatcactttggcagagtaattatcctgtgcactattaatagcaatgtcgccatgcacatttaccttgcagttaattgaataaaaatttaactggcatcagtcctaaaaaaattgatttcatccgcaggctattgacagaataattcagactggtctttcaggcatccagacacgctaccgcccctggctttttagctaccaatacactgatttagtttaatttttcacaccctctcagcatgcagtcgttgatgagaaagggttattacggaaattaacttccgaatataaggtgacattatggtaattgaatattggctttccaataatgcaggaggaagtgttacagctaacggaatagcaggcaagataacaattcggtaattggctatttttaagaattatattaagtgtcattcaatatggtttttaggagtttctttaggttgacaatatttaatatagtgtctccacatgcgatatttcttaaataatgttttattattaccacttttaattcagggataatgtgaggttattaccctcaaataatatgagataaatagtgctgcaacattgcatttttgccccgatttatccatgatcgaattgtgacatttgtcatacaacgaataggttttgtacttactatggaatggattgccgatccgtctatctgggccgggttaatcacgctgattgtgatcgaactggtcctcggcattgataacctggtctttattgccatcctcgccgaaaaactaccgccgaagcagcgtgaccgcgcacgggttaccgggctgctgctggcaatgttaatgcgcctgttactgctggcgtcaatctcctggctggtcaccctgactcaaccgctgttcagcttccgctcgtttacctttagcgcccgcgacttaatcatgctgtttggtggtttcttcctgttgttcaaagccacgatggagctgaacgaacggctggaagggaaagacagcaataatcccacacaacgcaaaggtgcgaagttctggggcgtggtgacgcaaattgtggtactggacgccattttctcactcgactcagtgattaccgccgtcgggatggtcgaccatttactggtcatgatggccgccgtggttatcgctatcagcctgatgttgatggccagcaagccgttaacgcaatttgttaacagtcacccgacgatcgttattctctgcttaagcttcctgttgatgattggctttagcctggtggcagaaggtttcggcttcgtcattccgaaaggctacctgtacgctgccattggtttctcggtgatgatcgaggcgctcaatcagttggctatctttaaccggcgacgttttctttccgctaaccagacgctgcgccagcggactaccgaagcggtaatgcgcctgcttagcgggcaaaaagaagatgcggaactggacgccgaaaccgcgtccatgctggtggatcatggtaaccagcagatctttaatccgcaggaacggcggatgattgagcgggtacttaatcttaaccagcgtaccgtcagcagcattatgacgtcgcgccacgatattgagcatatcgatctcaacgcgccggaagaagaaatccgccagttgctggagcgaaatcagcatacgcggctggtggttaccgacggtgatgacgcagaagatttgctcggtgttgttcacgttatcgacctgctacaacagtctctgcgcggcgaaccgctcaacctgcgggtgttgattcgccagccgctggtgttcccggaaaccttgccgttgttacctgccctggagcagttccgtaatgcccgcacgcactttgcttttgtggtggatgagtttggctcggtggaagggattgtgacattaagtgacgtcactgaaaccattgccggtaacttaccgaacgaagtggaagagatcgacgcccgccatgatattcagaagaatgcggacggttcctggacggcgaatggtcatatgccgctggaggatctggtgcaatatgtgccgctgccgctggatgaaaaacgtgaatatcacaccattgccgggctgttgatggagtatttgcagcgtattccaaaacctggcgaagaagttcaggtgggggattatttgcttaaaacgttgcaggtagaaagccatcgcgtgcagaaggtgcagattataccgctgcgtaaggatggcgagatggagtacgaggtgtgatggtatcggtcattttacccaatagccgaaaggaataagatgagggaaccgcgccatcggcgatttaccgccgggagcccgggttgccagggtggtggagattgagccaccctggcacgttcaccggcttgagcgttccatagtagcgaggaacatcaagtgaacggaacagccttcgatcttacatattcagaatataatgatgccgccacgaacgcctgatgcgacgctttacgcgtcttatcaggcctacaggactggtcacctggtaacctacatcttctccagcaacttcttcacatctttgccattacgggaatctttattccgctcggcccagtcattcaggcgacgtttcgcttcgtcctgtagatgtttgcgcagtaactgatccacttgcaggctgtaattgagttgctgccagttgccataaacccgcagcggtactggcgtttctttcaggaaatcaatcagtttgctttccccgttccagccacccacgacccgaatatcaaactgggtgtcgcaggtttgatctgccagattcaacatgccttcccctgtcagcgccagcacaggcgattgaccttgcatgtcgtttaacgtcacgacgccatccttcaacgtcaaatcggtggtaaagcggtcaagccgcgtcacgttatcaaagttttcagcggccttcacatcaccgccattacgctctaccgcttgctgaatcatctgctggaagttcatcccttccatgcgcgtgtcggtcatttcgacatgtgcctgtccttgccagttgtggcggaatgcgtcggcatctatgtcagcaccggagaaatcaccagccagtgacatttttccggtcaacgaaatcggatagttaaacgccttcagaatggtaccaatctcaacgttttccagccgtggctggaagtttatccgcggatttattgatgtcgcgtccagcgtgcccggcagtgaaacctgtccaccgttaagtttgccctgcagttgagtaatttccagcaaacccgacttgttggtcatttgcgtggcaacatctgtaaaattcattccgcgccagcgcacgttactggcctgcaacaaaatatcagccgtaaagccttgcagtccctgataggccggttcatcaatacgcgaagaaatgaccgggcgcggcaacgttgattggctctgcccctgctgcgcggcaccgttttcaccattcgcggtttcattaagcgggatgaggttgtcaagattcagttgcgggaattgcagcctcagctgccattccggtttctctgtcagcgtaacctgtgcttgcccgcttagcgtactatcattggcggtcaaactaatttggttaaatgaaaggcgtttatgtgactcctgccactgggcctggaaactcccctgcccctgaataccttgttttggtaaatcggcaccctgcaactgccagttaatttgttcaatagccgccgttaaatcatgcggataatcagaagcatctaccgtaccgttaagggatatcgtgagatcgcgctgatcgcgattaacccgcccggagaactcaaatgaaccacgatgttggggatcttgttccatttgcaggcgaatattgcggattgtcacctgctcgtcatcttcatgctggaacaccagcacgctgtccgccaccttaagactggatatatcaaacgaccatccgcgatcgtctgacagatccggcaaggtattgtcgcgcggtgcaaccggagcgtcttcactgcgcaccgcttccgtctgcggcgtcagttggatcactgccccttttagcatcacctgcttaacgctcagttgatgactcagtagtggtaaaagcgccacgtccagacgcatgttgtcggcgcgaaccagtggctggcttgcgccctgggcggtgagagacattcgcccggagaggatactaagctgcggccagacgtgccaacgcagtggcccgtcgagctgcaattgataaccgctacgtgcagcaacttgcttgaccatatagtcgcggaaatcattcggattcaccagcaacactaacgcagataacccggccaccagcacgaccaggagtatcatcagcgtcgtcagaaatcgtctcatggtatcctcaatgggcctgaattagtctttatcgattcggctggctaccgcgccctgctggttgcgatatttcgcatcttcacggcggttgtaaggtcgcaccgccgggccggaaagcggctcaaagctcagcgcaccaattaacatgcccggacgcagcgccagcggcagcttaccggagttgtagaactccagcacaatgcaaccagaccagcccggatcgatgcggtgcgcggtgacgtgcaccatcagccccagacgcgccagtgaggaacgcccgtccagccagcccaccagatcggctggcagcgtcaccgactccagcgtcaccgccagcgccagctctcctgggtgaagatagaacgcctcgccctcgtcgagaacgatctcatcgctcatcacgcggtcaagcgcggcgctcacttcatctttgggaccgctcagatcgataaacgctgccgtgtgaccacggaaggtacgaaatttattgcccaggcgtacatccaccgtcgcgccgttaatacgctccactggcggacgtgggttgatcgacaaacggccttcatcaagccaggcttcaatatctcggtcacacagacgcatggcattttctcctttcgcgcatcactcccttaacgccaattacgtcaagggcatactaggttatcactgaacggtacacaatttatcaagcttattcaaagaactgacttattttcgctttcaatatatcgatcgcgatgcggtttttcccgccgcgcggcacgataatgtccgcatattgtttagaaggctcaatgaattgcaggaacatcgggcgcacggttttttgatattgcgccatcactgaatccattgaacgcccacgctcgttaacgtcacgcttgatgcggcgcatcaggcagatatccagcggggtatcaacgaaaatggagaagttaagttcgtcacgcaaacgcgcatccgtcagcaacaaaatgccttcgagaatgatgaccttcttcggctcaaccgtcaccgtttctttcatacgcgtatgttcaacatagctgtaaaccggcaggtcaattgccgagccgcgtttcaacgcttgtaaatgctcaagcagcagactgtgatccatcgcgctgggatggtcgtagttggtcttaacgcgttcttccatcgacagatggctttgatctttgtaatagcagtcttcgggaattacgccgatgtgttcatcaccgacttgctcacgcaattcacgataaagggtactggcaataagactcttgccggaagccgatgcgccagcgataccgataatgacgcactgatgagactgatcagtcatatatttagcgacctgattaacctggatgttaggaagggggcgacgaagcgccaaacgcggcaattatagggatttcatccgtctgataccagtcgaatagcgttgccgcgcgctcagagttaattgttgacaaagaattcccgggggcaaattacgttgatcagttttatgtaaggtaaaaaatgttaaacgcagttgcgcaaattatccgcctttacgtcactttatgagcaattcgcatataaaatgtaaaacttttgtactagcataaacacagaaacgaatactggcgaccaggtcttgcggataaagcggtaatgagcaaacaatcacagcatgtattaattgccctgccccacccgctgcttcacctggtcagtttaggtttagtctcgtttatctttacccttttctcgcttgagctttcgcagtttggcacccaactcgccccactgtggttcccgacgtccatcatgatggtggcgttttatcgccatgccgggcgcatgtggccgggaattgcgctgagctgttcgctgggaaatatcgccgcatccatcctgcttttttccaccagctcgctgaacatgacctggacgaccatcaatattgttgaagccgtggtcggggcagtgctgctacgtaaattgctgccgtggtataaccccttgcaaaatctggctgactggctgcgtctggcactcggcagcgccattgttccgcctctgttggggggtgttctggttgtcctgctgacgcccggagacgatcctctcagggcatttttgatatgggtactgtcagaatccatcggcgctctggcactggtgccgctgggattgttatttaaaccacactatctgctgcgccatcgcaacccacggttgctttttgagtcgctgctcacgttagccatcacactgacgttaagctggctttcgatgctgtatctgccgtggccttttactttcattattgtgctgttgatgtggagcgccgtgcgtctgccacgaatggaagcctttttgatcttccttaccacggtgatgatggtgtcgctgatgatggccgcggatccctccctgcttgctacgccgcgtacgtacctgatgagccatatgccgtggctaccgtttttgctgatcctgctgcccgccaacatcatgaccatggtgatgtatgcctttcgtgcggaacgcaaacacatttccgaaagcgaaacccactttcggaacgcgatggaatattccgctatcggtatggcgttagtgggcaccgagggacaatggctgcaaaccaacaaagcgctctgccagtttctcgggtacagtcaggaagagctgcgcggactcacctttcagcaactgacctggccggaggatctcaataaagatctccaacaggttgaaaagctgataagcggtgaaataaacacctattcaatggaaaaacgctactacaaccgcaatggcgatgttgtctgggcgttgcttgccgtctcactggtgcgccacacggatggcacgccgctctattttatcgctcagattgaagacattaacgagctaaaacgcaccgaacaggtcaatcagcaactgatggagcgcatcactctggctaacgaagcgggcgggattggcatctgggagtgggagttgaagccgaatatttttagctgggataagcggatgttcgagctgtatgaaattcctccacatatcaaaccgaactggcaggtgtggtacgagtgcgtgctgccggaagatcgccagcatgccgaaaaagtgattcgtgattcgttgcaatcacgctcgccctttaaactggaatttcgcattaccgtaaaagacggtattcgccatatccgcgccctcgccaaccgggtactgaataaagaaggcgaagtcgaacgtctcctcggcatcaatatggatatgaccgaagtgaaacagcttaacgaggcattgtttcaggaaaaagagcgcctgcacattacgcttgattccatcggtgaagccgtggtctgtattgatatggcgatgaaaattacctttatgaatccagtggcggagaagatgagcggctggacgcaggaagaagcgttaggtgttccgctcctgacggtgttgcatattacttttggcgacaacggaccattaatggagaacatttacagtgccgacacctcacgttccgcgatcgagcaagatgtggtgttgcactgtcggagcggcggcagttacgacgtgcattacagtattacgccgttaagtactctggacggcagcaatattggttcggttctggtgattcaggacgttaccgaatcacgcaaaatgctgcgccagctgagctacagcgcctcccatgatgcactgacgcatctcgccaaccgcgccagttttgagaaacaactgcgtatcctgctgcaaacggtaaacagtacacatcagcgacatgccctggtgtttatcgatcttgatcgctttaaagcggtgaatgacagcgccgggcatgcggcgggtgacgctttgctgcgcgaactggcgtcgttaatgctgagtatgctgcgttccagcgacgtgctggcgcgactcggtggggatgaatttggtctgctgctaccagactgtaatgttgaaagcgcgcgttttatcgctacacgcattatcagtgccgtgaatgactatcactttatatgggaaggccgtgtgcatcgggtaggtgccagtgccgggattaccttgattgatgacaacaatcatcaggcggcagaagtgatgtcgcaggctgatatcgcctgttatgcctccaaaaatggtggccggggccgggtgacggtttacgaaccgcagcaagctgccgcacatagcgaacgggcggcgatgtcgcttgatgaacagtggcggatgattaaagagaatcagttgatgatgctcgcccacggtgtcgcttcgccacggatcccggaagcgcgtaatttgtggctgatttcacttaagctctggagttgcgaaggcgagattattgatgaacaaacatttcgtcgtagcttcagcgatccggcgcttagccatgctcttgaccgccgggtattccacgaatttttccagcaggccgcaaaagcggttgccagtaaaggcataagcatctccctccccctttccgttgccggtttgagtagcgccacgctggtgaatgatctgcttgagcagctggaaaatagccctctaccaccacggttattacatctgattattccggctgaagcgattttagatcacgcagaaagcgtgcaaaaactgcggctggcgggatgtcggatagtgctcagccaggtgggccgcgatctgcaaatcttcaactcgctgaaagcgaatatggcagattacctgctacttgatggtgagttatgcgccaacgtgcagggtaatttgatggatgagatgctgattacgattattcaggggcacgctcagcgactcgggatgaaaaccatcgccgggccagtcgttttacccttagtgatggatacgctttctggcatcggcgtcgatctgatttatggtgaggtgattgccgatgcccaaccgctggatttgctggtgaatagtagttatttcgcgattaactgaggcgtgcttccccatcgcctgatgcgacgctaacgcgtcttatcatgcctacaaatcgctcattccccaggccggataaggcgctcgcaccgcatccggcgaccaacgtcatgcttcgtctggttgccagccttccgtataccagatatgcaacagcgcataagaacgccagggcttccagcgctcggcataacggcggatttgcgccggtgtcattcccggaaatcgctgtttaatcagataatcatccggcaggaaaacatctttcgcctgccagccacgcaaagcaaaataattcgccgtccagcgcccgatacccggaaaagtttgcagcgttttcatcgcctgctccacatcgcccggtattgtcattggtaaggtgccctccagcgccgcatttgccagatgaatcagcgcctctgcccgtttcaacggcatacctaacgcttttaatgcctgcgggtctgctgctgccagccgctgaggcgtcgggaagcagatatactccggaaaatcatccagccgttcgccataaagctgtgccactctggcggtcaattttgccgccatcgccacgctcaccagttggcctaaaatcgcccgcacgccctgctcaaaagcatcaacacagccgggtaaacgcaatccgggccgcgccgcgcctaacctgcccaacgcaccgttaacaatttgtgggttacattgcagatcaaacaggcggctcattttcgccagacactctgcggcaacaggttctaaacctgcacttaaatttatgtgcagagtatggcgggctatatccggaatagcagtcaccacgccgcgatattcgcccaccgccagactacgggcataataactgtccgcgaccgtttccacactgctcaccgcacgggcggcgagaaatcccaacatccacgaccagtcatacggcggctgccagttcagggtatacatcgcatctccttattcatccgctttcagcataaacgttattcagacgctgcgctttgctttcatattccggttgtcgcgacggcaacatttcgctaaagtcacgccccttcttcaccggcatggggattatttcgtgtttattggttttgattacggtacagcaaactgttcagtggcggtcatgcgtgacggtaaaccgcatttgctaaaaatggaaaacgacagcacgctgctgccttcaatgctttgcgcgccaacgcgtgaagcggtaagcgaatggctgtaccgccatcatgatgttccggcagacgacgatgaaacgcaggcgctgttacgtcgggcgattcgttataaccgcgaagaagatatcgatgttacggcgaaaagcgtgcagttcggtctttcctcactggcacagtacattgatgatccagaagaagtgtggtttgtgaaatcaccaaaatcgttcctcggtgccagcggcttaaaaccgcagcaggtagcgctgtttgaggatctggtctgcgcaatgatgttgcacattcgccagcaggcgcaggcacagctgccagaagcgattactcaggcggtgattggtcgtccgatcaacttccaggggctgggcggtgatgaagcaaacacccaggcgcaagggattctggaacgcgcggcgaagcgtgccggattcagggacgtggtattccagtacgagccggtcgcggctgggctggattacgaagccaccttgcaggaagaaaaacgggtgctggtggtggatatcggcggtggtacgactgactgttcattgctgctgatggggccgcagtggcgttcgcgtctcgatcgtgaagccagcctgctgggtcacagtggttgccgtattggcggtaacgatctggatatcgcgctggcgtttaaaaacctgatgccactgctgggtatgggtggcgaaaccgaaaaaggcatcgccctgccgatcctgccgtggtggaatgcggttgccatcaacgacgtacctgcgcagagtgatttctacagtagtgccaacggtcgtctgcttaacgatctggtacgcgatgcccgcgaaccggaaaaagtggccctgttacagaaagtctggcgtcagcgtttaagctatcgcctggtgcgtagcgcagaagagtgcaaaattgctctttcaagcgtagcggaaacccgcgcctcactgccgtttatcagcaatgaactggctacgctgattagccagcgagggctggaaagcgccctcagccagccactgacgcggattctggaacaggtgcaactggccctggataacgcccaggaaaaaccggacgttatctacctgaccggcggtagcgcccgttctccgctgattaaaaaagcgctggcagaacagttgccgggcattccgattgcaggcggcgatgactttggctccgtcaccgccgggctggcacgctgggcggaagtggtgtttcgttaattgaaaaatggctcagcagcggcttaaatctgcctgcgcctgagccagtttttctgctgcctgacgtaacggttccatcaacggcatggtccgtgctggagcatgaaggcggaatcgctgcaactctgtcgcgccgactgtcaacgccgattccagccgatgtcgtttggcggtcattttcgccattaccgcttgtctgtctgctggcgttatcgcttcattcggcctgaacacaaaacggcgttcacagctcgctttccagtcgataaccgcctgggtcagatggtcgccaaaccctttcacttgcttaacgccacgacgggtaacatctgcggctgtttcaataccaaaagaccgtaacgccgctttacgcgcagggccaacgccgggaatagaggcaacatcaataaaaaatccctccagaaacttctgcttctgccgttcccttgcagtgtcatgaagtgctgccagagcgcgtttctcttcttccggtaacccgagaatttcgtccttcattttttcgagcatcgtccgtttggcgataaaaccttccaggccgcctacctgctggatctggcggactaaatggtcatagtccattttcgcacgattaaatgcctcacggcgttgctgaacttctgctttgtacgctttgcttgtcagactgccaataatccagatagccgccagcacaggaaccaaaataatataacgcggttctgcctgaaggccgcaaagcagcagcgataatgctgacagtgcgatctcaagcagaatgatgtattcgcgccgtaacaggcctaaaggaagcggcctgccagtcggttggaaatgatcgggtaatggcagttgcaatgctggcggtgctactgacgccatcaccatcgcccagactttcgccagcacaaaattcccgccggtggtaatgacctcttcgccgagatcaataaaatagataacaccttgattatccagcgcacaccacgggcagtcagtcaaatgagcggggtaaacatgcattgctgaaacgatacatttctttaactgttggcgtagagagtccagtgccgctacccacgctttagccgtcggacgcccggttgccacgccactttccgtgaatgcctgctgaaacatggcttcaacatcactcggtaacatcgatagcggaatagatcgtggcggcggttttaaaccacgtcgctgattatctgacgcgtaggcataacggaaatgggtaatatccgtctccagcgcattacccgcatcagagataagcggcacaccagaataaggatgccgcccaccaaacaagacgtgaaaaattagcaacgcaaggccaaaattatcgtgattttctgtgcgttcaaaaccgacaaatgatggcaaggtttgtagctctggcggcgtaaaatgcgacacgccgacttcgcataaatgcagtgtgccattggcgttaatttgaaaggagtcgctatcaatcagtaccactttgctgtcgcgacctaccataaaactgttctggtttacgtcacccacgacgtgcccgtgctcgtgaaccgtagcaaaagatgaagcaatattgcgcgcaacatagagtagaaaatcccacgcacaatgagggtaactctggcgacgatgtgccgggctatagatcatatgaatcggttctttaccagaaacttttggcatcataaaaccgataacttttccgcctcgtccaccgtgaagcgttgcctgcggccaggcgacataattcaacaactgcgcgtcagctgtcgcagccataaaggcaagtttgtcctgttttaaggcgggtggcggcgtgtgataaatcttggcgacgctatcgacaaactcctcgatatcataaaccgcgccttcaccacctttgcccagttcacggccaagagtggtcaattcacctgtcgatgtaaatacttttatatttgttttcataatatttcgcgggtagttatattatatttcaatgaataataacaactaaccattaaaattatttctatatggggaaaacccactcaagaataaaaatgataatgcaattttatcaggatacaattcaatttcggcctgataatgattaacttccacaggtttttgctaactttgactacaaagggattctggagaaaaaatgaaaaagatattacttatgttgagtctgctattttttactaccgcgggctttagtgaagtttcggatacgttagtgacgggaggttatgataaacaagcgatgtctgacgcgattaaacatgcgcggaaagaaaccgataaattcatcgaggttatgaataaaaaagatgccgatactttcgcagtcaaagccccgataaccgatcacggaagaaccgagcatttctggcttacggatgtcacttattctaacggcatgtttattggcgtaatcagcaatgaccctggtattgttacaaacgtagaatatggccaggagtggaaaatcaagaaagaagatatttcagactggatgtatacgcgcggggataaaatttacggcggttataccattgatcctttattggtcacctatccaaaagaagaagccgacgagctaagagcaaaattagttcgctaatcagccgttatatttattgtttaaactggcggttgaattgttgtcttcaaccgccatgagaaactcactctgcccacagcgccagtgccaacgttttatcatcatccgtacgctcgtttaccgccgggctggacaaaaactgctttaacaattcaggtaataaatcgagttgttcctgcgttgctgccgccagtccattgaaaaacggggtaaagaaaggcacatgaggagaattatccagcatatttaacgccagtcgctggataccatccgtaaatgctgcaactttgtgcgcacgcccagtgctggtgaaagtttccagtctggaaacggcatcttcgtcggtaatgaagtgcgtcatgttggcatattcacccgccatcggcgtgagaggcaattgcagaccgtgacccaaatctaccaccacgccgccatcgccaatctgcataatcaaggtgccgtcaggcgatgaaatcagtcccagaaatgtgcaggcaaaatcgcgaaccgctaattctttggcttccgcctcggcaaaaagtcgttgacgaatggtcagtaccatatttgtggcgaggacatcattaagccccaattccccgccctgcactttttgcgacatataagccatcgcttcattgacggcgagcatcgcgccttcgccaccctgcgagacactgcctgcgccatcagcgacaaataccgacaataatggctgctggtcatttaaccaggcaatctgcatctggcaggcatcctgacaaggcaagtccgcgctgatgtgcgacgttccaacggttgatgcatagaccagacgccagctcacactgacgtccagccttttggcgcttccagcacaacttccgttcccggcgtggagcgggaaaccgaacgcagcgaactggataaccagctaaacagttcacggaattgtaatccttgcagaggcaaaggctgacgaacgctaatttgtgccagcgtcttcatatccgccccctgaacaccgatggaaaagaaagcaaaccttttatcttcttccccccgaaacactttgttggctgcagcctgccactcatcggttggtgcaccatcggtaatcaggaaaatccacgggcgataatacgaaataccatttgcacgatactcacgtttccgctcctctaccatatccagggctttggtaatggccgcacccattggtgtatcgccctgggcaaacaggatgggcggaaaaaaattagcggcgctggtaaagggttgttccacatgcaccgggccgaacgtcacaatgccgagttccactctttttaaagccagcggatcagcaagcagttcatcacgaaaggtaaccaatccggcgttaagttcattaataggtctaccgttcatagaaccagaaacatccagcagcaaaatgcaggggcaacgtggttccgggttactggcaaaatcgctggtggcaaacgtgatttgttcgctcataagaaatcctttcttagagaattatcgaggtccggtatcataccgactgcaataatgaaataagagcaaacgaagaaactttcagaattaggcccggcggcgcagaaaattttgctattcgcctcgcaagaacggagagccgtcgattgacactaagggcggagtgacataatttcaggagtgagggttagggagaggtttccccctccccctggtgttcttagtaagcctggaagctaatcactaagagtatcaccagtatgatgacgtgcttcatcataaccctttccttattaaaagccctcttctccgggagaggctttcccgtttcagcgtcccgctgaaatcatcggcttacctcctttcgccctgaatgcagtctatcgctaacgcgtgaataaaatagtttcctctgtgattattgcgtaacgactcgcaaagaatatttgctggcaggatcgcagactacaaagcctgcggattgacaatcttatcgtgaaggcatactttcaggagtgagggtagagcggggtttcccccgccctggtagtcttagtaagcggggaagcttatgactaagagcaccacgatgatgagtagcttcatcatgaccctttccttatttatggccccttcctcgggaggggctttcccgtttcagcgtcccgctgaaatcgtcggcttacctcctttcgccatgcaagcagtctatcgctaacgcgtagataaaatagtttcctgtgttattactggatgcgtgctcgcaaatgtgcccgtcattcagacgattccagacagtgtttcataattcctccatttttctcccttattggctggctacactagtatcattccgcgaaacgtttcaggaagagaaactcttaacgatgaaaggtagttataaatcccgttgggtaatcgtaatcgtggtggttatcgccgccatcgccgcattctggttctggcaaggccgcaatgactcccggagtgcagccccaggggcgacgaaacaagcgcagcaatcgccagcgggtggtcgacgtggtatgcgttccggcccattagccccggttcaggcggcgaccgccgtagaacaggcagttccgcgttacctcaccgggcttggcaccattaccgccgctaataccgttacggtgcgcagccgcgtggacggccaactgatagcgttacatttccaggaaggccagcaggtcaaagcaggcgatttactggcagaaattgaccccagccagttcaaagttgcattagcacaagcccagggccaactggcaaaagataaagccacgcttgccaacgcccgccgtgacctggcgcgttatcaacaactggcaaaaaccaatctcgtttcccgccaggagctggatgcccaacaggcgctggtcagtgaaaccgaaggcaccattaaggctgatgaagcaagcgttgccagcgcgcagctgcaactcgactggagccggattaccgcaccagtcgatggtcgcgttggtctcaagcaggttgatgttggtaaccaaatctccagtggtgataccaccgggatcgtggtgatcacccagacgcatcctatcgatttagtctttaccctgccggaaagcgatatcgctaccgtagtgcaggcgcagaaagccggaaaaccgctggtggtagaagcctgggatcgcaccaactcgaagaaattaagtgaaggcacgctgttaagtctagataaccaaatcgatgccactaccggtacgattaaagtgaaagcacgctttaataatcaggatgatgcgctgtttcccaatcagtttgttaacgcgcgcatgttagtcgacaccgaacaaaacgccgtagtgatcccaacagccgccctgcaaatgggcaatgaaggccattttgtctgggtgctgaatagcgaaaacaaggtcagcaaacatctggtgacgccgggcattcaggacagtcagaaagtggtgatccgtgcaggtatttctgcgggcgatcgcgtggtgacagacggcattgatcgcctgaccgaaggggcgaaagtggaagtggtggaagcccagagcgccactactccggaagagaaagccaccagccgcgaatacgcgaaaaaaggagcacgctcctgatgcaggtgttacccccgagcagcacaggcggcccgtcgcgcctgtttattatgcgtcctgtggccaccacgctgctgatggtggcgatcttactcgccgggattatcggttatcgcgccctgcccgtttcggcgctgccggaagtggactatccgaccattcaggtggtcacgctctacccaggtgccagcccggatgtcatgacctctgccgttaccgcgccgctagaacgccagttcgggcagatgtctggcctgaaacagatgtcgtcgcaaagttccggcggtgcgtcagttatcactttgcagttccagctaacattaccgctcgatgtcgccgagcaggaagtgcaggccgcgattaacgctgcgaccaacttgttgccgagcgatctgcctaacccgccggtttacagcaaagtgaacccggcagatccgccgatcatgacgctcgccgtcacctcaaccgccatgccgatgacgcaagtggaagatatggtggaaacccgcgtcgcgcagaaaatctcgcagatttccggcgtcggcctggtgacgctttccggcggtcagcgtccggctgttcgcgtcaaacttaacgctcaggcgattgccgccctcggcctgaccagcgaaaccgtgcgcaccgccattaccggcgctaacgttaactcggcaaaaggtagcctcgacggcccttcccgtgcggtcacgctttccgcgaacgaccagatgcaatccgccgaagagtatcgccagctaatcatcgcctaccagaacggcgcgccaattcgtctgggcgatgtcgcaactgtagagcaaggtgcagaaaacagctggctcggcgcgtgggcgaacaaagaacaggccattgtgatgaatgttcagcgccagcccggtgctaacattatctccaccgccgacagcattcggcagatgctgccacagctcactgagagtctgccgaaatcggtgaaggtgacagtgctttccgatcgcaccaccaatatccgcgcatccgtcgatgatactcagtttgaattgatgatggctatcgcgctggtagtcatgattatctacctgtttttgcgcaatattccggcgaccatcattcccggtgttgctgtaccgctgtcgttaatcggcactttcgcggttatggtgtttctcgatttttcaatcaataacctgacactgatggcgttaactatcgccaccggattcgtggtcgatgacgccatcgtggtgatcgaaaacatttcccgctatatcgaaaaaggcgaaaaaccgttggcggcggcgctcaagggcgcaggtgaaatcggctttaccattatctcgctgaccttctcactgattgcggtgttgatcccactgctgtttatgggcgatatcgtcgggcgactgttccgcgaatttgctattaccctggcggtagcgattttgatctcagcggtggtgtcgctgaccctgacaccgatgatgtgcgcgcggatgctcagccaggagtcgttgcgtaaacagaaccgcttctcccgtgcctcggaaaaaatgttcgacaggataatcgccgcctatggtcgtggactggcgaaagtgctgaatcatccgtggctgaccttaagcgtggcactcagcacgctgctgcttagcgtgctgctgtgggtgttcattccgaaaggtttcttcccggtacaggacaatggcattattcagggcactttgcaggcaccgcaatccagctcctttgccaatatggcccagcgacaacgccaggtcgcggacgtgattttgcaggatccggcagtgcaaagcctgacctcatttgttggcgttgatggcactaacccgtcgctgaacagtgcacgtttacaaatcaacctcaaaccgttggatgaacgtgatgatcgggtgcaaaaagtcatcgcccgtctgcaaacggcggtagataaagtgccgggcgtcgatctcttcctgcaaccaacgcaggatctgactattgatactcaggtcagccgcacccagtaccagtttaccttgcaggccacgtcactggatgcgctcagtacctgggtgccacagttgatggaaaaactccagcaactgccacagctttctgatgtctccagcgactggcaggacaaagggctggtggcgtatgtcaatgttgatcgcgacagcgccagccgtctggggatcagcatggcggatgtcgataacgccctgtacaacgcgtttggtcagcggctgatttccactatttatactcaggccaaccagtatcgcgtggtgctggagcacaacaccgaaaataccccaggcctcgcggcgctggataccattcgcctgaccagcagcgacggcggcgtggtgccgctaagctcaattgccaaaattgagcagcgttttgcgccgctctccatcaaccatctggatcagttcccggtaacgaccatctcctttaacgtgccggataactattcgctgggcgatgcggtgcaggcgattatggacaccgaaaagacgctgaatctgccggtggatatcaccacgcagttccagggcagcaccctcgccttccagtcggcgctgggcagcactgtctggctgattgtcgcggcggtggtggcgatgtatatcgtgctcggcattctgtacgagagctttattcacccgatcaccattctctcgacgctacccaccgcaggggttggcgcactgctggcgttgctgattgctggtagcgaactggatgtgattgcgattatcggcattattttgctgatcggtatcgtgaagaagaacgccatcatgatgatcgacttcgcgctggctgctgagcgcgagcaaggcatgtcgccgcgcgaggcaatctaccaggcttgtctgttgcgttttcgtccgatcctgatgaccactctggcggctctgcttggcgcgctgccgctgatgttgagtaccggggtcggcgcggaactgcgtcgtccgttaggtatcggcatggtcggcggtctgattgtcagccaggtgctgacgctgtttaccacgccggtgatttatttgctgttcgaccgcctggcattgtggaccaaaagccgctttgcccgtcatgaagaggaggcgtaagtgaagttttttgccctcttcatttaccgcccggtggcgacgattttactgtcggttgccattaccctgtgcggcatactgggcttccgtatgctgccggtcgccccgctgccgcaggtcgattttccggtgattatcgtcagcgcctcgctgcccggtgcgtcaccagaaacaatggcgtcttccgttgccacgccgctggagcgctcacttgggcgcattgccggagtcagtgaaatgacctccagcagttcgctcggcagcacgcgtattattttgcagtttgattttgaccgggatatcaacggcgcagcgcgtgatgtgcaggcggcgatcaacgctgcacaaagtttgctgcccagtgggatgcccagccgcccgacctatcgcaaagcgaacccgtcggatgcgccaattatgatcctcacgctgacgtccgatacttattcgcagggtgaactgtacgatttcgcctcgacgcagctggctccgacgatttcgcaaatcgacggtgttggtgatgtcgatgtcggaggcagctcactgcccgccgtacgcgtcgggctgaatccgcaggcgctgtttaatcagggcgtgtcgctggacgacgtacgcaccgccgtcagcaatgccaacgtgcgtaaaccgcagggcgcgctggaagatggcactcaccgctggcagatccagaccaatgatgagctaaaaaccgccgctgaatatcagccgttgattattcactacaacaacggcggcgcggttcgtctgggcgatgtggcgacggtgaccgactcagtgcaggatgtgcgcaacgccgggatgaccaacgccaaaccggctattttactgatgatccgcaaactgccggaagccaatattatccagacggttgacagcatccgggcaaaattaccggagttgcaggaaaccattccggcggcgattgatctgcaaattgcccaggatcgctcccccaccattcgcgcctcgctggaagaagtcgagcaaacgctgattatctcggtggcgctggtgattctggtggtgtttttattcctgcgctcgggtcgcgccactattattcccgccgtttcggtgccggtttcgctgattggtacgtttgcggcgatgtacctgtgcggattcagtctcaataacctttcgttaatggcgctcaccatcgctactggtttcgtggtggatgacgccatcgtggtgctggaaaacattgcacgtcatctggaagcgggaatgaaaccgttgcaagccgcactgcaaggtactcgcgaagtcggttttacggtgctgtcgatgagtctgtcactggtggcggtgttcctgccgctgctgttgatgggcggattgccgggccgactgttacgcgaatttgccgtgacgctttctgtcgccattggtatatcgttgctggtttctctgacattaacgccaatgatgtgtggctggatgctgaaagccagcaagccgcgcgagcaaaagcgactgcgtggttttggtcgcatgttggtagccctgcaacaaggctacggcaagtcactaaaatgggtgctcaatcatacccgtctggtgggcgtggtgctgcttggcaccattgcgctgaatatctggctgtatatctcgatcccgaaaaccttcttcccggagcaggacactggcgtgttgatgggcgggattcaggcggatcagagtatttcgtttcaggcgatgcgcggtaagttgcaggatttcatgaaaattatccgtgacgatccggcagtggataatgtcaccggctttacaggcggttcgcgagtgaacagcgggatgatgtttatcaccctcaagccacgcgacgaacgcagcgaaacggcgcagcaaattatcgaccgtctgcgcgtaaaactggcgaaagaaccgggggcgaatctgttcctgatggcggtacaggatattcgcgttggtgggcgtcagtcgaacgccagctaccagtacacgttgttatccgacgacctggcggcactgcgagaatgggagccgaaaatccgcaaaaaactggcgacgttgccggaactggcggacgtgaactccgatcagcaggataacggcgcggagatgaatctggtttacgaccgcgacaccatggcacggctgggaatcgacgtacaagccgccaacagtctgttaaataacgccttcggtcagcggcaaatctcgaccatttaccagccgatgaaccagtataaagtggtgatggaagtggatccgcgctatacccaggacatcagtgcgctggaaaaaatgttcgttatcaataacgaaggcaaagcgatcccgctgtcgtatttcgctaaatggcaaccggcgaatgccccactatcggtgaatcatcagggattatcggcggcctcgaccatttcgtttaacctgccgaccggaaaatcgctctcggacgccagtgcggcgatcgatcgcgcaatgacccagcttggtgtgccttcgacggtgcgcggcagttttgccggcacggcgcaggtgttccaggagacgatgaactcgcaggtgatcctgattatcgccgccatcgccacggtgtatatcgtgctgggtatcctttacgagagttacgtacatccgctgacgattctctccaccctgccctcggcgggcgttggagcgctgttggcgctggagctgttcaatgccccgttcagcctaatcgccctgatagggatcatgctattaatcggcatcgtgaagaaaaacgccattatgatggtcgattttgcgcttgaagcccaacggcacggtaacctgacgccgcaggaagctattttccaggcctgtctgctgcgttttcgcccgattatgatgactaccctggcggcgctgtttggtgcgctgccgctggtattgtcgggcggcgacggctcggagctgcggcaacccctggggatcaccattgtcggcggactggtaatgagccagctccttacgctgtataccacgccggtggtgtatctctttttcgaccgtctgcggctgcgtttttcgcgtaaacctaaacaaacggtaaccgagtaaatgacagatcttcccgacagcacccgttggcaattgtggattgtggctttcggcttctttatgcagtcgctggacaccaccatcgtaaacaccgcccttccctcaatggcgcaaagcctcggggaaagtccgttgcatatgcacatggtcattgtctcttatgtgctgaccgtggcggtgatgctgcccgccagcggctggctggcggacaaagtcggcgtgcgcaatattttctttaccgccatcgtgctgtttactctcggttcactgttttgcgcgctttccggcacgctgaacgaactgttgctggcacgcgcgttacagggcgttggcggcgcgatgatggtgccggtcggcagattgacggtgatgaaaatcgtaccgcgcgagcaatatatggcggcgatgacctttgtcacgttacccggtcaggtcggtccgctgctcggtccggcgctcggcggtctgctggtggagtacgcatcgtggcactggatctttttgatcaacattccggtggggattatcggtgcgatcgccacattgctgttaatgccgaactacaccatgcagacgcggcgctttgatctctccggatttttattgctggcggttggcatggcggtattaaccctggcgctggacggcagtaaaggtacaggtttatcgccgctgacgattgcaggcctggtcgcagttggcgtggtggcactggtgctttatctgctgcacgccagaaataacaaccgtgccctgttcagtctgaaactgttccgtactcgtaccttttcgctgggcctggcggggagctttgccggacgtattggcagtggcatgttgccctttatgacaccggttttcctgcaaattggcctcggtttctcgccgtttcatgccggactgatgatgatcccgatggtgcttggcagcatgggaatgaagcgaattgtggtacaggtggtgaatcgctttggttatcgtcgggtactggtagcgaccacgctgggtctgtcgctggtcaccctgttgtttatgactaccgccctgctgggctggtactacgttttgccgttcgtcctgtttttacaagggatggtcaactcgacgcgtttctcctccatgaacaccctgacgctgaaagatctcccggacaatctggcgagcagcggcaacagcctgctgtcgatgattatgcaattgtcgatgagtatcggcgtcactatcgccgggctgttgctgggactttttggttcacagcatgtcagcgtcgacagcggcaccacacaaaccgtctttatgtacacctggcttagcatggcgttgatcatcgcccttccggcgttcatctttgccagagtgccgaacgatacgcatcaaaatgtagctatttcgcggcgaaaaaggagcgcgcaatgaagttctggcgacccggtattaccggcaaactgtttctggcgattttcgccacctgcattgtcttgctgatcagtatgcactgggcggtgcgtatcagttttgagcgtggctttattgattacatcaagcatggtaatgaacagcgattacaactgttaagtgatgcgcttggcgagcagtatgcgcagcatggcaactggcgcttcctgcgcaacaatgatcgctttgtctttcagatcctgcgttcatttgaacacgataattcggaagataaacccggcccgggtatgccaccgcacggctggcgtacccagttctgggtggttgatcaaaacaacaaagtgctggttggtccgcgagcgccgattccacctgacggtacacggcgacccattctggtcaacggtgcggaagttggcgcggtgatcgcctcccccgttgagcggttaacgcgcaatactgatatcaatttcgataaacaacagcggcaaaccagctggttgattgtcgccctggcaacgttactcgcggcacttgccacttttctgctggcgcgcggtttactggcaccggtaaaacgacttgtcgatggcacgcacaaactggcggcgggcgatttcactacccgcgtaacgcccaccagtgaagatgaactgggcaaactggcgcaagacttcaaccagcttgccagcacactggagaaaaaccagcaaatgcggcgcgattttatggccgatatttctcacgaactgcgtacgccattagcggtgctgcgcggtgaactggaagccattcaggatggcgtgcgtaaattcacgccggagacggtggcgtctttacaggcggaggtcggtacactgaccaaactggttgacgatctccatcagttgtcgatgtctgatgaaggcgctctcgcctatcaaaaagcaccggtagatttgatcccactgctggaagtggcgggcggcgcatttcgcgaacgattcgccagtcgtggcctgaaactgcaattttccctgccagacagtattaccgtatttggcgatcgcgaccgtttaatgcagttattcaataacttactggaaaacagcctgcgctacactgacagcggcggcagcctgcaaatctctgccgggcagcgcgacaaaacggtgcgcctgacctttgccgacagtgcgccaggtgtcagtgacgatcagctacaaaaattgtttgaacgtttttatcgcaccgaaggttcccgcaaccgtgccagcggcggttccgggctggggctggcgatttgcctgaacattgttgaagcacataatggtcgcattattgctgcccattcgccttttggcggggtaagcattacagtagagttaccgctggaacgggatttacagagagaagtatgaccgagttaccaatcgacgaaaacacaccgcgtattttgatcgtggaagatgaaccgaagctggggcagttgctcattgattatctgcgtgctgcgagctatgcgccgacgcttatcagccacggcgatcaggtactgccgtatgtgcgccagacaccaccggatctgatcctgttagatctgatgctccctggcaccgatggcctgacgctgtgccgggaaattcgtcgtttttctgacattccgatcgtgatggtgacggcaaaaatcgaagagatcgatcgcctgctggggctggagattggcgcagatgattatatctgtaagccgtacagcccacgggaagtggtagcgcgcgtcaaaaccattttgcgccgttgcaaaccgcagcgcgagttgcagcaacaggatgctgaaagcccgttgattatcgacgaaggtcgttttcaggcttcatggcgcggtaaaatgcttgacctgacgcctgcggaatttcgtctgctgaaaacgctctctcacgaaccaggaaaagtgttctcccgcgagcaattgctcaatcatctttatgacgactaccgcgtagtaaccgaccgcaccatcgacagccacattaaaaacctgcgccgcaagctggaatctctcgacgccgaacagtcatttatccgcgccgtttatggcgtcggttaccgctgggaagccgacgcctgccgcatcgtttagttttagcgacattattttgttagccggagatggcgttcagaccagatccggcaacattatcccacgcatggtcagcaaactgacattatctctccgccctggcaggcatcagaaaatcgctcatactttaatcggtaaacagcacctttagatgctgttttcgatacacaatttcaatcaaggagtcattatggctggttggtttgaactcagtaagagcagtgataatcagttccggtttgtgctaaaagcgggcaatggtgagactatcctcaccagcgagctttatacctcaaaaacctctgcggaaaagggcatcgcgtcggtgcgtagcaacagcccgcaagaagaacgctatgagaaaaaaacggcaagtaacggcaaattctatttcaatctgaaagccgctaatcatcaaattatcggctccagccagatgtacgccaccgcgcaatctcgtgaaaccggaattgcctccgttaaagccaatggcacaagccagacggtgaaagacaatacgtaattacgatgccgggcgtgggttgttggcgtccggcgctttaccagagccccccacagcgctacaatgcccgcccttaaagtgggggcactcccctaaccgcttcatcaggtgaagcggatctgacctgtcatcagaacgagagaattatgtttaaaccggaactcctttccccggcgggaacgctgaaaaatatgcgttacgctttcgcttatggcgcagatgctgtttatgcgggccagccgcgttattccctgcgtgtgcgcaacaacgaattcaaccacgaaaatcttcagctcggcatcaatgaagcccacgcgctggggaaaaagttttatgtcgtggtcaacattgcaccgcacaacgccaagctgaaaacctttatccgtgacctgaaaccggtggtggaaatggggccggatgcgctgattatgtccgatccagggctgattatgctggtgcgtgagcacttccctgaaatgccgatccacctttcggtgcaggctaacgccgtgaactgggcgacggtgaaattctggcagcaaatgggcctgacccgcgtgatcctctctcgcgagctgtcgctggaagagattgaagagatccgcaatcaggtgccggatatggagatcgagatcttcgttcacggcgcgctgtgcatggcctactccggtcgctgcctgctctctggctatatcaacaagcgcgacccgaaccagggcacctgcaccaacgcctgccgctgggagtacaacgtccaggaagggaaagaagatgatgttggcaacatcgtacacaagtacgagccgattccggtgcaaaatgttgagccgacgctgggtatcggcgcaccaaccgacaaagtgtttatgatcgaagaggcccagcgtccgggcgagtatatgaccgcgtttgaagatgagcacggcacttacatcatgaactcgaaagatctgcgcgccatcgcccatgtagaacgcctgaccaaaatgggcgtgcattcgctgaaaatcgaaggtcgtaccaaatctttctactattgtgcacgcaccgcacaggtttaccgcaaagctatcgatgacgccgctgcgggaaaaccgttcgataccagcctgctggaaactctggaaggtctggcgcatcgtggctataccgaaggtttcctgcgtcgtcatactcacgacgattatcagaactacgaatacggttattcagtttctgaccgccagcagtttgttggtgagtttaccggtgagcgcaagggggacctcgcggcggtagcggtgaaaaataaattctccgttggcgacagccttgagctgatgacgccgcaaggcaacattaattttacccttgagcacatggaaaacgccaaaggcgaagctatgccgatagcaccaggcgatggttatactgtgtggctcccggtcccgcaggatcttgagctcaattacgcgctgctgatgcgtaatttctccggggaaaccacgcgtaatccccacggtaagtgattaatttcgattatttttcccggatggaaaattcttagaaaccgatcacatacagctgcatttattaaggttatcatccgtttcgctgaaaaacataacccataaaatgctagctgtaccaggaaccacctccttagcctgtgtaatctcccttacacgggcttattttttacgcgtaatacaatgaaataaaaggatttatttctggtcacgtccacacattgaccacatcgacaaaaaagcccctcgactgaggggcttcctgtttctaattacatccacataatttgctgccctgacggcaacgggtgcggccttacgacgtggacttctcccggcttcacaatgtatcgctgtaccgactcataagtgatgaacgtggcgctgcaattcacgttctgacactggtgataacgctcttttgtcgtgtcagtgatatagcggcttgtacgcgcatgtgcggcatgctggcataaaggacaatgaaacatcgcgagcacctcttccggttttgttgatggtgccattttagttaatttacccttacaaaacaaacagataaaataaaaacatcactcattatcttctgtttcgtaccccacatcagaaagcctgacctcaagctctaatgacgtcgtgaagccgctattattcagaaaatgtgtcaccttagtgattgtccagtcctgctcgtctatgacgcgcttaaagccagacactttgaccggtgtttccgtgtaaatatctgcccgaccggtagccaggctgatggagaactctgctacacgggcttatttttttatgcataagccctatctctggtaaccgtcttccattgaccacatcgatagaatcctccttcatagcacgatgcctttcacttatcggcatcgtgctcccacaggttccggctacgcacagccagaacgcgcatatttgacgcttaccaaaaaatattctcactctccacatttgaatgtcagacgagcgacaccatgtaatcctacaccttctgtcttcagctcaactatttgcatttttttgccctgagtaacacagaaatgagttgcatcattttttactatattttctgcaccagatattctacccctggctaaagaagcttcggcttcggtgtagtattggttatcgagtttacgctgaatattacttttatatgcaagaccaaatttaccgatacttgtctcatcattatgcacagcacaaccagacataataaaaatactaattaatgatatagcagctatctttttcatctcaccttcccccattaaataccaacgacactctctagtgtttaaatataataatggcatgattattataattgaataggattataataaatgttctgtacaacatttcctacataagtaggaattacggacattgaggcccttcagggtaactccatgggggctttaatatattatattgaagatgccactgtttagttgaatattaggtatatgctcttttttgaaatttatcggtggcagccgttagtattcgctgtccccattgcaagctcctggtggtaaccactgaatcctccatacttgaactgactttttatcctccgactttcatcctgttctgactccaccttttgttttctgctctacactatctacagaccaatcataaaggcacatacgatcatggcagaatttcccgccagcttactgattcttaatggcaaaagtactgacaatctacccttgcgcgaagcaattatgctgttgcgtgaggaaggaatgacgatccatgtgcgggtcacctgggagaaaggcgatgccgcacgatatgtagaggaggcccggaagtttggcgtcgcaacggtgattgccggtggtggcgatggcaccattaatgaagtttctacggcgttgattcagtgtgagggggatgacatacccgcgctgggaattttgccattaggaaccgccaatgattttgccaccagtgtagggattcctgaggcactggataaggcgctgaaactggcaattgccggtgacgccattgcgatagatatggcgcaggtcaacaaacaaacctgttttattaatatggcgacaggcggatttgggacgcgtattaccacagaaacgccggaaaaattaaaagccgcgctgggtagcgtctcttacatcattcatggcttaatgcgtatggatactctgcaaccggaccgttgtgaaatccgcggtgaaaactttcactggcaaggtgacgccctggtcattggtattggtaacgggcgtcaggccggtggcggtcagcaattgtgtccgaacgcgttaattaacgatggcttgctgcaactgcgcatttttaccggcgatgaaatacttccggctctcgtatcaaccttaaaatctgacgaagataacccgaatattatcgaaggcgcttcgtcgtggtttgatattcaggcaccacacgacatcacctttaatcttgatggcgaaccgttgagtgggcaaaattttcatattgaaatacttccggcagcgttgcgttgtcgattaccaccagattgtccactgttgcgttaatcaaactattctctcttgaaccagggagaatccgtaatgccggatgcggtgtaaacaccttatccggcatacagaacaatactacaccgtaattaattttacccgcgtcttctgcaatgccagtttatccacctctgacacagcatcatcggtaataataatgtcaattttttcgattggtagtacctgattaaaaccgcgacggttaaatttcgatgaatcgagaacggcaatcactttattagcggctgtgaccatcgcaccgctaatagaataaccttcattaaaggtcgtaataccattaaccgcatcaataccatcagcaccgacaaacattaaatcggcattaatatcctgtaatgaacgctcggcaatggaaccatgcatcgagcgcgttttatggcggaccgtgccaccacagacgaccagagtaatgtctttattttcggaaagggcaaacgctgccgggagactgttggtaatcaccgtgatatttttggcggtcattaatccttcggcgataagcattgtcgtacttccgctgtcgagaataacggtctgatcttacccagcaatagtggacacgcggctaagtgagtaaactctcagtcagaggtgactcacatgacaaaaacagtatcaaccagtaaaaaaccccgtaaacagcattcgcctgaatttcgcagtgaagccctgaagcttgctgaacgcatcggtgttactgccgcagcccgtgaactcagcctgtatgaatcacaactctacaactggcgcagtaaacagcaaaatcagcagacgtcttctgaacgtgaactggagatgtctaccgagattgcacgtctcaaacgccagctggcagaacgggatgaagagctggctatcctccaaaaggccgcgacatacttcgcgaagcgcctgaaatgaagtatgtctttattgaaaaacatcaggctgagttcagcatcaaagcaatgtgccgcgtgctccgggtggcccgcagcggctggtatacgtggtgtcagcggcggacaaggataagcacgcgtcagcagttccgccaacactgcgacagcgttgtcctcgcggcttttacccggtcaaaacagcgttacggtgccccacgcctgacggatgaactgcgtgctcagggttacccctttaacgtaaaaaccgtggcggcaagcctgcgccgtcagggactgagggcaaaggcctcccggaagttcagcccggtcagctaccgcgcacacggcctgcctgtgtcagaaaatctgttggagcaggatttttacgccagtggcccgaaccagaagtgggcaggagacatcacgtacttacgtacagatgaaggctggctgtatctggcagtggtcattgacctgtggtcacgtgccgttattggctggtcaatgtcgccacgcatgacggcgcaactggcctgcgatgccctgcagatggcgctgtggcggcgtaagaggccccggaacgttatcgttcacacggaccgtggaggccagtactgttcagcagattatcaggcgcaactgaagcggcataatctgcgtggaagtatgagcgcaaaaggttgctgctacgataatgcctgcgtggaaagcttctttcattcgctgaaagtggaatgtatccatggagaacactttatcagccgggaaataatgcgggcaacggtgtttaattatatcgaatgtgattacaatcggtggcggcggcacagttggtgtggcggcctcagtccggaacaatttgaaaacaagaacctcgcttaggcctgtgtccatattacgtgggtaggatcagtcatcccttcgtggatcattttgactgccgcctgcgctattctgttttttggcgcgctggcgagctgaaatcgctctttaaacccgacttcctgggtctcggtttcactattaccagacattattttcgccgcaccgccatgaaagcgcgtaaccacgcctttttgttcgagaaagcgcaaatcggcacggattgtcgcttccgaggcagcaaatactcccgccagatcctgaacaagcacggttccctgttcattcactaattggatgatcttattccttcgctcgaatgaattcatcgtcatttacccatattcaattgtggctagtgtaaacgaagggggaccattggtgaatgatctgttttgcacaataccgggccagcatcacgctggcccgcggtttcagggaatgagcaacactttgcccggcatagcattacgagcgatgtcacgcaccgcctgggcgaagctttcaaagcttccacggtgagcgattaatggctccaggcttaacttacgttctgtcagcaaccggctcgccgtttcccactcctgccccggccaagggctggagtagttcatccaactgccgataaccgtcagctctttacgcaatattttgccaaacgttgccgatgttaaatgcagatcctgatgcaacgtgcccaccagcgccagttgggcatgaggaccggcaatctctaccgccagttcgacagtttgcggtacgccagccgtctcgaggataagctgattaaagcgcagttcgcgtaaaacgctctgcatttgcggcgcgctcatttcgctactgttaaatgtttgcatcgcaccgaaagattttgccagtgccagtttttctgaactaatgtcgatcgccgtcacactctttgctcccagcgcgacagcgcactgaatggccagcaggccaatggttccggcaccaataataataacgtttttattctcacaaccttgcgctaaatgaaaagcatgcagaccaacggtaatcggctcaataaaagccccatcctcaataggcatatccgtgggtagagcaaagacattttttcgcttaacgacaatatattcagcaaatccaccatcacgccgcgagccaataaaatcatattttgcgcactgggaataaaaccctttcagacactctggacaagtaaaacagggtaataacggcacacaggcaaccgcatcgccagggtgtaaatcatcaacaccggatcccaccgcatcaatatagccgctaaattcatggcctaacgttattggataataatgtgcaccatttttaaatatcctgggtaaatcggaaccacataagcccgagctggcaatttttacccgcacctcatcctgatgtttaatttcaggaatgacgctttctgcaacgcgcacgataccatcagtatcattcaccactgatttcataaaaactcctgattgttaagggggataacctccccctcaggtaaaaattattctgcgagaacgactttctcttgtttaataaagccacgcgctctacgccaggtcatgaaaataccggtcagataaattgcaccgataataatgaaaccgggaatattttgcggggagaaaacctgaatcagtaaccaggtaatgggagaaccgccctgatccattgaagccaccatacccccggcttttaacgccccagcattagccgccagttgggtgtgcaaaccaatagtttgcgtcgcgatccacagggtgatgctcataatgatgacacccgagattaaggtgcggaacagatttccacgatgcacggcgaccgccatcgccacgaagaagccgatggtggcaagatcgccaaacggcagcacctgattacccggcacacaaacagcaattaaaatggtgagtgggataaaaatcaggcttgccgataccaccgccgtatgtcccagcagcaacgccggatcaaggccaatcaggaactcctgaccgccgaacttcgcctgtaaacgactacgagcctgcttagcgatgggcgttaaaccatccatgatgggtttaatcacccgtggcattagcagcatcactgccgccgtttttaccgccagctgcaatacacctttgacatcgtaacccgcgaggatgccgataatcagccccatcacaaaacccacggtgacaggctcgccaaatggaccaaatttgcgctgaatatcgtcggcgctaaatttaattcggttaacgcctgggattttctcgatgatagcatcgaccagcaccgcaatcggccccatatacgccgacgtaccgtgcggaatagcaataccttccagctcaaagaaatttcgggtatcgcgggcaaaccagtcgccgagcttataaacaaacgccgcgtgaattaccacacctgccatccctatcatccatgaaccggttgccagatgcagcaacgcgccggtgaaggtcatatgccagatattccagatatcaacatttaccacccgcgtcatacgggtcagtaacatcgccacgttaaccagaatcgcaatcggaatcgccaccagcgcaatttgcgacgcccaggtcattggtgaagagcccggccagccaacatcgaccacatgcagattcaggtcgaaattttccgccatcgctttcgccgccgggccaatggaatccagcattaagccaatcacaaggccaatgccaacaaagccaatcccgatatgcagacccgctttaaagcaatcgcctgccttcatgcctaatattttagaaaaaataatgatgacaatcggcagcatcaccgtagggccgaggtcgagaatataacgcatgacttctgaaaacataggtcacccctgtaagatagtcagaattttattttgtaatgcttcgataccgataccagaaataaaaggcatgccgtgaactaacggaatatcgccaaaactacgatccactttggcagtggtgcatatcaaatgcacaccatccatataggtttctatttcattaacccgacactggattaattcaacaggaatattatgattctgacacaactctttaatttcttccgccgccatcgtagaggtcgcaaccgcgcctccgcaagcgacaataatcttgcgtttcataaatagtcctttttattgttacagagggatttattcgtctgaatctaaaacatactttgtgaagtattcctttaactgggtttcaggaagagtgattagtgtctcgacgatatcgggctgttgtaacttgccaaataaacagcgtaaaagtttcaattgctgctgcggattttccacaatcaacgcaataaccaacgataccgccacgtcgttatcatcatccgcttgctgaaaatgaactttatttgttggccttaacagataaatggctgacgacttagcatgaatcgcctcacaatgcggtattgcaatagcgtgctgctcaagcattatcccggtagggaattctgcttctctggcaattaatgcctgtggccaggtatcatgaaccacacctttggcgagcatctcattaccgatatgggttaaaacttcgctacgatcgacaaaagaaattccgctacgaacaaacaggttagtcatataccgtccttattccgcacagccgtagcgataggcgcgcaaaacatcataaattttatccataatcagctgatgcggtattgctgataattccccggactgaatgcgttcaaattgtttgggaagatactgactaatcatgcccagtgggatgtccacgccttcaagattcaccatcatcgtttcgacgctatttttaatccgactatgcggccagtaataacgaatacgatccgacaggctgtaacgaatatccagtaatgaatcgttaaaacccgtacgataatattttttccagtattgcggttcgtcgagcatcacttcttcaattaccgccaggcaaccgctgcgattttcaggggcgataagttcctgctcaatttgtgccagtgcaaatatcgcctcgcgtaaagcaaaggttaatgcgggaccgactttcaatattgcaaagtgatcgcggactaattcccaataagccgtccgggtctggtaatcggtagaatgtgcttcataaaccattcgggtgttttctatccattgcgccagcggctgcgcttcctgcggctgataatggataatattgctgtgatcaaattccacacccggctgcaccacgatggcaatcacacgtgttaacgcctctgtcagcccacgggcaataaaggccttttgatgcgtacgtaaagtattggcggcatcttcaacatgggtgatgtgtactgactgaatggcgctggcctcaccgcccggaaccggaacttcggtgccaatgacatagctcagttgctcacgctggcaatctgtcgccacactttccgcagcaaagcaaagcacagcagctcgttccgcaaccgtttctggtgctaacggtatgggatcccccgcgcaggacattgacgcatcaagatgaattttactgaagccggcacgaacatattcctttaccagctcgacggatttttccatcgccgcatccgcattttcttgctgccagcagtttggccccagatgatcgccgccgagaataatgcgttcgcgtgcaaacccaactttatcggcaatcgtaaaaacaaattcgcgaaagtctgccggtgtcattccggtataaccgccaaattgattgacctggtttgacgttgcttcaatcagcactttgcgcgtgctgttgcgatcaaatgccagcgccgcttcgataaccaacggatgggcagaacagactgaacatatgccgatatgttcaccagctttatgccgggcaattaacgttttcatgttttttccttgttaaatggcaggtgcgttatgccctgccctcgcagccacaatcggcaatcactttgctcaccacatcgcgcattgcggatttagccgactgcaaataatcccggggatcggtcgcttcagggtgctcggtcaggtaattttttaacgcctgcgagaaggcatttttcagctccgttgcaacgttgattttgcatatccccagtttgatggtttgctgaatatccttagtcgataaccctgacgcgccatgcagcaccagcggtaagttcacccactggcgaatgttctccagtctagaaaaatcaagcgccggtgcgctggcatacatcccatgagccgtgccgatggcgaccgccagggaatcaattccggttgcctcggcaaattcacgcgcctgagcggggttggtgtacaacgcatcggcttcattgacttgcacatcatcttcctggccgccaagttgccccagctccgcctcgacgctgacatcaaagcgatggcaaaaatccaccacctctttgacccgtgaaatattttgcgcaaaaggcaaatgcgaggcgtcaatcatgactgagcgcacgccagaacgaaccttctgagcgatatcgtcaaatttcgtgtgatggtcgagatgaattgccagtggatggtgatattgcttcgccatcgcgctgaccagcgccaacagattttctgtaccagcatgagtaaatgtgccaggcgttccggcgatgatgaccggcgcatgcaggttggcagcggtttctaccaccacttgcatcgtttcgagattgtgaatattgaatgccggaaccgcataaccgccgcgctgtgcgttgttcagcatctgctttgtcgataccacgtacattttcatatcctgtcgtttgttttcgatttcaaaatataatgaaattatttgtttttaaatatcgagataacgatcacaaaaacgacaatatgaaaattattcgaggagtgaaaggcaaaaaaacggcctcccgatagggaagccgtagcaaagtgcgcgtgtttttatgccggatgcggtgtaaacatacgtggcagtgctatgtaggcatgataagacgcttcagcgtcgcatcaggcataggttgccggatgcagcgtaaacgccttatccgtcctacggggtggtgttgttcgtataaggcgtatcaggcgatagtaattttgctatcgagataaacgtcctgcacggcgttaatcagtttcacgccgtcagccatcgatttcttgaacgctttacgtccaagaatcagccccattccgcctgcgcgtttgttgataaccgcagtacgcactgcatcgctgaggtcagtttcaccgcccgcagcaccgccggagtttatcaacccagcccgacccatatagcagttagctaactgataacgcaccagatcaatcgggttttcgctggtcaatttgctgtaaacacgatcgtcggtgtaaccgtaattaattgctttatagccgccgttattttccgccattttttgtttgacgatatctgcaccgatggttgccgccagatggtttgcctgaccggtcaggtcggcggaaacatggtaatcaacgccatctttcttaaaggcggagttacgcaaataggcccacagcactgtcaccatacccagctcgtgcgcacgttcaaaagccgcagaaatttcttcaatctggcgacgtgactcttccgagccaaaatagatagtcgcaccaaccgcaaccgcgcccatgttgaacgcctgctccacgctggcatacagcgtttgatcgtaggtattcgggtaacttagcgtctcgttgtgattaagtttgacgaggaatggaatgcgatgcgcataacgccgcgataccgacgccagcacgccgtaagttgacgccacacagttacagcccgcttcgatcgccagttcaacaatgtttttcgggtcaaagtagagcgggttagcagcaaatgaagctccggcagagtgctcaacgccctggtcaaccggcagaatagaaagatatcctgtgccagccagacgcccggtgttgtacaacgtctgcatattacgtaacaccgctggcgggcgattattgtcaatcattacgcggtctacgtagtcatgtccggggagataaagctggtcagaaggaattgtcatacaacggtgctgtaaaaggttgtcggcgtctttgccaagcaactgcgcaatatctgtcattactatgctcccgtaaattccgattggatatcggctatggattgtcctggcccgccttttgcgggcaatcataatcctggtcgttacgggcgagtttttccatcttttggatgttttttcagcgttttctgttggctcgattcatcagaaaaaatgttagcgcggtcaagttttcaccgcaaaggtatttaaaaggtattattaagtggtattgtcatcgcgtaccttacattacctgtcatgaaggaattaaaagatgaaaacaacagcaaagctgtcgttcatgatgtttgttgaatggtttatctggggcgcgtggtttgtgccattgtggttgtggttaagtaaaagcggttttagtgccggagaaattggctggtcgtatgcctgtaccgccattgcggcgatcctgtcgccaattctggttggctccatcactgaccgctttttctcggcgcaaaaagtgctggcggtattgatgttcgcaggcgcgctgctgatgtatttcgctgcgcaacagaccacttttgccgggttcttcccgttactgctggcctactcgctaacctatatgccgaccattgcgctgactaacagcatcgcttttgccaacgtgccggatgttgagcgtgatttcccgcgcattcgtgtgatgggcactatcggctggattgcctccggtctggcatgtggtttcttgccgcaaatactggggtatgccgatatctcaccgactaacatcccgctgctgattaccgccggaagttctgctctgctcggtgtgtttgcgtttttcctgcccgacacgccaccaaaaagcaccggcaaaatggatattaaagtcatgctcggcctggatgcgctgatcctgctgcgcgataaaaacttcctcgtctttttcttctgttcattcctgtttgcgatgccactagcgttctattacatctttgccaacggttatctgaccgaagttggcatgaaaaacgccaccggctggatgacgctcggccagttctctgaaatcttctttatgctggcattgccgtttttcactaaacgctttggtatcaaaaaggtattattgcttggtctggtcaccgctgcgatccgctatggcttctttatttacggtagtgcggatgaatatttcacctacgcgttactgttcctcggtattttgcttcacggcgtaagttacgatttttactacgttaccgcttacatctatgtcgataaaaaagcccccgtgcatatgcgtaccgctgcgcaggggctgatcacgctctgctgccagggcttcggcagtttgctcggctatcgtcttggcggtgtgatgatggaaaagatgttcgcttatcaggaaccggtaaacggactgactttcaactggtccgggatgtggactttcggcgcggtgatgattgccattatcgccgtgctgttcatgatttttttccgcgaatccgacaacgaaattacggctatcaaggtcgatgatcgcgatattgcgttgacacaaggggaagttaaatgaaaacagaacgtattctcggtgctctttatgggcaggcgttaggggatgcgatggggatgccctccgagctttggccacgcagccgcgttaaagcacactttggctggattgaccgttttcttcctggaccaaaggagaataacgcggcctgttattttaaccgcgccgaattcaccgacgatacctcgatggcgctgtgtctggcggatgcgttactggaacgtgaaggcaagatcgatccggatctgattgggcgtaatattctcgactgggcgctgcgtttcgacgcctttaacaaaaacgtactaggtccgacctcgaagattgcgcttaacgccattcgcgacggtaaacccgttgctgaactggaaaacaacggcgtgaccaacggcgcagcgatgcgcgtctcgccattaggttgtttgcttccggcgcgtgatgttgattcctttattgatgatgtagcgctggcgtccagcccgacccataaatccgatctggcggttgcaggcgcggtagtcatcgcatgggcgatttctcgtgccattgacggagaaagctggtcagcgattgttgattccctgccttcaattgcgcgacatgcacagcaaaaacgcatcactacgttcagcgcctcactggcggcgcggctggagattgcgctgaaaattgtgcgcaatgccgacggcaccgaatccgccagcgaacagctttaccaggtcgttggcgcaggtaccagcactattgagtccgttccgtgcgccattgcgctggttgaactggcacaaaccgacccgaatcgctgcgccgtcctgtgcgctaaccttggcggcgacacagacaccatcggtgctatggcgacggcaatttgcggcgcgttgcatggcgttaacgctatcgatcctgcgttaaaggcggaactggatgcggtaaatcagcttgatttcaaccgctatgccacagcgctggcgaaatatcgtcaacaacgggaggcggtatgagcggcgctcgattacacacgctgctgcctgaattaaccacgcgtcagtcggtgatggtcgtcggcgcggcggtcattgacgtgatcgccgacgcttatgccctcccctggcgtgggtgcgatatcgaactgaaacagcagagcgttaacgttggcggctgcgcactgaatattgccgtggcgttaaagcgcctcggcatcgaagcgggtaatgccttgccgctcggtcagggcgtgtgggcggagatgattcgcaaccggatggcaaaagagggcttaatcagcctgatcgataacgccgaaggtgataacggctggtgtctggcgctggttgagccggatggcgaacgcacttttatgtcattcagcggtgttgaaaatcagtggaatcgccagtggctggcgcgattaaccgttgcgcctggcagcctgctctatttttccggttatcaactggcctcgccctgcggcgaattgttagtggaatggctggaagagctgcaagacgtgacgccgtttatcgattttggcccacgtattggcgatatcccggatgcattactggcgcggatcatggcctgtcgacctttagtgtcgctcaatcgtcaagaggctgagattgccgccgaacgttttgctttatccgcagagataacaacacttggcaagcaatggcaggagaaatttgccgcgccgttgatcgttcgtctcgataaagaaggcgcatggtatttcagcaacgacgcttctggctgcattccggcatttccaacgcaagttgtcgacaccattggggcgggcgacagtcatgccggtggcgtacttgccgggctggcctctggtctgccactggcggatgccgtattactgggcaatgcagtggcgtcgtgggttgtcgggcatcggggcggtgattgtgcgccaacgcgcgaggaactactcctcgcacacaaaaacgtatagatcgctgcgacagtggctaatgctgtactcaataggccgttgctgttggtcaagcgccacttgcttgatcaccagcaccggtattttgctatctaactgaatatgtgactgaaactcggcatccggcatccgggcgctaacgcgggaacgcgtacgttgtgggtaaatgtgctggctgcggaaatagtcataaagtgaaatcccgatggcatcaacatcatgaattaaatgcgccggaacccacgattcctcaatcgataccgcttcttcatcgacatagcgaatacgcttaagcaaaaagacatcacttcctgcttcgaccgccagctgctgcgcgacttcttcgggacatttcacgacacgcttgttaacccatagcgtatcgggctttttcccgcgcaataccacctgctgagaaaaacctcgcgcttctttcaacgagtattcgaagatgttgttgatctgcgtgccgtaaccgcgcgaacgcgtcaccacaccctcttcttccagcgcctgcatcgccttgcgcaccgtaatgcgcgaaacgccggttaactgacttaaatcacgctcaccgggcaaaatattgccatgctccagcaccccgctgcgcacggcattttttaccgtttcggcaaacttaatataaagcggcgtgttatccgccgctaaaatacgctcgttcagttgggcaatcagctgggtatgcgcttgttccatttgtctttttcctgccggggagtctggtgggagtatatcactgcttcttatttaaggcgtttctttaatcccatcaacgaatgcctgcaactcctccaccgtgccattaaatacattaaaatccaccggaccattgatgccatctacctgtccacggtcggaatgctgccagaagcgccaggccattccgtcattgtccggacgacgttgatagtagtgagccacccaccacggatattcattgaaatagcccgccagattggtgtgataaaaaacggctcctgagtaaataatcggctttttccccgtacttttttcgaccatttttagccactgacttacccgcttgcgtaattcttttgccgataattttccccgttcttctacgtccagcacggcagggaaatcgccttgtgagaaatccaccgtttgcagaaataatctcgcctgaactgaagcggataccgacggggagaaataatgatacgccccacgcagcaggccattttcgcggcttagttgccagttacgcgaaaaataggggtccaccagcttttcgccttccgtcgccttaataaaagcaaactgtaagcggataccattgtcgcgcatttttgccacccgctgccagtcgatccgctcctgccagcgcgaaacatctattccgtgaatggtgtaactggcaggaatgcgaatagcgaaagatttaaccgggcgataaccgtagaagtggatgtagtctgtaatctgaactgctgtcgaatagaaaaaattcaccgtctgacgcggataaattgcaacgatggaaattagcccaagagcgcataatagagaggtgagtttttttcgactggtaattcttagctgcattggtttcatccctgaatgtcagtgccaaaggctgacaataaccaaagcagctatagtacggtgctcaccaccaggcgtggaagtggtgaaccggaccaataccgtgaccaacttccagcgtgtcggcctgggctaacgccgatgaaagccagctttttgcctcctgtacggtgtcagcccagtttgtatggcgcgggcgtagtgcagccaacgccgcagagagtgtacaaccagtgccgtgggtgtttttggtcataatgcgcggtgcggtaaaccgttgttcaccctcgcgggtaaacagccagtccgggctttgctcatcatccagatgaccacctttcattagcactgcgccacagcccatcgccaacagcgatcgcccttgttccagcatttcctgttcggtgcgcgcgtgtggcgcgtcgagcaaggcggcagcttcgggcaagtttggcgttattaatgaaacctgtggcaataatcgactgcgcagcgtagcaaccgccgaaggtgaaagcagcgggtcgccgctttttgccagcataacggtgtcgagtaccacgttttggatctgataacgttgcaaccgttctgccaccgcttcaacaatatcggtttccgccagcataccgattttagtggtatcgattcgcacatcgctgaacaccgaatcgagctgggcggcgacaaaatcaggctcaatgcgatacaccgactgtacgccacgggtattttgcgccaccagtgcagtaataactgagcaaccataagcgccaagtgccgagaaggttttaagatcggcctgaatccccgcaccaccactcggatcagtaccggcaatcgtcagagcgttaattcgtttcatgcctgcacctcctgcgtcaattgccagagcgcatcaaggaaatgtggaacaaaactgcctggcccctcgcttctggcgactgcgcgttctccggcttgtttcatccagtgacaggcagatgcgacattttccagcgtatcgcctggtaacgcacagcaggcagcgacaaccgccgataatgcacagccagttcctaccactttggtcattaacggatcaccaccgtgaataccaatgatacgatgtccatcggtaacataatccatctcgccagtgaccacgacgattgcgccagtttcccgtgccagtgtttgtgcagcgggtatcgcgttagctgcggcgtcagtggtatccactccccgtccgccattagcaatgccagctaatgccatgatttccgaagcattaccacgtatcgctgccggtttaaaagataaaagttcatgacaaaaatggcggcgataatcgagcgcacccaccgctactggatcaagcgtccagggtgtttgagagctttttgcttgctcaacggcagcacgcatcgcctgagcgcgtggctgcgtcagtgtgccaacgttaatcaacaaggcactggcgatagccgcaaactgactggcctcttcggtttcgataaccatcgctggcgatgcaccgagcgccagcaaggtattggcggtaaaggtttgcaccacatcattggtcatgcagtgcacaagaggggaatgttggtgaaaaaggtgtaacgcgtgcgcagattgcgctgaacccagcaggtcgacttgcatagtttgctcctgccataacgtgaagaagcaatgacctggtggtccgtgacttccctacgctggcattatccagatcaggtgatacgggtatttctcagccttcacgcagaagggcaccccgagtcgtttggttgcgatgataaatcgcagaggaggatggtaatgtccagcgcacgcgttgtaaacgaggaaaaacggcagttttacaatcgcgttaataaattatttgatatatgaatccagcaccttcagaacgacatccagatcttcttcacgttttagctcatccccctggtgaacgatgtgttccgtcagatgacctttaatcacttcccgcatcagaccgtttaccgcgccacggatagcagcaatctgttgtaaaactgcagcgcattcgtgcggctcgtcgagcattttcttgagcgccacgacctggccctgaatcttactggcacgcgctttcagtttctgtttatcacggattgtatgagacatggcaacacctggttaacaagaatatgaaaaatcatagcactattaatctactggggggtagtatcaggtactgggggggagtagaatcagattgccgaattaatactaagaattattatcatgaccgaatttacaactcttcttcagcaaggaaacgcctggttcttcatccccagcgccatcttacttggtgcgcttcatggcctggaaccagggcactcaaaaacgatgatggcggcgtttatcatcgccatcaaaggcaccattaaacaagcggtgatgctcggactggcagcaactatttcgcataccgcagtggtctggttaattgcctttggcgggatggtgatcagcaagcgctttactgctcaatcagcagaaccgtggctccagctgatttccgcagtgatcattattagcaccgcgttctggatgttctggcgtacctggcgcggcgaacgcaactggctggagaatatgcacgggcatgattatgagcatcatcatcacgatcacgaacatcaccacgaccatggacatcatcaccatcacgaacatggcgagtatcaggatgcccatgcacgagcccatgccaatgacattaaacgacgctttgatggtagagaggtcaccaactggcaaattttgttatttggcttaaccggtggccttatcccctgcccggcagcaattaccgtgctgttgatatgcattcagttgaaagccctgacactgggcgcaacactggtcgtcagtttcagcattggcctggcgttaacgcttgtcaccgtaggcgttggcgcagcaatcagcgttcagcaggtcgcaaaacgctggagcggatttaacactctcgctaaacgcgccccctatttttccagtctgttgattggcttagtcggtgtgtatatgggcgtacatggcttcatgggcataatgcgataactcaatcctttaggcttgcatgttatcttcagcccaggatgattcttaaatcagctatttccgctgactctctgctcgctaaggatgcttttagggcatcctttcatttacactttttacgaaatcatgggatcactaacaaaatatcgcttgtcagttatattgtatggcaggaaagatatgcgactgatattacagatccccaaagtggagagtttatgaccattaaaaataagatgttgctgggtgcgcttttgctggttaccagtgccgcctgggccgcaccagccaccgcgggttcgaccaatacctcgggaatttctaagtatgagttaagtagtttcattgctgactttaagcatttcaaaccaggggacaccgtaccagaaatgtaccgtaccgatgagtacaacattaagcagtggcagttgcgtaacctgcccgcgcctgatgccgggacgcactggacctatatgggtggcgcgtacgtgttgatcagcgacaccgacggtaaaatcattaaagcctacgacggtgagattttttatcatcgctaaaaaaagccccctcatcatgagggggaaatgcagacaccttgttattttttattattagccacttgctcgtcttgcttgttattagtcgtatttcacgttgattaatgcggttgcctccagtgcgccagatttaactttgtttgtatcgtagacgtagtaactggctgttatcggaattgaaaccgttgtatctgtaagttttgacttcgccgcaacttcctttaaatttgtatatcctttactgctgttagtgatatttaaaagtgtgactggcgaaccattactttcaagaataaatcctacgccattatcttccgcacctttcagtattgtgttgctgttggttaacaagtcagaacttgataaatacacctgcattttccgtgatgtttgattttgttgacctaataaatttttacaacgcagaataatatccccttgtttactatttattgttgctttgttacctgtggctggtaattgtgaaacgggaatactgtctaaagtaattaataaatcgtccggtttgcaggttgtggttatcgggttgtatgacaatgtcagattaaaggaatagacacctgcattttgtgccaatgcatttctgtagctatttacacatgcatcccatgacttgccacctaataaacacagtagaaattgtactgcggcactcccgcgtgtcgatgatgaagcactggataatgtcgcaacaccattaatcatcactgaaccgccgccccccgcagaaacattcacttttgcattactggccgcaggtgtcaccgtaactgaataaccactggtgaaactggtctgattatttgacaacgtgatgttgtttttattggtccattcaaaatgtaaatttaattttatggtatcgttataaagtccaacaataatatccgacgggctcataggggtgatagtatttgtacttacgcatgacgaatcattaaaattatgctcatatgtcgccatttgtgtttgagtaagtgcaaaatccccctgaacaaccaagttgtgctgaacagataactcactataacatgccgcatagctcacaggcataaccatcatcattaatataaatagcattatgcgaatttccatagaaccacctgactattactggcaaatataatttctactttcatcaatctctttaccgaaggtgattgtgcatgaaagtccttgttgcttatcaattgccacattaaccgatggcggtacttcattggtgcgaataaataactgacttccctggccgacaacgccaatattatgaccatggatatcattgacttcataaccaaacgttaatgattgcccatctgctcttaacgcttttataaaccatggcttgcgctgatcggtatcaaaattaaccagtacaaccgcgccgcgataaggggcggcaattttccggttgccacgtaattctgcttcgctatcgctttgcgacacatccagcatcaggtgattttcccgataaggtgtcattccgtcgtatatcaccactccattacggtttgttgtgcgatatttttgcccattgacataagcatctttaattcctggcgcattcatcacagcaaacgtttcggaaagacggttcgccagattaacgccacccgaccaggcgacaatgccccctgaaacactggctccagcctgtcgataagtactcgactgactataactgccattcactgtcgcaaccggcgcgttccaggtcaaattcgccccagctgtcgtttcatttccctgatgttgatgactcaggttgacaccataattgaactgatcccgactccctactgttcctgataatcccgtattatttgaggcaaacccctgatcatcaaacgtcgttgagttagacatatatatttgccgacgaggcgtcgaaacgtcatcaccccaatcaaagggaatcgatataaaaatattaaaacgtttctcttcatgatgattctcgtcataagcctggcttgccgcgagggtatagcttatccgtcgcaggttgttggaataactcaactgataatccttactactgccgctacgcccccagtaatctcgccataacgtacttaatgacacagacccccaaccttctggcaatgactggctcatattggcggaaaagctatttttgcggccaaaatcgttctggtaataatcggcaatgtcatagacatcgttttcatcacggcgataattatctttattgtttgcccaaacgtgatcgttaaatgtccggtaatcacgcgacgaataacgccaggccgccagaccaaaacgcgtcgacgtttggctcacaaatttgttgtaggcaatttgataactttgcccgtcaaacacatcgccgttgtcttgtttactatgcgacttagtggcatcgacggaaatggcaccaatgcgtgtattccagccagcccccaaagtaaacgcgtaataattattcgcgaccatcgagccaccatacagcgtcaataaattattaaaaccatactgataacccgcctggacaaaatcactttgtttgctcgccccttcaatatggctacgacccgccgctaaatcatatttcgacacgccgggttgcagcatatttggcaccgctgcataaggcaccagataggtggttaccgagccgtccgcctctttcacgctgacatcaagatctgctccaccaccggccaactgcaaatctgtaatcgcgaacgggccaggaggaacctctttctgataaaccacaaaaccattctgttcaatagttaccagcgcgttactctgagcaatcccctgcacccgtggcgtaaaattttgtttcgagttaggcaacatctgcatatcacgaaacaaccgcacacctctgaagcgaacagaatcaaaaatatcgcttgatgtgtacatatcacccacgcgaagcgtgccgagaagttgggcaaatccacgttccagatacagggtattgcttttccacacccctggattgttatttgttttactgaaactggcatcagaatgcagttgccaccccagtaaatttaacccgctgttaaaacgtacatatgtactcttgttattacccgacgctttatagtcgctgtaatactgactcagataataagaggtataaaacgcattaataccccgctcccagttttccggtggaacatagccactttccagttcttccacccaggcctgcgggacactgaaatcgagacgaaaaaccccgatatcccaggtatagctcccaccctgaacaagttgctcaaatgttaaacattgcttaccgctggcgaagttatcgctattaatgcctaaccgcttgataacttctcttgataaacatgtttcttgcgggttgtctttaacaataatctcatatttcccgcgccattgcttattgacataaatatcgatgtcatactgccccggtaagggttgattatcatcaagacgaatatttgcaacctgctggtctttcattccacctatcataaaatgggtatcaaaggtttcttcagctgcataagcttcaatgccgagcaataacgctacgattgctgatgcaagtggggtcattctcaacataggcagctcctgcaattaaattttgtcactaatatagttgccatggtcatcgataatggtcagatgccagttatttgcattattacttttgacattaacactctgactttctaagggggcaatcataatagtttcataattgactttgacattattagctttgacatccgaaatcgtcacccaattagctgagtcattttttatcaccaaaccattgccactgcgatttaccagcaattttttaaatgtcgctttatttaccggagcaatacccgctggccggtaaaacaacttaattctgttttgcatcgcaaacttcagtgcattcttaccttcttgctctggactatttggtggaatatccagaacattcagataaaaaatgctttctttattagtgggcagtttattcggcataattttgatttttacttgctgcccggaatttgcccctatttttgccactggtggcgttaacatgaaaggaacctgaattttttctggtggtaatgacgtatcgccatcatcaatccacgcctgcagcagcgaagaacggtttccctggttcatcaactgcaccatcacttctttattttctgccgggtaaataatgcgcgtcccgtagataacaattccggcatgtgcaggaaggaccatagaaaaaatgagtaaagataataatcctttcattttaatgcctcttaaattaaaaggccgccatgggatagcggccatgtttattacctggagaaacttacaattttatttattaatcctgcgccacacgcataaccagagaagataacacatcacctgattgcactgagttatctgtcagtttcaggtattttgctttaaacggaatagcatattgaccttccgctgttttataactctcaatgttaaaaggtgcagaaacatccaggacatcgctgttatcacctaaatagagatagtaacccacggtatcgttgctactggctatcgccttatcgttaccggttattttatcgttggtaatcaacgagagttttacaccagcaacttctttcgggcagctaatttttaacatgctgctggttacaccgactgcatcatcataggtagaatatttagctttaccttcaaagacactggttggtacagtcggcatattaatacttactgaatcaccacccgcttcgaatttacacggagattctgcaatattccccttaatagttaatgttccggtatcaacgtctgcagcaaatactccagcgctcataaaaaaagaagaaaagacagcggcagcaataattgaacgtttcataatatgttccttaataaaatttatttttggttgttaagagtctgtatctcttggaaacaaatttctcacatcaaaaaagttgccgcaatgtaaacacattgttttattgatttaaaacaaattaaccattgcaatataaatacaaaaaatatttaagagtattaactatttatcgcatctatcaattaatgtagatttatgtaaatggtattgttgatatcaataaaaaagccgaaatcatttatataaatgatttcggctttctaaatgcaattaaaatcaggttgccaaattaatcgtagcgatttaacacgattcgacgtttgctatcgctacctgcaacaaccacttctgtcgttacacctttgacgggcgaagaaaacagatgacgggtgtcaacattatacgttaactgaccacaatgctgttgaggttgaccattaaccatagccatactgcatgttgggggactgatcctgccattaatcgctaatgtggcagtctctgaagagaatgcgggagaagccaatccataggcaagaaaaataattcctgacagccaatacttattcattgaacgttatccctgtagtaaaggttatgcctggatagaatgagtgcataacaaactatagctgtacatccactacacagccacgaaggatgataatgaagcattgcctgtatgatcaatcgactttgtagagtttcggacgaaggtccgcagaatattcgcagtattaaataagtgttcattaatgcggcaaaaactaatacaccgcatcaatgtaacatctctgcggtgtatgaagaataaccagaatggttaataggcgttagaccgcgcggaaggaaatctcgcctggaatgacttcaccctgccagtagagctgagctgcaacgcggtcagccagctggcggtagatagcggtaaattcgctctccggacggctgataaccgttggcgtacctttatcgagatcctcacgtaaggagatgtgtaacggcatctgccccagcagctgtgtatggtatttttcagccagtttctctgcaccaccggtaccgaaaatcggttcatggtgaccacagttactgcaaatatgcacactcatgttctcgacaataccgagcaccggaacctcgactttctcgaacatcacaatgccttttttcgcatcgatcagcgcgatgtcctgcggggtggtgaccacgactgcaccggttactggaatgttttgcgccagcgtcaattgaatgtcaccggtgcctggcggcatatcaagcaccagatagtcgagatccggccacaaggtttcctgcaacatctgcattaacgccttgctcgccatcggtccacgccacaccatcgcattgtcgtcagtgaccagataaccaattgaattggttgccaggccatgagacataatcggtgccatatgggtaccgtccggcgaagttggacgctgattttctgcgcccaacattgttgggattgatgggccgtagatatcggcgtccagaatgccgactttcgccccttctgccgccagcgccagtgccaggtttaccgccgtggacgatttacccacgccgcctttaccggaactcaccgcgataatgttcttcacaccgttaattcccggctgattcttcacgcgtttcagagtggctatgttatgcgacagtttccagtcgatagctttcgccccggtgatgcgcagcagttcggcgctacattgctcttttaactcttcgaacgcgctatgccagacaaacggcataaccagttccacatgcaacgtgtcgtccatccaggcgacatggtgcaacgctttcagcgtggtgaggttatgcttcagggttgggtgctgaaaattggccagtgtcccggcgaccattgcgcgcaaggcttctggtgatttggcctgggattgttcgttcatcccgactccttttttgtatagataaaccatcagctgatagtttacctgaagaatatagagaagtacttacttaacattttcccatttggtactatctaaccccttttcactattaagaagtaatgcctactatgactcaagtcgcgaagaaaattctggtgacgtgcgcactgccgtacgctaacggctcaatccacctcggccatatgctggagcacatccaggctgatgtctgggtccgttaccagcgaatgcgcggccacgaggtcaacttcatctgcgccgacgatgcccacggtacaccgatcatgctgaaagctcagcagcttggtatcaccccggagcagatgattggcgaaatgagtcaggagcatcagactgatttcgcaggctttaacatcagctatgacaactatcactcgacgcacagcgaagagaaccgccagttgtcagaacttatctactctcgcctgaaagaaaacggttttattaaaaaccgcaccatctctcagctgtacgatccggaaaaaggcatgttcctgccggaccgttttgtgaaaggcacctgcccgaaatgtaaatccccggatcaatacggcgataactgcgaagtctgcggcgcgacctacagcccgactgaactgatcgagccgaaatcggtggtttctggcgctacgccggtaatgcgtgattctgaacacttcttctttgatctgccctctttcagcgaaatgttgcaggcatggacccgcagcggtgcgttgcaggagcaggtggcaaataaaatgcaggagtggtttgaatctggcctgcaacagtgggatatctcccgcgacgccccttacttcggttttgaaattccgaacgcgccgggcaaatatttctacgtctggctggacgcaccgattggctacatgggttctttcaagaatctgtgcgacaagcgcggcgacagcgtaagcttcgatgaatactggaagaaagactccaccgccgagctgtaccacttcatcggtaaagatattgtttacttccacagcctgttctggcctgccatgctggaaggcagcaacttccgcaagccgtccaacctgtttgttcatggctatgtgacggtgaacggcgcaaagatgtccaagtctcgcggcacctttattaaagccagcacctggctgaatcattttgacgcagacagcctgcgttactactacactgcgaaactctcttcgcgcattgatgatatcgatctcaacctggaagatttcgttcagcgtgtgaatgccgatatcgttaacaaagtggttaacctggcctcccgtaatgcgggctttatcaacaagcgttttgacggcgtgctggcaagcgaactggctgacccgcagttgtacaaaaccttcactgatgccgctgaagtgattggtgaagcgtgggaaagccgtgaatttggtaaagccgtgcgcgaaatcatggcgctggctgatctggctaaccgctatgtcgatgaacaggctccgtgggtggtggcgaaacaggaaggccgcgatgccgacctgcaggcaatttgctcaatgggcatcaacctgttccgcgtgctgatgacttacctgaagccggtactgccgaaactgaccgagcgtgcagaagcattcctcaatacggaactgacctgggatggtatccagcaaccgctgctgggccacaaagtgaatccgttcaaggcgctgtataaccgcatcgatatgaggcaggttgaagcactggtggaagcctctaaagaagaagtaaaagccgctgccgcgccggtaactggcccgctggcagatgatccgattcaggaaaccatcacctttgacgacttcgctaaagttgacctgcgcgtggcgctgattgaaaacgcagagtttgttgaaggttctgacaaactgctgcgcctgacgctggatctcggcggtgaaaaacgcaatgtcttctccggtattcgttctgcttacccggatccgcaggcactgattggtcgtcacaccattatggtggctaacctggcaccacgtaaaatgcgcttcggtatctctgaaggcatggtgatggctgccggtcctggcgggaaagatattttcctgctaagcccggatgccggtgctaaaccgggtcatcaggtgaaataatcccccttcaaggcgctgcatcgacagcgccttttctttataaattcctaaagttgttttcttgcgattttgtctctctctaacccgcataaatactggtagcatctgcattcaactggataaaattacagggatgcagaatgagacactttatctatcaggacgaaaaatcacataaattcagggcagttgagcaacagggaaacgagttgcatatcagttggggaaaagttggcaccaaagggcaaagccagataaaaagtttttcagatgctgcggcagcggcaaaagcggagcttaagctgattgcggagaaggtgaagaaggggtatgtggagcaagcgaaggataattctttgcaaccttcccaaacggtaacgggctctctcaaggtagcggacttatccaccattattcaggaacaaccctctttcgtagcagaaacccgtgcgcctgacaaaaatacagatgctgttttaccgtggctggcgaaagatattgctgtcgtttttccgcccgaagttgtacacaccacgttaagtcatcgccgctttcccggagttcctgttcagcaagcagacaaattgccccaattacgtcgcttagcctgtagtgtgtcgcaacgggataataaaacagccacatttgacttcagcgcctgttctttagaatggcaaaacaccgtcgcccaggcgatcagtcagatcgacggcctgaaaacaacacagttaccatcaccagtaatggctgtactcacggcacttgaaatgaaatgcacaagatataaagtgcgtgaggatgttatggatcagatcgtccaggaaggcggtctggaatatgctactgatgtaataatacaccttcaacagattgatattgaatgggattatgcgaataatgtcattattattctgccgtctggcattgcacctagctacttggagcaatattccagatttgaatgacgcctacgtaaacatttatcactgacggaagagtctctctggcaaaaatgtgcacaaaaacttattgccgcaattccacatattccagaatggcggcaaccattaattgctttgttattacccgaaaaaccagaaattgcacatgaaattgcccagcgtctactggggcaaaaaaaattaccctcgcttgagtggttaaaaatagtggcgactgatgagcacattcttgcctcattagaaaaatatcacgaaccatatgccatttttgatgattactattgtggtgcgatatggtcagccaccgtattacaggagcaaggtgttgcagccctgccccgatttgctccctatgccgcaagtgactactgcgccgatgtgttgcgtcatatcaatcatccgttcgcattgacactgcttatacgtgtagccgggcaaactaaacgctgtcacgatcggatgacgaaagccattgctgcgttcccacatgcagcaatggcggcactgacggaacttcttgggcaaaaagaagagaacagttggcgcattatgctaatgacaatgcttatctcacaaccagcactggcagaacaggtcattccctggctctcgacacccgcagttgccgtactgaaatcatgccagcaacaactgacacagccctcaaaccatgccagcgccgatctactgccagccgtagtagtctcccctccctggctttcgaaaaagaaaaaatcgccgattccggtgctggatttagcgccattaggcattgagccaatctgttatctgacagaagaaatcagtaatcaacttttggcgaaatatatctggtattcaaaacacatcacggttagccatgaagaaagtactaccaacctgttggcaaggatgggttttcaacgacggatcgctggtacatatattaaagctcccgaagcggtagttgaggcatggctaaatgaagattattcaaccttactaagtgaatttaaggtgtttcattcacctaccgggcattattggcagttggggattttgacaacattgccgctggagaaagcagtaaaagcatggaatgcccttaccctatctccacataccgataccgaatactccatgttacattttggactcaaagggttacctgggttagtaaactcacttgcacgctatccacaagaagccttgcccatcacgaattacttcgcagcgagtgagctggctcctgccgtcgcccgtgccttcaacaaactgaaaacgctacgcgaaaacgcccgtagctggctgttgaaatacccggaacatgcccttaccggcctgctgcctgcggcgctcggcaaagccggtgaagcacaggataacgcccgcgctgccttgcgtatgcttaccgaaaacggtcatcagccattactgcaagaaatcgcccgacgttataaccagccggaagtaaccgatgcggtgaacgctctgcttgcgctcgatcccttagataatcacccgacaaaaatccccactcttccggccttttatcagccatcgctctggacgcgcccggtattaaaagcaaatgcccaatcactgccagatagcgccctcctccacctcggtgaaatgctccgcttccctcaggaagaggctctgtatccgggattattgcaggtgaaagacgtctgttccgccgactcactggcgggatttgcctgggatctgtttaccgcctggcagaccgctggcgcgccgtcgaaagagagttgggcgttcactgcgttaggcgttctcggtaacgatgacaccgcccgcaaactgacgccattaatacgcgcctggcctggtgaatcccagcataaacgcgccaccgttgggttggatattctcgctgctatcggtagtgatatcgcccttatgcagcttaacggcatcgcccagaaactgaaattcaaagcattacaggagcgggcaaaagaaaaaattgccgacattgccgagagccgcgaactcacggtggcggagcttgaagatcgggttagcaccggatctcggtctggatgataacggttcgctgctgctggattttggcccacggcagttcaccgtcagctttgatgaaaccttaaaaccgtttgtgcgtgatgtttccggcagccgcctgaaagacctgcccaaaccgaacaaaagcgatgatgaaacgcgggcgaacgatgcggttaaccgctacaaattgctgaaaaaagatgcgcgtaccatcgccgcccagcaggtagcaaggctggaatccgccatgtgcctgcgccgccgctggtcgctggaaaacttccagctcttcctggttgagcatccgctggttcgtcacttaacccgccgtctgatttggggcgtttatagcgccgaaaaccagctactggcttgctttcgcgtagcagaagataacagctccagcaccgctgacgatgatcttttcaccctgccggaaggcgatatctctatcggcactcctcacgttctggaaatatcaccaacggatgctgccgcctttggtcagctttttgccgactacgaactgctaccaccgttccgccagctcgaccgtaacagctacgccctgacagaagccgagcgcaatgccagtgaactgacccgctgggcaggcagaaaatgcccgagtggtcgggtcatggggctggcgaataaaggctggataaagggcgaaccacaggatggaggctggatcggatggatgatcaaacctttgggtcgctggtcgttaatcatggaaatcgatgaaggctttgcggtaggcatgtcgccagccgaactcagcgctgagcagctcttaagcaagctgtggctatgggaaggcaaagcagaaagatatggctgggggagtaattcaacacaggaagcgcagttctccgtaatcgatgccatcaccgccagcgagctaattaacgatattgaagccctgtttgaataaggaaagagcatggacaaggaattaccgtggctggcggataacgcccaactggaactgaaatataaaaaaggcaaaacgccgctcagtcatcgtcgctggccgggcgaaccagtgtccgttatcactggaagtctcatccagacattgggtgatgaattgctacaaaaagctgagaagaaaaaaaacattgtctggcgttatgagaatttttcactggagtggcagtccgccatcacgcaggccatcaacttgatcggcgaacacaaaccctcaatcccggcccggacaatggcggcgctagcctgtatcgcgcaaaatgacagccaacagttgctcgacgaaatcgtccaacaagaggggctggaatatgcgactgaggtggtgattgcacgccagtttattgcgcggtgttatgagagtgatcctctggtagtgacattgcagtatcaggacgaggattatggctatggttatcgctcagaaacctataacgaattcgatctccgactgcgtaagcatctctctctggcagaggaaagctgctggcagcgttgcgccgacaaactcattgccgcactaccaggaataaacaaagttcgccgcccttttattgcgctgatcctcccggaaaaaccagaaatagccaatgagttggtaggccttgaatgcccgcgaactcattttcattctaaggagtggttaaaagttgttgctaatgaccccacagcggtgagaaaactcgaacactactggagccaggatatatttagcgatcgagaagccagctacatgtcgcatgaaaaccacttcggctacgcggcctgcgccgcccttttgcgcgaacaaggactggcagccattccgcgcctcgcgatgtatgcccataaagaagattgcggcagtctgctggtacaaattaaccatccgcaagtcatccgcaccttgctactggtggctgataaaaacaaacccagcctgcaacgtgtagctaaataccataaaaacttcccccatgcgacgctcgccgcactggcagaactgctggcgttaacagaaccaccagcccgccctggttatccaatcatcgaagacaaaaagctgcctgcacagcaaaaagcacgcgatgaatactggcgtacgctgttacaaacgctgatggcatcgcagccacaactggcagcagaagtgatgccgtggttaagtactcaaccccagtcagtgctgaagagttatttatcggcaccgcccaaaccggttattgatggcaccgataacagcaatctgccagaaatcctcgtttcaccaccgtggcgtagtaagaaaaaaatgacagctccacgtcttgatttggcaccgctcgaattaactccgcaagtttactggcaaccaggcgaacaagagaggcttgccgccactgagcctgcccgttatttcagcacggaatctcttgcgcaacgcatggaacaaaaaagtggacgagttgtattacaggaactgggttttggggatgatgtatggctgtttctgaattatatactccccggaaaactggatgctgcacgcaattcactctttgttcagtggcattactaccaggggcgggttgaagagatcctgaatggctggaactccccggaagcacaattagcagaacaggcgctccgcagcggtcacatagaagcgttaattaacatatgggaaaatgacaactactcacattatcgtccggaaaagagtgtctggaacctgtatttattggcacagttgccgcgtgagatggctttgaccttctggctgcgtatcaatgagaaaaagcatctgttcgcgggtgaggactattttctcagtatcctcggattggatgcgctaccaggtctgctgttggctttttcacatcgtccaaaagaaacatttccgttaattttaaattttggcgcaacagaactggcgctgcctgttgcccacgtctggcgacgtttcgcggcgcagcgtgatctggctcgccagtggattttacaatggccggaacatacggctagtgcacttatccctcttgtctttaccaaacccagcgataatagcgaagccgcattacttgccctgcgtttactgtacgaacagggacatggcgaattgctacaaaccgtggcaaaccgctggcagcgtacagatgtatggtctgccctggagcagttgcttaaacagggtccaatggacatttacccggcacgcattccaaaagcccctgatttctggcatccgcaaatgtggtccaggccgcgccttatcactaataatcaaactgttaccaatgacgctctggaaattatcggcgaaatgctgcgctttacccaggggggacgtttttatagcgggctggaacaactgaaaacgttctgccagccacaaacgctggcagcttttgcctgggatctcttcactgcgtggcaacaagctggtgcccccgcaaaagacaactgggcatttctggcgttaagtctctttggtgacgaaagcacggcacgggatctgacgacacagatcctcgcctggccacaagaaggcaaatctgcccgtgctgtcagcggcctgaacatccttaccctgatgaataatgatatggcgctgatacagctgcatcatatatcgcaacgggctaaatcccgccccttacgtgataacgcggcggaatttcttcaggtggtcgcagaaaatcgcgggctaagccaggaagagctagcggacagattagtcccaaccctgggccttgatgatccgcaggcgttgagttttgattttggtccccggcagtttaccgttcgcttcgatgaaaatctcaacccggttatctttgatcagcaaaacgttcgccagaaaagcgttccccgtttgcgcgccgatgacgatcaactgaaagcgcccgaggcactggcccgactaaaagggctaaaaaaagatgctactcaggtgagcaaaaacctgctcccgcgtcttgaaacggccctacgtaccacccgacgctggtcgctggcagattttcattctctgtttgttaatcatccctttacccgtctggttacccagcgattaatatggggggtttatccggcaaatgaaccgcgttgtttactcaaagcctttcgtgtggccgcagagggggagttctgcaatgcgcaagatgagccaattgacctgcctgcggacgctctgattggcattgcccacccgttagaaatgacagcagaaatgcgcagtgaatttgcacagctttttgccgattacgaaattatgccgccttttcgccagttgtcgcgccgcacggtgctgctcacacctgacgagtcaaccagtaacagcctgactcgctgggaaggtaaatccgctaccgttgggcaacttatgggaatgcgatacaaaggctgggagtcaggctatgaggacgcatttgtctataacctgggtgagtaccggctggtccttaagttttcacccggttttaaccactacaatgttgatagcaaagcgctaatgagcttccgttctcttcgagtgtaccgtgacaataaatccgtcacttttgccgaacttgatgtgtttgatttgagtgaggcgttaagcgcacctgacgtcattttccattaaaacacagcgggcagtgatgcaactgcccgttatcaacacgacttaccagcggggaaagcgatgatcgtgcaaaaagagctggttgctatttacgattatgaggtccctgtacctgaagatccgttttccttcagacttgagatccataaatgctctgaattatttacaggttccgtctatcgactggagcgattccggctacgtccaacatttcatcaacgtgatcgagaagatgctgacccgctaataaatgatgcgttgatttatataagagatgagtgtattgatgagcggaaattacgaggtgaatcacctgaaactgtaatagcaatttttaatcgtgaactacagaatatattcaaccaagaaatagaataatatactctaaataattcaaattggtccgatccggcgcaacgtcccaatggcctggattataaatctcattatcttaattgcaacggggtccagccgtggttataattcgttcgttggaacacgatgttgcacaggctgtggtgttaggcctgaaaatagtaaataaaagaacctgcctcaccagcaggtttttttatttactgtgatctgctttccagatatttttcgctcaaacaactaatgcgccaaacatttattgcgcgtaaaatatcgtttatttcattaatacatttcagggatgaatatatgtcaccgcagaataatcatctgcagcgtccgcctgctgctgtgttatacgccgatgaactggcaaaattaaaacaaaatgataacgcaccttgcccgcccggttggcagttaagtttgcctgcggcccgtgcttttatccttggcgacgaagcgcaaaatatcagccgtaaagtggtgattagcccctccgctgtcgaacgtatgttagtcactcttgctaccggccgcggtttgatgttggtgggggaaccgggtaccgcaaaatctcttctttctgaattactggcaaccgctattagcggcgatgccgggttaaccatccagggcggggcatctaccaccgaagatcaaatcaagtatggctggaactacgccctgcttatcaatcatggtccgtcaacggaagcgctggtccctgccccgctttatcagggaatgcgcgacggcaaaatcgtccgtttcgaagagataacgcgtacaccgctggaagtgcaggactgtctgttaggtatgctttctgacagggtgatgacggggccggaactcactggtgaagccagtcagctctatgcgcgagaaggctttaatattattgccactgccaatacccgcgatcgcggcgtcaatgaaatgagtgctgcgctaaagcgtcgcttcgattttgaaacggtttttccgattatggatttcgcccaggagttggaactggtcgccagtgcttcggcgcgtttgctggcccatagcggtattccgcataaagtgcctgacgcggtactggaattactggtccgcaccttccgcgatctgcgtgccaacggcgaaaagaaaacgtcaatggatacactgacagcgattatgtccaccgctgaagccgtgaacgtggcccatgctgtgggcgtccgcgcctggtttttagcgaatcgcgcgggggagcctgccgacctggtggaatgtattgccggaaccatcgtcaaagataacgaagaagatcgcgcgcgtctgcgccgttacttcgaacagcgtgtcgccacacataaagaagctcactggcaggcttattatcaagcccgccaccgcctgccgtgaggaaagatgcatgagcgagccgttaattgtcggcatccggcatcatagtccggcctgcgcccggctggtgaaatcgttaatcgaaagccagcggccacgatacgtgttgattgaaggcccggctgattttaatgaccgggtagacgaactgtttttagcccaccagcttccggtagctatttacagttattgccagtatcaggacggtgcagcccccgggcgtggtgcctggacgccatttgctgaattttcgccggagtggcaggcgctacaagccgcacgtcgcattcaggcacaaacttacttcatcgatttgccttgctgggcgcagagtgaagaagaggacgattcgcctgatacgcaagatgaaagccaggccttactgctgcgtgccacccgcatggataacagcgataccctgtgggatcacttgttcgaagatgaaagccagcaaactgcattaccctctgcgctggcgcactattttgcccaactgcggggcgacgcctccggcgatgcgctcaatcgtcagcgcgaagcctttatggcccgctggattggatgggcgatgcagcaaaataatggcgacgtgttagttgtctgcggtggctggcacgctccggcactggcaaagatgtggcgcgaatgccctcagaaaattaacaagccagaattgccctcgctggcagatgccgttacaggttgttatctcacaccctacagtgaaaagcgccttgatgtgctggcaggatacctttcaggaatgcctgccccggtatggcaaaactggtgctggcagtggggcttgcagaaggccggtgaacaactgctaaaaactatccttacccgtttgcgccagcacaaattgcccgcttctaccgcggatatggctgccgctcatctgcatgcgatggcgctggcacagttgcgcggtcatacactaccgttacgcactgactggctggatgccatagcaggctcgctgattaaagaagccctgaacgcgccgttgccgtggagctatcgcggcgttattcatcccgataccgatccgattctgctaacgttgatagacacattagcgggtgacggattcggtaaacttgccccttctacgccacaaccgcctctgccaaaagatgtcacctgcgaactggaacgtaccgcaatctcccttccggcggagcttaccttaaatcgctttacccccgatgggctggcgcaaagtcaggtgttacatcggctggcaatactggagatccctgggattgtacgccagcagggaagtacactgacacttgcaggcaacggtgaagaacgctggaaattaacccgcccgcttagccagcatgcggcattgattgaggccgcctgttttggtgccacactccaggaagccgcacgcaataaattagaagccgatatgctggacgcgggcggaatcggcagtatcaccacatgtcttagccaggcggcgttagcgggtctggcgtccttcagtcaacaattactggagcaactcacactattaatcgcccaggaaaatcaatttgccgaaatgggccaggcgctggaagtgctttatgccttatggcggctggatgaaattagcggtatgcaaggcgcgcagatattacaaacgacgttatgcgcgactatcgatcgcacgctgtggctgtgtgaatctaacggcagaccggatgaaaaggagtttcacgctcacctgcatagctggcaagcgctttgccatattctgcgcgatctacatagcggcgttaatttacccggcgtttctctttctgcggcggtagccttactggagcgacgcagtcaggcaattcatgccccggcgctggatcgcggcgcggctcttggcgcactaatgcgtctggaacatcccaacgccagtgccgaagcggcgctgacgatgctggcgcagttatccccggcacaatctggtgaggcgctgcacggtttgctggcgctggcccgccatcaactggcctgtcagccggcatttatcgccggtttcagcagtcatttaaatcaactgagtgaagccgattttattaacgccctgcccgatttacgcgcggcgatggcctggctaccaccacgagaacgcgggacgctggcgcatcaggtgcttgagcattatcaactggcgcaacttcccgtttcggcgctgcaaatgccgttgcattgtccaccacaggccattgcacatcatcaacaactcgaacagcaggcactggcatcgctgcaaaactggggagttttccatgtctgaactgaacgatcttctgaccacccgtgagctacaacgctggcgattaattcttggcgaagcggcagaaacgacgctttgtgggctggatgacaacgcccggcagatagaccacgcgctggagtggctgtatgggcgcgatcctgaacggctccagcgtggtgaacgttccggtggattaggtggctcaaatctcaccacccctgagtggatcaacagtattcacacgctgtttccgcagcaggtgattgagcggctggaaagcgatgccgtgctgcgctacggcattgaagatgtggtgacgaatctcgacgtgctggaacgtatgcagccttctgaaagcctgctacgcgctgttttgcacaccaaacatctgatgaaccccgaagtactggctgccgcccgccggatagtgtgccaggttgttgaagaaattatggctcgactggcaaaggaagttcgtcaggctttttctggtgtccgcgatcgccgtcgccgttcatttattccactggcgcgaaactttgatttcaaaagtactctgcgcgccaacctgcaacactggcacccgcaacacggcaagttgtatatcgaatccccccgctttaacagccgcattaaacgccaaagcgaacaatggcaactggtcttactggttgatcaaagcggatcgatggtcgattcggtgatccactctgcggtgatggcggcctgtttgtggcagttacccggcattcgtacccatctggtggcgtttgacacaagcgtcgttgatctcacggcagacgttgccgatccggtagagttattaatgaaagtacagttgggcggcgggaccaatatcgccagtgccgtggagtatggtcggcaacttattgaacaaccagcgaaaagcgtcattatcctcgtgagcgatttttacgaagggggttcatcatcattactgacgcatcaggtgaaaaagtgtgtccagagcggcatcaaagtgctgggactggcagcgctcgatagcaccgcaacaccttgctatgaccgcgatacggcccaggcgctggttaatgtcggcgcacaaatagccgccatgacgccgggcgagctggcatcatggcttgcggagaatcttcagtcatgaattcactacgtccggaattattagaactgacaccgcaggccctgacggcgttaagcaatgccggttttgttaagcgcagtcttaaggaactggaaaatggcaacgtcccggagatcagccatgagaacgacgctttaatcgccaccttcagtgacggtgtccgtacccagctggcgaacggccaggcactgaaagaggctcagtgcagttgcggggccaacggtatgtgccgtcatcgcgtgatgctggtgttaagttatcaacgactttgtgccaccactcagtctacggaaaaagaagaagagtgggatccggcaatctggctggaagaactggctacccttcccgatgctacccgcaaacgcgcacaggcgctggtcgctaaaggcatcaccattgagttgttctgtgcgccgggtgaaattccctctgcccgcttaccgatgagcgatgtgcgtttttattcccgcagcagtattcgtttcgcccgttgtgattgtattgaaggcacactttgcgaacatgtcgtactggcggtacaggccttcgtcgaggccaaagcgcagcaagcagaatttaaccatttaatctggcagatgcgcagcgaacacgtcacatcatctgacgatccgtttgccagcgaagaaggcaacgcgtgtcgtcaatatgttcagcaattaagccagacattatggcttggcggcatcagccagccgctcatccattacgaggcagcattcaaccgcgcattgcaggcggcagagacctgcaactggcgctgggtgagtgaatcgctacggcaactgcgcgccagcgttgatgccttccacgcccgcgccagccactataatgccggagaatgcttacatcagcttgcggcattaaacagtcgattaaattgcgcacaagagatggcccggcgcgacagtattggtgaagttcctcctgtgccgtggcgcacggtcgttggctctggcattgccggagaagcaaagcttgatcatctgcggctggtgtctttaggtatgcgttgctggcaggatattgagcattatggtttacgcatctggtttaccgatcccgacaccggcagtattttgcacctttcgcgcagttggccgcgaagtgaacaggaaaactcaccggcagctacgcgtcggctgtttagttttcaggctggcgcactggcgggcgggcaaattgtttcacaagcagcaaaacgcagtgccgatggcgagctgctgttagctacccgcaaccgcttaagcagcgttgtgccgctgtcgcctgatgcctggcaaatgttgagcgcgccgttacgccagccgggcattgtggctttgcgggaatatttacgccagcgtccccccgcctgcatacggcctcttaatcaggtcgataacttatttattctgccggtcgctgagtgtatttcgctcggttgggacagcagccgccagacgctggatgcgcaggtcattagcggcgaaggggaagataatgtgctgacgttatcattaccagcctcagccagcgcaccttatgccgttgaacgcatggcggcgcttttgcaacaaacagacgaccccgtgtgtctggtttctggctttgtcagttttgttgaagggcaattgacactggaaccacgggtgatgatgacaaaaacccgtgcctgggcgctggacgcagaaactacgcctgtggcaccgctaccttctgccagcgttttgcctgtgccgtctactgctcatcagttgctgatacgctgccaggcgttacttattcaactgctccataacggctggcgctatcaggaacagagtgctattggtcaggcatagttgctggcgaatgacctcaccgcggtgggtttttatcggctggcacatgtgttgggacaatttcgtaatacagaaagcgaggcacgggtagaagcaatgaataacggtgttttgctttgcgaacaattattccccatgcttcagcaacaaggatgaaatagtgctttttactaagagttctactccagttccggactgctcacgccacggtattaggcatatcctatatagcccctggtgagagtcaccagttccttgattaaataaaatggagttttacatgaaggctttcaataagctgttttccctcgttgttgcatctgttctggttttctctcttgctggctgcggtgacaaagaagaatcgaagaaattcagcgccaatctgaacggcactgaaattgccattacctatgtctacaaaggtgacaaggtgcttaagcaatcttctgaaaccaaaattcaatttgcctccattggtgcaaccaccaaagaagatgctgccaagacacttgagccgttaagcgccaaatacaaaaacatcgcgggtgttgaagaaaaattaacctataccgatacctacgcgcaggaaaacgtgactatcgatatggaaaaagtggattttaaagccctgcagggtatttcaggaatcaacgtttctgctgaagatgccaaaaaaggtatcactatggcgcaaatggaactggtgatgaaagccgctggttttaaagaagtgaaataatcggttggcggtcatgctctaaacatgaccgccaattttttagccttttttcacatgctggcgcgctgccagtccacgcagaaaataacgtaaaaattgatcgccgcattcgcggaagtttttatgatccggtgcgcgcatcatcgctgtaatttccggcatcgaaacgcggaactgctgttcggtgaggatagccagaatgtcatcggttttcagcgaaaacgcgatgcgtaattttttcagcacgatgttgttattaatgcgacgttccggctccagtgccggagcagactcatccttgccgcgtttttcataaatcaggccattgaggaatgacgacaaaacaatgtccggacaacgctgaaaaccctcttcgtcttctttacgtagccagacggcgatctgttccgcggtggcttcgacattacccagcgccagaatacgcaccaggtcattattattggctttcaaaatgtagcgcacgctgcgcagaatatcgttacttagcatgaggccttcaggtgttgatgaggcaaaaagccattttagcagtcttttacaggccaatcgcctcttttaagcttttcagataacggcggctgaccggcacggttaagccattacgcaaaatcaactcggcctggccgttatcttccagacgaatctcctgtaaatgcgcgaggttaaccagatactgacgatggcagcgcagtagtggtgtacgactttccagggtacgtaatgtcaattcggtaaagccctctttcccttcgtggctggtaacgtagacaccgctcatccgactgctgacaaatgccacatctttcatttgcagcaaataaatccgactatgccccgtacaagggataaatttcagcgcctgttgattttccggtaacagcgaaacatcctgcttgctgcgctcctgacgcaatcgcgccagcgttttctccagtcgcgcttcatcaattggcttcagcagataatcaaaggcatgttcttcaaaggctttaattgcgtattcgtcaaacgcagtgagaaaaacaatatacgggcgatgttccgggtcaagcatccccaccatttccagaccactgatgcgcggcatctggatatcgagaaacagcacatccgggcgcagtttatgcaccgcgccgatcccttccacggcgtttgaacactctccaacgatttcaatatcgctctgctcctgcaaaaatacacgcaggttctcccgtgctaacggttcatcatcgacaattaagactttaatcatgcctcgtccctccatggtagtcgtaacgttattcgggtgtaactatcaggctcacaggcgacgcttattccatagtcatcgccaaaccgttcacgtaaacgcttatccaccagattcatccccagcccactggcattggttaccggttgatacaaaccggcattgtcttcgatctccagcatcaaatgttgcccctcacgtcgggcgctgattgccactcgccctgtatccagcagttgtgatgtcccatgtttaatggcgttttccactatcggttgcagggtaaacgcgggcaattgctgctgggataattcttgcggaatagcaatgttgacctgcaaccgcgactggaagcgcgccttttcaatttgcagataagcattcacatgttcaatttcgtcggcgagagtaacaaactccgaaggccgctttaagtttttgcggaaaaaagtggaaagatactgcaccagctggctggcctgttcgctgtcgcggcggatcaccgctttaatggtgttaagcgcattaaacaaaaaatggggattcacctgggcgtgaagcagtttgatctctgactgggtgagcatcgctttttgccgctcatattgcccggcaaggatctgcgccgaaagcaattgcgcaatcccctcacccaacgtgcggttgattgaactgaataaacggtttttggcttcatacaatttgatggtgcccatcacccgctgattttcaccacgcaacggaattaccagcgtcgaccccagtttgcattgcggatgcaaagagcaacggtaaggtacttcgttgccatcagcgtagaccacttcaccggtttcaatcgcttttaaagtataagttgaagaaatcggtttgccgggtaaatggtggtcgtcaccaattccggtaaaggccagcaatttctctcgatcggtaatcgcgactgcaccaatatccagttcctgatacagcacctgagccactttcatgctgttcacttcgttaaacccctggcgcaaaatgccttccgtcgaggctgccactttcagcgcagtggcagaaaaagccgaagtgtatttttcaaacatcgcgcgtttatcgagcaatatacgcataaacagcgccgcgccgacggtattggtgaccatcattggcgcagcaatattactcaccagacgcaccgcatcttcataaggtcgggcgatcgcaaggatgatcagcatttgcaccatttcagcgacgaacgtgacggcaccggcggtaatggggttaaagactttatcagtgcgcccgcggcggatcaggatgctgtgtaccaggccaccgagtaatccttcaacgatggtcgagatcatgcaacttaacgcggtcatgccccccatcgaatatcgatgtaagccgccggtcagcccaaccagcccaccgacgaccggaccgccgagtaagccgcccattaccgcgcctatcgcacgggtattggcaatagaatcgtcaatgtgcaacccaaaccaggtgcccatgatgcagaagatggaaaagacgatgtagcagagaaatttatgcggcagacgaaccgtgacctgcattaacggtatgaataatggcgttttactcattaaccatgcaatgactaaaaaaacgcacatctgctgaagcagcagcaacaccagattaaaatcgtacatacccgcaaaccacacttccctttaaaacgcgtaacatacattgcctgcgtttaactttctttgaactcttgcagaaaaatgagaattcgtgagtacgatcactcaaaatcgcctggcaaaaataaaatcaccctatagatgcacaaaaaacgggcaaaactacctggttcgcaaaactgcgtctaaagttaaaccgggacctcgcgagcaagggtgagacgatggcgctttacacaattggtgaagtggcgttgctttgtgatattaatcctgtcacgttacgcgcgtggcagaggcgttacggattgctgaaaccgcaacggacagacggcggtcatcggctgttcaacgatgccgatattgaccggatccgcgagatcaaacgctggatcgacaacggcgtgcaggtcagcaaagttaaaatgctgctcagtaatgaaaatgttgatgtgcagaacggctggcgcgatcagcaagaaacattactgacttacctgcaaagcggcaatctacatagcctgcgaacgtggatcaaagagcgcggtcaggattaccccgcccagacactcaccacacatctgtttattcctctgcgccgacggcttcagtgccaacaaccgactctccaggcgctgctggcgatcctcgacggcgtactgatcaactacatcgccatttgtctggcttcggcacgtaaaaaacagggtaaagatgcgctggtggttggctggaatattcaggataccacccgtctgtggctggagggctggattgccagtcaacaaggatggcgcattgatgtcctcgcccactcgctcaatcaactacgccctgaactattcgaaggccgtacattgctggtgtggtgcggtgaaaatcgaacctccgcccaacagcagcaactcaccagttggcaagaacaaggccatgatattttcccactcggcatttaatgattcgttaacaaatgcgctttactgtacaatcctttcgttaacataaggagtgcattatgcgcatagctaaaattggggtcatcgccctgttcctgtttatggcgttaggcggaattggtggcgtcatgctcgcaggttatacctttattttgcgtgctggctaagcgcctgcaccagcctttcaaacaggcggtctgcgatgatcgccgccagtgccaccagtaacgccccctggatcacatacgcggtattaaatccgctaagcccgatgatgatgggcgtacccagcgtgctggcccctaccgttgaggcgatcgtcgccgtaccaatgttgataatcaccgaagttcgcacgcccgccagaatcaccggagccgccagcggtagctcgaccttacgcactcgctgaccacgactcattcccatacctttcgcaacttctgtcacgctggcatcaatcgctcccagcccggcaagtgtcgcctgcaggacgggcagcacaccgtaaaggatcaaggcgataatcgctggttgcagaccaaagccgatcaccggaacggcgatcgccagcactgcgacgggcggaaaagtctgtccaacggcggcaatagtttccaccagtgggcgaaattccgcgccccacgggcgagtgacagcaattccggcaccagtgccaatgatcaccgcaaacaaactcgaaattcccaccagccagaaatgagccagtgccagagctgcaaaactttcttgctgataaacgggtcgtggcagttgtgggaacaaggcagcaaacagcggctggctgtaaggcagccagaaaatcagcgccacaaacagagcaatgagccagaacagcggatcgcgcaacatcttcatacgcttacgcctccaccagcagatcctgaaaatgcagcgtgccgcaaggctggccctgcatgttcaccaccggcagcacctcgcatccccgcgcaacaaacagagagagcgcatcgcgtagcgtcatctcttctgccagtgcctcaccatctgctcgttcttcgcgacgcacgtaatccgccacactacgtaacgaaagcaggcgcacacccagttcactacgtccaaaaaactggcggacaaaatcattcgccggacgagtcagcatcgtcagcggattgccctgctgcactacttcaccgtgatccatcaataccagatgttctgccagccgtagcgcctcatcaatatcatgagtgaccagcacaatggtacgccccagcaaacggtgaatgcgcgtcatctcttgttgcaacgcgccgcgcgttaccgggtccagtgcgccaaaaggttcatccattagtaagacttgcggatcggcagccagtgcacgcgccactcccacacgttgctgctgaccaccggaaagctgatgcggataacgctcacgcaaatttgactccagccccagtagcgccattaattcgtcgatacgatcgtcaatccgcgcccgcgaccatttttgtaattgcggcacggtagcgatgttttgcgccacgctccagtgggggaacaggccaatagattgaatggcatagcccatccggcggcgcaactccagtactggcagcgagcgaatttcttctccggcaaagcggatctctccgctgtcatgctccaccaggcggttaatcattttcagggtggtggatttgccggagccagatgtgccaatcagcaccgaaaaactcccttcctgaaaattgagattgagatcgttaacggctttttgtgcgccgaacagtttgctgacatggctaaattcaatcattacgtttcaccttcagcagtgcgataagcaaatcgaacagcgcgtcggtaagcaccgccagaacaattaccgggatcacccccagcaacactaaatcaatggcgctgcttagcagcccctggaaaaccagcgcaccaaaaccgcctgcgccgattaacgccgcaatcaccgccatacctacagtttgcaccatcaccacccgcaggctgcgcagaaataccggtaacgccagcggtaactgaacatgcaggaaacgctgcgccccgctcatccccatcgctctggcgctttccagcacatcgcgcgggatctggttcaaaccgactaccacgccgcgcaccagcggcagcaaggcatagagcaccagcgcaatcagtgcgggtgtcattccggttcctgctatgccgagcgtccccagccacggaaaggccgtaaccagcgcggcaagcggcgcaatcaacaggccaaagagcgccaccgaaggcacggtctgaatcacattgagcagagaaaaaattgccccctgccgagcagtggaaaagtagcaccagatgcccaacggcacaccaatcactaacgcaggcagcaccgcaccaaacagcaacgtcagatgttgtgccagcgcgtcgtcaaacacatcctgacggttggcgtattctttcattagtgagagatcgttaagcgtgccggagtacagcaaccacagcggaataatggcaatctgcatatgcaacaaccagcgccacagcggatgcgtggagattcggcggatggcatcgctacaggccagcaatgccagcgccgcagccagccagaaaccactgccgaggctggtacgcgccagcgcactgccattttgcgccagttgggtcgccgcctttccagctccccacaccagcaatacgaagacgaattgcgccagaatgagtgcacaaatgctgccttttttaccgggaataaaacaggccgtcagccaggcgcaaccaacgcccaccagcatccagatcgtttgcggccacagctgccagagatgacgcccctcacccgaaactaaacgattaggcgcgtaactgataaacggcagcgccgctgcgattgccgtcagcaacagcagcagcgccagaacaggattaatacggaaataagtcacgggaaattacttcgtccaccctttttgtttcaggtagtcggcagccacttttttggcatccagtccttccacagcaatgctggcattcagttgctgcaatgtttttgcatcgaggctggcgaagactggctgtagccactgtgccatttgcggatactccctcaacaccgactcacgcaccactggtgcaggcgcgtagataggttgcacaccttgcggatcgcttaaggtttgcagccccagcgccgctaccgggccgtcagtgccgtaagccattgcagcattaacgccagaggtttgctgggcagcggctttgatcgtcaccgccgtgtcgccaccagccagtgacagcaactgatcctgaccgagcttaaagccataggctttttcaaacgcgggtaacgcatcggcgcgttcgataaactctgccgaggctgccagtttgaaggtgccgccctcttgcagataacgactcaggtcggcaagcgaagtgagtttatttttctctgccacatcctgacgcacggcgatagtccaggtgttatttgcaggcgcgggcgtcagccagattaacttgttgtgctccgaatcgagctttttgactttctcgtaaccttgctgcgcgtttttccacgctgcatcgttttcatctttaaagaagaaagcgccattgccggtatattccggatagatatccagttcaccggaagtaatcgccccgcgcaccacaggagtcgttccgagttgcactttattcaccgtcggtacgccgtggctttccagcacctgcaaaatgatattgccgagtagcgcaccttcggtatcgatttttgaaccgactttaacgggggaagccgcctgtagcggcaggctcacggctgccaacataaccagtgaacctgcccagagctttaagagtggcatgatgctttcctcattcttttactgttgttttcagcgaattaagagaaaagcatagttgataatggcggggttagcttgagcggaaggattcagttgcagaatcagataaatacttaagaggcatattcggtccggcgtttcctgccggatgcggcgcgagcgccttatccggcctacaaagggcgcaaacgtcgcgcccttactaaagcattacagcaactcaaactcgcctttcttaacgcgtgcggaatcagtgccgataaagacattgaacttgccaggctcggcgtcatatttcatctgttgattccagaacttcagcgcctcaatatcgatcgggaagctgacagtctgagtttcgcccggtttcagggtgattttctcaaagcctttcagctgtttcacagggcgactcatggaagccgtcacatcctgcaagtacatctgcactaccgtggcaccctcgcgcttaccggtgttcgtcacctgcacgctggcagtcactttgccgtcacgcttcatggtcggcgcagaaagtttcacatcagagacggtgaaagtggtgtagctcagcccatagccgaacggatacaacgccccgttagcttcatcaaaataacgcgaagtgtatttgttcggcttgtcggcattatacgggcgaccggtattcagatggctgtagtacaccgggatctgcccgacagaacgcgggaaggacattggcagcttgccggacgggttgtaatcgccaaacaatacatcggcaattgcattaccgccttcagtccccgcaaaccaggtttccagaatcgcatcagcctgctgatcttctttcaccagcgccagcggacgcccgttcatcagcaccagcaccagcggtttaccggtggctttcagcgccgcaatcaagtcacgttggctttgcggaatagtgatatcggtccggctggaggcttcgtgcgccatcccctgtgcttcaccgactacagccaccaccacatcagattgtttcgccgtctgcaccgcttcatcaatcatctcttgcggcgaacgcggatcgactttgaccgcttcttcatactgattcaggaaatcgataatgcctttgtcactggtaacgttcgcccctttggcatacagcactttaccgttttcaccgacggcatttttaatcccggtcagtacggtcacggattgatcggcaacaccggctgcggaccagctgcccatcacgtcacgtttactgtccgccagtggcccaaccaccgcaatggtggccgattttttcagcggtaacgtttcgagacggtttttcagcaacaccaagctttcgcgcgccacttcacgcgcttctttacggtgcaggcggctttcggcattggtatccaccgggtcagactctttcggccccaaatggctgtatgggtcgttaaacaaccccatatcatatttaacgttcagtacatggcgggcagcatcgtccagctctgccatcgtcactttgccggatttaatcaacccaggcagatacttcgagtagtactcgtcgctcatgctcatgttgattccggatttcagcgccacgcgcaccgcatcttccgggtctgccgccgtgccatgtttaatcagctctttgattgcaccgtgatcggaaacggtgatgcctttaaagccccactggtcgcgcagaacatctttcagcagccaggaatcggaggtggctggcgtgccgttcagcgagttcagcgccaccatcaccgcgccgctgcctgcgtccagccccgctttgtacggcggcatataatcattaaacaggcgctgcggactcatatcgacggtgttgtactctttaccgccttctaccgcgccgtatgcggcaaagtgtttgacgctggtcatcaccgagtagcgatctgccgggcttttaccctgcatcgcttccaccatggttttacccattgttgaggtgagatacgtatcttcgccaaaaccttcggaagcacgtccccagcgcggatcgcgcgagacatcgaccatcggtgcccaggtcatattcaggccatcatctgccgcttcataagcagagacacgtccgaccgttttcactgcatcgaggttaaaagacgaggccagaccgaggctaatcgggaacaccgtgcgctgaccgtgcagcacgtcgtaagcaaagaaaagaggaattttcaggcggcttaattccatcacctgatcctgcatggcgcggatatcctgacgggttacggtgttgaaaatcgccccaacctgaccgtctttgatcatctcgcggatcgcctctttcgggttatccgggccgacgctgattaagcgcagctgaccaattttctcatcaactgtcattttcttaagcagttcggtgacgaacgcatcccgcgcttcgggcgttaatggatggttgccgaataaatcatccgccagtgctggctgcagggccagactcaccgcgattcctactgaacatagccatttcatatggatttttcttcctttgttgcccgacgtggcagcgaaaatggtgcaaaaaccgtagtttgccataagcatgatggagagagaaaaagaatgctcagtttattgtctgaattttcaaaatattcactcgctgaattgttatacaaggcgctattctagtttgtgatattttttcgccaccacaaggagtggaaaatgtcttccatgacaacaactgataataaagcctttttgaatgaacttgctcgtctggtgggttcttcacacctgctcaccgatcccgcaaaaacggcccgctatcgcaagggcttccgttctggtcagggcgacgcgctggctgtcgttttccctggctcactactagaattgtggcgggtgctgaaagcctgcgtcaccgccgacaaaattattctgatgcaggccgccaatacaggcctgaccgaaggatcgacgccaaacggtaacgattatgatcgcgatgtcgttatcatcagcaccctgcgtctcgacaagctgcacgttcttggcaagggcgaacaggtgctggcctatccgggcaccacgctctattcgctggaaaaagccctcaaaccgctgggacgcgaaccgcactcagtgattggatcatcgtgtataggcgcatcggtcatcggcggtatttgtaacaactccggcggctcgctggtgcaacgtggcccggcgtataccgaaatgtcgttattcgcgcgtataaatgaagacggcaaactgacgctggtgaaccatctggggattgatctgggcgaaacgccggagcagatccttagcaagctggatgatgatcgcatcaaagatgacgatgtgcgtcacgatggtcgtcacgcccacgattatgactatgtccaccgcgttcgtgatattgaagccgacacgcccgcacgttataacgccgatcctgatcggttatttgaatcttctggttgcgccgggaagctggcggtctttgcagtacgtcttgataccttcgaagcggaaaaaaatcagcaggtgttttatatcggcaccaaccagccggaagtgctgaccgaaatccgccgtcatattctggctaacttcgaaaatctgccggttgccggggaatatatgcaccgggatatctacgatattgcggaaaaatacggcaaagacaccttcctgatgattgataagttaggcaccgacaagatgccgttcttctttaatctcaagggacgcaccgatgcgatgctggagaaagtgaaattcttccgtccgcattttactgaccgtgcgatgcaaaaattcggtcacctgttccccagccatttaccgccgcgcatgaaaaactggcgcgataaatacgagcatcatctgctgttaaaaatggcgggcgatggcgtgggcgaagccaaatcgtggctggtggattatttcaaacaggccgaaggcgatttctttgtctgtacgccggaggaaggcagcaaagcgtttttacaccgtttcgccgctgcgggcgcagcaattcgttatcaggcggtgcattccgatgaagtcgaagacattctggcgttggatatcgctctgcggcgtaacgacaccgagtggtatgagcatttaccgccggagatcgacagccagctggtgcacaagctctattacggccattttatgtgctatgtcttccatcaggattacatagtgaaaaaaggcgtggatgtgcatgcgttaaaagaacagatgctggaactgctacagcagcgcggcgcgcagtaccctgccgagcataacgtcggtcatttgtataaagcaccggagacgttgcagaagttctatcgcgagaacgatccgaccaacagcatgaatccggggatcggtaaaaccagtaaacggaaaaactggcaggaagtggagtaaaaattacggatggcagagtatcgccatccgaattcacttaatcgttctgtgccgtctgccccgccgccgccatttgggcggctttttgttttttatagctcaacgctgctgccggcacaggcatcactttaccggtttcaatccaggtacgcaggcggctggcatcggcaaaatgggtatatttgccaaacgcgtccatcactaccagcgccaccggtttattattgataaccgtacgcatcaccagacaatggcccgccgcattggtaaagccggttttggttaactgaatattccagttatcgcgatacaccagatgattagtattgcggaacggcagcgtatacgtcggattagagaaggttgccatatcttcccgggtagtacttaactgcccgatcaacggatattgtttgctggcaatgagcagtttggttaagtcacgggcagttgaaacgttatgcaccgacaatccggtaggttcaacaaagcgcgtgttgttcattccgagcgatttcgctttcgcattcattgccttaataaaggctttgtaaccaccgggataatggtgcgcaaggcttgccgccgcgcggttttctgaagacatcagcgccagcaacagcatatctttacggctgatttcgctattcagtcgtacgcgcgaatagacccctttcatctccggcgtctggctgatatccacttttagtttttcatccagcggcagtcgtgcatccagcacaaccatcgcggtcattaatttgctgatagacgcaatcggacgcaccagatccgggtggttcgaatagatcactttgttggtattcagatcaacaatcatcgcgctaccggaggcaatttccggttgtgaagcggtggtagcggctgccgttttcgcaacggcctgcggtgcaaaaggcacagccagcatcagggccaggctaaataaagaaactcgaaatttcggcatgatgagcattcagatagtggttcacgcgcacgggttgcgcaccgccggagtaaggatttactgaggctagcgacgccatcataacgagcaaaaagtgcgatcgtcaaaggagaatcgtgaggaaatgctgcattgctgacatttacgccagcaatgcaacgtcaaagaactttctagaacaaacgataaccgtagccccatagtataacggttagggcgagcagcacttccagtaccagcacgccaatcgccagcgtcgaactagagaagctaaggccttcctctttgttgatattcaggaagctcggaataccaaggtaaagcaggtagccggtgtaaaacagcgccaccgtgccgaccagcgcacacaaccagaccagtggataaagcgccaccagaccgcttaaaaacagcggagttgcaacgtagcccgcgaagaccatgcagtgcgcaagtgacggacgctgcggataattacgcgccatccaccagatgacccgccccatcaccgcgaccccagccagcataacgccgtaaaacaagacagccagcgccagtccggtaaaccaggataacttcaggatagtgccatcgccaaaattccagccaatctgtgtagtgccaatgaaggcgcaaatcaccggaatcgccgccatcagcaaaacgtggtgggtgtaatggtgagaaatcgtttcgttttcgcgattaatcacctgcatttcacgatcgggatgggaaaacagtccccagacatggctcataccgcccccttgttgtgagttcatgaacctgacagttcaagtataagtcagcttgtgattattttttgttcgcccatgtaattttcactgtctgatgaacgtcctttttcagcgtgaatgattcacagggtgtatgcttactggcaaccaaagggagacagactggcctatggatctcaatacacttatctcacaatatggttatgccgcgctggtgatcggtagcctggcggaaggtgaaaccgtgactttgctgggaggcgttgcggcgcatcaggggctattaaagttcccgctggtggtactttctgtggcgcttggcggcatgattggcgaccaggtgctctatctgtgcgggcggcggtttggcggcaagctgttacgccgtttctcgaaacatcaggataaaattgagcgggcgcagaaacttatccaacgccatccgtatctgtttgtcattggtacgcgctttatgtatggctttcgggtgattggcccgacgctgattggtgccagccagctgccgccgaaaatctttctgccgctgaatattctcggcgcatttgcctgggcgttgatttttaccactattggttacgctggtggtcaggtgattgcgccgtggttgcacaatctcgaccagcatttgaagcactgggtctggttgattctggtcgtggttctggtggtgggcgtgcgctggtggctgaaacgacgcgggaagaaaaagccggatcatcaggcgtaaaaccattgccctggataaggcgttcgcgccgcatccgacatccggagtaccatgcctgatacgacgcttgtgcgtcttttcatgccgaccaaaatattacccaatgaaatatccacgcacctcactgcgctattctgggttgaactgtggattcgccaacataaagccgccatccactatcaacgactgcccggtggtgtaatttgcgccctccgaacaaagccacaccaccaggctggcaatctcatgcgttgcgccaaaacgccgcaagggaatcgaaggctccgcgtcgggcttcacgtcgctgtcatccatgccattcattggcgtggcgatcgccccaggcgcgactgcgttcaccaaaatcttatgcctgaccagctccagcgccatcgctttggttaacccaccgagcgcatgtttagcggctgtgtaggcgctggcatccggcagcggcgtatgttcatgtaccgacgtaatgttgatgatgcgaccgccctgcccttgtttcaccatctgacgagccgcaatttgcgagcataagaatgcaccatcgacatcaacggtaaaaatcttgcgccactcatcaaaagccatatcaagaaacggcgctttggtcattgcacccgcattattcaccagcacatcaatgcgccccagccgttgaatgagtttctccagcgccagtgccccttctggtagattgccgagatccagctgcacgatctccgcacgtacgccgtggctaactacctcacgcgcggtatcttttgccccttcttcatctgagtgccaggtaataccaatatcaaacccctgctgcgccagtaataacgcgcactctttgccgatccccgaatcggaggcggtaataatcgcaacctgtgccatcgagttctccacttaacgctgaataaacgttaagtatagaaggcgcatatcatcagcgtttgtaccccccgcccaacgcaccagtgagttgaatggaggcatccagccactgcccttgcaataacaggccattggcccgctcacgcagcgcggggattctggcttcgctgacgcgggaaccagcaatgatgcccgcgttaaagcgcgcctgcgcaagacctaccacacgcaaggcatcgcgctcaatttgcgcctgatgctggtttttctccgccagtgtctgaacctgactggctgcccgcgccacgtcattcaccgcttcaaccaccgctttgttgtagctggcgatagacaagttgctttcggcttttgcgatatcgagattggcgttaagacgaccactatcgaaaatgggtagcgtcaggcctgccgtaacgcccatttgctgcgcggaatgacggaacagatcgcttaagtgcaacgcatcctgttgcaggaaggccatcaggttgatgtcaggataaaatgccgcttttgccgcatcaatggtgcttagcgatgactcaacgtaccagtgcgccgcctgcaaatctgcccgccgggccagtaaggagtaccccagttcatcaggaagctggcttgccactttcggcaacgcgaccggtttaagcttcaatgactttgtctggttatttgtaagtgcgcttaaccgtgcctcaataattttcattttccccgcgacatcgttgagctgctgccgggttttgctggcattaatatcggtttccacaccttcaactgaagaagtaatcccgttctgatatagctggcgatcggtcgcgataatggtgttctgctctttttctatttgctgcaagaccgtgtttaacgccgcctgggtttgccactcccagtacaggcgggctacgctgccagccagcaattggcgggtttgctcgcgttccgccgcccgtgctttaaccgtacccaggcgggcagtaacctccgcccgattctttccccagatatcgagatgccagcccgccgttaagccaaaagtaccgttggtgtaccacgggccggtcgtacctgcggccggatcgttcagagcaaacggccccattaagccttctgccgacattttttgccgctccatatccgccgaaaagtcgatctgcggaccatcctgagtggcaactgccttcgcctgggcttcagctagctgaatgcgctgttcagccacctgcatatccggtgcgttctgtagtgcattgttaattaaggaagtgagttgattatcgtgatactccagccaccattggctgtctggccaaccattttcagcgccgtgggtaatgcggtgtcaacttgtgcagcgggcgtttgctggcttaacgcctggcgggtttcatgcataggcgcacacccggccagcatcagtaacagcggaaaacaggcgatggctggataaaaggaatcacgattcatgggggaataatcaggtaagaaaaggtgcgcggagattaccgtgtgttgcgatatattttttagtttcgcgtggcaatacatcagtggcaataaaacgacatatccagaaaaatatacactaagtgaatgatatcttccgatttatcttaatcgtttatggataacggcaaagggcttcgttttttcctatacttattcagcactcacaaataaaggaacgccaatgaaaattatactctgggctgtattgattattttcctgattgggctactggtggtgactggcgtatttaagatgatattttaaaattaattaatgtcatcaggtccgaaaataacgagaatatttcagtctctcatcctgttgcgctcctgtcatgtgcattgcttcatataatcactggcgcaaggagcgcgcagggggcggccaatcgccgccgccccctgcacccccgggctctggcgaacaaaatcgccgctgcgcggtgccctcggcttatcccttacggctaccgggtcgggcgcgaggtaacatccctgtaaaacgcgccctcagcccacatccatgtgggctgccccggccttcagggaacgcctcggcaattttgacgccaccaaacaaccgtgcggcctattgataaagagctaacacattgtcaaaaaacatcactatggttttttagagtttctcgatatcaattgcctgaatagcccttgcaatatcaggggaattattcaacacccgaacatgctgaaataattccgttgcttcatcgtattctttacgcaaataactcaaccactgtttaatccgcgcaacgtgatataacccggtatcgccctgcttttccagacgggtatatttttgcagcaaagcaaccacctccggccacggcattcgcggttcgttatattttaccacccggctcaggttgggaatattgagcgccccgcgaccaatcatcactgcgtcgcagccgctgatcgccatgcattgttgcgcgctctgccagtcccagatttcaccgttggcaatcaccggaatattcagccgctggcgaatatcgccaatcgcctgccagtcaatatgctccgcgcggtaaccctgctctttcgtccgcccatgcaccaccagctccgtagcgccagcctgttgaaccgcatcggcgatttcaaatttcttctcaccgctgtcccagcccagacgcactttcacgctgacgggcaaatgcgccggtacagcttcacgcatcgcttttgcaccctggtagatgagttcaggatctttgagtaacgtcgccccgccgccgctaccgttaaccgttttcgacgggcagccgcaattgagatccacgccccaggaacctaactccaccgcacgggcggcgttctctgccagccattgtgggaactgacctaacaactgcacgcgcaccagcgtaccagatggtgtccggctggcgttttgtagctcagggcaaatgcgatgaaagacttttaccggcagcagttgatccaccacgcggacaaactcggtgatgcacagatcgtagtcgttaacttcggtcagcaattcacgcaccagagagtcaagcactccctccatcggtgccagtaacacacgcatatcatcacccgcaaaaaaatgaggcgctatgttagcgcctatggtcagcggattaaaggtctgcaaagagggattgctgcaaactgcaatccctctctatgcttgatgtatgcctgagttcgctgcgcattgcgtaatgccggggagcgaaaaaataagcgctgatttcttaatgtgatcggtagcacgttttacgaattaattgtatgatgaatccatctcatctggggtgttgattatgagtaagacactgaacattatctggcaatatttacgcgctttcgtcctgatttatgcctgcctgtatgcaggcattttcattgcttccctgctaccggtaaccattccgggcagcatcatcgggatgctgatcctgtttgtcctgctggccttgcaaattcttccggcaaaatgggtcaatccggggtgctacgtactgattcgctatatggcgctattgtttgtgccgattggcgtaggcgtcatgcaatattttgatttgctccgcgcacagtttggcccggtagtggtttcctgtgcagtcagtacgctggtggtttttctggtggtgagctggagttcgcaactggtacacggtgaacgtaaagtcgtaggtcagaaaggatcagaagaatgatggcgaatatctggtggtcattaccgctgacattgattgtcttttttgccgcccgcaaactggcggcacggtataagtttcccttgcttaacccgtcgctggtagcaatggtggtgatcattccttttttaatgctgactggcatctcttacgacagctactttaaaggtagcgaagtgctaaacgatctgctgcaaccggcggtcgtcgcgctggcctatcctttatatgagcagctacaccagatccgcgcgcgctggaaatcgatcatcaccatctgttttatcggcagcgtggttgcgatggtgacggggacttccgtggcattgttgatgggcgcttcaccggaaatcgccgcgtcaatcctgccgaaatcagtcaccacgcctattgcaatggcggttggcggcagtattggcggtattccggcaatcagcgcagtttgcgtgattttcgtcggcatcctcggcgcggtatttggccatacattgcttaatgcgatgcgtattcgtaccaaagctgcgcgcggtctggcaatggggactgcctcgcacgccctcggtacggcgcgctgcgccgagctggattatcaggaaggtgcatttagttcgctagcgctggtgttatgcgggataattacttcgctgatcgcaccgttccttttcccgattattctggcagtaatgggctaaaatttgcgatgcgtcgcgcatttttgatgtatgtttcacgcgttgcataattaatgagattcagatcacatataaagccacaacgggttcgtaaactgttatcccattacatgattatgaggcaacgccatgcatccacgttttcaaaccgcttttgcccaacttgcggataacttgcaatctgcactggaacctattctggcagacaagtacttccccgctttgttgaccggggagcaagtctcatcgctgaagagcgcaacggggctggacgaagacgcgctggcattcgcactacttccgctggcggcggcctgtgcgcgtacgccattgtcgaattttaatgttggcgcaattgcgcgcggtgtgagcggaacctggtatttcggtgccaatatggaatttattggtgcgacaatgcagcaaaccgttcatgccgaacaaagcgcgatcagccacgcctggttgagtggtgaaaaagcgcttgcagccatcaccgttaactacacgccttgtggtcactgccgtcagtttatgaatgaactgaacagcggtctggatctgcgtattcatctgccgggccgcgaggcacacgcgctgcgtgactatctgccagatgcctttgggccgaaagatctggagattaaaacgctgctgatggacgaacaggatcacggctatgcgctgacgggtgatgcgctttctcaggcagcgattgcggcggcaaaccgttcgcacatgccttacagtaagtcgccaagcggtgtcgcgctggaatgtaaagacggtcgtattttcagtggcagctacgctgaaaacgccgcattcaacccgactctgccaccgttgcagggagcgttaattctgttgaatctcaagggttatgattacccggatatccagcgcgcggttctggcagaaaaagccgatgcgccgttgattcagtgggatgccacctccgcaacgctgaaagctctcggctgtcacagtatcgaccgagtgcttctcgcttaagcctggtgccggatgcggcgtgaacgccttgtccggcttgccagccctctcctggtgtcgaaattcccggcaaacagtttgccgtttcttgcgcaaaaccagcgggtaaagtagcctgatggaaattttccttagatcgagtctcctgcatgttaaagcgcgtgttcctcagcctgttagtcctgatcggcttgctgctgttgactgtgctcggcctcgatcgctggatgagctggaaaaccgcgccttatatctacgacgaattgcaggatctcccctaccgccaggtcggtgtggtgctcggaacagcaaaatattatcgtactggcgtaattaatcagtattatcgctaccgcattcaaggagcgattaatgcctataacagcggtaaggtaaattatctattactgagcggcgataacgcattgcaaagttataatgagccgatgaccatgcgcaaagatttaatcgctgctggtgtcgacccatcagatattgttctcgattacgcaggctttcgtacgctggattccatcgtgcgtacacgcaaagttttcgatactaatgatttcattattatcacccaacgtttccactgtgagcgagcattatttattgcgctgcatatggggattcaggctcagtgttatgccgtaccgtcaccgaaagatatgctgtcagtacgtattcgtgaatttgccgcccgtttcggtgcgctggctgacctttatatttttaaacgtgaaccgcgttttttagggccgctggtccctattccggctatgcaccaggtaccggaagatgcgcaggggtatcccgccgtcacacccgaacagttacttgaattacaaaagaaacaaggaaagtagttatggatgtacagcagttttttgtcgttgccgtttttttccttatcccgatattttgtttccgcgaagcatggaaaggctggcgcgcaggcgcgattgataaacgggttaaaaatgcaccggaaccggtgtatgtctggcgagcaaaaaatcccggactctttttcgcttatatggtggcatatatcggcttcggaattttatctatcggcatgattgtttatcttattttctatcgttaatattcccctctccagttaattattgagaataattattacttcacctgataagctgcggatatcacattcctaaccgcagctatttgtgaatcttttcacagtttaaattcccccgcacgcttagccttaatatcagtacattattatttactaaacgctcgccttaattacctatagcattaaggaagatcacatgccgcaacaaaattatctggatgaactcactccggcttttacgtctttactggcgattaaagaagcctctcgctgtttattatgtcacgacgctccctgtagtcaggcttgcccggcacagaccgatccggggaaatttattcgctcaatctactttcgtaattttaaaggcgctgccgagacaattcgcgaaaataatgccctcggtgccgtttgtgccagagtgtgcccgacggagaaattatgccaaagcggttgtacccgtgccggtgttgatgctcccattgatatcggccgcttacagcgttttgttactgattttgaacaacaaaccggaatggaaatttatcagcccggtactaaaacgctcggcaaagtcgcgattattggcgcaggtcctgccggattgcaggccagtgtgacactgacaaaccagggttatgacgtcacgatttatgagaaagaagcgcaccccggtggctggttgcgtaacggtattccgcaattccggttaccgcaatcagtgctggatgcagagatcgcccgtattgaaaaaatgggcgtgaccattaagtgcaacaacgaagtcggtaacacactcacccttgagcagctgaaagcagaaaaccgcgcggtactggtcaccgtggggttatcaagcggttccgggctaccgctgtttgagcatagtgacgttgagattgccgtcgacttcttgcaacgtgcacgacaggcgcaaggcgatatcagcattccacaaagcgcattaattatcggcggcggtgatgtcgcgatggacgtagccagcacgctgaaagttctcggctgtcaggcggtaacttgcgtagcgcgtgaagagttagatgagtttccggcaagcgaaaaagagtttaccagcgcccgggagctgggcgtttcgatcatcgatggattcacgccagtagccgtggaaggcaataaagtcacgtttaagcatgtacggttatcgggcgaactgacgatggcggcagataaaattattctcgccgtcggtcagcatgccagactagatgcctttgcggagttagagccgcagcgtaacaccatcaaaacacaaaattaccagacccgcgacccgcaagtctttgctgctggcgatattgttgagggtgacaaaaccgtggtctatgccgtgaaaaccgggaaagaagccgccgaggcgattcatcactatttagagggagcttgctcatgttaacgaaagatctttcgattactttttgcggcgtgaagtttcccaacccgttctgcctctcttcttcgccggtaggcaactgctatgagatgtgtgccaaagcctacgacacaggttggggcggtgtggtgtttaaaacgatcggcttttttatcgccaacgaagtctcgccgcgttttgatcatctggtgaaagaagataccggttttatcggcttcaaaaatatggagcagattgctgaacatccgttggaagagaatctggccgccctgcgtcggctgaaggaagattacccggacaaagtattgatcgcttcgatcatgggggaaaatgagcagcaatgggaggagctggcgcgcctggtgcaagaagctggcgcggatatgatcgagtgtaacttctcctgtccgcaaatgacttctcatgcgatgggtagcgatgtcgggcaaagcccggagctggtagaaaaatattgtcgggcagtgaaacggggttccacgctgccaatgctggcgaagatgacgccgaatatcggtgatatgtgcgaagtggcgctggcggcgaagcgcggcggcgcagatggcattgcggcgattaacaccgttaaatccatcaccaatatcgatcttaatcagaaaatcggtatgccgatcgttaacggaaaatcgagtatttccggatattccggtaaagcggtaaaaccgatcgccctgcgcttcattcagcaaatgcgcacccatccagaactgcgcgatttcccaatcagcggtatcggcggcattgaaacctgggaggatgcggctgagtttttattgctcggcgcagcaacgttacaggtgaccaccggcatcatgcagtacgggtatcggatagtggaagatatggcaagcgggttgtcgcattatctcgccgatcagggatttgattcgctgcaggagatggtaggtctggcgaataacaatattgtcccggcggaagatttagaccgcagttatattgtctatccccgtatcaatcttgataaatgtgttggctgtggacgctgttatatttcctgttacgacggcggtcaccaggcgatggaatggagcgagaaaacccgcacaccgcattgtaataccgagaaatgtgtgggttgtctgctttgtggtcacgtctgcccggtgggttgtattgagctcggggaagtgaagtttaagaaaggcgagaaagaacacccggtaacgttgtaaaaccagagacgcatccggcatttggttcctgtcgccggatgcggcttgaacgccttatccggcctacaaaaccatacaaatcagtatgttgagcttattgtaggccggataaaacgcgccagcgttgcatccggcatttggctcctgttgccggatgcggcgtgaacgccttatccggcctacaaaaccacacagatcatgatgttatgtgcgtttatgaccgaatgcggaccacattcacatcatttcttacgcgcgtatttcagtgaatccagcgctacggcgaagataataatcgcccctttgatgatgtactgccagtatgggtttacgccgatatacgtcaggccatagttgatgacggtaaaaataattaccccggtcaccacgccaatcaccgtccccacaccgccgctgaacgatacaccgcctaccacgcacgccgcgatagcatccagctcatacataaagccgaggttgttggtggcagagccgatacgtccggcttctaacatcccgccaaaggcatagaacacgccagacaacgcgtagatcatcagcaggttcaggccgacgttgacaccagatacttttgccgcttccgggttaccgccaatggcaaaaatgttcttaccgaagcgggttttgttccacaacacccagacgaacgccaccgcaatcaacgcgtagaaggtgatgtaagagagacggaaactccccagcgcgacaaagccctgagcaaaggtagagaagccactgtcaaaaccagaaattggcgacgccccgacaaagtcgtaatagagcgagttgatgccatagacgatgatcatcgtgccgagcgtggtaatgaacggcgtcacgttgagataagcgataatcagaccgttgatcaaaccgatcaccgcaccaatggcacagacaatcagaataaccagcgcaatcggcatcgtcgccatttccgggaacactttgttggcgttatccatggactgcaataatgtcgcagccaccactgccgccagccctacctgacgaccagcagaaagatcggtcccctgggtgacaattaaccctgccacaccgagcgcgataataatacgcaccgatgactgggtgagaatattacttaagttcaacagacttaaaaatgttgggtcctggaaaataataatcgccagcaaaactaaaagaacgacgtaaataccgccctctttcaggtaagtaagaaaacttttcttatttaacgcactcatgggaagcccctaatcttaaaggtgcaaagacgcaagacgcagaatttcgttttgcgttgttgtttttgtatcgacaattccggaaacgagaccattgctcatgaccagaatacggtctgttatccctaacaactcaggcatttcagaggagataataataatccccttgcctttcttcgccagttcggcaattaactgataaatttcaaacttcgccccgacatcaataccgcgcgtcggttcatcgagcattaatatttctggttgcgttagtagccagcgaccaataatcaccttttgctgattaccaccggagagcgaaccaatttgcgtccgatgacccggcgtttttacccgcatcgaatcaatcacccactgggtatcgcttttcatccgcgagttatccagtaaaccaactttatttttgtagttgcgaatattggaaattaacgagttaaaaccaatatccagataggcataaattcccgttgagcggcgctcctcagttaccagtgcaaatccatggtttatggcttcgttggcattatggttattgatctgtttgccgtgcaacgttatggtgccagccgatttctcgcgaataccaaataacgtctcaacaatatcggtacgtttcgcccccaccagaccggcaataccgaggatctcccctttatgcagatcaaacgagacatcgcgaatcgacggctggcgcagtgacgtcaggttacgtacctcgaggatgacttcgcccggtttgttttctttgtcagggaaacgctggttaagagaacgcccaaccatcatggcgatgatcttgtccatcgtcagtcctgccagcggttcggtggcgatccactgaccgtcgcgcaatacggtaacttcatcacataactggaagatttcttccattttatgcgagatataaacaataccgcagccgcgctcttttaatttacgaataatagtgaacagatgattgacctctttttcggttaacgaagaagtcggttcatccataatcacaattttcgcgttataggaaaacgctttggcgatttcgatcatctgcatttgcgaaacggataatgtgccgacgcgcgcacgcggatcgatatcaatatccagttcgtcaaaaatcgctttggtttcgcggtacattttgtcctgatcgacaaacatgcctttggtgggatatcgccccagccacatgttatccatcaccgaacgttgtaataccaggtttaactcctggtgtaccatcgaaataccattttccagggcttcttttgcagaatggaaatcgatctctttaccctggaataaaatggtgccggagtctttttgataaataccaaacaggcattttaataatgtcgattttcctgcaccgttttcccccattaatgcatggatagaatgtggccggacttttaaattaacgttatcaagtgccttaacaccaggaaaggacttgttgataccgctcatttccaacaagtattccccggaggacggagtcgttgagctgaccatataattttaccttgttggccatacaataagggcgcagtaatagactgcgcccaatcagtcttatttcttgctgaattcagccaggttgtctttatctacgccaacataaggtacgcggaccactttgttgtcgattttccagttggtgccatcagccgcacctttaccatcggccaggtttttcgccagatcaaaggtcgctttcgcctggttgttagcatcgttcagtacggtgcccgccagtgcaccggatttcaccagcgccagcgcttctggcagcgcatcgacgccaaacaccggaatgctggacttgttgtgtgctttcagcgcttcaaccgcgcccattgccatcgcatcgttgttggcgataaccacttcgattttgttggcgttcgggccagacagccaggcgtccatcttatctttcgcctgagcggtgtcccacattgcggtatctaactgtaactgttcagttttgatgcctttatcgttcaattctttaatcacgtaagtggtacgtgcttctgcatccggatggcccggttcacctttcagcagtacgaactgaatctgaccgtctttgttcagatcccaaccctgattcgccgcccagtgtttagcaatcaaatcgccttgaataatgccggactctttggagtcagtgccaacgtagtaggctttgtcgtagctatccagcgccttacgagacggttctttgttgaagaaaaccaccggcacgttttgcccacgcgctttctcaatcaccgtacccgcagctgccgggtcaaccaggttgattgccagtgccttcacccctttcgccagcaatacgtcgatctgatcgttctgcttggactggtcattctgagaatcattcatcagcagctgaacatctggcgcggctttcgcatcttgctcaatagccttgcgcactacagacataaagttatcgtcgtacttatagattgttacaccaatgcgagtatcagcagcgtgtgcagcggcaccgaataacatgctggccatcacagcagacagggttaacaccttcttattcatggtatctccggtttttcttatgcagggtagtgcttgagataaatgctcggcggggcagtagagttaatgaagtgttactgaacgccgaagctcactttttaaaattcgttcttccatgcccggtaacgctccagaaaacggctttaattgttgttatgacgctgttacctcggcaaaagtgattattcactgttacatacgggttacaacgttaaaacggtgcaatcatagctatcacattgttaagatactgtgaaatcactcacagattgaaagcggttacatcgcctgatttgttgagttagtgatcgccgccgcattctggcgtgttgcgacagaatggcgacgcactaacgtcggcataaaacagtggctggcacgaggatcaatattgcctgctgccccctgcaaggccagttcggtggctaatttcgccattgaagcaatgggataacgcacggtcgttaattgcgggtcggtgtaacgggcgatgggaatatcatcgaaaccgatgattgagagatgtaacggaatcgcaatgccattatcttttaatgctgtcagtgcgccagcggccatattgtcgttataagcaaatacagcggtaagttgtagattgcgccccagcagttcaaccatcgccgcctcaccgcccggcatgtccggcgtaccagcgccaatccagctttccggcggaataatatcctgctctttcaacgcactcatccagcctgctttacgcatggcgtcatcttcaatgccgtggctggaagaaagataaccaatacgttgatgaccgttattcagcaacatgcgcgtcgccattcgggcaccgctgagattatccaggcaaacgcaacgatgggcgtaccccggcacaacgcggttgattaacaccataccgggaatgttatccataaattgcgccagttcatcgtcactcaatgcttttgagtgaacaatcaacgcattacaacgctggcgaattaacacctcaatggcgtgacgctctttttccgcttcatgatagctattgccgattagcacgtatttctgatgctgctgagcgaccagatccaccgcttttaccagcgcgccgaaaaacgcatcagaaacgtccatcaccaccacgccaatggtgtcgctaacctgagttgccagcgcctgggcattggcgtttggccgataatccagctcactcacggctttcattactgcttcacgcgtgtcggcactgaccagcgtgctgttattgagcacccgggaaaccgttgccacagagacgccagcctgacgcgctacatcacgaatggtgatcatattcactacctgttatgagattgcagtaaatgactgcttgctggcggctattttgtcagcactgaatacaggacttcgtgaatcgagtcacagcaatggaaacggttacagccgttttgttaacgaatgtgatccagatcgttatcttgatgttttagatattgccggtccggcagcacgcaaagttaactgacgccagagccattccaccggcccctggcggaagtaacgcagccagataacagagaagaggatattcgccagccataccggaataacaaacgccagcagctccaggcggtcaaaatgcataaacaaaccgaggtggtaaaaaagcgtggtacaaatcagcgtttgcaatagatagttggtcagcgccatccgtccgacgcaggcgatcgcaagcaccagcttaaagcggctcaattgcggccagaagccataaaacagcgacgcatagccaatcgcctgaaacggcgcactcagttcccgcggcatttgaagtaagaaggcacaccagcgatacgcccagtccagctgccattgcagggcgatggcaggaaggttaatggtcaccccaatcgccaccagcacaaaaccagtacgacgatagtgacgtaagctgaactgccctttcagccagccgctgcgcatcagcgccgcaccaatgagcatcatccctgccagttgccagccatactgtgcgcccagtgccagtaaactgttgccaacaccatcggcacgattactgatcgcttcaacgccgccgtgaagcttccagtatttttcatacaaaatagccgatgcatccggcgtccaggcgcggctggtctggctgtcggaaatcagccccaataacagcaaaacgccaagccccaccagataaagcatgacgcctgtattaaacaggctttttaccgatggcgcatcgcgcaccagccgccagcagattaagcccaccagcccgtaagccagcaaaatatcgccgtcccagaacaataaaccgtgaataaagcccaacaagactaacagcgttaaccgcgactggatccagcgtctgccacggggcagcaacatttgcaggcccgcaccaaacagtagcgcaaaaagcgtgaggaatttcacctggccgatgagatcaagaaatgcccaagtccatgcatcccgcggcgtaatagcaccgtaccaggcgggattgagataagccgcctttggtagcccaaaggcgctgatgtttaatagcaggatccccagaatggcgacgccgcgaacaaaatcgagcgtgacgttgcgctccatggttcctgccttttaatcagttgtgatgacgcacagcgcgcagaaactcgtggcgcgtattctgactggatttgaacaatccaccaagagaggtcgttgtcgtggcactggttgcatcgcggatgccacgcgccttcacgcagtaatgcaccgcgtcgatcgagacagccacgttattggtgcccagcagcgtttgtagcgcaataagaatttgctgcgtcagacgttcctgcacctgcggacgctgggcaaagaactgcacaatgcggttaatttttgacagaccgatcaccgaatctttcgggatataggccaccgtcgctttgccatcgatggtaacaaaatggtgttcacaggtgctggtcagagtgatatcgcgcacggtgaccatttcatcgaccttcattttgttttcaatgagggtgattttcgggaaattggcgtaatccagaccggagaaaatttcatcgacatacattttagcgatgcgatgcggcgtttccatcaaactgtcatcagccaggtcgagattcagcagctgcatgatttcggtcatatgaccagcaataaggcttttgcgcgtttcgttatccatttcatgcacgggcgggcgcagcggtgtttccagtcctcgcgcaactaacgcttcatgaaccagggccgcttctttactgagtgatggcatttatgatttctcctgcaggtgtgacgcctccgccctgcgtgggggcaaagttattaagctgatttacagcctgattattgtgcgtgaggcggcgcacataatccagtattcacagcgataattattgtaattgccgctgcctttcatcagcagatgttaaaacatcgttatgcaaatacggaagtgaaagttactcacagcacattgaataaacggtatgatgaagaaattgcaaacaacacaacaaggagccacgcatggaaatgctcgaagagcaccgctgttttgaaggctggcagcaacgctggcgacacgactccagtaccttaaactgcccgatgacgttcagtatctttctccctccacctcgtgatcacactccgccaccagtgctgtactggctttccggattaacctgcaatgacgagaacttcaccaccaaggcgggtgcccagcgggtagcggcggaactggggattgtactggtgatgccagacaccagcccgcgcggcgaaaaggttgccaacgacgatggctacgatttaggccagggcgcaggcttttatcttaatgccacgcaaccgccgtgggcgacgcattaccggatgtatgattatctgcgcgatgaattaccggcgctggttcagtcgcaatttaatgtcagcgaccgctgcgccattagcggtcactcaatgggtggtcacggtgcgctgattatggcgctgaaaaatccgggtaaatacaccagcgtttcggcctttgcgccaattgtgaatccgtgcagcgtcccgtggggaatcaaagcgtttagcagctatttaggtgaggacaaaaatgcatggctggaatgggacagttgcgcactgatgtatgccagtaacgcgcaggatgcgatcccgacgcttatcgatcagggcgataatgatcagtttcttgccgaccagttgcaacctgcggtactggcagaagccgcgcgccagaaagcgtggccgatgacgctgcgtattcagccgggatatgatcacagttactacttcatcgcctcttttatagaggatcacctgcgcttccatgcgcagtatttactgaagtgaaagtccgcccggttcgccgggcatcttctcatcagaagcgataatccactgccataaagtaacgacgtccgtcttcgttatagctgtagtcgtcacgactgagatccttgtcgccaaggttcagcacgcctgcgcgcagtttgacgtctttagtcacctgccaggccgcgccggtattccagatggtataaccgcccggtgttttagccgtcgcgctgtcggcgcgtttctgcccggtatagtgcccagaaacatagaatgaccagtcttccagcgccagcggtttccagtccagcgtaccgttagcagtatggaacggcagatcggatagcggtttgttttcgccgttgctgacatcacgaccatcgttgtaggtgtagttgatcgacagtttccattcatcgttgaacggaattttcagttcggtttccacgccctgaatacgagctttgttaacgttgtagtagctaaataccggtatgcgccgtccgttagcgcccgtctcaaaaccaacaaagttttggtagcccggtgcagcgttgacgtcagacgtacggctgatgctgatacgatctttcacatcgttacggaaaacggtaacgctggattcaaccccttccagccagccttcttcacccatgtagtaaagccccagctcccaactttcgctggtttctggtttcagatccgggctacccacaatcttacatgcgccacggcaggaattgctcgtccagtcagggctaagttgcaacagagaaggtgctttaaatgccgtcgcccagccccctttcaccgttacggtgtcggtggcgttataaaccaggtaggcacgcggactccagtgttcaccgtaggtttcgtgatcgtccatacgcacgccggtcgtcagcgccagcggctcgaagatccgccattcatcttccacaaacagcgcgtactggctggcagacgttttggagctggttcccccggtcaggttcaccgcatcgctaagtttgtcgtgacgccattcaccgccaaccgtgagaaactgattaatcgccgtcagcggcaacgtgtatttgccgtcgaccgtattgctttcggaagttatcgggctgctgttgccagggtttttgttctcgactttctcaccgtagtatttcagttcgctggtgccgtaatcccaacgcccattatggctgacggagtagttctggcgttccaggcggtttttgtccagcgagtcggaatcacgatcctgacggtcgaaaccgtatccggcagtaaaatcgtgattttgattcggtgtccaggcaaattcgacattgccgtcgcggctggagaatccttcaatacgcggcgtttctccggtatcggtggtcgttgagttttgcgggtcatccttttcacgttttgccaggctgccgtaagctttcattcccagcacaccatcaattaatggtccactggtaaagaactgaccgttataggtgtcaccgcgatcgcgatgttcctgaatggtggtatcgacggtaacggtacccgaccatttctgaccgatttttttggtgatgatattcactacaccgccgagcgcatcggaaccgtacagcgacgacatcgggccacggaccacttcaatacgttcgatggaatcgaccgggatccagttcagatcgaaatcattgtggcggaagacggcattgcgggagttcacgcgtttaccgtcgacgagaatcagggtatagctgctgtccagaccacgaatactaacgcccttacggttatccccttcgttcgtcagttgtacgccaggcacttctttgaggacatccttcagattctgtaccggttttcgctgcaggtcttcctgggtaatgacgctgatactggcaggtgcatctttaagattttgttccacggaagatgcagtgacaaccatcgtttcgccatcatcatcgaccgctaacacaggccatgcacaagaaatagcggacaaacacagcccgacccgtacgaaagggttcaacctaaacattccatatctccatgaggtaactacgaaaataaaatgggttatcgctcacatcttcttcacgtccccttgcgtacggcagcatcgcggtggacttattttttatgcaggtgatcatcccagaaagccggaacagcctctgatttgtcagccttttttgattgcggcgtaacgataatgcaaacgataacaattatcaatccaaatgttaaattttatatccgcatgatttgtcagggaaatggaattgaaaaagccctctcggttgagagggcttagcaaggaagggaggaaacttatttcttatcgttctgcgggaacttcatttcgctgtagcgtacgaagtgagttcctttaatcagcttgtagccgaaccaaataatcaggaacagcgggataccaatatacgttgccgctacgccgccccagtcaatagtatctttcaggaacgcttcgtagttctggcccaaagtgataatcagacacagaatgaatgcgaagatcggccccagtgggaagaaacctgaacggtacggcagatcgttaatgtcgtgtccctgcaatacgtaaccgcgacggaagcgatagtggctaatggcaatccccagccaggcgataaaacccgtcatcccggaggtgttcagcagccacaggtataccgtctggttgccaaacatggaggtcaggaagcacagaccggcaatcaccgtcgtcgcatacagcgcattacgcggcacgccaccacgcgacagtttagcgaaaatgcgcggcgctttaccgtcacacgccagggtgtacagcatacgagtagacgcatacataccggagttacccgctgacagcaccgccgtcagaataactgcgttcatcaccgccgccgcagagagcagacccgcgtgctggaacaccagggtgaacggactaacgctgatgtctttaacatcgttacgcagcaggctcggatcggtgtacggaataatcaggctgataatcaggatcgcgaacacatagaacaacaggattcgccagaacacctgacgtaccgcgcgtggaatgtttttcgccggatcttcggactcgcctgcagcaataccgatcagctcggttccctggaaagagaagccgacaatcatagctacgccgatcatcgccgcaaaaccaccagcaaacggcgcttcgccgattgtccagttgctccagcccgcaggctgcgcgcctttgaagataccgataatcatcagcacgccaacgatgataaagacaataactgtcgtgactttgatcagtgagaaccagtattccgcttcaccaaagccacgaactgagatgtagttcagcaggaagataacgccgaggaacaacgcactccagatccagcccggtgtatccgggaaccaccagctcatgaccagctgagctgcaaccaggtcaacggcgatagtcaccgcccagttgtaccagtagttccagcccagcgcgaagccaaagccttcttcaacatagttctgaccgtaagtggcaaacgaaccggaaaccggcatatatgcagccagttcaccgagactggtcatcaggaagtaaaccatcaggccaatcagcatatacgagagcaatgccccgcccggacctgcctgagaaatcgttgcgccagaggcaacaaaaagacctgtaccgatggaaccgccaatggcaatcatcgtcaggtgacgcgcctttaattcacggcgtaagcccggcgcttctgtggttttagtttcggaaaccatacaaaaatgctatccatcttaaaaatgaggcgcgattgtagcagacgattggcaatccttccggcagaaatacacggttataagacaccttcatgatcgcccagggattataagtaaagcagccaatctcttttctggcgaatgcatgctgaaggcgctgcgtcacgaaatcgacacagcaccagcatgttcttgtacagcaacttaacgcggcacatttgcgggatcgcaatagtccagaaagcgccgtagcgcgttggaaaggtgtttttgccgatgatgtatacgccacaacgtacgcatcaggcgcggcagagggaccgcaacttcacttaatgtgcctgcctgcaattgatcttcaatcacacgtcgcgacaggcaactaattcccaacccatgacgcaccgcatgtttgattgcctcggagttacctaattccatcgccatctcaaacttcggtaaatgtgacagcaacagataatcgacaatctcccgcgtgccggaaccgcgttcacgcaggatccacggcgcagcggccagctgttctaaggtgaccggaccacgggccaacggcgaagtcggcgcggcgaaaaccaccagctcgtcttccagccacggttcagaaatgatttcagtgctgtggcacggtccttcaataaagccaatatcaacgcggaaatccagcaccgcttgcatcacgtcctggctattcccaacgctaagttcaatcggcaactgcggataatcatggcgataacgggcgataactgcaggcagaatgtagttaccgatggtactactggcatagatacgaatcgcgccgttgtcttcgcgaaacagttgttcgatttcaaccgcctgttcaagcaatgccaacgcacgcggatagagcagccgcccgtgttcattaacaaccagtcttttccccacgcgatcaaacagttgcacgccaagctgcccttccaggtcggtcaaggctgcgctcactgctgattgcgacaacgccagcatcaccgacgcctgggtggttgatccacttttcaatacttctgcaaaaacttccaactgccggagggtgatgtgcatagtcgcttaccacttataaagattaattataaatatataatcaattttatttttaaaccagttagtcgtaaccttatgcccggttaaaggagagggttatgacgaatatcaccttacagaaacaacatcgtacactgtggcattttattccggggttagccctgagtgcagttatcaccggggtcgccctgtggggtggttccattcccgcggttgcgggtgccgggtttagtgccctcaccctcgcaatcttgttggggatggttttaggcaacaccatctatccgcacatctggaaaagctgtgacggtggtgtgctgtttgccaagcaatatttattacgtctgggtatcattctttatggcttccgtctgacgttctcgcaaattgccgatgtcggtatcagtgggatcatcattgacgtgttgacgctgtccagtaccttcctgctggcttgcttcctggggcagaaagtgtttggtctggataagcacaccagctggttgatcggtgccggtagcagtatctgtggtgctgccgcggtactggcgactgagccggtagtgaaagcggaagccagtaaagtaaccgtggctgttgcaaccgttgttatcttcgggaccgtcgcgattttcctctacccggcgatatatccgctgatgtctcaatggtttagtccggaaactttcggtatctacattggttctactgtgcacgaagtggcgcaggtggtggcggcaggtcatgccatcagcccggatgcggaaaacgcagcagttatttccaaaatgctgcgcgtgatgatgctggctccgttcctcatcctgctggcggcgcgtgttaaacagctgtctggggcgaacagcggcgagaaaagcaaaatcactattccgtggtttgccatcttgttcatcgtagttgccatctttaactcgttccacctgttaccgcagagcgtggtgaacatgctggtaacgctggataccttcctgctggcaatggcgatggcggcgctgggtctgaccactcacgtcagcgcgctgaaaaaagctggggcgaaacctctgctgatggcactggtactgtttgcctggctgattgttggtggtggtgcgattaactatgtgattcaaagcgtcatcgcataaaccactacatcttgctcctgttaacccgctatcattaccgttttcctccagcgggtttaacaggagtcctcgcatgaaatacattggagcgcacgttagtgctgctggcggtctggcaaatgccgcaattcgcgccgccgaaatcgacgcaaccgcgtttgccttgttcaccaaaaaccaacgtcagtggcgtgccgcaccgctcacgacgcaaaccatcgatgaattcaaagccgcctgtgaaaaatatcactacacatcggcgcaaattcttccccacgacagttatctgattaacctcggacatccggtcactgaagctctggaaaaatcgcgcgatgcctttatagatgaaatgcagcgttgcgaacagctggggctttctttgctcaacttccaccctggcagccatctgatgcagatttcagaagaggattgccttgcgcgtattgccgaatccatcaacattgcgctggataaaactcaaggtgtgacagcggtgatagaaaacaccgccggtcagggcagtaacttagggtttaaattcgaacatctcgcggcgattatcgacggcgtggaagataaatcccgcgtcggcgtctgcattgatacctgccatgctttcgctgccgggtatgatttgcgtactccagccgaatgcgagaaaacattcgcggattttgcccgtactgtcggctttaagtatctgcgcgggatgcaccttaacgatgcgaaaagcacctttggcagccgcgttgaccgccatcatagcctcggtgaaggcaatatcggtcatgatgcgttccgctggatcatgcaggacgaccgtttcgacggcattccgctgatcctcgaaaccatcaacccggatatctgggcagaagagatcgcctggctgaaagcgcaacaaactgaaaaagcggtagcctgaagatgaataaccgggaaaaggagatccttgcaattttacggcgtaacccgctgattcagcagaacgaaattgcggacatgctgcaaatcagccgttcgcgcgttgcggcgcatattatggatttaatgcgcaaaggccggattaaaggcaaaggttacattctcaccgagcaggaatactgcgtagtggtggggacaatcaatatggatattcgcgggatggcggatatccgttacccgcaatcggcttctcatcccggtacaattcattgctcagcgggcggcgtgggacgcaacatcgcccacaatctggcgctgttaggccgtgacgtccatttgctttcagtgattggcgatgacttttatggcgaaatgctcctggaagaaacgcgccgtgccggcgtgaatgtctccggctgcgttcgtttgcatggtcaaagcacatcgacgtatctggcaattgccaatcgagacgatcaaaccgtgctggcgattaacgatacccatctgctggaacagttgacaccgcaactactgaacgggtcgcgcgatttacttcgtcatgcgggcgtggtactggctgattgcaacctgacagccgaggcgctggaatgggtctttaccctcgctgatgaaatcccggtgtttgtcgataccgtttcagaattcaaagcgggcaaaatcaaacactggctggcgcatattcacaccctgaaacccactttaccggagctggaaattttatggggacaggcgatcaccagcgatgctgaccgtaataccgcagtgaatgcattgcatcagcaaggtgttcagcaactgtttgtttatttgcccgatgagtcagtttattgcagcgaaaaggatggagaacaatttttgctgaccgcgccagcgcatacgacagtagacagttttggtgctgacgatggttttatggcgggcctggtatatagctttcttgaaggatacagtttccgcgacagcgcccgttttgcggtagcctgcgcggcaatttcgcgcgccagcggcagcttaaacaaccctaccctgtctgccgataacgcgctttcattagtgccaatggtgtaacaatgttgccggatgcgacgcttaacgcgtcttatccggcctacaaatcaggcaatttcagcaagtaaatgtaggcctgataagcttgcgcatcaggcaatgacactcaagctaaaccaataaagaacccggcaatggtcgcactcatcaagttggaaagcgtcgccgccgccagcgcccgtaaaccaagctgggcgatttccggcgcacggtgtggcgcaaccgcagaaaacgcccccaccaccaccccgatagaaccaaagttagcgaaaccgcacaacgcgaaggaaataatcgccacagttttagcatcgagagtgccagccgtttgcagatagggtgagaaattgagataagcgacaaattcatttattgccagtttctgtccaatcaaactcccggcaagattcgcatcactccagtccacacccatcacccacgccagtggagccagcaggtaacctaaaatggactccagcgaggcatgttcaaaaccaaaccagccaccaacgccgccgataataccgttaatcaacgcaattattgcaacaaatgccatcaccactgttgccacacctgcggcgattttcagcccggtcattgcccctgtcgcagcggcttcaataatgctttttggcggtgtttcggtgaaagagaggttattaaaggaaacctgcgaagattccgttgccgggcttaacaggcgggcaaacaagatcccgccagggatcgccattaatgatgccgccagcagatattccacaggcacgcccagtgcggcgtaaccaatcattgtcgaaccagcaatcgaggccatgccactacaaatcgctgtaaataattcattgcgattcagacgatcgataaagggtttgacgattgccggaatttcgttttgcccgaggaaaatggtggtgaccgcgacgaatgactcgatcttgctgatatttaatgctttctggaagataccgccgagaattcgaattaaaatccccatcacaccgatgtagtagagaatactcaccagcgcggtgacgaagataattgccggtaacaccctgaaaccaaagataaatcctgcaccatcaaataaggtatccattttcggtccgaccagagaaccgaagataaatgcgctacccgcgtcgctgtacgccatcactttatgcacgccaaaagcgactttttcagcgacccaacgccctggcggtaaccaaagcataatgccgccaatcacgacctgtaacactaacgccgcgccaacggtacgcaggctgatcttcttcttgtttactgacagtaaaaacgcaatcgtcagcaataccaccattcccagaacacttctcatgacatccatagtgattatctcttcatgtcatattgggcgacggctttctgcccatcagaaatagccaggcctgcatcttgcgataccggcccggcttgttatcaacacttaatgggttttgatgtagccgcgcacgcactcttcgactaatccccagaaccagtctgtatcaatagtgatgccgactttggtattggcgggcttgccaagaacgcccagctcgtcgcagacggtacgcccatagcaagggccactgttgacgtccacttcgacgtacatctcctgggttttaatgccatcagggttaatcagataaccgatgcaggtggcgtcgtgcaccgggccgccagcaaggccgtagttttcgaactgcgttttgagagtgaagttcatgatgtcgctgaacagctctccggcggggccgcctgccctttccatccgagcaatcacgtccggggtgcaaacggtctggttggtgagatcgaggcccatcatcactaatggaacgccggaggtgaacactacgcgtgcggcttccgggtcggcaaagatgttgaactcggcagatggcgtgaagttgcctgtaccgtaagcgccgcccattagcacaatttcacggattttgggcaggatcgcgggttgcatacgcattgccaccgcgatatttgaaagcggaccaaccggcaccagagtgatatcgccatcgcttgccatcagggtatcaatgatatatttcaccgcatgagtgctttctgcctggcgggtcagcggctcgaataccgggccatccagtccggtttcaccgtgaatattatcggcaacgatttgttgacgcataatgggctgcggcatccccgcataaaccggaacattaatctccagtttctggcaaacattcaggccattaattaatgttttatcaagcgtctgattacccgctacaatagtgatgcctaataaatctattgccggatgtttcgccgccatcattatagcaatagcatcatcatgacccggatcacaatccagaataatttttctcttttccattgtttatttcctctgtttccagttgcgttattttttctacagcaaagaaaattcgaccgggccgatgattgaatcttaacaacagcgtacgtatgctaaatatgagaaatctcatagcggataaacatcgtgaaagaaatccacaataatgatcttaagcagcaattgatgagtgaatccgcgtttaaggattgctttttaacggatgtttcagccgatacgcggctgtttcattttttagcgcgtgactacattgtgcaggaagggcaacagccgtcctggctgttttacctgacgcgaggccgcgccaggctttacgccacgctagctaatggtcgcgtgtcgctgatcgatttctttgccgccccctgttttattggcgagattgagttaatcgataaagaccatgaaccgcgtgcggtgcaggctattgaagagtgttggtgccttgcgctccctatgaaacattaccgtccgctgttattaaacgacacgctatttttacgaaaactctgcgtcaccttaagtcataaaaattatcgtaatattgtttctttaactcagaatcaatcatttccgttagtgaatcgcctggcagcatttatattactctcgcaggaaggtgatctttatcacgaaaagcatacgcaagcggcagagtatttaggcgtttcttatcgacatcttttatatgttctcgcgcagttcattcacgacggtttattaattaaaagcaagaaagggtatctcattaaaaacagaaagcagttgtcaggactggcgctggagatggacccggagaataaattctccgggatgatgcagtaaaaattattttcaatagcgcgattgccggatgcaacgcttaatacgttttatccggtctacaaatcgagcattacgccagaccaataaagaacccggcaatagtcgcactcatcaggttggaaagcgttgctgctgccagcgcccgtaaaccaagctgggcgatttccggcgcgcgttttggcgaaatagccgaaaatgcgccaacgacaacaccgatagaaccaaagttagcaaaaccacaaagcgcaaaggagataatcgcaatggttttcacttccagcgtgccgcccgtttgcaggtatggggagaaactcaggtaagcgacgaattcgttaatcgccagtttctgcccaatcaggctacccgcaagattggcatcactccagtccacacccatgatccacgccagcggtgccagcacatagccaaaaatactttccagagaggcattggcgaaaccaaaccagccgccaattccgccgataatgccgttgatcagcgcaataattgcgacaaacgccattaccaccgtcgccacaccagcggcgatttttagcccggtcatcgcaccgctcgccgccgcttcgataaagctttttggcggcgtttcgctgaacgacagattttcaaatgtgacctgcgaaggctcggttgccgggctaagaatacgtgcaaacaaaatcccgccagggatcgccatcagcgatgccgctaacaggtagtcaattggtacgcccattccggcataaccaatcatcatcgaaccagcaatggacgccatcccgctacaaattgcggtaaacaactcgttgcgattcatgcgatcgataaacggtttaacgatcgccgggatctcattttgcccgaggaaaatagtagtaaccgcaacaaaagattcgattttgctgatgttgagggctttctggaaaatgctgccaaggatgcgaatcagcagccccatcacgccaatgtagtacagcagactgatgagcgcagtaacgaaaataatcgccggaagtacgcgaaaggcgaagataaaacccgcaccgtcaaacaggacatccattttcggcccaaccagcgaaccaaaaatgaaggcgctaccggcatcactgtaagacatcactttatgaacgcctaatgccgcctgttctactgcccattttcccggtgggaagtagagcatgatgccaccaatagcgatttgcagcagcagtgcggctccaaccgtgcgcaaactgatgctctttttattcactgacaacagaaatgctattgccagtaacaccaccatccccacaacacttctcattatatccataatgattttcccttcatgccggtaaacccggcgtcagcgccaggttttggtatgcttgatgagtacgggcgacggctttctgcccgtcagaaattaacccgcgagacgctgatattctttggcaatttcgctcgccagaatggcgttgttgaacaccagctggatgttggatttcaggctgtcaccgccggtcagttcagcaacgcgcgccagcaggaatggcgtactttctttaccaatgactccctgagcttcagcttcagctaccgcctgatcgatcgccgcattgatagtgtgttccggcatagcaaactgttccgggatcgggttcgctaccacgaggccaccgttcagaccgctttgccatttcaccaccattgcacgggcaatttcgctggcgctgtcgagacgaatgctgacgtcaaacgggctggtgcggcagaaaaacgcaggcagcgctttagtctgatagccaattaacggcacaccgaaggtttctaaatactcagtggttaatcctaaatcgagaatagatttcgccccggcacaaacaacggtgacattagtatttgccagttcttgcaaatcggcagaaatatcgaaggtatgttccgccccgcgatgcacaccaccaattcccccggtggcaaatactttaattccggcaagcgccgcaataatcatcgttgaagccacagtggttgcgccattttttccggcggcaacaacaaaaggtaaatcgcgacgactaactttggtcacgttatgcccttcacgacccagtaattcaatttcttctttgcttaaccccactttcatcacgccgccaataatggcgatcgtggcaggtacagcgccctgtttacgaatagtttcttcaacttcaattgcggtctgggcattttgtgggaacggcatcccgtgagaaataatggtcgattccagcgccacaaccggttttttgttttttaaagcgtcctgcacttccggggaaatttgtaataattcaggggaaatttttaattcagacattctgcgttctccactaacgatataacgttggcaatcgataaatcggggttattggtgtattcacaggagagcgccattgacgaacatccctgtgcgaaacgaacagattcggcaaacggcattccgtctacccaacacgaagcaagtcccgccatcatggcatcgcccgctccggtaacattaataacattggttttgatcggcgcagaccagccactttcaccgctgatatcgctgtaataaacgccgtcgccgcccatgctcaataccagtcggttcaggccatgttgatggaaccaggcagcaacttttgccacatcttcacgccctgacagcgcaatcccactcagggtttccgcttcaaggcggtttggcttgagagtgtggatctgatttagacggtcgcgcactttgacacatttccatgccgaaaccggatcgacaaatacgggtacgttggcggcattatccagaatccatgccagtgcctcttcactgatattacagtccgcgacaatgacctttgccctctgaataaattcaccgtgctgtgcgagatattcagctgtaatagcgttgctaatattcatgtcatttatagcaaccagcatttcaccggtattatcgagtaatgataaataactcgacgtattttctcccggcacaatcaggcatttatcgacataaacgccagattgattggtttgcgttagcagcgattgaccataaaaatcactgcctacggcgctcagtagccaggctttgttacccagcaacgccaggttttgtgcaatattgcgccctactccaccaggcgtaaattttattttacctggatttgaatccgcataatttaatgattcatgtgaatatccggcgacatcaatattcgccgaacctataattacgacataatccttttcgcgcatagcacgtcctctggtaaaaaattaccaaccctgtcaatccacaagaatatagatactgcaaagacggtttaaacatgtgttcatatttaaacatgtgctcatagtatgcatgttttacgtaaagtaaattaccgccagagaggcaaaatgggcagatttgagcaggctcacaaaatgcgattaaatgcctgaattacaaaagcgaggaatttgtgacgggatgcacagaacagaacaataaaaaagggcagaaaataatctgcccttgaggaaataacctgagtgtttgatgaacgtttgaagtttctactgaaagataaaaccatttaaattcataaaattacattcacaaaccggtcattctctttgcgctcatcaaatgttacaggacaggaaatttctgccctgtaacacaccttttattacgctgctttcgctactgcgtccacttccggacgtttcaggaaggcataggccaaacccgccaccagcgtaccggcaataattgctaccaggtaacccaataccggcgtaatagcgccagggatcagcagaacaaacagaccaccgtgcggtgccatcagtttcgcaccaatcgccattgagattgcgccagtcagcgccccacccacgatacagcacggcagcacacgcatcggatcacgagcagcaaacggaattgcaccttccgaaatgaagcacagtcccaataccagagcggctttgccaccttcctgctgcgctttgtcgaatttgcgacgcgccaccattgttgccagacccattgccagcggtggcaccatacctgccgccataatcgccgccatcgggccataggtttgagtactcagcagacccacaccgaatgcgtacgctgctttgtttaccggaccgcccatgtcagtacacatcatgccaccgaggatcgcccccagcagaaccgcattcgcagtccccatggtctgcagccagtgagtcagcccttcgagaatgccagcaactggtttaccgatcaggtagatcatcgccagaccgaccaccagactggaaattagcggaatgatcaggatcggtttcagcgcctccatactctgtggcagtttcaattgcgtactgattaacttcgcaatgtaaccagccaggaagcccgcaataataccaccaatgaagccagaaccggtgctgaccgccagcataccgccaatcagacccggagtgaggcccggacgatcggcaatggaaaaggcaatataacctgccagtaccggcaccatcagcgcaaaggctgaaccaccaccaatctgcatcagcgccgcagccaacgtacccggctctttaaacgcttcgataccaaaagcaaaagaaagcgcgatacacagaccacctgcaacgaccatcggcagcatgtaagaaacgcccgtcagcaagtgacggtatgcgcctgcactctctttcttactttcagtggtcgccgtttgagctttgcccgccggttcatacggcgttgcttcagcaaccgctttatccagttcctgcgcggttttcttcagcgccagaccggtagaggtacgatacatcggtttaccagcaaatttcgccagatccacttcgatatctgccgccacaatcaccagatccgctgctgcgacttcttcgggagtgattgcattacccgcgccaacagaaccacgggtttcaactttcacccaccagccacgttttttcgcttcggtttcaatggcttcagccgccataaaggtgtgtgctacgccagtcgggcaagcagtcaccgcaactacgcgtttcggaccgctggcggcaactggtgctgtcgcagcgaccggcgcagtgtaaggtttcgcatggcctttggcttcactcaggaacagctcagggtgcgcaactgcccgggaaatatcgcccagccagacatttttaccgttcagcgcgctgtcgttcgggatggaatcaccgagaacaatcgccatttcagcgtcgttcggattgtcgatgatttccagttttgcttttcgcgccgccgcgcccagcagggtcttcgccatataggcgcgtgcctgaccgagattagcgtcaataatcagcagcgttttcattatgcctctcctgctgtcagttaaaaggttgtaagtcgacgcgcgccatcattgcggccaactgcggacgatcggtaatacccacattgctttgacttaccgccagggctgcaacagctgtcgccagacgcagtgtgtgttcactggattcacgcatcagcaagccataaatcaggccaccaaccatagaatcccctgcgccaacggtgcttacgacatcgactgacggtggtttggcgatccattcgccggaggcattaacccaaagcgcgccttcggcacccagtgaaataacaacatgcgcgatgccttgttcacgtagcgcatgtgcagcttcaatcacatctttcatttcaggcagtttacggcctgcccagatttccagctcgcggcggttaggtttcaccagccacggtgccgctttcaaacctgctactaacgcttcacggctactatcaaagataatgcaaggacactgactacgcaggcgagtcatccagtcggtgaacgcttccgggctgacgcctgacggtaagcttccgctgacacagaccatatcgaactgaccgagccagctcagagaatcagtcacaaagcgttcccagtcggcgggggtgacttcaaaacccgagaagttgaagtcggtcacttcgccgtctttttccgtcagcttaacgttaattcgggtgcgcccctgtacaacctggaaacggttggcaatgcccagctcgctgaacagttgctgaaaaccatcctgattgtctttacccaggaagccgccaacggtgacatcaattcccaggtcttttaatactttggccacgttgatgcctttacccgccgcatgcagaccggtggttttcaccaggttcacttcgccgcgttcaatttccgggcagaaaccaacaaggtcataagccggattaagggtgatagtagcaacacgtctgctcattatgcgccctccccaagaccagcagcgatagcgtcgccgattgctttcagcgcctgttcagcatctgcaccctgggcggtaaagcgtaggcgatgacctttcttaacgccaagtgccacaactttcatcagactacgtccgtttgccggtttgccggtaccatcaaggtttgtcacggtaatatcactgttaaattgtttaatggtattgaccagcatggtacctggacgagcatgcaggccgtgttcattgcgcaccacaaactccgcgcttaacacgtcgtcggtcggcgcatcatcgctggtcagcagcgccagcaacgttgccgcatccgctttcagcaagcggtcagctttattgtcgagcaataaatcagcgagacgcttaagaaccgcgatgggctgatcgtcattcatcgccacactcaccagcatggctgccgtttcgccgtccacatcaaaagcatttgccgcacggcttaccgcaatcgcgctacgcagattgccttcggcgctatcgctcagccagataccctgtccgagattcagcggttgttcattgatggctttggtgacgaaagtggcgtcaactgcccccgcctctttcagacgcgcagcgttcagcgcctgaagagtcagcagatcgctggcgacgatatccagtgtcagcatttcgttgtcgagcttcagctgctcactctgcttttcgcccatcagtaatgcgcgaagttcttctgctgttgttgctgacttcagttgttcagcaacggaatcatcgctcagtacgtgggtcagctggcgtagcaggcccagatgttcatccgagctggcagcaataccgattgccacgtacgctacctgaccgtcaccccaggtgacgccttccgggaactgaaatacctgaacgccggttttcagcacctgatcgcgggtgtcggtagtgccgtgtggaatagcaataccattgccgaggaacgttgaggtttgctgttcgcgcgccagcatgccattgacgtagccttctgctacattaccggcctgcaccagcgccgcagcgacctggcgaatcgcctcttctttgtctccggccttttcgcccggatggatgtcctgtacggataactggaacatagttctcctctcttgctgaattgaaacgattcagcctctatgagaaaaaaagcgccaacctggcttagggttaaagacaagatcgcgctgaaacgtttcaagaaagcataatacttctgtttcagcacgcaaggaaagccgtaaagttatgagcaaaagtttgatgtgctgcacaattttttgccatttttcctaattgctgatgggaaaatccgttatcagcaatttcatttcagcagcgtcagcagccaatcagcaacagtgaaatggcattttgactattcgtggcgcttttgatttcgctgtctgtttattttctgacaagcagcgtaaactccgcgtcttcctcttccagtgatcgaccagcatgcataactcccccgcagtctccagcgcgaaatcgtttgacctgacctcgacggcgtttttaatcgttgcctttctcaccggtattgcgggcgctctgcaaaccccgacactcagtatttttcttaccgatgaagtacatgcccgtccggcgatggtgggattcttctttaccggcagcgctgtcattgggattctggtaagtcagtttctcgccgggcgctctgataagcgcggcgatcgcaaatcgctgattgtcttttgctgcctgttaggcgtgctggcctgcaccctttttgcctggaatcgcaactactttgttttgctattcgttggcgtctttcttagcagctttggctcgaccgctaacccgcaaatgtttgcccttgcccgtgaacatgccgacaaaaccggacgtgaggcggtgatgttcagctcttttttacgcgctcaggtttcactggcatgggtcattggcccaccgctggcttatgccttagcgatgggtttcagctttacggtaatgtatctgagcgcagcggtagcgtttattgtttgcggtgtgatggtgtggctgtttttaccgtcgatgcgaaaagagcttccgctggcgaccggcacgatcgaagcgccgcgccgtaaccgtcgcgatacgctgctgctgtttgtcatttgtacattgatgtggggctcgaacagcctgtacatcatcaacatgccgctatttattatcaacgaactgcatcttcccgagaaactggccggtgtgatgatggggaccgccgccgggctggaaatcccgacgatgttgattgccggatatttcgccaaacgtctgggtaagcgtttcttaatgcgcgttgctgccgtgggtggcgtctgtttttacgcaggaatgctgatggcgcattcacctgtcattctgttgggcttgcagctgctaaatgctatttttattggcattctgggcggcatcgggatgctctattttcaggatctgatgcccggtcaggcgggttcagccaccacgctctataccaacacttcgcgcgtgggctggatcatcgcaggatcagtggcgggcatcgtcgccgagatctggaattatcacgctgtgttctggtttgcgatggtgatgattatcgccactctgttttgcttactgcggattaaagatgtttaaggcgcggtcagcatttccagatcgataagccaggtcatggcctgctgacgcgagttaccgcacatttcagcgctggcttgtaagcctgcacagactttcggtcgcagtggcgaggtgaaaattttacagcgttgctgttcatcaagctgaatgcagggcgtattggcgggcttgccatctggcataccgggaatagggctggaaattgaaggggcagtgcaacacgccccgcaacccggacggcattccatacgttgttctcttaaggttaaccaccggattgatgagcgcgcacagtaccaccttttttgcaccagcaaaagtgcgaataccacttgcccgaaaggcccgtcgcgagtactttgtcgcgatatttttgacattttcgactacaggaatttttcgatgccaagagcgaacgaaattaaaaaaggtatggtactgaattacaacggcaaactgctgctggttaaggatattgatattcagtcgcccactgcccgcggtgccgctacgctgtacaaaatgcgtttttctgatgtccgtaccgggctgaaagtagaagagcgtttcaaaggtgatgatatcgttgacaccgtgacgctgacccgccgttacgttgacttctcctatgtcgatggcaacgaatatgtctttatggataaagaagactataccccgtataccttcaccaaagatcagattgaagaagagttgctgtttatgccagagggcggcatgccggacatgcaggtgctgacctgggacggtcaactgctggcgcttgagctgccgcagaccgttgatctggaaatcgttgaaaccgcaccaggcatcaaaggggcatctgccagcgcccgtaacaaaccggcgacattgagcactggtctggtgattcaggtaccagaatacttaagcccgggcgaaaaaattcgtatccatatcgaagaacgccgttatatggggcgtgctgactaacttcagccgcatgcagaaaagggatagctcaggctgtcccttttttaatttattataccaatcttctattttgcgcttcctgaacaccttacgccctcaattttcactcgttgattgatcgccctcacacttcatcgcattaacaatccagaccaatttcaattgctgtcatataactttacactgtcgttgttaattaatcgttactaagacgtgactcctatgaatacaatcgcctccgttacgctcccgcatcatgtacacgctccacgctatgatcgccagcagttgcaatcacgtatcgttcattttggctttggagcctttcaccgcgctcatcaggcgttactgaccgatcgtgtgctgaatgcccagggcggcgactgggggatctgtgaaatcagcttgttcagcggtgatcaactgatgagccagctccgcgcacagaaccatttatataccgtgctggagaaaggtgcggacggcaatcaggtgataattgtcggtgccgttcacgaatgccttaatgcaaaactggattccttagcggcaattattgagaaattttgcgagccacaggtggcaattgtttccctgacgattaccgaaaaaggctattgtattgacccggccaccggtgcactcgacaccagtaatccgcggattattcacgatctacaaacccctgaagaacctcactccgcaccgggtattctcgtcgaagcactgaaacgccgccgtgagcgcggccttacaccgtttaccgtgctctcctgcgacaatattcccgacaatggtcatgtggtgaaaaacgcggtgctgggaatggcagaaaaacgttcgccagaactcgccgggtggataaaagagcacgtcagttttccgggaaccatggtcgaccgcattgttccggctgcaaccgacgaatcactggtggaaatcagccagcatctgggggtgaatgatccctgcgcgattagctgcgaaccgtttatccagtgggtggtggaagataacttcgtcgctgggcgtcctgcctgggaagtcgcaggtgtacaaatggtgaatgatgtcctgccatgggaagagatgaaactgcggatgcttaatggcagccactcttttctcgcttatctgggttacctctcaggattcgcccatatcagtgattgcatgcaggatcgcgcatttcgccatgccgccagaacattaatgctggatgagcaagcgccgacactgcaaattaaagatgtcgatttaacacaatatgcggataagttaattgcacgttttgctaatccggcgctgaaacataagacctggcaaatcgcgatggatggcagccagaaattaccgcaacgcatgctggcaggtattcgcatacatcaggggcgcgaaacggactggtcgttgctggcattaggcgttgcaggctggatgcgttacgtcagcggcgttgatgatgccggaaatgccattgatgttcgcgatccgcttagcgataaaattcgcgaacttgttgcgggcagcagcagtgaacaacgcgtaaccgccctgctttccctgcgtgaagttttcggtgatgatctgccagataacccgcattttgtgcaggccatcgaacaagcctggcaacaaatcgtacaattcggcgcacatcaggcgctattaaacaccctcaaaatttaacgatttctgcggttaaagcggatgaagctcaccttcgtccgctctccccttctcttttctgccttttttagccaggattaacgctcagttaacttaccagagtattgcggagccgttgtgaccaggaccaacctcatcaccggttttctcggcagcgggaaaaccacgtcgattcttcatctgttagcccataaagatcccaacgaaaaatgggcggtactggttaatgaatttggggaagtcggaattgatggtgctttgctcgccgatagcggcgcattgctgaaagagatccccggcggctgcatgtgctgcgttaatggtttacccatgcaggtagggttgaataccttactgcgtcagggaaaaccagaccgcttgttgatagagccgaccgggctgggccatccgaaacagatcctcgatctgttaaccgcaccagtctatgaaccgtggatagatctgcgcgccaccttgtgcattctcgatccgcgcttgctgctggacgaaaaaagcgccagcaatgaaaacttccgtgaccagctggctgccgcagacatcattgtcgccaataaatccgaccgtacgacgcccgaaagtgagcaagcgctacagcgttggtggcagcaaaatggtggcgatcgacaattaattcacagtgagcatgggaaagttgacggtcatcttctggatttgccgcgtcgcaatttagccgagttgcccgccagcgccgcgcattctcatcagcatgtcgtgaaaaaagggttagcagcgttaagcctgccagagcatcaacgctggcgtcgcagtctgaacagcgggcaaggatatcaggcctgcggctggatattcgacgctgatacggtattcgacaccattggcattctggaatgggcgcgacttgcaccggtggaacgcgtcaaaggcgtgctgcgtattcccgaagggctggtgcgaatcaaccgtcagggcgatgacctgcacattgaaacgcaaaacgttgcgccaccggacagccgtattgagctgatttccagcagcgaagctgactggaatgccttgcagagcgcgctgttgaagcttcgtttagcgactaccgcgtaaggttgcctgcgtttttcagtaagataattagagaaaatatgattaaaaatttgccgcaaatagtgttgttgaatattgtcggcctcgcgctgtttctttcctggtatatccccgttaatcatggattctggttgccgattgatgcggatattttttatttctttaatcagaaactggtcgaaagtaaggcctttttgtggctggttgcattgaccaacaatcgcgccttcgacggttgttcactgctggcgatgggtatgttgatgctgagtttctggctgaaagaaaacgcccctggcagacgacgtatcgtgattattggtctggtcatgctattaactgcagtggtattaaaccagctgggtcaggcattaattcctgtaaaacgggccagcccaacattgacttttaccgatattaaccgcgtcagcgaactgctctctgttcccacgaaagatgcctcacgagatagctttcccggcgatcacggcatgatgctgcttattttttcggcattcatgtggcgttatttcggcaaagttgcaggccttatcgcccttattatttttgtggtttttgcatttcccagagtaatgattggcgcacactggtttactgacatcattgtcggttcgatgaccgtgatattgatcggtttgccctgggtgttgctgacgccattaagtgatcgattaatcaccttttttgacaaatcactaccaggaaaaaacaaacatttccaaaacaaataactcacagtaattaacatcatcagggttatttttatagtgaggataatcctgatgatgcgcaccgtgctttcatctatcgaacgcaaaaatcattctctaagtaaatgaatggattgcatgcgtttcactcaattgtactttaattgaccaaccccgcttattaactttctgtatcactttttcttataaaaaatcatgtaaaaccgctcgccaagaccgcaccaatcgggtaatctcgaactcgttttgcctcggcggtagattatcctcacagcatataattttgtgcgttagtccacagatttggccttaaggaattgtttcaacatgcccaggtaattagtctcgtgtcgcttggcatttttttataacgatatttgtcgttaaggacttcaagggaaaacaaacaacatggtcaaatctcaaccgattttgagatatatcttgcgcgggattcccgcgattgcagtagcggttctgctttctgcatgtagtgcaaataacaccgcaaagaatatgcatcctgagacacgtgcagtgggtagtgaaacatcatcactgcaagcttctcaggatgaatttgaaaacctggttcgtaatgtcgacgtaaaatcgcgaattatggatcagtatgctgactggaaaggcgtacgttatcgtctgggcggcagcactaaaaaaggtatcgattgttctggtttcgtacagcgtacattccgtgagcaatttggcttagaacttccgcgttcgacttacgaacagcaggaaatgggtaaatctgtttcccgcagtaatttgcgtacgggtgatttagttctgttccgtgccggttcaacgggacgccatgtcggtatttatatcggcaacaatcagtttgtccatgcttccaccagcagtggtgttattatttccagcatgaatgaaccgtactggaagaagcgttacaacgaagcacgccgggttctcagccgcagctaataaaccgtttggatgcaatcccttggctatcctgacgagttaactgaaagcactgcttaggcagtgcttttttgttttcattcatcagagaaaatgatgtttccgcgtcttgatccaggctatagtccggtcattgttatcttttaaatgttgtcgtaatttcaggaaattaacggaatcatgttcatacgcgctcccaattttggacgtaagctcctgcttacctgcattgttgcaggcgtaatgattgcgatactggtgagttgccttcagtttttagtggcctggcataagcacgaagtcaaatacgacacactgattaccgacgtacaaaagtatctcgatacctattttgccgacctgaaatccactactgaccggctccagccgctgaccttagatacctgccagcaagctaaccccgaactgaccgcccgcgcagcgtttagcatgaatgtccgaacgtttgtgctggtgaaagataaaaaaacattctgttcatctgcgaccggtgagatggacattccactcaatgaattgattccggcgctcgacattaataaaaacgtcgatatggcgatcttacccggcacgccgatggtgccgaacaaacccgcaatcgtcatctggtatcgcaaccctttgctgaaaaatagcggcgtctttgccgctctgaatctcaacctgacgccttcactcttttatagttcacggcaggaagattacgatggcgtcgccctcattattggcaatactgcgctatctaccttttcttcacgtttgatgaacgttaacgaattaaccgacatgccagtccgtgaaactaaaattgcgggcattcctctgaccgttcggctttatgcagatgactggacatggaacgatgtgtggtacgcatttttactgggcggcatgagtggaactgtcgttggcctgctctgctattacctgatgagcgtacgtatgcgccccggcagagaaatcatgaccgccatcaagcgcgaacaattttacgtggcgtatcaaccggtggtggatacacaagctttgcgagtaacgggcctggaagtactgctacgctggcggcatcctgtcgcgggagaaattcccccggatgccttcattaactttgccgaatcgcaaaagatgattgtgccgctgactcagcacctgtttgagttaattgcccgcgatgccgcagaattagaaaaagtgctgccggtaggcgtcaaatttggtattaacattgcgccggaccatctgcacagcgaaagctttaaagcagatatccagaaactgctcacttccctgcccgcacaccatttccagattgtgctggaaattaccgagcgcgatatgttgaaagagcaagaagccacacaactcttcgcctggctgcactcggtcggcgtagaaattgctattgatgacttcggcaccgggcacagcgcgcttatctatcttgagcgttttacgctcgattatctgaaaattgaccgtggatttatcaacgccatcggtacggaaacgatcacttcccccgtacttgacgcggtgctgacgctggcgaaacgcctcaatatgctgacggttgctgaaggggtcgaaacgccggaacaggcgcgatggctaagcgaacgcggcgttaatttcatgcaaggctactggattagccgcccgttaccgctggacgattttgttcgctggctaaagaaaccgtatacgccgcagtggtaaggtgtgcttacgtcccttattattcatagtgaaagcatgccggattgcggctaatgatgagtaaaaggaaatccgttgcagatgattgtgcgcatactgctgctgtttatcgctctgttcacctttggtgtgcaggcgcaggctatcaaggaaagctatgcctttgccgtgctgggcgaaccccggtacgcgtttaatttcaaccattttgattatgtgaaccccgccgcgccaaaaggtgggcagataacgttgtcagccctcggcaccttcgataatttcaaccgctatgcactgcgcggcaacccgggcgcacgcaccgagcagctgtacgacacgctatttacgacttccgatgacgaaccaggcagttattacccgctgattgctgaaagcgcacgctatgctgacgattattcctgggtggaggtcgctattaatccgcgcgcccgttttcatgatggttcgcccattactgcccgcgatgtagagtttacttttcaaaaatttatgaccgaaggcgtgccgcaatttcgtctggtctacaaaggcaccaccgtcaaagccattgcaccgttaaccgtgcgcattgagttagctaaacccggcaaagaagatatgctgagtctgttttcgctgccggtatttccagaaaagtactggaaggatcacaaacttagcgacccgctcgccacgcctccgcttgccagtggtccgtaccgcgttacgtcctggaaaatggggcaaaatattgtctattcccgtgtgaaagattactgggcagcaaacttaccggtaaaccgtggacgctggaatttcgacaccattcgctacgattattacctcgatgataatgtcgcctttgaagcgtttaaagcaggtgcctttgatttgcgtatggaaaacgacgccaaaaactgggccacgcgttataccggtaaaaatttcgataaaaaatacatcatcaaagatgagcaaaagaacgaatcagcccaggatacgcgttggctggcgtttaatatccaacgtccggtattcagcgatcgccgggtccgggaagctatcactctcgcctttgactttgaatggatgaacaaggcgttgttttacaatgcctggagtcgcacgaacagttattttcagaataccgaatacgcggccagaaattaccccgacgccgcggagctggtgcttctggcaccaatgaaaaaagatctaccgtcagaagtcttcacacaaatctaccagccgccggtatccaaaggcgatggctacgatcgtgacaacctgttaaaagccgacaaacttctcaacgaagcgggctgggtgctgaagggtcagcaacgcgttaatgccacaacgggtcagccactcagctttgaattattgcttcccgcaagcagcaatagtcagtgggtattgccgttccagcacagcctgcaacggctgggtatcaacatggacattcgcaaggtggataactcgcaaatcactaaccgcatgcgcagtcgcgactatgacatgatgccgcgcgtatggcgggcgatgccgtggcccagttccgatttacagatttcctggtcatcggaatatatcaattccacttataatgcccccggcgtgcaaagcccggttatcgactcgctgatcaaccaaattattgccgcgcagggaaataaagaaaaattactgccgttggggcgagcactggatcgcgtattaacgtggaattattacatgctgccaatgtggtacatggcggaagaccgtctcgcctggtgggataaattctcccagccggccgtgcgccccatctatagcctcggtatcgatacctggtggtatgacgtcaataaagcggccaaactgccgtccgccagcaaacagggagagtagatgggcgcttacctgattcgccgtctgttgctggtgatcccaacattatgggcgattatcaccatcaactttttcatcgtgcaaattgcgcctggcggtccggtcgaccaggccatcgccgccattgagtttggtaatgccggagtattacccggcgcaggcggtgaaggtgttcgtgccagccatgcgcaaacgggtgtcggcaatatcagcgacagtaattaccgtggcggacgcggattagatccagaagtgatcgctgagatcactcatcgctacggttttgataagccgatccacgaacgttacttcaaaatgctctgggactacatccgctttgattttggcgatagcctgtttcgcagcgcctcggtgctgacgctgattaaagacagtctgccggtttccatcaccctcggattgtggagcacgctgattatctatctggtgtcgattccgttaggcattcgcaaagctgtttataatgggagccgctttgacgtctggagtagcgcatttatcatcatcggctacgccattccggcctttttgtttgccatcctgctgattgtcttcttcgcgggcggcagctatttcgacctgttccctctacgcggcctggtttccgctaactttgattcgctgccgtggtatcagaaaatcaccgattatctgtggcatatcacgctgccggtgctggcgacagtgattggtggctttgcggcgctgaccatgctgacaaaaaactcattccttgatgaagtgcgcaagcaatacgtggtgaccgcgcgtgcgaaaggggtaagtgaaaaaaatattctctggaaacatgtgttccgcaacgccatgctgctggtgattgccggttttccggcgacgtttatcagcatgttttttaccggctcgctgctgattgaggtgatgttttcactcaatggtctgggcttactgggctacgaagcgaccgtctcgcgcgattatcctgtaatgtttggtaccttgtatattttcaccctgattggcctgctgctgaatattgtcagtgatatcagctatacgctggttgatccgcgtattgattttgagggacgttaatgtcgcgactcagccccgtcaatcaggcccgttgggcgcgttttcgtcataaccgtcgcggctactggtcgttatggattttcctcgtcttgtttggtttgagtttgtgttctgaacttatcgccaacgataaaccgttgctggtgcgttatgacggcagttggtatttcccgttattgaaaaactacagcgaaagcgattttggcggcccgctggcaagtcaggctgattatcaggacccgtggctgaaacaacggctggaaaataacggctgggtactgtgggcaccgattcgctttggtgctaccagtatcaactttgctaccaataagcccttcccttctccaccctcccggcaaaactggctgggaacggatgccaacggcggcgatgtgctggcacgcattctctatggcacgcggatctcggttctgtttggcctgatgctgactctctgttccagcgtgatgggcgtgctggcgggggcgctacaaggctattacggcggtaaagtcgatctctggggacaacgctttattgaagtatggtcggggatgccgacgctgtttttgattattttactttccagcgtcgtacagcctaacttctggtggctgctggcaattactgtcttgtttggctggatgagtctggtcggcgtggtgcgggcggagtttttacgtactcgtaatttcgactacattcgtgcggcacaggcgcttggcgtcagcgatcgcagtatcatcctgcgtcatatgttgcctaatgccatggtcgcgaccctcacctttttaccgtttattttatgtagttcgataaccaccctgacctcgctcgatttcctcggcttcggtctaccgctcggttcaccgtcactcggtgaactgctgttacaagggaaaaataaccttcaggccccgtggcttgggatcaccgccttcttgtcggtggcgatattattgtctttgctgatctttattggtgaagccgtccgcgacgcatttgatcctaataaggcggtgtagcatgacgcaaactctgttagcgattgaaaatttgtcggtgggttttcgccatcagcaaaccgtacgtacagtagtcaatgatgtttcactacagattgaggctggcgaaacgctggcgctggtgggtgagtcaggttcaggcaaaagcgttaccgcgctgtcaattttacgcctgctcccttccccgccggttgaatatctctccggcgatattcgttttcatggcgaatcgctgcttcacgccagcgatcaaacgttgcgcggtgtacgcggtaataagatcgccatgatttttcaggaaccgatggtgtcgttaaatccattgcataccctggaaaaacagctttatgaagtgctttcactccaccgcgggatgcgtcgggaagcggctcgtggcgaaattcttaactgccttgatcgcgttggtatccgccaggcggcaaaacggctgacagattatccgcatcagctctccggcggcgaacggcagcgggtgatgattgcgatggcgctgttaacgcgaccggaattattaattgccgatgaaccgaccaccgcactggacgtctctgtccaggcgcagattttacagctgttgcgcgaactgcaaggcgagctgaatatgggcatgctgtttattactcataacctcagcattgtcagaaaactggcccaccgcgtggcggtaatgcaaaacggtcgctgtgtcgagcaaaattacgccgctacgctatttgcatcacccactcatccttacacacaaaagctactcaacagtgaaccgtcaggcgatccagtgccgttgccagaacctgcctcaacgttgctggatgttgaacagcttcaggttgccttccccattcgcaaagggattttgaagcgcattgtggatcataatgtggtggtgaaaaacatcagttttacgctacgagcgggtgaaacactgggtttagtgggcgagtccggttccgggaaaagtacgacgggactggcgctgctgcgactgattaattctcagggcagcatcatctttgacggtcagccactgcaaaatttaaatcgccgccagctgttacctattcgtcatcgcattcaggtggtatttcaggatccaaactcctcgctcaacccacgactcaacgttttgcagattattgaggaaggcttacgggttcaccagccgacgctttctgccgcacaacgcgaacaacaagtgatagccgtgatgcatgaagtgggattagatcctgaaacacgccaccgttatccggcggagttctctggtggtcagcgacaacgtattgcgattgccagggcattaattcttaagccctcgctgatcatacttgatgaaccgacatcatcactcgacaaaacggtacaggcgcaaatattgacgctattgaaatcattgcaacaaaagcatcaactggcctatttgtttatcagccacgatttgcacgttgtccgcgcgttatgtcatcaggttatcatactgcgacaaggggaagtagtggaacaaggaccgtgcgcgcgcgtgtttgccacaccgcagcaggagtatacgcgtcagctactggcgttgagctgacgcttaaaaaggattgtagtttgaaaagggttcggcaattgccacaccaaaatttttcaatcggcatgttgcagcaaactcgtcctggcgatttacaaacaggcacggctcaccttcacactccagcaccgaacatggaacttcgatgtcgcttaacgcctggcttagtttatacatcaccgaccatgcattatcaccatccgggctaagcaatttaagcgccaccaggctgttgtcaccgcacggtccattttgcggaatcggttcaaccttcgaacctgcgaaaccagcagaccagcgatagttctgcggcagtcgatggacgattgagagttgtaatgaagtcacttattttccccggaagcacattcacttcacaatttgtttacatcaattttaacacatcatcaacaatccgtctttatacagatcgtaaagattgatgcctcgcctgcgtggcctctatggctctgatttaagtaatatctgcgggcgtggtcacgtttgcggggctatatgtacccgtttctgcgatctaactcaacctttttaactacaatgatgtgactttttacataaattgattttacataaaataaacatatatcgggggaatgatagatttgtggttgacatgcatcaacaaaggaagccttttagcttcctcgttgtgcaatagatcaccgttttttcggccgactggcgtacagacagaagagaatggagctggttgcgcagaatgcaattgaccaaatcatcggccatgcagagttaaaggtcgcaagagaaagcaatgcgccaacaattgcccctatgccaaaacggaaggttcctgccagcgaagatgccgttcccgccatatggggaaactcatcaagaatgaccgccatcgcattggatgacaccatcgacacgcagcccacaaacgccgcaacgccaaccaccagcgaccaaaatcccagccccagcagcgcactgatgaccatccacgctgccataataaattgtatccacaaccccgagcggaacatatttaacgcgccaatgcggcggacgaagcggctgttaaagatggtcatcacgaacagaaaaacaatgtttagcgcaaagtaataaccaaagttttccggcgcgacgtggttaatttcaatataaacaaacggtccggcgcttaagaatgagaacatcccggcaaagctgaaaccactggcaagcatgtagctcaggacacgtttatggcggaacagcgccgcaaagttaccaatagtggtacgaatgtgaaatggctgacgacgctccggtggtaaggtttctttaatcaggaagaaaatcattgccgaagccagaatcgccgctaatgccaggatccagaagatgtaatgccagctcagccacaccagcacccagccgccaactatcggtgccatcagcggtgcaatggttgtcaccagcatgacaaacgacatcatccgcgagaactcttctttcgggtaaatatcgcgcatcagggcgttaatgaccacgctggccgcagccgcagccagcccgtggaagaaacgcatcacaatcagctgatcgatggtgtttgccaacgcacacgccaccgcggcggcggcaaacaccagcgtaccgccgagcaccaccggcttacgcccgaagctgtctgccatcggcccgtagattaactgccccaacgcaaagcccagaatataagtactgagggtcatctgcgtactgcccgccggtacgccaaactgcgctgaaattaccggtagcgcgggcagatacatatcaatcgacagcggcatcaacatggccagcaggccaaggataaaaacaatagcaaacgacgaatgctgtcgggtggtcacaacgggctcctgaaagtcattgaaaagttagacgacgctggcaatttcttcttcagttaacggacgatattcaccgggggctaaatcagcatccagcgtaataccgccaatacgttcacgatgcagctcaaccacgtggttacccacggcggcgaacatgcgtttcacctgatgataacgcccttcgctgatggtcagacgaacctgcgttggggtaatcacttccagcaccgcaggcttagtgagatctttttcgttatgcagctgcacgcctttagcaaattgctctgccgtatcgtcagctacaggtgattccagtgtcaccagataggtcttctcgcaatgatggcgcggagaagtaatgcggtgcgaccactgaccatcatcagtcatcagcaccagaccggtggtatcaatatccaaccgccccgccgcatgcagtttccacgctaccggttcatcaagaaaatagagcaccgttgggtgatcagggtcgtccgtggagcaaacatagccctgaggcttattgagcatgaagtaacgtggaccgtgttgctgcgccagcgggttgccatcgtaagcgacatcatgttcaggaagcagtttgaacgctgcattacggacgatttcgccatcgacggtgacacgattgccgcggatttcacgcccggcaatagcacggctaacgccgagttgctgtgcgataaatttatcaagtcgcatgtgtgtgattttgcctgtaaaaacggaggtcgggcattgacccgaaaatctgaactgttgtctgcccagtatagcggtctaataacatccctcaagggaaaaagatccatggcatactattagcagaataatctacctacgcgagaccatgatttttacacttcgcccatatcagcaagaagccgtggatgccacgctcaaccattttcgtcgtcataaaacccctgccgttatcgtgctgcccaccggcgcaggtaaaagcctggtgatagcggaactggcacggctggctcgtggtcgcgtgctggtgctggcacacgttaaagaactggtggcgcaaaaccatgcaaagtatcaggcgctggggctggaagccgatatttttgccgccgggctaaagcgcaaagagagccacggtaaagtggtatttggcagcgtgcagtctgtcgcccgtaatcttgatgcctttcagggtgaattttcgctgttgattgtcgatgaatgtcaccgtattggtgacgatgaagagagccagtatcagcaaatcctcactcacctgacaaaagtgaatccccacttacgcctgctggggctgactgccacgccttttcgattgggcaaaggctggatctaccagtttcattatcacggcatggtacgcggcgatgagaaagcccttttccgtgactgcatttatgagctgccgctgcgttatatgattaaacacggctatctgacgccgccagaacgactggatatgccagtagtgcaatacgatttcagccgcttgcaggcacagagtaacgggctgttcagcgaagccgatctcaaccgtgagctgaaaaaacaacaacgtattaccccgcacatcatcagccagattatggagtttgctgcaacgcgcaaaggggtgatgatttttgccgcgacggttgaacacgcaaaagagattgtgggattactgcctgccgaagatgcagcactgattactggcgacacccccggcgctgagcgcgatgtgttaattgaaaattttaaagcccagcgttttcgctatctggtcaacgtcgcggtactgaccaccggatttgacgccccgcacgtcgatcttatcgccattctgcgccctaccgaatcagtgagtctttaccaacaaattgtcgggcgcggtctgcgtctcgctccgggcaagactgattgcttaattcttgattatgcgggtaatcctcacgatctctacgcgccggaagttggtacaccaaaaggcaaaagtgacaacgttccggtacaggttttctgccctgcctgcggttttgccaacaccttttgggggaaaacgaccgccgacgggacattgattgaacactttggtcgtcgctgtcagggatggtttgaagatgacgacggtcatcgcgaacaatgtgacttccgtttccgttttaaaaattgcccgcaatgtaacgcggaaaacgatattgccgcccgccgctgccgcgaatgtgacaccgtactggttgatccggacgatatgttaaaagcggcgctacgactgaaagacgcgctggtattacgctgtagcggcatgtctttgcaacatgggcacgacgagaaaggcgaatggttgaaaatcacctattacgatgaagacggcgcggatgtgagtgagcgtttccgtctgcaaacacctgcccagcgtaccgccttcgagcagctttttatccgcccgcatacgcgcacaccgggcatcccgctgcgctggatcaccgccgccgatatcctcgcccagcaagccttattgcgacacccggattttgtcgtcgcccgcatgaaaggccagtactggcaggtgcgtgaaaaagtgttcgattacgaaggtcgttttcgtctggcgcacgaattacgcggttaatggtagttttgattgatgtataaggcgattgagtatagaatctcgcccgcttttgcatacgcaaagcagatcacttacctgttgctgggtcgcctgtagcaggattaatttaagagagaaagaaatgtttactatcaacgcagaagtacgtaaagagcagggtaagggtgcgagccgccgcctgcgtgccgctaacaagttcccggcaatcatctacggtggcaaagaagcgccgctggctatcgagctggatcacgacaaagtcatgaacatgcaagctaaagctgaattctacagcgaagttctgaccatcgttgttgacggtaaagaaatcaaagttaaagctcaggacgtacagcgtcacccgtacaaaccgaagctgcagcacatcgacttcgttcgcgcttaattgctgaataagttgtaaaaaaccccgctccggcggggttttttgtatctgcagattatgcctgattacggtattgctattttttgcaggccagataaggcgttcacgccgcatctggcattcagaacacaaaaccgattaattgccgccagacgtccggcgctgcaattggtcgcgcaaattcggcggcgtgcctttaatggtcaaggtatcggttgctggatcccagaagatgcgttcacctaacagcatcgcatcaaagttaatagtcaagccaccgccgctaccggcaaacttcgtcaactgacgcagtgtgctacggtctgccgggaagctctcttccagttcgtagcctttttcagccgcaaactccgtgaagctcacttcgcttacgcctgccagctctttcgacagcgatttcagttcgatctcttcgcctgcctgcagctgctcattacagtagctataaacctgctggcgcacgttctgtcgctctgctttatccagttgtgcttcggcagtgaaatcatcaaccgcttgcaacagcccacggttttgcgctttcgcgtttaacccttcgctggccccgaggaaatccataaagaaatccgccactttgcgccctactcgccctttcaggaaagtgagatagcgggtggactctggattggtttcccattcggttaaatcgatacgcgcaacaatatccgcatgattgatatcaagataatgggttgggttgatgtcgagattttcgttaacgcgcatactgctcaggttgctcagaactgccaccagcaaatactccaccgccagatagcgatagtggcaaaacagcacgaatccaccgtcagcaaaaggatatttcgctaattcgtcacgcaggcggccggttgccgcgcggctaaatgccaggaagtcctcttcgccctgacgctgtaagcgcagcgtctgcgccagttcactctcttcgctaaacaagccgtaagctttatttttggcgctatagacccgatgcagttctgccaccatctcaacgacggtttctgtcggttccagcaatgaatcgcgcaacaccagctcaaggttctgctcatcacgcttgataagctggtgcagagcaatctggttgatatccagactcatgataaactctcctttaagaccgggcggtattcaaccaccgccggttaagcgacgcaataaaagatggcggtcattttacagaaggcagcgtaacgagaatgatttaacgcataaaaaagcagaaaaaaaaccgttgctacggtaatatgttgccctttcatcaactaactgatttcgatttatgccacaaatttcccgctacagtgatgaacaggttgaacaattgctcgcagagctgctcaacgtactggaaaaacataaggctccgaccgacctttccctgatggtgttaggcaacatggtcactaaccttatcaacaccagcattgccccggcccaacgccaggcaattgccaactcttttgcccgcgccttacagtcctctatcaacgaagacaaagcgcactaagggaaacagataacaggttatggtaactcatcgtcagcgctaccgtgaaaaagtctcccagatggtcagttgggggcactggtttgcactgttcaatattctgctttcgctcgtcattggcagccgttacctgtttatcgccgactggccgacaacgcttgctggtcgcatttattcctacgtaagcattatcggccatttcagcttcctggtgttcgccacctacttgctgatcctcttcccgctgacctttatcgtcggctcccagaggctgatgaggtttttgtccgtcattctggcaacggcgggaatgacgctattactgatcgatagcgaagtctttactcgtttccatctccatcttaatcccatcgtctggcaactggttatcaacccagacgaaaatgagatggcgcgcgactggcagctgatgttcatcagcgtgccggttattttattgcttgaactggtgtttgcgacgtggagctggcaaaagctgcgcagcctgacgcgtcgtcgacgcttcgcgcgcccgctggccgcattcttatttatcgcctttatcgcctcgcatgtggtgtatatctgggccgatgccaacttctatcgcccgatcaccatgcagcgcgctaacctgccgctttcgtacccgatgacggcgcgacgttttcttgagaagcatggtctgcttgatgcgcaggagtatcaacgccgtcttattgagcaaggtaatccagacgccgtttccgttcagtatccgttaagcgaactgcgctatcgcgatatgggcaccgggcagaatgtgctgttgattactgtcgatggcctgaactactcacgcttcgagaagcagatgcctgcgctggcaggttttgctgagcaaaatatttcgttcacgcgccatatgagctccggcaacactacagacaacggcatctttggcctgttctatggcatctcgccgagctatatggacggcattctgtcgacccgtacgcctgcggcattaattactgcgcttaatcagcaaggctatcagctggggttattctcatcagatggctttaccagcccgctgtatcgccaggcattgttgtcagatttctcgatgccgagcgtacgcacccaatccgacgagcagaccgccacgcagtggatcaactggctgggacgctacgcacaagaagataaccgctggttctcgtgggtttctttcaatggtactaacattgacgacagcaatcagcaggcatttgcacggaaatatagccgggcggcaggcaatgtcgatgaccagatcaaccgcgtgctcaatgcactgcgtgattctggcaaactggacaatacggtggtgattatcactgccggtcggggtattccactgagcgaagaggaagaaacctttgactggtcccacggtcatctgcaggtgccattagtgattcactggccaggcacgccggcgcagcgtattaatgctctgactgatcataccgatctgatgacgacgctgatgcaacgcctgctacatgtcagcacacctgccagcgaatattcgcaaggtcaggatttgttcaaccctcaacgccgtcattactgggttaccgcagcggataacgatacgctggcaattaccaccccgaaaaagacgctggtactgaacaataacggtaaataccgcacttacaacttacgtggtgaaagagtgaaagatgaaaaaccacagttaagtttgttattgcaagtgctgacagacgagaagcgttttatcgctaactgattaattataaatcagttagcgaaatatcttacttgcaatcggtgtggaaaacggtagtattagcagccacgagtcggcacgtagcgcagcctggtagcgcaccgtcatggggtgtcgggggtcggaggttcaaatcctctcgtgccgaccaaaaatcccaagaaaaaaccaacccttacggttggtttttttatatctgcaattaattcgataaacagaccgtgacacatcacagcctgtttattttctgttatcagaacgtccagaccacacccgcctgagtattccacggcgattctacccctgcgccattgccatagctgactgacaaatgaccgcttaacgtcggggtaaacgatgaccttataccagcctgataaacgccactggttccagccacatcattattaaatttgccatcgtcattaactttcacctggttagaatcggcgtattcctgacgcacggccgctttcagccagggttccagcgtcgtaccgttttgcaggtccatgtgatagcttaccgccgttcccgcttcagcgcgtaatatccgggtatttcccacatccgcgcgcatgccgtttgataacgtgtagtcctgaccatctgtggtaaagccggtaaaggccagatagggtctaacactccacaatccgtcaacccaacggaacccgctctcaacatgagcacccgcgccgttactattgtaatcgccaaacgctgttgccccattactcatcttgccatggatggtgttggcaaaacggtcaactttcaccaccccatcaacataggcaccgttctgatgctcccaaccggcataagcccccagggtatagctatcgatattacctttgccgccgcgatcaaaaccaatatcagaatgagagtaaccaaagatcaagccgcgaattgtactgctttcttcacgggagaaacggctatcgataccgagcgtcaggcccgtcaatgtttgctcaaaaccagctcccgcatcagtggtcacgttgttgcgggtgttaattgccgaactccacatcgccgtatcgtaactaacgccttttacgctaccaagacgctcacgcacggtgtccagttctgcatcaaataccagcggttgtgcggccgccatattcagcacatcagtggttgaaggggtaatttgcgcgcgattctctgccagactccagctatggttgccattatccagcaaggtatattcatacgtaccgatatcaacaacgcctccggcattgcccaacgtaaatgcagcatcaccgccgcccgttgttaccagtgtaaggctatctcctgctgccgggctggcaccggtgtccgtcacgaatattttgaaatcacctgttgcctgaccggtgacgttgagctgatcgctctgatgattagccatatcggtacgcatataaaaattgccgtttcccgacagggtattggtggtcaacgtaatgaaattttccgcacttgccgtcactgatgaacgagtcactggctcatccatcataatcacatttgcgtcagacatcgcaaggttggctaagttgaggagggtgttttggttcgtcgtagtgatatcggcaatgatggtccatacgctattttcgagcgaaacgtccgctttgctggtatccacggcaccatgcgttctaaaagaagcgccctcagaaaccactaccttacccaccaacattgcgggtgcataatttatttgcggcttcatgacctcaagaatgccatcattccctctgactgaaacgttaaccattgtgccagcccagacgttagcgcggccattgttgataaccatattttcagagatggcttttgaggaatacgtgatacttccattctgatatgatcgaccgagatcatataccgcatttgcctgcactttcgtaccagtatcctttcccagcgattgcatagtggcatgcttatcaaggatagtatcaatggcctgcgtgtcctccataacaatgagcccggaaccatcatccagttcataattttttgacacaccatcttttatactaaattggcctttactgtttggaccactcacttccagcgcattcgttgagacaattaattttccgcctgcttttttatcaacgccagttacagtcccgccatccataacctccagtaagccgccactatctacagtggtattataagcgaagtcattttcttcaactcgcaaacttccgccgttttccaacaacatattattagcaataccattcttgatatcgaactgaccgagacggtttgttccgaatacctccatggcccgcgtggttgttttaatagcaccgcctgctttctgatctaccgcaaatgcaaatcccccctctttaacctccagtagtcctcccttttcgatagcgacaaagacggcccccccatctttttcaacgattaagcgcccgcctttaatcgtggtatcattcgctgcgccataaacctgtagcacaccattattgagcgtagtctggtttgccgcgccacccatttgaacaatttgataaccgtcatttaatactgagtattctgcggcgccattcatttcaatgtactgataccctccgttaatttcagtattattacttacaccaaattcttttatatgctgttctccgccaggattgattttcgtattattggcggtcccataaaccagctggatatctttttccaggacaacaccatcaactgtctcaccatactcaacagttgatgccaatgctatgggtgaatataaggaaggtgcgaataagcggggaaattcttctcggctgactcagtcatttcatttcttcatgtttgagccgattttttctcccgtaaatgccttgaatcagcctatttagaccgtttcttcgccatttaaggcgttatccccagtttttagtgagatctctcccactgacgtatcatttggtccgcccgaaacaggttggccagcgtgaataacatcgccagttggttatcgtttttcagcaaccccttgtatctggctttcacgaagccgaactgtcgcttgatgatgcgaaatgggtgctccaccctggcccggatgctggctttcatgtattcgatgttgatggccgttttgttcttgcgtggatgctgtttcaaggttcttaccttgccggggcgctcggcgatcagccagtccacatccacctcggccagctcctcgcgctgtggcgccccttggtagccggcatcggctgagacaaattgctcctctccatgcagcagattacccagctgattgaggtcatgctcgttggccgcggtggtgaccaggctgtgggtcaggccactcttggcatcgacaccaatgtgggccttcatgccaaagtgccactgattgcctttcttggtctgatgcatctccggatcgcgttgctgctctttgttcttggtcgagctgggtgcctcaatgatggtggcatcgaccaaggtgccttgagtcatcatgacgcctgcttcggccagccagcgattgatggtcttgaacaattggcgggccagttgatgctgctccagcaggtggcggaaattcatgatggtggtgcggtccggcaaggcgctatccagggataaccgggcaaacagacgcatggaggcgatttcgtacagagcatcttccatcgcgccatcgctcaggttgtaccaatgctgcatgcagtgaatgcgtagcatggtttccagcggataaggtcgccggccattaccagccttggggtaaaacggctcgatgacttccaccatgttttgccatggcagaatctgctccatgcgggacaagaaaatctcttttctggtctgacggcgcttactgctgaattcactgtcggcgaaggtaagttgatgactcatgatgaaccctgttctatggctccagatgacaaacatgatctcatatcagggacttgttcgcaccttccataacgctgtagccaccagaacagatattgcggaacgacaaagagaaacagaaccagattgatgcattgagctttcatcctatgaaattaattgctgttaaaagcattgggtacagaaaatacccatagctccatacccggagtcagtttttaaaaactgtttaaagaaatgcacaagtattgtgattgattttttagttgtttttcttgatgagaagctgatgcaaaattccgtctttataatgaaaatgatgccaaagcgaacgacaaggttgtagttttcactacatgtccatacataaaatggggtaacattcacgcgcctggtagcgttaccaacgctacgctcaaacataatgattctaataaaacctcaggagactactatgcctgaagcaacaccttttcaggtgatgattgtggatgatcatccacttatgcgacgcggtgttcgtcagttactggagcttgatcctggctctgaagtggtcgccgaagcgggcgacggcgcgagcgctatcgatctggcgaatagactggatatcgacgtgatcttgctggatctcaatatgaaaggtatgagtggcctggatactctcaatgccttgcgcagggatggcgttaccgcgcaaattattatcctgaccgtatccgatgcctccagcgatgtctttgcgctgatagacgcaggcgcagacggttatctgttgaaagacagcgacccggaagtattgctggaagcgattcgtgccggagcgaaaggcagcaaagtctttagcgaacgcgtcaatcagtacttacgtgaacgtgaaatgtttggcgcggaagaagatcccttcagcgtgctgacggagcgcgagctggatgttctgcacgagctggcacaggggctgtcaaataaacagattgcctcggtgttgaatatttccgagcagacagtaaaagtacatattcgcaatctgctgcgtaaactcaatgtccgctcacgcgtggcggccaccattctgttcctgcaacaacgcggggcacaataaaaatagcccgatggatttatcatcgggctgagatttatgacaaacgcaaaactgcctgatgcgctacgcttatcaggcctacgtggatcgatcaatttattgaatttacacaattttgtaggccggataaggcgttcacgccgcatccggcataaactaagcgcactttgtcaacagtctagcccgatggcatcaccatcgggcctctttttatttactctcctgcggcgacaaatgttgcatcgcctgcgcgatactacgttcaatcaccgcacggcgagtatcgttggcaggtaagagtttcaacatcatctcccacgcggcaacggcttcgccaaatcgctgctgctcaaaggcattaaacgcatacatgcttagcacacggatattgctatggtccgttctcaccagctgacgtagcagttcaccgccgaggcggttgtcgttgggatcagatgaacgagtcaacgcttcagcgtatcccagtgcagcatcactgtttttcggatcgaggcgatacgcagtggcgtatgcatcggtggcgatactggcgttacccagcgccatgccaacgcggcccaacataatccagccttctatatctcccggatttttttgcagttgagtacgcatccccagcgcaagacgcgacatctcttcttcgttgagcggatcggctttcggatccagcgccctgtccagcaacgccggagcctgtgccgtggcctgctgccagattttcacctgctgataattgccagtctggtagtagctgacgccagccacaattaacgccaccacaatacccggcagataaacaacatatccggcacgcttaccttccggcacgctttgttcaggaaacgcttccggcaccacgcgtacccgacgccgcgagcgggcgtatatgacccaaccgccaatgccaatagccactactggcagcacccacagcagcacggtcagcggcgttaacggcggatcgtaagtgacgaagttgccgtaacgcgccaccatataatcgacaatctcttttttacttttaccttcctgcatcagttcatacactttctgacgcaggtcggtggcaatcatcgagttggaatcggcaatgctgttgttctggcatttcgggcagcgcagttcttcagtgagctgacggaactgttgttcctgtgcttcatctttaaactgcaacacatcgatggtcgccagcgctgagccggagatcatcagcatcagcacgcccaataaaaacctcattgtgcggcctccttactgtatttctcccacagcggcttgatctcttcttcccagacgcgaggattcagatcgcccgcatggcgatagcgaatgatgccgttgccgtcaataagaaacgtttctggcgcgccatagacaccgagatccagccctaacatgccatcgccatcaaacaggcttagcgcgtaaggattgcccagctctttcagccagctgattgccttctggcgatcgtctttatagttcatgccgaccacgcggatgccctgcgcagaaagctgattcagatattgatgttccgcacggcaggtcggacaccaggtcgcccagacgttaagcagtactggtttgccctgagtcagcacatccgcctgataaaactgccccggattgtccagtgattcgagacgaaacttcggcacaggcttgccaatgagcgccgattccagattggtcggatcatccccttcggcattacgcgccagctgccacagcagcgccgcggcaatcgccaggaagataatcaacggaattaacaatactttgcgcttcatacggcctccggcgcagttttttgcggactcacgcgcttacgatagcgaggatcaaacagacacagcagtccgcccaacgccatcatcagcccgcccgcccaaatccagcgaacaaatggtttgtagtaaagacgcacggcccacgcgccgttttccagctcttcaccgagggccgcgtacaggtcacgcgtgatgccgccgtcaattgccgcttcggtcatcatcgacccggcagtgttgtaataacgtttttccgcatacagcaccgtttccggcttgccatcgcgcgttacgccgatagtcgccacaccgccacgccagttcgggccagtcacctctttgacatcacggaaggtgaagcgatattcatgaatatcgacgctatcgccggacttcatgcgcacatcacgctcaacgctatagttctggctaaaggcaatgccaacaattgtcactgccagcccaaggtgagccgccaccatcccccaataactgaaggtggttttcgtgccgcgtgaaatacgtagcgcagcttccgcaattgccagcaccgcaatccagcaggccattgccaggccgagcaccgtcatcgccacaactttgctttcgaacagccacggcaacagcagcgacagcaccagcgtagagatgaaggcgataatcaataaattgcggatcttacgcgggcgatcccgcccccagcgcaccagaggaccgacaccaagcagtagcgcaaacggcaccatcagccaggtaaacatggtgttgaagaacggttcgccaatcgaaatactgcccagtcccagttgcttatgcaccaacggcagcagcgtccccagcaacaccaccagcatcgcagcgaccagcaaaacattgttcgctaacagcaaagattcccgcgaccacagcgcattgtttacgcgtgagcgaactttgtgtccacgcgcggcaaacagcagcagcgaaccgccaatcaccagcaccataaaggcgaggataaacataccgcgcgccggatcagacgcaaacgcgtgtaccgataccagcacgccggaacgcacgaggaaagtccccaacagacacaacgagaaggcactgattgccagcagtaatgtccacgctttgaagctggcgcgttgttcagtgaccgccagtgagtgcatcagcgcagtccccaccagccacggcataaacgaggcgttttctaccggatcccagaaccaccagccaccccagccgagttcgtaataggcccatgcggaaccgagcacgatgccgagcgtcaggaagatccacgctgccagcgtccacggacgagtaaaacgcgcataagtgctgtccagacgcccgctcagcaaagaagcaatggcaaaagcaaacgccaccgagaaacccacgtaccccatataaagcagaggcggatggaagatcagccccggatcctgcaatagcgggttaagatcgcgaccttcaatcgggaagttcggcaacgtgcgagagaacgggttagaggtaaagagaatgaacagcaaaaagccgacactgaccatccccattatcgccagtacacgggccacaatatccagcggaatacgctgactaaaaatcgccaccgcaaaggtccagccgctcatcagcagcacccacagcagtagcgagccttcatgcgcgccccaggtagccgccacgcgataccacaccggaagctgggtattggagttgctggcaacataggtgacggtgaagtcgttgaccacgaaagcattgaccagcaccagaaatgcgccagccacagacataaacagcagccaggcaaacaagcgggaagacgccatcatgcgcgcatctccgcgcgccacgccccatagcggatacacggacagcagcagcgcaattcccagcgccaggcacagcagtccgttaccaatttctggcatcatgatgctgggtccttataaacactcgccgggcgacggtggttagcttccatcgctttctcaacttctggcggcgtatagttttcatcgtgtttcgccagcacttctttcgcgaggatatgattgcctttttccagttcgccctgcaccacaacgccctgcccttcacggaacagatccggcaaaatgccttcgtaagagacatccactgagccttcagcatcgtaaatggtgaaggtcactttcagcgaattgggatcgcgctgcacactacccggcatcaccatcccgccaacgcgcagacgctgaccgacttccggcatttgctgagtttcacgcttgccgtagagaatttcccccggcgtataaaagagatcgatattcgagcgcagcgcatatagcaccagaccgatagtcagcgccagccctgccaacacggcacaggcaatccacaagcggtttttacggcgaatattcatgcagcctcctgctgttgcgcagcacgtaaacgcgcctcacgcgcccgctgttgcgccacgccacgcagaattgcgcgatgttgcatcaccgagtgcacgaccaaaaccaccagcggaataacggtcatcaccaccgccagccagacaaaaaaggcgtaaccgcccattgcgaaaaattcattccaggaagcaaatgcaggggtcatttacggcctcttttcagtatcagttcactcacccacggacggcgtttttccatcagcaaaatcaaattacgcatccgcatcagcgtcagcgtggcagacaggagcaggaagccaaaaatcgaccagcgcagcggcgaacgcatcgccggatcgatactttgctgcatccgcgttgatccctgatgcagggtgttccaccactccacggagtaatgaataatcggcagattcaccacgccaatcagcaccaggatacctgccgcacggcccgccagacggcggtcgtcgaaggcgtgccacagggcaatcacacccacatacaaaaacagcagcaccagttcagaagtcagacgtgcatcccatacccaccaggtgccccacatcggttttccccatgcagagccggtaaccagggcaataaaggtaaacacggcaccaatgggggccatcgccgccaccgccaggttggccattttcatctgccagacaaggccaataaacgctgccactgccattgatgcataaatgcccatcgaccagatcgccgcaggcacatgcaggtagataatgcggtagctatttccctgctgataatcagccggagcaaagccgaatccccagatccagccgacggtaagcacgaccacactggcaattgccagccacggtataaaccagccacagatttgatacagccgtggtgggatcgccagttgatgcagtgttttccacatagtttcgataccagactcgaacaaaaatcagtaatccagcgttattgaatgctgattcgtaacgctgccgccgtcgcaaaaggacttaatgtcgcggtgcctgccagcaacgcgcctaaaattgccagatacccgtcaacgggcaaatgcatagaagccgcgtccatcgcggcggtggcaaagatgagtaatgggatagtcagcggtaacaccagtatgctgagcagcacaccaccgcgcttaagtcccactgtcagcgccacgcccggtgcaccgagaaagccaagcgtaggcgttcccagcagcagcgtcagcgccatcacttgccagccataaacatccattcccagtagcattgctaccagtggcgaaaggatgagtaacggcagaccggttaccatccagtgcgccatcaccttcgccagcacaacggcgggcaagggtaacggcaacaacatcaattgttcaagactgccgtcctgcaaatcgtcacggaacagtcgttccagcgccagcaaggatgaaagcagcgcagcaacccagataatgcccggtgcaatacgcgccagcagttgcggctccggaccgatactgagcggaaaaagggtaattacaatcaggaagaaccacagcgggttggcgatttcggcgctatggcgaaacgctacacgcagctcaagacggaaaatgcgccagaacatcatgcggccctcgtttgcgtcagtgaaatgcggcgaattttactttcagcaacgttgagcggctggtgggtagtcagaatcacaatccccccctgctccgtatgctgcgccatacgctgggtcagacgatcgacaccgttaacgtcaatcgcggtaaaaggctcgtcgaggatccataacgtggcacgggtcagccacagacgcgctaaagcgacgcggcgttgttgcccggccgagagctgatttacaggaatatcttcgaatccggcaagcccggcctgcgccagggcttccagacattgtgcggtatcgccatcgcgatgataaaagtgcagattttctaacgccgtcagccgggttttgatccccggctgatggcctatccataacaggttttgatggtagctgtcgcgtacctgatgcaagggctgcccttgccagagaacctcgcctgcgtcagggcgagacaaccccgtcagcaaacggagaagcgttgtcttccccgcgccgttgctaccggtgatttgtacccactctcctgcgttcagcgtaaatgacaagccactaaataaggttcgttcatcccgctcacaaagtaactctctggcttcaagcatacccacgcaataaccctgttaaaaacctggctcgacttcacgcatatcgggcagcttgtgcgctatccctttatggcaatcaatacaggtttgcccatctttcaccgcctggtcatgcatcttcgcggcaaccgatttctgggcggttgtatccatatactcgaagttgtgacagttacggcactcctgcgagttattgtccttcatgcgccgccactcattctgtgccatcgtcagacgatgagcttcaaatttctgcggcgtgtcaataacgccaaaaattttaccatacagctctttacttgctttgagcttgcgtatcatcttcggcacaaactcgtgcggaacgtgacaatccggacaggtcgcacggacgccgctacggttgttgtagtgcacggaatccatgtattcctgatacaccgtgttgcgcatttcgtggcagctaatgcagaactcttcggtattggctttttccatcccggtgttaaagccaccccagaagacgatgccgccaacaaaaccgatcaacagcagcgtccccagcgccagacggctgggggtacgccaccatttccacaggcgcttaatcagaccaggcttacggtcagaatttcccataataacctcttatttcccgtaaccttttgatggggtaaaggtattccccacgattggcgcggtatcggcctgcggtacgtgacattgcagacagaaataacgacgcggagccacttccgcgcccactttgccgtcgctgtccataaagtgagtaggactgatacgcggcgcgccagtggtgcgatagctttcgacaccgtggcactgcaagcagcgattggtattggtcgttacctgataaccttcaacgctatgcgggatcattggcggctgattcacatagttcagcggcatccgatcctgctcttttggcatccgaatggccccttcctgtgtcccggatacttccggcgactggctaaaatcgacgccattagccgcccaaaccgcgccgcttaccaccagggccagcatcgccgtccattgacacagcgctttcttcaggtcatggcttttcatgatttcgctcccgaactccatcgtgtagttattgtaaatacatcctcagaacagacatccacgcagcgaccgcacgtcatgcaatcgcggctggtgacctgcaccgggctttgttcatccagcaccggggcacgtagcacatgcggttccgggcaaacatgaaaacaatccatacagcggttacatttctgccgatcggtggccgcaacggtaatcacacctttgctacccagcacgccatacagcgcgccaaccggacaaatgtgcccgcaccagccgtgttcaacgaccagtagatcaaataaaaacagcgcgagaataagcagcgcgccgctgccgaagcccattaccaggctacgccccatcagagaaacggggttgatccattcccaaatgagcgtgccagttaaggctgatcccaccagaatgaccaccaacagcacgtagcgaatgtggcgagggatcgtcgcagactgattgaggtcaaagcgcctgcgtaaccagttcgctaagtcggtaatcgggttcagcgggcagacccagctgcaaaataatcgctttcccgccagggcgtagagcacggtgataatcaccgcaccggtcaacgccaccgtggcaggcagatgaccactggcaagactttgcagcgtcatcagcggatcggtcagcggaacggtgtcgaataacaggctactgctgtagttgccgtgcaagatccacacaccaaaccatggaccgctcaaaaacatccccagcacgaagaactgacaaaggcgacgtaacaccagccaacggtgactgcgccaccagccttttttctccagcgcctcgcgcccggcgtcacgtttacgatttgccattgttcccctccagccagccgaagcggtaatggtgacctaactcccctttcgccagtgacagcggtaacaccttgattgccggttgttccagcacgcatactttttcgcacttaccgcaaccggtacaggcgtcgctgtgaaccgtcggcagaaagcgggcgtgcttaccggtacgcgtgttgcgctccagctccagggtgatggcctcatcaattttcgggcattcgcgataacaaacatcgcagcgcagcccctgaaagttgagacagttttcctggtccaccagtaccgccagccccatccgcgcgtcgtcgatcgattcaatctcacgatccagcgcaccgcttgggcacactttggcgcacggaatgtcctcacacatttcgcaaggaatatcccgtgcgacaaaatatggcgtgcccgccgacagaccagaggccagcgtcgccagttttaaggtgtcgtaagggcaagcctgaacacactgaccgcaacgcacacaggcactggcaaaggcgttctcgtttatggctccgggcgggcgcaaccgcacgccagatgcgcgtgcggtttgctgttgtaaccccagcgccacacccacggcagccagcccgcctgctgtgcgaacgacatcgcgcagaaagcggcggcgaccattttgaggtttcgctgaccgggacataatggcttacaccttctccagtttgaccgcgcacttcttgaagtccgtctctttcgagagcggatcggtcgcatccagcgtcagtttgttaaccaactgtgcggcgtcgaagaacggcatgtacaccaggccctgtggcggacggttacgaccgcgcgtttcaacaatcgagatcacttcgccacggcgagaaaccactttcactttgtcgccacggcgcagatcgcgcgctttcgcatccagcgggtgaataaacaggaccgcttccgggaaggcgcggtgcagttctggtacacggcgagtcatactgccggtgtgccagtgctccagaacgcgtccggtagagagccacaggtcgtactcttcatccggtgcttccgccgccggttcgaatggcagtgcgaagatcaccgctttgccatccggtttaccgtagaacttatagccttcgcccgctttcacgtacgggtcgttaccttcgctgtaacgccactgcgtttctttaccgttcaccaccggccagcgcagaccgcgcgctttgtggtagtcatcgaacggtgccagatcgtgaccgtgaccgcgaccaaaccatgcgtactcttcgaacagccctttttgcagatagaagcccagctcgcgggattcatcgttcagctgatcttccgccagttcggataccgggaatttgctcacttccggtgtggcatacagcacttcgtacagcgttttgccacgcagttccggtttcttcgccagcagatcttccggccatacttcttcagttttgaagcggcgggagaactggactaactgccagagatccgatttcgcttcgcccggtgcctgtacctgttgacgccagaactgagtacggcgttcggcgttaccgtaagcgccctctttctctacccacattgcggtcggcaggatcaagtcggcggccagcgcactgactgtcggatacggatcggagacgatgatgaagttgcgcggatcgcgccagcccggcatacgctcttcattgatgttcggcccggcctgcatgttgttggtacacatggtccagtaaacattcagtttgccgtctttcagcgcacggtcttgtgccaccgcgtgcagaccgattttcgccggaatggtgccgctcgggatattccacttcttctcgcagatatcacggtgtttctcgttggtcaccaccatgtccgcaggcagacggtgagcaaaggtgcccacttcacgcgcagtaccacacgcagaaggttgcccggtcagggagaacggaccgcaacccggctgggaaattttgccggtcagcaggtgcaggttgtagaccaggttgttagcccacacgccacgagtatgctggttgaagcccatcgtccagtaggagatgactttcttgttcggatcggcatacagctgcgccagttgttctaactggtctttcggcacgccggtcatttcggcagttttttccagcgtatactcggcaacgaaggctttgtaatcttcaaagctcatcggttcggaggcgtcagaacccggattcttcgctgctttttccagcggatgggtcggacgtaaaccgtagccgatgtccgtcgcccctttgcgcaggttaacgtgcttgctgaagaagtcctgatttatcgcattgttttgaatgatatagttggcgatgtagttcaggatcaccaggtcagattgcggcgtaaagatgatgccgttatccgccagctcgaagctacgatgctggtaggtagaaagcaccgccacggtgacgttctggttagagagacgacggttagtgatgcgcgaccagaggatcgggtgcatttccgccatgtttgcgccccacagcacaaacgcgtcagcctgctcgatgtcgtcatagcagcccatcggctcatccataccaaaggtacgcataaagccaactactgccgacgccatacagtgacgcgcgttcgggtcgatgttgttcgaacggaagcccgctttaaacagcttggacgcggcataaccttcccagatagtccactgaccagaaccgaacataccgatcgattccggccctttttctttcagggcggttttgaatttctcttccatcacatcgaaggcctgatcccaggtgattggggtaaattcgccttctttgtcatatttaccgtttttcatacgcagcagcggctgcgtcaaacggtctttaccgtacatgattttgggcaggaaatagcccttaatgcagttcaggccacggttaaccggtgcgtccgggtcgccctgacaggccaccacacgtccctgctgcgttccgaccagaacgccgcaaccagtaccgcagaaacggcacggcgctttatcccatttgatggcttcctgctgaccaacaacggcgcgggcaacgcccggcacgctgagaccggcagccgccgcagcggccgcaacggcgttagctttcataaagctacgacgactgagtttcatggtgtttcctcaccttgctcttcctgctggtgataaaccagcgacaccgccagcacgccctctacgttgcgtactgactcaatggtttggatcagcgtttcgctgtcttctgcttccaccaccacaatcaactgaccgctcggcgcgtcgctgacagcaacttcacagccgggaaaggcgttcagttgggtgctgatgtctgaaattcgttcgcttttggcctgcacgaccaggctgcaaacttgccagttagtgtgcatggagatactccgcagttatggctgataccggacagctggctgcacatgctccacatccgttgcaaagttggctattaagttgcggctggtagatcccggagagcgtcgggcgaaagataattgccattggctcacagctatcctgacagcggcggcattcaactgactgatacgccaggcacgcgtccccgatggtgaactgcaaatcccaggccctggtgtggcgcggagaaaatagcgattcggggcaagcctgcgcgcaggcgtaacagaagctgcactcgttatttttgaaattaacgctcggatagccgcccgcgccgcgttgcagaatgttgttttcacaagcattaatacaggcgtcgcagcgggtgcaatgggtcagaaaatgagattcatcaccggaccagggcggacggataccgttactggctttgcgccagcgaccagtgagtatgccccgacgggatgcatcaatcttcacattgaccttccatcattaacgcgctctgaaaattgagagcgaccaaataaaccgcataattaataagccatttttatagccgctaagatattaaaggatgtgtcaaagatgcataccccgatcggggtaaaacctgtagcaggatcaaaagagtggcgggaagcgtggcaaaaacgggcttttgctcacatttcaaatggttataaatatatttatatagcgattgattcaccagagatatttctgctggtttgctctctcattagaatttaacactaaaagagcaggtaaaattgtctgaatgttctttaagttattcataaagcaaattaataaatctgatgaatatgttaaccttcagcgacatcatcggtgaaaacctataaatgaagaaggaaagcaaaaaaatgaagaccattctacctgcagtattgtttgccgctttcgctaccacttccgcctgggcggcagaaagcgtccagccactggaaaaaatcgcgccttatccacaagctgaaaaagggatgaagcgtcaggtgattcagttaaccccgcaagaagatgaatctaccctgaaagtagaactgttaatcggtcagacgctggaagtcgattgcaatttgcatcgtctcggcgggaagctggaaaacaaaacgctggaaggctggggctatgattattatgtctttgataaagtcagttccccggtttcaacgatgatggcctgcccggatggcaagaaagagaagaaatttgtcaccgcgtatctgggcgatgctggaatgctgcgttacaacagcaagctgccgatcgtggtgtatacgccagacaatgtagatgtgaagtaccgcgtctggaaggcggaagagaaaattgacaacgcggtagttcgctaaactgccgtgaagtgcggcaccccgtaggtcagacaaggcggtcacgccgcatccgacatccaacgcccgagccggttgcctgatgcgacgctggcgcgtcttatcaggcctacaccgctgtgaagtgcggcaccccgtaggtcagacaaggcggtcacgccgcatccgacatccaacgcccgagccggttgcctgatgcgacgctggcgcgtcttatcaggcctacaccgctgtgaagtgctccaccccgtaggtcggataaggcggttacgccgcatccgacatctaacgcccaagccggttgcctgatgcgacgctggcgcgtcttatcaggcctacaccgctgtgaagtgctccaccccgtaggttggataaggcggttacgccgcatccgacatccaacgtccgagccggttgcctgatgcgacgctggcgcgtcttatcaggcctacaccgctgtgaagtgctccaccccgtaggtcggataaggcggttacgccgcatccgacatctaacgcccaagccggttgcctgatgcgacgctggcgcgtcttatcaggcctacaccgctgtgaagtgctccaccccgtaggttggataaggcggttacgccgcatccaacatctaacgcccgagccggttgcctgatgcgacgctggcgcgtcttatcagcatacgccacatccggcataccatgccggatgtggcgtatcattacaacgcaatatccgccacttctttttgaacgggttgcggtttcaactgcggtttcggcgtactatctgctgcctgcggcttgtcgtagttcaaccccagcacttcgctggtgtactgcaactcgcgttctgttgccgctacatcaccgttcagcttgcgtccataagacggaacgatcgctttcaacgtagcctgccattgcgggctggaaacacgatcgccaaatactttttccagcagattcaacataatcggcgcggcggttgacgcccctggcgatgcccccaggagcgcggcaatggttccttgctggtcactgacgacttcagtacccagacgcagtacgccacctttctcggcatcacgcttgataatctgcacgcgctgccccgcttgccacaaacgccagtcctcttttttcgcctgcggatagtactctttcaacgcttcaaaacgatcctcttcactcaacatcacctgactcaccagatatttcaccagatcgaaattatccagcccgacgtgcatcatcggcatcacgttagaggtggtggtggaactcattagatcccacaatgaaccgtttttgaggaatttggttgagaaggtggcaaatggcccaaacagcactacgcgtttaccgtccagaacgcgggtatcgatatgcggaaccgacatcggtggtgcgccaacggatgctttaccgtaaaccttcgccagatggtgattaaccacgtccgggttttccgaaacaaggaactgtccgcccaccgggaaaccggcgtagtctttcgcttccggaatccccgattcctgtaacagcttcagcgccgcaccgcccgcgccgataaagacaaatttggcacgaatgttctgtgcagtgccatttttcagatcggcaacggtaacggtccaggtgttatcgtcattacgctttagggcgcggacttcgctgctgagttgcagcgagaagttagatttcttctgcaaggaagcaattaactggcgggtgatctcgccgtagttcacatcggtaccaatttccgtacgcgtggctgccactttctgttgcggatcgcgcccttccatcactaacggtgcccactctttgatctgcgcgtgatcttcagagtaacgcataccgcgaaacagcgagctttgttgcaacgcggcgtaacgggcgcgcaggaaattgacgttatcctcgccccagacaaagctcatatgcggaacggtattgataaatgaacgcggagtacgcagcacgccgcgctcaacctggtgcgcccagaactggcgggaaatctgaaatgcttcgttaatggcgactgctttttcaatactgatgctgccatcggcgttttgcggggtgtagttcagttccatcagtgcagaatgcccggttccggcgttattccagccgttcgaactctcctgcgcgacaccctccaggcgctccaccatggtcatcgaccattcaggctccagctcgcgtaaataggtccccaacgtggcgctcataatgccgccgccaatcaacagtacatcagtttcctgctcctcggacgctttcgcttttgccgccatcgaaacggcattaagccccacggccatcgagaagagcatggcagtcacttttttcatcttgttaatgccttacttttagtcgctttattgcaggtgagatttgcgcggcatcaacggtaacacttaagtaacaacatttaaataatgtttataaattatattctaattttagaaacattataatttcgttgattaattatagggttattagaaatgaagggatttttagcatattgacctgacggcagcagtccgccaggtcagcgtcgtaatattatgccgtccgggcaacggcatcacgcgaagcggcatcgcgctcttcgcccgtcagctcgctaagttgcccattgcgcatttccagcaggcggtcggcgtggataaagtaatgatcatcatgactgatagcgaaaatagttttacccatctcctgcatcagcggcagcaacacctgataaaactcacgacggaagtgtggatcctgatccgccgcccattcatccagcaggataatatcgcgttcttctgccagcgccagcaacagcgccacgcgttttttctgcccttttgataacttcaggttaacaatacgcccgttgcttaactcaagcttatgagccattttcagctgcgccagccacttctcaaccagttgcgggttagcgggtttaccctccggccccagcagttgatcaaacagccagacatcggtaaacactgccgaaaacagtttgcgataatcttccggttgttcgccgctgacaggtttgccatccagcaagatttcgccgctttgtggctgatacaagcccgtcaacaacatcgccagcgtcgattttccgctaccgttgccgccaatcagaaacagcagctcgccacgtttgatggtgagattaatcggaccaacggaaaacgcgttatcctgataagcaaacgtcacgttacgcagctccagcgtttgccagttgggaaacgcctgcgggcgcggaaactctgctttgaaaggcgcgagcgcgaatttgttcagcttgttaaacgccacctgcgccgtcagcagcgtcggcaatgcgccaaccgccgaaagcagcggcgtacgcaggaataaaagcgtcaacgaataggtcgcggcaacgttggtatcagcccaaccgaggctgttcgccatccagaacaccaggccgattgcgcccagcatcatgatgtttgaccagttcacggcactaagatggaaggtgtctgcgcgaataatatggtggcgatactcttgcgcatcaggaatgtagaggttgttaaacacatactcggcgcgttcccggttcagagtcagctctttgcgcccttcaagtacagtttgaaaatccgtgtacagcttgtcttcggtttcacgcagggtcgccatatgtttgtacacccgcgccaccagcacaaaaccgccccagatggtgatcgccatccagatagccgttaccagcaacattttgcccgacagcatccacagatacgccgctgaaccgatagtgagaatgatcccctgcaccagttccggcagacgcacaaaagcaatggtgatattgcgcacatcgctggttaaccccgccagcaacgaggcgctaccgagttgttcaatgcgctcgacgtgagtatccagaatccgcttgataaattcactacgcagtcggtaaacgaagtgatgccccaaagtggtgagcgccagttgcgatccgagagtgactgccatcaacagcagcaataatcccagaaactccggcaacaccagcagactggtatccgccgtttcgataaggcgctgattgataaaagcaattaagccaatgcctaatgccgcactggcgaggcttagcgccatcacactgataaatggccagcgatactgccgccagacaagtacaagaagttccatgcagaaaacccggacaatgaattacagcccgcagtttaaacatcttcgcgcgcacagcaataataattcttatttttattcttttttacctgcctgacggaatgtcaggttgtagcggcagtcgatggtgagtggatgaaaccccgctttcaacggttgaataccgtgataaaacagccgcgattcaccgccccataccaccacatcgccatgttccaacaacaaacgtttgagcggatcatttcgtttcaggccgccaaattgaaaaatcgcgggtaagcccagagaaacagaaacaattggcgcgcgcagatccggttcgtctttatcctgatgcagcgacagtttcgcgccaggagcgtagcggttgataagacaagcatctggctggaaatctggatagcccgccgccgtagccgcacgttgacataaattatgaaaactctgtggcatggcgggccacggtttatttgtttgcggatcaatgggcgaatagagataaccttgccgatgggtcgtccagcccagatgcccacagttggtcatcgccaccgacatggtatatcccccgggggtgaccatctggcgaaacggcgactggctggcaacgtcattaatatcgcggatcagttgctccgcagcgttaaaagcaaaacgccgtaaaattaccgcaccagccgccagtggctcttgccacggttcagcatcggcaaacagatccaacattacctctcctcattttcagcttcgcggcgcagcagttgcgctttacgcgacacgccccagcggtaaccggaaagtgtgccatcaccacggaccacccgatgacagggtattatgatagccagcttgttggcggcacaggcgctggcaacggcccgtaccgctttcggtttgccgatggcgttagccagttgctgataactgacggtttcaccgcaaggtatcgtgcgcagtgcctgccagacttgttgctgaaaagcagtgccgcgaatgtccagcggtaacgtcagcggcgtatcgcgttgattgaggctggcgatcacttcacgcacatgttgctgaaacatcagatcggcaggcgcgttgtcggcagcgggaaacatctgctgcaactcgctgattagtgtcgcgtcatcatcgcccagcaatatcgcgcaaatcccccgctcgctttctgccaccaggcaacgacccagctcacaatcagccagcgcgtaacgcaccgccagattttcgccaccgtgacggaattgtttagccgtcatgcccagcgtttcgtcagctttgcgatagtaactgctgctgtcggggaatccggcgttaagaatagacgtcgtcacgctctcccctttcgccagcgattcgcgcaaacggcgagcgcgccaggcctgttgccaggctttaggcgtcattccggtagtcgctttaaacaaccgatgtagatgaaatggactcatcgccacctggtcggctaaggcttccagcgttacaggcgtttcctgttccagcagtcgacacgcgtgggtgattttatccaaccgatgttgctgggcattggctttttctggctgacaacgtttgcaggggcgaaagccagcggcgagtgcctcgctggcatttgcgtagaaggagacgttttcccgcaaagcatgtctggcgcggcaagacggacggcaaaagatgcctgtggtacgcacggcgaaaacgaattcgccgtcggcattcgggtcgcgggctaagacagattgccagcgttgatcgtcagttaagcatgtggcttttttcataatcagctccctggttaaggatagcctttaggctgcccggtcaccatcacgcaaaaaccaacaatcttgcgctttaatttttttcgctgacaaggaagcttttaaactgtggtgacatccaggttttaaagctatcgccttctttggtgatcatataaaccgccagcccttcccggcgaacaacctctttagctttctccggcccgagtaccatcaagccagtatcccaggcatcggcttccagcgccgtcggagcaatcaccgtcacggataccagattgtgttcgatgggacgcccggtttgcggatcgataacatgggaaagacgtttgccgtccagttcgtaatagttacggtagctgccagaggtgctaatcccatgaccgttgatatccaccacagcctgaaccgcgttttctttatcggttggtttttgaatcgctacccgccacggcaggccttcaccgttcataccacggctgttcagcgcgccgcccaccgacaccagatagcgggaaatcccttcctgctccatcaagcgtgccaaatgatcggccgcatagccttcgccgacggtggagagatcgacatataaatccggcaggtctttttgcagatattgctgatgcgactgattgatgaccgtcaggtgctgtaagccggttttggctttcatcgcatcgatctgttcctggctcggaatttgaaccggctgttgttccgggccaaagccccacagattcaccagcggcccgacggttatatccatcgcgccatcggtcttcgcgccaatgcgcagcgaggtggtgacgatatcggccatcgcttcacttaccggccacggcgataaactttgcgagtcgttaaagcgcatcagcgcggaatcttttttataggtcgaaagcagctgatcgtcggcgtccagttgggtctgaatcttttctttaagttcggcgctgcgtttggcgtcaatgcccgggatgctggcacgccagaaggtacccatagttttgccttcaagaacggtaacttcagtagcgtgggttttggcgggttgtggtttttgatcgcaaccaacaaagaagagcgcggcagccagcagtgccacgcgggtaaagcttatttccatacgtgattatcctcatgcgaacggtcgcaagagtacaccaaaaaactgagtttgtacgctgaaaacaatgaaaaaagggcccgcaggccctttgttcgatatcaatcgagattagaactggtaaaccagacccagagctacgatgttatcagtgttgatgccagcgtcacgagtgaactggttgtcgtccagcaggttgattttgtagtcaacgtaggtggacatgtttttgttgaagtagtaggtagcaccaacatcaacatatttcaggatatcttcgtcgtcgtagccacgacccaggtttttacctttagactgcaggtaagccagggacggacgcagaccgaagtcgaactggtactgagcaacagcttcgaagttctgtgctttgttcgcccaacccagggaacctacgcgagttgcgttgtaggtctgggtgtactgagcagccaggtagatgttgttagcgtcgtatttcagaccaccagtgtaggtttcagcacggtcgccgttaccgatgtaagcagcggtgttctgagcatcagtacgtttggagctggagatcgcaccaccgataccgaaaccttcgtaatcataagtgatagaaccgccgacgccgtcgccgttttgacgcagtgcgtcacgaccgttgttagttacgccactagtaaagccttcaccagatgggttgccgtttttaccctggtactgaacagcaaagttcaggccgtcaaccagaccgaagaagtcagtgttacggtaggtcgcgaagccgttaccacgctgctgcatgaagttgtcagaaccgtaggtgtcaccaccgaattctggcagtacgtcggtccaggaagttacgtcataaacaacgccgtagttacgaccgtagtcgaaagaacccacatcctggaatttcagacctgcgaatgccacacgggtccaggagttgttttcgttttcagcgctgttgccctggatctgatattcccactggccgtaaccggtcagctggtcagtaacctgagtttcacctttgaagccaagacgcatgtaggtctggtcgccatctacatctttgttgtcagagaaatagtgcaggccgtctactttaccgtacagatctaatttgttgccgtctttgttgtaaacttcagcagcgtttgctgcgcctgctaccagcagagctgggaccaggagggacagtactttaactttcatgttattaaccctctgttatatgcctttatttgcttttttatgccactgcatactgattaaccctcattaatcagtcggcaagtccattctccccaaaaatgcagaataatccaacacgaatatgatactaaaacttttaagatgtttcatttatcgctatagatgtttcaaaatgtaaatgcaagggaactttttaagattattgcggaatggcgaaataagcacctaacatcaagcaataataattcaaggttaaaatcaataacttattcttaagtatttgacagcactgaatgtcaaaacaaaaccttcactcgcaactagaataactcccgctatcatcattaactttatttattaccgtcattcatttctgaatgtctgtttacccctatttcaaccggatgcctcgcattcggttttttttacccttctttacacacttttcattattctgtgctaccacagaaaaactataacgcttgttaactatttcacaaataattaacatccgcataatttccagcaatctttgtttatttgcaattatttttgttgggctttttgtaggttatttgtacagcaaaatggcgcttgtacatctatttcccccaatgcaggatgataaatatcacgggagaatagagaatcatcaatcaggtaagagtctggaatttcacactgtaccctttatactgccctatcacttcgcgaagttttaacaggtcataaacacgaatgcgtcagaaagagacaacggccacgacccgcttttcactcctaccggggagcattacccgcttctttttactgttgatcattgtgttactggtgacgatgggtgtaatggtacaaagcgccgttaacgcctggctgaaagataaaagttaccagattgtcgacattacccatgctatccaaaagcgcgtcgataactggcgttacgtgacctggcagatctacgacaacattgccgcgacgacctccccctcctccggcgaaggtttacaagagacgcgcctgaaacaggatgtctactatctggagaaaccacgccgcaaaacggaagcgttaatctttggctctcacgacaactcaacgcttgagatgactcagcggatgtccacttatctggatacattgtggggcgcagaaaatgtaccgtggtcgatgtattacctgaatggtcaggataacagtctggtgctgatctcaaccctaccccttaaagatctcacctccggatttaaagaatcgaccgtcagcgacattgttgattcacgtcgtgcagagatgttgcaacaggccaacgccctcgatgaacgcgaaagcttttctaacatgcgccgcctggcctggcagaacggtcattactttacattgcgtactacctttaaccagccaggacatctggcaacggtcgtggcttttgatctgccgattaatgatttgatcccaccgggtatgccgctggacagtttccgccttgagccagacgcgacggcaacgggaaacaatgataatgagaaagaagggacggatagcgtcagtatccactttaacagtacgaagattgaaatctcctcggcactcaactctaccgatatgcgcctggtctggcaggttccttatggcaccttattgctggatacgttgcaaaacattctgctgccactgctgctgaacatcggtttgctggcgctggcgttatttggctataccacattccgccatttctccagccgcagtacagaaaacgtccccagcacggcggtcaataacgaattgcgcattttacgggcaatcaatgaagagatagtctcactgctgccgctcggcctgctggttcacgatcaggaatcgaaccgcactgtcataagtaacaaaattgccgatcatttgctgccgcatttgaatctgcaaaacatcaccaccatggcggaacagcatcaggggattattcaggcgacgatcaataacgagctgtatgagatccgcatgttccgcagccaggtcgcgccgcgcacacaaattttcattattcgcgatcaggatcgcgaagtgctggtaaacaagaaactcaagcaggcgcagcgtctgtatgagaaaaaccagcaggggcggatgatctttatgaaaaacattggcgatgcgctgaaagaacccgcacagtccctggcggagagcgcggctaaactcaacgccccggaaagcaaacaactggcgaatcaggcagatgtgctggtgcggctggttgatgaaatacagttagcgaacatgcttgcggatgatagctggaaaagtgagacggtgctgttctccgtgcaggatttaattgatgaagttgtgccttcagtgttgcctgccatcaagcgtaaaggtctgcaactgctgattaacaatcatctgaaagcacacgatatgcgccgcggcgatcgcgatgccttacgacgtattttgctgctactgatgcaatatgccgtgacctcaacgcaattgggaaaaatcacccttgaggttgatcaggatgagtcctccgaagaccgcctgacgttccgcattctggacacgggagaaggcgtaagtattcatgaaatggataatttgcacttcccgtttatcaaccagacccaaaacgatcgctatggcaaggcggacccgctggcattctggctgagcgatcaactggcacgtaaactgggcggtcatttaaacatcaaaacgcgggatgggcttggtacacgctactctgtgcatatcaaaatgctcgcagctgacccggaagttgaagaggaagaagagcgtttactggatgatgtctgcgtaatggtggatgttacttcggcagaaattcggaatattgtcactcgccagttagaaaattggggtgcaacctgtatcacacccgatgaaagattaattagtcaagattatgatatctttttaacggataatccgtctaatcttactgcctctggcttgcttttaagcgatgatgagtctggcgtacgggaaattgggcctggtcaattgtgcgtcaacttcaatatgagcaacgctatgcaggaagcggtcttacaattaattgaagtgcaactggcgcaggaagaggtgacagaatcgcctctgggcggagatgaaaatgcgcaactccatgccagcggctattatgcgctctttgtagacacagtaccggatgatgttaagaggctgtatactgaagcagcaaccagtgactttgctgcgttagcccaaacggctcatcgtcttaaaggcgtatttgccatgctaaatctggtacccggcaagcagttatgtgaaacgctggaacatctgattcgtgagaaggatgttccaggaatagaaaaatacatcagcgacattgacagttatgtcaagagcttgctgtagcaaggtagcctattacatgaacaatatgaacgtaattattgccgatgaccatccgatagtcttgttcggtattcgcaaatcacttgagcaaattgagtgggtgaatgttgtcggcgaatttgaagactctacagcactgatcaacaacctgccgaaactggatgcgcatgtgttgattaccgatctctccatgcctggcgataagtacggcgatggcattaccttaatcaagtacatcaagcgccatttcccaagcctgtcgatcattgttctgactatgaacaacaacccggcgattcttagtgcggtattggatctggatatcgaagggatcgtgctgaaacaaggtgcaccgaccgatctgccgaaagctctcgccgcgctgcagaaagggaagaaatttaccccggaaagcgtttctcgcctgttggaaaaaatcagtgctggtggttacggtgacaagcgtctctcgccaaaagagagtgaagttctgcgcctgtttgcggaaggcttcctggtgaccgagatcgctaaaaagctgaaccgcagtattaaaaccatcagtagccagaagaaatctgcgatgatgaagctgggtgtcgagaacgatatcgccctgctgaattatctctcttcagtgaccttaagtccggcagataaagactaatcacctgtaggccagataagacgcgttagtgtcttatctggcatttgcaccgattgccggatgcggcgtaaacgccttatccggcctacgattcccattatttcaacaaattacattaaagtaggccagataagacgcgtcagcgtcgcatctggcatttgcactgaatgccggatgcggcgtaaacgccttatccgtcctacgaatcccgcgatttcctgaccctctcggcatataacgtcagcgtctgttttatcacatccagcgttaccggcttcgacaggcagctgtccataccggactccagacaccgctgcttctcttcagccaacgcattagcagttactccgattaccggcaacgtcagtcccaactgacgaatgcgttgcgtcaagcggtaaccatccatatttggcatgttgacgtcgctaagcacgatatcaatatgattcttgctaagtacattaagcgcatcgacgccatcattcgcggttttacattgatagcccaacgatcccaactgatctgccagcaaacgccggttaatcggatgatcatccacgaccagaatcatcatatcgtcattatcgctgaccgctttgtccgttgacggcagagcgttagcaggatcgtcgctctccatctcgatcaaataaatacgcgccaacaatgccggtagctcatgcggagcagccacactgtgtacccactcccctggcgctttctccagcggaataccaatatggcgacgacagaaggtcactaccgctctgccctgccattttttactcactacctcgtcagtgatcaacacatcttcgggagtcggttcctgcccttcgtatgttgtaacgacgatgccgctgcgctgcaaactggtttccaggaactgacagagcgacgcattgcggaccgccagccagcagcgtttaccactcaacccttccacgccttttttctgcgggtactgagcgccgtacaacggaatacgcacggtaaactggctgcccattcccggttctgaatctaccgagatatcgccgtccatcatgctgatcagtttttcacaaatcgccagacccagaccggtcccctggaaattacgctgtacgcccgttccgacctggaagaagggatcaaacaagcgcaccacttctttcgccggtatccccacgccggtatcgcgaacacggatagagagataatcgccatccgcgcgaacatgcaaaactatacagccggtatcggtgaattttatggcgttactcaacaggttggagatgacctgctgtaaacgcatcgggtcgccatttaaggccactggcacatccggttcaataaagcagtacaagcctaactgcttgcgtaccaccagcggtaaatagttggcggtgatgtggttcatcacttcacgcggtgaaaactcacgcggttcgatcttcaactgttccgattcaatcttcgagaaatcgagaatatcgctgataattttcaacaacaggctggaagagttgttcattgccgtcaccagccgatcgacgcctttcggtaactctttggtttgcaacagatccaggttaccgataatgccatacagcggcgttcgcagctcatgactgacggtggcaaggaacatcgattttgactggctcgcctgttccgctgcttgtgccatctcctgcaacgactcttccatcttcacgcgcgaagaaacatccaccagcacacaaatggccacgttttcattacgatagcgcgaatggacgaagctgatttgcagattggtattgttgctggtcaggacatcaacaaaattgacctgctgcccacagataatttgcgtcagtcgttggcggtcctcatgcgtaagcatattgagataggtatgcgccagttcgttacttaaaatattgacgccatcagcggtacgcaaaatgcagatacccactggcgcggaggcgacaatcttgcgattgaactgctcatgttcttccagtcgcagggcgtcgctttccgccggaatgaaaatacgtcgctcgtacatccgtgcgagagtaaacaatgcagctccggcaagcacattcagcaaaattgcgttaaggatcaacatgcgaatgcgttccagcaccttatcaaccggcaccgaatacacgatgcttagcgatgagggtggcagatttttcttcagcaccagctcccggaacccttccgtatagccaaaccaggagcgttcctgcatccagcgaggatcgcccttaattttactttctggtccggtaagcgaaatcagggtatgaccattttcatcaagaatggtaacccccatcggcaacgtacccggtaagaaaaagttctccatccggatggtctgctcgacacccaaaagcgcctgcaaccggttcgccagataaactggcgtcaacgcgtaaaaatacccgacgccagggcgcggaccttcgctgatccagtagaggttactgccgctatcatcttgtggtgcatttcgatatttattgatgcgttcatgcaaagctttcaacgcggtatcgcgttccactggcatatcacgcagaccgaaattggccatgcagaggttatcgctgccgattaaaaatacccggtttagatcgtaagccgcagaaaaattatcgcgccagtagcgcataaaccacgccaatgactccagagaacctcgccaggtgttactcattgcggaacaatcggagtcggcaaacagcggttcaaacgcaggcacatccgcctgcgtttctcgtccacgcggggaaagcacaccgttttctgccgataagcgattttcggcgatgtacttcagctctttcatcacatcagaggtgcgttgaataaagcgctgagcctgatcggaactcagattaaattcctgacgaatttccgattctcgctgatgtaacgcattaacgatgtaaaaaacggatgaaaaagcaatcaacagccagagcactaacgccaatgctctgaacatgtagcgcgaggctttcagggttgtacgaaaagaagcaaggtatttcaaaggggcgaagctccgcctcaggtgaccgatggagtgtggttaaggtagcggtaaaagcgtgttaccgcaatgttctctcttctctggaatatgatacaccgccgagaaatcatcaccttaacctctgataatcgtcatataccggacaagactagtggatttcagcatgcattatatgaagtggatttatccacgccgcttacgcaatcaaatgatcctgatggcaatcctgatggtcattgtcccaacgcttactattggttatatcgtagaaacggaaggacgttcagcagtcttatctgaaaaagagaaaaaactttctgccgtggtcaacctgcttaatcaggcactaggcgatcgctatgatctctacatcgacttaccacgtgaggagcgtatccgcgcattaaatgcagaacttgcccccattaccgaaaatatcactcacgccttccctggcatcggtgctggttattacaacaaaatgctggatgcgataatcacctacgcgccttcagcgctatatcagaataatgtcggcgttaccattgccgcagatcaccctggtcgcgaagtgatgcgtacaaatacccctttagtttattcaggcaggcaggtgcgcggcgatattttgaattcaatgctccccattgagcgtaatggtgaaatcctcggctatatctgggccaatgaattaaccgaagatattcgccgccaggcctggaaaatggatgtgaggattatcattgtgctcaccgctggtttgctgataagcctgctgttgattgtccttttctcccgtcgcctgagcgccaatattgatatcatcaccgatggcctctcgactctggcacaaaatattcccactcgattaccacaattgcccggtgaaatggggcaaatcagtcagagtgttaataacctcgcccaggcactgcgtgaaacgcggacacttaacgatctgattattgaaaacgctgccgatggcgtcattgccattgaccgccagggtgatgtaaccaccatgaacccagcagcagaagttatcactggctatcaacgccatgaactggtagggcagccttactccatgttgttcgacaatactcagttctacagtccagtactggatacgctggaacatggcaccgaacatgtggcgctggagatcagttttccaggtcgtgaccgcaccattgaactcagtgtcactaccagtcgtattcataacacgcacggtgaaatgataggtgctttggtgattttctctgatttaactgcccgcaaagaaacccagcgccgcatggcgcaagcagaacgcctcgccacactgggtgagctgatggctggcgtcgcgcatgaagtacgtaatccgttaacggctattcgtggttatgtacagatcttgcgccaacaaaccagtgacccaatacatcaggaatatctgtccgtagtactcaaagaaatcgattcaattaacaaagttattcagcaattgctcgaattttcacgtccacgccacagtcaatggcaacaagtcagcctcaatgcattggttgaagaaactctggtactggtacaaaccgccggcgtacaagcgcgggtcgacttcataagcgaactggataatgaattaagcccgattaacgccgatcgtgaactgctcaaacaggtactactgaatatcctgatcaatgccgtccaggctatcagcgcacgagggaaaattcgcattcaaacctggcaatacagcgactcacaacaggccatttcgatagaggacaacggctgtggcattgatctctcgctgcaaaaaaagatcttcgatccctttttcaccacc
